European Patent Application EP 4 640 059 A1, published October 29, 2025. Title: ISOLATED BACTERIOPHAGE AGAINST XYLELLA FASTIDIOSA. Applicant: BIOLINE AGROSCIENCES FRANCE. The sequence listing filed with the application follows.

SEQUENCE LISTING (46 sequences)

SEQ ID NO: 1 - DNA, 44415 bp, unidentified
  source 1..44415: mol_type = genomic DNA
cgtccggtcccaccagcgtgagcatgcccttctgctctccggtcttctcgtccgtcgtgatgtagtacgtggacaagtccttgtggatgtcgtcgcgtctggcaagcgccttggtgaacggcaggttgcggtagcccagcgcctcgatcacgtcggcagcggtggagtacacgccgggatcgctcttgctttcccatgcagcatcaggctcggtgtagccagggaactcgaacagcatgtcctcgttgcggaacttctgcttggtcaagtcatcgaccttcaccttcttggtcttgtactctcccttgttcttgccgctgccgtacgtggtgtagcgccagaggttgtcgaagtcctcggccggtggcgtcgccgtcgtggtaccatcgaccagcacgtagtgcacctcgtccttctgcacgtaagtcggcccaccctcggtggacatgatcggaaccttggccgtgtacttcaccttgccgccgaagatcagcgcgctcttgtggaagcggctgttccagttgaaggtcaggccctcgggcagctcggggatgaagccgttgagttcggcggtcgccgttgcaagctcgacctccaactccttcgccttcgtaagcgcccagtccttgtccacgtacatgccgttgtactcggcttcgatggtgaagcacagcgcacccatgttgaggagcgccgagcgcagaccaccacgtgcacggaaggcggcgagctgtccgaggaacatcttctcggtgttaccgatgtcgcccacgtcgtcggtgtcgttggtgccgaggaggtaatccatcagcagcgtcttgtcgatgtcgcaggtgtccacgcccgcagcccacagggacttgactgcatcgtccttcaagttgccgccgtagcgtggagccgtctcgtccatgctcgccatgtggaactcttgcgtcatgccgtgcagcaggtactccgcaagctggcagtcccacaccatgccgccgccgtcgatgaactcgatccatgcctgccggttgagtgggccttggcagatggcgtgcaggatgtcgaacttgatgttgaacccgacgaggaactgctgcccgtaacacagctcacgcagccacccatcgggtgcgccgcccatgtactggttgtctatcccgactcgggtgtcgtagtacaggccggtgttccgtgcgtcacccttccgcttgtagccaatcgccacgatcttgttcatgtcgtagaacggattggccttgcgcttcaggatggaacggatcgtggtttcgaggtcgaaggaagtgaagctcacagcggccaccgttgcagggccagctggtacatttcatccgacgcatcgccatccaagtccagcccgtcgcgcacccaacgtaacacgatgatgcggtcctgcttgtccttgatgttgcggcgcttgcagatggtggtggcctcgaccgcgcgctgataccagccggagtcggcggtcaccatgacgttgaacacgccgttgcgcagcgcataccacgtggtgctgtagtcctcgtcctcctcgtagtgtccatcggcaccggagcacagggtccatccctgatcgaccagcttttcgatggcctcgtggaagtcctgcaccagcacgaggaagtcgatgtccgtgtcggtcacgggcggctcgactgtgtagctgctgccggtgcggctggacgtgatgacgcccacgttgcgcggcaggtagatgttcggttcggtactcacggtgtgttacctccgggcttggtgatccagaacgtgaagcacgggatcagattgatgcaccagcgcttgttgtgcggcgagtagtgcacgccgatccaagtgctgtgtttgttccgcagccatccccacttccactgcggcgcgtcgttgcggccttcgatgtagcctgcgtcgtgcaccttgcgcagcagcttggcaaggtggattgcttgcgcgttgctcacgcagttgaaggtcttcgcctcggtggattcaccggggaagctgaccgacaccgtgaacccggtggctacgatgtgaattggcttgctcatgctgcctcctgatagaagcgggcacgctctgcatccatcatcacttcttcccgaacgtcacgcttgccgcctgcgcggtgcagcttgttcttcggggtgccgatgtagcggaagcgttccatcgctgggtcattgagcttgccgcccatgatgatgaagtcgcacgcaccctgcttgccggtcttgctgtccttcagtgcggactgcggcgggtactggattccctcaccctcggcgctgatctgcgaagtcgccacgcccacggcgtcgtacttcacacaccagttgcgagcggcctgatacatcgcctccaacatctgatcggtacgctgcccgccgttggtcatgccaccggtgaacgtgatgttgtcgatcatgtcgaagatgatgaagccggggttggtctgcttgatgatggcctcgacttcaccggagttgaacccgtggatgtcgtagaactgcatgcggtggatgtccccgcccatcgcatcttcgatgcgcttgcggatgctaccatccttcgcccactccaccatctcagggatggtagcgccgagcagcgactgataccaccgctgcttgatgcgcttgcccggcccctcgttgttgagccagatgccggtgcgcttctggtccggccaaacgttgtcgagctgcgtgatccagtggctggactcgctggtcaggaacgtggtcttgcctgcgtcgggacgcatggcgtagatgccgaagtcaccaccacgcagagcgcgcaggttcttcgccaacgtgggcagtcggaagtggatgccgatgtcgtgctcgtccatctgcatcagttcctcgggcgtctcctgcaccagcgggagccgcgccttgcgatccattcggtcggtgatcgtctcggccaagccgtacagctcgtcgcgcaggctgaactcagcgccgccattccactgcacgatcttgctgaccgcagtggtggcaagctccaactccaacagcttctcgatcatgccctgctctgcctcgggcgggaccggctcgcgcatctgcttcagcagaactttgagcagggacttcttgtcgtcgggctgcgtcttccacttgaactccatggcccagccatcgaacacatcgaacggcaagtccttcgtgtccgggaactccttgtagtacgcacgcaacgcatcgagcatcagcacggtcagctcgtccagcccatcacgtggtgcgctgggtaccagccggtcgaacttgccacggttggtgcacaaccgcagcagcgtggtgtcaagactcatcaggttctccttcgggttcgtacttggaatcgagctggtgataccgggtgttgcgcgtctcgaacttgcgcccgccgtccgccacatacagcaccgtcgaggtgtgcacgatgtcgcagtcgccgaggttcggatgcgcaagcacgccgccgagcgtggcacggaagccaacgacgggcgggatgatagcgcgccggtagcgcacgatgggtttgctcattgcagcttctccttgatgtagtcggtcgtgtaatacttcgggtcacgtggtgacgtgatgttcctgtagtccagaccaaacgcacgtagacgcgcagcgattactcgcgcactgtcttggccgggattgctaccgttgcttctacctctgtcgtcatcgagccacgtcgctacacgttggcctcgatcagtcagctgcttcaacactttgttgtgcagcttggtgccgagcaacgaccacgcttcggttaccagtcccaccttgtatgcactgagcgggtcttcgcacagtacgatggtgtcacctgtgcccacgccgtagcgtgcgacaagtccgtctttcggaacgtcaggtgttagccacttcggctgtctcgttgccgaccgggctgtccagtataccacgttgtcgccttcagtgatcggtagtaccacccgcccgatgcttgggcaccagtacagccgcagcttctcgatcatctgaagcgagagtcccatcttgaagaaccacaccttagcgtcgagcggccactcgcgggtgtcgtatacccgtggctctggcaactcaacagtcgcacgcactctgcgttcgctcgtctgctcggcgtggattcgtgcaagcttggcctcgatactctcgtgctcacgcttgaatcctgtgccaccgcacctgaaacagaatgcggtggacttgtcgtgctctcgtgagataagcaagggcgtaccctccccgcactcatgggccacacgtgtgcggccaccaacaggcaggcgctcggcatgtggtagccagtcgttgtcgggaagggtatcgctcatgctatcctcgcttggttattcccagacctcgaagatgtcgtggctggtggcgtacaggacggagccgttgccgtccgtgctgacgatcagacgggagccgtcttcactggtcagcttggacacgacgaacccggtgcccttcggcagcttgttggtctgccgcgtgtcgatcaggtacgcattctggccgggcttcagctcgtcgccacgcttgacgacggccacgctgggtgacggcggggcgaggctcacgactgcccgccttcgccacccgcagccttggcggcagcggcttcggcggcgaggcgctgggcctcggcaacggcggcgtcgatttcttcctgcgccttcagcacttcctcggccgacatcagcagggcgctgctgtcgatcaggttcagctcggcatccagaccttcgccggtctgcaccttcagttgcagcacgcccttgtcgttcttgccggtggcgacgatcacgccggacaggacgcgcttgttcagggcacgaccgaacaggtaggacacggcgtcgcccgccttcagcgcttcgatggcggcgctgttggcctcgacggcatccagcttggcgagcttctcgttcaggccatcgaccttggcctgcgccttggcgatgtcttccagcagctcggcgcgcttggcttcgtagtggctgacggtggtctgctcggtggtgttttcgttcgacatgtagatggttcctcttgacggttgataggatggcccgtacgtgggccagtcgtagcctacccggctcgggttactgaaagatcagctcgctgttgtacccaccgccgccattgtagaagcggcgacgcagcacgctctcctcacccagcaccagcagacggtccacgatggcgcggatggcgctcatgtactggtccaccagctcgctgtgcaagttcaggtcgaagcggatcacggtcaccgcctcgtcgtccagtgcgccggtgtccttgcggacgtacaggccacggccattggtcatggtcgcaccgccgatcagcttcacggcggcggcaatctccggctgcacgttgagcagtcggctgtcgggcacagtcacctcgacccagcttcccatgcgcaggctcatgctgcacctgccagtgcggactgcacgttgggctgcaacgatgcaccggaacgcagctcggcagcacgacgcttcatgcgggagcgcagcttgcgacgctgcttgttgttcccgccgaggctatcggccacgcgcttcagctggttgttgccgacgatgcgggtctgaccctgccccttctgcacggggaagtagtcctgccccagcatcttgcgcaggatcgggttgtcgatgggaatcagcggcacgctgacgtgcaggtgccggctggtgtccggcgcaggcggcggcgtgtcgtcgtcatcgtggcgcggcttcaccgctgcgaccaccttgtccttgacgtacttggccgcagccttgatcttgtccatgaaacccatggttacttcctcctcgttccgaagtgattgaactccaactcatgccacacgtagtacgtggtgccgagcgggtcagtgtctgccttccagttgcgctggtcgcagtagtcgttggctgcgccgaggtcatcgaacgtcagcgagaacccagtggaagccgggccggtgcggaaccggcacagcttgccgtcgtcgtcatggtactggccgacgacaacccacgggccacgacccacgatccagtacagcaggatcaggatgcgcagccagagcttacgcatagtacggctcgacacggtagcccatgttctcgccgcccagcgactcggcattgaacacggcgcgcgctgcatcgcgggtcgggaacagcacgttgtactcgctcttgttgtactcgttgccgtcgatgcgcacggtggcgctcgggtgctggttgtagcagctgacatcggagtcgctgcggtcttcggcgaaggcgtaggtgatacgccaacccagcggcttgcgcaccggcttgcggatgctctcgcccacttcgaggatgtgccagttgaagaacgacccgccgtagctgttgagcacatccgcctcggcacgcacggcggcgcggcggtcgaagatggcgagctggttcgggtacgtgccgtcacgcagcgagtccagcaggctggtggtggcacccttggtgcgcagctcggcgatcaccgcatccagttcctcttgggtcggggtgcggccggtgccattggcgacgacgccagtgatgacgccatcgttgctgttcttggggatcgagacgatgaagtataccttacgcatggtggttctcctgattgacgggtgggatttcgatttcctctatcgagtagagggtgggcaccttctcgtggtgcttgcggtggtgttcgatggcttgctcgcacgcctcgtggctggtgtgatgtccgccgaggatgtaatccccgacagccacacccttcacggtaacgagcggcagcgccttcaccacaaggcgcaggctgacctcacgcataccagcgctccacgctgtgctcatgggtcacgaactctttccactggcgcggctgctcgcacagctggatcggcttgcgctccccactacggatgcgcttgtaagttacggggatcatgcaatgtgccctcctgttgggcgtggttccaaagctacgccctcgttagaaggcgcagcggtagatcacgcgcggctcgggtgccacttcacgcggtagcggcggagacggttcggatcgttgccgacgtgcgaggcgatggcgttgcgtgcagcctgcgcagtggtgaacgtgccgctgagtccgatcacagtggacgtattccaacccagctggtgagggcgccgcgcatgcttggtgaagaactcggcggtgtagaagccgcgatccttctccgggccatcgggagtgccttcgggcaccacacggtacgcatcctcgctgatgccctgcaccttggcccgcgccttcagcatgcggtacgcagcattgcggctgcgctgcggcaggcccagctcacgcacctgcgcccagttggcgagggcgatgctgccgtggcgcagattgaactgcacgatccagcccttggtcttcgtcttgttgaccagcccggtctgcgatgcagtcagggcgacgtggcgtgcgctctggtcgtccatcaggacatccggcagcttacgcggcaggttgtcgggcattgccaggccgggcaacaccatgcggccggtcacgctgccgaggaagtccagctgcgaggcatccaacaccaccggaggcaacggagacagcaggcacgccatcacccgcgcctcgatagcagcgaagtcaagttcacgcatgccgtagcccacggtgaacgtcggcggtgcgatcaggtcgcgcagcagctgtgcctcgacatcgctgtcacggcaggccgcaatcacgtcgtcctcgaattgcaggatggcgtcacgctcgaagctctcgacaccgaagtcgcgcagctcaccgtgcagcacggcgaactcattggacagcttgcggttggagtacgggtctgcctttgcggtcagtgcacaggcgatgtgaagggccgagcgcagcagggatgcttcgcgctgggtcactcgaaggttgatcttgggttccatgttacacgttctccttcttcttggtgggcttcggcacagcgcgggcagcgttgatgacggcctgttcctcctcggtcggcacgtagccttcctcggtcgccttttccagacggcccagcagcttgtgcaggtcggcggcgaacgagaacgcctctgcgggcttctcggtcttgaagtcgtaccacgccttcgcggcggcacgttccagcacgtcggccagagcttcgccctcgactcgcttgctcttggcaaacttcatgggcgcgctcgccttggtttccttgtcgtcgttcggagccatcgggccgaactcggacaggtacaggcgcagggcttcatgcttcatgccgttgcccacggcgagacacagatcggaagcgagcgtaacgtcgccgtggatgtgtgcgtggttgatgaccgcaatcgcggcctgctgaatctggtccaccagcttggtgcgggcggtgttgatcgacttgatggcgcgcttgatgtcagcgcttccggtgatgatgtccatggtggttcccttcaggttgggtccgtgccgattgcacgacactaggccctcttgcgaaggcccagtagcttgcatttaagcgagtcggatgtcgaatgaacgcccaccgcacggcaggacgtagagcgccgacacagagccggccggatgcttcatgatggcccgattgtaggaatcgcgggcagcttccacgtagtggcgagagaacttgaaccggatcacaggtaagccctcctgtcagcggcgtggttcgcccggttcgtcccgctgttaccctcgacaacaaacacagatcgctttccggcggttccgtggcgggcttcgtagcgctcggcttggcgcttgcgctcggcaagcttgcggtcatgctccgtggtgcgcaggtccatcacgcttgccgtccgggtgaactggcagaagcggcgcttacgctgggtgcggtcgagattggcattgatcgagccttgcatgttgtgcctccattggcactggtgggaaaactaacagattgatgcgccctcagaaagccgtcgagtcggtcaatccctcattctcgattagagccgttgcatcgcctatcgtgggcgcacactgaccaccggatttgcctgcatggtcatcgcaaagggagggcgcatcaatctgctagcccttcgggctgtcaaccctactccggctagcagtgccattgtcaccgtgtggcccgtagagccttttcacgaaacgcacagtattccatgcgataggaggctcaccacctccttatgaccggcttcccaccttggcagtgggttacttcccgtggccgactctcacggcagatgggaagccctaagcgttaggcttaggtaaagcggcaccagtgttgcaagtctggtggattctatgggcctttgaaatcccagttcatccggttatccgctagtgctacgttgcagcttggcggtccacgtcaactctcggccactattggctgtggttggcacgcttcccgttacaccctacccgttagcggtagtcctacgccatccaatgtggctgctcctcagagcgtggtgccatactagcacccttgttgcatcctgtcaagcccttggctcgctcgggtctctaacccgttgggcgtcctgtcgccaccatcccaccatgtacgtcggtggtccacgtgttgcaaggcctcaaagggctatctgtgccgccttgtcaagctatccgttagaggaccatgtgcgctcctgttagtgtcttgaccggtgtcccggtctcacctcagcctcaacacccgtaatctctcacgtctagccttaccgctaggtcgctccgctgttccggtggctaccacttgccgcctatcatagctaactgctagcttagtgtcaagcgtggttcggtagctcctcgcatcccttaccagtgactcccgtgtacccttagcccacttgttggcggcgccactacggatcacgtcactcgacttgcgttgcagcttactaccattgcggccgtgtgtctactactgcttgcatcgcaagcgtcaaccgttggcctagcgggtagctaactaatcagctcgacagagtaccgatagacggtgattcaggttgagccgactgtgtgctataggtgtaccaaaaggccgaaacgatacagatggccctcgcacgcctacagctgcggttcgcatggtagcaggtagggtagcccctgtcaagccccttgcggccctcctgaagccctgtcgctgccccagtgacgccattgaaccacaccgcaccggccacgtcaacacctttcgccaagagatttattaacgattcagccaaggcagcgcggtccagccatacaggcagcaggcgcacgcccacccgcacgcccacccgcaggcacccacgcacggccacgcacacgcacgctcaggcccacgcaggcaggcacacgggtacacccacgcggaaccttgacgcgggcgcacagacgcgcacacaggcgcacacgcgggcacgcacccacgcacacccgcaggcgcgtaacgcgagggcgtacgggggcacgcgcgggagcttctattggagtgacccccgcgcatttccgaagcaaattttggtccggctacccacgtggccttactcctaagcctcgcgaactggtgcctttagcttgacgataggcccggagctgtagacatcgtgagctatcgcagcagccatggccttagccacagacttgctcgcatgataggcccctagagctagcgccttgccactgccatcgaagtacggagcctcctcgacccactgctgcttaccagtagtgaccgtgagtacgccgtccttaaccacaagcaccgtcgcggacttgccaacgtgctcctcgtagccttcgcccgctttaagcgcagcgagaaccgggcgaagcactgtgaaatccccggtgacacccagcagcacagggccggtgggtgtcgatacgggcatgatcttacgcacggtgtgcttgtggtcgccctgcgtggcctgactatcggcccacaggtgcttgccgtcccatgcgatggtggtcatttgtcacccgtacaccggcgcttaccggtaccgcacacctcggccttccacgcacgcagcgcagccttgtccttgttgcacagaacggtgtccatgcggcggtcctgcgcgagcttgaccaccttgtcctgcgaggaggtggtgcccttctccccaccgaggtaggtgatgtggcagtctgcaagcagggagtcgtcagggaccggcaggttcgcgcaggaggtcagcgacatcagcaggaacagtgccatcccggtactccggggcagcgtcaagaacttcttcagtgcgaacacgcacgtcctccttctctttgatgtaggtcgcgtacccggtagcctgcgtctgcgccgccttggcggtagcggtcgtgccgacttgggcagtttccagcttctccaccttgcgttgcaggccgtagacgtacagaccgaagcacacgaacatggtcacgaccagcagcaagccaaccagcttgccgccgagccgcgcgatcacttcacttggggtttccacggttggatcacctcgttgttggggcgcaagcacagagcaaactctgcgtcgcggcgcttggggatgccggagcaacggctgctggacagtcggcagtcgagcttaccgacgtagacccagcgcaggaactccttgcagctaccttcacgatcccctgcgttcgctttgcgcagcatggtgctgtcggcgaacgccttctcacctacgttgaacacgaagtctgtgtaggcgtcgatctggttgcggttaacgggggccttcaggtgcttgcgcacgccctgctgggcgatctgtaggtcttcgatcagccacttgtcgcactgtgccttcgttgccgtcatgcccatcgctacgcccttggtgtggccgtagcagatggtcggcacccggccggtgtcgaggtacgcagcgtagcgtaccccttcgtggccttgggtgaatgacagcagcgttgccgaaatgccgatgaagatgccgccgatcaggccgaacagccccttgttgctggtatcttggttctgctgctggttcatggttgctccttacggggtcagtgggtcgtcatccgggtccagatcgaccggagtgtgcgggccggagttcggacccgaggacgcggtgcgtgcgcccgcagcgatcagggcgtccagcacgagggtggcgtccttctggaactgcgcgagcagctgcgctgcggttgcgggatgctgctctgcgtgctccatgagggcgagcagttcgcggtgcaggtagttgccacggccgaacagacccgtgtagttgctggtgaagtcggacttctgcattggttacctccggtaacggtcgagtagggatggacggccacgttgcagcggactcttgcgggtcgctgccttcatgccggtcggatcgttgatccagtcttggaactctcgctgctgctgcttggcgatggccttgttctggtccagtgcaagctgcgcaacccagtgacgcacgctaccttccagtgcatcgagccggtcatcgtgtgcgatgctgcccttctgctgcgtgatcttcgccatctggtggaacaggctgtagacctgacgcttgccgctggtggcgtagcgctgggtgtactcgtgatccatttcaaccacggattccagcatgaccagcgagccgcgagccatgacaggttcgagagtgccgatgatacgggcttccttgttgccggtcacgaactcctcgcggatgtcgcccttgtatcccttctccgtgccgcgatcttctcgcaggacaggcaggaacaccttggcgaacgcgccgtagcccatgttcttttcgatgctgatgacgttcggcttgtacttcaccgcaatgcggcgcagttctagcaagccatcaccgtcgtagccaccgggcacagctcccacggccaacacgtacacggtggagttgaggaaggcggtcacggcgaaggccgtctcgtctccgttggcaccaccaccggccgggtcgatctgcatgtgcacgccctgcacgggggcagtctcggtgctcatgtcgtgcggcatcatcatcacgaagccgtacccactggactggaagctgcgctggtgagcgttgctcaggccacgggtgatcgtcagcgggaagcggtcgccaccaccggggatcacgatcaggttatcggtcttcagcgggaagcgcagcgcatccatcagccgcgtgttgagcatgtagttcagctgatagctggacggtccacgctgacgcagctcggactggtgcttctgctcaccggccaacagctcgtcggtgcactggccctcgtcgcccatcgggccaccaccgaacgccaacatcgggtcggcttctaggcgctgcacgatagacggtgccagatgcgggccgtagtgctcgcgctgtgccggggtcgggtagcgaccgggccagatgcgaacgtcgtagccacgtccgggcagggtgttgtagatggagtcgccggtctgcggcgtgccgaggtacaggatgcgacccggagtaccgggcttgccggtgcagatggccgagaactccaacgtgatggtcagcagcagctcacggttcgcggcagtgcggctgttcttgttggactccacgtcgtcggcgatcagcaggtccgcacgcttacccggcaggttgccggtgacgccgatgcacgccacgctcggggacttgtcgattcccttcagcgagtggtgcacgtcgaacgcatccacggaggtacggtcgcccgcgttcttgtccgggcggatgcactccaacgtcggcaccgtgaggatgatgcgctgaatcagcgtagcaatctcggatgcctgcgtgccgcctgccgatacgatcagcacacggtgagtgggatcgtggatcaggcagaagacggcgtagatggcagcgatggtggacttcgcctcgcctcgctgcgcctgcaccattgcgaggtgcgggccatactgcatgtagttggcgatgtcgtactgcatccacgtcggctcgaaccccagcaccttcataatgtcgcgcatgaaggtggcgaagtgccggtagtggttctgcaacagctccaacttcttgcggcgcacgtcggccgcttcagctgattcacgcattgttggctacgctccccggaaagtgaacgatgttgtcgagtgcacgctgcaactcgtcgtcgtcagccggaggcagcgagtgcttgcccagctcgtcttccagctcgccgagtgccttgttggcctcgcgcgtcgccgtgatgttgttgtccttcaggaacttgatcgccgcattgatgtcggctgcggtgcacagctcgccatcttggatgcgctgcatcagcgcacgcgcgaccagttcgtgcagcgcaccgagtgcgccctcacttgccggattcgacatccttgcctcccatgatctttcggtgctcgcgtgcccgccagtagaactgagcgacggcgtacagaatggcgagcgtagttacgatggcagcaccgtacgtgctgatgaagttgaggtagaccgcgccgagcgtaagcggcgaggttcggacgacctcattgaccacactcggcggggtcatgctgttctcctgtaggttagggccagtcgtcgggattgccgacgagcttccattgcaggcggttgacgttgttcatgcccaccgcaatcaggtcgccggggattcccgaggcgatcacatgttcggttgcgaagcgctcacgctgcgcgcgtacgcacaggttgctgccgttcttgtacgacaggagcacgtcgctctgcgtggcgaagacagcccgcttctcgtccatgcacaggcgcggagtggtagcaccggggatcaccatggtctgcatcgaagcagccaccgtgtcgtaccagtagaacttgcacacaccgcccgccatgtacgccacgtgcgggcgcatggtctggtcgaaggccagtgcgatctgcgtgatcccggagtcggtcagcacggtgaccggggcaacgccgtcgcggtaaacgacgacgctgctgccgtcactctcggcagtccacagcgcagcttggaggtcgtccactgctgcgttgagagtcagcccgccctgctcgaagtcaatgagcgggcgggtgcgccgattctgctgctccacccagtcaccgcgttggatgctttgggagacagtggggatcatggcgtgtaccggctccaagaaacccgcatgcgcaagttcgccgtctccgatccggtcttggtgatacccggattgaagccgacttggaaggtcacgcacgcggagagtcccattgcagccgtgatcggaccaccgggcacgttgttgatcgacatccggcaaacgcagtcacggtagtaagtacccggaacataggctacctgctgaagctgcaagtcagagaagctggcaatcgtccccggcggatactggtcggtgatagctccggtgccgtcgccagtaccgccgtagaagtagtagcacccccacacgtagtccgaccaagcgactgccgactgaccgttcataccgccgctgcggcccattgcaataggcttacaggtaacagtggtgctaacacccttgatcgtctcagtagtgacaaccggcgtggtatctgcgtacatgcgcagctcgtaagtaaccacgaggatttcatccgacagcaccgtgatggtggtcgggttacctgcggagtccttgataagcgcacgggtggtcaggatgtacgcgccggtattgttgttgtatgctttggcaccaagctccgacagaacgccagtagcggtaccagccgggaactggtactggcagcgggagtaggcgtagtacggggcagtggtagtcccaccgctgtccgaggacgtacgaccaacctgcgccacctgtgcaccaagagcggtatcggtgaatgccggggtggcgctgccactaccgactgccaagtaagcaatgaggtcgtacatgctgcgaggatagccgctgccggtatcacccagtgcgtccataccaccgtccgtgataaggttgctctgccagtcggctacaacttcgagagtatcgagggacttacccttgctgatggtgaacacgccagcaatgccgaggtgattgtggatcatgcgaagctccatgatacgaagccagaccggagtcgtgcagtcgcgtcgagcggctggttgactacagggtgctgcttcagggtgaaggaatggaaagaactcgacagcttcgccgtctccgggtcaggcgtgtagtccttacggatggatcggatgtcgaacgaaacgaaagcgctcccgtacaacgtgctctccgggtcggcggcataatcctgcctagagcttcggagttcccagcttacgaaggaggaacccagcgacgcagtatccaaaggctggagcatgtcgatgttgctgtacccagcaaagctgctggtcagcatcgcggcatcgaactggtagaagctgtagagcttggacgtaacgtagatgccctgctcctcgatacgaccggaccagtaggccacacggttcaacccgtccgtgaccttgatgctaaggaagtaggagctgtcgtcgttctgacccagtacgtacttgtggttccacttaacggtgtccacccacagcggtttgttctgcttgctgcggaacgccgacagtacaacctgcacgtacttcgtgtccttgggcgcagcgccttcggcaacggactggtgccacgcaccgttgctgccggaggaaaccatgttgccccagttgcgttgcagctcggtcccatcctccttgcggtagatgatcgacacacgagcaccggccttgcccttggagcttgcgccctgctggacctcggcggtgcatcggatgtagtcgttgaccttggcagggatcagcgggttgagcaggtcgctgccgcccgtcttgatgttggcgaagcgcgcgctgtacacgccgctgtcggtgtcgtagtctgagccagtgccaatcgaccagccttcgccattcgatccaccgcccggcaaccacgtgccgtcgtcgcctgcctcgaagtcgccgttgggcacgagggtttcctcgtccacgacttcagtgaaagccgcccacttgacgacgacttccttggtgatgttgtccacccgtaccgcagcgcccgaagggagcgtcgattcgatgacctccacggtgcagcggccgactgggttgttgatggacaggcgagactcgtaagcctcgcccgccgtgtacccttccagcacgcccgtcaccgacaggccatctgcaacctcgtccgccatgagcggtcggccgtacagcctgaagtgattagccatgcttactccttagccaagtcgcccgagagcaaccacgtgttggtgtcgccgtcgatgcacgttgcagtgatgacggagttggtgccgcgagttgcggcggtgcagccgaccgggacttcgagcgtcacgcccacgtcgccagtgatgaccacagggcctgccttctgctgcacgctgaagtagctgcccgaggcgagcttggtttcaccgtcgcccacttcggggatcaggttgatgttgacggcgcaacctccggcgtacgtgcagcgcacgagtccgtactcggtagccttggcggcgtagtaagtcggaccctctgccgtgatgatcggcacccgcaggctcgcagcggtgatcggcgcaggcccggtgtagggcttggcgtaaccacgcagcacggcgaaccagatgctgccctcggcaggaaccgtggcgaagcggatgaagctgggatcggtgccgtcagcgagcgtgacctgatagtccacgtccggctgcatgccgatgccgttgacgtacacgtcgtagaagcccgcgccggatacgtccgcgcccaccatgtcgaagtcggtgtcacccacctgatcgccagtccaagcaccggaccagacgcgcggggcgacggacacgataccaccagctgccagcaactcggtgacctgcttgtagatgttctggataatctcgttcaggtccacgatcacaccgacctgctggtcgatgctaagggtggcgatgttgagtgagtcgaacatttcctgaatgatcttcaggagctggtcgttgctgaggttaaggtttgtcttgctgatgatgctaccgttaacgtagtcaacgagcatctgctgcaccggagtgctgcggtagatgtagagcttgcgcccagcggcgacggcaggcgagactcggacggtactagcgtcatcgtcttcgctcaggacttccacggtgtgcggagtccggtcggtcagcagctgagtctcctcgtccagcagtccgctcatggcgtacacgtgggacgggttgatgtagccaccggtaaagctgatctgccagtcagtggtcacgccatcggcgtcgaacacgtctgtcgcgtagcgcagctgcgggtctggaactgccatgctgcctcctgtttgctataggtgtaccaaaagggtgggccgtccttggccctgatcttactcctccttccactggctggctgcgcccttcagcagcgggatcaccatcggcagtcgcccgcccggaatcacgtcggccagattctccggcttgccagcaatgccctgagcgaagtcgttgatgactcccagcgacggcgcgaactgcccgcccaccacttccttgcggttgccgaactgcccaccggccagctgcttcagccacgtcggaccctgcgtatcggtggcgtactcgtaccagccgcccgccacgccagtgcccacgtccagcacatcgttgagcatacccgtcgccgacacgtagttcagcgtggccttgcccagcgccagaggcgacaggatgttctggtcgatggcctcgtcgcgctcctgatcgttcatcagggccacgcgggacagcacccgcagggcttgcagcggagccgccacagccatcgcagcagcgatcaggcccgccgtctgccatgcaccgtagttgcccacgtaccggcccagctgcttctgctgcgcgaccagcgagaacgtgcggtgctggaacagcagcttcagccagccgttgtgcgcccacttgccagtctcgccgatgaaggtgtcctgaagaatctgcgaggtgccacggttgatcgcgttgtagaacgccaaccatgcctgccgatccgccagcccctcgacgttgcgcgggtctactgcttccagcttaccatccgcgccccagcgcacgacctgatcctgcgtagcccgcaggcggttcagcaggttgtcgtcaatgcccatgtccttcagggcggtgtcagcttcagcaccatcacgcaggaacttcacgcccttggcgatcagcacttccgcgaagccacgctgctgcacagcaagcacggcccgctgccccgagaggatgcggttcgcatgcgctgccttctgcaccagcgaggtcaggaagcctgcgcgctcgctaccatacatcgacgcctgcgtgtccagcgagttgaacatgtgtaggtcgtaaccggcgagaccgaagccgcgaccgctgatgaactcgaagccgtcgaggatttggttgccgctgtcctcgcccttcaggatgcgcatgatttcgctgcgcatgcggggagcgatacggattgcgtcagccacaccagcagcaccaacagcggcgaggccgttgctgtactccgctgcctgattgatgcccgcgccgcccagctggatggccgaggtcagcagacgcgcattcgccagaacagtcggatcgccggtaccgaccgggcgaccaaggaactcggacatcacctgctcgaacgccttcagctccacatcgttggcaccggtcaggcgcattgcttcgcgcgccacgttgatgcctgcgtcgccgaggatgccgtgcttcgccagagcgatgtcaccagcaacacgtcccgcgtacttgcggtagttgtccatcacgcggttgtcgagatagtccatcagacggaacttaccgtcagcgtcctcgtactgcttggtcacgtcgaggtcgatacgcgccttggtgtgcttcgcaccgccacggctgtacttgcccatgaccttctgaatctcctcctcgttgagcgacatcgcccgcagagtgtcgcgcagcgtgtccgcctgcgactccgagaagacctgacccggcgcttcgatgacacccgcagccttgcgctcgatgcgttccagatacttggtagcgaacttatcgaggaagtcgtccccatacagctcgcccatcacctcgaactgatcgcgcatcgcctgacggataccctcgcgtcgcaccggaccagcagcagcgatgctgccgcccagccacgtacgggactcgtagccctccacgtcctcctccggcagacgctgtgcgcccaccgtaccggccgcgcgctgctctgctgccatgcggttgtagccacggtccaactcacgggccattgccttcactgcctcgtgcgcatccgggatgtccccgccgttgaagcgagtctcgcggtacagcttcactgcgtactcgaagtccgcgcgagccttccagcccgtggcgaagtccttgatcgcaccgataccgcgcacgtccgcacgccacaggcgataggccgcttcccactgacgcgggcgggtgcccatgaacgactcaaaccgaccatgccgatccatcgctgcggtgctgtgtcggcctgctgcaccctcgggattctccaacagggtgatcgcaagcatgcgggcaactggcgacttggacgacattagagtcgtgctcgtagcttccagcccgaagcgctgcatgatggtggacagcttcgccgcgtcgatgccgtactgcgcactgaagcgttcggagcgtgccatcacttcggcgacctgcacacgcatcgcgtcatcactgacggacttgtccagaccggtgcgctggtagaaagccttgcgctcgcggttcgacttgaagatcgagttggcgagcatgccacgcgtctgccgggtaccggcctgcgtgtcgcgcacttccgcgccgaggttgtcaccgacgaccgacatcaggcgttcgagcgcggactcctgattcttcagacccatcactcgcgcgatcttatccttcagccactcccacgcattcgggcgggtgttgcccggcgcgggcatctgacgcagcaccgcctgcacagcgcggttcgtcaggccgtaggaaatcagctcgtcagtgttggcgaggaagcctgcctgcggctggttgatgcgcgtctccatcgcagcggtggtcagcgtggagtccacactgccgatgctgttgttgatatgggtcagcagttcttccatttcctgcccgaacaccgagttgctgcgcagctcacgcagcgtggcagcgtgcagcatttcgtgcaccaccacttccggcgtgtagttccgcatcgccatcgcgtccagtccggcgttgtagccaccggccacacgcatacccggacccatgttggcaccggcgaaccacttgtcgagttccgattccggcacgatcttcaccgtgctcagccgcccgccacgcttcagcgcgttggcgatagcacgcacgtcctccgggatagaggcgttggattccagatacttcagcacgccatcgacgttaccgcccttgatacctgcggtcttccatgcgcgttccagcagcgggtcatgctgatcgacccggccacccacgctgtcgttgtaccgcccggtcgttgcgtccacgttgcccgcgtcccgtgcgagtgcaccagtggtgcctgcggtggtggtcgtctcctgcacgtcgggacgggcgaagatacggaagtcgtcaggcacgtcggccataccagcgcgcagccaatccacagcctcctgcttggcaagctggtggatgcggttgttcaccagcaccgggttggcgtcctcgcccagctcggccacagcgcgcgccttcaggtcggccgaccacgcttcgccgtaagcggcagcgttgcctgcggacaggtcgatggttgccttgtcacgaatctgcgcagccgagcgcacgcccggaatgtgcatcgcggtgcctatggtggtagcgaatgcagcgtcggtcatgaagtccgcgaagttgcggcgctcgcccatgccaaccagcgcggcgtccgtgatgacggaaccgaccgcgttctccgcagcagccgacgcgagcgacgcgcccacgcgcccttcggcaacgagtgcagccgagccgatgcccagcgccttagcgcctgcggcagtgacgccgccgatagcccagttgcccggatcggtgaagcctgccaccatgtcgtaaccgaagctaccccagccagtctgctgatccttgatgcgcatggagtggcggcgcaggaactgtcggtcgctgacgtacttcagctcgttcggcgagtacgctgcatcgcggatgtcttcgagttcgtcggcagtcatccacggcttctcccattccttcgggtcgtacttccaaccttccggaacgttctcgtcctcgcgcgcaaactggttgctgatcgcagcaccgatgccgctgtcgaacgcagcgccccacttgtcgaggaaggtcagcgagttgcgcagctcctcgtccgcgcggtcctgcgcgagcgcctgttcggtctgatccagcagcgccttgcgagcgccggtgttcagcacgtccacttcctgacgcacccaccacggcacaacctgatccgatgcacggacagcctgagccttgcctacggcctgcgcggcggtgccaccttcctgtgctacctgacccatcgacagctcggcgatgcccgcacgaatcttgccgatgtgttccttcgctgccgacgccagagcgttgcggccttcgatgggcgcacccgtccacgcatccgggatggacgcaccggaccacgtacggtcgcgcatgttcgggttgccctgccatgcggcgttgaggtctgcctgcgtggtggtcaggctgcgcggctgcgccgacactgcgggagcggacgcaccgcccagcacgctcggtgcataggctgcgttctcctgcccccagttcttcggattggtgccgccttggtagatgcgcagcgccttcgtcacgtcgcccttggcaagctgcatgttctcgcgcatgatgtcggcatacagctcgatgctgtcttggaagttgcgcatgtcgtacttgcgaccgttgcgcgcttcccacgttgcctgcgtggtgggcatgacttggaagtcgccctgtgctcctgccttgctgcggatcacaccgtcagcgtccttggcggcacgcccgttgccggactctactcgccactgaccgcgcacgatggactccggcactcccgcataagcggcagccttggcaatctgctggtcttgggtcagccccgaaagatcgagtgccattgtctatctccttacagtttgggttggatggaaatgctctgctgaatcgtaccgtcgttcatgcgaacgtagccctgcggtaccggggcctgcaactgacgctgctgcttggtgtgcttctcgtactcgtccttgatgtcgcgcccgtacaccggcacaaccttccagcccttctcgccaacagcgttgacgtacagcaccggctcgccgttctcgctgtccttcatgcggaacacgtcagccttcagcccggtgctcggctcgatgttgacccggcgcagtgctgcgtcgatggccttctcgatggcgggtccggtttccttcgtgtccatgaagcccagccatgcaccgacgctgccgatcactcggccttcgtcgtcgcgtccgttttcccatgcgtacttgcctgcgtcttccagaccgtaggccagcttggcgtgagtagccgcagcctgcaagccttccgcagaagtgtccagcagaccaccggtgtcagtgaccgagcggacgatggcgcgagcatacgcagcgcggccagagtcgcccagcttgttgccgaacatgccgaggtacttggggttgagcttggcgatagcttccgtaacacgagcctgagtagcctcggattccttacggctgttcgcgtcgaactgcgtcggatcgtcggtggtgatttctccacgggccacctcgtaagcaagctcgaagttcacgccaccattctccaacgcttgcagcttgttgaagaacgtgttgacgctatctccgaagtacagcgcagcggtagtcgcgccagtcagtcggccctgcacgggctgaccgttcgtgtcgatgcgtgcggcggtggtctgcttcagttccttccactgctggtacagtgcagccgctgccgtgttcggctgatcgcggagcacagcgcgcgccgtggtctggaactggtcggccacacccttcagcacagcgcctcgcccggtgttggcgttccacaccagctgcgacatggcgaccttggggttcgcggccatcgtggcattccatgcctgcaccgtgttcgcctcgatcagctccttgtccacgccggggatgttgatcgtctgcgcgtacgtgccgcgcttgaacgcttcgatgccaccacggatgtcctcctcctgcgcggccagcttctgctggtcggtcagcgcggccttggccgcagcgttacgctggttgatgacggcttcctgtgcgcggatgtgcgcgcctgcggactgtgccatgatcgaagccaactgcgtaccggagtacagcggtgcgtcgcttccagtctcggcggcgtaggtcgagttcatttcctcgatcatcgcctgcgacggcttggcaccaatgccctccgatgcgtacatggagacgagcgccatcttctcggcctgctccgggttggcatcgagccagtcggaacggtaacgatcctgcgcctgcttcacgtactgctggattcccagctgcccgtccgggtcgatggcgttcagaacgcccttgctgttgaggaacttcagcgtgtggaactcgccgcgatccgcagcgccacgatagaacgcagtgatcgcggacttgtacgactcgtccgtctggtagcgcgagggcgacagtccgtccagcagggacagctgcgcctgcgtcagcgcctcggtggccttctcgtccatgggacggttggtaccgagcatcgccgtgcgcttcgccagttcgttgaagccggtggacgccgacgagttcgcagcgtactgcgccttcaccagctcctgctgctgccatgccgtgcgctccttggtgtgcaggtccatgagggaacccgcgcgatccatgaaggtcttctgcaacaccgtgtccgcgaaaccgttgccggtcatgcgggcagtggcgaggtcgttgaactccttcgccatcgcctcgggaggaagctgacgcaactccggcatacgccgaagcaagtcgctctccatttcgttgacctgcgagagcgtgttatacatgctcgcgccaatctcgtagttggtgtctccgaagattttcttgtaccacggttcggtcgcagcaatctcgtccatggtcttaccagcgcgggcggcaacgaagccgtcccacatctgctgctgcttcagcttggcggtgttcggcgctgccagctcctgcaagaactctggcaggttgctgtccggcatcgtcataccaccagtgcttgcgaaccagtcgttgccggattgaaccggcccgacctgattcacaccagcgccttgaatgctggtgttgcccgacagtgctggggtggcgttgatgccaccctgcaatgcggactgcgtgttgaaggtaaccgtgccgatgtcagccattaccatgcacctcctgagttgcctccgctgccgctatcgaaccagccgaggccggacgtagtggtggagaagttgtcgtagttgttgccgaagttgccggtgaccttcgccccagtcacggactgcttgccggtgccgtcgttgtacccgaaggtagtggacgcccacgacttgccgccgcgatcattggactgctgccacgcctgcataccgttctgcgctgcgttgctgaaggactgagaggcaccagtgaagttgccgttgtccgcctgccacgtgccgaccgcgaagtctgccacggcctcgcctgccatcggcccaccgaagtaggtagccacggccacgccgatcagcttgcccaagcgacgcttcattgcctgcggctcgatgtgctgcgagtagtcgaactgcccgaacgaacggctcatgtccatcccgttccacgcgcgcgacatgatctgcgcagtctgcgatgcgccccgcgaggcgaggagcgagacagcgttggcctgcgtctcctgatccatttccgcctgcaaccgcaccatcgaatccatcaggtctgcggacgagccgccgacaccgacagcaccagcctgcgcctgaagtgcgccacgcgcgttcgccagttggagctgggagttaagcccagccccttggcgcgcacgcagctcctcggacagcgcttccatgttggagttgtactccttcgcggcggcgtccagttgggcgttgttcttcagggaccgcatgaaatcagcgaagccggtcttggcgacctcgctgcggttctggttgtcggtctgcgcaacggctgcacggtagttcgcacgggcaacgcgggtggtgttgttcgcttgcaggatcgtattaaccgaacccattagctaaccctccgtacattgttgaaagtctgacccgtccagctcaggccggtcacccggagcgggagccaatccttgctgcgaatctcgtaggtgcactcgcgcacttcgcgcccgacgctgatgttgagctgcccccggtacaccggttgccgcgcgatcagattgtcggagtcgccgaggatgcggccctcgaagtccgtagtggtcacattgctgttgcgggttgccaccgtggcgatcatgcctgccgtgttctccacgtccaccgtcaccttgttgagggacatgcgtccatcgagtacggcctgaccgttctggtcccgagggaacggattggtcgggatcaccagagcttcggacaccacgccgtattccagcgcaccagcagcgaggtcatcgaactggttaaggaagtcagacgcctgcgcgtagggacaacccagcaggaagtacgggctagtgctattgacggcgatgcttgcgctcgcagtctgtacgcccgtaggtgtaccaaaactcgcccagctgtcgaggcacgcatgcgagtccggctcgcccttcgggtcgaacacgtcgcacgccaccagcgacccgcgcgcagtgaacacgaggccgttcttcttgtagctgctcacgccgatgatttcgcccagcgccgggtggtaccggaacttcgaccacgcatccacgatgcgctgcccgttgttcttgttgtcctcgtaccggtacaggtagaagtcctgcgggtgctcgcgagtgcggaacatgacgaggttcggcgcagtgagcggggtgatctgcaacggagtgcccgacagccacgagtccagctcgttggacatttcgtccgtcaccgtctgctgcccgttgagcgcgcccactcgcatctggtgcaggctcgtgccttcgctgccgtactgcgcataaaagatgtagttgcccgaggtctgcgccttcgcgtcaaccgaatccttgttggcactgaacgctttaatcagcggattcttcggactgaacaccgagtcgccgctgatgccgtactgctgacggtcaccgaagatcacgaggttgccgttgtagagcgtcgcgtgccggagcacatcgccctcgctgccgtgcgcgaagatttcgatggggtcgctgtcttcgatggtgacggccgagccgcgccagaagttcaggtagtccgccgagcgtgaggcgttgacgtagttctgtgcgccgatgaccagccggtcttggaagacggacagcatcgtgatcggcttgtcgatgaaccacgggatcggcgaggtcagaccatcgcctgccactcgcgcaccgtaggccggatgctcgccgctgctcggagccagagacgtgaggcccgcaccgttgcgtgcgatgtagcctacaccgttgtagatgtagagctgcgacacgaggttgtcgatggtgcactccacgccgggcgcttcgtaccagtccaccgacccgtagccggaagtctcgccgttctccaactcagcgcgcaggtagtacgactcgtccgcgcctgcaccactcggccgcacgcgaatgaccttgccgtgccagtggaacttgacggcgtaggtcgcgtctgtaatttcctgccctgcggcgtagaaggtcgtgccgtctccctcgtcgtcaaccgtgatgtccttgaactggtcatcgtcaatgatgatcccgcccttgatgtacgttgccgacacgcctgcatcgaccagcaaatccgacagctgctccgcgatgtactccgggcgcgtctgctcagcgctcgtcacgatccactcgttgaccgcagagttgtactcgttcactcggtcgttgacgtacttctggtacgccgcgtccggctccgtgccaccgggaaggtagaacgggatgtcgctggtgtcgagcgttccggggtacgatgcggtaaccgtcttgaacgttaccgtcagcaccgtgttgtccgtccgcgtcaggttcaccgtgtacgtggtgttgtacttcccggtgcgcacccatgctgcgaggcgctggatgttcgtctgctcctgccacacgttcgtgctggtggccgaggggatcgtggtgttgcccgcgatgtagacgtagctgccgatggccgtgagcgacgatgcgcctccgctgaccagcgtgttgacccacgtgctgttctcgtacaccagagggatgaacgactcgtccgtcttgttgtagaggaacgcgaaggactcgctgcccaaggtcgaggcgtcgcgccggtacagcagcgcgtactccttgccctcctgcatgaagtcgaacacgtccatgttgcgcagctcggccgaggtgacaacggcttgggaagcagcgaaccgcgtaccacgacggcgcacgaggccgttcaccggatcggacagcacgttgatctgctcgtgcgtctgtcccggccgacgacgatgcgccggtttctgactgacaccctgaaggatgtcgggataggttccgcctgcctttgccatgttgtctccttagccggggaatgtgacgtggctgtgccacgggtgaccgctgtagttccagtaacgggaacgcagcacgtccacggatgcgcgagcgaacagcgggttcgccttgatctggcggatgtgctcggccttcaagttgatgtaactgtcatcgcgctgctgcttgatcttggcgtacttggtgttgtcgccgtcgaagtcagactggaaccgcagcaccgagtcgtcgcgcacgaacatctgcacctcgtaggggaggtcatcgaagtccagcagccgcaccagcttggcctgcacgttgtggtcgaactcgtaggtgttgcgcttgcggtcgtacagtcggcgtccgcgctgcaccacgtggccgaaccggctcgggttgcagtccagcttcagcacgtccgtggggaccatgatgtacttgctcgttgcctgcggcttcagctccacccattcggtgttgaaccacagcgagagtgaggacacgtcacggtgcacgcggtcgatcaagtcaacggcgtcgtccttgtatacgtggtcatcttccagcgtgttgagcttcgtctcgcccatcgtcttcaagcaggcgttcacgatgtcgagcttggtgatgaatgccatggtgtctcctgagaggaacaaggcagagacgccggagcgcccctgccgggatgttgcttagtccgcagccagagccagagcggccggtgcgtactcgatgtcctgcgagccgatttcgtcgtccacgaaacggacacggacgacccagcctgcggtgccacgggtgtcgtagtggacgccgacgacggtaccaacggagttggcgggcagaccggccacgccagttgcggcgacgacgcggttggaaatctcgaacggtcggtcaaagaccatgatgttgctcctgtgttggtggaagaagggcgcggtttgagttacccgaaggattcagggaccgcgcccagcggattaggcaaccttgtcgatgcggcccgcgttctcgacgcgatccagaccaacggcgaaggacatccacgagtccacgaagtagcacttcgaggcatcgctccaccacaccgaggactgcaacggcagcgcttcggcgatcagcagggccttcggcgacacggccacggcgatcagggtgctgaagtcgccgtcgtagaagtcgtcgttgtcgtcgttcgacagcaggtgaccttcgatcacggtgttcggcaggttctcgctcgacagcaccgggacgccccagccgtggaaggtcgggatgccggtcagcttgttgccgtccgaggtcaggtactcgccgttgctgatctgctcggcctgctgcaacaggtagaagatcgccgggcgcacgatcaggaccacgccatcgcgctgcggcttgaccttcttctcctcctccatgcgggagaacagtttgccgatggcggcgtacaccttggccggatcgttctcgtcaccagcggcggacagcacgacctgcgtggcaccgaagtggccctcgggcgcgcggccgttgcgggtgaagatcgactgcgtggcagcagcggccttcgcggcggcgatgctgatggtcaggtccacgaactcggcgatttcctgaccctgctcgatggcgatttccttgcgggtgtcgatgtcggtgaagatttcgtccagctgccagatgctgtgacgcgacagcagcatggtatcgacggtcaccgacgccttgctgaagtccaccggggtgccgtccggcgcgtcaccgcgcttcagcttctgaagcttggtacggccgatggccttcttggtcagggtgttggtgcccttgacctgcttgcgcgggaagaacttttccagcaccgagctggacacgtaggtgtgctcgacatcgccggtgaactgttcgaggatcagggcgttctcgttgccggactggttgacctgattcggcagaaccgggacagtcgggaagatggtgctcatgctttgtgttgctccttggtcttagtggatgacgcgcgcgttgagtgcacgcagttcttcggagtgggccgcaccacggatgcccttctcggcaaccagcttgcggtactcagcgcggtactgctccttcgtgataggagcgacgccgttgatcgacgcggcgggggcggcggcgttggtagccggtgcgcccttgacggtcgtcgcgggattggcctgtgccagagccatcaggtaacgcgcggtcgcctgagcgccgaagccaccagccgacagcgattcgcttgcctgcttcagttggtcggcgggcaggttggcccgtgcgaactgctggatcgcagcccagttctctgcgccacccacggcttcgtggacagcagcaacgttcgcggcgtgcgctgcggttgcagcggcggtgacacgagcgatgctctccttcgccagagcgaggatcggtgcggaacccttggccttgtcgccgaggacttccagcttggcttccagcagggcgaagttgcccttcgctgcttcggtcagttcgcggctgtcgatgtcgaggcccacggtgttgacgaagtattcggccgcgatgttcaggccgttgtcgccgtagtccgggatcgacaccgcagtcggcgcagcgttcgccggggcggcgggctgtgcgggagcggcaggttcgagactcagcgcgtcagcagccggaggtgcagcaggagctgcgggctgtgccggtgcggccggagcgggctggccgttgggcaacagcttgtcgtctgcgggagccggagctgccggtgcgggctggttgccgttcgaggttgcgatcacggttgcgccgggaccaccgcccggaggtgcgttggaactcattgtgtctgtgtctccatgttgttggcgttgtcgatctgctgggatgcgttctgcatggcgagctgctgctgtgcacgctgctgcatcatctggccgtactcggcctcagtcagcacgtagacgttcgggtccaagccaccagcggcggcgaggtctgcgatccacgcggacagcttcagtcgttcgagaatctgcggcggcagtgcgaggacgttggcgaggttgctgccgaactccaacagccggtcacggtcacccgtacgggagagcgcggccaagccggtgatgatgacaggctccaagtccttgcctcggatgtcgcggcccgtcaggttcatcacccaaaaggcgactggtacctgcacgtccgcagcgatccgggagtagccgccacccagcccgccttccagttcttcggcgaccatgcggatttcctgcgcggtcacacgttccgcctgacgagtcaccgccgtctgcaacaggaagcctgcgccgatgcggttgatgtaggtggactggattgcttggttggtttgcagcacgccatcgacgcctgcgttaatcagctcgatgtcacccttcatgccgggaatggccgcgccattgggcgacgccatgaagtcctcgacggaggtctgacctgcggggttaaccagccaccggaactcggaggcgaggatcgcgccctgcactgcggcctcggacagcatcgagagcgactggaagtcggcctcgtagtcttcgaccaagccggagccgtagtcatcgcctgcggccaagtcccagctaaccgcccggtagggcagcttgtctgcggtgtaggtcgaggagaagttggcgggcagcttgcagttgcaaatccacacgtcttcgttgtacttgccggtcttgtggtccagcttgacccacttgtactcccacaccatgccgtcgtcatcgggcttgaagtccgggtgcgcgacaatggcagcgagcgctgcgggttccagctgggtcttgtgcaccttctcccgaaggatcagttcgtagacctcgccggtgcgggtgcgcttgaccacgtagtgccgcatgttgagcacgcggatcgtgtccttctccaacaccatgagggcgttgcccagcacgatcagcatcttcagcaggtcgtacagccgggagcggatggagcgcttgtccagttcgagactggcatcctgctcggccttcgcaagcatcgcctgcatggcctgcaagtcagcgccttgctcctgcgcagcctgcttcgccttgcgcttcagctccaaccggaagaacgggcgggacggtgcgaacagcgacatcatcagcttgttcgccagatggttcactgcctgcgcgccgagagactggaacccgtgggtcagcggctcggtgtcctgatcgcggttcttgcgagggaacagcttgggcacggtccagctcgaatagcgttcgagtcggtacatgatgccctgtcgcttgttgtcgtaagcctcgaactggcggtgagcggtttggatcggatggtccatgctcacctcacaacaggtctgacccggccacggtcgtcagccgggaagctgcggtcgtggtcacgggtcgggtgtaagtggagcgggcggtcttgcgtcggccgatcaggtcggcagtctgcaagtcgaggtcggaagttcccagccgcacatcgacggtatcgacgggggcactcagcaacttctcggcgtactcagatgcggcctgctgtgcagctgcctgtgccatctgatcggccatcgcctgaatctggtagttcgtggattgagtttggaggttggtctgcttgtcgatagcagcagcttgcttcagcgctgctcgcttggcggacccaccaccaacgatgctacccataggttaactccttcgcttggtgaattggggagcatgccgttccagcaggtagccgtagcgtgcatacatccgtgtgagtgctcgggagttccgagctagtgcaccgcctgcgctcagtgagtcgcagtggttgatgtcagccagatgttccatcacggctatgtaccggtcgaaggaactgcccggcccaattcgcagcaccatgttctcaacgaacgtagtacggttcttggagtaccacggtgtgacaatggcaaagcacagcaggtaggcttcatcaatgattactgcatccactagaccctgtgttatcagggccactgtgtaatcagggtcatcacagttgtagctcacagaagattctctgttgtctaccttactatcttctctagatgacagatacaaagcggccgttaaagccgccttgatctgctcactatcacccgtcgttggtgttcggtacggaggaatcaacggtgaaaccctcctgtaagatgttcaggacgcgggccatccccaactgcatacctgcctccaagggcgtggtattcgagttgacggacagcgacagcccggacagcttccgcacggcggccagctggttcgggtggagcgtcatcaggactttcactttggcgtcttcggccatggtgtctcctctgtgctataggtgtaccaaaaggtccggcaccggttccgcttaccttcgcggccgctccaaccggacctcagttgcctcgtgctataggtgtactgaaactccgtcagctgaagaagtacggagaatcaaggacttgccgaaggtccagctcgcccatcggcggcggctccggcaggaacgggtaggccgagtggaaggccgacagcacgtcgtgccgctcgtacatcgacacgaacacctcccggatgatccggtacagtgccgcgctgtcggcggcgtgggtgccgaagtcgtcgtgaatcatggcgaaggcgtcgatgccttcggccttggccgcgttgaccaccagcgtcaggtggcttgcgtcgaggctgtgcacgaagttcggggcgatgccgttgcggtgccgggacttcttcaccgcgtccgtgctcttgcgcagggacagcttggcgttgccgcacagcttggtgttgatgcggtgctcctcggactcccagtagacctgcaccaccgggaacccggacggcgtgatccaccggatgcggtcgtacccttggttgaggatcgacccggagccgcgctgcaaccactccatcgcgcccgctgcggcgaccacggtgtcggcgatggcctcacccatgcgcttgctcaggaagcgcgctgcggggccgtacagggccttgtcgagcgaggggaacttcccacacttcaggtagtcttcgatgatgaagtccgcccacgaggactgccgcgagccgtacggcagggtcatcacgctgcgcttcaccagcgagcgtgtgaggccgtggtcgagccacagcgtgcggtacccttcggcatcctcgtcctcgcctagcaggacggcagtcacgcggtctgccaccatctggtagatgtcattcggcagcggtgctgggatcaggttcgtcgccacgccgcctgctgcgtcgcgcagcatcgccgagaagttctgaagcccattgcacgaaccgtccatgccgactgcgatgcggctcaggaagcgatccccgaacacttgccactgctcgtactccatgcaccagctcagaaattgcagcggcttgtcggcggtcttccactcgtcgttgttcaccgggtccgcagcgaacgccatgatctggtcgtgatgctccgctacccacttcacacgatccggcagagacgccttgtcgtatccccatcggtttgctcctgtgatgcagaaccaatccttcgcgtccttagtcagcagcggcttgccatcggcgaactccaagagcgccttctgcaagtccgaaccctgcggcgacacgccggtggtctgaacgtacttgcggccacggaagtcagcgaagtacacgaagtagatgctcgggtactcggcgaacttgcgcgccaccttcattgcgttgtagaaacgattgcccttgttctgtcgcaggcgctcgtcggtgtgccagttggacatgtcgcgcttccactgcttgaactccaactcctgattgtgggacatggtttccttggtcatgtccttcgtcagccactccggcttgcgcggcttcggcagctcgccctgagaaatgatttcctccatgtcgtgcaccttggcgatggccgacacagcttccatcagtcgcttgttgatgcgccacggcacgcgctgcaatgcgttgatcgcagccatctcgttgcgcagctcggcagcgcggtactcgtcgcgggtctgagcgtaggtcttcaccatccacggattgagtcggcgcatttccttcgtgtggaatccaccgttgtcgatgtccacccagtccatcggcggctcgacgcacggcaggtagaacggcgtggcctcgatcacgaagtcgctgatctgagtaatcagcttgcgcacctcgtcggtcagcacgatcttgacgtgcgtcttggtctggaacttgcggtacgctgcgcctgcactggcagcagtctcggtgaccacgccaatctccaacatgcccagctgcgcaagctgatcgcacaggtacgcgccgacctgatcgcgctgtgcctgtccccactccacgaactcgatgccgttcttgcgtccttgcatcttcatcaccgtcatgcggtggttctcgttgacagagagcttgcggtccatgtcgttcatcaggtggtagaacagagtcggctccgcgtcggcgaactgcgtcagcaggtactcatggtacacgttgatgccaacgttcttcaacacgtcgcggtcgctgccttcgccgtgcttgtctcgcatgcaggaggtaagggcaccgcgaacggcgacgaaggccacagcctcgtaccactcgcgtgcctgttcctcggcgctgacgggctgtccacgcttgttctgacgctcgggatcgtacttggcgcgcagaagtggcacgtgcgcttgcgcacggccgattcgcggagagtcgatgtccgcacggatgcgctccgcaagcggaagcacgaaccggcgatacactgcttgggcgtaggggttgttgtccgcgccgcccttctcctcgttgcgggcgatggacttctccatgcgctccttaccgaaggcgtaggtttccagttcgagttccacttgcgagagcattgttacctccgttgctgccgcacggtgtagtcgcgcggcgggtagcgtttcaggataccgcgcatgatttccatgtgcaggtcgtggatgatgtgcggccacgcctcaccgccgatatcctcggccatgcacgtggcagcagcgccgaacaagtcggcaccgtaccgggcgcgcaccgaaacctcgacgcggcccatccatgccgaggactggctgaagtccagctccggcttctcgaaagtgatcgcgtccatcagcccctccgctcgtcaaggaacttggcgaacgcttcctgcaccttgtcgcgcagcgtctcgttcggccacagggaaccggcgtactcgccgaaaggaacgctgatgcgcagctccaccgtgtcgcgctccatgttgtgccatgcttgcacctcgacgctcacaggtctgcctccttcttgtcgtgacggatgcccttgtatcgcggctcgcgcagcaggccgtacttgctgaaggacatcgcctcgatttccacgatgcctcccacgctaggcagctcgctctcgctgtgcggcacgccgctgccaacctcctgcgtcttgccttctccgaggtcaacgacgaccgtgtacacggcgcggccggtcttctcgccgactgcttcgttgatgccgagcacacgcaggtccagcgtcagggtcggcttgatcttgacgacttcgccgttggttcccttgtcgcccttcacccacttgccgctcggcttgcgcaggatcagcccgtcgtacgcgccgccctcgcacagcagcttcgccgcttccatgctgcccagctcttggtcgatcaggaagccctgcgactcggcgtagaacaccggcgcggtgccctcggcgatggcgtggcccatgctcggcaggcggctgacgcgctcctgatacacgaggtcgctgaaaccctgctcccattcttccagcgtcacgaagtcgaacaccacgaacatcggctcggtgtactgcgtgccgtccttcttgcggaacatgccgctgacggtgggctggtcgatctgcgggtgccagtattcgccgaagtacacgccgaccgggaagaacggcgcggatgcgagagcgttctcgatgtggtgtgcgctgacgacctgctcaccggtgcgggagaacaggtcaaccacgccacgatccaccggctgcatctgcacgtcgcccaccttgatggcatgcaggcccttgttcaccgtgggcacccagtggccgcgcttgatggcgaccatgttgcagccgtcgtacttcggctgtgcgatgtactcggtgcgaagctgctcctcggtgggccgcagcttcttcttgatcttgtcctgctcgactgccttgtggacgatgtagctcatgcgtagtccctccaaatctggaacatggcgagcggcacttcgtaccacggaacgtagcgctcccagtacgtggccttgccgtcgtaccactgcacgcggaagttgcccttggtgaaggcgcggttgatcttgaagccgcgcttgcgcttcttgtagccgggagcaacccggacattctggcgaggcacatcaaacatcggcgctgtcctccttcttggtgccgtcacccagcgcggcgttgaaccgtgcgatgcgggacgacatgaactggttgacgatggtgccgatccacagcttgcgcggagcgagcgaaccacggtagccttcccacgcatcggcgatgcgggtatacagctcggcctgatcttcgtcgggcaggttcgggaacccggccttgaccgcattctgcaatgcctcctcgtggtcggcactctcgccccacgcaacggcgttctcgtaggacttgatgagcatggcggtctggttcttgtagagcattcagttctccttcgacgggaatggaacgaaacctgcgaggcccctcatcacgaggatgcagaatgcgtcgtcagggtatgtacgatgccagagtgagttggcccactcgacatcgaactgcttgcgggtacggtgctcctctaggaagcgcgcccactcggcctcatgtgggacgtaccgatgcacttggccgcagcgggcgcaggccatcagtcacccttgctgaaccagcggcggatgatgtactggcggatgaagctgatcgctgtgaacgcaatgccgatggcgtgcgccgacagcagcggatgctcgggatgccacagcaccggaagcagcgcgatgttcgctgcgtagttgatgctgtagccgatgccgatgttcacccaagcctctttgatggagcgcgccttactctgcgccactggccttctcctcctcgcgcagttccagctccaacaggaacagctcgttgatgatgtggtgcgcccggtggtggatgcccgtctccgggtccagcttctcgccgaggcagcgcttgttgtcgtgtcggtagctcgcgtcctgataccgttcgagcgccttctcgacatgctgccacgagtgcgctttgtacttctgcgcgccgaaggtcagggtgtcgatgactcgggccagtgcacgcggcacgccctcatgcagcagacgggcctgcggcttgcccccgtcatccttcaggccgacgccacggtcggacagtgtgcgacggtcctcgtcgcggtagctcagttcgggcattggtacctctcgtctggtggtggtcacgcctccgatgctgagaagctgtcggagggaatcgggaacgcagcagctcggcttaactcgaccgtcgaagaagacctcgacatcacgagcgaacacgcggcttacctgtccacgcagcccgatcattgcgggcgcattgccgatgtactgtacccgcatgccgctgcggatgtcggtgatcttcatgtcggttccttatgccgggacggtgatgtgcttgcgcgcctcggcgctggtcgtgagcttgcgcccacggctgtagccgtcgcacacggtgcactgaagcaggaggtaggtaccgacctgcgtgcgggccggatcatcctgcgggatcatttcgttgcagccgcacttgttgcagcggtgctcgctgccgtcggccttgtagtacactgcgacgttcggatgctgcgagtaccaaccgcgcagcttcttgtactccaacttcatggacttcacgtcgatgcggttgtacgcttcgcactcgtcccatgctccgggcaggctctgcatgcaggccacccacaggtcgaagccggggaagttgtggtggtcgtacttgcgcagctccggcacgatcacgccggtggtgtactccaacttctgcgaggtgaaggcgaactcggtgcggttcagcagcatcgggtcgatcacctgcaccggagacacgggcggcaggccgaggattgcgaggcgagccttgatcttgcgaaggtcgaacttcttgccgttgcgagcgagcacgaagtcggcggcgttgagcagtgcccacagcgccttgccctgcttgcgatcatcgaacacgtcgcgcacgttgcgctggtccatgtagaacgacgcctcgtcgtccagccattcgcaagcgaacgacatcagcgaccagtcacgcttgatctgcttgacgctgaagttgttgttgaacatgccccagccatagaactcgatggggaacgtctcgatgtcgaggcagagaatcttcgggccgcgcttcggtgctcggcgaatgaactgggtaagggtcacggtgtctccttgttgatagcccgacgctttcgcgctttcgcattgcgagcgatacgcttctcgtcgtcggtcttgtaggtaggatgcaggtaccccgtgatgttggtgaggtgcgaccgcaggtagttggggatgcccgcacagaatgcgaacacgtcgcgcacgccgtaccggcctgcgttgttctcgaccttgccgagcagggagttgcatccgcgatggagcaccccgcgcacagcgccggtcttgtggtcatggtccagcaccggatcgagcggagccttcaggccgaactgtccctgacagagacagcaccggttgccttgctccgctgcgagcttgatgcgcagcagcttgacctgtgttgcagtgagtcgcttcatgctttgtatgcctccaagattgcacgcttctcgttcacgtcctcggcgaggtcatagaacgcctgcttcagcttcggcccgaacacgtcgagcttcagcacgtcgagcagttctgcgtcacgatccgtccgcatccacagcagcacggcttgctcggcgaatgtcttgcgccagtcggcacccaacacttcgctgtacttgccgctcacgatctgcaccgcttcgaggttggtcttcgtctcgaacagcagctgctccgctgtcaccttgcccaccttcggcagacccggtatgttgtcggcggtgtcgccgtggagcatctgcatccagaaccacttgtgaccgtactgcaatccgttctcgccaacgatgtcgtaagcgccgagcggaacctctgtgatgtcgtagccgtcccagtctacgtgcacgccgcagaacattcgcatgtccttgtcggcgctgtgcaccacgtgcaggatgttgtggtgcaatgctgcaccctcgttgacgtacgcgatgccatcgtcggcctcacgggtcagccagattttgggagtgaaagcgtcgccctcgtatgtctccatccactcacgaaggaacgcccagttgttgggcttgcggcctgcttggcgctgaccctgatacggctgcgtggtagcagcgaggaagcgatcacccttggtagacgcggcgtgcgtcaggtgcatgacgatcttgcccgctccgctgacatgcttcagctgtgcgcagcgggagagcacgttgcgtcgtgcatcccccgccgagcagttctcgctaccagccgcgaagtacgccatgtagtccccatcaacgtgagcgatcacgcgcgggttgtgctgacgtaccacctgcaccggcatcggggagcgctcaccggccgctgccatgagagcgctcaggtccatcaggcgatgcctgccatcgggtcgctaccgtccaccgggaacggcggcttgtcgtcggccggagcagcgtcggtgggcgcggcgttcgccacgtcgccgaccacttcgtccagcgcatcgacgccttccttggtgaccgtggtgctgcccgccaacttggcggcggcgtagtcgtagcacggaagacccttgaagttcagcgccgcagcgatgcgcagctgcgtcttgttcttcgactgcgcctcgtgggtgaccttgccggtcttctcgtccttgcgctccgggtactcgccggggatgtagatgctgtcccacatgtcggcgtcggcgaagtcccacacgaacgcacccagcggggtgatctgctgcggcaccgggatcacggtgtccacgaacttgccggtcgggatgccgttctccatttccggcaccggcatgaccggcttgcggatggaagccttgtcgatttcggcgaaggtcttgttcgggtcgcgcttgcccggcttgtggatgacttccagcagcacaccctgacccagcagctgcacgaagtggcgctcctcggtgcgcaggcggctgaagattttgaagtagtgcgccttctcgttggtggacaggccgagggtcagcgtcatgcgcaccggcaccggaccattgtcggtttcgatgtgcgggtgctgcttaccggtcagctcgaacacgatggcgacttcatcctgcgtcttcttcttgccctcgaactcgaactcgtgcttgcccagctcgtagtacccgacgatgcgggcggtggtcacaccggcagcgggcggggtgtagtcgaagctgccaccactggcgaccgactgatccttaccctgcgtggcgaccttgttcaacagtgcgtcaagactcatgcgtgttgttctccttattcaaacgacgggttgtgattacctacgaagtccttgcggatcgacgcgcggtactcgatgaccagaccggcgaactctgcgggagggttcttctcctccatcatgttgtcgcccatcttggtttcacacgggacgccaagcggcagcgtccagttgaaccaccactccatatacaccgacgcttccagcatcgaggcgtgcagcagagcagcggccttggttgcgatgtcgccgtgtgcatccacgtagacggcatcgtgcacctgattcacgagcaacgcacggcccaaccattccttcggttcggtcacgtacttccggtagaaggcgcgcaggctgacgtacatcgccgccttggcccattcaccaccggtgccttgcatcgggtagttcttgatttccgtgggcgagaacgactgcgcacagccacccttgctcgcgggcttgttggcgatgaacaccggggacggtgactcgctgaaggaatacatcttgccgtccggcgtggtccagtgcgaccggccaagctgacacgtcagcccatgcggcacgccttgctgccccgcgttgggatgcggaacgaagcgctgagtgctgacgcggttgcgcttgatgtgctcgaccatgcggtcgatgtactcgcccagctccgggtaacgctcggcctcaccgcgcaccagcgcctcgacttcttcctccgacatgccggtggtcgcagcgatcttcgccacgcccgcaccgtacgcacgctggaaggagaacaccttcgcgttgccgcgcttcttcttccacttcttgtgctcgggatgcttgtcgtccttgctcgccttcaggatgaagtcgtagtcgtacttgccttgctcaccccacgcctgctctgcacggaggcagtgcatgtcgaggccctgcttcaagtcctcgatcagctgacggcactcggtgaggattgcctgcacgtagatttcgagggaggtgtagtccgactggatgatcttgccaccccggtgccgggacacgaaggcgcgcttgatctgcgaacccttctcctccaacgtctcctcgtccagctcgcccttgctcacgttctgcaagttcggatcgctggaagacaagcggccggtaaccgtgttggtcatgttgagcttgtggtggatgatgt

SEQ ID NO: 2 - DNA, 44415 bp, unidentified
  source 1..44415: mol_type = genomic DNA
ccgtcgatgaactcgatccatgcctgccggttgagtgggccttggcagatggcgtgcaggatgtcgaacttgatgttgaacccgacgaggaactgctgcccgtaacacagctcacgcagccacccatcgggtgcgccgcccatgtactggttgtctatcccgactcgggtgtcgtagtacaggccggtgttccgtgcgtcacccttccgcttgtagccaatcgccacgatcttgttcatgtcgtagaacggattggccttgcgcttcaggatggaacggatcgtggtttcgaggtcgaaggaagtgaagctcacagcggccaccgttgcagggccagctggtacatttcatccgacgcatcgccatccaagtccagcccgtcgcgcacccaacggaacacgatgatgcggtcctgcttgtccttgatgttgcggcgcttgcagatggtggtggcctcgaccgcgcgctgataccagccggagtcggcggtcaccatgacgttgaacacgccgttgcgcagcgcataccacgtggtgctgtagtcctcgtcctcctcgtagtgtccatcggcaccggagcacagggtccatccctgatcgaccagcttttcgatggcctcgtggaagtcctgcaccagcacgaggaagtcgatgtccgtgtcggtcacgggcggctcgactgtgtagctgctgccggtgcggctggacgtgatgacgcccacgttgcgcggcaggtagatgttcggttcggtactcacggtgtgttacctccgggcttggtgatccagaacgtgaagcacgggatcagattgatgcaccagcgcttgttgtgcggcgagtagtgcacgccgatccaagtgctgtgtttgttccgcagccatccccacttccactgcggcgcgtcgttgcggccttcgatgtagcctgcgtcgtgcaccttgcgcagcagcttggcaaggtggattgcttgcgcgttgctcacgcagttgaaggtcttcgcctcggtggattcaccggggaagctgaccgacaccgtgaacccggtggctacgatgtgaattggcttgctcatgctgcctcctgatagaagcgggcacgctctgcatccatcatcacttcttcccgaacgtcacgcttgccgcctgcgcggtgcagcttgttcttcggggtgccgatgtagcggaagcgttccatcgctgggtcattgagcttgccgcccatgatgatgaagtcgcacgcaccctgcttgccggtcttgctgtccttcagtgcggactgcggcgggtactggattccctcaccctcggcgctgatctgcgaagtcgccacgcccacggcgtcgtacttcacacaccagttgcgagcggcctgatacatcgcctccaacatctgatcggtacgctgcccgccgttggtcatgccaccggtgaacgtgatgttgtcgatcatgtcgaagatgatgaagccggggttggtctgcttgatgatggcctcgacttcaccggagttgaacccgtggatgtcgtagaactgcatgcggtggatgtccccgcccatcgcatcttcgatgcgcttgcggatgctaccatccttcgcccactccaccatctcagggatggtagcgccgagcagcgactgataccaccgctgcttgatgcgcttgcccggcccctcgttgttgagccagatgccggtgcgcttctggtccggccaaacgttgtcgagctgcgtgatccagtggctggactcgctggtcaggaacgtggtcttgcctgcgtcgggacgcatggcgtagatgccgaagtcaccaccacgcagagcgcgcaggttcttcgccaacgtgggcagtcggaagtggatgccgatgtcgtgctcgtccatctgcatcagttcctcgggcgtctcctgcaccagcgggagccgcgccttgcgatccattcggtcggtgatcgtctcggccaagccgtacagctcgtcgcgcaggctgaactcagcgccgccattccactgcacgatcttgctgaccgcagtggtggcaagctccaactccaacagcttctcgatcatgccctgctctgcctcgggcgggaccggctcgcgcatctgcttcagcagaactttgagcagggacttcttgtcgtcgggctgcgtcttccacttgaactccatggcccagccatcgaacacatcgaacggcaagtccttcgtgtccgggaactccttgtagtacgcacgcaacgcatcgagcatcagcacggtcagctcgtccagcccatcacgtggtgcgctgggtaccagccggtcgaacttgccacggttggtgcacaaccgcagcagcgtggtgtcaagactcatcaggttctccttcgggttcgtacttggaatcgagctggtgataccgggtgttgcgcgtctcgaacttgcgcccgccgtccgccacatacagcaccgtcgaggtgtgcacgatgtcgcagtcgccgaggttcggatgcgcaagcacgccgccgagcgtggcacggaagccaacgacgggcgggatgatagcgcgccggtagcgcacgatgggtttgctcattgcagcttctccttgatgtagtcggtcgtgtaatacttcgggtcacgtggtgacgtgatgttcctgtagtccagaccaaacgcacgtagacgcgcagcgattactcgcgcactgtcttggccgggattgctaccgttgcttctacctctgtcgtcatcgagccacgtcgctacacgttggcctcgatcagtcagctgcttcaacactttgttgtgcagcttggtgccgagcaacgaccacgcttcggttaccagtcccaccttgtatgcactgagcgggtcttcgcacagtacgatggtgtcacctgtgcccacgccgtagcgtgcgacaagtccgtctttcggaacgtcaggtgttagccacttcggctgtctcgttgccgaccgggctgtccagtataccacgttgtcgccttcagtgatcggtagtaccacccgcccgatgcttgggcaccagtacagccgcagcttctcgatcatctgaagcgagagtcccatcttgaagaaccacaccttagcgtcgagcggccactcgcgggtgtcgtatacccgtggctctggcaactcaacagtcgcacgcactctgcgttcgctcgtctgctcggcgtggattcgtgcaagcttggcctcgatactctcgtgctcacgcttgaatcctgtgccaccgcacctgaaacagaatgcggtggacttgtcgtgctctcgtgagataagcaagggcgtaccctccccgcactcatgggccacacgtgtgcggccaccaacaggcaggcgctcggcatgtggtagccagtcgttgtcgggaagggtatcgctcatgctatcctcgcttggttattcccagacctcgaagatgtcgtggctggtggcgtacaggacggagccgttgccgtccgtgctgacgatcagacgggagccgtcttcactggtcagcttggacacgacgaacccggtgcccttcggcagcttgttggtctgccgcgtgtcgatcaggtacgcattctggccgggcttcagctcgtcgccacgcttgacgacggccacgctgggtgacggcggggcgaggctcacgactgcccgccttcgccacccgcagccttggcggcagcggcttcggcggcgaggcgctgggcctcggcaacggcggcgtcgatttcttcctgcgccttcagcacttcctcggccgacatcagcagggcgctgctgtcgatcaggttcagctcggcatccagaccttcgccggtctgcaccttcagttgcagcacgcccttgtcgttcttgccggtggcgacgatcacgccggacaggacgcgcttgttcagggcacgaccgaacaggtaggacacggcgtcgcccgccttcagcgcttcgatggcggcgctgttggcctcgacggcatccagcttggcgagcttctcgttcaggccatcgaccttggcctgcgccttggcgatgtcttccagcagctcggcgcgcttggcttcgtagtggctgacggtggtctgctcggtggtgttttcgttcgacatgtagatggttcctcttgacggttgataggatggcccgtacgtgggccagtcgtagcctacccggctcgggttactgaaagatcagctcgctgttgtacccaccgccgccattgtagaagcggcgacgcagcacgctctcctcacccagcaccagcagacggtccacgatggcgcggatggcgctcatgtactggtccaccagctcgctgtgcaagttcaggtcgaagcggatcacggtcaccgcctcgtcgtccagtgcgccggtgtccttgcggacgtacaggccacggccattggtcatggtcgcaccgccgatcagcttcacggcggcggcaatctccggctgcacgttgagcagtcggctgtcgggcacagtcacctcgacccagcttcccatgcgcaggctcatgctgcacctgccagtgcggactgcacgttgggctgcaacgatgcaccggaacgcagctcggcagcacgacgcttcatgcgggagcgcagcttgcgacgctgcttgttgttcccgccgaggctatcggccacgcgcttcagctggttgttgccgacgatgcgggtctgaccctgccccttctgcacggggaagtagtcctgccccagcatcttgcgcaggatcgggttgtcgatgggaatcagcggcacgctgacgtgcaggtgccggctggtgtccggcgcaggcggcggcgtgtcgtcgtcatcgtggcgcggcttcaccgctgcgaccaccttgtccttgacgtacttggccgcagccttgatcttgtccatgaaacccatggttacttcctcctcgttccgaagtgattgaactccaactcatgccacacgtagtacgtggtgccgagcgggtcagtgtctgccttccagttgcgctggtcgcagtagtcgttggctgcgccgaggtcatcgaacgtcagcgagaacccagtggaagccgggccggtgcggaaccggcacagcttgccgtcgtcgtcatggtactggccgacgacaacccacgggccacgacccacgatccagtacagcaggatcaggatgcgcagccagagcttacgcatagtacggctcgacacggtagcccatgttctcgccgcccagcgactcggcattgaacacggcgcgcgctgcatcgcgggtcgggaacagcacgttgtactcgctcttgttgtactcgttgccgtcgatgcgcacggtggcgctcgggtgctggttgtagcagctgacatcggagtcgctgcggtcttcggcgaaggcgtaggtgatacgccaacccagcggcttgcgcaccggcttgcggatgctctcgcccacttcgaggatgtgccagttgaagaacgacccgccgtagctgttgagcacatccgcctcggcacgcacggcggcgcggcggtcgaagatggcgagctggttcgggtacgtgccgtcacgcagcgagtccagcaggctggtggtggcacccttggtgcgcagctcggcgatcaccgcatccagttcctcttgggtcggggtgcggccggtgccattggcgacgacgccagtgatgacgccatcgttgctgttcttggggatcgagacgatgaagtataccttacgcatggtggttctcctgattgacgggtgggatttcgatttcctctatcgagtagagggtgggcaccttctcgtggtgcttgcggtggtgttcgatggcttgctcgcacgcctcgtggctggtgtgatgtccgccgaggatgtaatccccgacagccacacccttcacggtaacgagcggcagcgccttcaccacaaggcgcaggctgacctcacgcataccagcgctccacgctgtgctcatgggtcacgaactctttccactggcgcggctgctcgcacagctggatcggcttgcgctccccactacggatgcgcttgtaagttacggggatcatgcaatgtgccctcctgttgggcgtggttccaaagctacgccctcgttagaaggcgcagcggtagatcacgcgcggctcgggtgccacttcacgcggtagcggcggagacggttcggatcgttgccgacgtgcgaggcgatggcgttgcgtgcagcctgcgcagtggtgaacgtgccgctgagtccgatcacagtggacgtattccaacccagctggtgagggcgccgcgcatgcttggtgaagaactcggcggtgtagaagccgcgatccttctccgggccatcgggagtgccttcgggcaccacacggtacgcatcctcgctgatgccctgcaccttggcccgcgccttcagcatgcggtacgcagcattgcggctgcgctgcggcaggcccagctcacgcacctgcgcccagttggcgagggcgatgctgccgtggcgcagattgaactgcacgatccagcccttggtcttcgtcttgttgaccagcccggtctgcgatgcagtcagggcgacgtggcgtgcgctctggtcgtccatcaggacatccggcagcttacgcggcaggttgtcgggcattgccaggccgggcaacaccatgcggccggtcacgctgccgaggaagtccagctgcgaggcatccaacaccaccggaggcaacggagacagcaggcacgccatcacccgcgcctcgatagcagcgaagtcaagttcacgcatgccgtagcccacggtgaacgtcggcggtgcgatcaggtcgcgcagcagctgtgcctcgacatcgctgtcacggcaggccgcaatcacgtcgtcctcgaattgcaggatggcgtcacgctcgaagctctcgacaccgaagtcgcgcagctcaccgtgcagcacggcgaactcattggacagcttgcggttggagtacgggtctgcctttgcggtcagtgcacaggcgatgtgaagggccgagcgcagcagggatgcttcgcgctgggtcactcgaaggttgatcttgggttccatgttacacgttctccttcttcttggtgggcttcggcacagcgcgggcagcgttgatgacggcctgttcctcctcggtcggcacgtagccttcctcggtcgccttttccagacggcccagcagcttgtgcaggtcggcggcgaacgagaacgcctctgcgggcttctcggtcttgaagtcgtaccacgccttcgcggcggcacgttccagcacgtcggccagagcttcgccctcgactcgcttgctcttggcaaacttcatgggcgcgctcgccttggtttccttgtcgtcgttcggagccatcgggccgaactcggacaggtacaggcgcagggcttcatgcttcatgccgttgcccacggcgagacacagatcggaagcgagcgtaacgtcgccgtggatgtgtgcgtggttgatgaccgcaatcgcggcctgctgaatctggtccaccagcttggtgcgggcggtgttgatcgacttgatggcgcgcttgatgtcagcgcttccggtgatgatgtccatggtggttcccttcaggttgggtccgtgccgattgcacgacactaggccctcttgcgaaggcccagtagcttgcatttaagcgagtcggatgtcgaatgaacgcccaccgcacggcaggacgtagagcgccgacacagagccggccggatgcttcatgatggcccgattgtaggaatcgcgggcagcttccacgtagtggcgagagaacttgaaccggatcacaggtaagccctcctgtcagcggcgtggttcgcccggttcgtcccgctgttaccctcgacaacaaacacagatcgctttccggcggttccgtggcgggcttcgtagcgctcggcttggcgcttgcgctcggcaagcttgcggtcatgctccgtggtgcgcaggtccatcacgcttgccgtccgggtgaactggcagaagcggcgcttacgctgggtgcggtcgagattggcattgatcgagccttgcatgttgtgcctccattggcactggtgggaaaactaacagattgatgcgccctcagaaagccgtcgagtcggtcaatccctcattctcgattagagccgttgcatcgcctatcgtgggcgcacactgaccaccggatttgcctgcatggtcatcgcaaagggagggcgcatcaatctgctagcccttcgggctgtcaaccctactccggctagcagtgccattgtcaccgtgtggcccgtagagccttttcacgaaacgcacagtattccatgcgataggaggctcaccacctccttatgaccggcttcccaccttggcagtgggttacttcccgtggccgactctcacggcagatgggaagccctaagcgttaggcttaggtaaagcggcaccagtgttgcaagtctggtggattctatgggcctttgaaatcccagttcatccggttatccgctagtgctacgttgcagcttggcggtccacgtcaactctcggccactattggctgtggttggcacgcttcccgttacaccctacccgttagcggtagtcctacgccatccaatgtggctgctcctcagagcgtggtgccatactagcacccttgttgcatcctgtcaagcccttggctcgctcgggtctctaacccgttgggcgtcctgtcgccaccatcccaccatgtacgtcggtggtccacgtgttgcaaggcctcaaagggctatctgtgccgccttgtcaagctatccgttagaggaccatgtgcgctcctgttagtgtcttgaccggtgtcccggtctcacctcagcctcaacacccgtaatctctcacgtctagccttaccgctaggtcgctccgctgttccggtggctaccacttgccgcctatcatagctaactgctagcttagtgtcaagcgtggttcggtagctcctcgcatcccttaccagtgactcccgtgtacccttagcccacttgttggcggcgccactacggatcacgtcactcgacttgcgttgcagcttactaccattgcggccgtgtgtctactactgcttgcatcgcaagcgtcaaccgttggcctagcgggtagctaactaatcagctcgacagagtaccgatagacggtgattcaggttgagccgactgtgtgctataggtgtaccaaaaggccgaaacgatacagatggccctcgcacgcctacagctgcggttcgcatggtagcaggtagggtagcccctgtcaagccccttgcggccctcctgaagccctgtcgctgccccagtgacgccattgaaccacaccgcaccggccacgtcaacacctttcgccaagagatttattaacgattcagccaaggcagcgcggtccagccatacaggcagcaggcgcacgcccacccgcacgcccacccgcaggcacccacgcacggccacgcacacgcacgctcaggcccacgcaggcaggcacacgggtacacccacgcggaaccttgacgcgggcgcacagacgcgcacacaggcgcacacgcgggcacgcacccacgcacacccgcaggcgcgtaacgcgagggcgtacgggggcacgcgcgggagcttctattggagtgacccccgcgcatttccgaagcaaattttggtccggctacccacgtggccttactcctaagcctcgcgaactggtgcctttagcttgacgataggcccggagctgtagacatcgtgagctatcgcagcagccatggccttagccacagacttgctcgcatgataggcccctagagctagcgccttgccactgccatcgaagtacggagcctcctcgacccactgctgcttaccagtagtgaccgtgagtacgccgtccttaaccacaagcaccgtcgcggacttgccaacgtgctcctcgtagccttcgcccgctttaagcgcagcgagaaccgggcgaagcactgtgaaatccccggtgacacccagcagcacagggccggtgggtgtcgatacgggcatgatcttacgcacggtgtgcttgtggtcgccctgcgtggcctgactatcggcccacaggtgcttgccgtcccatgcgatggtggtcatttgtcacccgtacaccggcgcttaccggtaccgcacacctcggccttccacgcacgcagcgcagccttgtccttgttgcacagaacggtgtccatgcggcggtcctgcgcgagcttgaccaccttgtcctgcgaggaggtggtgcccttctccccaccgaggtaggtgatgtggcagtctgcaagcagggagtcgtcagggaccggcaggttcgcgcaggaggtcagcgacatcagcaggaacagtgccatcccggtactccggggcagcgtcaagaacttcttcagtgcgaacacgcacgtcctccttctctttgatgtaggtcgcgtacccggtagcctgcgtctgcgccgccttggcggtagcggtcgtgccgacttgggcagtttccagcttctccaccttgcgttgcaggccgtagacgtacagaccgaagcacacgaacatggtcacgaccagcagcaagccaaccagcttgccgccgagccgcgcgatcacttcacttggggtttccacggttggatcacctcgttgttggggcgcaagcacagagcaaactctgcgtcgcggcgcttggggatgccggagcaacggctgctggacagtcggcagtcgagcttaccgacgtagacccagcgcaggaactccttgcagctaccttcacgatcccctgcgttcgctttgcgcagcatggtgctgtcggcgaacgccttctcacctacgttgaacacgaagtctgtgtaggcgtcgatctggttgcggttaacgggggccttcaggtgcttgcgcacgccctgctgggcgatctgtaggtcttcgatcagccacttgtcgcactgtgccttcgttgccgtcatgcccatcgctacgcccttggtgtggccgtagcagatggtcggcacccggccggtgtcgaggtacgcagcgtagcgtaccccttcgtggccttgggtgaatgacagcagcgttgccgaaatgccgatgaagatgccgccgatcaggccgaacagccccttgttgctggtatcttggttctgctgctggttcatggttgctccttacggggtcagtgggtcgtcatccgggtccagatcgaccggagtgtgcgggccggagttcggacccgaggacgcggtgcgtgcgcccgcagcgatcagggcgtccagcacgagggtggcgtccttctggaactgcgcgagcagctgcgctgcggttgcgggatgctgctctgcgtgctccatgagggcgagcagttcgcggtgcaggtagttgccacggccgaacagacccgtgtagttgctggtgaagtcggacttctgcattggttacctccggtaacggtcgagtagggatggacggccacgttgcagcggactcttgcgggtcgctgccttcatgccggtcggatcgttgatccagtcttggaactctcgctgctgctgcttggcgatggccttgttctggtccagtgcaagctgcgcaacccagtgacgcacgctaccttccagtgcatcgagccggtcatcgtgtgcgatgctgcccttctgctgcgtgatcttcgccatctggtggaacaggctgtagacctgacgcttgccgctggtggcgtagcgctgggtgtactcgtgatccatttcaaccacggattccagcatgaccagcgagccgcgagccatgacaggttcgagagtgccgatgatacgggcttccttgttgccggtcacgaactcctcgcggatgtcgcccttgtatcccttctccgtgccgcgatcttctcgcaggacaggcaggaacaccttggcgaacgcgccgtagcccatgttcttttcgatgctgatgacgttcggcttgtacttcaccgcaatgcggcgcagttctagcaagccatcaccgtcgtagccaccgggcacagctcccacggccaacacgtacacggtggagttgaggaaggcggtcacggcgaaggccgtctcgtctccgttggcaccaccaccggccgggtcgatctgcatgtgcacgccctgcacgggggcagtctcggtgctcatgtcgtgcggcatcatcatcacgaagccgtacccactggactggaagctgcgctggtgagcgttgctcaggccacgggtgatcgtcagcgggaagcggtcgccaccaccggggatcacgatcaggttctcggtcttcagcgggaagcgcatcgcatccatcagccgcgtgttgagcatgtagttcagctgatagctggacggtccacgctgacgcagctcggactggtgcttctgctcaccggccaacagctcgtcggtgcactggccctcgtcgcccatcgggccaccaccgaacgccaacatcgggtcggcttctaggcgctgcacgatagacggtgccagatgcgggccgtagtgctcgcgctgtgccggggtcgggtagcgaccgggccagatgcgaacgtcgtagccacgtccgggcagggtgttgtagatggagtcgccggtctgcggcgtgccgaggtacaggatgcgacccggagtaccgggcttgccggtgcagatggccgagaactccaacgtgatggtcagcagcagctcacggttcgcggcagtgcggctgttcttgttggactccacgtcgtcggcgatcagcaggtccgcacgcttacccggcaggttgccggtgacgccgatgcacgccacgctcggggacttgtcgattcccttcagcgagtggtgcacgtcgaacgcatccacggaggtacggtcgcccgcgttcttgtccgggcggatgcactccaacgtcggcaccgtgaggatgatgcgctgaatcagcgtagcaatctcggatgcctgcgtgccgcctgccgatacgatcagcacacggtgagtgggatcgtggatcaggcagaagacggcgtagatggcagcgatggtggacttcgcctcgcctcgctgcgcctgcaccattgcgaggtgcgggccatactgcatgtagttggcgatgtcgtactgcatccacgtcggctcgaaccccagcaccttcataatgtcgcgcatgaaggtggcgaagtgccggtagtggttctgcaacagctccaacttcttgcggcgcacgtcggccgcttcagctgattcacgcattgttggctacgctccccggaaagtgaacgatgttgtcgagtgcacgctgcaactcgtcgtcgtcagccggaggcagcgagtgcttgcccagctcgtcttccagctcgccgagtgccttgttggcctcgcgcgtcgccgtgatgttgttgtccttcaggaacttgatcgccgcattgatgtcggctgcggtgcacagctcgccatcttggatgcgctgcatcagcgcacgcgcgaccagttcgtgcagcgcaccgagtgcgccctcacttgccggattcgacatccttgcctcccatgatctttcggtgctcgcgtgcccgccagtagaactgagcgacggcgtacagaatggcgagcgtagttacgatggcagcaccgtacgtgctgatgaagttgaggtagaccgcgccgagcgtaagcggcgaggttcggacgacctcattgaccacactcggcggggtcatgctgttctcctgtaggttagggccagtcgtcgggattgccgacgagcttccattgcaggcggttgacgttgttcatgcccaccgcaatcaggtcgccggggattcccgaggcgatcacatgttcggttgcgaagcgctcacgctgcgcgcgtacgcacaggttgctgccgttcttgtacgacaggagcacgtcgctctgcgtggcgaagacagcccgcttctcgtccatgcacaggcgcggagtggtagcaccggggatcaccatggtctgcatcgaagcagccaccgtgtcgtaccagtagaacttgcacacaccgcccgccatgtacgccacgtgcgggcgcatggtctggtcgaaggccagtgcgatctgcgtgatcccggagtcggtcagcacggtgaccggggcaacgccgtcgcggtaaacgacgacgctgctgccgtcactctcggcagtccacagcgcagcttggaggtcgtccactgctgcgttgagagtcagcccgccctgctcgaagtcaatgagcgggcgggtgcgccgattctgctgctccacccagtcaccgcgttggatgctttgggagacagtggggatcatggcgtgtaccggctccaagaaacccgcatgcgcaagttcgccgtctccgatccggtcttggtgatacccggattgaagccgacttggaaggtcacgcacgcggagagtcccattgcagccgtgatcggaccaccgggcacgttgttgatcgacatccggcaaacgcagtcacggtagtaagtacccggaacataggctacctgctgaagctgcaagtcagagaagctggcaatcgtccccggcggatactggtcggtgatagctccggtgccgtcgccagtaccgccgtagaagtagtagcacccccacacgtagtccgaccaagcgactgccgactgaccgttcataccgccgctgcggcccattgcaataggcttacaggtaacagtggtgctaacacccttgatcgtctcagtagtgacaaccggcgtggtatctgcgtacatgcgcagctcgtaagtaaccacgaggatttcatccgacagcaccgtgatggtggtcgggttacctgcggagtccttgataagcgcacgggtggtcaggatgtacgcgccggtattgttgttgtatgctttggcaccaagctccgacagaacgccagtagcggtaccagccgggaactggtactggcagcgggagtaggcgtagtacggggcagtggtagtcccaccgctgtccgaggacgtacgaccaacctgcgccacctgtgcaccaagagcggtatcggtgaatgccggggtggcgctgccactaccgactgccaagtaagcaatgaggtcgtacatgctgcgaggatagccgctgccggtatcacccagtgcgtccataccaccgtccgtgataaggttgctctgccagtcggctacaacttcgagagtatcgagggacttacccttgctgatggtgaacacgccagcaatgccgaggtgattgtggatcatgcgaagctccatgatacgaagccagaccggagtcgtgcagtcgcgtcgagcggctggttgactacagggtgctgcttcagggtgaaggaatggaaagaactcgacagcttcgccgtctccgggtcaggcgtgtagtccttacggatggatcggatgtcgaacgaaacgaaagcgctcccgtacaacgtgctctccgggtcggcggcataatcctgcctagagcttcggagttcccagcttacgaaggaggaacccagcgacgcagtatccaaaggctggagcatgtcgatgttgctgtacccagcaaagctgctggtcagcatcgcggcatcgaactggtagaagctgtagagcttggacgtaacgtagatgccctgctcctcgatacgaccggaccagtaggccacacggttcaacccgtccgtgaccttgatgctaaggaagtaggagctgtcgtcgttctgacccagtacgtacttgtggttccacttaacggtgtccacccacagcggtttgttctgcttgctgcggaacgccgacagtacaacctgcacgtacttcgtgtccttgggcgcagcgccttcggcaacggactggtgccacgcaccgttgctgccggaggaaaccatgttgccccagttgcgttgcagctcggtcccatcctccttgcggtagatgatcgacacacgagcaccggccttgcccttggagcttgcgccctgctggacctcggcggtgcatcggatgtagtcgttgaccttggcagggatcagcgggttgagcaggtcgctgccgcccgtcttgatgttggcgaagcgcgcgctgtacacgccgctgtcggtgtcgtagtctgagccagtgccaatcgaccagccttcgccattcgatccaccgcccggcaaccacgtgccgtcgtcgcctgcctcgaagtcgccgttgggcacgagggtttcctcgtccacgacttcagtgaaagccgcccacttgacgacgacttccttggtgatgttgtccacccgtaccgcagcgcccgaagggagcgtcgattcgatgacctccacggtgcagcggccgactgggttgttgatggacaggcgagactcgtaagcctcgcccgccgtgtacccttccagcacgcccgtcaccgacaggccatctgcaacctcgtccgccatgagcggtcggccgtacagcctgaagtgattagccatgcttactccttagccaagtcgcccgagagcaaccacgtgttggtgtcgccgtcgatgcacgttgcagtgatgacggagttggtgccgcgagttgcggcggtgcagccgaccgggacttcgagcgtcacgcccacgtcgccagtgatgaccacagggcctgccttctgctgcacgctgaagtagctgcccgaggcgagcttggtttcaccgtcgcccacttcggggatcaggttgatgttgacggcgcaacctccggcgtacgtgcagcgcacgagtccgtactcggtagccttggcggcgtagtaagtcggaccctctgccgtgatgatcggcacccgcaggctcgcagcggtgatcggcgcaggcccggtgtagggcttggcgtaaccacgcagcacggcgaaccagatgctgccctcggcaggaaccgtggcgaagcggatgaagctgggatcggtgccgtcagcgagcgtgacctgatagtccacgtccggctgcatgccgatgccgttgacgtacacgtcgtagaagcccgcgccggatacgtccgcgcccaccatgtcgaagtcggtgtcacccacctgatcgccagtccaagcaccggaccagacgcgcggggcgacggacacgataccaccagctgccagcaactcggtgacctgcttgtagatgttctggataatctcgttcaggtccacgatcacaccgacctgctggtcgatgctaagggtggcgatgttgagtgagtcgaacatttcctgaatgatcttcaggagctggtcgttgctgaggttaaggtttgtcttgctgatgatgctaccgttaacgtagtcaacgagcatctgctgcaccggagtgctgcggtagatgtagagcttgcgcccagcggcgacggcaggcgagactcggacggtactagcgtcatcgtcttcgctcaggacttccacggtgtgcggagtccggtcggtcagcagctgagtctcctcgtccagcagtccgctcatggcgtacacgtgggacgggttgatgtagccaccggtaaagctgatctgccagtcagtggtcacgccatcggcgtcgaacacgtctgtcgcgtagcgcagctgcgggtctggaactgccatgctgcctcctgtttgctataggtgtaccaaaagggtgggccgtccttggccctgatcttactcctccttccactggctggctgcgcccttcagcagcgggatcaccatcggcagtcgcccgcccggaatcacgtcggccagattctccggcttgccagcaatgccctgagcgaagtcgttgatgactcccagcgacggcgcgaactgcccgcccaccacttccttgcggttgccgaactgcccaccggccagctgcttcagccacgtcggaccctgcgtatcggtggcgtactcgtaccagccgcccgccacgccagtgcccacgtccagcacatcgttgagcatacccgtcgccgacacgtagttcagcgtggccttgcccagcgccagaggcgacaggatgttctggtcgatggcctcgtcgcgctcctgatcgttcatcagggccacgcgggacagcacccgcagggcttgcagcggagccgccacagccatcgcagcagcgatcaggcccgccgtctgccatgcaccgtagttgcccacgtaccggcccagctgcttctgctgcgcgaccagcgagaacgtgcggtgctggaacagcagcttcagccagccgttgtgcgcccacttgccagtctcgccgatgaaggtgtcctgaagaatctgcgaggtgccacggttgatcgcgttgtagaacgccaaccatgcctgccgatccgccagcccctcgacgttgcgcgggtctactgcttccagcttaccatccgcgccccagcgcacgacctgatcctgcgtagcccgcaggcggttcagcaggttgtcgtcaatgcccatgtccttcagggcggtgtcagcttcagcaccatcacgcaggaacttcacgcccttggcgatcagcacttccgcgaagccacgctgctgcacagcaagcacggcccgctgccccgagaggatgcggttcgcatgcgctgccttctgcaccagcgaggtcaggaagcctgcgcgctcgctaccatacatcgacgcctgcgtgtccagcgagttgaacatgtgtaggtcgtaaccggcgagaccgaagccgcgaccgctgatgaactcgaagccgtcgaggatttggttgccgctgtcctcgcccttcaggatgcgcatgatttcgctgcgcatgcggggagcgatacggattgcgtcagccacaccagcagcaccaacagcggcgaggccgttgctgtactccgctgcctgattgatgcccgcgccgcccagctggatggccgaggtcagcagacgcgcattcgccagaacagtcggatcgccggtaccgaccgggcgaccaaggaactcggacatcacctgctcgaacgccttcagctccacatcgttggcaccggtcaggcgcattgcttcgcgcgccacgttgatgcctgcgtcgccgaggatgccgtgcttcgccagagcgatgtcaccagcaacacgtcccgcgtacttgcggtagttgtccatcacgcggttgtcgagatagtccatcagacggaacttaccgtcagcgtcctcgtactgcttggtcacgtcgaggtcgatacgcgccttggtgtgcttcgcaccgccacggctgtacttgcccatgaccttctgaatctcctcctcgttgagcgacatcgcccgcagagtgtcgcgcagcgtgtccgcctgcgactccgagaagacctgacccggcgcttcgatgacacccgcagccttgcgctcgatgcgttccagatacttggtagcgaacttatcgaggaagtcgtccccatacagctcgcccatcacctcgaactgatcgcgcatcgcctgacggataccctcgcgtcgcaccggaccagcagcagcgatgctgccgcccagccacgtacgggactcgtagccctccacgtcctcctccggcagacgctgtgcgcccaccgtaccggccgcgcgctgctctgctgccatgcggttgtagccacggtccaactcacgggccattgccttcactgcctcgtgcgcatccgggatgtccccgccgttgaagcgagtctcgcggtacagcttcactgcgtactcgaagtccgcgcgagccttccagcccgtggcgaagtccttgatcgcaccgataccgcgcacgtccgcacgccacaggcgataggccgcttcccactgacgcgggcgggtgcccatgaacgactcaaaccgaccatgccgatccatcgctgcggtgctgtgtcggcctgctgcaccctcgggattctccaacagggtgatcgcaagcatgcgggcaactggcgacttggacgacattagagtcgtgctcgtagcttccagcccgaagcgctgcatgatggtggacagcttcgccgcgtcgatgccgtactgcgcactgaagcgttcggagcgtgccatcacttcggcgacctgcacacgcatcgcgtcatcactgacggacttgtccagaccggtgcgctggtagaaagccttgcgctcgcggttcgacttgaagatcgagttggcgagcatgccacgcgtctgccgggtaccggcctgcgtgtcgcgcacttccgcgccgaggttgtcaccgacgaccgacatcaggcgttcgagcgcggactcctgattcttcagacccatcactcgcgcgatcttatccttcagccactcccacgcattcgggcgggtgttgcccggcgcgggcatctgacgcagcaccgcctgcacagcgcggttcgtcaggccgtaggaaatcagctcgtcagtgttggcgaggaagcctgcctgcggctggttgatgcgcgtctccatcgcagcggtggtcagcgtggagtccacactgccgatgctgttgttgatatgggtcagcagttcttccatttcctgcccgaacaccgagttgctgcgcagctcacgcagcgtggcagcgtgcagcatttcgtgcaccaccacttccggcgtgtagttccgcatcgccatcgcgtccagtccggcgttgtagccaccggccacacgcatacccggacccatgttggcaccggcgaaccacttgtcgagttccgattccggcacgatcttcaccgtgctcagccgcccgccacgcttcagcgcgttggcgatagcacgcacgtcctccgggatagaggcgttggattccagatacttcagcacgccatcgacgttaccgcccttgatacctgcggtcttccatgcgcgttccagcagcgggtcatgctgatcgacccggccacccacgctgtcgttgtaccgcccggtcgttgcgtccacgttgcccgcgtcccgtgcgagtgcaccagtggtgcctgcggtggtggtcgtctcctgcacgtcgggacgggcgaagatacggaagtcgtcaggcacgtcggccataccagcgcgcagccaatccacagcctcctgcttggcaagctggtggatgcggttgttcaccagcaccgggttggcgtcctcgcccagctcggccacagcgcgcgccttcaggtcggccgaccacgcttcgccgtaagcggcagcgttgcctgcggacaggtcgatggttgccttgtcacgaatctgcgcagccgagcgcacgcccggaatgtgcatcgcggtgcctatggtggtagcgaatgcagcgtcggtcatgaagtccgcgaagttgcggcgctcgcccatgccaaccagcgcggcgtccgtgatgacggaaccgaccgcgttctccgcagcagccgacgcgagcgacgcgcccacgcgcccttcggcaacgagtgcagccgagccgatgcccagcgccttagcgcctgcggcagtgacgccgccgatagcccagttgcccggatcggtgaagcctgccaccatgtcgtaaccgaagctaccccagccagtctgctgatccttgatgcgcatggagtggcggcgcaggaactgtcggtcgctgacgtacttcagctcgttcggcgagtacgctgcatcgcggatgtcttcgagttcgtcggcagtcatccacggcttctcccattccttcgggtcgtacttccaaccttccggaacgttctcgtcctcgcgcgcaaactggttgctgatcgcagcaccgatgccgctgtcgaacgcagcgccccacttgtcgaggaaggtcagcgagttgcgcagctcctcgtccgcgcggtcctgcgcgagcgcctgttcggtctgatccagcagcgccttgcgagcgccggtgttcagcacgtccacttcctgacgcacccaccacggcacaacctgatccgatgcacggacagcctgagccttgcctacggcctgcgcggcggtgccaccttcctgtgctacctgacccatcgacagctcggcgatgcccgcacgaatcttgccgatgtgttccttcgctgccgacgccagagcgttgcggccttcgatgggcgcacccgtccacgcatccgggatggacgcaccggaccacgtacggtcgcgcatgttcgggttgccctgccatgcggcgttgaggtctgcctgcgtggtggtcaggctgcgcggctgcgccgacactgcgggagcggacgcaccgcccagcacgctcggtgcataggctgcgttctcctgcccccagttcttcggattggtgccgccttggtagatgcgcagcgccttcgtcacgtcgcccttggcaagctgcatgttctcgcgcatgatgtcggcatacagctcgatgctgtcttggaagttgcgcatgtcgtacttgcgaccgttgcgcgcttcccacgttgcctgcgtggtgggcatgacttggaagtcgccctgtgctcctgccttgctgcggatcacaccgtcagcgtccttggcggcacgcccgttgccggactctactcgccactgaccgcgcacgatggactccggcactcccgcataagcggcagccttggcaatctgctggtcttgggtcagccccgaaagatcgagtgccattgtctatctccttacagtttgggttggatggaaatgctctgctgaatcgtaccgtcgttcatgcgaacgtagccctgcggtaccggggcctgcaactgacgctgctgcttggtgtgcttctcgtactcgtccttgatgtcgcgcccgtacaccggcacaaccttccagcccttctcgccaacagcgttgacgtacagcaccggctcgccgttctcgctgtccttcatgcggaacacgtcagccttcagcccggtgctcggctcgatgttgacccggcgcagtgctgcgtcgatggccttctcgatggcgggtccggtttccttcgtgtccatgaagcccagccatgcaccgacgctgccgatcactcggccttcgtcgtcgcgtccgttttcccatgcgtacttgcctgcgtcttccagaccgtaggccagcttggcgtgagtagccgcagcctgcaagccttccgcagaagtgtccagcagaccaccggtgtcagtgaccgagcggacgatggcgcgagcatacgcagcgcggccagagtcgcccagcttgttgccgaacatgccgaggtacttggggttgagcttggcgatagcttccgtaacacgagcctgagtagcctcggattccttacggctgttcgcgtcgaactgcgtcggatcgtcggtggtgatttctccacgggccacctcgtaagcaagctcgaagttcacgccaccattctccaacgcttgcagcttgttgaagaacgtgttgacgctatctccgaagtacagcgcagcggtagtcgcgccagtcagtcggccctgcacgggctgaccgttcgtgtcgatgcgtgcggcggtggtctgcttcagttccttccactgctggtacagtgcagccgctgccgtgttcggctgatcgcggagcacagcgcgcgccgtggtctggaactggtcggccacacccttcagcacagcgcctcgcccggtgttggcgttccacaccagctgcgacatggcgaccttggggttcgcggccatcgtggcattccatgcctgcaccgtgttcgcctcgatcagctccttgtccacgccggggatgttgatcgtctgcgcgtacgtgccgcgcttgaacgcttcgatgccaccacggatgtcctcctcctgcgcggccagcttctgctggtcggtcagcgcggccttggccgcagcgttacgctggttgatgacggcttcctgtgcgcggatgtgcgcgcctgcggactgtgccatgatcgaagccaactgcgtaccggagtacagcggtgcgtcgcttccagtctcggcggcgtaggtcgagttcatttcctcgatcatcgcctgcgacggcttggcaccaatgccctccgatgcgtacatggagacgagcgccatcttctcggcctgctccgggttggcatcgagccagtcggaacggtaacgatcctgcgcctgcttcacgtactgctggattcccagctgcccgtccgggtcgatggcgttcagaacgcccttgctgttgaggaacttcagcgtgtggaactcgccgcgatccgcagcgccacgatagaacgcagtgatcgcggacttgtacgactcgtccgtctggtagcgcgagggcgacagtccgtccagcagggacagctgcgcctgcgtcagcgcctcggtggccttctcgtccatgggacggttggtaccgagcatcgccgtgcgcttcgccagttcgttgaagccggtggacgccgacgagttcgcagcgtactgcgccttcaccagctcctgctgctgccatgccgtgcgctccttggtgtgcaggtccatgagggaacccgcgcgatccatgaaggtcttctgcaacaccgtgtccgcgaaaccgttgccggtcatgcgggcagtggcgaggtcgttgaactccttcgccatcgcctcgggaggaagctgacgcaactccggcatacgccgaagcaagtcgctctccatttcgttgacctgcgagagcgtgttatacatgctcgcgccaatctcgtagttggtgtctccgaagattttcttgtaccacggttcggtcgcagcaatctcgtccatggtcttaccagcgcgggcggcaacgaagccgtcccacatctgctgctgcttcagcttggcggtgttcggcgctgccagctcctgcaagaactctggcaggttgctgtccggcatcgtcataccaccagtgcttgcgaaccagtcgttgccggattgaaccggcccgacctgattcacaccagcgccttgaatgctggtgttgcccgacagtgctggggtggcgttgatgccaccctgcaatgcggactgcgtgttgaaggtaaccgtgccgatgtcagccattaccatgcacctcctgagttgcctccgctgccgctatcgaaccagccgaggccggacgtagtggtggagaagttgtcgtagttgttgccgaagttgccggtgaccttcgccccagtcacggactgcttgccggtgccgtcgttgtacccgaaggtagtggacgcccacgacttgccgccgcgatcattggactgctgccacgcctgcataccgttctgcgctgcgttgctgaaggactgagaggcaccagtgaagttgccgttgtccgcctgccacgtgccgaccgcgaagtctgccacggcctcgcctgccatcggcccaccgaagtaggtagccacggccacgccgatcagcttgcccaagcgacgcttcattgcctgcggctcgatgtgctgcgagtagtcgaactgcccgaacgaacggctcatgtccatcccgttccacgcgcgcgacatgatctgcgcagtctgcgatgcgccccgcgaggcgaggagcgagacagcgttggcctgcgtctcctgatccatttccgcctgcaaccgcaccatcgaatccatcaggtctgcggacgagccgccgacaccgacagcaccagcctgcgcctgaagtgcgccacgcgcgttcgccagttggagctgggagttaagcccagccccttggcgcgcacgcagctcctcggacagcgcttccatgttggagttgtactccttcgcggcggcgtccagttgggcgttgttcttcagggaccgcatgaaatcagcgaagccggtcttggcgacctcgctgcggttctggttgtcggtctgcgcaacggctgcacggtagttcgcacgggcaacgcgggtggtgttgttcgcttgcaggatcgtattaaccgaacccattagctaaccctccgtacattgttgaaagtctgacccgtccagctcaggccggtcacccggagcgggagccaatccttgctgcgaatctcgtaggtgcactcgcgcacttcgcgcccgacgctgatgttgagctgcccccggtacaccggttgccgcgcgatcagattgtcggagtcgccgaggatgcggccctcgaagtccgtagtggtcacattgctgttgcgggttgccaccgtggcgatcatgcctgccgtgttctccacgtccaccgtcaccttgttgagggacatgcgtccatcgagtacggcctgaccgttctggtcccgagggaacggattggtcgggatcaccagagcttcggacaccacgccgtattccagcgcaccagcagcgaggtcatcgaactggttaaggaagtcagacgcctgcgcgtagggacaacccagcaggaagtacgggctagtgctattgacggcgatgcttgcgctcgcagtctgtacgcccgtaggtgtaccaaaactcgcccagctgtcgaggcacgcatgcgagtccggctcgcccttcgggtcgaacacgtcgcacgccaccagcgacccgcgcgcagtgaacacgaggccgttcttcttgtagctgctcacgccgatgatttcgcccagcgccgggtggtaccggaacttcgaccacgcatccacgatgcgctgcccgttgttcttgttgtcctcgtaccggtacaggtagaagtcctgcgggtgctcgcgagtgcggaacatgacgaggttcggcgcagtgagcggggtgatctgcaacggagtgcccgacagccacgagtccagctcgttggacatttcgtccgtcaccgtctgctgcccgttgagcgcgcccactcgcatctggtgcaggctcgtgccttcgctgccgtactgcgcataaaagatgtagttgcccgaggtctgcgccttcgcgtcaaccgaatccttgttggcactgaacgctttaatcagcggattcttcggactgaacaccgagtcgccgctgatgccgtactgctgacggtcaccgaagatcacgaggttgccgttgtagagcgtcgcgtgccggagcacatcgccctcgctgccgtgcgcgaagatttcgatggggtcgctgtcttcgatggtgacggccgagccgcgccagaagttcaggtagtccgccgagcgtgaggcgttgacgtagttctgtgcgccgatgaccagccggtcttggaagacggacagcatcgtgatcggcttgtcgatgaaccacgggatcggcgaggtcagaccatcgcctgccactcgcgcaccgtaggccggatgctcgccgctgctcggagccagagacgtgaggcccgcaccgttgcgtgcgatgtagcctacaccgttgtagatgtagagctgcgacacgaggttgtcgatggtgcactccacgccgggcgcttcgtaccagtccaccgacccgtagccggaagtctcgccgttctccaactcagcgcgcaggtagtacgactcgtccgcgcctgcaccactcggccgcacgcgaatgaccttgccgtgccagtggaacttgacggcgtaggtcgcgtctgtaatttcctgccctgcggcgtagaaggtcgtgccgtctccctcgtcgtcaaccgtgatgtccttgaactggtcatcgtcaatgatgatcccgcccttgatgtacgttgccgacacgcctgcatcgaccagcaaatccgacagctgctccgcgatgtactccgggcgcgtctgctcagcgctcgtcacgatccactcgttgaccgcagagttgtactcgttcactcggtcgttgacgtacttctggtacgccgcgtccggctccgtgccaccgggaaggtagaacgggatgtcgctggtgtcgagcgttccggggtacgatgcggtaaccgtcttgaacgttaccgtcagcaccgtgttgtccgtccgcgtcaggttcaccgtgtacgtggtgttgtacttcccggtgcgcacccatgctgcgaggcgctggatgttcgtctgctcctgccacacgttcgtgctggtggccgaggggatcgtggtgttgcccgcgatgtagacgtagctgccgatggccgtgagcgacgatgcgcctccgctgaccagcgtgttgacccacgtgctgttctcgtacaccagagggatgaacgactcgtccgtcttgttgtagaggaacgcgaaggactcgctgcccaaggtcgaggcgtcgcgccggtacagcagcgcgtactccttgccctcctgcatgaagtcgaacacgtccatgttgcgcagctcggccgaggtgacaacggcttgggaagcagcgaaccgcgtaccacgacggcgcacgaggccgttcaccggatcggacagcacgttgatctgctcgtgcgtctgtcccggccgacgacgatgcgccggtttctgactgacaccctgaaggatgtcgggataggttccgcctgcctttgccatgttgtctccttagccggggaatgtgacgtggctgtgccacgggtgaccgctgtagttccagtaacgggaacgcagcacgtccacggatgcgcgagcgaacagcgggttcgccttgatctggcggatgtgctcggccttcaagttgatgtaactgtcatcgcgctgctgcttgatcttggcgtacttggtgttgtcgccgtcgaagtcagactggaaccgcagcaccgagtcgtcgcgcacgaacatctgcacctcgtaggggaggtcatcgaagtccagcagccgcaccagcttggcctgcacgttgtggtcgaactcgtaggtgttgcgcttgcggtcgtacagtcggcgtccgcgctgcaccacgtggccgaaccggctcgggttgcagtccagcttcagcacgtccgtggggaccatgatgtacttgctcgttgcctgcggcttcagctccacccattcggtgttgaaccacagcgagagtgaggacacgtcacggtgcacgcggtcgatcaagtcaacggcgtcgtccttgtatacgtggtcatcttccagcgtgttgagcttcgtctcgcccatcgtcttcaagcaggcgttcacgatgtcgagcttggtgatgaatgccatggtgtctcctgagaggaacaaggcagagacgccggagcgcccctgccgggatgttgcttagtccgcagccagagccagagcggccggtgcgtactcgatgtcctgcgagccgatttcgtcgtccacgaaacggacacggacgacccagcctgcggtgccacgggtgtcgtagtggacgccgacgacggtaccaacggagttggcgggcagaccggccacgccagttgcggcgacgacgcggttggaaatctcgaacggtcggtcaaagaccatgatgttgctcctgtgttggtggaagaagggcgcggtttgagttacccgaaggattcagggaccgcgcccagcggattaggcaaccttgtcgatgcggcccgcgttctcgacgcgatccagaccaacggcgaaggacatccacgagtccacgaagtagcacttcgaggcatcgctccaccacaccgaggactgcaacggcagcgcttcggcgatcagcagggccttcggcgacacggccacggcgatcagggtgctgaagtcgccgtcgtagaagtcgtcgttgtcgtcgttcgacagcaggtgaccttcgatcacggtgttcggcaggttctcgctcgacagcaccgggacgccccagccgtggaaggtcgggatgccggtcagcttgttgccgtccgaggtcaggtactcgccgttgctgatctgctcggcctgctgcaacaggtagaagatcgccgggcgcacgatcaggaccacgccatcgcgctgcggcttgaccttcttctcctcctccatgcgggagaacagtttgccgatggcggcgtacaccttggccggatcgttctcgtcaccagcggcggacagcacgacctgcgtggcaccgaagtggccctcgggcgcgcggccgttgcgggtgaagatcgactgcgtggcagcagcggccttcgcggcggcgatgctgatggtcaggtccacgaactcggcgatttcctgaccctgctcgatggcgatttccttgcgggtgtcgatgtcggtgaagatttcgtccagctgccagatgctgtgacgcgacagcagcatggtatcgacggtcaccgacgccttgctgaagtccaccggggtgccgtccggcgcgtcaccgcgcttcagcttctgaagcttggtacggccgatggccttcttggtcagggtgttggtgcccttgacctgcttgcgcgggaagaacttttccagcaccgagctggacacgtaggtgtgctcgacatcgccggtgaactgttcgaggatcagggcgttctcgttgccggactggttgacctgattcggcagaaccgggacagtcgggaagatggtgctcatgctttgtgttgctccttggtcttagtggatgacgcgcgcgttgagtgcacgcagttcttcggagtgggccgcaccacggatgcccttctcggcaaccagcttgcggtactcagcgcggtactgctccttcgtgataggagcgacgccgttgatcgacgcggcgggggcggcggcgttggtagccggtgcgcccttgacggtcgtcgcgggattggcctgtgccagagccatcaggtaacgcgcggtcgcctgagcgccgaagccaccagccgacagcgattcgcttgcctgcttcagttggtcggcgggcaggttggcccgtgcgaactgctggatcgcagcccagttctctgcgccacccacggcttcgtggacagcagcaacgttcgcggcgtgcgctgcggttgcagcggcggtgacacgagcgatgctctccttcgccagagcgaggatcggtgcggaacccttggccttgtcgccgaggacttccagcttggcttccagcagggcgaagttgcccttcgctgcttcggtcagttcgcggctgtcgatgtcgaggcccacggtgttgacgaagtattcggccgcgatgttcaggccgttgtcgccgtagtccgggatcgacaccgcagtcggcgcagcgttcgccggggcggcgggctgtgcgggagcggcaggttcgagactcagcgcgtcagcagccggaggtgcagcaggagctgcgggctgtgccggtgcggccggagcgggctggccgttgggcaacagcttgtcgtctgcgggagccggagctgccggtgcgggctggttgccgttcgaggttgcgatcacggttgcgccgggaccaccgcccggaggtgcgttggaactcattgtgtctgtgtctccatgttgttggcgttgtcgatctgctgggatgcgttctgcatggcgagctgctgctgtgcacgctgctgcatcatctggccgtactcggcctcagtcagcacgtagacgttcgggtccaagccaccagcggcggcgaggtctgcgatccacgcggacagcttcagtcgttcgagaatctgcggcggcagtgcgaggacgttggcgaggttgctgccgaactccaacagccggtcacggtcacccgtacgggagagcgcggccaagccggtgatgatgacaggctccaagtccttgcctcggatgtcgcggcccgtcaggttcatcacccaaaaggcgactggtacctgcacgtccgcagcgatccgggagtagccgccacccagcccgccttccagttcttcggcgaccatgcggatttcctgcgcggtcacacgttccgcctgacgagtcaccgccgtctgcaacaggaagcctgcgccgatgcggttgatgtaggtggactggattgcttggttggtttgcagcacgccatcgacgcctgcgttaatcagctcgatgtcacccttcatgccgggaatggccgcgccattgggcgacgccatgaagtcctcgacggaggtctgacctgcggggttaaccagccaccggaactcggaggcgaggatcgcgccctgcactgcggcctcggacagcatcgagagcgactggaagtcggcctcgtagtcttcgaccaagccggagccgtagtcatcgcctgcggccaagtcccagctaaccgcccggtagggcagcttgtctgcggtgtaggtcgaggagaagttggcgggcagcttgcagttgcaaatccacacgtcttcgttgtacttgccggtcttgtggtccagcttgacccacttgtactcccacaccatgccgtcgtcatcgggcttgaagtccgggtgcgcgacaatggcagcgagcgctgcgggttccagctgggtcttgtgcaccttctcccgaaggatcagttcgtagacctcgccggtgcgggtgcgcttgaccacgtagtgccgcatgttgagcacgcggatcgtgtccttctccaacaccatgagggcgttgcccagcacgatcagcatcttcagcaggtcgtacagccgggagcggatggagcgcttgtccagttcgagactggcatcctgctcggccttcgcaagcatcgcctgcatggcctgcaagtcagcgccttgctcctgcgcagcctgcttcgccttgcgcttcagctccaaccggaagaacgggcgggacggtgcgaacagcgacatcatcagcttgttcgccagatggttcactgcctgcgcgccgagagactggaacccgtgggtcagcggctcggtgtcctgatcgcggttcttgcgagggaacagcttgggcacggtccagctcgaatagcgttcgagtcggtacatgatgccctgtcgcttgttgtcgtaagcctcgaactggcggtgagcggtttggatcggatggtccatgctcacctcacaacaggtctgacccggccacggtcgtcagccgggaagctgcggtcgtggtcacgggtcgggtgtaagtggagcgggcggtcttgcgtcggccgatcaggtcggcagtctgcaagtcgaggtcggaagttcccagccgcacatcgacggtatcgacgggggcactcagcaacttctcggcgtactcagatgcggcctgctgtgcagctgcctgtgccatctgatcggccatcgcctgaatctggtagttcgtggattgagtttggaggttggtctgcttgtcgatagcagcagcttgcttcagcgctgctcgcttggcggacccaccaccaacgatgctacccataggttaactccttcgcttggtgaattggggagcatgccgttccagcaggtagccgtagcgtgcatacatccgtgtgagtgctcgggagttccgagctagtgcaccgcctgcgctcagtgagtcgcagtggttgatgtcagccagatgttccatcacggctatgtaccggtcgaaggaactgcccggcccaattcgcagcaccatgttctcaacgaacgtagtacggttcttggagtaccacggtgtgacaatggcaaagcacagcaggtaggcttcatcaatgattactgcatccactagaccctgtgttatcagggccactgtgtaatcagggtcatcacagttgtagctcacagaagattctctgttgtctaccttactatcttctctagatgacagatacaaagcggccgttaaagccgccttgatctgctcactatcacccgtcgttggtgttcggtacggaggaatcaacggtgaaaccctcctgtaagatgttcaggacgcgggccatccccaactgcatacctgcctccaagggcgtggtattcgagttgacggacagcgacagcccggacagcttccgcacggcggccagctggttcgggtggagcgtcatcaggactttcactttggcgtcttcggccatggtgtctcctctgtgctataggtgtaccaaaaggtccggcaccggttccgcttaccttcgcggccgctccaaccggacctcagttgcctcgtgctataggtgtactgaaactccgtcagctgaagaagtacggagaatcaaggacttgccgaaggtccagctcgcccatcggcggcggctccggcaggaacgggtaggccgagtggaaggccgacagcacgtcgtgccgctcgtacatcgacacgaacacctcccggatgatccggtacagtgccgcgctgtcggcggcgtgggtgccgaagtcgtcgtgaatcatggcgaaggcgtcgatgccttcggccttggccgcgttgaccaccagcgtcaggtggcttgcgtcgaggctgtgcacgaagttcggggcgatgccgttgcggtgccgggacttcttcaccgcgtccgtgctcttgcgcagggacagcttggcgttgccgcacagcttggtgttgatgcggtgctcctcggactcccagtagacctgcaccaccgggaacccggacggcgtgatccaccggatgcggtcgtacccttggttgaggatcgacccggagccgcgctgcaaccactccatcgcgcccgctgcggcgaccacggtgtcggcgatggcctcacccatgcgcttgctcaggaagcgcgctgcggggccgtacagggccttgtcgagcgaggggaacttcccacacttcaggtagtcttcgatgatgaagtccgcccacgaggactgccgcgagccgtacggcagggtcatcacgctgcgcttcaccagcgagcgtgtgaggccgtggtcgagccacagcgtgcggtacccttcggcatcctcgtcctcgcctagcaggacggcagtcacgcggtctgccaccatctggtagatgtcattcggcagcggtgctgggatcaggttcgtcgccacgccgcctgctgcgtcgcgcagcatcgccgagaagttctgaagcccattgcacgaaccgtccatgccgactgcgatgcggctcaggaagcgatccccgaacacttgccactgctcgtactccatgcaccagctcagaaattgcagcggcttgtcggcggtcttccactcgtcgttgttcaccgggtccgcagcgaacgccatgatctggtcgtgatgctccgctacccacttcacacgatccggcagagacgccttgtcgtatccccatcggtttgctcctgtgatgcagaaccaatccttcgcgtccttagtcagcagcggcttgccatcggcgaactccaagagcgccttctgcaagtccgaaccctgcggcgacacgccggtggtctgaacgtacttgcggccacggaagtcagcgaagtacacgaagtagatgctcgggtactcggcgaacttgcgcgccaccttcattgcgttgtagaaacgattgcccttgttctgtcgcaggcgctcgtcggtgtgccagttggacatgtcgcgcttccactgcttgaactccaactcctgattgtgggacatggtttccttggtcatgtccttcgtcagccactccggcttgcgcggcttcggcagctcgccctgagaaatgatttcctccatgtcgtgcaccttggcgatggccgacacagcttccatcagtcgcttgttgatgcgccacggcacgcgctgcaatgcgttgatcgcagccatctcgttgcgcagctcggcagcgcggtactcgtcgcgggtctgagcgtaggtcttcaccatccacggattgagtcggcgcatttccttcgtgtggaatccaccgttgtcgatgtccacccagtccatcggcggctcgacgcacggcaggtagaacggcgtggcctcgatcacgaagtcgctgatctgagtaatcagcttgcgcacctcgtcggtcagcacgatcttgacgtgcgtcttggtctggaacttgcggtacgctgcgcctgcactggcagcagtctcggtgaccacgccaatctccaacatgcccagctgcgcaagctgatcgcacaggtacgcgccgacctgatcgcgctgtgcctgtccccactccacgaactcgatgccgttcttgcgtccttgcatcttcatcaccgtcatgcggtggttctcgttgacagagagcttgcggtccatgtcgttcatcaggtggtagaacagagtcggctccgcgtcggcgaactgcgtcagcaggtactcatggtacacgttgatgccaacgttcttcaacacgtcgcggtcgctgccttcgccgtgcttgtctcgcatgcaggaggtaagggcaccgcgaacggcgacgaaggccacagcctcgtaccactcgcgtgcctgttcctcggcgctgacgggctgtccacgcttgttctgacgctcgggatcgtacttggcgcgcagaagtggcacgtgcgcttgcgcacggccgattcgcggagagtcgatgtccgcacggatgcgctccgcaagcggaagcacgaaccggcgatacactgcttgggcgtaggggttgttgtccgcgccgcccttctcctcgttgcgggcgatggacttctccatgcgctccttaccgaaggcgtaggtttccagttcgagttccacttgcgagagcattgttacctccgttgctgccgcacggtgtagtcgcgcggcgggtagcgtttcaggataccgcgcatgatttccatgtgcaggtcgtggatgatgtgcggccacgcctcaccgccgatatcctcggccatgcacgtggcagcagcgccgaacaagtcggcaccgtaccgggcgcgcaccgaaacctcgacgcggcccatccatgccgaggactggctgaagtccagctccggcttctcgaaagtgatcgcgtccatcagcccctccgctcgtcaaggaacttggcgaacgcttcctgcaccttgtcgcgcagcgtctcgttcggccacagggaaccggcgtactcgccgaaaggaacgctgatgcgcagctccaccgtgtcgcgctccatgttgtgccatgcttgcacctcgacgctcacaggtctgcctccttcttgtcgtgacggatgcccttgtatcgcggctcgcgcagcaggccgtacttgctgaaggacatcgcctcgatttccacgatgcctcccacgctaggcagctcgctctcgctgtgcggcacgccgctgccaacctcctgcgtcttgccttctccgaggtcaacgacgaccgtgtacacggcgcggccggtcttctcgccgactgcttcgttgatgccgagcacacgcaggtccagcgtcagggtcggcttgatcttgacgacttcgccgttggttcccttgtcgcccttcacccacttgccgctcggcttgcgcaggatcagcccgtcgtacgcgccgccctcgcacagcagcttcgccgcttccatgctgcccagctcttggtcgatcaggaagccctgcgactcggcgtagaacaccggcgcggtgccctcggcgatggcgtggcccatgctcggcaggcggctgacgcgctcctgatacacgaggtcgctgaaaccctgctcccattcttccagcgtcacgaagtcgaacaccacgaacatcggctcggtgtactgcgtgccgtccttcttgcggaacatgccgctgacggtgggctggtcgatctgcgggtgccagtattcgccgaagtacacgccgaccgggaagaacggcgcggatgcgagagcgttctcgatgtggtgtgcgctgacgacctgctcaccggtgcgggagaacaggtcaaccacgccacgatccaccggctgcatctgcacgtcgcccaccttgatggcatgcaggcccttgttcaccgtgggcacccagtggccgcgcttgatggcgaccatgttgcagccgtcgtacttcggctgtgcgatgtactcggtgcgaagctgctcctcggtgggccgcagcttcttcttgatcttgtcctgctcgactgccttgtggacgatgtagctcatgcgtagtccctccaaatctggaacatggcgagcggcacttcgtaccacggaacgtagcgctcccagtacgtggccttgccgtcgtaccactgcacgcggaagttgcccttggtgaaggcgcggttgatcttgaagccgcgcttgcgcttcttgtagccgggagcaacccggacattctggcgaggcacatcaaacatcggcgctgtcctccttcttggtgccgtcacccagcgcggcgttgaaccgtgcgatgcgggacgacatgaactggttgacgatggtgccgatccacagcttgcgcggagcgagcgaaccacggtagccttcccacgcatcggcgatgcgggtatacagctcggcctgatcttcgtcgggcaggttcgggaacccggccttgaccgcattctgcaatgcctcctcgtggtcggcactctcgccccacgcaacggcgttctcgtaggacttgatgagcatggcggtctggttcttgtagagcattcagttctccttcgacgggaatggaacgaaacctgcgaggcccctcatcacgaggatgcagaatgcgtcgtcagggtatgtacgatgccagagtgagttggcccactcgacatcgaactgcttgcgggtacggtgctcctctaggaagcgcgcccactcggcctcatgtgggacgtaccgatgcacttggccgcagcgggcgcaggccatcagtcacccttgctgaaccagcggcggatgatgtactggcggatgaagctgatcgctgtgaacgcaatgccgatggcgtgcgccgacagcagcggatgctcgggatgccacagcaccggaagcagcgcgatgttcgctgcgtagttgatgctgtagccgatgccgatgttcacccaagcctctttgatggagcgcgccttactctgcgccactggccttctcctcctcgcgcagttccagctccaacaggaacagctcgttgatgatgtggtgcgcccggtggtggatgcccgtctccgggtccagcttctcgccgaggcagcgcttgttgtcgtgtcggtagctcgcgtcctgataccgttcgagcgccttctcgacatgctgccacgagtgcgctttgtacttctgcgcgccgaaggtcagggtgtcgatgactcgggccagtgcacgcggcacgccctcatgcagcagacgggcctgcggcttgcccccgtcatccttcaggccgacgccacggtcggacagtgtgcgacggtcctcgtcgcggtagctcagttcgggcattggtacctctcgtctggtggtggtcacgcctccgatgctgagaagctgtcggagggaatcgggaacgcagcagctcggcttaactcgaccgtcgaagaagacctcgacatcacgagcgaacacgcggcttacctgtccacgcagcccgatcattgcgggcgcattgccgatgtactgtacccgcatgccgctgcggatgtcggtgatcttcatgtcggttccttatgccgggacggtgatgtgcttgcgcgcctcggcgctggtcgtgagcttgcgcccacggctgtagccgtcgcacacggtgcactgaagcaggaggtaggtaccgacctgcgtgcgggccggatcatcctgcgggatcatttcgttgcagccgcacttgttgcagcggtgctcgctgccgtcggccttgtagtacactgcgacgttcggatgctgcgagtaccaaccgcgcagcttcttgtactccaacttcatggacttcacgtcgatgcggttgtacgcttcgcactcgtcccatgctccgggcaggctctgcatgcaggccacccacaggtcgaagccggggaagttgtggtggtcgtacttgcgcagctccggcacgatcacgccggtggtgtactccaacttctgcgaggtgaaggcgaactcggtgcggttcagcagcatcgggtcgatcacctgcaccggagacacgggcggcaggccgaggattgcgaggcgagccttgatcttgcgaaggtcgaacttcttgccgttgcgagcgagcacgaagtcggcggcgttgagcagtgcccacagcgccttgccctgcttgcgatcatcgaacacgtcgcgcacgttgcgctggtccatgtagaacgacgcctcgtcgtccagccattcgcaagcgaacgacatcagcgaccagtcacgcttgatctgcttgacgctgaagttgttgttgaacatgccccagccatagaactcgatggggaacgtctcgatgtcgaggcagagaatcttcgggccgcgcttcggtgctcggcgaatgaactgggtaagggtcacggtgtctccttgttgatagcccgacgctttcgcgctttcgcattgcgagcgatacgcttctcgtcgtcggtcttgtaggtaggatgcaggtaccccgtgatgttggtgaggtgcgaccgcaggtagttggggatgcccgcacagaatgcgaacacgtcgcgcacgccgtaccggcctgcgttgttctcgaccttgccgagcagggagttgcatccgcgatggagcaccccgcgcacagcgccggtcttgtggtcatggtccagcaccggatcgagcggagccttcaggccgaactgtccctgacagagacagcaccggttgccttgctccgctgcgagcttgatgcgcagcagcttgacctgtgttgcagtgagtcgcttcatgctttgtatgcctccaagattgcacgcttctcgttcacgtcctcggcgaggtcatagaacgcctgcttcagcttcggcccgaacacgtcgagcttcagcacgtcgagcagttctgcgtcacgatccgtccgcatccacagcagcacggcttgctcggcgaatgtcttgcgccagtcggcacccaacacttcgctgtacttgccgctcacgatctgcaccgcttcgaggttggtcttcgtctcgaacagcagctgctccgctgtcaccttgcccaccttcggcagacccggtatgttgtcggcggtgtcgccgtggagcatctgcatccagaaccacttgtgaccgtactgcaatccgttctcgccaacgatgtcgtaagcgccgagcggaacctctgtgatgtcgtagccgtcccagtctacgtgcacgccgcagaacattcgcatgtccttgtcggcgctgtgcaccacgtgcaggatgttgtggtgcaatgctgcaccctcgttgacgtacgcgatgccatcgtcggcctcacgggtcagccagattttgggagtgaaagcgtcgccctcgtatgtctccatccactcacgaaggaacgcccagttgttgggcttgcggcctgcttggcgctgaccctgatacggctgcgtggtagcagcgaggaagcgatcacccttggtagacgcggcgtgcgtcaggtgcatgacgatcttgcccgctccgctgacatgcttcagctgtgcgcagcgggagagcacgttgcgtcgtgcatcccccgccgagcagttctcgctaccagccgcgaagtacgccatgtagtccccatcaacgtgagcgatcacgcgcgggttgtgctgacgtaccacctgcaccggcatcggggagcgctcaccggccgctgccatgagagcgctcaggtccatcaggcgatgcctgccatcgggtcgctaccgtccaccgggaacggcggcttgtcgtcggccggagcagcgtcggtgggcgcggcgttcgccacgtcgccgaccacttcgtccagcgcatcgacgccttccttggtgaccgtggtgctgcccgccaacttggcggcggcgtagtcgtagcacggaagacccttgaagttcagcgccgcagcgatgcgcagctgcgtcttgttcttcgactgcgcctcgtgggtgaccttgccggtcttctcgtccttgcgctccgggtactcgccggggatgtagatgctgtcccacatgtcggcgtcggcgaagtcccacacgaacgcacccagcggggtgatctgctgcggcaccgggatcacggtgtccacgaacttgccggtcgggatgccgttctccatttccggcaccggcatgaccggcttgcggatggaagccttgtcgatttcggcgaaggtcttgttcgggtcgcgcttgcccggcttgtggatgacttccagcagcacaccctgacccagcagctgcacgaagtggcgctcctcggtgcgcaggcggctgaagattttgaagtagtgcgccttctcgttggtggacaggccgagggtcagcgtcatgcgcaccggcaccggaccattgtcggtttcgatgtgcgggtgctgcttaccggtcagctcgaacacgatggcgacttcatcctgcgtcttcttcttgccctcgaactcgaactcgtgcttgcccagctcgtagtacccgacgatgcgggcggtggtcacaccggcagcgggcggggtgtagtcgaagctgccaccactggcgaccgactgatccttaccctgcgtggcgaccttgttcaacagtgcgtcaagactcatgcgtgttgttctccttattcaaacgacgggttgtgattacctacgaagtccttgcggatcgacgcgcggtactcgatgaccagaccggcgaactctgcgggagggttcttctcctccatcatgttgtcgcccatcttggtttcacacgggacgccaagcggcagcgtccagttgaaccaccactccatatacaccgacgcttccagcatcgaggcgtgcagcagagcagcggccttggttgcgatgtcgccgtgtgcatccacgtagacggcatcgtgcacctgattcacgagcaacgcacggcccaaccattccttcggttcggtcacgtacttccggtagaaggcgcgcaggctgacgtacatcgccgccttggcccattcaccaccggtgccttgcatcgggtagttcttgatttccgtgggcgagaacgactgcgcacagccacccttgctcgcgggcttgttggcgatgaacaccggggacggtgactcgctgaaggaatacatcttgccgtccggcgtggtccagtgcgaccggccaagctgacacgtcagcccatgcggcacgccttgctgccccgcgttgggatgcggaacgaagcgctgagtgctgacgcggttgcgcttgatgtgctcgaccatgcggtcgatgtactcgcccagctccgggtaacgctcggcctcaccgcgcaccagcgcctcgacttcttcctccgacatgccggtggtcgcagcgatcttcgccacgcccgcaccgtacgcacgctggaaggagaacaccttcgcgttgccgcgcttcttcttccacttcttgtgctcgggatgcttgtcgtccttgctcgccttcaggatgaagtcgtagtcgtacttgccttgctcaccccacgcctgctctgcacggaggcagtgcatgtcgaggccctgcttcaagtcctcgatcagctgacggcactcggtgaggattgcctgcacgtagatttcgagggaggtgtagtccgactggatgatcttgccaccccggtgccgggacacgaaggcgcgcttgatctgcgaacccttctcctccaacgtctcctcgtccagctcgcccttgctcacgttctgcaagttcggatcgctggaagacaagcggccggtaaccgtgttggtcatgttgagcttgtggtggatgatgccgtccggtcccaccagcgtgagcatgcccttctgctctccggtcttctcgtccgtcgtgatgtagtacgtggacaagtccttgtggatgtcgtcgcgtctggcaagcgccttggtgaacggcaggttgcggtagcccagcgcctcgatcacgtcggcagcggtggagtacacgccgggatcgctcttgctttcccatgcagcatcaggctcggtgtagccagggaactcgaacagcatgtcctcgttgcggaacttctgcttggtcaagtcatcgaccttcaccttcttggtcttgtactctcccttgttcttgccgctgccgtacgtggtgtagcgccagaggttgtcgaagtcctcggccggtggcgtcgccgtcgtggtaccatcgaccagcacgtagtgcacctcgtccttctgcacgtaagtcggcccaccctcggtggacatgatcggaaccttggccgtgtacttcaccttgccgccgaagatcagcgcgctcttgtggaagcggctgttccagttgaaggtcaggccctcgggcagctcggggatgaagccgttgagttcggcggtcgccgttgcaagctcgacctccaactccttcgccttcgtaagcgcccagtccttgtccacgtacatgccgttgtactcggcttcgatggtgaagcacagcgcacccatgttgaggagcgccgagcgcagaccaccacgtgcacggaaggcggcgagctgtccgaggaacatcttctcggtgttaccgatgtcgcccacgtcgtcggtgtcgttggtgccgaggaggtaatccatcagcagcgtcttgtcgatgtcgcaggtgtccacgcccgcagcccacagggacttgactgcatcgtccttcaagttgccgccgtagcgtggagccgtctcgtccatgctcgccatgtggaactcttgcgtcatgccgtgcagcaggtactccgcaagctggcagtcccacaccatgccgcct

SEQ ID NO: 3 - DNA, 44415 bp, unidentified
  source 1..44415: mol_type = genomic DNA
gataggcccggagctgtagacatcgtgagctatcgcagcagccatggccttagccacagacttgctcgcatgataggcccctagagctagcgccttgccactgccatcgaagtacggagcctcctcgacccactgctgcttaccagtagtgaccgtgagtacgccgtccttaaccacaagcaccgtcgcggacttgccaacgtgctcctcgtagccttcgcccgctttaagcgcagcgagaaccgggcgaagcactgtgaaatccccggtgacacccagcagcacagggccggtgggtgtcgatacgggcatgatcttacgcacggtgtgcttgtggtcgccctgcgtggcctgactatcggcccacaggtgcttgccgtcccatgcgatggtggtcatttgtcacccgtacaccggcgcttaccggtaccgcacacctcggccttccacgcacgcagcgcagccttgtccttgttgcacagaacggtgtccatgcggcggtcctgcgcgagcttgaccaccttgtcctgcgaggaggtggtgcccttctccccaccgaggtaggtgatgtggcagtctgcaagcagggagtcgtcagggaccggcaggttcgcgcaggaggtcagcgacatcagcaggaacagtgccatcccggtactccggggcagcgtcaagaacttcttcagtgcgaacacgcacgtcctccttctctttgatgtaggtcgcgtacccggtagcctgcgtctgcgccgccttggcggtagcggtcgtgccgacttgggcagtttccagcttctccaccttgcgttgcaggccgtagacgtacagaccgaagcacacgaacatggtcacgaccagcagcaagccaaccagcttgccgccgagccgcgcgatcacttcacttggggtttccacggttggatcacctcgttgttggggcgcaagcacagagcaaactctgcgtcgcggcgcttggggatgccggagcaacggctgctggacagtcggcagtcgagcttaccgacgtagacccagcgcaggaactccttgcagctaccttcacgatcccctgcgttcgctttgcgcagcatggtgctgtcggcgaacgccttctcacctacgttgaacacgaagtctgtgtaggcgtcgatctggttgcggttaacgggggccttcaggtgcttgcgcacgccctgctgggcgatctgtaggtcttcgatcagccacttgtcgcactgtgccttcgttgccgtcatgcccatcgctacgcccttggtgtggccgtagcagatggtcggcacccggccggtgtcgaggtacgcagcgtagcgtaccccttcgtggccttgggtgaatgacagcagcgttgccgaaatgccgatgaagatgccgccgatcaggccgaacagccccttgttgctggtatcttggttctgctgctggttcatggttgctccttacggggtcagtgggtcgtcatccgggtccagatcgaccggagtgtgcgggccggagttcggacccgaggacgcggtgcgtgcgcccgcagcgatcagggcgtccagcacgagggtggcgtccttctggaactgcgcgagcagctgcgctgcggttgcgggatgctgctctgcgtgctccatgagggcgagcagttcgcggtgcaggtagttgccacggccgaacagacccgtgtagttgctggtgaagtcggacttctgcattggttacctccggtaacggtcgagtagggatggacggccacgttgcagcggactcttgcgggtcgctgccttcatgccggtcggatcgttgatccagtcttggaactctcgctgctgctgcttggcgatggccttgttctggtccagtgcaagctgcgcaacccagtgacgcacgctaccttccagtgcatcgagccggtcatcgtgtgcgatgctgcccttctgctgcgtgatcttcgccatctggtggaacaggctgtagacctgacgcttgccgctggtggcgtagcgctgggtgtactcgtgatccatttcaaccacggattccagcatgaccagcgagccgcgagccatgacaggttcgagagtgccgatgatacgggcttccttgttgccggtcacgaactcctcgcggatgtcgcccttgtatcccttctccgtgccgcgatcttctcgcaggacaggcaggaacaccttggcgaacgcgccgtagcccatgttcttttcgatgctgatgacgttcggcttgtacttcaccgcaatgcggcgcagttctagcaagccatcaccgtcgtagccaccgggcacagctcccacggccaacacgtacacggtggagttgaggaaggcggtcacggcgaaggccgtctcgtctccgttggcaccaccaccggccgggtcgatctgcatgtgcacgccctgcacgggggcagtctcggtgctcatgtcgtgcggcatcatcatcacgaagccgtacccactggactggaagctgcgctggtgagcgttgctcaggccacgggtgatcgtcagcgggaagcggtcgccaccaccggggatcacgatcaggttctcggtcttcagcgggaagcgcagcgcatccatcagccgcgtgttgagcatgtagttcagctgatagctggacggtccacgctgacgcagctcggactggtgcttctgctcaccggccaacagctcgtcggtgcactggccctcgtcgcccatcgggccaccaccgaacgccaacatcgggtcggcttctaggcgctgcacgatagacggtgccagatgcgggccgtagtgctcgcgctgtgccggggtcgggtagcgaccgggccagatgcgaacgtcgtagccacgtccgggcagggtgttgtagatggagtcgccggtctgcggcgtgccgaggtacaggatgcgacccggagtaccgggcttgccggtgcagatggccgagaactccaacgtgatggtcagcagcagctcacggttcgcggcagtgcggctgttcttgttggactccacgtcgtcggcgatcagcaggtccgcacgcttacccggcaggttgccggtgacgccgatgcacgccacgctcggggacttgtcgattcccttcagcgagtggtgcacgtcgaacgcatccacggaggtacggtcgcccgcgttcttgtccgggcggatgcactccaacgtcggcaccgtgaggatgatgcgctgaatcagcgtagcaatctcggatgcctgcgtgccgcctgccgatacgatcagcacacggtgagtgggatcgtggatcaggcagaagacggcgtagatggcagcgatggtggacttcgcctcgcctcgctgcgcctgcaccattgcgaggtgcgggccatactgcatgtagttggcgatgtcgtactgcatccacgtcggctcgaaccccagcaccttcataatgtcgcgcatgaaggtggcgaagtgccggtagtggttctgcaacagctccaacttcttgcggcgcacgtcggccgcttcagctgattcacgcattgttggctacgctccccggaaagtgaacgatgttgtcgagtgcacgctgcaactcgtcgtcgtcagccggaggcagcgagtgcttgcccagctcgtcttccagctcgccgagtgccttgttggcctcgcgcgtcgccgtgatgttgttgtccttcaggaacttgatcgccgcattgatgtcggctgcggtgcacagctcgccatcttggatgcgctgcatcagcgcacgcgcgaccagttcgtgcagcgcaccgagtgcgccctcacttgccggattcgacatccttgcctcccatgatctttcggtgctcgcgtgcccgccagtagaactgagcgacggcgtacagaatggcgagcgtagttacgatggcagcaccgtacgtgctgatgaagttgaggtagaccgcgccgagcgtaagcggcgaggttcggacgacctcattgaccacactcggcggggtcatgctgttctcctgtaggttagggccagtcgtcgggattgccgacgagcttccattgcaggcggttgacgttgttcatgcccaccgcaatcaggtcgccggggattcccgaggcgatcacatgttcggttgcgaagcgctcacgctgcgcgcgtacgcacaggttgctgccgttcttgtacgacaggagcacgtcgctctgcgtggcgaagacagcccgcttctcgtccatgcacaggcgcggagtggtagcaccggggatcaccatggtctgcatcgaagcagccaccgtgtcgtaccagtagaacttgcacacaccgcccgccatgtacgccacgtgcgggcgcatggtctggtcgaaggccagtgcgatctgcgtgatcccggagtcggtcagcacggtgaccggggcaacgccgtcgcggtaaacgacgacgctgctgccgtcactctcggcagtccacagcgcagcttggaggtcgtccactgctgcgttgagagtcagcccgccctgctcgaagtcaatgagcgggcgggtgcgccgattctgctgctccacccagtcaccgcgttggatgctttgggagacagtggggatcatggcgtgtaccggctccaagaaacccgcatgcgcaagttcgccgtctccgatccggtcttggtgatacccggattgaagccgacttggaaggtcacgcacgcggagagtcccattgcagccgtgatcggaccaccgggcacgttgttgatcgacatccggcaaacgcagtcacggtagtaagtacccggaacataggctacctgctgaagctgcaagtcagagaagctggcaatcgtccccggcggatactggtcggtgatagctccggtgccgtcgccagtaccgccgtagaagtagtagcacccccacacgtagtccgaccaagcgactgccgactgaccgttcataccgccgctgcggcccattgcaataggcttacaggtaacagtggtgctaacacccttgatcgtctcagtagtgacaaccggcgtggtatctgcgtacatgcgcagctcgtaagtaaccacgaggatttcatccgacagcaccgtgatggtggtcgggttacctgcggagtccttgataagcgcacgggtggtcaggatgtacgcgccggtattgttgttgtatgctttggcaccaagctccgacagaacgccagtagcggtaccagccgggaactggtactggcagcgggagtaggcgtagtacggggcagtggtagtcccaccgctgtccgaggacgtacgaccaacctgcgccacctgtgcaccaagagcggtatcggtgaatgccggggtggcgctgccactaccgactgccaagtaagcaatgaggtcgtacatgctgcgaggatagccgctgccggtatcacccagtgcgtccataccaccgtccgtgataaggttgctctgccagtcggctacaacttcgagagtatcgagggacttacccttgctgatggtgaacacgccagcaatgccgaggtgattgtggatcatgcgaagctccatgatacgaagccagaccggagtcgtgcagtcgcgtcgagcggctggttgactacagggtgctgcttcagggtgaaggaatggaaagaactcgacagcttcgccgtctccgggtcaggcgtgtagtccttacggatggatcggatgtcgaacgaaacgaaagcgctcccgtacaacgtgctctccgggtcggcggcataatcctgcctagagcttcggagttcccagcttacgaaggaggaacccagcgacgcagtatccaaaggctggagcatgtcgatgttgctgtacccagcaaagctgctggtcagcatcgcggcatcgaactggtagaagctgtagagcttggacgtaacgtagatgccctgctcctcgatacgaccggaccagtaggccacacggttcaacccgtccgtgaccttgatgctaaggaagtaggagctgtcgtcgttctgacccagtacgtacttgtggttccacttaacggtgtccacccacagcggtttgttctgcttgctgcggaacgccgacagtacaacctgcacgtacttcgtgtccttgggcgcagcgccttcggcaacggactggtgccacgcaccgttgctgccggaggaaaccatgttgccccagttgcgttgcagctcggtcccatcctccttgcggtagatgatcgacacacgagcaccggccttgcccttggagcttgcgccctgctggacctcggcggtgcatcggatgtagtcgttgaccttggcagggatcagcgggttgagcaggtcgctgccgcccgtcttgatgttggcgaagcgcgcgctgtacacgccgctgtcggtgtcgtagtctgagccagtgccaatcgaccagccttcgccattcgatccaccgcccggcaaccacgtgccgtcgtcgcctgcctcgaagtcgccgttgggcacgagggtttcctcgtccacgacttcagtgaaagccgcccacttgacgacgacttccttggtgatgttgtccacccgtaccgcagcgcccgaagggagcgtcgattcgatgacctccacggtgcagcggccgactgggttgttgatggacaggcgagactcgtaagcctcgcccgccgtgtacccttccagcacgcccgtcaccgacaggccatctgcaacctcgtccgccatgagcggtcggccgtacagcctgaagtgattagccatgcttactccttagccaagtcgcccgagagcaaccacgtgttggtgtcgccgtcgatgcacgttgcagtgatgacggagttggtgccgcgagttgcggcggtgcagccgaccgggacttcgagcgtcacgcccacgtcgccagtgatgaccacagggcctgccttctgctgcacgctgaagtagctgcccgaggcgagcttggtttcaccgtcgcccacttcggggatcaggttgatgttgacggcgcaacctccggcgtacgtgcagcgcacgagtccgtactcggtagccttggcggcgtagtaagtcggaccctctgccgtgatgatcggcacccgcaggctcgcagcggtgatcggcgcaggcccggtgtagggcttggcgtaaccacgcagcacggcgaaccagatgctgccctcggcaggaaccgtggcgaagcggatgaagctgggatcggtgccgtcagcgagcgtgacctgatagtccacgtccggctgcatgccgatgccgttgacgtacacgtcgtagaagcccgcgccggatacgtccgcgcccaccatgtcgaagtcggtgtcacccacctgatcgccagtccaagcaccggaccagacgcgcggggcgacggacacgataccaccagctgccagcaactcggtgacctgcttgtagatgttctggataatctcgttcaggtccacgatcacaccgacctgctggtcgatgctaagggtggcgatgttgagtgagtcgaacatttcctgaatgatcttcaggagctggtcgttgctgaggttaaggtttgtcttgctgatgatgctaccgttaacgtagtcaacgagcatctgctgcaccggagtgctgcggtagatgtagagcttgcgcccagcggcgacggcaggcgagactcggacggtactagcgtcatcgtcttcgctcaggacttccacggtgtgcggagtccggtcggtcagcagctgagtctcctcgtccagcagtccgctcatggcgtacacgtgggacgggttgatgtagccaccggtaaagctgatctgccagtcagtggtcacgccatcggcgtcgaacacgtctgtcgcgtagcgcagctgcgggtctggaactgccatgctgcctcctgtttgctataggtgtaccaaaagggtgggccgtccttggccctgatcttactcctccttccactggctggctgcgcccttcagcagcgggatcaccatcggcagtcgcccgcccggaatcacgtcggccagattctccggcttgccagcaatgccctgagcgaagtcgttgatgactcccagcgacggcgcgaactgcccgcccaccacttccttgcggttgccgaactgcccaccggccagctgcttcagccacgtcggaccctgcgtatcggtggcgtactcgtaccagccgcccgccacgccagtgcccacgtccagcacatcgttgagcatacccgtcgccgacacgtagttcagcgtggccttgcccagcgccagaggcgacaggatgttctggtcgatggcctcgtcgcgctcctgatcgttcatcagggccacgcgggacagcacccgcagggcttgcagcggagccgccacagccatcgcagcagcgatcaggcccgccgtctgccatgcaccgtagttgcccacgtaccggcccagctgcttctgctgcgcgaccagcgagaacgtgcggtgctggaacagcagcttcagccagccgttgtgcgcccacttgccagtctcgccgatgaaggtgtcctgaagaatctgcgaggtgccacggttgatcgcgttgtagaacgccaaccatgcctgccgatccgccagcccctcgacgttgcgcgggtctactgcttccagcttaccatccgcgccccagcgcacgacctgatcctgcgtagcccgcaggcggttcagcaggttgtcgtcaatgcccatgtccttcagggcggtgtcagcttcagcaccatcacgcaggaacttcacgcccttggcgatcagcacttccgcgaagccacgctgctgcacagcaagcacggcccgctgccccgagaggatgcggttcgcatgcgctgccttctgcaccagcgaggtcaggaagcctgcgcgctcgctaccatacatcgacgcctgcgtgtccagcgagttgaacatgtgtaggtcgtaaccggcgagaccgaagccgcgaccgctgatgaactcgaagccgtcgaggatttggttgccgctgtcctcgcccttcaggatgcgcatgatttcgctgcgcatgcggggagcgatacggattgcgtcagccacaccagcagcaccaacagcggcgaggccgttgctgtactccgctgcctgattgatgcccgcgccgcccagctggatggccgaggtcagcagacgcgcattcgccagaacagtcggatcgccggtaccgaccgggcgaccaaggaactcggacatcacctgctcgaacgccttcagctccacatcgttggcaccggtcaggcgcattgcttcgcgcgccacgttgatgcctgcgtcgccgaggatgccgtgcttcgccagagcgatgtcaccagcaacacgtcccgcgtacttgcggtagttgtccatcacgcggttgtcgagatagtccatcagacggaacttaccgtcagcgtcctcgtactgcttggtcacgtcgaggtcgatacgcgccttggtgtgcttcgcaccgccacggctgtacttgcccatgaccttctgaatctcctcctcgttgagcgacatcgcccgcagagtgtcgcgcagcgtgtccgcctgcgactccgagaagacctgacccggcgcttcgatgacacccgcagccttgcgctcgatgcgttccagatacttggtagcgaacttatcgaggaagtcgtccccatacagctcgcccatcacctcgaactgatcgcgcatcgcctgacggataccctcgcgtcgcaccggaccagcagcagcgatgctgccgcccagccacgtacgggactcgtagccctccacgtcctcctccggcagacgctgtgcgcccaccgtaccggccgcgcgctgctctgctgccatgcggttgtagccacggtccaactcacgggccattgccttcactgcctcgtgcgcatccgggatgtccccgccgttgaagcgagtctcgcggtacagcttcactgcgtactcgaagtccgcgcgagccttccagcccgtggcgaagtccttgatcgcaccgataccgcgcacgtccgcacgccacaggcgataggccgcttcccactgacgcgggcgggtgcccatgaacgactcaaaccgaccatgccgatccatcgctgcggtgctgtgtcggcctgctgcaccctcgggattctccaacagggtgatcgcaagcatgcgggcaactggcgacttggacgacattagagtcgtgctcgtagcttccagcccgaagcgctgcatgatggtggacagcttcgccgcgtcgatgccgtactgcgcactgaagcgttcggagcgtgccatcacttcggcgacctgcacacgcatcgcgtcatcactgacggacttgtccagaccggtgcgctggtagaaagccttgcgctcgcggttcgacttgaagatcgagttggcgagcatgccacgcgtctgccgggtaccggcctgcgtgtcgcgcacttccgcgccgaggttgtcaccgacgaccgacatcaggcgttcgagcgcggactcctgattcttcagacccatcactcgcgcgatcttatccttcagccactcccacgcattcgggcgggtgttgcccggcgcgggcatctgacgcagcaccgcctgcacagcgcggttcgtcaggccgtaggaaatcagctcgtcagtgttggcgaggaagcctgcctgcggctggttgatgcgcgtctccatcgcagcggtggtcagcgtggagtccacactgccgatgctgttgttgatatgggtcagcagttcttccatttcctgcccgaacaccgagttgctgcgcagctcacgcagcgtggcagcgtgcagcatttcgtgcaccaccacttccggcgtgtagttccgcatcgccatcgcgtccagtccggcgttgtagccaccggccacacgcatacccggacccatgttggcaccggcgaaccacttgtcgagttccgattccggcacgatcttcaccgtgctcagccgcccgccacgcttcagcgcgttggcgatagcacgcacgtcctccgggatagaggcgttggattccagatacttcagcacgccatcgacgttaccgcccttgatacctgcggtcttccatgcgcgttccagcagcgggtcatgctgatcgacccggccacccacgctgtcgttgtaccgcccggtcgttgcgtccacgttgcccgcgtcccgtgcgagtgcaccagtggtgcctgcggtggtggtcgtctcctgcacgtcgggacgggcgaagatacggaagtcgtcaggcacgtcggccataccagcgcgcagccaatccacagcctcctgcttggcaagctggtggatgcggttgttcaccagcaccgggttggcgtcctcgcccagctcggccacagcgcgcgccttcaggtcggccgaccacgcttcgccgtaagcggcagcgttgcctgcggacaggtcgatggttgccttgtcacgaatctgcgcagccgagcgcacgcccggaatgtgcatcgcggtgcctatggtggtagcgaatgcagcgtcggtcatgaagtccgcgaagttgcggcgctcgcccatgccaaccagcgcggcgtccgtgatgacggaaccgaccgcgttctccgcagcagccgacgcgagcgacgcgcccacgcgcccttcggcaacgagtgcagccgagccgatgcccagcgccttagcgcctgcggcagtgacgccgccgatagcccagttgcccggatcggtgaagcctgccaccatgtcgtaaccgaagctaccccagccagtctgctgatccttgatgcgcatggagtggcggcgcaggaactgtcggtcgctgacgtacttcagctcgttcggcgagtacgctgcatcgcggatgtcttcgagttcgtcggcagtcatccacggcttctcccattccttcgggtcgtacttccaaccttccggaacgttctcgtcctcgcgcgcaaactggttgctgatcgcagcaccgatgccgctgtcgaacgcagcgccccacttgtcgaggaaggtcagcgagttgcgcagctcctcgtccgcgcggtcctgcgcgagcgcctgttcggtctgatccagcagcgccttgcgagcgccggtgttcagcacgtccacttcctgacgcacccaccacggcacaacctgatccgatgcacggacagcctgagccttgcctacggcctgcgcggcggtgccaccttcctgtgctacctgacccatcgacagctcggcgatgcccgcacgaatcttgccgatgtgttccttcgctgccgacgccagagcgttgcggccttcgatgggcgcacccgtccacgcatccgggatggacgcaccggaccacgtacggtcgcgcatgttcgggttgccctgccatgcggcgttgaggtctgcctgcgtggtggtcaggctgcgcggctgcgccgacactgcgggagcggacgcaccgcccagcacgctcggtgcataggctgcgttctcctgcccccagttcttcggattggtgccgccttggtagatgcgcagcgccttcgtcacgtcgcccttggcaagctgcatgttctcgcgcatgatgtcggcatacagctcgatgctgtcttggaagttgcgcatgtcgtacttgcgaccgttgcgcgcttcccacgttgcctgcgtggtgggcatgacttggaagtcgccctgtgctcctgccttgctgcggatcacaccgtcagcgtccttggcggcacgcccgttgccggactctactcgccactgaccgcgcacgatggactccggcactcccgcataagcggcagccttggcaatctgctggtcttgggtcagccccgaaagatcgagtgccattgtctatctccttacagtttgggttggatggaaatgctctgctgaatcgtaccgtcgttcatgcgaacgtagccctgcggtaccggggcctgcaactgacgctgctgcttggtgtgcttctcgtactcgtccttgatgtcgcgcccgtacaccggcacaaccttccagcccttctcgccaacagcgttgacgtacagcaccggctcgccgttctcgctgtccttcatgcggaacacgtcagccttcagcccggtgctcggctcgatgttgacccggcgcagtgctgcgtcgatggccttctcgatggcgggtccggtttccttcgtgtccatgaagcccagccatgcaccgacgctgccgatcactcggccttcgtcgtcgcgtccgttttcccatgcgtacttgcctgcgtcttccagaccgtaggccagcttggcgtgagtagccgcagcctgcaagccttccgcagaagtgtccagcagaccaccggtgtcagtgaccgagcggacgatggcgcgagcatacgcagcgcggccagagtcgcccagcttgttgccgaacatgccgaggtacttggggttgagcttggcgatagcttccgtaacacgagcctgagtagcctcggattccttacggctgttcgcgtcgaactgcgtcggatcgtcggtggtgatttctccacgggccacctcgtaagcaagctcgaagttcacgccaccattctccaacgcttgcagcttgttgaagaacgtgttgacgctatctccgaagtacagcgcagcggtagtcgcgccagtcagtcggccctgcacgggctgaccgttcgtgtcgatgcgtgcggcggtggtctgcttcagttccttccactgctggtacagtgcagccgctgccgtgttcggctgatcgcggagcacagcgcgcgccgtggtctggaactggtcggccacacccttcagcacagcgcctcgcccggtgttggcgttccacaccagctgcgacatggcgaccttggggttcgcggccatcgtggcattccatgcctgcaccgtgttcgcctcgatcagctccttgtccacgccggggatgttgatcgtctgcgcgtacgtgccgcgcttgaacgcttcgatgccaccacggatgtcctcctcctgcgcggccagcttctgctggtcggtcagcgcggccttggccgcagcgttacgctggttgatgacggcttcctgtgcgcggatgtgcgcgcctgcggactgtgccatgatcgaagccaactgcgtaccggagtacagcggtgcgtcgcttccagtctcggcggcgtaggtcgagttcatttcctcgatcatcgcctgcgacggcttggcaccaatgccctccgatgcgtacatggagacgagcgccatcttctcggcctgctccgggttggcatcgagccagtcggaacggtaacgatcctgcgcctgcttcacgtactgctggattcccagctgcccgtccgggtcgatggcgttcagaacgcccttgctgttgaggaacttcagcgtgtggaactcgccgcgatccgcagcgccacgatagaacgcagtgatcgcggacttgtacgactcgtccgtctggtagcgcgagggcgacagtccgtccagcagggacagctgcgcctgcgtcagcgcctcggtggccttctcgtccatgggacggttggtaccgagcatcgccgtgcgcttcgccagttcgttgaagccggtggacgccgacgagttcgcagcgtactgcgccttcaccagctcctgctgctgccatgccgtgcgctccttggtgtgcaggtccatgagggaacccgcgcgatccatgaaggtcttctgcaacaccgtgtccgcgaaaccgttgccggtcatgcgggcagtggcgaggtcgttgaactccttcgccatcgcctcgggaggaagctgacgcaactccggcatacgccgaagcaagtcgctctccatttcgttgacctgcgagagcgtgttatacatgctcgcgccaatctcgtagttggtgtctccgaagattttcttgtaccacggttcggtcgcagcaatctcgtccatggtcttaccagcgcgggcggcaacgaagccgtcccacatctgctgctgcttcagcttggcggtgttcggcgctgccagctcctgcaagaactctggcaggttgctgtccggcatcgtcataccaccagtgcttgcgaaccagtcgttgccggattgaaccggcccgacctgattcacaccagcgccttgaatgctggtgttgcccgacagtgctggggtggcgttgatgccaccctgcaatgcggactgcgtgttgaaggtaaccgtgccgatgtcagccattaccatgcacctcctgagttgcctccgctgccgctatcgaaccagccgaggccggacgtagtggtggagaagttgtcgtagttgttgccgaagttgccggtgaccttcgccccagtcacggactgcttgccggtgccgtcgttgtacccgaaggtagtggacgcccacgacttgccgccgcgatcattggactgctgccacgcctgcataccgttctgcgctgcgttgctgaaggactgagaggcaccagtgaagttgccgttgtccgcctgccacgtgccgaccgcgaagtctgccacggcctcgcctgccatcggcccaccgaagtaggtagccacggccacgccgatcagcttgcccaagcgacgcttcattgcctgcggctcgatgtgctgcgagtagtcgaactgcccgaacgaacggctcatgtccatcccgttccacgcgcgcgacatgatctgcgcagtctgcgatgcgccccgcgaggcgaggagcgagacagcgttggcctgcgtctcctgatccatttccgcctgcaaccgcaccatcgaatccatcaggtctgcggacgagccgccgacaccgacagcaccagcctgcgcctgaagtgcgccacgcgcgttcgccagttggagctgggagttaagcccagccccttggcgcgcacgcagctcctcggacagcgcttccatgttggagttgtactccttcgcggcggcgtccagttgggcgttgttcttcagggaccgcatgaaatcagcgaagccggtcttggcgacctcgctgcggttctggttgtcggtctgcgcaacggctgcacggtagttcgcacgggcaacgcgggtggtgttgttcgcttgcaggatcgtattaaccgaacccattagctaaccctccgtacattgttgaaagtctgacccgtccagctcaggccggtcacccggagcgggagccaatccttgctgcgaatctcgtaggtgcactcgcgcacttcgcgcccgacgctgatgttgagctgcccccggtacaccggttgccgcgcgatcagattgtcggagtcgccgaggatgcggccctcgaagtccgtagtggtcacattgctgttgcgggttgccaccgtggcgatcatgcctgccgtgttctccacgtccaccgtcaccttgttgagggacatgcgtccatcgagtacggcctgaccgttctggtcccgagggaacggattggtcgggatcaccagagcttcggacaccacgccgtattccagcgcaccagcagcgaggtcatcgaactggttaaggaagtcagacgcctgcgcgtagggacaacccagcaggaagtacgggctagtgctattgacggcgatgcttgcgctcgcagtctgtacgcccgtaggtgtaccaaaactcgcccagctgtcgaggcacgcatgcgagtccggctcgcccttcgggtcgaacacgtcgcacgccaccagcgacccgcgcgcagtgaacacgaggccgttcttcttgtagctgctcacgccgatgatttcgcccagcgccgggtggtaccggaacttcgaccacgcatccacgatgcgctgcccgttgttcttgttgtcctcgtaccggtacaggtagaagtcctgcgggtgctcgcgagtgcggaacatgacgaggttcggcgcagtgagcggggtgatctgcaacggagtgcccgacagccacgagtccagctcgttggacatttcgtccgtcaccgtctgctgcccgttgagcgcgcccactcgcatctggtgcaggctcgtgccttcgctgccgtactgcgcataaaagatgtagttgcccgaggtctgcgccttcgcgtcaaccgaatccttgttggcactgaacgctttaatcagcggattcttcggactgaacaccgagtcgccgctgatgccgtactgctgacggtcaccgaagatcacgaggttgccgttgtagagcgtcgcgtgccggagcacatcgccctcgctgccgtgcgcgaagatttcgatggggtcgctgtcttcgatggtgacggccgagccgcgccagaagttcaggtagtccgccgagcgtgaggcgttgacgtagttctgtgcgccgatgaccagccggtcttggaagacggacagcatcgtgatcggcttgtcgatgaaccacgggatcggcgaggtcagaccatcgcctgccactcgcgcaccgtaggccggatgctcgccgctgctcggagccagagacgtgaggcccgcaccgttgcgtgcgatgtagcctacaccgttgtagatgtagagctgcgacacgaggttgtcgatggtgcactccacgccgggcgcttcgtaccagtccaccgacccgtagccggaagtctcgccgttctccaactcagcgcgcaggtagtacgactcgtccgcgcctgcaccactcggccgcacgcgaatgaccttgccgtgccagtggaacttgacggcgtaggtcgcgtctgtaatttcctgccctgcggcgtagaaggtcgtgccgtctccctcgtcgtcaaccgtgatgtccttgaactggtcatcgtcaatgatgatcccgcccttgatgtacgttgccgacacgcctgcatcgaccagcaaatccgacagctgctccgcgatgtactccgggcgcgtctgctcagcgctcgtcacgatccactcgttgaccgcagagttgtactcgttcactcggtcgttgacgtacttctggtacgccgcgtccggctccgtgccaccgggaaggtagaacgggatgtcgctggtgtcgagcgttccggggtacgatgcggtaaccgtcttgaacgttaccgtcagcaccgtgttgtccgtccgcgtcaggttcaccgtgtacgtggtgttgtacttcccggtgcgcacccatgctgcgaggcgctggatgttcgtctgctcctgccacacgttcgtgctggtggccgaggggatcgtggtgttgcccgcgatgtagacgtagctgccgatggccgtgagcgacgatgcgcctccgctgaccagcgtgttgacccacgtgctgttctcgtacaccagagggatgaacgactcgtccgtcttgttgtagaggaacgcgaaggactcgctgcccaaggtcgaggcgtcgcgccggtacagcagcgcgtactccttgccctcctgcatgaagtcgaacacgtccatgttgcgcagctcggccgaggtgacaacggcttgggaagcagcgaaccgcgtaccacgacggcgcacgaggccgttcaccggatcggacagcacgttgatctgctcgtgcgtctgtcccggccgacgacgatgcgccggtttctgactgacaccctgaaggatgtcgggataggttccgcctgcctttgccatgttgtctccttagccggggaatgtgacgtggctgtgccacgggtgaccgctgtagttccagtaacgggaacgcagcacgtccacggatgcgcgagcgaacagcgggttcgccttgatctggcggatgtgctcggccttcaagttgatgtaactgtcatcgcgctgctgcttgatcttggcgtacttggtgttgtcgccgtcgaagtcagactggaaccgcagcaccgagtcgtcgcgcacgaacatctgcacctcgtaggggaggtcatcgaagtccagcagccgcaccagcttggcctgcacgttgtggtcgaactcgtaggtgttgcgcttgcggtcgtacagtcggcgtccgcgctgcaccacgtggccgaaccggctcgggttgcagtccagcttcagcacgtccgtggggaccatgatgtacttgctcgttgcctgcggcttcagctccacccattcggtgttgaaccacagcgagagtgaggacacgtcacggtgcacgcggtcgatcaagtcaacggcgtcgtccttgtatacgtggtcatcttccagcgtgttgagcttcgtctcgcccatcgtcttcaagcaggcgttcacgatgtcgagcttggtgatgaatgccatggtgtctcctgagaggaacaaggcagagacgccggagcgcccctgccgggatgttgcttagtccgcagccagagccagagcggccggtgcgtactcgatgtcctgcgagccgatttcgtcgtccacgaaacggacacggacgacccagcctgcggtgccacgggtgtcgtagtggacgccgacgacggtaccaacggagttggcgggcagaccggccacgccagttgcggcgacgacgcggttggaaatctcgaacggtcggtcaaagaccatgatgttgctcctgtgttggtggaagaagggcgcggtttgagttacccgaaggattcagggaccgcgcccagcggattaggcaaccttgtcgatgcggcccgcgttctcgacgcgatccagaccaacggcgaaggacatccacgagtccacgaagtagcacttcgaggcatcgctccaccacaccgaggactgcaacggcagcgcttcggcgatcagcagggccttcggcgacacggccacggcgatcagggtgctgaagtcgccgtcgtagaagtcgtcgttgtcgtcgttcgacagcaggtgaccttcgatcacggtgttcggcaggttctcgctcgacagcaccgggacgccccagccgtggaaggtcgggatgccggtcagcttgttgccgtccgaggtcaggtactcgccgttgctgatctgctcggcctgctgcaacaggtagaagatcgccgggcgcacgatcaggaccacgccatcgcgctgcggcttgaccttcttctcctcctccatgcgggagaacagtttgccgatggcggcgtacaccttggccggatcgttctcgtcaccagcggcggacagcacgacctgcgtggcaccgaagtggccctcgggcgcgcggccgttgcgggtgaagatcgactgcgtggcagcagcggccttcgcggcggcgatgctgatggtcaggtccacgaactcggcgatttcctgaccctgctcgatggcgatttccttgcgggtgtcgatgtcggtgaagatttcgtccagctgccagatgctgtgacgcgacagcagcatggtatcgacggtcaccgacgccttgctgaagtccaccggggtgccgtccggcgcgtcaccgcgcttcagcttctgaagcttggtacggccgatggccttcttggtcagggtgttggtgcccttgacctgcttgcgcgggaagaacttttccagcaccgagctggacacgtaggtgtgctcgacatcgccggtgaactgttcgaggatcagggcgttctcgttgccggactggttgacctgattcggcagaaccgggacagtcgggaagatggtgctcatgctttgtgttgctccttggtcttagtggatgacgcgcgcgttgagtgcacgcagttcttcggagtgggccgcaccacggatgcccttctcggcaaccagcttgcggtactcagcgcggtactgctccttcgtgataggagcgacgccgttgatcgacgcggcgggggcggcggcgttggtagccggtgcgcccttgacggtcgtcgcgggattggcctgtgccagagccatcaggtaacgcgcggtcgcctgagcgccgaagccaccagccgacagcgattcgcttgcctgcttcagttggtcggcgggcaggttggcccgtgcgaactgctggatcgcagcccagttctctgcgccacccacggcttcgtggacagcagcaacgttcgcggcgtgcgctgcggttgcagcggcggtgacacgagcgatgctctccttcgccagagcgaggatcggtgcggaacccttggccttgtcgccgaggacttccagcttggcttccagcagggcgaagttgcccttcgctgcttcggtcagttcgcggctgtcgatgtcgaggcccacggtgttgacgaagtattcggccgcgatgttcaggccgttgtcgccgtagtccgggatcgacaccgcagtcggcgcagcgttcgccggggcggcgggctgtgcgggagcggcaggttcgagactcagcgcgtcagcagccggaggtgcagcaggagctgcgggctgtgccggtgcggccggagcgggctggccgttgggcaacagcttgtcgtctgcgggagccggagctgccggtgcgggctggttgccgttcgaggttgcgatcacggttgcgccgggaccaccgcccggaggtgcgttggaactcattgtgtctgtgtctccatgttgttggcgttgtcgatctgctgggatgcgttctgcatggcgagctgctgctgtgcacgctgctgcatcatctggccgtactcggcctcagtcagcacgtagacgttcgggtccaagccaccagcggcggcgaggtctgcgatccacgcggacagcttcagtcgttcgagaatctgcggcggcagtgcgaggacgttggcgaggttgctgccgaactccaacagccggtcacggtcacccgtacgggagagcgcggccaagccggtgatgatgacaggctccaagtccttgcctcggatgtcgcggcccgtcaggttcatcacccaaaaggcgactggtacctgcacgtccgcagcgatccgggagtagccgccacccagcccgccttccagttcttcggcgaccatgcggatttcctgcgcggtcacacgttccgcctgacgagtcaccgccgtctgcaacaggaagcctgcgccgatgcggttgatgtaggtggactggattgcttggttggtttgcagcacgccatcgacgcctgcgttaatcagctcgatgtcacccttcatgccgggaatggccgcgccattgggcgacgccatgaagtcctcgacggaggtctgacctgcggggttaaccagccaccggaactcggaggcgaggatcgcgccctgcactgcggcctcggacagcatcgagagcgactggaagtcggcctcgtagtcttcgaccaagccggagccgtagtcatcgcctgcggccaagtcccagctaaccgcccggtagggcagcttgtctgcggtgtaggtcgaggagaagttggcgggcagcttgcagttgcaaatccacacgtcttcgttgtacttgccggtcttgtggtccagcttgacccacttgtactcccacaccatgccgtcgtcatcgggcttgaagtccgggtgcgcgacaatggcagcgagcgctgcgggttccagctgggtcttgtgcaccttctcccgaaggatcagttcgtagacctcgccggtgcgggtgcgcttgaccacgtagtgccgcatgttgagcacgcggatcgtgtccttctccaacaccatgagggcgttgcccagcacgatcagcatcttcagcaggtcgtacagccgggagcggatggagcgcttgtccagttcgagactggcatcctgctcggccttcgcaagcatcgcctgcatggcctgcaagtcagcgccttgctcctgcgcagcctgcttcgccttgcgcttcagctccaaccggaagaacgggcgggacggtgcgaacagcgacatcatcagcttgttcgccagatggttcactgcctgcgcgccgagagactggaacccgtgggtcagcggctcggtgtcctgatcgcggttcttgcgagggaacagcttgggcacggtccagctcgaatagcgttcgagtcggtacatgatgccctgtcgcttgttgtcgtaagcctcgaactggcggtgagcggtttggatcggatggtccatgctcacctcacaacaggtctgacccggccacggtcgtcagccgggaagctgcggtcgtggtcacgggtcgggtgtaagtggagcgggcggtcttgcgtcggccgatcaggtcggcagtctgcaagtcgaggtcggaagttcccagccgcacatcgacggtatcgacgggggcactcagcaacttctcggcgtactcagatgcggcctgctgtgcagctgcctgtgccatctgatcggccatcgcctgaatctggtagttcgtggattgagtttggaggttggtctgcttgtcgatagcagcagcttgcttcagcgctgctcgcttggcggacccaccaccaacgatgctacccataggttaactccttcgcttggtgaattggggagcatgccgttccagcaggtagccgtagcgtgcatacatccgtgtgagtgctcgggagttccgagctagtgcaccgcctgcgctcagtgagtcgcagtggttgatgtcagccagatgttccatcacggctatgtaccggtcgaaggaactgcccggcccaattcgcagcaccatgttctcaacgaacgtagtacggttcttggagtaccacggtgtgacaatggcaaagcacagcaggtaggcttcatcaatgattactgcatccactagaccctgtgttatcagggccactgtgtaatcagggtcatcacagttgtagctcacagaagattctctgttgtctaccttactatcttctctagatgacagatacaaagcggccgttaaagccgccttgatctgctcactatcacccgtcgttggtgttcggtacggaggaatcaacggtgaaaccctcctgtaagatgttcaggacgcgggccatccccaactgcatacctgcctccaagggcgtggtattcgagttgacggacagcgacagcccggacagcttccgcacggcggccagctggttcgggtggagcgtcatcaggactttcactttggcgtcttcggccatggtgtctcctctgtgctataggtgtaccaaaaggtccggcaccggttccgcttaccttcgcggccgctccaaccggacctcagttgcctcgtgctataggtgtactgaaactccgtcagctgaagaagtacggagaatcaaggacttgccgaaggtccagctcgcccatcggcggcggctccggcaggaacgggtaggccgagtggaaggccgacagcacgtcgtgccgctcgtacatcgacacgaacacctcccggatgatccggtacagtgccgcgctgtcggcggcgtgggtgccgaagtcgtcgtgaatcatggcgaaggcgtcgatgccttcggccttggccgcgttgaccaccagcgtcaggtggcttgcgtcgaggctgtgcacgaagttcggggcgatgccgttgcggtgccgggacttcttcaccgcgtccgtgctcttgcgcagggacagcttggcgttgccgcacagcttggtgttgatgcggtgctcctcggactcccagtagacctgcaccaccgggaacccggacggcgtgatccaccggatgcggtcgtacccttggttgaggatcgacccggagccgcgctgcaaccactccatcgcgcccgctgcggcgaccacggtgtcggcgatggcctcacccatgcgcttgctcaggaagcgcgctgcggggccgtacagggccttgtcgagcgaggggaacttcccacacttcaggtagtcttcgatgatgaagtccgcccacgaggactgccgcgagccgtacggcagggtcatcacgctgcgcttcaccagcgagcgtgtgaggccgtggtcgagccacagcgtgcggtacccttcggcatcctcgtcctcgcctagcaggacggcagtcacgcggtctgccaccatctggtagatgtcattcggcagcggtgctgggatcaggttcgtcgccacgccgcctgctgcgtcgcgcagcatcgccgagaagttctgaagcccattgcacgaaccgtccatgccgactgcgatgcggctcaggaagcgatccccgaacacttgccactgctcgtactccatgcaccagctcagaaattgcagcggcttgtcggcggtcttccactcgtcgttgttcaccgggtccgcagcgaacgccatgatctggtcgtgatgctccgctacccacttcacacgatccggcagagacgccttgtcgtatccccatcggtttgctcctgtgatgcagaaccaatccttcgcgtccttagtcagcagcggcttgccatcggcgaactccaagagcgccttctgcaagtccgaaccctgcggcgacacgccggtggtctgaacgtacttgcggccacggaagtcagcgaagtacacgaagtagatgctcgggtactcggcgaacttgcgcgccaccttcattgcgttgtagaaacgattgcccttgttctgtcgcaggcgctcgtcggtgtgccagttggacatgtcgcgcttccactgcttgaactccaactcctgattgtgggacatggtttccttggtcatgtccttcgtcagccactccggcttgcgcggcttcggcagctcgccctgagaaatgatttcctccatgtcgtgcaccttggcgatggccgacacagcttccatcagtcgcttgttgatgcgccacggcacgcgctgcaatgcgttgatcgcagccatctcgttgcgcagctcggcagcgcggtactcgtcgcgggtctgagcgtaggtcttcaccatccacggattgagtcggcgcatttccttcgtgtggaatccaccgttgtcgatgtccacccagtccatcggcggctcgacgcacggcaggtagaacggcgtggcctcgatcacgaagtcgctgatctgagtaatcagcttgcgcacctcgtcggtcagcacgatcttgacgtgcgtcttggtctggaacttgcggtacgctgcgcctgcactggcagcagtctcggtgaccacgccaatctccaacatgcccagctgcgcaagctgatcgcacaggtacgcgccgacctgatcgcgctgtgcctgtccccactccacgaactcgatgccgttcttgcgtccttgcatcttcatcaccgtcatgcggtggttctcgttgacagagagcttgcggtccatgtcgttcatcaggtggtagaacagagtcggctccgcgtcggcgaactgcgtcagcaggtactcatggtacacgttgatgccaacgttcttcaacacgtcgcggtcgctgccttcgccgtgcttgtctcgcatgcaggaggtaagggcaccgcgaacggcgacgaaggccacagcctcgtaccactcgcgtgcctgttcctcggcgctgacgggctgtccacgcttgttctgacgctcgggatcgtacttggcgcgcagaagtggcacgtgcgcttgcgcacggccgattcgcggagagtcgatgtccgcacggatgcgctccgcaagcggaagcacgaaccggcgatacactgcttgggcgtaggggttgttgtccgcgccgcccttctcctcgttgcgggcgatggacttctccatgcgctccttaccgaaggcgtaggtttccagttcgagttccacttgcgagagcattgttacctccgttgctgccgcacggtgtagtcgcgcggcgggtagcgtttcaggataccgcgcatgatttccatgtgcaggtcgtggatgatgtgcggccacgcctcaccgccgatatcctcggccatgcacgtggcagcagcgccgaacaagtcggcaccgtaccgggcgcgcaccgaaacctcgacgcggcccatccatgccgaggactggctgaagtccagctccggcttctcgaaagtgatcgcgtccatcagcccctccgctcgtcaaggaacttggcgaacgcttcctgcaccttgtcgcgcagcgtctcgttcggccacagggaaccggcgtactcgccgaaaggaacgctgatgcgcagctccaccgtgtcgcgctccatgttgtgccatgcttgcacctcgacgctcacaggtctgcctccttcttgtcgtgacggatgcccttgtatcgcggctcgcgcagcaggccgtacttgctgaaggacatcgcctcgatttccacgatgcctcccacgctaggcagctcgctctcgctgtgcggcacgccgctgccaacctcctgcgtcttgccttctccgaggtcaacgacgaccgtgtacacggcgcggccggtcttctcgccgactgcttcgttgatgccgagcacacgcaggtccagcgtcagggtcggcttgatcttgacgacttcgccgttggttcccttgtcgcccttcacccacttgccgctcggcttgcgcaggatcagcccgtcgtacgcgccgccctcgcacagcagcttcgccgcttccatgctgcccagctcttggtcgatcaggaagccctgcgactcggcgtagaacaccggcgcggtgccctcggcgatggcgtggcccatgctcggcaggcggctgacgcgctcctgatacacgaggtcgctgaaaccctgctcccattcttccagcgtcacgaagtcgaacaccacgaacatcggctcggtgtactgcgtgccgtccttcttgcggaacatgccgctgacggtgggctggtcgatctgcgggtgccagtattcgccgaagtacacgccgaccgggaagaacggcgcggatgcgagagcgttctcgatgtggtgtgcgctgacgacctgctcaccggtgcgggagaacaggtcaaccacgccacgatccaccggctgcatctgcacgtcgcccaccttgatggcatgcaggcccttgttcaccgtgggcacccagtggccgcgcttgatggcgaccatgttgcagccgtcgtacttcggctgtgcgatgtactcggtgcgaagctgctcctcggtgggccgcagcttcttcttgatcttgtcctgctcgactgccttgtggacgatgtagctcatgcgtagtccctccaaatctggaacatggcgagcggcacttcgtaccacggaacgtagcgctcccagtacgtggccttgccgtcgtaccactgcacgcggaagttgcccttggtgaaggcgcggttgatcttgaagccgcgcttgcgcttcttgtagccgggagcaacccggacattctggcgaggcacatcaaacatcggcgctgtcctccttcttggtgccgtcacccagcgcggcgttgaaccgtgcgatgcgggacgacatgaactggttgacgatggtgccgatccacagcttgcgcggagcgagcgaaccacggtagccttcccacgcatcggcgatgcgggtatacagctcggcctgatcttcgtcgggcaggttcgggaacccggccttgaccgcattctgcaatgcctcctcgtggtcggcactctcgccccacgcaacggcgttctcgtaggacttgatgagcatggcggtctggttcttgtagagcattcagttctccttcgacgggaatggaacgaaacctgcgaggcccctcatcacgaggatgcagaatgcgtcgtcagggtatgtacgatgccagagtgagttggcccactcgacatcgaactgcttgcgggtacggtgctcctctaggaagcgcgcccactcggcctcatgtgggacgtaccgatgcacttggccgcagcgggcgcaggccatcagtcacccttgctgaaccagcggcggatgatgtactggcggatgaagctgatcgctgtgaacgcaatgccgatggcgtgcgccgacagcagcggatgctcgggatgccacagcaccggaagcagcgcgatgttcgctgcgtagttgatgctgtagccgatgccgatgttcacccaagcctctttgatggagcgcgccttactctgcgccactggccttctcctcctcgcgcagttccagctccaacaggaacagctcgttgatgatgtggtgcgcccggtggtggatgcccgtctccgggtccagcttctcgccgaggcagcgcttgttgtcgtgtcggtagctcgcgtcctgataccgttcgagcgccttctcgacatgctgccacgagtgcgctttgtacttctgcgcgccgaaggtcagggtgtcgatgactcgggccagtgcacgcggcacgccctcatgcagcagacgggcctgcggcttgcccccgtcatccttcaggccgacgccacggtcggacagtgtgcgacggtcctcgtcgcggtagctcagttcgggcattggtacctctcgtctggtggtggtcacgcctccgatgctgagaagctgtcggagggaatcgggaacgcagcagctcggcttaactcgaccgtcgaagaagacctcgacatcacgagcgaacacgcggcttacctgtccacgcagcccgatcattgcgggcgcattgccgatgtactgtacccgcatgccgctgcggatgtcggtgatcttcatgtcggttccttatgccgggacggtgatgtgcttgcgcgcctcggcgctggtcgtgagcttgcgcccacggctgtagccgtcgcacacggtgcactgaagcaggaggtaggtaccgacctgcgtgcgggccggatcatcctgcgggatcatttcgttgcagccgcacttgttgcagcggtgctcgctgccgtcggccttgtagtacactgcgacgttcggatgctgcgagtaccaaccgcgcagcttcttgtactccaacttcatggacttcacgtcgatgcggttgtacgcttcgcactcgtcccatgctccgggcaggctctgcatgcaggccacccacaggtcgaagccggggaagttgtggtggtcgtacttgcgcagctccggcacgatcacgccggtggtgtactccaacttctgcgaggtgaaggcgaactcggtgcggttcagcagcatcgggtcgatcacctgcaccggagacacgggcggcaggccgaggattgcgaggcgagccttgatcttgcgaaggtcgaacttcttgccgttgcgagcgagcacgaagtcggcggcgttgagcagtgcccacagcgccttgccctgcttgcgatcatcgaacacgtcgcgcacgttgcgctggtccatgtagaacgacgcctcgtcgtccagccattcgcaagcgaacgacatcagcgaccagtcacgcttgatctgcttgacgctgaagttgttgttgaacatgccccagccatagaactcgatggggaacgtctcgatgtcgaggcagagaatcttcgggccgcgcttcggtgctcggcgaatgaactgggtaagggtcacggtgtctccttgttgatagcccgacgctttcgcgctttcgcattgcgagcgatacgcttctcgtcgtcggtcttgtaggtaggatgcaggtaccccgtgatgttggtgaggtgcgaccgcaggtagttggggatgcccgcacagaatgcgaacacgtcgcgcacgccgtaccggcctgcgttgttctcgaccttgccgagcagggagttgcatccgcgatggagcaccccgcgcacagcgccggtcttgtggtcatggtccagcaccggatcgagcggagccttcaggccgaactgtccctgacagagacagcaccggttgccttgctccgctgcgagcttgatgcgcagcagcttgacctgtgttgcagtgagtcgcttcatgctttgtatgcctccaagattgcacgcttctcgttcacgtcctcggcgaggtcatagaacgcctgcttcagcttcggcccgaacacgtcgagcttcagcacgtcgagcagttctgcgtcacgatccgtccgcatccacagcagcacggcttgctcggcgaatgtcttgcgccagtcggcacccaacacttcgctgtacttgccgctcacgatctgcaccgcttcgaggttggtcttcgtctcgaacagcagctgctccgctgtcaccttgcccaccttcggcagacccggtatgttgtcggcggtgtcgccgtggagcatctgcatccagaaccacttgtgaccgtactgcaatccgttctcgccaacgatgtcgtaagcgccgagcggaacctctgtgatgtcgtagccgtcccagtctacgtgcacgccgcagaacattcgcatgtccttgtcggcgctgtgcaccacgtgcaggatgttgtggtgcaatgctgcaccctcgttgacgtacgcgatgccatcgtcggcctcacgggtcagccagattttgggagtgaaagcgtcgccctcgtatgtctccatccactcacgaaggaacgcccagttgttgggcttgcggcctgcttggcgctgaccctgatacggctgcgtggtagcagcgaggaagcgatcacccttggtagacgcggcgtgcgtcaggtgcatgacgatcttgcccgctccgctgacatgcttcagctgtgcgcagcgggagagcacgttgcgtcgtgcatcccccgccgagcagttctcgctaccagccgcgaagtacgccatgtagtccccatcaacgtgagcgatcacgcgcgggttgtgctgacgtaccacctgcaccggcatcggggagcgctcaccggccgctgccatgagagcgctcaggtccatcaggcgatgcctgccatcgggtcgctaccgtccaccgggaacggcggcttgtcgtcggccggagcagcgtcggtgggcgcggcgttcgccacgtcgccgaccacttcgtccagcgcatcgacgccttccttggtgaccgtggtgctgcccgccaacttggcggcggcgtagtcgtagcacggaagacccttgaagttcagcgccgcagcgatgcgcagctgcgtcttgttcttcgactgcgcctcgtgggtgaccttgccggtcttctcgtccttgcgctccgggtactcgccggggatgtagatgctgtcccacatgtcggcgtcggcgaagtcccacacgaacgcacccagcggggtgatctgctgcggcaccgggatcacggtgtccacgaacttgccggtcgggatgccgttctccatttccggcaccggcatgaccggcttgcggatggaagccttgtcgatttcggcgaaggtcttgttcgggtcgcgcttgcccggcttgtggatgacttccagcagcacaccctgacccagcagctgcacgaagtggcgctcctcggtgcgcaggcggctgaagattttgaagtagtgcgccttctcgttggtggacaggccgagggtcagcgtcatgcgcaccggcaccggaccattgtcggtttcgatgtgcgggtgctgcttaccggtcagctcgaacacgatggcgacttcatcctgcgtcttcttcttgccctcgaactcgaactcgtgcttgcccagctcgtagtacccgacgatgcgggcggtggtcacaccggcagcgggcggggtgtagtcgaagctgccaccactggcgaccgactgatccttaccctgcgtggcgaccttgttcaacagtgcgtcaagactcatgcgtgttgttctccttattcaaacgacgggttgtgattacctacgaagtccttgcggatcgacgcgcggtactcgatgaccagaccggcgaactctgcgggagggttcttctcctccatcatgttgtcgcccatcttggtttcacacgggacgccaagcggcagcgtccagttgaaccaccactccatatacaccgacgcttccagcatcgaggcgtgcagcagagcagcggccttggttgcgatgtcgccgtgtgcatccacgtagacggcatcgtgcacctgattcacgagcaacgcacggcccaaccattccttcggttcggtcacgtacttccggtagaaggcgcgcaggctgacgtacatcgccgccttggcccattcaccaccggtgccttgcatcgggtagttcttgatttccgtgggcgagaacgactgcgcacagccacccttgctcgcgggcttgttggcgatgaacaccggggacggtgactcgctgaaggaatacatcttgccgtccggcgtggtccagtgcgaccggccaagctgacacgtcagcccatgcggcacgccttgctgccccgcgttgggatgcggaacgaagcgctgagtgctgacgcggttgcgcttgatgtgctcgaccatgcggtcgatgtactcgcccagctccgggtaacgctcggcctcaccgcgcaccagcgcctcgacttcttcctccgacatgccggtggtcgcagcgatcttcgccacgcccgcaccgtacgcacgctggaaggagaacaccttcgcgttgccgcgcttcttcttccacttcttgtgctcgggatgcttgtcgtccttgctcgccttcaggatgaagtcgtagtcgtacttgccttgctcaccccacgcctgctctgcacggaggcagtgcatgtcgaggccctgcttcaagtcctcgatcagctgacggcactcggtgaggattgcctgcacgtagatttcgagggaggtgtagtccgactggatgatcttgccaccccggtgccgggacacgaaggcgcgcttgatctgcgaacccttctcctccaacgtctcctcgtccagctcgcccttgctcacgttctgcaagttcggatcgctggaagacaagcggccggtaaccgtgttggtcatgttgagcttgtggtggatgatgccgtccggtcccaccagcgtgagcatgcccttctgctctccggtcttctcgtccgtcgtgatgtagtacgtggacaagtccttgtgaatgtcgtcgcgtctggcaagcgccttggtgaacggcaggttgcggtagcccagcgcctcgatcacgtcggcagcggtggagtacacgccgggatcgctcttgctttcccatgcagcatcaggctcggtgtagccagggaactcgaacagcatgtcctcgttgcggaacttctgcttggtcaagtcatcgaccttcaccttcttggtcttgtactctcccttgttcttgccgctgccgtacgtggtgtagcgccagaggttgtcgaagtcctcggccggtggcgtcgccgtcgtggtaccatcgaccagcacgtagtgcacctcgtccttctgcacgtaagtcggcccaccctcggtggacatgatcggaaccttggccgtgtacttcaccttgccgccgaagatcagcgcgctcttgtggaagcggctgttccagttgaaggtcaggccctcgggcagctcggggatgaagccgttgagttcggcggtcgccgttgcaagctcgacctccaactccttcgccttcgtaagcgcccagtccttgtccacgtacatgccgttgtactcggcttcgatggtgaagcacagcgcacccatgttgaggagcgccgagcgcagaccaccacgtgcacggaaggcggcgagctgtccgaggaacatcttctcggtgttaccgatgtcgcccacgtcgtcggtgtcgttggtgccgaggaggtaatccatcagcagcgtcttgtcgatgtcgcaggtgtccacgcccgcagcccacagggacttgactgcatcgtccttcaagttgccgccgtagcgtggagccgtctcgtccatgctcgccatgtggaactcttgcgtcatgccgtgcagcaggtactccgcaagctggcagtcccacaccatgccgccgccgtcgatgaactcgatccatgcctgccggttgagtgggccttggcagatggcgtgcaggatgtcgaacttgatgttgaacccgacgaggaactgctgcccgtaacacagctcacgcagccacccatcgggtgcgccgcccatgtactggttgtctatcccgactcgggtgtcgtagtacaggccggtgttccgtgcgtcacccttccgcttgtagccaatcgccacgatcttgttcatgtcgtagaacggattggccttgcgcttcaggatggaacggatcgtggtttcgaggtcgaaggaagtgaagctcacagcggccaccgttgcagggccagctggtacatttcatccgacgcatcgccatccaagtccagcccgtcgcgcacccaacggaacacgatgatgcggtcctgcttgtccttgatgttgcggcgcttgcagatggtggtggcctcgaccgcgcgctgataccagccggagtcggcggtcaccatgacgttgaacacgccgttgcgcagcgcataccacgtggtgctgtagtcctcgtcctcctcgtagtgtccatcggcaccggagcacagggtccatccctgatcgaccagcttttcgatggcctcgtggaagtcctgcaccagcacgaggaagtcgatgtccgtgtcggtcacgggcggctcgactgtgtagctgctgccggtgcggctggacgtgatgacgcccacgttgcgcggcaggtagatgttcggttcggtactcacggtgtgttacctccgggcttggtgatccagaacgtgaagcacgggatcagattgatgcaccagcgcttgttgtgcggcgagtagtgcacgccgatccaagtgctgtgtttgttccgcagccatccccacttccactgcggcgcgtcgttgcggccttcgatgtagcctgcgtcgtgcaccttgcgcagcagcttggcaaggtggattgcttgcgcgttgctcacgcagttgaaggtcttcgcctcggtggattcaccggggaagctgaccgacaccgtgaacccggtggctacgatgtgaattggcttgctcatgctgcctcctgatagaagcgggcacgctctgcatccatcatcacttcttcccgaacgtcacgcttgccgcctgcgcggtgcagcttgttcttcggggtgccgatgtagcggaagcgttccatcgctgggtcattgagcttgccgcccatgatgatgaagtcgcacgcaccctgcttgccggtcttgctgtccttcagtgcggactgcggcgggtactggattccctcaccctcggcgctgatctgcgaagtcgccacgcccacggcgtcgtacttcacacaccagttgcgagcggcctgatacatcgcctccaacatctgatcggtacgctgcccgccgttggtcatgccaccggtgaacgtgatgttgtcgatcatgtcgaagatgatgaagccggggttggtctgcttgatgatggcctcgacttcaccggagttgaacccgtggatgtcgtagaactgcatgcggtggatgtccccgcccatcgcatcttcgatgcgcttgcggatgctaccatccttcgcccactccaccatctcagggatggtagcgccgagcagcgactgataccaccgctgcttgatgcgcttgcccggcccctcgttgttgagccagatgccggtgcgcttctggtccggccaaacgttgtcgagctgcgtgatccagtggctggactcgctggtcaggaacgtggtcttgcctgcgtcgggacgcatggcgtagatgccgaagtcaccaccacgcagagcgcgcaggttcttcgccaacgtgggcagtcggaagtggatgccgatgtcgtgctcgtccatctgcatcagttcctcgggcgtctcctgcaccagcgggagccgcgccttgcgatccattcggtcggtgatcgtctcggccaagccgtacagctcgtcgcgcaggctgaactcagcgccgccattccactgcacgatcttgctgaccgcagtggtggcaagctccaactccaacagcttctcgatcatgccctgctctgcctcgggcgggaccggctcgcgcatctgcttcagcagaactttgagcagggacttcttgtcgtcgggctgcgtcttccacttgaactccatggcccagccatcgaacacatcgaacggcaagtccttcgtgtccgggaactccttgtagtacgcacgcaacgcatcgagcatcagcacggtcagctcgtccagcccatcacgtggtgcgctgggtaccagccggtcgaacttgccacggttggtgcacaaccgcagcagcgtggtgtcaagactcatcaggttctccttcgggttcgtacttggaatcgagctggtgataccgggtgttgcgcgtctcgaacttgcgcccgccgtccgccacatacagcaccgtcgaggtgtgcacgatgtcgcagtcgccgaggttcggatgcgcaagcacgccgccgagcgtggcacggaagccaacgacgggcgggatgatagcgcgccggtagcgcacgatgggtttgctcattgcagcttctccttgatgtagtcggtcgtgtaatacttcgggtcacgtggtgacgtgatgttcctgtagtccagaccaaacgcacgtagacgcgcagcgattactcgcgcactgtcttggccgggattgctaccgttgcttctacctctgtcgtcatcgagccacgtcgctacacgttggcctcgatcagtcagctgcttcaacactttgttgtgcagcttggtgccgagcaacgaccacgcttcggttaccagtcccaccttgtatgcactgagcgggtcttcgcacagtacgatggtgtcacctgtgcccacgccgtagcgtgcgacaagtccgtctttcggaacgtcaggtgttagccacttcggctgtctcgttgccgaccgggctgtccagtataccacgttgtcgccttcagtgatcggtagtaccacccgcccgatgcttgggcaccagtacagccgcagcttctcgatcatctgaagcgagagtcccatcttgaagaaccacaccttagcgtcgagcggccactcgcgggtgtcgtatacccgtggctctggcaactcaacagtcgcacgcactctgcgttcgctcgtctgctcggcgtggattcgtgcaagcttggcctcgatactctcgtgctcacgcttgaatcctgtgccaccgcacctgaaacagaatgcggtggacttgtcgtgctctcgtgagataagcaagggcgtaccctccccgcactcatgggccacacgtgtgcggccaccaacaggcaggcgctcggcatgtggtagccagtcgttgtcgggaagggtatcgctcatgctatcctcgcttggttattcccagacctcgaagatgtcgtggctggtggcgtacaggacggagccgttgccgtccgtgctgacgatcagacgggagccgtcttcactggtcagcttggacacgacgaacccggtgcccttcggcagcttgttggtctgccgcgtgtcgatcaggtacgcattctggccgggcttcagctcgtcgccacgcttgacgacggccacgctgggtgacggcggggcgaggctcacgactgcccgccttcgccacccgcagccttggcggcagcggcttcggcggcgaggcgctgggcctcggcaacggcggcgtcgatttcttcctgcgccttcagcacttcctcggccgacatcagcagggcgctgctgtcgatcaggttcagctcggcatccagaccttcgccggtctgcaccttcagttgcagcacgcccttgtcgttcttgccggtggcgacgatcacgccggacaggacgcgcttgttcagggcacgaccgaacaggtaggacacggcgtcgcccgccttcagcgcttcgatggcggcgctgttggcctcgacggcatccagcttggcgagcttctcgttcaggccatcgaccttggcctgcgccttggcgatgtcttccagcagctcggcgcgcttggcttcgtagtggctgacggtggtctgctcggtggtgttttcgttcgacatgtagatggttcctcttgacggttgataggatggcccgtacgtgggccagtcgtagcctacccggctcgggttactgaaagatcagctcgctgttgtacccaccgccgccattgtagaagcggcgacgcagcacgctctcctcacccagcaccagcagacggtccacgatggcgcggatggcgctcatgtactggtccaccagctcgctgtgcaagttcaggtcgaagcggatcacggtcaccgcctcgtcgtccagtgcgccggtgtccttgcggacgtacaggccacggccattggtcatggtcgcaccgccgatcagcttcacggcggcggcaatctccggctgcacgttgagcagtcggctgtcgggcacagtcacctcgacccagcttcccatgcgcaggctcatgctgcacctgccagtgcggactgcacgttgggctgcaacgatgcaccggaacgcagctcggcagcacgacgcttcatgcgggagcgcagcttgcgacgctgcttgttgttcccgccgaggctatcggccacgcgcttcagctggttgttgccgacgatgcgggtctgaccctgccccttctgcacggggaagtagtcctgccccagcatcttgcgcaggatcgggttgtcgatgggaatcagcggcacgctgacgtgcaggtgccggctggtgtccggcgcaggcggcggcgtgtcgtcgtcatcgtggcgcggcttcaccgctgcgaccaccttgtccttgacgtacttggccgcagccttgatcttgtccatgaaacccatggttacttcctcctcgttccgaagtgattgaactccaactcatgccacacgtagtacgtggtgccgagcgggtcagtgtctgccttccagttgcgctggtcgcagtagtcgttggctgcgccgaggtcatcgaacgtcagcgagaacccagtggaagccgggccggtgcggaaccggcacagcttgccgtcgtcgtcatggtactggccgacgacaacccacgggccacgacccacgatccagtacagcaggatcaggatgcgcagccagagcttacgcatagtacggctcgacacggtagcccatgttctcgccgcccagcgactcggcattgaacacggcgcgcgctgcatcgcgggtcgggaacagcacgttgtactcgctcttgttgtactcgttgccgtcgatgcgcacggtggcgctcgggtgctggttgtagcagctgacatcggagtcgctgcggtcttcggcgaaggcgtaggtgatacgccaacccagcggcttgcgcaccggcttgcggatgctctcgcccacttcgaggatgtgccagttgaagaacgacccgccgtagctgttgagcacatccgcctcggcacgcacggcggcgcggcggtcgaagatggcgagctggttcgggtacgtgccgtcacgcagcgagtccagcaggctggtggtggcacccttggtgcgcagctcggcgatcaccgcatccagttcctcttgggtcggggtgcggccggtgccattggcgacgacgccagtgatgacgccatcgttgctgttcttggggatcgagacgatgaagtataccttacgcatggtggttctcctgattgacgggtgggatttcgatttcctctatcgagtagagggtgggcaccttctcgtggtgcttgcggtggtgttcgatggcttgctcgcacgcctcgtggctggtgtgatgtccgccgaggatgtaatccccgacagccacacccttcacggtaacgagcggcagcgccttcaccacaaggcgcaggctgacctcacgcataccagcgctccacgctgtgctcatgggtcacgaactctttccactggcgcggctgctcgcacagctggatcggcttgcgctccccactacggatgcgcttgtaagttacggggatcatgcaatgtgccctcctgttgggcgtggttccaaagctacgccctcgttagaaggcgcagcggtagatcacgcgcggctcgggtgccacttcacgcggtagcggcggagacggttcggatcgttgccgacgtgcgaggcgatggcgttgcgtgcagcctgcgcagtggtgaacgtgccgctgagtccgatcacagtggacgtattccaacccagctggtgagggcgccgcgcatgcttggtgaagaactcggcggtgtagaagccgcgatccttctccgggccatcgggagtgccttcgggcaccacacggtacgcatcctcgctgatgccctgcaccttggcccgcgccttcagcatgcggtacgcagcattgcggctgcgctgcggcaggcccagctcacgcacctgcgcccagttggcgagggcgatgctgccgtggcgcagattgaactgcacgatccagcccttggtcttcgtcttgttgaccagcccggtctgcgatgcagtcagggcgacgtggcgtgcgctctggtcgtccatcaggacatccggcagcttacgcggcaggttgtcgggcattgccaggccgggcaacaccatgcggccggtcacgctgccgaggaagtccagctgcgaggcatccaacaccaccggaggcaacggagacagcaggcacgccatcacccgcgcctcgatagcagcgaagtcaagttcacgcatgccgtagcccacggtgaacgtcggcggtgcgatcaggtcgcgcagcagctgtgcctcgacatcgctgtcacggcaggccgcaatcacgtcgtcctcgaattgcaggatggcgtcacgctcgaagctctcgacaccgaagtcgcgcagctcaccgtgcagcacggcgaactcattggacagcttgcggttggagtacgggtctgcctttgcggtcagtgcacaggcgatgtgaagggccgagcgcagcagggatgcttcgcgctgggtcactcgaaggttgatcttgggttccatgttacacgttctccttcttcttggtgggcttcggcacagcgcgggcagcgttgatgacggcctgttcctcctcggtcggcacgtagccttcctcggtcgccttttccagacggcccagcagcttgtgcaggtcggcggcgaacgagaacgcctctgcgggcttctcggtcttgaagtcgtaccacgccttcgcggcggcacgttccagcacgtcggccagagcttcgccctcgactcgcttgctcttggcaaacttcatgggcgcgctcgccttggtttccttgtcgtcgttcggagccatcgggccgaactcggacaggtacaggcgcagggcttcatgcttcatgccgttgcccacggcgagacacagatcggaagcgagcgtaacgtcgccgtggatgtgtgcgtggttgatgaccgcaatcgcggcctgctgaatctggtccaccagcttggtgcgggcggtgttgatcgacttgatggcgcgcttgatgtcagcgcttccggtgatgatgtccatggtggttcccttcaggttgggtccgtgccgattgcacgacactaggccctcttgcgaaggcccagtagcttgcatttaagcgagtcggatgtcgaatgaacgcccaccgcacggcaggacgtagagcgccgacacagagccggccggatgcttcatgatggcccgattgtaggaatcgcgggcagcttccacgtagtggcgagagaacttgaaccggatcacaggtaagccctcctgtcagcggcgtggttcgcccggttcgtcccgctgttaccctcgacaacaaacacagatcgctttccggcggttccgtggcgggcttcgtagcgctcggcttggcgcttgcgctcggcaagcttgcggtcatgctccgtggtgcgcaggtccatcacgcttgccgtccgggtgaactggcagaagcggcgcttacgctgggtgcggtcgagattggcattgatcgagccttgcatgttgtgcctccattggcactggtgggaaaactaacagattgatgcgccctcagaaagccgtcgagtcggtcaatccctcattctcgattagagccgttgcatcgcctatcgtgggcgcacactgaccaccggatttgcctgcatggtcatcgcaaagggagggcgcatcaatctgctagcccttcgggctgtcaaccctactccggctagcagtgccattgtcaccgtgtggcccgtagagccttttcacgaaacgcacagtattccatgcgataggaggctcaccacctccttatgaccggcttcccaccttggcagtgggttacttcccgtggccgactctcacggcagatgggaagccctaagcgttaggcttaggtaaagcggcaccagtgttgcaagtctggtggattctatgggcctttgaaatcccagttcatccggttatccgctagtgctacgttgcagcttggcggtccacgtcaactctcggccactattggctgtggttggcacgcttcccgttacaccctacccgttagcggtagtcctacgccatccaatgtggctgctcctcagagcgtggtgccatactagcacccttgttgcatcctgtcaagcccttggctcgctcgggtctctaacccgttgggcgtcctgtcgccaccatcccaccatgtacgtcggtggtccacgtgttgcaaggcctcaaagggctatctgtgccgccttgtcaagctatccgttagaggaccatgtgcgctcctgttagtgtcttgaccggtgtcccggtctcacctcagcctcaacacccgtaatctctcacgtctagccttaccgctaggtcgctccgctgttccggtggctaccacttgccgcctatcatagctaactgctagcttagtgtcaagcgtggttcggtagctcctcgcatcccttaccagtgactcccgtgtacccttagcccacttgttggcggcgccactacggatcacgtcactcgacttgcgttgcagcttactaccattgcggccgtgtgtctactactgcttgcatcgcaagcgtcaaccgttggcctagcgggtagctaactaatcagctcgacagagtaccgatagacggtgattcaggttgagccgactgtgtgctataggtgtaccaaaaggccgaaacgatacagatggccctcgcacgcctacagctgcggttcgcatggtagcaggtagggtagcccctgtcaagccccttgcggccctcctgaagccctgtcgctgccccagtgacgccattgaaccacaccgcaccggccacgtcaacacctttcgccaagagatttattaacgattcagccaaggcagcgcggtccagccatacaggcagcaggcgcacgcccacccgcacgcccacccgcaggcacccacgcacggccacgcacacgcacgctcaggcccacgcaggcaggcacacgggtacacccacgcggaaccttgacgcgggcgcacagacgcgcacacaggcgcacacgcgggcacgcacccacgcacacccgcaggcgcgtaacgcgagggcgtacgggggcacgcgcgggagcttctattggagtgacccccgcgcatttccgaagcaaattttggtccggctacccacgtggccttactcctaagcctcgcgaactggtgcctttagcttgac

SEQ ID NO: 4 - DNA, 44415 bp, unidentified
  source 1..44415: mol_type = genomic DNA
gcgctgccttggctgaatcgttaataaatctcttggcgaaaggtgttgacgtggccggtgcggtgtggttcaatggcgtcactggggcagcgacagggcttcaggagggccgcaaggggcttgacaggggctaccctacctgctaccatgcgaaccgcagctgtaggcgtgcgagggccatctgtatcgtttcggccttttggtacacctatagcacacagtcggctcaacctgaatcaccgtctatcggtactctgtcgagctgattagttagctacccgctaggccaacggttgacgcttgcgatgcaagcagtagtagacacacggccgcaatggtagtaagctgcaacgcaagtcgagtgacgtgatccgtagtggcgccgccaacaagtgggctaagggtacacgggagtcactggtaagggatgcgaggagctaccgaaccacgcttgacactaagctagcagttagctatgataggcggcaagtggtagccaccggaacagcggagcgacctagcggtaaggctagacgtgagagattacgggtgttgaggctgaggtgagaccgggacaccggtcaagacactaacaggagcgcacatggtcctctaacggatagcttgacaaggcggcacagatagccctttgaggccttgcaacacgtggaccaccgacgtacatggtgggatggtggcgacaggacgcccaacgggttagagacccgagcgagccaagggcttgacaggatgcaacaagggtgctagtatggcaccacgctctgaggagcagccacattggatggcgtaggactaccgctaacgggtagggtgtaacgggaagcgtgccaaccacagccaatagtggccgagagttgacgtggaccgccaagctgcaacgtagcactagcggataaccggatgaactgggatttcaaaggcccatagaatccaccagacttgcaacactggtgccgctttacctaagcctaacgcttagggcttcccatctgccgtgagagtcggccacgggaagtaacccactgccaaggtgggaagccggtcataaggaggtggtgagcctcctatcgcatggaatactgtgcgtttcgtgaaaaggctctacgggccacacggtgacaatggcactgctagccggagtagggttgacagcccgaagggctagcagattgatgcgccctccctttgcgatgaccatgcaggcaaatccggtggtcagtgtgcgcccacgataggcgatgcaacggctctaatcgagaatgagggattgaccgactcgacggctttctgagggcgcatcaatctgttagttttcccaccagtgccaatggaggcacaacatgcaaggctcgatcaatgccaatctcgaccgcacccagcgtaagcgccgcttctgccagttcacccggacggcaagcgtgatggacctgcgcaccacggagcatgaccgcaagcttgccgagcgcaagcgccaagccgagcgctacgaagcccgccacggaaccgccggaaagcgatctgtgtttgttgtcgagggtaacagcgggacgaaccgggcgaaccacgccgctgacaggagggcttacctgtgatccggttcaagttctctcgccactacgtggaagctgcccgcgattcctacaatcgggccatcatgaagcatccggccggctctgtgtcggcgctctacgtcctgccgtgcggtgggcgttcattcgacatccgactcgcttaaatgcaagctactgggccttcgcaagagggcctagtgtcgtgcaatcggcacggacccaacctgaagggaaccaccatggacatcatcaccggaagcgctgacatcaagcgcgccatcaagtcgatcaacaccgcccgcaccaagctggtggaccagattcagcaggccgcgattgcggtcatcaaccacgcacacatccacggcgacgttacgctcgcttccgatctgtgtctcgccgtgggcaacggcatgaagcatgaagccctgcgcctgtacctgtccgagttcggcccgatggctccgaacgacgacaaggaaaccaaggcgagcgcgcccatgaagtttgccaagagcaagcgagtcgagggcgaagctctggccgacgtgctggaacgtgccgccgcgaaggcgtggtacgacttcaagaccgagaagcccgcagaggcgttctcgttcgccgccgacctgcacaagctgctgggccgtctggaaaaggcgaccgaggaaggctacgtgccgaccgaggaggaacaggccgtcatcaacgctgcccgcgctgtgccgaagcccaccaagaagaaggagaacgtgtaacatggaacccaagatcaaccttcgagtgacccagcgcgaagcatccctgctgcgctcggcccttcacatcgcctgtgcactgaccgcaaaggcagacccgtactccaaccgcaagctgtccaatgagttcgccgtgctgcacggtgagctgcgcgacttcggtgtcgagagcttcgagcgtgacgccatcctgcaattcgaggacgacgtgattgcggcctgccgtgacagcgatgtcgaggcacagctgctgcgcgacctgatcgcaccgccgacgttcaccgtgggctacggcatgcgtgaacttgacttcgctgctatcgaggcgcgggtgatggcgtgcctgctgtctccgttgcctccggtggtgttggatgcctcgcagctggacttcctcggcagcgtgaccggccgcatggtgttgcccggcctggcaatgcccgacaacctgccgcgtaagctgccggatgtcctgatggacgaccagagcgcacgccacgtcgccctgactgcatcgcagaccgggctggtcaacaagacgaagaccaagggctggatcgtgcagttcaatctgcgccacggcagcatcgccctcgccaactgggcgcaggtgcgtgagctgggcctgccgcagcgcagccgcaatgctgcgtaccgcatgctgaaggcgcgggccaaggtgcagggcatcagcgaggatgcgtaccgtgtggtgcccgaaggcactcccgatggcccggagaaggatcgcggcttctacaccgccgagttcttcaccaagcatgcgcggcgccctcaccagctgggttggaatacgtccactgtgatcggactcagcggcacgttcaccactgcgcaggctgcacgcaacgccatcgcctcgcacgtcggcaacgatccgaaccgtctccgccgctaccgcgtgaagtggcacccgagccgcgcgtgatctaccgctgcgccttctaacgagggcgtagctttggaaccacgcccaacaggagggcacattgcatgatccccgtaacttacaagcgcatccgtagtggggagcgcaagccgatccagctgtgcgagcagccgcgccagtggaaagagttcgtgacccatgagcacagcgtggagcgctggtatgcgtgaggtcagcctgcgccttgtggtgaaggcgctgccgctcgttaccgtgaagggtgtggctgtcggggattacatcctcggcggacatcacaccagccacgaggcgtgcgagcaagccatcgaacaccaccgcaagcaccacgagaaggtgcccaccctctactcgatagaggaaatcgaaatcccacccgtcaatcaggagaaccaccatgcgtaaggtatacttcatcgtctcgatccccaagaacagcaacgatggcgtcatcactggcgtcgtcgccaatggcaccggccgcaccccgacccaagaggaactggatgcggtgatcgccgagctgcgcaccaagggtgccaccaccagcctgctggactcgctgcgtgacggcacgtacccgaaccagctcgccatcttcgaccgccgcgccgccgtgcgtgccgaggcggatgtgctcaacagctacggcgggtcgttcttcaactggcacatcctcgaagtgggcgagagcatccgcaagccggtgcgcaagccgctgggttggcgtatcacctacgccttcgccgaagaccgcagcgactccgatgtcagctgctacaaccagcacccgagcgccaccgtgcgcatcgacggcaacgagtacaacaagagcgagtacaacgtgctgttcccgacccgcgatgcagcgcgcgccgtgttcaatgccgagtcgctgggcggcgagaacatgggctaccgtgtcgagccgtactatgcgtaagctctggctgcgcatcctgatcctgctgtactggatcgtgggtcgtggcccgtgggttgtcgtcggccagtaccatgacgacgacggcaagctgtgccggttccgcaccggcccggcttccactgggttctcgctgacgttcgatgacctcggcgcagccaacgactactgcgaccagcgcaactggaaggcagacactgacccgctcggcaccacgtactacgtgtggcatgagttggagttcaatcacttcggaacgaggaggaagtaaccatgggtttcatggacaagatcaaggctgcggccaagtacgtcaaggacaaggtggtcgcagcggtgaagccgcgccacgatgacgacgacacgccgccgcctgcgccggacaccagccggcacctgcacgtcagcgtgccgctgattcccatcgacaacccgatcctgcgcaagatgctggggcaggactacttccccgtgcagaaggggcagggtcagacccgcatcgtcggcaacaaccagctgaagcgcgtggccgatagcctcggcgggaacaacaagcagcgtcgcaagctgcgctcccgcatgaagcgtcgtgctgccgagctgcgttccggtgcatcgttgcagcccaacgtgcagtccgcactggcaggtgcagcatgagcctgcgcatgggaagctgggtcgaggtgactgtgcccgacagccgactgctcaacgtgcagccggagattgccgccgccgtgaagctgatcggcggtgcgaccatgaccaatggccgtggcctgtacgtccgcaaggacaccggcgcactggacgacgaggcggtgaccgtgatccgcttcgacctgaacttgcacagcgagctggtggaccagtacatgagcgccatccgcgccatcgtggaccgtctgctggtgctgggtgaggagagcgtgctgcgtcgccgcttctacaatggcggcggtgggtacaacagcgagctgatctttcagtaacccgagccgggtaggctacgactggcccacgtacgggccatcctatcaaccgtcaagaggaaccatctacatgtcgaacgaaaacaccaccgagcagaccaccgtcagccactacgaagccaagcgcgccgagctgctggaagacatcgccaaggcgcaggccaaggtcgatggcctgaacgagaagctcgccaagctggatgccgtcgaggccaacagcgccgccatcgaagcgctgaaggcgggcgacgccgtgtcctacctgttcggtcgtgccctgaacaagcgcgtcctgtccggcgtgatcgtcgccaccggcaagaacgacaagggcgtgctgcaactgaaggtgcagaccggcgaaggtctggatgccgagctgaacctgatcgacagcagcgccctgctgatgtcggccgaggaagtgctgaaggcgcaggaagaaatcgacgccgccgttgccgaggcccagcgcctcgccgccgaagccgctgccgccaaggctgcgggtggcgaaggcgggcagtcgtgagcctcgccccgccgtcacccagcgtggccgtcgtcaagcgtggcgacgagctgaagcccggccagaatgcgtacctgatcgacacgcggcagaccaacaagctgccgaagggcaccgggttcgtcgtgtccaagctgaccagtgaagacggctcccgtctgatcgtcagcacggacggcaacggctccgtcctgtacgccaccagccacgacatcttcgaggtctgggaataaccaagcgaggatagcatgagcgatacccttcccgacaacgactggctaccacatgccgagcgcctgcctgttggtggccgcacacgtgtggcccatgagtgcggggagggtacgcccttgcttatctcacgagagcacgacaagtccaccgcattctgtttcaggtgcggtggcacaggattcaagcgtgagcacgagagtatcgaggccaagcttgcacgaatccacgccgagcagacgagcgaacgcagagtgcgtgcgactgttgagttgccagagccacgggtatacgacacccgcgagtggccgctcgacgctaaggtgtggttcttcaagatgggactctcgcttcagatgatcgagaagctgcggctgtactggtgcccaagcatcgggcgggtggtactaccgatcactgaaggcgacaacgtggtatactggacagcccggtcggcaacgagacagccgaagtggctaacacctgacgttccgaaagacggacttgtcgcacgctacggcgtgggcacaggtgacaccatcgtactgtgcgaagacccgctcagtgcatacaaggtgggactggtaaccgaagcgtggtcgttgctcggcaccaagctgcacaacaaagtgttgaagcagctgactgatcgaggccaacgtgtagcgacgtggctcgatgacgacagaggtagaagcaacggtagcaatcccggccaagacagtgcgcgagtaatcgctgcgcgtctacgtgcgtttggtctggactacaggaacatcacgtcaccacgtgacccgaagtattacacgaccgactacatcaaggagaagctgcaatgagcaaacccatcgtgcgctaccggcgcgctatcatcccgcccgtcgttggcttccgtgccacgctcggcggcgtgcttgcgcatccgaacctcggcgactgcgacatcgtgcacacctcgacggtgctgtatgtggcggacggcgggcgcaagttcgagacgcgcaacacccggtatcaccagctcgattccaagtacgaacccgaaggagaacctgatgagtcttgacaccacgctgctgcggttgtgcaccaaccgtggcaagttcgaccggctggtacccagcgcaccacgtgatgggctggacgagctgaccgtgctgatgctcgatgcgttgcgtgcgtactacaaggagttcccggacacgaaggacttgccgttcgatgtgttcgatggctgggccatggagttcaagtggaagacgcagcccgacgacaagaagtccctgctcaaagttctgctgaagcagatgcgcgagccggtcccgcccgaggcagagcagggcatgatcgagaagctgttggagttggagcttgccaccactgcggtcagcaagatcgtgcagtggaatggcggcgctgagttcagcctgcgcgacgagctgtacggcttggccgagacgatcaccgaccgaatggatcgcaaggcgcggctcccgctggtgcaggagacgcccgaggaactgatgcagatggacgagcacgacatcggcatccacttccgactgcccacgttggcgaagaacctgcgcgctctgcgtggtggtgacttcggcatctacgccatgcgtcccgacgcaggcaagaccacgttcctgaccagcgagtccagccactggatcacgcagctcgacaacgtttggccggaccagaagcgcaccggcatctggctcaacaacgaggggccgggcaagcgcatcaagcagcggtggtatcagtcgctgctcggcgctaccatccctgagatggtggagtgggcgaaggatggtagcatccgcaagcgcatcgaagatgcgatgggcggggacatccaccgcatgcagttctacgacatccacgggttcaactccggtgaagtcgaggccatcatcaagcagaccaaccccggcttcatcatcttcgacatgatcgacaacatcacgttcaccggtggcatgaccaacggcgggcagcgtaccgatcagatgttggaggcgatgtatcaggccgctcgcaactggtgtgtgaagtacgacgccgtgggcgtggcgacttcgcagatcagcgccgagggtgagggaatccagtacccgccgcagtccgcactgaaggacagcaagaccggcaagcagggtgcgtgcgacttcatcatcatgggcggcaagctcaatgacccagcgatggaacgcttccgctacatcggcaccccgaagaacaagctgcaccgcgcaggcggcaagcgtgacgttcgggaagaagtgatgatggatgcagagcgtgcccgcttctatcaggaggcagcatgagcaagccaattcacatcgtagccaccgggttcacggtgtcggtcagcttccccggtgaatccaccgaggcgaagaccttcaactgcgtgagcaacgcgcaagcaatccaccttgccaagctgctgcgcaaggtgcacgacgcaggctacatcgaaggccgcaacgacgcgccgcagtggaagtggggatggctgcggaacaaacacagcacttggatcggcgtgcactactcgccgcacaacaagcgctggtgcatcaatctgatcccgtgcttcacgttctggatcaccaagcccggaggtaacacaccgtgagtaccgaaccgaacatctacctgccgcgcaacgtgggcgtcatcacgtccagccgcaccggcagcagctacacagtcgagccgcccgtgaccgacacggacatcgacttcctcgtgctggtgcaggacttccacgaggccatcgaaaagctggtcgatcagggatggaccctgtgctccggtgccgatggacactacgaggaggacgaggactacagcaccacgtggtatgcgctgcgcaacggcgtgttcaacgtcatggtgaccgccgactccggctggtatcagcgcgcggtcgaggccaccaccatctgcaagcgccgcaacatcaaggacaagcaggaccgcatcatcgtgttccgttgggtgcgcgacgggctggacttggatggcgatgcgtcggatgaaatgtaccagctggccctgcaacggtggccgctgtgagcttcacttccttcgacctcgaaaccacgatccgttccatcctgaagcgcaaggccaatccgttctacgacatgaacaagatcgtggcgattggctacaagcggaagggtgacgcacggaacaccggcctgtactacgacacccgagtcgggatagacaaccagtacatgggcggcgcacccgatgggtggctgcgtgagctgtgttacgggcagcagttcctcgtcgggttcaacatcaagttcgacatcctgcacgccatctgccaaggcccactcaaccggcaggcatggatcgagttcatcgacggcggcggcatggtgtgggactgccagcttgcggagtacctgctgcacggcatgacgcaagagttccacatggcgagcatggacgagacggctccacgctacggcggcaacttgaaggacgatgcagtcaagtccctgtgggctgcgggcgtggacacctgcgacatcgacaagacgctgctgatggattacctcctcggcaccaacgacaccgacgacgtgggcgacatcggtaacaccgagaagatgttcctcggacagctcgccgccttccgtgcacgtggtggtctgcgctcggcgctcctcaacatgggtgcgctgtgcttcaccatcgaagccgagtacaacggcatgtacgtggacaaggactgggcgcttacgaaggcgaaggagttggaggtcgagcttgcaacggcgaccgccgaactcaacggcttcatccccgagctgcccgagggcctgaccttcaactggaacagccgcttccacaagagcgcgctgatcttcggcggcaaggtgaagtacacggccaaggttccgatcatgtccaccgagggtgggccgacttacgtgcagaaggacgaggtgcactacgtgctggtcgatggtaccacgacggcgacgccaccggccgaggacttcgacaacctctggcgctacaccacgtacggcagcggcaagaacaagggagagtacaagaccaagaaggtgaaggtcgatgacttgaccaagcagaagttccgcaacgaggacatgctgttcgagttccctggctacaccgagcctgatgctgcatgggaaagcaagagcgatcccggcgtgtactccaccgctgccgacgtgatcgaggcgctgggctaccgcaacctgccgttcaccaaggcgcttgccagacgcgacgacatccacaaggacttgtccacgtactacatcacgacggacgagaagaccggagagcagaagggcatgctcacgctggtgggaccggacggcatcatccaccacaagctcaacatgaccaacacggttaccggccgcttgtcttccagcgatccgaacttgcagaacgtgagcaagggcgagctggacgaggagacgttggaggagaagggttcgcagatcaagcgcgccttcgtgtcccggcaccggggtggcaagatcatccagtcggactacacctccctcgaaatctacgtgcaggcaatcctcaccgagtgccgtcagctgatcgaggacttgaagcagggcctcgacatgcactgcctccgtgcagagcaggcgtggggtgagcaaggcaagtacgactacgacttcatcctgaaggcgagcaaggacgacaagcatcccgagcacaagaagtggaagaagaagcgcggcaacgcgaaggtgttctccttccagcgtgcgtacggtgcgggcgtggcgaagatcgctgcgaccaccggcatgtcggaggaagaagtcgaggcgctggtgcgcggtgaggccgagcgttacccggagctgggcgagtacatcgaccgcatggtcgagcacatcaagcgcaaccgcgtcagcactcagcgcttcgttccgcatcccaacgcggggcagcaaggcgtgccgcatgggctgacgtgtcagcttggccggtcgcactggaccacgccggacggcaagatgtattccttcagcgagtcaccgtccccggtgttcatcgccaacaagcccgcgagcaagggtggctgtgcgcagtcgttctcgcccacggaaatcaagaactacccgatgcaaggcaccggtggtgaatgggccaaggcggcgatgtacgtcagcctgcgcgccttctaccggaagtacgtgaccgaaccgaaggaatggttgggccgtgcgttgctcgtgaatcaggtgcacgatgccgtctacgtggatgcacacggcgacatcgcaaccaaggccgctgctctgctgcacgcctcgatgctggaagcgtcggtgtatatggagtggtggttcaactggacgctgccgcttggcgtcccgtgtgaaaccaagatgggcgacaacatgatggaggagaagaaccctcccgcagagttcgccggtctggtcatcgagtaccgcgcgtcgatccgcaaggacttcgtaggtaatcacaacccgtcgtttgaataaggagaacaacacgcatgagtcttgacgcactgttgaacaaggtcgccacgcagggtaaggatcagtcggtcgccagtggtggcagcttcgactacaccccgcccgctgccggtgtgaccaccgcccgcatcgtcgggtactacgagctgggcaagcacgagttcgagttcgagggcaagaagaagacgcaggatgaagtcgccatcgtgttcgagctgaccggtaagcagcacccgcacatcgaaaccgacaatggtccggtgccggtgcgcatgacgctgaccctcggcctgtccaccaacgagaaggcgcactacttcaaaatcttcagccgcctgcgcaccgaggagcgccacttcgtgcagctgctgggtcagggtgtgctgctggaagtcatccacaagccgggcaagcgcgacccgaacaagaccttcgccgaaatcgacaaggcttccatccgcaagccggtcatgccggtgccggaaatggagaacggcatcccgaccggcaagttcgtggacaccgtgatcccggtgccgcagcagatcaccccgctgggtgcgttcgtgtgggacttcgccgacgccgacatgtgggacagcatctacatccccggcgagtacccggagcgcaaggacgagaagaccggcaaggtcacccacgaggcgcagtcgaagaacaagacgcagctgcgcatcgctgcggcgctgaacttcaagggtcttccgtgctacgactacgccgccgccaagttggcgggcagcaccacggtcaccaaggaaggcgtcgatgcgctggacgaagtggtcggcgacgtggcgaacgccgcgcccaccgacgctgctccggccgacgacaagccgccgttcccggtggacggtagcgacccgatggcaggcatcgcctgatggacctgagcgctctcatggcagcggccggtgagcgctccccgatgccggtgcaggtggtacgtcagcacaacccgcgcgtgatcgctcacgttgatggggactacatggcgtacttcgcggctggtagcgagaactgctcggcgggggatgcacgacgcaacgtgctctcccgctgcgcacagctgaagcatgtcagcggagcgggcaagatcgtcatgcacctgacgcacgccgcgtctaccaagggtgatcgcttcctcgctgctaccacgcagccgtatcagggtcagcgccaagcaggccgcaagcccaacaactgggcgttccttcgtgagtggatggagacatacgagggcgacgctttcactcccaaaatctggctgacccgtgaggccgacgatggcatcgcgtacgtcaacgagggtgcagcattgcaccacaacatcctgcacgtggtgcacagcgccgacaaggacatgcgaatgttctgcggcgtgcacgtagactgggacggctacgacatcacagaggttccgctcggcgcttacgacatcgttggcgagaacggattgcagtacggtcacaagtggttctggatgcagatgctccacggcgacaccgccgacaacataccgggtctgccgaaggtgggcaaggtgacagcggagcagctgctgttcgagacgaagaccaacctcgaagcggtgcagatcgtgagcggcaagtacagcgaagtgttgggtgccgactggcgcaagacattcgccgagcaagccgtgctgctgtggatgcggacggatcgtgacgcagaactgctcgacgtgctgaagctcgacgtgttcgggccgaagctgaagcaggcgttctatgacctcgccgaggacgtgaacgagaagcgtgcaatcttggaggcatacaaagcatgaagcgactcactgcaacacaggtcaagctgctgcgcatcaagctcgcagcggagcaaggcaaccggtgctgtctctgtcagggacagttcggcctgaaggctccgctcgatccggtgctggaccatgaccacaagaccggcgctgtgcgcggggtgctccatcgcggatgcaactccctgctcggcaaggtcgagaacaacgcaggccggtacggcgtgcgcgacgtgttcgcattctgtgcgggcatccccaactacctgcggtcgcacctcaccaacatcacggggtacctgcatcctacctacaagaccgacgacgagaagcgtatcgctcgcaatgcgaaagcgcgaaagcgtcgggctatcaacaaggagacaccgtgacccttacccagttcattcgccgagcaccgaagcgcggcccgaagattctctgcctcgacatcgagacgttccccatcgagttctatggctggggcatgttcaacaacaacttcagcgtcaagcagatcaagcgtgactggtcgctgatgtcgttcgcttgcgaatggctggacgacgaggcgtcgttctacatggaccagcgcaacgtgcgcgacgtgttcgatgatcgcaagcagggcaaggcgctgtgggcactgctcaacgccgccgacttcgtgctcgctcgcaacggcaagaagttcgaccttcgcaagatcaaggctcgcctcgcaatcctcggcctgccgcccgtgtctccggtgcaggtgatcgacccgatgctgctgaaccgcaccgagttcgccttcacctcgcagaagttggagtacaccaccggcgtgatcgtgccggagctgcgcaagtacgaccaccacaacttccccggcttcgacctgtgggtggcctgcatgcagagcctgcccggagcatgggacgagtgcgaagcgtacaaccgcatcgacgtgaagtccatgaagttggagtacaagaagctgcgcggttggtactcgcagcatccgaacgtcgcagtgtactacaaggccgacggcagcgagcaccgctgcaacaagtgcggctgcaacgaaatgatcccgcaggatgatccggcccgcacgcaggtcggtacctacctcctgcttcagtgcaccgtgtgcgacggctacagccgtgggcgcaagctcacgaccagcgccgaggcgcgcaagcacatcaccgtcccggcataaggaaccgacatgaagatcaccgacatccgcagcggcatgcgggtacagtacatcggcaatgcgcccgcaatgatcgggctgcgtggacaggtaagccgcgtgttcgctcgtgatgtcgaggtcttcttcgacggtcgagttaagccgagctgctgcgttcccgattccctccgacagcttctcagcatcggaggcgtgaccaccaccagacgagaggtaccaatgcccgaactgagctaccgcgacgaggaccgtcgcacactgtccgaccgtggcgtcggcctgaaggatgacgggggcaagccgcaggcccgtctgctgcatgagggcgtgccgcgtgcactggcccgagtcatcgacaccctgaccttcggcgcgcagaagtacaaagcgcactcgtggcagcatgtcgagaaggcgctcgaacggtatcaggacgcgagctaccgacacgacaacaagcgctgcctcggcgagaagctggacccggagacgggcatccaccaccgggcgcaccacatcatcaacgagctgttcctgttggagctggaactgcgcgaggaggagaaggccagtggcgcagagtaaggcgcgctccatcaaagaggcttgggtgaacatcggcatcggctacagcatcaactacgcagcgaacatcgcgctgcttccggtgctgtggcatcccgagcatccgctgctgtcggcgcacgccatcggcattgcgttcacagcgatcagcttcatccgccagtacatcatccgccgctggttcagcaagggtgactgatggcctgcgcccgctgcggccaagtgcatcggtacgtcccacatgaggccgagtgggcgcgcttcctagaggagcaccgtacccgcaagcagttcgatgtcgagtgggccaactcactctggcatcgtacataccctgacgacgcattctgcatcctcgtgatgaggggcctcgcaggtttcgttccattcccgtcgaaggagaactgaatgctctacaagaaccagaccgccatgctcatcaagtcctacgagaacgccgttgcgtggggcgagagtgccgaccacgaggaggcattgcagaatgcggtcaaggccgggttcccgaacctgcccgacgaagatcaggccgagctgtatacccgcatcgccgatgcgtgggaaggctaccgtggttcgctcgctccgcgcaagctgtggatcggcaccatcgtcaaccagttcatgtcgtcccgcatcgcacggttcaacgccgcgctgggtgacggcaccaagaaggaggacagcgccgatgtttgatgtgcctcgccagaatgtccgggttgctcccggctacaagaagcgcaagcgcggcttcaagatcaaccgcgccttcaccaagggcaacttccgcgtgcagtggtacgacggcaaggccacgtactgggagcgctacgttccgtggtacgaagtgccgctcgccatgttccagatttggagggactacgcatgagctacatcgtccacaaggcagtcgagcaggacaagatcaagaagaagctgcggcccaccgaggagcagcttcgcaccgagtacatcgcacagccgaagtacgacggctgcaacatggtcgccatcaagcgcggccactgggtgcccacggtgaacaagggcctgcatgccatcaaggtgggcgacgtgcagatgcagccggtggatcgtggcgtggttgacctgttctcccgcaccggtgagcaggtcgtcagcgcacaccacatcgagaacgctctcgcatccgcgccgttcttcccggtcggcgtgtacttcggcgaatactggcacccgcagatcgaccagcccaccgtcagcggcatgttccgcaagaaggacggcacgcagtacaccgagccgatgttcgtggtgttcgacttcgtgacgctggaagaatgggagcagggtttcagcgacctcgtgtatcaggagcgcgtcagccgcctgccgagcatgggccacgccatcgccgagggcaccgcgccggtgttctacgccgagtcgcagggcttcctgatcgaccaagagctgggcagcatggaagcggcgaagctgctgtgcgagggcggcgcgtacgacgggctgatcctgcgcaagccgagcggcaagtgggtgaagggcgacaagggaaccaacggcgaagtcgtcaagatcaagccgaccctgacgctggacctgcgtgtgctcggcatcaacgaagcagtcggcgagaagaccggccgcgccgtgtacacggtcgtcgttgacctcggagaaggcaagacgcaggaggttggcagcggcgtgccgcacagcgagagcgagctgcctagcgtgggaggcatcgtggaaatcgaggcgatgtccttcagcaagtacggcctgctgcgcgagccgcgatacaagggcatccgtcacgacaagaaggaggcagacctgtgagcgtcgaggtgcaagcatggcacaacatggagcgcgacacggtggagctgcgcatcagcgttcctttcggcgagtacgccggttccctgtggccgaacgagacgctgcgcgacaaggtgcaggaagcgttcgccaagttccttgacgagcggaggggctgatggacgcgatcactttcgagaagccggagctggacttcagccagtcctcggcatggatgggccgcgtcgaggtttcggtgcgcgcccggtacggtgccgacttgttcggcgctgctgccacgtgcatggccgaggatatcggcggtgaggcgtggccgcacatcatccacgacctgcacatggaaatcatgcgcggtatcctgaaacgctacccgccgcgcgactacaccgtgcggcagcaacggaggtaacaatgctctcgcaagtggaactcgaactggaaacctacgccttcggtaaggagcgcatggagaagtccatcgcccgcaacgaggagaagggcggcgcggacaacaacccctacgcccaagcagtgtatcgccggttcgtgcttccgcttgcggagcgcatccgtgcggacatcgactctccgcgaatcggccgtgcgcaagcgcacgtgccacttctgcgcgccaagtacgatcccgagcgtcagaacaagcgtggacagcccgtcagcgccgaggaacaggcacgcgagtggtacgaggctgtggccttcgtcgccgttcgcggtgcccttacctcctgcatgcgagacaagcacggcgaaggcagcgaccgcgacgtgttgaagaacgttggcatcaacgtgtaccatgagtacctgctgacgcagttcgccgacgcggagccgactctgttctaccacctgatgaacgacatggaccgcaagctctctgtcaacgagaaccaccgcatgacggtgatgaagatgcaaggacgcaagaacggcatcgagttcgtggagtggggacaggcacagcgcgatcaggtcggcgcgtacctgtgcgatcagcttgcgcagctgggcatgttggagattggcgtggtcaccgagactgctgccagtgcaggcgcagcgtaccgcaagttccagaccaagacgcacgtcaagatcgtgctgaccgacgaggtgcgcaagctgattactcagatcagcgacttcgtgatcgaggccacgccgttctacctgccgtgcgtcgagccgccgatggactgggtggacatcgacaacggtggattccacacgaaggaaatgcgccgactcaatccgtggatggtgaagacctacgctcagacccgcgacgagtaccgcgctgccgagctgcgcaacgagatggctgcgatcaacgcattgcagcgcgtgccgtggcgcatcaacaagcgactgatggaagctgtgtcggccatcgccaaggtgcacgacatggaggaaatcatttctcagggcgagctgccgaagccgcgcaagccggagtggctgacgaaggacatgaccaaggaaaccatgtcccacaatcaggagttggagttcaagcagtggaagcgcgacatgtccaactggcacaccgacgagcgcctgcgacagaacaagggcaatcgtttctacaacgcaatgaaggtggcgcgcaagttcgccgagtacccgagcatctacttcgtgtacttcgctgacttccgtggccgcaagtacgttcagaccaccggcgtgtcgccgcagggttcggacttgcagaaggcgctcttggagttcgccgatggcaagccgctgctgactaaggacgcgaaggattggttctgcatcacaggagcaaaccgatggggatacgacaaggcgtctctgccggatcgtgtgaagtgggtagcggagcatcacgaccagatcatggcgttcgctgcggacccggtgaacaacgacgagtggaagaccgccgacaagccgctgcaatttctgagctggtgcatggagtacgagcagtggcaagtgttcggggatcgcttcctgagccgcatcgcagtcggcatggacggttcgtgcaatgggcttcagaacttctcggcgatgctgcgcgacgcagcaggcggcgtggcgacgaacctgatcccagcaccgctgccgaatgacatctaccagatggtggcagaccgcgtgactgccgtcctgctaggcgaggacgaggatgccgaagggtaccgcacgctgtggctcgaccacggcctcacacgctcgctggtgaagcgcagcgtgatgaccctgccgtacggctcgcggcagtcctcgtgggcggacttcatcatcgaagactacctgaagtgtgggaagttcccctcgctcgacaaggccctgtacggccccgcagcgcgcttcctgagcaagcgcatgggtgaggccatcgccgacaccgtggtcgccgcagcgggcgcgatggagtggttgcagcgcggctccgggtcgatcctcaaccaagggtacgaccgcatccggtggatcacgccgtccgggttcccggtggtgcaggtctactgggagtccgaggagcaccgcatcaacaccaagctgtgcggcaacgccaagctgtccctgcgcaagagcacggacgcggtgaagaagtcccggcaccgcaacggcatcgccccgaacttcgtgcacagcctcgacgcaagccacctgacgctggtggtcaacgcggccaaggccgaaggcatcgacgccttcgccatgattcacgacgacttcggcacccacgccgccgacagcgcggcactgtaccggatcatccgggaggtgttcgtgtcgatgtacgagcggcacgacgtgctgtcggccttccactcggcctacccgttcctgccggagccgccgccgatgggcgagctggaccttcggcaagtccttgattctccgtacttcttcagctgacggagtttcagtacacctatagcacgaggcaactgaggtccggttggagcggccgcgaaggtaagcggaaccggtgccggaccttttggtacacctatagcacagaggagacaccatggccgaagacgccaaagtgaaagtcctgatgacgctccacccgaaccagctggccgccgtgcggaagctgtccgggctgtcgctgtccgtcaactcgaataccacgcccttggaggcaggtatgcagttggggatggcccgcgtcctgaacatcttacaggagggtttcaccgttgattcctccgtaccgaacaccaacgacgggtgatagtgagcagatcaaggcggctttaacggccgctttgtatctgtcatctagagaagatagtaaggtagacaacagagaatcttctgtgagctacaactgtgatgaccctgattacacagtggccctgataacacagggtctagtggatgcagtaatcattgatgaagcctacctgctgtgctttgccattgtcacaccgtggtactccaagaaccgtactacgttcgttgagaacatggtgctgcgaattgggccgggcagttccttcgaccggtacatagccgtgatggaacatctggctgacatcaaccactgcgactcactgagcgcaggcggtgcactagctcggaactcccgagcactcacacggatgtatgcacgctacggctacctgctggaacggcatgctccccaattcaccaagcgaaggagttaacctatgggtagcatcgttggtggtgggtccgccaagcgagcagcgctgaagcaagctgctgctatcgacaagcagaccaacctccaaactcaatccacgaactaccagattcaggcgatggccgatcagatggcacaggcagctgcacagcaggccgcatctgagtacgccgagaagttgctgagtgcccccgtcgataccgtcgatgtgcggctgggaacttccgacctcgacttgcagactgccgacctgatcggccgacgcaagaccgcccgctccacttacacccgacccgtgaccacgaccgcagcttcccggctgacgaccgtggccgggtcagacctgttgtgaggtgagcatggaccatccgatccaaaccgctcaccgccagttcgaggcttacgacaacaagcgacagggcatcatgtaccgactcgaacgctattcgagctggaccgtgcccaagctgttccctcgcaagaaccgcgatcaggacaccgagccgctgacccacgggttccagtctctcggcgcgcaggcagtgaaccatctggcgaacaagctgatgatgtcgctgttcgcaccgtcccgcccgttcttccggttggagctgaagcgcaaggcgaagcaggctgcgcaggagcaaggcgctgacttgcaggccatgcaggcgatgcttgcgaaggccgagcaggatgccagtctcgaactggacaagcgctccatccgctcccggctgtacgacctgctgaagatgctgatcgtgctgggcaacgccctcatggtgttggagaaggacacgatccgcgtgctcaacatgcggcactacgtggtcaagcgcacccgcaccggcgaggtctacgaactgatccttcgggagaaggtgcacaagacccagctggaacccgcagcgctcgctgccattgtcgcgcacccggacttcaagcccgatgacgacggcatggtgtgggagtacaagtgggtcaagctggaccacaagaccggcaagtacaacgaagacgtgtggatttgcaactgcaagctgcccgccaacttctcctcgacctacaccgcagacaagctgccctaccgggcggttagctgggacttggccgcaggcgatgactacggctccggcttggtcgaagactacgaggccgacttccagtcgctctcgatgctgtccgaggccgcagtgcagggcgcgatcctcgcctccgagttccggtggctggttaaccccgcaggtcagacctccgtcgaggacttcatggcgtcgcccaatggcgcggccattcccggcatgaagggtgacatcgagctgattaacgcaggcgtcgatggcgtgctgcaaaccaaccaagcaatccagtccacctacatcaaccgcatcggcgcaggcttcctgttgcagacggcggtgactcgtcaggcggaacgtgtgaccgcgcaggaaatccgcatggtcgccgaagaactggaaggcgggctgggtggcggctactcccggatcgctgcggacgtgcaggtaccagtcgccttttgggtgatgaacctgacgggccgcgacatccgaggcaaggacttggagcctgtcatcatcaccggcttggccgcgctctcccgtacgggtgaccgtgaccggctgttggagttcggcagcaacctcgccaacgtcctcgcactgccgccgcagattctcgaacgactgaagctgtccgcgtggatcgcagacctcgccgccgctggtggcttggacccgaacgtctacgtgctgactgaggccgagtacggccagatgatgcagcagcgtgcacagcagcagctcgccatgcagaacgcatcccagcagatcgacaacgccaacaacatggagacacagacacaatgagttccaacgcacctccgggcggtggtcccggcgcaaccgtgatcgcaacctcgaacggcaaccagcccgcaccggcagctccggctcccgcagacgacaagctgttgcccaacggccagcccgctccggccgcaccggcacagcccgcagctcctgctgcacctccggctgctgacgcgctgagtctcgaacctgccgctcccgcacagcccgccgccccggcgaacgctgcgccgactgcggtgtcgatcccggactacggcgacaacggcctgaacatcgcggccgaatacttcgtcaacaccgtgggcctcgacatcgacagccgcgaactgaccgaagcagcgaagggcaacttcgccctgctggaagccaagctggaagtcctcggcgacaaggccaagggttccgcaccgatcctcgctctggcgaaggagagcatcgctcgtgtcaccgccgctgcaaccgcagcgcacgccgcgaacgttgctgctgtccacgaagccgtgggtggcgcagagaactgggctgcgatccagcagttcgcacgggccaacctgcccgccgaccaactgaagcaggcaagcgaatcgctgtcggctggtggcttcggcgctcaggcgaccgcgcgttacctgatggctctggcacaggccaatcccgcgacgaccgtcaagggcgcaccggctaccaacgccgccgcccccgccgcgtcgatcaacggcgtcgctcctatcacgaaggagcagtaccgcgctgagtaccgcaagctggttgccgagaagggcatccgtggtgcggcccactccgaagaactgcgtgcactcaacgcgcgcgtcatccactaagaccaaggagcaacacaaagcatgagcaccatcttcccgactgtcccggttctgccgaatcaggtcaaccagtccggcaacgagaacgccctgatcctcgaacagttcaccggcgatgtcgagcacacctacgtgtccagctcggtgctggaaaagttcttcccgcgcaagcaggtcaagggcaccaacaccctgaccaagaaggccatcggccgtaccaagcttcagaagctgaagcgcggtgacgcgccggacggcaccccggtggacttcagcaaggcgtcggtgaccgtcgataccatgctgctgtcgcgtcacagcatctggcagctggacgaaatcttcaccgacatcgacacccgcaaggaaatcgccatcgagcagggtcaggaaatcgccgagttcgtggacctgaccatcagcatcgccgccgcgaaggccgctgctgccacgcagtcgatcttcacccgcaacggccgcgcgcccgagggccacttcggtgccacgcaggtcgtgctgtccgccgctggtgacgagaacgatccggccaaggtgtacgccgccatcggcaaactgttctcccgcatggaggaggagaagaaggtcaagccgcagcgcgatggcgtggtcctgatcgtgcgcccggcgatcttctacctgttgcagcaggccgagcagatcagcaacggcgagtacctgacctcggacggcaacaagctgaccggcatcccgaccttccacggctggggcgtcccggtgctgtcgagcgagaacctgccgaacaccgtgatcgaaggtcacctgctgtcgaacgacgacaacgacgacttctacgacggcgacttcagcaccctgatcgccgtggccgtgtcgccgaaggccctgctgatcgccgaagcgctgccgttgcagtcctcggtgtggtggagcgatgcctcgaagtgctacttcgtggactcgtggatgtccttcgccgttggtctggatcgcgtcgagaacgcgggccgcatcgacaaggttgcctaatccgctgggcgcggtccctgaatccttcgggtaactcaaaccgcgcccttcttccaccaacacaggagcaacatcatggtctttgaccgaccgttcgagatttccaaccgcgtcgtcgccgcaactggcgtggccggtctgcccgccaactccgttggtaccgtcgtcggcgtccactacgacacccgtggcaccgcaggctgggtcgtccgtgtccgtttcgtggacgacgaaatcggctcgcaggacatcgagtacgcaccggccgctctggctctggctgcggactaagcaacatcccggcaggggcgctccggcgtctctgccttgttcctctcaggagacaccatggcattcatcaccaagctcgacatcgtgaacgcctgcttgaagacgatgggcgagacgaagctcaacacgctggaagatgaccacgtatacaaggacgacgccgttgacttgatcgaccgcgtgcaccgtgacgtgtcctcactctcgctgtggttcaacaccgaatgggtggagctgaagccgcaggcaacgagcaagtacatcatggtccccacggacgtgctgaagctggactgcaacccgagccggttcggccacgtggtgcagcgcggacgccgactgtacgaccgcaagcgcaacacctacgagttcgaccacaacgtgcaggccaagctggtgcggctgctggacttcgatgacctcccctacgaggtgcagatgttcgtgcgcgacgactcggtgctgcggttccagtctgacttcgacggcgacaacaccaagtacgccaagatcaagcagcagcgcgatgacagttacatcaacttgaaggccgagcacatccgccagatcaaggcgaacccgctgttcgctcgcgcatccgtggacgtgctgcgttcccgttactggaactacagcggtcacccgtggcacagccacgtcacattccccggctaaggagacaacatggcaaaggcaggcggaacctatcccgacatccttcagggtgtcagtcagaaaccggcgcatcgtcgtcggccgggacagacgcacgagcagatcaacgtgctgtccgatccggtgaacggcctcgtgcgccgtcgtggtacgcggttcgctgcttcccaagccgttgtcacctcggccgagctgcgcaacatggacgtgttcgacttcatgcaggagggcaaggagtacgcgctgctgtaccggcgcgacgcctcgaccttgggcagcgagtccttcgcgttcctctacaacaagacggacgagtcgttcatccctctggtgtacgagaacagcacgtgggtcaacacgctggtcagcggaggcgcatcgtcgctcacggccatcggcagctacgtctacatcgcgggcaacaccacgatcccctcggccaccagcacgaacgtgtggcaggagcagacgaacatccagcgcctcgcagcatgggtgcgcaccgggaagtacaacaccacgtacacggtgaacctgacgcggacggacaacacggtgctgacggtaacgttcaagacggttaccgcatcgtaccccggaacgctcgacaccagcgacatcccgttctaccttcccggtggcacggagccggacgcggcgtaccagaagtacgtcaacgaccgagtgaacgagtacaactctgcggtcaacgagtggatcgtgacgagcgctgagcagacgcgcccggagtacatcgcggagcagctgtcggatttgctggtcgatgcaggcgtgtcggcaacgtacatcaagggcgggatcatcattgacgatgaccagttcaaggacatcacggttgacgacgagggagacggcacgaccttctacgccgcagggcaggaaattacagacgcgacctacgccgtcaagttccactggcacggcaaggtcattcgcgtgcggccgagtggtgcaggcgcggacgagtcgtactacctgcgcgctgagttggagaacggcgagacttccggctacgggtcggtggactggtacgaagcgcccggcgtggagtgcaccatcgacaacctcgtgtcgcagctctacatctacaacggtgtaggctacatcgcacgcaacggtgcgggcctcacgtctctggctccgagcagcggcgagcatccggcctacggtgcgcgagtggcaggcgatggtctgacctcgccgatcccgtggttcatcgacaagccgatcacgatgctgtccgtcttccaagaccggctggtcatcggcgcacagaactacgtcaacgcctcacgctcggcggactacctgaacttctggcgcggctcggccgtcaccatcgaagacagcgaccccatcgaaatcttcgcgcacggcagcgagggcgatgtgctccggcacgcgacgctctacaacggcaacctcgtgatcttcggtgaccgtcagcagtacggcatcagcggcgactcggtgttcagtccgaagaatccgctgattaaagcgttcagtgccaacaaggattcggttgacgcgaaggcgcagacctcgggcaactacatcttttatgcgcagtacggcagcgaaggcacgagcctgcaccagatgcgagtgggcgcgctcaacgggcagcagacggtgacggacgaaatgtccaacgagctggactcgtggctgtcgggcactccgttgcagatcaccccgctcactgcgccgaacctcgtcatgttccgcactcgcgagcacccgcaggacttctacctgtaccggtacgaggacaacaagaacaacgggcagcgcatcgtggatgcgtggtcgaagttccggtaccacccggcgctgggcgaaatcatcggcgtgagcagctacaagaagaacggcctcgtgttcactgcgcgcgggtcgctggtggcgtgcgacgtgttcgacccgaagggcgagccggactcgcatgcgtgcctcgacagctgggcgagttttggtacacctacgggcgtacagactgcgagcgcaagcatcgccgtcaatagcactagcccgtacttcctgctgggttgtccctacgcgcaggcgtctgacttccttaaccagttcgatgacctcgctgctggtgcgctggaatacggcgtggtgtccgaagctctggtgatcccgaccaatccgttccctcgggaccagaacggtcaggccgtactcgatggacgcatgtccctcaacaaggtgacggtggacgtggagaacacggcaggcatgatcgccacggtggcaacccgcaacagcaatgtgaccactacggacttcgagggccgcatcctcggcgactccgacaatctgatcgcgcggcaaccggtgtaccgggggcagctcaacatcagcgtcgggcgcgaagtgcgcgagtgcacctacgagattcgcagcaaggattggctcccgctccgggtgaccggcctgagctggacgggtcagactttcaacaatgtacggagggttagctaatgggttcggttaatacgatcctgcaagcgaacaacaccacccgcgttgcccgtgcgaactaccgtgcagccgttgcgcagaccgacaaccagaaccgcagcgaggtcgccaagaccggcttcgctgatttcatgcggtccctgaagaacaacgcccaactggacgccgccgcgaaggagtacaactccaacatggaagcgctgtccgaggagctgcgtgcgcgccaaggggctgggcttaactcccagctccaactggcgaacgcgcgtggcgcacttcaggcgcaggctggtgctgtcggtgtcggcggctcgtccgcagacctgatggattcgatggtgcggttgcaggcggaaatggatcaggagacgcaggccaacgctgtctcgctcctcgcctcgcggggcgcatcgcagactgcgcagatcatgtcgcgcgcgtggaacgggatggacatgagccgttcgttcgggcagttcgactactcgcagcacatcgagccgcaggcaatgaagcgtcgcttgggcaagctgatcggcgtggccgtggctacctacttcggtgggccgatggcaggcgaggccgtggcagacttcgcggtcggcacgtggcaggcggacaacggcaacttcactggtgcctctcagtccttcagcaacgcagcgcagaacggtatgcaggcgtggcagcagtccaatgatcgcggcggcaagtcgtgggcgtccactaccttcgggtacaacgacggcaccggcaagcagtccgtgactggggcgaaggtcaccggcaacttcggcaacaactacgacaacttctccaccactacgtccggcctcggctggttcgatagcggcagcggaggcaactcaggaggtgcatggtaatggctgacatcggcacggttaccttcaacacgcagtccgcattgcagggtggcatcaacgccaccccagcactgtcgggcaacaccagcattcaaggcgctggtgtgaatcaggtcgggccggttcaatccggcaacgactggttcgcaagcactggtggtatgacgatgccggacagcaacctgccagagttcttgcaggagctggcagcgccgaacaccgccaagctgaagcagcagcagatgtgggacggcttcgttgccgcccgcgctggtaagaccatggacgagattgctgcgaccgaaccgtggtacaagaaaatcttcggagacaccaactacgagattggcgcgagcatgtataacacgctctcgcaggtcaacgaaatggagagcgacttgcttcggcgtatgccggagttgcgtcagcttcctcccgaggcgatggcgaaggagttcaacgacctcgccactgcccgcatgaccggcaacggtttcgcggacacggtgttgcagaagaccttcatggatcgcgcgggttccctcatggacctgcacaccaaggagcgcacggcatggcagcagcaggagctggtgaaggcgcagtacgctgcgaactcgtcggcgtccaccggcttcaacgaactggcgaagcgcacggcgatgctcggtaccaaccgtcccatggacgagaaggccaccgaggcgctgacgcaggcgcagctgtccctgctggacggactgtcgccctcgcgctaccagacggacgagtcgtacaagtccgcgatcactgcgttctatcgtggcgctgcggatcgcggcgagttccacacgctgaagttcctcaacagcaagggcgttctgaacgccatcgacccggacgggcagctgggaatccagcagtacgtgaagcaggcgcaggatcgttaccgttccgactggctcgatgccaacccggagcaggccgagaagatggcgctcgtctccatgtacgcatcggagggcattggtgccaagccgtcgcaggcgatgatcgaggaaatgaactcgacctacgccgccgagactggaagcgacgcaccgctgtactccggtacgcagttggcttcgatcatggcacagtccgcaggcgcgcacatccgcgcacaggaagccgtcatcaaccagcgtaacgctgcggccaaggccgcgctgaccgaccagcagaagctggccgcgcaggaggaggacatccgtggtggcatcgaagcgttcaagcgcggcacgtacgcgcagacgatcaacatccccggcgtggacaaggagctgatcgaggcgaacacggtgcaggcatggaatgccacgatggccgcgaaccccaaggtcgccatgtcgcagctggtgtggaacgccaacaccgggcgaggcgctgtgctgaagggtgtggccgaccagttccagaccacggcgcgcgctgtgctccgcgatcagccgaacacggcagcggctgcactgtaccagcagtggaaggaactgaagcagaccaccgccgcacgcatcgacacgaacggtcagcccgtgcagggccgactgactggcgcgactaccgctgcgctgtacttcggagatagcgtcaacacgttcttcaacaagctgcaagcgttggagaatggtggcgtgaacttcgagcttgcttacgaggtggcccgtggagaaatcaccaccgacgatccgacgcagttcgacgcgaacagccgtaaggaatccgaggctactcaggctcgtgttacggaagctatcgccaagctcaaccccaagtacctcggcatgttcggcaacaagctgggcgactctggccgcgctgcgtatgctcgcgccatcgtccgctcggtcactgacaccggtggtctgctggacacttctgcggaaggcttgcaggctgcggctactcacgccaagctggcctacggtctggaagacgcaggcaagtacgcatgggaaaacggacgcgacgacgaaggccgagtgatcggcagcgtcggtgcatggctgggcttcatggacacgaaggaaaccggacccgccatcgagaaggccatcgacgcagcactgcgccgggtcaacatcgagccgagcaccgggctgaaggctgacgtgttccgcatgaaggacagcgagaacggcgagccggtgctgtacgtcaacgctgttggcgagaagggctggaaggttgtgccggtgtacgggcgcgacatcaaggacgagtacgagaagcacaccaagcagcagcgtcagttgcaggccccggtaccgcagggctacgttcgcatgaacgacggtacgattcagcagagcatttccatccaacccaaactgtaaggagatagacaatggcactcgatctttcggggctgacccaagaccagcagattgccaaggctgccgcttatgcgggagtgccggagtccatcgtgcgcggtcagtggcgagtagagtccggcaacgggcgtgccgccaaggacgctgacggtgtgatccgcagcaaggcaggagcacagggcgacttccaagtcatgcccaccacgcaggcaacgtgggaagcgcgcaacggtcgcaagtacgacatgcgcaacttccaagacagcatcgagctgtatgccgacatcatgcgcgagaacatgcagcttgccaagggcgacgtgacgaaggcgctgcgcatctaccaaggcggcaccaatccgaagaactgggggcaggagaacgcagcctatgcaccgagcgtgctgggcggtgcgtccgctcccgcagtgtcggcgcagccgcgcagcctgaccaccacgcaggcagacctcaacgccgcatggcagggcaacccgaacatgcgcgaccgtacgtggtccggtgcgtccatcccggatgcgtggacgggtgcgcccatcgaaggccgcaacgctctggcgtcggcagcgaaggaacacatcggcaagattcgtgcgggcatcgccgagctgtcgatgggtcaggtagcacaggaaggtggcaccgccgcgcaggccgtaggcaaggctcaggctgtccgtgcatcggatcaggttgtgccgtggtgggtgcgtcaggaagtggacgtgctgaacaccggcgctcgcaaggcgctgctggatcagaccgaacaggcgctcgcgcaggaccgcgcggacgaggagctgcgcaactcgctgaccttcctcgacaagtggggcgctgcgttcgacagcggcatcggtgctgcgatcagcaaccagtttgcgcgcgaggacgagaacgttccggaaggttggaagtacgacccgaaggaatgggagaagccgtggatgactgccgacgaactcgaagacatccgcgatgcagcgtactcgccgaacgagctgaagtacgtcagcgaccgacagttcctgcgccgccactccatgcgcatcaaggatcagcagactggctggggtagcttcggttacgacatggtggcaggcttcaccgatccgggcaactgggctatcggcggcgtcactgccgcaggcgctaaggcgctgggcatcggctcggctgcactcgttgccgaagggcgcgtgggcgcgtcgctcgcgtcggctgctgcggagaacgcggtcggttccgtcatcacggacgccgcgctggttggcatgggcgagcgccgcaacttcgcggacttcatgaccgacgctgcattcgctaccaccataggcaccgcgatgcacattccgggcgtgcgctcggctgcgcagattcgtgacaaggcaaccatcgacctgtccgcaggcaacgctgccgcttacggcgaagcgtggtcggccgacctgaaggcgcgcgctgtggccgagctgggcgaggacgccaacccggtgctggtgaacaaccgcatccaccagcttgccaagcaggaggctgtggattggctgcgcgctggtatggccgacgtgcctgacgacttccgtatcttcgcccgtcccgacgtgcaggagacgaccaccaccgcaggcaccactggtgcactcgcacgggacgcgggcaacgtggacgcaacgaccgggcggtacaacgacagcgtgggtggccgggtcgatcagcatgacccgctgctggaacgcgcatggaagaccgcaggtatcaagggcggtaacgtcgatggcgtgctgaagtatctggaatccaacgcctctatcccggaggacgtgcgtgctatcgccaacgcgctgaagcgtggcgggcggctgagcacggtgaagatcgtgccggaatcggaactcgacaagtggttcgccggtgccaacatgggtccgggtatgcgtgtggccggtggctacaacgccggactggacgcgatggcgatgcggaactacacgccggaagtggtggtgcacgaaatgctgcacgctgccacgctgcgtgagctgcgcagcaactcggtgttcgggcaggaaatggaagaactgctgacccatatcaacaacagcatcggcagtgtggactccacgctgaccaccgctgcgatggagacgcgcatcaaccagccgcaggcaggcttcctcgccaacactgacgagctgatttcctacggcctgacgaaccgcgctgtgcaggcggtgctgcgtcagatgcccgcgccgggcaacacccgcccgaatgcgtgggagtggctgaaggataagatcgcgcgagtgatgggtctgaagaatcaggagtccgcgctcgaacgcctgatgtcggtcgtcggtgacaacctcggcgcggaagtgcgcgacacgcaggccggtacccggcagacgcgtggcatgctcgccaactcgatcttcaagtcgaaccgcgagcgcaaggctttctaccagcgcaccggtctggacaagtccgtcagtgatgacgcgatgcgtgtgcaggtcgccgaagtgatggcacgctccgaacgcttcagtgcgcagtacggcatcgacgcggcgaagctgtccaccatcatgcagcgcttcgggctggaagctacgagcacgactctaatgtcgtccaagtcgccagttgcccgcatgcttgcgatcaccctgttggagaatcccgagggtgcagcaggccgacacagcaccgcagcgatggatcggcatggtcggtttgagtcgttcatgggcacccgcccgcgtcagtgggaagcggcctatcgcctgtggcgtgcggacgtgcgcggtatcggtgcgatcaaggacttcgccacgggctggaaggctcgcgcggacttcgagtacgcagtgaagctgtaccgcgagactcgcttcaacggcggggacatcccggatgcgcacgaggcagtgaaggcaatggcccgtgagttggaccgtggctacaaccgcatggcagcagagcagcgcgcggccggtacggtgggcgcacagcgtctgccggaggaggacgtggagggctacgagtcccgtacgtggctgggcggcagcatcgctgctgctggtccggtgcgacgcgagggtatccgtcaggcgatgcgcgatcagttcgaggtgatgggcgagctgtatggggacgacttcctcgataagttcgctaccaagtatctggaacgcatcgagcgcaaggctgcgggtgtcatcgaagcgccgggtcaggtcttctcggagtcgcaggcggacacgctgcgcgacactctgcgggcgatgtcgctcaacgaggaggagattcagaaggtcatgggcaagtacagccgtggcggtgcgaagcacaccaaggcgcgtatcgacctcgacgtgaccaagcagtacgaggacgctgacggtaagttccgtctgatggactatctcgacaaccgcgtgatggacaactaccgcaagtacgcgggacgtgttgctggtgacatcgctctggcgaagcacggcatcctcggcgacgcaggcatcaacgtggcgcgcgaagcaatgcgcctgaccggtgccaacgatgtggagctgaaggcgttcgagcaggtgatgtccgagttccttggtcgcccggtcggtaccggcgatccgactgttctggcgaatgcgcgtctgctgacctcggccatccagctgggcggcgcgggcatcaatcaggcagcggagtacagcaacggcctcgccgctgttggtgctgctggtgtggctgacgcaatccgtatcgctccccgcatgcgcagcgaaatcatgcgcatcctgaagggcgaggacagcggcaaccaaatcctcgacggcttcgagttcatcagcggtcgcggcttcggtctcgccggttacgacctacacatgttcaactcgctggacacgcaggcgtcgatgtatggtagcgagcgcgcaggcttcctgacctcgctggtgcagaaggcagcgcatgcgaaccgcatcctctcggggcagcgggccgtgcttgctgtgcagcagcgtggcttcgcggaagtgctgatcgccaagggcgtgaagttcctgcgtgatggtgctgaagctgacaccgccctgaaggacatgggcattgacgacaacctgctgaaccgcctgcgggctacgcaggatcaggtcgtgcgctggggcgcggatggtaagctggaagcagtagacccgcgcaacgtcgaggggctggcggatcggcaggcatggttggcgttctacaacgcgatcaaccgtggcacctcgcagattcttcaggacaccttcatcggcgagactggcaagtgggcgcacaacggctggctgaagctgctgttccagcaccgcacgttctcgctggtcgcgcagcagaagcagctgggccggtacgtgggcaactacggtgcatggcagacggcgggcctgatcgctgctgcgatggctgtggcggctccgctgcaagccctgcgggtgctgtcccgcgtggccctgatgaacgatcaggagcgcgacgaggccatcgaccagaacatcctgtcgcctctggcgctgggcaaggccacgctgaactacgtgtcggcgacgggtatgctcaacgatgtgctggacgtgggcactggcgtggcgggcggctggtacgagtacgccaccgatacgcagggtccgacgtggctgaagcagctggccggtgggcagttcggcaaccgcaaggaagtggtgggcgggcagttcgcgccgtcgctgggagtcatcaacgacttcgctcagggcattgctggcaagccggagaatctggccgacgtgattccgggcgggcgactgccgatggtgatcccgctgctgaagggcgcagccagccagtggaaggaggagtaagatcagggccaaggacggcccacccttttggtacacctatagcaaacaggaggcagcatggcagttccagacccgcagctgcgctacgcgacagacgtgttcgacgccgatggcgtgaccactgactggcagatcagctttaccggtggctacatcaacccgtcccacgtgtacgccatgagcggactgctggacgaggagactcagctgctgaccgaccggactccgcacaccgtggaagtcctgagcgaagacgatgacgctagtaccgtccgagtctcgcctgccgtcgccgctgggcgcaagctctacatctaccgcagcactccggtgcagcagatgctcgttgactacgttaacggtagcatcatcagcaagacaaaccttaacctcagcaacgaccagctcctgaagatcattcaggaaatgttcgactcactcaacatcgccacccttagcatcgaccagcaggtcggtgtgatcgtggacctgaacgagattatccagaacatctacaagcaggtcaccgagttgctggcagctggtggtatcgtgtccgtcgccccgcgcgtctggtccggtgcttggactggcgatcaggtgggtgacaccgacttcgacatggtgggcgcggacgtatccggcgcgggcttctacgacgtgtacgtcaacggcatcggcatgcagccggacgtggactatcaggtcacgctcgctgacggcaccgatcccagcttcatccgcttcgccacggttcctgccgagggcagcatctggttcgccgtgctgcgtggttacgccaagccctacaccgggcctgcgccgatcaccgctgcgagcctgcgggtgccgatcatcacggcagagggtccgacttactacgccgccaaggctaccgagtacggactcgtgcgctgcacgtacgccggaggttgcgccgtcaacatcaacctgatccccgaagtgggcgacggtgaaaccaagctcgcctcgggcagctacttcagcgtgcagcagaaggcaggccctgtggtcatcactggcgacgtgggcgtgacgctcgaagtcccggtcggctgcaccgccgcaactcgcggcaccaactccgtcatcactgcaacgtgcatcgacggcgacaccaacacgtggttgctctcgggcgacttggctaaggagtaagcatggctaatcacttcaggctgtacggccgaccgctcatggcggacgaggttgcagatggcctgtcggtgacgggcgtgctggaagggtacacggcgggcgaggcttacgagtctcgcctgtccatcaacaacccagtcggccgctgcaccgtggaggtcatcgaatcgacgctcccttcgggcgctgcggtacgggtggacaacatcaccaaggaagtcgtcgtcaagtgggcggctttcactgaagtcgtggacgaggaaaccctcgtgcccaacggcgacttcgaggcaggcgacgacggcacgtggttgccgggcggtggatcgaatggcgaaggctggtcgattggcactggctcagactacgacaccgacagcggcgtgtacagcgcgcgcttcgccaacatcaagacgggcggcagcgacctgctcaacccgctgatccctgccaaggtcaacgactacatccgatgcaccgccgaggtccagcagggcgcaagctccaagggcaaggccggtgctcgtgtgtcgatcatctaccgcaaggaggatgggaccgagctgcaacgcaactggggcaacatggtttcctccggcagcaacggtgcgtggcaccagtccgttgccgaaggcgctgcgcccaaggacacgaagtacgtgcaggttgtactgtcggcgttccgcagcaagcagaacaaaccgctgtgggtggacaccgttaagtggaaccacaagtacgtactgggtcagaacgacgacagctcctacttccttagcatcaaggtcacggacgggttgaaccgtgtggcctactggtccggtcgtatcgaggagcagggcatctacgttacgtccaagctctacagcttctaccagttcgatgccgcgatgctgaccagcagctttgctgggtacagcaacatcgacatgctccagcctttggatactgcgtcgctgggttcctccttcgtaagctgggaactccgaagctctaggcaggattatgccgccgacccggagagcacgttgtacgggagcgctttcgtttcgttcgacatccgatccatccgtaaggactacacgcctgacccggagacggcgaagctgtcgagttctttccattccttcaccctgaagcagcaccctgtagtcaaccagccgctcgacgcgactgcacgactccggtctggcttcgtatcatggagcttcgcatgatccacaatcacctcggcattgctggcgtgttcaccatcagcaagggtaagtccctcgatactctcgaagttgtagccgactggcagagcaaccttatcacggacggtggtatggacgcactgggtgataccggcagcggctatcctcgcagcatgtacgacctcattgcttacttggcagtcggtagtggcagcgccaccccggcattcaccgataccgctcttggtgcacaggtggcgcaggttggtcgtacgtcctcggacagcggtgggactaccactgccccgtactacgcctactcccgctgccagtaccagttcccggctggtaccgctactggcgttctgtcggagcttggtgccaaagcatacaacaacaataccggcgcgtacatcctgaccacccgtgcgcttatcaaggactccgcaggtaacccgaccaccatcacggtgctgtcggatgaaatcctcgtggttacttacgagctgcgcatgtacgcagataccacgccggttgtcactactgagacgatcaagggtgttagcaccactgttacctgtaagcctattgcaatgggccgcagcggcggtatgaacggtcagtcggcagtcgcttggtcggactacgtgtgggggtgctactacttctacggcggtactggcgacggcaccggagctatcaccgaccagtatccgccggggacgattgccagcttctctgacttgcagcttcagcaggtagcctatgttccgggtacttactaccgtgactgcgtttgccggatgtcgatcaacaacgtgcccggtggtccgatcacggctgcaatgggactctccgcgtgcgtgaccttccaagtcggcttcaatccgggtatcaccaagaccggatcggagacggcgaacttgcgcatgcgggtttcttggagccggtacacgccatgatccccactgtctcccaaagcatccaacgcggtgactgggtggagcagcagaatcggcgcacccgcccgctcattgacttcgagcagggcgggctgactctcaacgcagcagtggacgacctccaagctgcgctgtggactgccgagagtgacggcagcagcgtcgtcgtttaccgcgacggcgttgccccggtcaccgtgctgaccgactccgggatcacgcagatcgcactggccttcgaccagaccatgcgcccgcacgtggcgtacatggcgggcggtgtgtgcaagttctactggtacgacacggtggctgcttcgatgcagaccatggtgatccccggtgctaccactccgcgcctgtgcatggacgagaagcgggctgtcttcgccacgcagagcgacgtgctcctgtcgtacaagaacggcagcaacctgtgcgtacgcgcgcagcgtgagcgcttcgcaaccgaacatgtgatcgcctcgggaatccccggcgacctgattgcggtgggcatgaacaacgtcaaccgcctgcaatggaagctcgtcggcaatcccgacgactggccctaacctacaggagaacagcatgaccccgccgagtgtggtcaatgaggtcgtccgaacctcgccgcttacgctcggcgcggtctacctcaacttcatcagcacgtacggtgctgccatcgtaactacgctcgccattctgtacgccgtcgctcagttctactggcgggcacgcgagcaccgaaagatcatgggaggcaaggatgtcgaatccggcaagtgagggcgcactcggtgcgctgcacgaactggtcgcgcgtgcgctgatgcagcgcatccaagatggcgagctgtgcaccgcagccgacatcaatgcggcgatcaagttcctgaaggacaacaacatcacggcgacgcgcgaggccaacaaggcactcggcgagctggaagacgagctgggcaagcactcgctgcctccggctgacgacgacgagttgcagcgtgcactcgacaacatcgttcactttccggggagcgtagccaacaatgcgtgaatcagctgaagcggccgacgtgcgccgcaagaagttggagctgttgcagaaccactaccggcacttcgccaccttcatgcgcgacattatgaaggtgctggggttcgagccgacgtggatgcagtacgacatcgccaactacatgcagtatggcccgcacctcgcaatggtgcaggcgcagcgaggcgaggcgaagtccaccatcgctgccatctacgccgtcttctgcctgatccacgatcccactcaccgtgtgctgatcgtatcggcaggcggcacgcaggcatccgagattgctacgctgattcagcgcatcatcctcacggtgccgacgttggagtgcatccgcccggacaagaacgcgggcgaccgtacctccgtggatgcgttcgacgtgcaccactcgctgaagggaatcgacaagtccccgagcgtggcgtgcatcggcgtcaccggcaacctgccgggtaagcgtgcggacctgctgatcgccgacgacgtggagtccaacaagaacagccgcactgccgcgaaccgtgagctgctgctgaccatcacgttggagttctcggccatctgcaccggcaagcccggtactccgggtcgcatcctgtacctcggcacgccgcagaccggcgactccatctacaacaccctgcccggacgtggctacgacgttcgcatctggcccggtcgctacccgaccccggcacagcgcgagcactacggcccgcatctggcaccgtctatcgtgcagcgcctagaagccgacccgatgttggcgttcggtggtggcccgatgggcgacgagggccagtgcaccgacgagctgttggccggtgagcagaagcaccagtccgagctgcgtcagcgtggaccgtccagctatcagctgaactacatgctcaacacgcggctgatggatgcgctgcgcttcccgctgaagaccgagaacctgatcgtgatccccggtggtggcgaccgcttcccgctgacgatcacccgtggcctgagcaacgctcaccagcgcagcttccagtccagtgggtacggcttcgtgatgatgatgccgcacgacatgagcaccgagactgcccccgtgcagggcgtgcacatgcagatcgacccggccggtggtggtgccaacggagacgagacggccttcgccgtgaccgccttcctcaactccaccgtgtacgtgttggccgtgggagctgtgcccggtggctacgacggtgatggcttgctagaactgcgccgcattgcggtgaagtacaagccgaacgtcatcagcatcgaaaagaacatgggctacggcgcgttcgccaaggtgttcctgcctgtcctgcgagaagatcgcggcacggagaagggatacaagggcgacatccgcgaggagttcgtgaccggcaacaaggaagcccgtatcatcggcactctcgaacctgtcatggctcgcggctcgctggtcatgctggaatccgtggttgaaatggatcacgagtacacccagcgctacgccaccagcggcaagcgtcaggtctacagcctgttccaccagatggcgaagatcacgcagcagaagggcagcatcgcacacgatgaccggctcgatgcactggaaggtagcgtgcgtcactgggttgcgcagcttgcactggaccagaacaaggccatcgccaagcagcagcagcgagagttccaagactggatcaacgatccgaccggcatgaaggcagcgacccgcaagagtccgctgcaacgtggccgtccatccctactcgaccgttaccggaggtaaccaatgcagaagtccgacttcaccagcaactacacgggtctgttcggccgtggcaactacctgcaccgcgaactgctcgccctcatggagcacgcagagcagcatcccgcaaccgcagcgcagctgctcgcgcagttccagaaggacgccaccctcgtgctggacgccctgatcgctgcgggcgcacgcaccgcgtcctcgggtccgaactccggcccgcacactccggtcgatctggacccggatgacgacccactgaccccgtaaggagcaaccatgaaccagcagcagaaccaagataccagcaacaaggggctgttcggcctgatcggcggcatcttcatcggcatttcggcaacgctgctgtcattcacccaaggccacgaaggggtacgctacgctgcgtacctcgacaccggccgggtgccgaccatctgctacggccacaccaagggcgtagcgatgggcatgacggcaacgaaggcacagtgcgacaagtggctgatcgaagacctacagatcgcccagcagggcgtgcgcaagcacctgaaggcccccgttaaccgcaaccagatcgacgcctacacagacttcgtgttcaacgtaggtgagaaggcgttcgccgacagcaccatgctgcgcaaagcgaacgcaggggatcgtgaaggtagctgcaaggagttcctgcgctgggtctacgtcggtaagctcgactgccgactgtccagcagccgttgctccggcatccccaagcgccgcgacgcagagtttgctctgtgcttgcgccccaacaacgaggtgatccaaccgtggaaaccccaagtgaagtgatcgcgcggctcggcggcaagctggttggcttgctgctggtcgtgaccatgttcgtgtgcttcggtctgtacgtctacggcctgcaacgcaaggtggagaagctggaaactgcccaagtcggcacgaccgctaccgccaaggcggcgcagacgcaggctaccgggtacgcgacctacatcaaagagaaggaggacgtgcgtgttcgcactgaagaagttcttgacgctgccccggagtaccgggatggcactgttcctgctgatgtcgctgacctcctgcgcgaacctgccggtccctgacgactccctgcttgcagactgccacatcacctacctcggtggggagaagggcaccacctcctcgcaggacaaggtggtcaagctcgcgcaggaccgccgcatggacaccgttctgtgcaacaaggacaaggctgcgctgcgtgcgtggaaggccgaggtgtgcggtaccggtaagcgccggtgtacgggtgacaaatgaccaccatcgcatgggacggcaagcacctgtgggccgatagtcaggccacgcagggcgaccacaagcacaccgtgcgtaagatcatgcccgtatcgacacccaccggccctgtgctgctgggtgtcaccggggatttcacagtgcttcgcccggttctcgctgcgcttaaagcgggcgaaggctacgaggagcacgttggcaagtccgcgacggtgcttgtggttaaggacggcgtactcacggtcactactggtaagcagcagtgggtcgaggaggctccgtacttcgatggcagtggcaaggcgctagctctaggggcctatcatgcgagcaagtctgtggctaaggccatggctgctgcgatagctcacgatgtctacagctccgggcctatcgtcaagctaaaggcaccagttcgcgaggcttaggagtaaggccacgtgggtagccggaccaaaatttgcttcggaaatgcgcgggggtcactccaatagaagctcccgcgcgtgcccccgtacgccctcgcgttacgcgcctgcgggtgtgcgtgggtgcgtgcccgcgtgtgcgcctgtgtgcgcgtctgtgcgcccgcgtcaaggttccgcgtgggtgtacccgtgtgcctgcctgcgtgggcctgagcgtgcgtgtgcgtggccgtgcgtgggtgcctgcgggtgggcgtgcgggtgggcgtgcgcctgctgcctgtatggctggacc

SEQ ID NO: 5 - DNA, 44415 bp, unidentified
  source 1..44415: mol_type = genomic DNA
gctgccttggctgaatcgttaataaatctcttggcgaaaggtgttgacgtggccggtgcggtgtggttcaatggcgtcactggggcagcgacagggcttcaggagggccgcaaggggcttgacaggggctaccctacctgctaccatgcgaaccgcagctgtaggcgtgcgagggccatctgtatcgtttcggccttttggtacacctatagcacacagtcggctcaacctgaatcaccgtctatcggtactctgtcgagctgattagttagctacccgctaggccaacggttgacgcttgcgatgcaagcagtagtagacacacggccgcaatggtagtaagctgcaacgcaagtcgagtgacgtgatccgtagtggcgccgccaacaagtgggctaagggtacacgggagtcactggtaagggatgcgaggagctaccgaaccacgcttgacactaagctagcagttagctatgataggcggcaagtggtagccaccggaacagcggagcgacctagcggtaaggctagacgtgagagattacgggtgttgaggctgaggtgagaccgggacaccggtcaagacactaacaggagcgcacatggtcctctaacggatagcttgacaaggcggcacagatagccctttgaggccttgcaacacgtggaccaccgacgtacatggtgggatggtggcgacaggacgcccaacgggttagagacccgagcgagccaagggcttgacaggatgcaacaagggtgctagtatggcaccacgctctgaggagcagccacattggatggcgtaggactaccgctaacgggtagggtgtaacgggaagcgtgccaaccacagccaatagtggccgagagttgacgtggaccgccaagctgcaacgtagcactagcggataaccggatgaactgggatttcaaaggcccatagaatccaccagacttgcaacactggtgccgctttacctaagcctaacgcttagggcttcccatctgccgtgagagtcggccacgggaagtaacccactgccaaggtgggaagccggtcataaggaggtggtgagcctcctatcgcatggaatactgtgcgtttcgtgaaaaggctctacgggccacacggtgacaatggcactgctagccggagtagggttgacagcccgaagggctagcagattgatgcgccctccctttgcgatgaccatgcaggcaaatccggtggtcagtgtgcgcccacgataggcgatgcaacggctctaatcgagaatgagggattgaccgactcgacggctttctgagggcgcatcaatctgttagttttcccaccagtgccaatggaggcacaacatgcaaggctcgatcaatgccaatctcgaccgcacccagcgtaagcgccgcttctgccagttcacccggacggcaagcgtgatggacctgcgcaccacggagcatgaccgcaagcttgccgagcgcaagcgccaagccgagcgctacgaagcccgccacggaaccgccggaaagcgatctgtgtttgttgtcgagggtaacagcgggacgaaccgggcgaaccacgccgctgacaggagggcttacctgtgatccggttcaagttctctcgacactacgtggaagctgcccgcgattcctacaatcgggccatcatgaagcatccggccggctctgtgtcggcgctctacgtcctgccgtgcggtgggcgttcattcgacatccgactcgcttaaatgcaagctactgggccttcgcaagagggcctagtgtcgtgcaatcggcacggacccaacctgaagggaaccaccatggacatcatcaccggaagcgctgacatcaagcgcgccatcaagtcgatcaacaccgcccgcaccaagctggtggaccagattcagcaggccgcgattgcggtcatcaaccacgcacacatccacggcgacgttacgctcgcttccgatctgtgtctcgccgtgggcaacggcatgaagcatgaagccctgcgcctgtacctgtccgagttcggcccgatggctccgaacgacgacaaggaaaccaaggcgagcgcgcccatgaagtttgccaagagcaagcgagtcgagggcgaagctctggccgacgtgctggaacgtgccgccgcgaaggcgtggtacgacttcaagaccgagaagcccgcagaggcgttctcgttcgccgccgacctgcacaagctgctgggccgtctggaaaaggcgaccgaggaaggctacgtgccgaccgaggaggaacaggccgtcatcaacgctgcccgcgctgtgccgaagcccaccaagaagaaggagaacgtgtaacatggaacccaagatcaaccttcgagtgacccagcgcgaagcatccctgctgcgctcggcccttcacatcgcctgtgcactgaccgcaaaggcagacccgtactccaaccgcaagctgtccaatgagttcgccgtgctgcacggtgagctgcgcgacttcggtgtcgagagcttcgagcgtgacgccatcctgcaattcgaggacgacgtgattgcggcctgccgtgacagcgatgtcgaggcacagctgctgcgcgacctgatcgcaccgccgacgttcaccgtgggctacggcatgcgtgaacttgacttcgctgctatcgaggcgcgggtgatggcgtgcctgctgtctccgttgcctccggtggtgttggatgcctcgcagctggacttcctcggcagcgtgaccggccgcatggtgttgcccggcctggcaatgcccgacaacctgccgcgtaagctgccggatgtcctgatggacgaccagagcgcacgccacgtcgccctgactgcatcgcagaccgggctggtcaacaagacgaagaccaagggctggatcgtgcagttcaatctgcgccacggcagcatcgccctcgccaactgggcgcaggtgcgtgagctgggcctgccgcagcgcagccgcaatgctgcgtaccgcatgctgaaggcgcgggccaaggtgcagggcatcagcgaggatgcgtaccgtgtggtgcccgaaggcactcccgatggcccggagaaggatcgcggcttctacaccgccgagttcttcaccaagcatgcgcggcgccctcaccagctgggttggaatacgtccactgtgatcggactcagcggcacgttcaccactgcgcaggctgcacgcaacgccatcgcctcgcacgtcggcaacgatccgaaccgtctccgccgctaccgcgtgaagtggcacccgagccgcgcgtgatctaccgctgcgccttctaacgagggcgtagctttggaaccacgcccaacaggagggcacattgcatgatccccgtaacttacaagcgcatccgtagtggggagcgcaagccgatccagctgtgcgagcagccgcgccagtggaaagagttcgtgacccatgagcacagcgtggagcgctggtatgcgtgaggtcagcctgcgccttgtggtgaaggcgctgccgctcgttaccgtgaagggtgtggctgtcggggattacatcctcggcggacatcacaccagccacgaggcgtgcgagcaagccatcgaacaccaccgcaagcaccacgagaaggtgcccaccctctactcgatagaggaaatcgaaatcccacccgtcaatcaggagaaccaccatgcgtaaggtatacttcatcgtctcgatccccaagaacagcaacgatggcgtcatcactggcgtcgtcgccaatggcaccggccgcaccccgacccaagaggaactggatgcggtgatcgccgagctgcgcaccaagggtgccaccaccagcctgctggactcgctgcgtgacggcacgtacccgaaccagctcgccatcttcgaccgccgcgccgccgtgcgtgccgaggcggatgtgctcaacagctacggcgggtcgttcttcaactggcacatcctcgaagtgggcgagagcatccgcaagccggtgcgcaagccgctgggttggcgtatcacctacgccttcgccgaagaccgcagcgactccgatgtcagctgctacaaccagcacccgagcgccaccgtgcgcatcgacggcaacgagtacaacaagagcgagtacaacgtgctgttcccgacccgcgatgcagcgcgcgccgtgttcaatgccgagtcgctgggcggcgagaacatgggctaccgtgtcgagccgtactatgcgtaagctctggctgcgcatcctgatcctgctgtactggatcgtgggtcgtggcccgtgggttgtcgtcggccagtaccatgacgacgacggcaagctgtgccggttccgcaccggcccggcttccactgggttctcgctgacgttcgatgacctcggcgcagccaacgactactgcgaccagcgcaactggaaggcagacactgacccgctcggcaccacgtactacgtgtggcatgagttggagttcaatcacttcggaacgaggaggaagtaaccatgggtttcatggacaagatcaaggctgcggccaagtacgtcaaggacaaggtggtcgcagcggtgaagccgcgccacgatgacgacgacacgccgccgcctgcgccggacaccagccggcacctgcacgtcagcgtgccgctgattcccatcgacaacccgatcctgcgcaagatgctggggcaggactacttccccgtgcagaaggggcagggtcagacccgcatcgtcggcaacaaccagctgaagcgcgtggccgatagcctcggcgggaacaacaagcagcgtcgcaagctgcgctcccgcatgaagcgtcgtgctgccgagctgcgttccggtgcatcgttgcagcccaacgtgcagtccgcactggcaggtgcagcatgagcctgcgcatgggaagctgggtcgaggtgactgtgcccgacagccgactgctcaacgtgcagccggagattgccgccgccgtgaagctgatcggcggtgcgaccatgaccaatggccgtggcctgtacgtccgcaaggacaccggcgcactggacgacgaggcggtgaccgtgatccgcttcgacctgaacttgcacagcgagctggtggaccagtacatgagcgccatccgcgccatcgtggaccgtctgctggtgctgggtgaggagagcgtgctgcgtcgccgcttctacaatggcggcggtgggtacaacagcgagctgatctttcagtaacccgagccgggtaggctacgactggcccacgtacgggccatcctatcaaccgtcaagaggaaccatctacatgtcgaacgaaaacaccaccgagcagaccaccgtcagccactacgaagccaagcgcgccgagctgctggaagacatcgccaaggcgcaggccaaggtcgatggcctgaacgagaagctcgccaagctggatgccgtcgaggccaacagcgccgccatcgaagcgctgaaggcgggcgacgccgtgtcctacctgttcggtcgtgccctgaacaagcgcgtcctgtccggcgtgatcgtcgccaccggcaagaacgacaagggcgtgctgcaactgaaggtgcagaccggcgaaggtctggatgccgagctgaacctgatcgacagcagcgccctgctgatgtcggccgaggaagtgctgaaggcgcaggaagaaatcgacgccgccgttgccgaggcccagcgcctcgccgccgaagccgctgccgccaaggctgcgggtggcgaaggcgggcagtcgtgagcctcgccccgccgtcacccagcgtggccgtcgtcaagcgtggcgacgagctgaagcccggccagaatgcgtacctgatcgacacgcggcagaccaacaagctgccgaagggcaccgggttcgtcgtgtccaagctgaccagtgaagacggctcccgtctgatcgtcagcacggacggcaacggctccgtcctgtacgccaccagccacgacatcttcgaggtctgggaataaccaagcgaggatagcatgagcgatacccttcccgacaacgactggctaccacatgccgagcgcctgcctgttggtggccgcacacgtgtggcccatgagtgcggggagggtacgcccttgcttatctcacgagagcacgacaagtccaccgcattctgtttcaggtgcggtggcacaggattcaagcgtgagcacgagagtatcgaggccaagcttgcacgaatccacgccgagcagacgagcgaacgcagagtgcgtgcgactgttgagttgccagagccacgggtatacgacacccgcgagtggccgctcgacgctaaggtgtggttcttcaagatgggactctcgcttcagatgatcgagaagctgcggctgtactggtgcccaagcatcgggcgggtggtactaccgatcactgaaggcgacaacgtggtatactggacagcccggtcggcaacgagacagccgaagtggctaacacctgacgttccgaaagacggacttgtcgcacgctacggcgtgggcacaggtgacaccatcgtactgtgcgaagacccgctcagtgcatacaaggtgggactggtaaccgaagcgtggtcgttgctcggcaccaagctgcacaacaaagtgttgaagcagctgactgatcgaggccaacgtgtagcgacgtggctcgatgacgacagaggtagaagcaacggtagcaatcccggccaagacagtgcgcgagtaatcgctgcgcgtctacgtgcgtttggtctggactacaggaacatcacgtcaccacgtgacccgaagtattacacgaccgactacatcaaggagaagctgcaatgagcaaacccatcgtgcgctaccggcgcgctatcatcccgcccgtcgttggcttccgtgccacgctcggcggcgtgcttgcgcatccgaacctcggcgactgcgacatcgtgcacacctcgacggtgctgtatgtggcggacggcgggcgcaagttcgagacgcgcaacacccggtatcaccagctcgattccaagtacgaacccgaaggagaacctgatgagtcttgacaccacgctgctgcggttgtgcaccaaccgtggcaagttcgaccggctggtacccagcgcaccacgtgatgggctggacgagctgaccgtgctgatgctcgatgcgttgcgtgcgtactacaaggagttcccggacacgaaggacttgccgttcgatgtgttcgatggctgggccatggagttcaagtggaagacgcagcccgacgacaagaagtccctgctcaaagttctgctgaagcagatgcgcgagccggtcccgcccgaggcagagcagggcatgatcgagaagctgttggagttggagcttgccaccactgcggtcagcaagatcgtgcagtggaatggcggcgctgagttcagcctgcgcgacgagctgtacggcttggccgagacgatcaccgaccgaatggatcgcaaggcgcggctcccgctggtgcaggagacgcccgaggaactgatgcagatggacgagcacgacatcggcatccacttccgactgcccacgttggcgaagaacctgcgcgctctgcgtggtggtgacttcggcatctacgccatgcgtcccgacgcaggcaagaccacgttcctgaccagcgagtccagccactggatcacgcagctcgacaacgtttggccggaccagaagcgcaccggcatctggctcaacaacgaggggccgggcaagcgcatcaagcagcggtggtatcagtcgctgctcggcgctaccatccctgagatggtggagtgggcgaaggatggtagcatccgcaagcgcatcgaagatgcgatgggcggggacatccaccgcatgcagttctacgacatccacgggttcaactccggtgaagtcgaggccatcatcaagcagaccaaccccggcttcatcatcttcgacatgatcgacaacatcacgttcaccggtggcatgaccaacggcgggcagcgtaccgatcagatgttggaggcgatgtatcaggccgctcgcaactggtgtgtgaagtacgacgccgtgggcgtggcgacttcgcagatcagcgccgagggtgagggaatccagtacccgccgcagtccgcactgaaggacagcaagaccggcaagcagggtgcgtgcgacttcatcatcatgggcggcaagctcaatgacccagcgatggaacgcttccgctacatcggcaccccgaagaacaagctgcaccgcgcaggcggcaagcgtgacgttcgggaagaagtgatgatggatgcagagcgtgcccgcttctatcaggaggcagcatgagcaagccaattcacatcgtagccaccgggttcacggtgtcggtcagcttccccggtgaatccaccgaggcgaagaccttcaactgcgtgagcaacgcgcaagcaatccaccttgccaagctgctgcgcaaggtgcacgacgcaggctacatcgaaggccgcaacgacgcgccgcagtggaagtggggatggctgcggaacaaacacagcacttggatcggcgtgcactactcgccgcacaacaagcgctggtgcatcaatctgatcccgtgcttcacgttctggatcaccaagcccggaggtaacacaccgtgagtaccgaaccgaacatctacctgccgcgcaacgtgggcgtcatcacgtccagccgcaccggcagcagctacacagtcgagccgcccgtgaccgacacggacatcgacttcctcgtgctggtgcaggacttccacgaggccatcgaaaagctggtcgatcagggatggaccctgtgctccggtgccgatggacactacgaggaggacgaggactacagcaccacgtggtatgcgctgcgcaacggcgtgttcaacgtcatggtgaccgccgactccggctggtatcagcgcgcggtcgaggccaccaccatctgcaagcgccgcaacatcaaggacaagcaggaccgcatcatcgtgttccgttgggtgcgcgacgggctggacttggatggcgatgcgtcggatgaaatgtaccagctggccctgcaacggtggccgctgtgagcttcacttccttcgacctcgaaaccacgatccgttccatcctgaagcgcaaggccaatccgttctacgacatgaacaagatcgtggcgattggctacaagcggaagggtgacgcacggaacaccggcctgtactacgacacccgagtcgggatagacaaccagtacatgggcggcgcacccgatgggtggctgcgtgagctgtgttacgggcagcagttcctcgtcgggttcaacatcaagttcgacatcctgcacgccatctgccaaggcccactcaaccggcaggcatggatcgagttcatcgacggcggcggcatggtgtgggactgccagcttgcggagtacctgctgcacggcatgacgcaagagttccacatggcgagcatggacgagacggctccacgctacggcggcaacttgaaggacgatgcagtcaagtccctgtgggctgcgggcgtggacacctgcgacatcgacaagacgctgctgatggattacctcctcggcaccaacgacaccgacgacgtgggcgacatcggtaacaccgagaagatgttcctcggacagctcgccgccttccgtgcacgtggtggtctgcgctcggcgctcctcaacatgggtgcgctgtgcttcaccatcgaagccgagtacaacggcatgtacgtggacaaggactgggcgcttacgaaggcgaaggagttggaggtcgagcttgcaacggcgaccgccgaactcaacggcttcatccccgagctgcccgagggcctgaccttcaactggaacagccgcttccacaagagcgcgctgatcttcggcggcaaggtgaagtacacggccaaggttccgatcatgtccaccgagggtgggccgacttacgtgcagaaggacgaggtgcactacgtgctggtcgatggtaccacgacggcgacgccaccggccgaggacttcgacaacctctggcgctacaccacgtacggcagcggcaagaacaagggagagtacaagaccaagaaggtgaaggtcgatgacttgaccaagcagaagttccgcaacgaggacatgctgttcgagttccctggctacaccgagcctgatgctgcatgggaaagcaagagcgatcccggcgtgtactccaccgctgccgacgtgatcgaggcgctgggctaccgcaacctgccgttcaccaaggcgcttgccagacgcgacgacatccacaaggacttgtccacgtactacatcacgacggacgagaagaccggagagcagaagggcatgctcacgctggtgggaccggacggcatcatccaccacaagctcaacatgaccaacacggttaccggccgcttgtcttccagcgatccgaacttgcagaacgtgagcaagggcgagctggacgaggagacgttggaggagaagggttcgcagatcaagcgcgccttcgtgtcccggcaccggggtggcaagatcatccagtcggactacacctccctcgaaatctacgtgcaggcaatcctcaccgagtgccgtcagctgatcgaggacttgaagcagggcctcgacatgcactgcctccgtgcagagcaggcgtggggtgagcaaggcaagtacgactacgacttcatcctgaaggcgagcaaggacgacaagcatcccgagcacaagaagtggaagaagaagcgcggcaacgcgaaggtgttctccttccagcgtgcgtacggtgcgggcgtggcgaagatcgctgcgaccaccggcatgtcggaggaagaagtcgaggcgctggtgcgcggtgaggccgagcgttacccggagctgggcgagtacatcgaccgcatggtcgagcacatcaagcgcaaccgcgtcagcactcagcgcttcgttccgcatcccaacgcggggcagcaaggcgtgccgcatgggctgacgtgtcagcttggccggtcgcactggaccacgccggacggcaagatgtattccttcagcgagtcaccgtccccggtgttcatcgccaacaagcccgcgagcaagggtggctgtgcgcagtcgttctcgcccacggaaatcaagaactacccgatgcaaggcaccggtggtgaatgggccaaggcggcgatgtacgtcagcctgcgcgccttctaccggaagtacgtgaccgaaccgaaggaatggttgggccgtgcgttgctcgtgaatcaggtgcacgatgccgtctacgtggatgcacacggcgacatcgcaaccaaggccgctgctctgctgcacgcctcgatgctggaagcgtcggtgtatatggagtggtggttcaactggacgctgccgcttggcgtcccgtgtgaaaccaagatgggcgacaacatgatggaggagaagaaccctcccgcagagttcgccggtctggtcatcgagtaccgcgcgtcgatccgcaaggacttcgtaggtaatcacaacccgtcgtttgaataaggagaacaacacgcatgagtcttgacgcactgttgaacaaggtcgccacgcagggtaaggatcagtcggtcgccagtggtggcagcttcgactacaccccgcccgctgccggtgtgaccaccgcccgcatcgtcgggtactacgagctgggcaagcacgagttcgagttcgagggcaagaagaagacgcaggatgaagtcgccatcgtgttcgagctgaccggtaagcagcacccgcacatcgaaaccgacaatggtccggtgccggtgcgcatgacgctgaccctcggcctgtccaccaacgagaaggcgcactacttcaaaatcttcagccgcctgcgcaccgaggagcgccacttcgtgcagctgctgggtcagggtgtgctgctggaagtcatccacaagccgggcaagcgcgacccgaacaagaccttcgccgaaatcgacaaggcttccatccgcaagccggtcatgccggtgccggaaatggagaacggcatcccgaccggcaagttcgtggacaccgtgatcccggtgccgcagcagatcaccccgctgggtgcgttcgtgtgggacttcgccgacgccgacatgtgggacagcatctacatccccggcgagtacccggagcgcaaggacgagaagaccggcaaggtcacccacgaggcgcagtcgaagaacaagacgcagctgcgcatcgctgcggcgctgaacttcaagggtcttccgtgctacgactacgccgccgccaagttggcgggcagcaccacggtcaccaaggaaggcgtcgatgcgctggacgaagtggtcggcgacgtggcgaacgccgcgcccaccgacgctgctccggccgacgacaagccgccgttcccggtggacggtagcgacccgatggcaggcatcgcctgatggacctgagcgctctcatggcagcggccggtgagcgctccccgatgccggtgcaggtggtacgtcagcacaacccgcgcgtgatcgctcacgttgatggggactacatggcgtacttcgcggctggtagcgagaactgctcggcgggggatgcacgacgcaacgtgctctcccgctgcgcacagctgaagcatgtcagcggagcgggcaagatcgtcatgcacctgacgcacgccgcgtctaccaagggtgatcgcttcctcgctgctaccacgcagccgtatcagggtcagcgccaagcaggccgcaagcccaacaactgggcgttccttcgtgagtggatggagacatacgagggcgacgctttcactcccaaaatctggctgacccgtgaggccgacgatggcatcgcgtacgtcaacgagggtgcagcattgcaccacaacatcctgcacgtggtgcacagcgccgacaaggacatgcgaatgttctgcggcgtgcacgtagactgggacggctacgacatcacagaggttccgctcggcgcttacgacatcgttggcgagaacggattgcagtacggtcacaagtggttctggatgcagatgctccacggcgacaccgccgacaacataccgggtctgccgaaggtgggcaaggtgacagcggagcagctgctgttcgagacgaagaccaacctcgaagcggtgcagatcgtgagcggcaagtacagcgaagtgttgggtgccgactggcgcaagacattcgccgagcaagccgtgctgctgtggatgcggacggatcgtgacgcagaactgctcgacgtgctgaagctcgacgtgttcgggccgaagctgaagcaggcgttctatgacctcgccgaggacgtgaacgagaagcgtgcaatcttggaggcatacaaagcatgaagcgactcactgcaacacaggtcaagctgctgcgcatcaagctcgcagcggagcaaggcaaccggtgctgtctctgtcagggacagttcggcctgaaggctccgctcgatccggtgctggaccatgaccacaagaccggcgctgtgcgcggggtgctccatcgcggatgcaactccctgctcggcaaggtcgagaacaacgcaggccggtacggcgtgcgcgacgtgttcgcattctgtgcgggcatccccaactacctgcggtcgcacctcaccaacatcacggggtacctgcatcctacctacaagaccgacgacgagaagcgtatcgctcgcaatgcgaaagcgcgaaagcgtcgggctatcaacaaggagacaccgtgacccttacccagttcattcgccgagcaccgaagcgcggcccgaagattctctgcctcgacatcgagacgttccccatcgagttctatggctggggcatgttcaacaacaacttcagcgtcaagcagatcaagcgtgactggtcgctgatgtcgttcgcttgcgaatggctggacgacgaggcgtcgttctacatggaccagcgcaacgtgcgcgacgtgttcgatgatcgcaagcagggcaaggcgctgtgggcactgctcaacgccgccgacttcgtgctcgctcgcaacggcaagaagttcgaccttcgcaagatcaaggctcgcctcgcaatcctcggcctgccgcccgtgtctccggtgcaggtgatcgacccgatgctgctgaaccgcaccgagttcgccttcacctcgcagaagttggagtacaccaccggcgtgatcgtgccggagctgcgcaagtacgaccaccacaacttccccggcttcgacctgtgggtggcctgcatgcagagcctgcccggagcatgggacgagtgcgaagcgtacaaccgcatcgacgtgaagtccatgaagttggagtacaagaagctgcgcggttggtactcgcagcatccgaacgtcgcagtgtactacaaggccgacggcagcgagcaccgctgcaacaagtgcggctgcaacgaaatgatcccgcaggatgatccggcccgcacgcaggtcggtacctacctcctgcttcagtgcaccgtgtgcgacggctacagccgtgggcgcaagctcacgaccagcgccgaggcgcgcaagcacatcaccgtcccggcataaggaaccgacatgaagatcaccgacatccgcagcggcatgcgggtacagtacatcggcaatgcgcccgcaatgatcgggctgcgtggacaggtaagccgcgtgttcgctcgtgatgtcgaggtcttcttcgacggtcgagttaagccgagctgctgcgttcccgattccctccgacagcttctcagcatcggaggcgtgaccaccaccagacgagaggtaccaatgcccgaactgagctaccgcgacgaggaccgtcgcacactgtccgaccgtggcgtcggcctgaaggatgacgggggcaagccgcaggcccgtctgctgcatgagggcgtgccgcgtgcactggcccgagtcatcgacaccctgaccttcggcgcgcagaagtacaaagcgcactcgtggcagcatgtcgagaaggcgctcgaacggtatcaggacgcgagctaccgacacgacaacaagcgctgcctcggcgagaagctggacccggagacgggcatccaccaccgggcgcaccacatcatcaacgagctgttcctgttggagctggaactgcgcgaggaggagaaggccagtggcgcagagtaaggcgcgctccatcaaagaggcttgggtgaacatcggcatcggctacagcatcaactacgcagcgaacatcgcgctgcttccggtgctgtggcatcccgagcatccgctgctgtcggcgcacgccatcggcattgcgttcacagcgatcagcttcatccgccagtacatcatccgccgctggttcagcaagggtgactgatggcctgcgcccgctgcggccaagtgcatcggtacgtcccacatgaggccgagtgggcgcgcttcctagaggagcaccgtacccgcaagcagttcgatgtcgagtgggccaactcactctggcatcgtacataccctgacgacgcattctgcatcctcgtgatgaggggcctcgcaggtttcgttccattcccgtcgaaggagaactgaatgctctacaagaaccagaccgccatgctcatcaagtcctacgagaacgccgttgcgtggggcgagagtgccgaccacgaggaggcattgcagaatgcggtcaaggccgggttcccgaacctgcccgacgaagatcaggccgagctgtatacccgcatcgccgatgcgtgggaaggctaccgtggttcgctcgctccgcgcaagctgtggatcggcaccatcgtcaaccagttcatgtcgtcccgcatcgcacggttcaacgccgcgctgggtgacggcaccaagaaggaggacagcgccgatgtttgatgtgcctcgccagaatgtccgggttgctcccggctacaagaagcgcaagcgcggcttcaagatcaaccgcgccttcaccaagggcaacttccgcgtgcagtggtacgacggcaaggccacgtactgggagcgctacgttccgtggtacgaagtgccgctcgccatgttccagatttggagggactacgcatgagctacatcgtccacaaggcagtcgagcaggacaagatcaagaagaagctgcggcccaccgaggagcagcttcgcaccgagtacatcgcacagccgaagtacgacggctgcaacatggtcgccatcaagcgcggccactgggtgcccacggtgaacaagggcctgcatgccatcaaggtgggcgacgtgcagatgcagccggtggatcgtggcgtggttgacctgttctcccgcaccggtgagcaggtcgtcagcgcacaccacatcgagaacgctctcgcatccgcgccgttcttcccggtcggcgtgtacttcggcgaatactggcacccgcagatcgaccagcccaccgtcagcggcatgttccgcaagaaggacggcacgcagtacaccgagccgatgttcgtggtgttcgacttcgtgacgctggaagaatgggagcagggtttcagcgacctcgtgtatcaggagcgcgtcagccgcctgccgagcatgggccacgccatcgccgagggcaccgcgccggtgttctacgccgagtcgcagggcttcctgatcgaccaagagctgggcagcatggaagcggcgaagctgctgtgcgagggcggcgcgtacgacgggctgatcctgcgcaagccgagcggcaagtgggtgaagggcgacaagggaaccaacggcgaagtcgtcaagatcaagccgaccctgacgctggacctgcgtgtgctcggcatcaacgaagcagtcggcgagaagaccggccgcgccgtgtacacggtcgtcgttgacctcggagaaggcaagacgcaggaggttggcagcggcgtgccgcacagcgagagcgagctgcctagcgtgggaggcatcgtggaaatcgaggcgatgtccttcagcaagtacggcctgctgcgcgagccgcgatacaagggcatccgtcacgacaagaaggaggcagacctgtgagcgtcgaggtgcaagcatggcacaacatggagcgcgacacggtggagctgcgcatcagcgttcctttcggcgagtacgccggttccctgtggccgaacgagacgctgcgcgacaaggtgcaggaagcgttcgccaagttccttgacgagcggaggggctgatggacgcgatcactttcgagaagccggagctggacttcagccagtcctcggcatggatgggccgcgtcgaggtttcggtgcgcgcccggtacggtgccgacttgttcggcgctgctgccacgtgcatggccgaggatatcggcggtgaggcgtggccgcacatcatccacgacctgcacatggaaatcatgcgcggtatcctgaaacgctacccgccgcgcgactacaccgtgcggcagcaacggaggtaacaatgctctcgcaagtggaactcgaactggaaacctacgccttcggtaaggagcgcatggagaagtccatcgcccgcaacgaggagaagggcggcgcggacaacaacccctacgcccaagcagtgtatcgccggttcgtgcttccgcttgcggagcgcatccgtgcggacatcgactctccgcgaatcggccgtgcgcaagcgcacgtgccacttctgcgcgccaagtacgatcccgagcgtcagaacaagcgtggacagcccgtcagcgccgaggaacaggcacgcgagtggtacgaggctgtggccttcgtcgccgttcgcggtgcccttacctcctgcatgcgagacaagcacggcgaaggcagcgaccgcgacgtgttgaagaacgttggcatcaacgtgtaccatgagtacctgctgacgcagttcgccgacgcggagccgactctgttctaccacctgatgaacgacatggaccgcaagctctctgtcaacgagaaccaccgcatgacggtgatgaagatgcaaggacgcaagaacggcatcgagttcgtggagtggggacaggcacagcgcgatcaggtcggcgcgtacctgtgcgatcagcttgcgcagctgggcatgttggagattggcgtggtcaccgagactgctgccagtgcaggcgcagcgtaccgcaagttccagaccaagacgcacgtcaagatcgtgctgaccgacgaggtgcgcaagctgattactcagatcagcgacttcgtgatcgaggccacgccgttctacctgccgtgcgtcgagccgccgatggactgggtggacatcgacaacggtggattccacacgaaggaaatgcgccgactcaatccgtggatggtgaagacctacgctcagacccgcgacgagtaccgcgctgccgagctgcgcaacgagatggctgcgatcaacgcattgcagcgcgtgccgtggcgcatcaacaagcgactgatggaagctgtgtcggccatcgccaaggtgcacgacatggaggaaatcatttctcagggcgagctgccgaagccgcgcaagccggagtggctgacgaaggacatgaccaaggaaaccatgtcccacaatcaggagttggagttcaagcagtggaagcgcgacatgtccaactggcacaccgacgagcgcctgcgacagaacaagggcaatcgtttctacaacgcaatgaaggtggcgcgcaagttcgccgagtacccgagcatctacttcgtgtacttcgctgacttccgtggccgcaagtacgttcagaccaccggcgtgtcgccgcagggttcggacttgcagaaggcgctcttggagttcgccgatggcaagccgctgctgactaaggacgcgaaggattggttctgcatcacaggagcaaaccgatggggatacgacaaggcgtctctgccggatcgtgtgaagtgggtagcggagcatcacgaccagatcatggcgttcgctgcggacccggtgaacaacgacgagtggaagaccgccgacaagccgctgcaatttctgagctggtgcatggagtacgagcagtggcaagtgttcggggatcgcttcctgagccgcatcgcagtcggcatggacggttcgtgcaatgggcttcagaacttctcggcgatgctgcgcgacgcagcaggcggcgtggcgacgaacctgatcccagcaccgctgccgaatgacatctaccagatggtggcagaccgcgtgactgccgtcctgctaggcgaggacgaggatgccgaagggtaccgcacgctgtggctcgaccacggcctcacacgctcgctggtgaagcgcagcgtgatgaccctgccgtacggctcgcggcagtcctcgtgggcggacttcatcatcgaagactacctgaagtgtgggaagttcccctcgctcgacaaggccctgtacggccccgcagcgcgcttcctgagcaagcgcatgggtgaggccatcgccgacaccgtggtcgccgcagcgggcgcgatggagtggttgcagcgcggctccgggtcgatcctcaaccaagggtacgaccgcatccggtggatcacgccgtccgggttcccggtggtgcaggtctactgggagtccgaggagcaccgcatcaacaccaagctgtgcggcaacgccaagctgtccctgcgcaagagcacggacgcggtgaagaagtcccggcaccgcaacggcatcgccccgaacttcgtgcacagcctcgacgcaagccacctgacgctggtggtcaacgcggccaaggccgaaggcatcgacgccttcgccatgattcacgacgacttcggcacccacgccgccgacagcgcggcactgtaccggatcatccgggaggtgttcgtgtcgatgtacgagcggcacgacgtgctgtcggccttccactcggcctacccgttcctgccggagccgccgccgatgggcgagctggaccttcggcaagtccttgattctccgtacttcttcagctgacggagtttcagtacacctatagcacgaggcaactgaggtccggttggagcggccgcgaaggtaagcggaaccggtgccggaccttttggtacacctatagcacagaggagacaccatggccgaagacgccaaagtgaaagtcctgatgacgctccacccgaaccagctggccgccgtgcggaagctgtccgggctgtcgctgtccgtcaactcgaataccacgcccttggaggcaggtatgcagttggggatggcccgcgtcctgaacatcttacaggagggtttcaccgttgattcctccgtaccgaacaccaacgacgggtgatagtgagcagatcaaggcggctttaacggccgctttgtatctgtcatctagagaagatagtaaggtagacaacagagaatcttctgtgagctacaactgtgatgaccctgattacacagtggccctgataacacagggtctagtggatgcagtaatcattgatgaagcctacctgctgtgctttgccattgtcacaccgtggtactccaagaaccgtactacgttcgttgagaacatggtgctgcgaattgggccgggcagttccttcgaccggtacatagccgtgatggaacatctggctgacatcaaccactgcgactcactgagcgcaggcggtgcactagctcggaactcccgagcactcacacggatgtatgcacgctacggctacctgctggaacggcatgctccccaattcaccaagcgaaggagttaacctatgggtagcatcgttggtggtgggtccgccaagcgagcagcgctgaagcaagctgctgctatcgacaagcagaccaacctccaaactcaatccacgaactaccagattcaggcgatggccgatcagatggcacaggcagctgcacagcaggccgcatctgagtacgccgagaagttgctgagtgcccccgtcgataccgtcgatgtgcggctgggaacttccgacctcgacttgcagactgccgacctgatcggccgacgcaagaccgcccgctccacttacacccgacccgtgaccacgaccgcagcttcccggctgacgaccgtggccgggtcagacctgttgtgaggtgagcatggaccatccgatccaaaccgctcaccgccagttcgaggcttacgacaacaagcgacagggcatcatgtaccgactcgaacgctattcgagctggaccgtgcccaagctgttccctcgcaagaaccgcgatcaggacaccgagccgctgacccacgggttccagtctctcggcgcgcaggcagtgaaccatctggcgaacaagctgatgatgtcgctgttcgcaccgtcccgcccgttcttccggttggagctgaagcgcaaggcgaagcaggctgcgcaggagcaaggcgctgacttgcaggccatgcaggcgatgcttgcgaaggccgagcaggatgccagtctcgaactggacaagcgctccatccgctcccggctgtacgacctgctgaagatgctgatcgtgctgggcaacgccctcatggtgttggagaaggacacgatccgcgtgctcaacatgcggcactacgtggtcaagcgcacccgcaccggcgaggtctacgaactgatccttcgggagaaggtgcacaagacccagctggaacccgcagcgctcgctgccattgtcgcgcacccggacttcaagcccgatgacgacggcatggtgtgggagtacaagtgggtcaagctggaccacaagaccggcaagtacaacgaagacgtgtggatttgcaactgcaagctgcccgccaacttctcctcgacctacaccgcagacaagctgccctaccgggcggttagctgggacttggccgcaggcgatgactacggctccggcttggtcgaagactacgaggccgacttccagtcgctctcgatgctgtccgaggccgcagtgcagggcgcgatcctcgcctccgagttccggtggctggttaaccccgcaggtcagacctccgtcgaggacttcatggcgtcgcccaatggcgcggccattcccggcatgaagggtgacatcgagctgattaacgcaggcgtcgatggcgtgctgcaaaccaaccaagcaatccagtccacctacatcaaccgcatcggcgcaggcttcctgttgcagacggcggtgactcgtcaggcggaacgtgtgaccgcgcaggaaatccgcatggtcgccgaagaactggaaggcgggctgggtggcggctactcccggatcgctgcggacgtgcaggtaccagtcgccttttgggtgatgaacctgacgggccgcgacatccgaggcaaggacttggagcctgtcatcatcaccggcttggccgcgctctcccgtacgggtgaccgtgaccggctgttggagttcggcagcaacctcgccaacgtcctcgcactgccgccgcagattctcgaacgactgaagctgtccgcgtggatcgcagacctcgccgccgctggtggcttggacccgaacgtctacgtgctgactgaggccgagtacggccagatgatgcagcagcgtgcacagcagcagctcgccatgcagaacgcatcccagcagatcgacaacgccaacaacatggagacacagacacaatgagttccaacgcacctccgggcggtggtcccggcgcaaccgtgatcgcaacctcgaacggcaaccagcccgcaccggcagctccggctcccgcagacgacaagctgttgcccaacggccagcccgctccggccgcaccggcacagcccgcagctcctgctgcacctccggctgctgacgcgctgagtctcgaacctgccgctcccgcacagcccgccgccccggcgaacgctgcgccgactgcggtgtcgatcccggactacggcgacaacggcctgaacatcgcggccgaatacttcgtcaacaccgtgggcctcgacatcgacagccgcgaactgaccgaagcagcgaagggcaacttcgccctgctggaagccaagctggaagtcctcggcgacaaggccaagggttccgcaccgatcctcgctctggcgaaggagagcatcgctcgtgtcaccgccgctgcaaccgcagcgcacgccgcgaacgttgctgctgtccacgaagccgtgggtggcgcagagaactgggctgcgatccagcagttcgcacgggccaacctgcccgccgaccaactgaagcaggcaagcgaatcgctgtcggctggtggcttcggcgctcaggcgaccgcgcgttacctgatggctctggcacaggccaatcccgcgacgaccgtcaagggcgcaccggctaccaacgccgccgcccccgccgcgtcgatcaacggcgtcgctcctatcacgaaggagcagtaccgcgctgagtaccgcaagctggttgccgagaagggcatccgtggtgcggcccactccgaagaactgcgtgcactcaacgcgcgcgtcatccactaagaccaaggagcaacacaaagcatgagcaccatcttcccgactgtcccggttctgccgaatcaggtcaaccagtccggcaacgagaacgccctgatcctcgaacagttcaccggcgatgtcgagcacacctacgtgtccagctcggtgctggaaaagttcttcccgcgcaagcaggtcaagggcaccaacaccctgaccaagaaggccatcggccgtaccaagcttcagaagctgaagcgcggtgacgcgccggacggcaccccggtggacttcagcaaggcgtcggtgaccgtcgataccatgctgctgtcgcgtcacagcatctggcagctggacgaaatcttcaccgacatcgacacccgcaaggaaatcgccatcgagcagggtcaggaaatcgccgagttcgtggacctgaccatcagcatcgccgccgcgaaggccgctgctgccacgcagtcgatcttcacccgcaacggccgcgcgcccgagggccacttcggtgccacgcaggtcgtgctgtccgccgctggtgacgagaacgatccggccaaggtgtacgccgccatcggcaaactgttctcccgcatggaggaggagaagaaggtcaagccgcagcgcgatggcgtggtcctgatcgtgcgcccggcgatcttctacctgttgcagcaggccgagcagatcagcaacggcgagtacctgacctcggacggcaacaagctgaccggcatcccgaccttccacggctggggcgtcccggtgctgtcgagcgagaacctgccgaacaccgtgatcgaaggtcacctgctgtcgaacgacgacaacgacgacttctacgacggcgacttcagcaccctgatcgccgtggccgtgtcgccgaaggccctgctgatcgccgaagcgctgccgttgcagtcctcggtgtggtggagcgatgcctcgaagtgctacttcgtggactcgtggatgtccttcgccgttggtctggatcgcgtcgagaacgcgggccgcatcgacaaggttgcctaatccgctgggcgcggtccctgaatccttcgggtaactcaaaccgcgcccttcttccaccaacacaggagcaacatcatggtctttgaccgaccgttcgagatttccaaccgcgtcgtcgccgcaactggcgtggccggtctgcccgccaactccgttggtaccgtcgtcggcgtccactacgacacccgtggcaccgcaggctgggtcgtccgtgtccgtttcgtggacgacgaaatcggctcgcaggacatcgagtacgcaccggccgctctggctctggctgcggactaagcaacatcccggcaggggcgctccggcgtctctgccttgttcctctcaggagacaccatggcattcatcaccaagctcgacatcgtgaacgcctgcttgaagacgatgggcgagacgaagctcaacacgctggaagatgaccacgtatacaaggacgacgccgttgacttgatcgaccgcgtgcaccgtgacgtgtcctcactctcgctgtggttcaacaccgaatgggtggagctgaagccgcaggcaacgagcaagtacatcatggtccccacggacgtgctgaagctggactgcaacccgagccggttcggccacgtggtgcagcgcggacgccgactgtacgaccgcaagcgcaacacctacgagttcgaccacaacgtgcaggccaagctggtgcggctgctggacttcgatgacctcccctacgaggtgcagatgttcgtgcgcgacgactcggtgctgcggttccagtctgacttcgacggcgacaacaccaagtacgccaagatcaagcagcagcgcgatgacagttacatcaacttgaaggccgagcacatccgccagatcaaggcgaacccgctgttcgctcgcgcatccgtggacgtgctgcgttcccgttactggaactacagcggtcacccgtggcacagccacgtcacattccccggctaaggagacaacatggcaaaggcaggcggaacctatcccgacatccttcagggtgtcagtcagaaaccggcgcatcgtcgtcggccgggacagacgcacgagcagatcaacgtgctgtccgatccggtgaacggcctcgtgcgccgtcgtggtacgcggttcgctgcttcccaagccgttgtcacctcggccgagctgcgcaacatggacgtgttcgacttcatgcaggagggcaaggagtacgcgctgctgtaccggcgcgacgcctcgaccttgggcagcgagtccttcgcgttcctctacaacaagacggacgagtcgttcatccctctggtgtacgagaacagcacgtgggtcaacacgctggtcagcggaggcgcatcgtcgctcacggccatcggcagctacgtctacatcgcgggcaacaccacgatcccctcggccaccagcacgaacgtgtggcaggagcagacgaacatccagcgcctcgcagcatgggtgcgcaccgggaagtacaacaccacgtacacggtgaacctgacgcggacggacaacacggtgctgacggtaacgttcaagacggttaccgcatcgtaccccggaacgctcgacaccagcgacatcccgttctaccttcccggtggcacggagccggacgcggcgtaccagaagtacgtcaacgaccgagtgaacgagtacaactctgcggtcaacgagtggatcgtgacgagcgctgagcagacgcgcccggagtacatcgcggagcagctgtcggatttgctggtcgatgcaggcgtgtcggcaacgtacatcaagggcgggatcatcattgacgatgaccagttcaaggacatcacggttgacgacgagggagacggcacgaccttctacgccgcagggcaggaaattacagacgcgacctacgccgtcaagttccactggcacggcaaggtcattcgcgtgcggccgagtggtgcaggcgcggacgagtcgtactacctgcgcgctgagttggagaacggcgagacttccggctacgggtcggtggactggtacgaagcgcccggcgtggagtgcaccatcgacaacctcgtgtcgcagctctacatctacaacggtgtaggctacatcgcacgcaacggtgcgggcctcacgtctctggctccgagcagcggcgagcatccggcctacggtgcgcgagtggcaggcgatggtctgacctcgccgatcccgtggttcatcgacaagccgatcacgatgctgtccgtcttccaagaccggctggtcatcggcgcacagaactacgtcaacgcctcacgctcggcggactacctgaacttctggcgcggctcggccgtcaccatcgaagacagcgaccccatcgaaatcttcgcgcacggcagcgagggcgatgtgctccggcacgcgacgctctacaacggcaacctcgtgatcttcggtgaccgtcagcagtacggcatcagcggcgactcggtgttcagtccgaagaatccgctgattaaagcgttcagtgccaacaaggattcggttgacgcgaaggcgcagacctcgggcaactacatcttttatgcgcagtacggcagcgaaggcacgagcctgcaccagatgcgagtgggcgcgctcaacgggcagcagacggtgacggacgaaatgtccaacgagctggactcgtggctgtcgggcactccgttgcagatcaccccgctcactgcgccgaacctcgtcatgttccgcactcgcgagcacccgcaggacttctacctgtaccggtacgaggacaacaagaacaacgggcagcgcatcgtggatgcgtggtcgaagttccggtaccacccggcgctgggcgaaatcatcggcgtgagcagctacaagaagaacggcctcgtgttcactgcgcgcgggtcgctggtggcgtgcgacgtgttcgacccgaagggcgagccggactcgcatgcgtgcctcgacagctgggcgagttttggtacacctacgggcgtacagactgcgagcgcaagcatcgccgtcaatagcactagcccgtacttcctgctgggttgtccctacgcgcaggcgtctgacttccttaaccagttcgatgacctcgctgctggtgcgctggaatacggcgtggtgtccgaagctctggtgatcccgaccaatccgttccctcgggaccagaacggtcaggccgtactcgatggacgcatgtccctcaacaaggtgacggtggacgtggagaacacggcaggcatgatcgccacggtggcaacccgcaacagcaatgtgaccactacggacttcgagggccgcatcctcggcgactccgacaatctgatcgcgcggcaaccggtgtaccgggggcagctcaacatcagcgtcgggcgcgaagtgcgcgagtgcacctacgagattcgcagcaaggattggctcccgctccgggtgaccggcctgagctggacgggtcagactttcaacaatgtacggagggttagctaatgggttcggttaatacgatcctgcaagcgaacaacaccacccgcgttgcccgtgcgaactaccgtgcagccgttgcgcagaccgacaaccagaaccgcagcgaggtcgccaagaccggcttcgctgatttcatgcggtccctgaagaacaacgcccaactggacgccgccgcgaaggagtacaactccaacatggaagcgctgtccgaggagctgcgtgcgcgccaaggggctgggcttaactcccagctccaactggcgaacgcgcgtggcgcacttcaggcgcaggctggtgctgtcggtgtcggcggctcgtccgcagacctgatggattcgatggtgcggttgcaggcggaaatggatcaggagacgcaggccaacgctgtctcgctcctcgcctcgcggggcgcatcgcagactgcgcagatcatgtcgcgcgcgtggaacgggatggacatgagccgttcgttcgggcagttcgactactcgcagcacatcgagccgcaggcaatgaagcgtcgcttgggcaagctgatcggcgtggccgtggctacctacttcggtgggccgatggcaggcgaggccgtggcagacttcgcggtcggcacgtggcaggcggacaacggcaacttcactggtgcctctcagtccttcagcaacgcagcgcagaacggtatgcaggcgtggcagcagtccaatgatcgcggcggcaagtcgtgggcgtccactaccttcgggtacaacgacggcaccggcaagcagtccgtgactggggcgaaggtcaccggcaacttcggcaacaactacgacaacttctccaccactacgtccggcctcggctggttcgatagcggcagcggaggcaactcaggaggtgcatggtaatggctgacatcggcacggttaccttcaacacgcagtccgcattgcagggtggcatcaacgccaccccagcactgtcgggcaacaccagcattcaaggcgctggtgtgaatcaggtcgggccggttcaatccggcaacgactggttcgcaagcactggtggtatgacgatgccggacagcaacctgccagagttcttgcaggagctggcagcgccgaacaccgccaagctgaagcagcagcagatgtgggacggcttcgttgccgcccgcgctggtaagaccatggacgagattgctgcgaccgaaccgtggtacaagaaaatcttcggagacaccaactacgagattggcgcgagcatgtataacacgctctcgcaggtcaacgaaatggagagcgacttgcttcggcgtatgccggagttgcgtcagcttcctcccgaggcgatggcgaaggagttcaacgacctcgccactgcccgcatgaccggcaacggtttcgcggacacggtgttgcagaagaccttcatggatcgcgcgggttccctcatggacctgcacaccaaggagcgcacggcatggcagcagcaggagctggtgaaggcgcagtacgctgcgaactcgtcggcgtccaccggcttcaacgaactggcgaagcgcacggcgatgctcggtaccaaccgtcccatggacgagaaggccaccgaggcgctgacgcaggcgcagctgtccctgctggacggactgtcgccctcgcgctaccagacggacgagtcgtacaagtccgcgatcactgcgttctatcgtggcgctgcggatcgcggcgagttccacacgctgaagttcctcaacagcaagggcgttctgaacgccatcgacccggacgggcagctgggaatccagcagtacgtgaagcaggcgcaggatcgttaccgttccgactggctcgatgccaacccggagcaggccgagaagatggcgctcgtctccatgtacgcatcggagggcattggtgccaagccgtcgcaggcgatgatcgaggaaatgaactcgacctacgccgccgagactggaagcgacgcaccgctgtactccggtacgcagttggcttcgatcatggcacagtccgcaggcgcgcacatccgcgcacaggaagccgtcatcaaccagcgtaacgctgcggccaaggccgcgctgaccgaccagcagaagctggccgcgcaggaggaggacatccgtggtggcatcgaagcgttcaagcgcggcacgtacgcgcagacgatcaacatccccggcgtggacaaggagctgatcgaggcgaacacggtgcaggcatggaatgccacgatggccgcgaaccccaaggtcgccatgtcgcagctggtgtggaacgccaacaccgggcgaggcgctgtgctgaagggtgtggccgaccagttccagaccacggcgcgcgctgtgctccgcgatcagccgaacacggcagcggctgcactgtaccagcagtggaaggaactgaagcagaccaccgccgcacgcatcgacacgaacggtcagcccgtgcagggccgactgactggcgcgactaccgctgcgctgtacttcggagatagcgtcaacacgttcttcaacaagctgcaagcgttggagaatggtggcgtgaacttcgagcttgcttacgaggtggcccgtggagaaatcaccaccgacgatccgacgcagttcgacgcgaacagccgtaaggaatccgaggctactcaggctcgtgttacggaagctatcgccaagctcaaccccaagtacctcggcatgttcggcaacaagctgggcgactctggccgcgctgcgtatgctcgcgccatcgtccgctcggtcactgacaccggtggtctgctggacacttctgcggaaggcttgcaggctgcggctactcacgccaagctggcctacggtctggaagacgcaggcaagtacgcatgggaaaacggacgcgacgacgaaggccgagtgatcggcagcgtcggtgcatggctgggcttcatggacacgaaggaaaccggacccgccatcgagaaggccatcgacgcagcactgcgccgggtcaacatcgagccgagcaccgggctgaaggctgacgtgttccgcatgaaggacagcgagaacggcgagccggtgctgtacgtcaacgctgttggcgagaagggctggaaggttgtgccggtgtacgggcgcgacatcaaggacgagtacgagaagcacaccaagcagcagcgtcagttgcaggccccggtaccgcagggctacgttcgcatgaacgacggtacgattcagcagagcatttccatccaacccaaactgtaaggagatagacaatggcactcgatctttcggggctgacccaagaccagcagattgccaaggctgccgcttatgcgggagtgccggagtccatcgtgcgcggtcagtggcgagtagagtccggcaacgggcgtgccgccaaggacgctgacggtgtgatccgcagcaaggcaggagcacagggcgacttccaagtcatgcccaccacgcaggcaacgtgggaagcgcgcaacggtcgcaagtacgacatgcgcaacttccaagacagcatcgagctgtatgccgacatcatgcgcgagaacatgcagcttgccaagggcgacgtgacgaaggcgctgcgcatctaccaaggcggcaccaatccgaagaactgggggcaggagaacgcagcctatgcaccgagcgtgctgggcggtgcgtccgctcccgcagtgtcggcgcagccgcgcagcctgaccaccacgcaggcagacctcaacgccgcatggcagggcaacccgaacatgcgcgaccgtacgtggtccggtgcgtccatcccggatgcgtggacgggtgcgcccatcgaaggccgcaacgctctggcgtcggcagcgaaggaacacatcggcaagattcgtgcgggcatcgccgagctgtcgatgggtcaggtagcacaggaaggtggcaccgccgcgcaggccgtaggcaaggctcaggctgtccgtgcatcggatcaggttgtgccgtggtgggtgcgtcaggaagtggacgtgctgaacaccggcgctcgcaaggcgctgctggatcagaccgaacaggcgctcgcgcaggaccgcgcggacgaggagctgcgcaactcgctgaccttcctcgacaagtggggcgctgcgttcgacagcggcatcggtgctgcgatcagcaaccagtttgcgcgcgaggacgagaacgttccggaaggttggaagtacgacccgaaggaatgggagaagccgtggatgactgccgacgaactcgaagacatccgcgatgcagcgtactcgccgaacgagctgaagtacgtcagcgaccgacagttcctgcgccgccactccatgcgcatcaaggatcagcagactggctggggtagcttcggttacgacatggtggcaggcttcaccgatccgggcaactgggctatcggcggcgtcactgccgcaggcgctaaggcgctgggcatcggctcggctgcactcgttgccgaagggcgcgtgggcgcgtcgctcgcgtcggctgctgcggagaacgcggtcggttccgtcatcacggacgccgcgctggttggcatgggcgagcgccgcaacttcgcggacttcatgaccgacgctgcattcgctaccaccataggcaccgcgatgcacattccgggcgtgcgctcggctgcgcagattcgtgacaaggcaaccatcgacctgtccgcaggcaacgctgccgcttacggcgaagcgtggtcggccgacctgaaggcgcgcgctgtggccgagctgggcgaggacgccaacccggtgctggtgaacaaccgcatccaccagcttgccaagcaggaggctgtggattggctgcgcgctggtatggccgacgtgcctgacgacttccgtatcttcgcccgtcccgacgtgcaggagacgaccaccaccgcaggcaccactggtgcactcgcacgggacgcgggcaacgtggacgcaacgaccgggcggtacaacgacagcgtgggtggccgggtcgatcagcatgacccgctgctggaacgcgcatggaagaccgcaggtatcaagggcggtaacgtcgatggcgtgctgaagtatctggaatccaacgcctctatcccggaggacgtgcgtgctatcgccaacgcgctgaagcgtggcgggcggctgagcacggtgaagatcgtgccggaatcggaactcgacaagtggttcgccggtgccaacatgggtccgggtatgcgtgtggccggtggctacaacgccggactggacgcgatggcgatgcggaactacacgccggaagtggtggtgcacgaaatgctgcacgctgccacgctgcgtgagctgcgcagcaactcggtgttcgggcaggaaatggaagaactgctgacccatatcaacaacagcatcggcagtgtggactccacgctgaccaccgctgcgatggagacgcgcatcaaccagccgcaggcaggcttcctcgccaacactgacgagctgatttcctacggcctgacgaaccgcgctgtgcaggcggtgctgcgtcagatgcccgcgccgggcaacacccgcccgaatgcgtgggagtggctgaaggataagatcgcgcgagtgatgggtctgaagaatcaggagtccgcgctcgaacgcctgatgtcggtcgtcggtgacaacctcggcgcggaagtgcgcgacacgcaggccggtacccggcagacgcgtggcatgctcgccaactcgatcttcaagtcgaaccgcgagcgcaaggctttctaccagcgcaccggtctggacaagtccgtcagtgatgacgcgatgcgtgtgcaggtcgccgaagtgatggcacgctccgaacgcttcagtgcgcagtacggcatcgacgcggcgaagctgtccaccatcatgcagcgcttcgggctggaagctacgagcacgactctaatgtcgtccaagtcgccagttgcccgcatgcttgcgatcaccctgttggagaatcccgagggtgcagcaggccgacacagcaccgcagcgatggatcggcatggtcggtttgagtcgttcatgggcacccgcccgcgtcagtgggaagcggcctatcgcctgtggcgtgcggacgtgcgcggtatcggtgcgatcaaggacttcgccacgggctggaaggctcgcgcggacttcgagtacgcagtgaagctgtaccgcgagactcgcttcaacggcggggacatcccggatgcgcacgaggcagtgaaggcaatggcccgtgagttggaccgtggctacaaccgcatggcagcagagcagcgcgcggccggtacggtgggcgcacagcgtctgccggaggaggacgtggagggctacgagtcccgtacgtggctgggcggcagcatcgctgctgctggtccggtgcgacgcgagggtatccgtcaggcgatgcgcgatcagttcgaggtgatgggcgagctgtatggggacgacttcctcgataagttcgctaccaagtatctggaacgcatcgagcgcaaggctgcgggtgtcatcgaagcgccgggtcaggtcttctcggagtcgcaggcggacacgctgcgcgacactctgcgggcgatgtcgctcaacgaggaggagattcagaaggtcatgggcaagtacagccgtggcggtgcgaagcacaccaaggcgcgtatcgacctcgacgtgaccaagcagtacgaggacgctgacggtaagttccgtctgatggactatctcgacaaccgcgtgatggacaactaccgcaagtacgcgggacgtgttgctggtgacatcgctctggcgaagcacggcatcctcggcgacgcaggcatcaacgtggcgcgcgaagcaatgcgcctgaccggtgccaacgatgtggagctgaaggcgttcgagcaggtgatgtccgagttccttggtcgcccggtcggtaccggcgatccgactgttctggcgaatgcgcgtctgctgacctcggccatccagctgggcggcgcgggcatcaatcaggcagcggagtacagcaacggcctcgccgctgttggtgctgctggtgtggctgacgcaatccgtatcgctccccgcatgcgcagcgaaatcatgcgcatcctgaagggcgaggacagcggcaaccaaatcctcgacggcttcgagttcatcagcggtcgcggcttcggtctcgccggttacgacctacacatgttcaactcgctggacacgcaggcgtcgatgtatggtagcgagcgcgcaggcttcctgacctcgctggtgcagaaggcagcgcatgcgaaccgcatcctctcggggcagcgggccgtgcttgctgtgcagcagcgtggcttcgcggaagtgctgatcgccaagggcgtgaagttcctgcgtgatggtgctgaagctgacaccgccctgaaggacatgggcattgacgacaacctgctgaaccgcctgcgggctacgcaggatcaggtcgtgcgctggggcgcggatggtaagctggaagcagtagacccgcgcaacgtcgaggggctggcggatcggcaggcatggttggcgttctacaacgcgatcaaccgtggcacctcgcagattcttcaggacaccttcatcggcgagactggcaagtgggcgcacaacggctggctgaagctgctgttccagcaccgcacgttctcgctggtcgcgcagcagaagcagctgggccggtacgtgggcaactacggtgcatggcagacggcgggcctgatcgctgctgcgatggctgtggcggctccgctgcaagccctgcgggtgctgtcccgcgtggccctgatgaacgatcaggagcgcgacgaggccatcgaccagaacatcctgtcgcctctggcgctgggcaaggccacgctgaactacgtgtcggcgacgggtatgctcaacgatgtgctggacgtgggcactggcgtggcgggcggctggtacgagtacgccaccgatacgcagggtccgacgtggctgaagcagctggccggtgggcagttcggcaaccgcaaggaagtggtgggcgggcagttcgcgccgtcgctgggagtcatcaacgacttcgctcagggcattgctggcaagccggagaatctggccgacgtgattccgggcgggcgactgccgatggtgatcccgctgctgaagggcgcagccagccagtggaaggaggagtaagatcagggccaaggacggcccacccttttggtacacctatagcaaacaggaggcagcatggcagttccagacccgcagctgcgctacgcgacagacgtgttcgacgccgatggcgtgaccactgactggcagatcagctttaccggtggctacatcaacccgtcccacgtgtacgccatgagcggactgctggacgaggagactcagctgctgaccgaccggactccgcacaccgtggaagtcctgagcgaagacgatgacgctagtaccgtccgagtctcgcctgccgtcgccgctgggcgcaagctctacatctaccgcagcactccggtgcagcagatgctcgttgactacgttaacggtagcatcatcagcaagacaaaccttaacctcagcaacgaccagctcctgaagatcattcaggaaatgttcgactcactcaacatcgccacccttagcatcgaccagcaggtcggtgtgatcgtggacctgaacgagattatccagaacatctacaagcaggtcaccgagttgctggcagctggtggtatcgtgtccgtcgccccgcgcgtctggtccggtgcttggactggcgatcaggtgggtgacaccgacttcgacatggtgggcgcggacgtatccggcgcgggcttctacgacgtgtacgtcaacggcatcggcatgcagccggacgtggactatcaggtcacgctcgctgacggcaccgatcccagcttcatccgcttcgccacggttcctgccgagggcagcatctggttcgccgtgctgcgtggttacgccaagccctacaccgggcctgcgccgatcaccgctgcgagcctgcgggtgccgatcatcacggcagagggtccgacttactacgccgccaaggctaccgagtacggactcgtgcgctgcacgtacgccggaggttgcgccgtcaacatcaacctgatccccgaagtgggcgacggtgaaaccaagctcgcctcgggcagctacttcagcgtgcagcagaaggcaggccctgtggtcatcactggcgacgtgggcgtgacgctcgaagtcccggtcggctgcaccgccgcaactcgcggcaccaactccgtcatcactgcaacgtgcatcgacggcgacaccaacacgtggttgctctcgggcgacttggctaaggagtaagcatggctaatcacttcaggctgtacggccgaccgctcatggcggacgaggttgcagatggcctgtcggtgacgggcgtgctggaagggtacacggcgggcgaggcttacgagtctcgcctgtccatcaacaacccagtcggccgctgcaccgtggaggtcatcgaatcgacgctcccttcgggcgctgcggtacgggtggacaacatcaccaaggaagtcgtcgtcaagtgggcggctttcactgaagtcgtggacgaggaaaccctcgtgcccaacggcgacttcgaggcaggcgacgacggcacgtggttgccgggcggtggatcgaatggcgaaggctggtcgattggcactggctcagactacgacaccgacagcggcgtgtacagcgcgcgcttcgccaacatcaagacgggcggcagcgacctgctcaacccgctgatccctgccaaggtcaacgactacatccgatgcaccgccgaggtccagcagggcgcaagctccaagggcaaggccggtgctcgtgtgtcgatcatctaccgcaaggaggatgggaccgagctgcaacgcaactggggcaacatggtttcctccggcagcaacggtgcgtggcaccagtccgttgccgaaggcgctgcgcccaaggacacgaagtacgtgcaggttgtactgtcggcgttccgcagcaagcagaacaaaccgctgtgggtggacaccgttaagtggaaccacaagtacgtactgggtcagaacgacgacagctcctacttccttagcatcaaggtcacggacgggttgaaccgtgtggcctactggtccggtcgtatcgaggagcagggcatctacgttacgtccaagctctacagcttctaccagttcgatgccgcgatgctgaccagcagctttgctgggtacagcaacatcgacatgctccagcctttggatactgcgtcgctgggttcctccttcgtaagctgggaactccgaagctctaggcaggattatgccgccgacccggagagcacgttgtacgggagcgctttcgtttcgttcgacatccgatccatccgtaaggactacacgcctgacccggagacggcgaagctgtcgagttctttccattccttcaccctgaagcagcaccctgtagtcaaccagccgctcgacgcgactgcacgactccggtctggcttcgtatcatggagcttcgcatgatccacaatcacctcggcattgctggcgtgttcaccatcagcaagggtaagtccctcgatactctcgaagttgtagccgactggcagagcaaccttatcacggacggtggtatggacgcactgggtgataccggcagcggctatcctcgcagcatgtacgacctcattgcttacttggcagtcggtagtggcagcgccaccccggcattcaccgataccgctcttggtgcacaggtggcgcaggttggtcgtacgtcctcggacagcggtgggactaccactgccccgtactacgcctactcccgctgccagtaccagttcccggctggtaccgctactggcgttctgtcggagcttggtgccaaagcatacaacaacaataccggcgcgtacatcctgaccacccgtgcgcttatcaaggactccgcaggtaacccgaccaccatcacggtgctgtcggatgaaatcctcgtggttacttacgagctgcgcatgtacgcagataccacgccggttgtcactactgagacgatcaagggtgttagcaccactgttacctgtaagcctattgcaatgggccgcagcggcggtatgaacggtcagtcggcagtcgcttggtcggactacgtgtgggggtgctactacttctacggcggtactggcgacggcaccggagctatcaccgaccagtatccgccggggacgattgccagcttctctgacttgcagcttcagcaggtagcctatgttccgggtacttactaccgtgactgcgtttgccggatgtcgatcaacaacgtgcccggtggtccgatcacggctgcaatgggactctccgcgtgcgtgaccttccaagtcggcttcaatccgggtatcaccaagaccggatcggagacggcgaacttgcgcatgcgggtttcttggagccggtacacgccatgatccccactgtctcccaaagcatccaacgcggtgactgggtggagcagcagaatcggcgcacccgcccgctcattgacttcgagcagggcgggctgactctcaacgcagcagtggacgacctccaagctgcgctgtggactgccgagagtgacggcagcagcgtcgtcgtttaccgcgacggcgttgccccggtcaccgtgctgaccgactccgggatcacgcagatcgcactggccttcgaccagaccatgcgcccgcacgtggcgtacatggcgggcggtgtgtgcaagttctactggtacgacacggtggctgcttcgatgcagaccatggtgatccccggtgctaccactccgcgcctgtgcatggacgagaagcgggctgtcttcgccacgcagagcgacgtgctcctgtcgtacaagaacggcagcaacctgtgcgtacgcgcgcagcgtgagcgcttcgcaaccgaacatgtgatcgcctcgggaatccccggcgacctgattgcggtgggcatgaacaacgtcaaccgcctgcaatggaagctcgtcggcaatcccgacgactggccctaacctacaggagaacagcatgaccccgccgagtgtggtcaatgaggtcgtccgaacctcgccgcttacgctcggcgcggtctacctcaacttcatcagcacgtacggtgctgccatcgtaactacgctcgccattctgtacgccgtcgctcagttctactggcgggcacgcgagcaccgaaagatcatgggaggcaaggatgtcgaatccggcaagtgagggcgcactcggtgcgctgcacgaactggtcgcgcgtgcgctgatgcagcgcatccaagatggcgagctgtgcaccgcagccgacatcaatgcggcgatcaagttcctgaaggacaacaacatcacggcgacgcgcgaggccaacaaggcactcggcgagctggaagacgagctgggcaagcactcgctgcctccggctgacgacgacgagttgcagcgtgcactcgacaacatcgttcactttccggggagcgtagccaacaatgcgtgaatcagctgaagcggccgacgtgcgccgcaagaagttggagctgttgcagaaccactaccggcacttcgccaccttcatgcgcgacattatgaaggtgctggggttcgagccgacgtggatgcagtacgacatcgccaactacatgcagtatggcccgcacctcgcaatggtgcaggcgcagcgaggcgaggcgaagtccaccatcgctgccatctacgccgtcttctgcctgatccacgatcccactcaccgtgtgctgatcgtatcggcaggcggcacgcaggcatccgagattgctacgctgattcagcgcatcatcctcacggtgccgacgttggagtgcatccgcccggacaagaacgcgggcgaccgtacctccgtggatgcgttcgacgtgcaccactcgctgaagggaatcgacaagtccccgagcgtggcgtgcatcggcgtcaccggcaacctgccgggtaagcgtgcggacctgctgatcgccgacgacgtggagtccaacaagaacagccgcactgccgcgaaccgtgagctgctgctgaccatcacgttggagttctcggccatctgcaccggcaagcccggtactccgggtcgcatcctgtacctcggcacgccgcagaccggcgactccatctacaacaccctgcccggacgtggctacgacgttcgcatctggcccggtcgctacccgaccccggcacagcgcgagcactacggcccgcatctggcaccgtctatcgtgcagcgcctagaagccgacccgatgttggcgttcggtggtggcccgatgggcgacgagggccagtgcaccgacgagctgttggccggtgagcagaagcaccagtccgagctgcgtcagcgtggaccgtccagctatcagctgaactacatgctcaacacgcggctgatggatgcgctgcgcttcccgctgaagaccgagaacctgatcgtgatccccggtggtggcgaccgcttcccgctgacgatcacccgtggcctgagcaacgctcaccagcgcagcttccagtccagtgggtacggcttcgtgatgatgatgccgcacgacatgagcaccgagactgcccccgtgcagggcgtgcacatgcagatcgacccggccggtggtggtgccaacggagacgagacggccttcgccgtgaccgccttcctcaactccaccgtgtacgtgttggccgtgggagctgtgcccggtggctacgacggtgatggcttgctagaactgcgccgcattgcggtgaagtacaagccgaacgtcatcagcatcgaaaagaacatgggctacggcgcgttcgccaaggtgttcctgcctgtcctgcgagaagatcgcggcacggagaagggatacaagggcgacatccgcgaggagttcgtgaccggcaacaaggaagcccgtatcatcggcactctcgaacctgtcatggctcgcggctcgctggtcatgctggaatccgtggttgaaatggatcacgagtacacccagcgctacgccaccagcggcaagcgtcaggtctacagcctgttccaccagatggcgaagatcacgcagcagaagggcagcatcgcacacgatgaccggctcgatgcactggaaggtagcgtgcgtcactgggttgcgcagcttgcactggaccagaacaaggccatcgccaagcagcagcagcgagagttccaagactggatcaacgatccgaccggcatgaaggcagcgacccgcaagagtccgctgcaacgtggccgtccatccctactcgaccgttaccggaggtaaccaatgcagaagtccgacttcaccagcaactacacgggtctgttcggccgtggcaactacctgcaccgcgaactgctcgccctcatggagcacgcagagcagcatcccgcaaccgcagcgcagctgctcgcgcagttccagaaggacgccaccctcgtgctggacgccctgatcgctgcgggcgcacgcaccgcgtcctcgggtccgaactccggcccgcacactccggtcgatctggacccggatgacgacccactgaccccgtaaggagcaaccatgaaccagcagcagaaccaagataccagcaacaaggggctgttcggcctgatcggcggcatcttcatcggcatttcggcaacgctgctgtcattcacccaaggccacgaaggggtacgctacgctgcgtacctcgacaccggccgggtgccgaccatctgctacggccacaccaagggcgtagcgatgggcatgacggcaacgaaggcacagtgcgacaagtggctgatcgaagacctacagatcgcccagcagggcgtgcgcaagcacctgaaggcccccgttaaccgcaaccagatcgacgcctacacagacttcgtgttcaacgtaggtgagaaggcgttcgccgacagcaccatgctgcgcaaagcgaacgcaggggatcgtgaaggtagctgcaaggagttcctgcgctgggtctacgtcggtaagctcgactgccgactgtccagcagccgttgctccggcatccccaagcgccgcgacgcagagtttgctctgtgcttgcgccccaacaacgaggtgatccaaccgtggaaaccccaagtgaagtgatcgcgcggctcggcggcaagctggttggcttgctgctggtcgtgaccatgttcgtgtgcttcggtctgtacgtctacggcctgcaacgcaaggtggagaagctggaaactgcccaagtcggcacgaccgctaccgccaaggcggcgcagacgcaggctaccgggtacgcgacctacatcaaagagaaggaggacgtgcgtgttcgcactgaagaagttcttgacgctgccccggagtaccgggatggcactgttcctgctgatgtcgctgacctcctgcgcgaacctgccggtccctgacgactccctgcttgcagactgccacatcacctacctcggtggggagaagggcaccacctcctcgcaggacaaggtggtcaagctcgcgcaggaccgccgcatggacaccgttctgtgcaacaaggacaaggctgcgctgcgtgcgtggaaggccgaggtgtgcggtaccggtaagcgccggtgtacgggtgacaaatgaccaccatcgcatgggacggcaagcacctgtgggccgatagtcaggccacgcagggcgaccacaagcacaccgtgcgtaagatcatgcccgtatcgacacccaccggccctgtgctgctgggtgtcaccggggatttcacagtgcttcgcccggttctcgctgcgcttaaagcgggcgaaggctacgaggagcacgttggcaagtccgcgacggtgcttgtggttaaggacggcgtactcacggtcactactggtaagcagcagtgggtcgaggaggctccgtacttcgatggcagtggcaaggcgctagctctaggggcctatcatgcgagcaagtctgtggctaaggccatggctgctgcgatagctcacgatgtctacagctccgggcctatcgtcaagctaaaggcaccagttcgcgaggcttaggagtaaggccacgtgggtagccggaccaaaatttgcttcggaaatgcgcgggggtcactccaatagaagctcccgcgcgtgcccccgtacgccctcgcgttacgcgcctgcgggtgtgcgtgggtgcgtgcccgcgtgtgcgcctgtgtgcgcgtctgtgcgcccgcgtcaaggttccgcgtgggtgtacccgtgtgcctgcctgcgtgggcctgagcgtgcgtgtgcgtggccgtgcgtgggtgcctgcgggtgggcgtgcgggtgggcgtgcgcctgctgcctgtatggctggaccgc

SEQ ID NO: 6 - DNA, 44482 bp, unidentified
  source 1..44482: mol_type = genomic DNA
tcccggccacccgtcaagcacaatctgcgagagatttattaaccattcagccaaggcggcacggtccagccatacaggcagcgcaagcgtacacgcgccgtaggcgcaggcaggcgcacccgcccacgcaggcacacgcacggccgcacaggcgcgcccacacgccacgcgcaggcaggcacaggcacacacccacgcggaaccttgacgcgggcgcacagccgcgcacacaggcgcacacgcgagcacgcaggcgggcgcacccgcaggcgcgtaacgcacgggcgtatgggggcacgcgcgggagcttctattggagtgacccccgcgcatttgggaagcaaattttggtccggctacccgcgtggccttatgactaagccttgcgaactggtgcctttagcttgatgataggcccggagctgtacacatcgtgagctatcgccgcagccattgccttagccacagacttgctcgcatggtacgcccctagagctagcgccttgccgctgccatcgaagtacggagcctcctcgacccactgctgcttaccagtagtgaccgtgagtacgccgtccttaatcacaagcaccgtcgcggacttgccaacgtgctcctcgtagccttcgcccgctttaagcgcagcgagaaccgggcgaagcactgtgaagtccccggtgacacccagcagcacagggccggtgggtgtcgatacgggcatgatcttgcggacggtgtgcttgtggtcgccctgtgtggcctgactatcggcccacaggtgcttgccgtcccatgcgatggtggtcacttgtcccccgtacaccggcgcttgccggtaccgcacacttcttccttccacgcacgcagcgcggccttgtccttgttgcacagaacggtgtccatgcggcggtcttgtgcgagcttgaccaccttgtcctgactggaagtcgtcccgcgctcaccaccgaggtaggtgatgtggcagtccttcagcagatcatcgctgggaaccggcaggttcgcgcaggaggtcagcgacatcagcaggaacagtgccgtcacgatactcgggaacggcgtcgagagcttcttcagtgcgaacacgcacgtcctccttctctttgatgtaggttgcgtacccggtagcctgagtctgcgcagccttggcggtagcggtcgtgccgacttgggcagtttccagcttctccaccttgcgttgcagaccgtagacgtacagaccgaagcacacgaacatggtcacgaccagcagcaggccgatagccttgccgccgagccgcgcgatcacttcacttggggtttccacggttggatcacctcgttgttggggcgcaggcagagggcaaactctgcatcgcggcgcttgggaatgccggagcagcggctgctggacagtcggcagtcgagcttgccaacgtagacccagcgcaggaactccttgcagctaccttcacgatcccctgcgttcgccttgcgcagcatggtgctgtctgcgaacgccttctcgcctacgttgaacacgaagtccgtgtaagcgtcgatctggttgcggttaacgggaaccttcaggtgcttgcgcacgccctgctgggcgatctgtaggtcttcgatcagccacttgtcgcactgtgccttcgttgccgtcatgcccatcgctacgcccttggtgtggccgtagcagatggtcggcacccggccggtgtcgaggtacgcagcgtagcgtaccccttcgtggccttgggtgaatgacagcagcgttgccgaaatgccgatgaagatgccgccgatcaggccgaacagccccttgttgctggtatcttggttctgctgctggttcatggttgctccttacggggtcagcgggtcatcatccgggtccagatcgaccggagtgtgcgggccggagttcggacccgaggactgcgtgcgcgcaccggcagcgatcagggcgtcgagcacgagggtcgcgtccttctggaactgagcgagcagctgcgctgcggttgcgggatgctgctccgcatgctccacgagggcaagcagttcgcggtgcaggtagttgccacggccgaacaggcccgtgtagttgctggtgaagtcggacttctgcattggttacctccggtaacggtcgagtagggatggacggccacgttgcagcggactctttcgggtcgctgccttcatgccggtcggatcgttgatccagtcttggaactctcgctgctgctgcttggcgatggccttgttctggtccagtgcaagctgcgcaacccagtgacgcacgctaccttccagcgcatcgaggcggtcatcgtgtgcgatgctgcccttctgctgcgtgatcttcgccatctggtggaacaggctgtagacctgacgcttcccgctggatgcgtagcgctgggtgtactcgtgatccatttcaaccacggattccagcatgaccagcgagccacgagccatgacaggttcgagcgtgccgatgatgcgggcttccttgttgccggtcacgaactcctcgcggatgtcacccttgtatcccttctcggtaccgcgatcttctcgcagcacaggcaggaacaccttggcgaacgcgccgtagcccatgttcttttcgatgctgatgacgtttggcttgtacttcaccgcgatgcggcggagttcgagcaggccgtcaccgtcgtagccaccgggcacagcgcccacggccaacacgtacacggtggagttgaggaaggcggtcacggcgaacgccgtctcgtctccgtttgcaccgccaccggccgggtcgatctgcatgtgcacaccctgcaccggggcagtctcggtgctcatgtcgtgcggcatcatcatcacgaagccgtagccgctggactggaagctgcgctggtgcgcgttgctcaggccacgagtgatcgtcagcgggaagcggtcgccgccacccggaatcacgatcaggttctccgtcttcagcgggaagcggagcgcgtccatcagccgcgtgttgagcatgtagttcagctggtagctggacggtccacgctgacgcagttcggactggtgcttctgctcaccggccaacagctcgtcggtgcactgcccctcgtcgcccatcgggccaccaccgaacgccaacatcgggtcggcttcgagacgctgcacgatggacggtgccagatgcgggccgtagtgctcgcgctgtgccggggtcggatagcgaccgggccagatgcgaacgtcgtagccacgtccgggcagggtgttgtagatggagtcgccggtctgcggcgtgccgaggtacaggatgcgccccggagtgccgggcttgccggtgcagatcgcggagaactccaacgtgatggtcagcagcagctcgcggttcgcggcagtgcggctgttcttgttggactccacgtcgtcggcgatcaggaggtcggctcgcttacccggcaggttgccggtgacgccgatacacgccacgctcggggacttgtcgatgcccttcagcgagtggtgcacgtcgaaggcgtccacactggtgcggtcgcccgcgttcttgtccgggcggatgcactccaacgtcggcaccgtgaggatgatgcgctgaattagcgtagcaatctcggatgcctgcgtgccgcctgccgatacgatcagcacacggtgggtgggatcgtggatcaagcagaagacggcgtagatcgcggcgatggtggacttcgcctcgcctcgctgcgcctgcaccattgcgaggtgcgggccgtactgcatgtagttggcgatgtcgtactgcatccacgtcggctcgaaccccagcaccttcataatgtcgcgcatgaaggtggcgaagtggcggtagtggttctgcaacagctccaacttgcggcgacggatgtctgccgcttcggctgattcacgcattggctacgctccccggaaagttcacgatgttgtcgagcgctgcttgcagctcggtgtcgtcggcctgcggcagcgagtgcttgccgagttcgtcttccagttcgccgagcgccttgttggcctcgcgcgtagccgtgatgttgttgtccttcaggaacttgatcgcggcattgatgtcggctgcggtacacagctcgccgttggcgaggcgttccttcagtaccgtggcgacaagttcgtggagtgcgccaagcgcgccctcacttgcggggttcgacatccttccctcccatgatcttgcggtgctcgcgcgcgcgccagtagaactgggcgactgcgtacagaatggcgagcgtagttacgatggcagcaccatacgtgctgatgaagttgaggtagaccgcgccgagcgtaagcggcgaggttcggacgacctcattgaccacactcggcggggtcatgctgttctcctgtaggttagggccagtcgtcgggattgccgacgagcttccattgcaggcggttgacgttgttcataccaaccgcgatcaggtcaccggggattccggtggcgatcacgtgttcggttgcgaagcgctcgcgctgtgctcggacgcacaggttgctcccgttcttgtaggacagtagcacgtcgctctgcgtggcgaagatcgcccgcttctcgtccatgcacagacgtggcgtagtagcaccggggatcaccatggtctgcatggaagcagccaccgtgtcgtaccagtagaacttgcacacaccacctgccatgtacgcgatgtgtgggcgcatggtctggtcgaatgccagtgcgatctgcgtgatgcccgagtctgtcagcacggtgacaggagcaacgccgtcgcggtaaacgacaacgctgctgccatcactctcggcggtccacaacgcggcctgaaggtcgtccacggatgcgttgagagccagcccgccctgctcgaagtcgatgagcgggcgggtgcgccgattctgctgctctacccagtcaccacgttggatgctttgggagacagtggggatcatggcgtgtaccggctccaagaaactcgcatgcgcaggttcgccgtctccgagccggtcttggtgatgcccggactgaagccaacttggaacgaggcgcaagccgagaggcccatagcagccgtgatcggaccaccgggtacgttgttgatcgacatgcgacacaccacgtcccgatagtggctaccggcaacgtaggccacatactgaatatgcaagtccgagtagctgacgttggttcccggaggatactggtctgtgatcgcgccggtcccgtctccggttccgccgtagaagtagtagcagccccaaacgtagtccgaccacgcaatggccgattgcccactgagcgaaccactccggccgagggcgatgggcttgcaagtcacagtggtgctgacgcccttgatcgtctcagtcgtcaccaccggagtcgtgtcgatgtagagacgcagctcgtaggtcaccacgaggatttcatccgacagcaccgtgatggtggtcgggttacctgcggagtccttgataagcgcgcgcgtggtgaggatgtaggtaccgttgctgctgttgtacgccttggcacccagttcggaaaggacgccggtagcggtgcctgccgggaactggtactggcagcgggagtaggcgtagtacggagccgtggtggtgccgccgttgtccgaagtcgtacggccaacctgcgcaacctgcgcgccgagagcagtgtcggtgaacgcaggggttgcgctaccgctgcccactgccaagtaggcaatgaggtcgtacatgctgcggggatacccgctgccggagtcacccagtgcgtccatgccaccgtcggtgataaggttgctctgccagtcggcgacaacttccagagtgtcgagggacttacccttgctgatagtgaacacaccggcgatgccgaggtgattgtggatcatgagaagctccatgatacgaagccggaccggagtcgagcagtcgcgtcgagcggctgattgacaacaaggtgctgcttcatggtgaaggaatggaaggaactcgacagtcgcgccatctccgggtcgggtgtgtagtccttgcgaatggatcggatgtcgaacgaaacgaaagagctaccgtaggaaaggctctcctcagcggcgtaatcctgacgcgagctgcgcagttcccagcttacgaaggaggaacccagcgacgcagtatccaaaggaggcagcatgtcgatgttgctgtacccagcaaagctgctggtcagcatcgcggcatcgaactggtagaagctgtagagcttcgacgtaacgtagatgccctgctcctcgatacgaccggaccagtaggccacacggttcaacccatccgtgaccttgatgctcaggaagtaggagctgtcgtcgttctgacccagcacgtacttgtggttccacttaacggtgtccacccacagcggcttgttctgcttgctgcggaacgccgacagcacaacctgcacgtacttcgtgtccttgggcgcggcaccttcggcaacagactggtgccacgcaccgttgctgccggaggaaaccatgttgccccagttacgttgtagctcggtcccatcttccttgcggtagatgatcgacacgcgagcaccagccttgcccttggagcttgcgccctgctggacttcggcggtgcatcggatgtagtcgttgaccttggcagggatcagagggttgagtaagtcgctaccgcccgtcttgatgttggcgaagcgcgcgctgtatacgccgctgtccgtgtcgtagtccgagccggtgccaatcgaccagccttcgccgttcgatccgccgcccggcacccacgtgccgtcgtcgcctgcctcgaagtcgccgttgggtacgagggtttcctcatccacgacttcagtgaaagccgcccactttacgacgacttccttggtgatgttgtccacccgtaccgcagcgcccgaagggagcgtcgattcgatgacctccacggtgcagcggccgactgggttgttgatggacaggcgagactcgtaagcctcgcccgccgtgtacccttccagcacgcccgtcaccgacaggccatctgcaacctcgtccgccatcagcggtcggccgtacagcctgaagtgattagccatgcttactccttagccaagtcgcccgagagcaaccacgtgttggtgtcgccgtcgatgcacgttgcagtgacgacggagttggtgccgcgagtcgcggcggtgcagccgaccgggacttcgatggtcacgcctgcgtcgccagtgatgaccactgggcctgccttctgctggacgctgaagtagctgcccgaggcgagcttcgtctcaccgtcgcccacttcggggatcaggttgatgttgacggcgcagcctccggcatacgtgcagcgcacgaggccgtactcggtatccttggcggcgtagtaggtcggaccctctgccgggatgatcggcactcgcaggctcgcagcggtgatcggcgcaggcccggtgtaaggcttggcgtaaccacgcagcacggcgaaccagatgctgccctcggcgggaaccgtggcgaagcggatgaagctgggatcggtatcgtcggccagagtgacctgatagtccacgtccggctgcatgccgataccgttgacgtacacgtcgtagaagccagcgccggacacgtccgcgcccaccatgtcgaagtcggtgtcgtccacctgatcgccggtccatgcaccggaccagacgcgcggggcgacggacacgataccaccagcggccagcaactcggtgacctgcttgtagatgttctggataatctcgttcaggtccacgatcacaccgacctgctggtcaatgctaagggtggcgatgttgagcgagtcgaacatttcctgaatgatcttcaggagctggtcgttgctgaggttaaggttggtcttgctgatgatgctaccgttaacgtagtcaacgagcatctgctgcaccggagtgctgcggtagatgtagagcttgcgcccagcggcgactgcaggcgagacacggacggtgctagcgtcatcgtcctcgctcaggacttccacggtgtgcggagtccggtcggtcagcagctgagtctcctcgtccagcagtccgctcatggcgtacacgtgggacgggttgatgtagccaccggtaaagctgatctgccagtcagtggtcacgccatcggcgtcgaacacgtctgtcgcgtagcgcagctgcgggtctggaactgccatgctgcctcctgtttgctataggtgtaccaaaaagggtgggccatccttggccctgattctcactcctccttccactggctggccgcgcccttcagcagcgggatcaccatgggcagtcgcccgcccggaatcacgtcggccagattctccggcttgccagcgatgccctgagcgaagtcgttgatgacgcccagcgcgggcgcgaactgcccgcccaccacttccttgcggttgccgaactgcccaccggccagctgcttcagccacgtcggaccctgcgtgtcggtggcgtactcgtaccagccaccagccacaccggtgcccacgtccagcacatcgttgagcatgcccgtcgccgacacgtagttcagcgtggccttgcccagcgccagaggcgacaggatgttctggtcgatggcttcgtcgcgctcctgatcgttcatcaggaccacgcgggacagcacgcgcagggcttgcagcggcgcagccacggccatcgccgcagcgatcaggcccgcagtctgccacgcaccgtagttgcccacgtagcggcccagctgcttctgctgcgcgaccagcgagaacgtgcggtgctggaacagcagcttcaaccaaccgttgtgcgcccacttgccagtctcgccgatgaaggtgtcctgaagaatctgcgaggtgccacggttgatcgcgttgtagaacgccaaccatgcctgccgatccgccagtccctcgacgttgcgcgggtccaccgcttccagcttaccgtcagcgccccagcgcacgacccgatcctgcgtcgcccgcaggcggttcagcaggttgtcgtcaatgcccatgtccttcagggcggtgtcagcctcggcaccatcgcgcaggaacttcacgcccttggcgatcagcacttccgcgaagccgcgctgctgcacggcgagcacagcccgctgccccgaaaggatgcggttcgcatgcgctgccttctgcaccagcgaggtcaggaagcccgcgcgctcgctgccgtacatcgacgcctgcgtgtccaacgagttgaacatgtgcaggtcgtaaccggcgaggccgaagccgcgaccgctgatgaactcgaagccgtcgaggatttggttgccgctgtcctcgcccttcaggatgcgcatgatttcgctgcgcatgcgaggagcgatgcgaatcgcgtcagccacaccagcagcaccaacagcggcgaggccgttgctgtactctgctgcctgattgatgcccgcaccgcccagctggatagccgaagtcagcaggcgtgcgttcgccagaacagtcggatcaccggtgcccaccgggcgaccgaggaactcggacatcacctgctcgaacgccttcagctccacgtcgttggcaccggtcaggcgcattgcttcgcgcgccacgttgatgcctgcgtcaccgaggataccgtgcttcgccagagcgatgtcaccagcaacccggcccgcgtacttgcggtagttgtccatcactcggttgtcgaggtagtccatcagacggaacttaccgtcagcatcttcgtactgcttggtcacgtcgaggtcgatacgcgccttggtgtgcttcgcaccgccacggctgtacttgcccatcaccttctgaatctcctcctcgttgagcgacatcgcccgcagagtgtcgcgcagcgtgtccgcctgcgactccgagaagacctgacccggtgcttcgatgatacccgcagccttgcgctcgatgcgttccagatacttggtagcgaacttgtcgaggaagtcatccccgtacagctcacccatcacctcgaactgatcgcgcattgcctgacggatgccctcacggcgaaccggaccagcagcagcgatgctaccacccagccacgtacgggactcgtagccctccacgtcttcctccggcagacgctgtgcgcccaccgtaccggccgcgcgctgctctgctgccatgcggttgtagccacggtccagctcacgggccattgccttcactgcctcgtgcgcatccgggatgtccccgccgttgaagcgagtctcgcggtacagcttcactgcgtactcgaagtccgcacgtgccttccagcccgtggcgaagtccttgatcgcaccgatgccgcgcacgtccgcacgccacaagcggtaggccgcttcccactgacgcgggcgcgtacccatgaacgactcgaaccgaccatgccgatccatcgccgctgtgctgtgtcggcctgctgcaccctccgggttctccaacagggtgatcgcaagcatgcgagcgacaggcgacttggacgacatcagggtcgtgctcgtagcttccagcccgaagcgctgcatgatggtggacagcttcgcagcgtcgatgccgtactgcgcactgaagcgctccgagcgtgccatcacctctgcgacctgcactcgcatcgcgtcgtcgctgacggacttgtccagaccggtgcgctggtagaacgccttgcgctcgcggttcgacttgaagatcgagttggcgagcatgccacgggtctgccgggacgcggcctgagtgtcgcgcacttcagcaccgaggttgtcaccgaccacagacatcagacgttcgagcgcggactcctgattcttcaggcccatcactcgcgcgatcttgtccttcagccactcccacgcattcggacgggtgttgcccggcgcaggcatctgacgcagcaccgcctgcacggcgcggttcgtcaggccgtaggaaatcagctcgtcggtgttggcgaggaagcctgcctgcggctggttgatgcgcgtctccatcgcagcggtggtcagcgtggagtccacactgccgatgctgttgttgatgtgggtcagcagttcttccatttcctgaccgaacaccgagttgctgcgcagctcacgcagggtggcagcgtgcagcatttcgtgcaccaccacttccggcgtgtagttccgcatcgccatcgcgtccagcccggcgttgtagccaccggccactcgcatacccggacccatgttggcaccggcaaaccacttgtcgagttcagactccggcacgatcttcaccgtgctcagacgaccgccgcgcttcagcgcattggcgatagcacgcacgtcctcggggatcgaggcgttggattccagatacttcagcacgccatcgacgttgccgccacggatgcctgcggccttccacgcacgttccagcagcggatcatgctgatcgactcgaccacccacgctgtcgttgtaacgaccggtcgaggcgtccacgttgtccacgtcacgcgccagtgcaccagtggtgcctgcggtggtggtcgtctcctgcacgtcgggacgcgcgaagatgcggaagtcgtccggcacatcagccataccagcgcgcagccaatcgactgcttcctgcttggcaagctggtggatgcggttgttgaccagcaccgggttggcgttgtcgccaagctcggccacagctcgcgccttcaggtcagccgaccacgcttcgccgtaagcggcagcgttgcctgcggacaggtcgatggtagccttgtcccgaatctgcgcagccgagcgcacgcccggaatgtgcatcgcggtaccgatggtggtggcgaacgctgcgtcggtcataaagtccgcgaagttgcggcgctcacccataccaaccagcgcggcgtccgtaatgacggaaccgaccgcgttctccgcagcagcggacgcgagggacgcaccgacgcggccttcggcaaccagagccgccgagcctacgcccagcaccttggcacccgcagcagtcacgccgccgatggcccagttgcccggatcggtgaagcctgccactaggtcgtagccgaagctcgaccagccggtctgctgatccttgatgcgcattgagctgcgacgcatgtactgtcggtcgctcacgtacttcagctcgttcggcgagtacgcagcatcgcggatgtcttccagttcgtcggcagtcatccacgacttctcccactccttcgggtcgtacttccaaccttccggcacgttctcgtcctcacgcgcgagctggttgctgatcgcagcaccgatgccgctatcgaaagcagcgccccacttgtcgaggaaggtaagcgagttgcgcagttcctcgtccgcacggtcctgtgcgagagcctgctcggtctgatccagcagcgccttgcgtgcgccggtgttcagaacgtccacttcctgacgaacccaccacggcacaacctgatccgatgcacggacagcctgcgccttacccacagcctccgctgcggtgccgccttcctgagccacctgccccatcgacagttcggcgatgcccgcgcgaatcttgccgatgtgttccttcgctgccgacgccagagcgttgcggccttcgatgggcgcgccagtccacgcatccgggatggatgcaccggaccacgtgcggtcgcgcatgttcgggtttccctgccatgcggcgttgaggtctgcctgtgtggtagtcaggctgcgcggctgcgatgacactgcgggagcggatgcgccgcccagcacactcggtgcgtaagccgcgttctcttgcccccagttcttctggttggtaccaccttggtagatgcgcagcgccttcgtcacgtcacccttggcaagctgcatgttctcgcgcatgatgtcggcatacagctcgatgctgtcttggaagttgcgcatgtcgtacttgcgaccgttgcgcgcttcccacgttgcctgcgtggtgggcatgacttggaagtcgccctgtgctcctgccttgctgcggatcacaccgtcagcgtccttggcggcgcgcccgttgccggactctactcgccactgaccgcgcacgatggactccggcactcccgcataagcggcagccttggcaatctgctggtcttgggtcagccccgaaagatcgagtgccattgtctatctccttacagtttgggttggatggaaatgctctgctgaatcgtaccgtcgttcatacgaacgtagccctgcggtaccggggcctgcaactgacgctgctgcttggtgtgcttctcgtactcggccttgatgtcgcgcccatacaccggcacaaccttccagcccttctcgccaacagcgttgacgtacagcaccggctcgccgttctcgctatccttcatgcggaacacgtcagccttcaggccagctcccggctcgatgttgacccggcgtagcgctgcgtcgatggccttctcgatagcgggtccggtttccttcgtgtccatgaagcccagccatgcaccgacgcctccggtcactcgaccttcatcatcgcgcccgttctcccacgcgtacttgcctgcgtcttccagaccgtaggccagcttggcgtgagtagccgcagcctgcaagccttccgcagacgtgtccagcagaccaccgctgtcggtgaccgagcgtacgatggcgcgagcatacgcagcgcggccagagtcgcccagcttgttgccgaacatgccgaggtacttggggttgagcttggcgatagcttccgtaacacgagcctgagtagcctcggattccttacggctggtcgcgtcgaactgcgtagggtcttcggtggtgatttctccacgggccacctcgtaggcaagctcgaagttcacgccaccattctccagagcttgcagcttgttgaagaacgtgttgacgctatccccgaagtacagcgcagcagtagtcgcgccagtcagtcggccctgtacgggctgaccgttcgtgtcgatgcgtgcggcggtggtctgcttcagctccttccactgctggtacagtgcggccgctgccgtgttaggctgatcgcggagcacagcgcgtgccgtggtctggaactggtcggccacccccttcagcacagcgcctcgaccggtgttggcgttccacaccagctgcgacatggcgaccttggggttcgatgccatcgtggcgttccatgcctgcaccgtgtttgcttcgatcagctccttgtccactccggggatgttgatcgtctgcgcgtacgtgccgcgcttgaacgcttcgatgccaccacggatgtcctcctcctgcgcggccagcttctgctgatcggtcagcgcggccttggccgcagcgttgcgctggttgatgacggcttcctgtgcgcggatgtgtgcgcctgcggactgcgccatgatcgaagccagctgtgtgccggagtacagcggtgcgtcgcttcccgtctcggcggcgtaggtcgagttcatttcctcgatcatcgcctgcgacggcttggcaccaatgccctccgatgcgtacatggagacgagcgccatcttctcggcctgctccgggttggcgtcgagccagtcggaacggtaccggtcctgcgcttgcttcacgtactgctggattccaagctgcccatcagggtcaatggcgctcagcacgcccttgctgttgaggaacttcagcgtgtggaactcgccacgatccgcagcgccacggtagaacgccgtgatcgcggacttgtaggactcgtccgtctggtagcgcgaaggcgacagcccatccagcaaggacagctgcgcctgcgtcagcgcctcggtagccttctcgtccattggccggttggtgccgagcatcgccgtgcgcttcgccagttcgttgaagccggtggacgccgacgagttcgcagcgtactgtgctttcaccagctcctgctgctgccacgccgtacgctccttggtgtgcaggtccatgagagaaccagcgcgatccatgaaggtcttctgcaacaccgtgtccgcgaaaccgttgccggtcatccgggcagtggcgaggtcgttgaactccttcgccatcgcctcgggaggaagctgccgcaactccggcatgcggcgcagcaagtcgctctccatttcattgacctgcgagagcgtgttatacatgctcgcgccaatctcgtagttggtgtcgccgaagattttcttgtaccacggttcggtcgcagcaatctcgtccatggtcttaccagcgcgggcggctacgaagccatcccacatctgctgctgcttcagcttggcggtgttcggcgctgccagctcctgcaagaactctggcaggttgctgtccggcatcgtcataccaccagtgcttgcgaaccagtcgttgccggattgaaccgggccgaccggattcacaccagcgccttgaatgctggtgttgcccgacagtgcgggggtggcgttgatgccaccctgcaatgcggactgcgtgttgaaggtaaccgtgccgatgtcagccattaccatgcacctcctgagttgcccccgctgccgctatcgaaccagccgaggccggacgtagtggtggagaagttgtcgtagttgttgccgaagttgccagtgaccttcgccccagtcacggcctgcttgccggtgccgtcgttgtacccgaaggtagtggacgcccacgacttgccgccgcgatcattggactgctgccatgcctgcatgccgttctgcgctgcgttgctgaaggactgagaggcaccagtgaagttgccgttgtccgcctgccacgtgccgaccgcgaagtctgccacggcctcgcccgccatcggcccaccgaagtaggtagcaacggccacgccgatcagcttgcccaagcgacgcttcatcgcctgcggctcgatgtgctgcgagtagtcgaactgcccgaacgaacggctcatgtccatcccgttccacgcacgcgacatgacctgcgcagtctgcgaggcaccacgcgaggcgaggagagcaacagcgttggcctgcgtctcctgatccatttccgcctgcaaccgcaccatcgaatccatcaggtctgcggacgagccgccgacaccgacagcaccggcctgcgcctgaagtgcaccccgcgcgttcgccagttggagctgggagttaagcccagccccttggcgcgcacgcagctcctccgacagcgcctccatgttggagttgtactccttcgcggctgcgtccagttgggcgttgttcttcagggaccgcatgaaatcagcgaagccggtcttggcgacctcgctgcggttctgattgtcggtctgcgcaacggctgcacggtagttcgcacgggcaactcgggtggtgttgttcgcttgcaggatcgtattaaccgaacccattagctaaccctccgtacattgttgaaagtctgacccgtccagctcaggccggtcacccggagcgggagccaatccttgctgcgaatctcgtaggtgcactcgcgcacttcgcgtccaacgctgatgttgagctgcccccggtacaccggttgccgcgcgatcaggttgtcggagtcgccgaggatgcggccctcgaagtccgtggtggtcacgttgctgttgcgtgtggtcaccgcagcgagcatgcccgcagtatcctctacgtccaccgtcaccttgttgagtgacatgcgtccgtcgagtacggcctgaccattctgatcccgagggaacgggttggtcgggatcaccacagcctcggacaccacaccgtattccagcgcaccagcgtcgaggtcatcgaactgggtaaggaagtcggacgcctgagcgtaaggacagccgagcaggaagtacgggctagtgctattgacggcgatgctcgcgctcgcggtcagtacgcccgtaggtgtaccaaaactcgcccagctatcgaggcacgcatgcgagtccggctcgcccttcgggtcgaacacgtcgcacgccaccagcgatccgcgtgcggtgaacacgaggccgttcttcttgtagctgctcacgccgatgatttcgcccagcgccgggtggtattggaacttcgaccacgagtccacgacacgctgcccgttgttcttgttgtcctcgtaccggtacaggtagaagtcctgcgggtgctctcgcgtgcggaacatgacgaggttcggtgccgtgagcggagtgatctgcaacggcgtgcccgacagccacgagtccagctcgttggacatttcgtccgtcaccgtctgctgcccgttgagtgcgccgactcgcatctgatgcaggctcgtgccttcgctgccgtactgcgcgtagaagatgtagttgcccgaggtctgcgccttcgcatccaccgaatccttgttggcactgaacgccttaatcagtggattcttgggactgaacaccgagtcgccgctgatgccatactgctgccggtcaccgaagatcacgaggtttccgttgtagagcgtagcgtgccggagcacgtcgccctcgctaccgtgagcgaagatttcgatggggtcgctgtcttcgatggtaacggcagagccacgccagaagttcaggtagtccgccgagcgcgaggagttgacgtagttctgtgctccgatcaccagccggtcttggaagacggacagcatcgtgatcggcttgtcgatgaaccacgggatcggcgaggtcagcccgtcgcctgccacccgcgcgccgtaagccggatgctcaccgctgcccggagccagagacgtgaggccagcgccgttacgcgcgatgtagcccacaccgttgtagatgtagagctgggacacgaggttgtcgatggtgcactccacgccgggcgcttcataccagtccaccgagccgtagcccgaagtctccccgttctccaactccgcacgcaggtagtacgactcgtcagcgcctgcaccgctcgggcgcacgcggatgatcttgccgtgccaatggaacttgacggcataggtcgcgtcggtaatctcctgccctgcggcatagaaggtcgtgccgtcgccctcgtcgtcaaccgttatgtccttgaactggtcgtcgtcaatcacgataccgcccttgatgtacgtcgccgacacgcctgcatcgaccagcaaatccgacagctgctcggcgatgtactccgggcgcgtctgctcggcgctcgtcacgatccactcgttgactgcggagttgtactcgttcactctgtcgttgacatacttctggtacgccgggtccggctccgtaccaccgggtaggtagaacgggatgtcgctggtgtcgagcgtgccgggatacgatgcggtcaccgtcttgaacgtcaccgtaagcaccgtgttgtccgtccgcgtcaggttcaccgtgtacgtggtgttgtacttaccgctgcgcacccacgctgcgaggcgctggatgttcgtctgctcctgccacacgttcgtgctagtggcggacgggatcgtggtgttgcccgcgatgtagacgtagctgccgatggctgcgagcgacgatgcgccaccgctgaccagcgtgttgacccacgtgctgttctcgtacaccagcgggatgaacgactcgtccgtcttgttgtagaggaacgcgaaggactcgcttcccaaggtcgaggcgtcgcgccgatacagcagtgcatactccttgccctcctgcatgaagtcgaacacgtccatgttgcgcagctcggccgaggtgacaacggcttgggaagcagcgaaccgcgtaccacgacggcgcacgaggccgttcaccggatcggacagcacgttgatctgctcgtgcgtctggcccggacgacgacggtgcgccggtttctgactgacaccctgaaggatgtcgggataggttccgcctgcctttgccatgttgcctccttagccggggaaagtgtagtggctatgccacgggtgtccgctgtagttgaagtaccgctgacgcagcacgtccacggatgcacgagcgaacagcgggttcgccttgatctggcggatgtgctcggacttcaggttgatgtagctgtcgtcgcgctgctgcttgatctttgcgtacttggtgttgtcgccatcgaagtccgactggaagcgcagcactgcgtcgtcgcgcacgaacatctgcacctcgtaggggaggtcatcgaagtccagcagccgaaccatcttggcctgcacgttgtgatcgaactcgtatgtgttgcgcttgcggtcgtacagtcggcgtccgcgctgtaccacgtggccgaaccggctcgggttacagtccagcttcagcacgtccgtggggaccatgatgtacttgctcgttgcctgcggcttcagctccacccattcggtgttgaaccacagcgcgagcgacgacacgtcgcgggtaacgcggtcgatcaagtcaactgcgtcgtccttgtatacgtggtcatcttccagcgtgttgagcttcgtctcgcccatcgtcttcaagcaggcgttcacgatgtcgagcttggtgatgaatgccatggtgtctcctgagaggaacaaggcagagacgccggagcgccccctgccgggatgttgcttagtccgcagccagagccagcgaggccggtgcgtactcgatgtcctgcgagccgatttcgtcatcaacgaaacggacgcgcacgacccagcccgagccgatggcgtcgtaatggacgcctacgacggtgccaacggagttggcgggcagaccggccacgccagttgcggcgacgacgcggttggaaatctcgaacggtcgatcaaagaccatgatgttgctcctgtgttggtggaaggcgaggcgcggtttgagttacccgaaggattcagggaccgcgcctagcggattaggcaaccttgtcgatgcggcccgcgttctcgacgcgatccagaccaacggcgaaggacatccacgagtccacgaagtagcacttcgaggcgtcgctccaccacaccgaggactgcaacggcagcgcttcggcgatcagcagggccttcggcgacacggccacagcgatcagggtgctgaagtcgccgtcgtagaagtcgtcgttgtcgtcgttcgacagcaggtgaccttcgatcacggtgttcggcaggttctcgctcgacagcaccgggacgccccagccgtggaaggtcgggatgccggtcagcttgttgccgtccgaggtcaggtactcgccgttgctgatctgctctgcctgctgcaacaggtagaagatcgccgggcgcacgatcaggaccacgccatcacgctgcggcttgaccttcttctcctcctccatgcgggagaacagcttgccgatggcggcgtacaccttggccggatcgttctcgtcaccggcggcggcgagcacgacctgcgtggcaccgaagtggccctcgggcgcgcggccgttgcgggtgaagatcgactgcgtggcagcagcggccttggcggcggcgatgctgatggtcaggtccacgaactcggcgatttcctgaccctgctcgatggcgatttccttgcgggtgtcgatgtcggtgaagatttcgtccagctgccagatgctgtgacgcgacagcagcatggtatcgacggtcaccgacgccttgctgaagtccaccggggtgccgtccggcgcgtcaccgcgcttcagcttctgaagcttggtacggccgatggccttcttggtcagggtgttggtgcccttgacctgcttgcgcgggaagaacttttccagcaccgagctggacacgtaggtgtgctcgacatcgccggtgaactgttcgaggatcagcgcgttctcgttgccggactggttgacctgattcggcagaaccgggacggtcgggaagatggtgctcatgctttatgttgctccttggttcttagtggatgacgcgcgcgttgagtgcacgcagttcttcggagtgggccgcaccacggatgcccttctcggcaaccagcttgcggtactcagcgcggtactgctccttcgtgagaggagcgacgccgttgatcgacgcggcgggagcggcggcattggtagccggtgcgcccttgacggtcgtcgcgggattggcctgtgccagagccatcaggtaacgcgcggtcgcctgagcgccgaagccaccagccgacagcgattcgcttgcctgcttcagttggtcggcgggcaggttggcccgtgcgaactgctggatcgcagcccagttctctgcgccacccacggcctcgtggacagcagcaacgttcgcggtgtgtgctgcggttgcggcagcggtgacgcgagcgatgctctccttcgccagagcgaggatcggtgcggaacccttggccttgtcgccgaggacttccagcttggcttccagcagggcgaagttgcccttcgctgcttcggtcagttcgcggctgtcgatgtcgaggcccacggtgttgacgaagtattcggccgcgatgttcaggccgttgtcgccgtagtccgggatcgccacagcagtcggcgcgccattcgccggggcggcgggctgtgcgggagccgcaggttcgagactcagcgcgtcagcagccggaggtgcagcaggagctgcgggctgtgccggtgcggcgggtgcaggctgaccgttgggcagcagcttgtcgtccacgggagccggagctgccggtgcgggctggttgccgttcgaggttgcgatcacggttgcgccgggaccaccgcccggaggtgcgttggaactcattgtgtctgtgtctccatgttgttggcgttatcgacctgctgcgatgcgttctgcatgaccagctgctgctgtgcacgctgctgcatcatctggccgtactcggcctcagtcagtacgtagatgttcgggtccaagccaccagcggcggcgaggtctgcgatccacgcggacagcttcagtcgttcgagaatctgcggcggcagcgcgaggacgttggctaggttgctgccgaactccaacagccggtcacggtcacccgtacgggagagcgcggccaagccggtgatgatgacaggctccaagtccttgcctcggatgtcgcggcccgtcaggttcatcacccaaaaggcaacgggtacctgcacgtcagcggcgatacgggagtaaccaccacccagcccgccttccagttcttcggcgaccatgcggatttcctgcgcggtcacacgttccgcctgacgagtcaccgccgtctgcaacaggaagcctgcgccgatgcggttgatgtaggtggactggattgcttggttggtttgcagcacaccatcgacgcctgcgttaatcagctcgatgtcgcccttcatgccgggaatggccgcgccgtttggcgatgccatgaagtcctcgacggaggtctgacctgcggggttcaccagccaccggaactcggaagcgaggatcgcgccctgtactgcggcctcggacagcatcgagagcgactggaagtcggcctcgtagtcttcgaccaagccggagccgtagtcatcgcctgcggccaagtcccagctcaccgcccggtagggcagcttgtctgcggtgtaggtcgaggagaagttggcgggcagcttgcagttgcaaatccacacgtcttcgttgtacttgccggtcttgtggtccagcttgacccacttgtactcccacaccattccgtcgtcatcgggcttgaagtccgggtgcgcgacaatggcagcgagtgcggctggttccagctgggtcttgtgcaccttctcccgaaggatcagctcgtacacctcgccggtgcgggtgcgcttgaccacgtagtgccgcatgttgagcacgcggatcgtgtccttctccaacaccatgagggcgttgcctagtacgatcagcatcttcagcaggtcgtacagtcgggatcggattgagcgcttgtccagttcgagactggcatcctgctcggccttcgcaagcatcgcctgcatggcctgcaagtcagcgccctgttcctgagcagcctgcttcgccttgcgcttcagctccaatcggaagaagggtcgggacggagcgaacagcgacatcatcagcttgttcgccagatggttcactgcctgcgcgccgagagactggaacccgtgggtcagcggctcggtatcctgatcgcggttcttgcgagggaacagcttcggcacagtccagcccgaatagcgttcgagtcggtacatgatgccctgacgcttgttgtcgtaagcctcgaactggcggtgagcggtttggatcgaatggtccatgctcacctcacaacaggtctgacccggccacagtcgtcagccgggaagctgcggtcgtggtcacgggtcgggtgtaggtggagcgggcggtcttgcgtcggccgatcaggtcggcagtctgcaagtcgaggtcggaagttcccagccgcacatcgacggtatcgacgggggcactcagcaacttctcggcgtactcagatgcggcctgctgtgcagctgcctgtgccatctgatcggccatcgcctgaatctggtagttcgtggattgagtttggaggttggtctgcttgtcgatagcagcagcttgcttcagcgctgcccgcttggcggacccaccaccaacgatgctacccataggttaactccttcgcttggtgaattggggagcatgccgttccagcaggtagccgtagcgtgcatacatccgtgtgagcgctcgtgagttccgagctagtgcaccgcctgcgctcagtgagtcgcagtggttgatgtcagccagatgttccatcacggctatgtaccggtcgaaggaactgcccggcccaattcgcagcaccatgttctcaacgaacgtagtacggttcttggagtaccacggtgtgacaatggcaaagcatagtaggtaagcttcatcaatgattactgcatccactagaccctgtgttatcagggccactgtgtaatcaggatcatcacagttgtagctcacagaagattctctgttgtctaccttactatcttctctagatgacagatacaaagcggccgttaaagccgccttgatctgctcactatcacccgtcgttggtgttcggtacggaggaatcaacggtgaaaccctcctgtaagatgttcaggacgcgggccatccccaactgcatacctgcctccaagggcgtggtatttgagttgacggacagcgacagcccggacagtcgccgcacggcggccagctggttcgggtggagcgtcatcaggactttcactttggcgtcttcggccatggtgtctcctctgtgctataggtgtaccaaaaggtccggcaccggttccgcttactctcgcggccgctccaaccggacctcagttgcctcgtgctataggtgtactgaaactccgtcagctgaagaagtacggagaatcaaggacttgccgcaggtccagctcgcccatcggcggcggctccggcaggaacgggtaggccgagtggaaggccgagagcacatcgtgccgctcgtacatcgacacgaacacctcccggatgatccggtacagggccgcgctgtcggcggcatgggtgccgaagtcgtcgtggatcatggcgaaggcgtcgatgccctcggccttggccgcgttgaccaccagcgtcaggtggcttgcgtcgaggctgtgcacgaagttcggggcgatgccgttgcggtgccgggacttcttcaccgcgtccgtgctcttgcgcagggacagcttggcgttgccgcacagcttggtgttgatgcggtgctcctcggattcccagtagacctgcaccaccgggaatccggacggcgtgatccaccggatgcggtcgtacccttggttgaggatcgacccggagccgcgctgcaaccactccatcgcgcccgctgcggcgaccacggtgtcggcgatggcctcacccatgcgcttgctcaggaagcgcgctgcggggccgtacagggccttgtcgagcgaggggaacttgccgcacttcaggtagtcttcgatgatgaagtccgcccacgaagactgccgggagccgtagggcagggtcatcacgctacgcttcaccagcgaacgtgtgaggccatggtcgagccacagcgtacggtacccttcggcatcctcgtcctcgcccagcaggatcgcagtcacgcggtctgcgaccatctggtagatgtcattcggcagcggtgccgggatcaggttagtcgccaccccgcctgctgcgtcgcgcagcatcgccgagaagttctgaagcccattgcacgaaccgtccatgccgactgcgatgcggctcaggaagcgatccccgaacacttgccactgctcgtactccatgcaccagctcagaaattgcagcggcttgtcggcggtcttccactcgtcgttgtgcaccgggtccgcagcgaacgccattatctggtcgtgatgctccgctacccacttcacacgatccggcagagacgccttgtcgtatccccatcggtttgctcctgtgatgcagaaccaatccttcgcgtccttcgtcagcaacggcttaccatcggcgaactccaagagtgccttctgcaagtccgaaccctgcggcgacacgccggtcgtctgcacgtacttgcggccgcggaagtcagcgaagtacacgaagtagatgctcgggtactcggcgaacttgcgcgccaccttcattgcgttgtagaatcgattgcccttgttctgccgcaggcgctcgtcggtgtgccagttggacatgtcgcgcttccactgcttgaactccaactcctgattgtgggacatggtttccttggtcatgtccttcgtcagccactccggcttgcgcggcttcggcagctcgccttgcgaaatgatttcctccatgtcgtgcaccttggcgatggccgacacggcttccatcagccgcttgttgatgcgccacggcacgcgctgcaatgcgttgatcgcggacatttcgttgcgcagctcggcggcgcggtactcgtctcgcgtctgagcgtaggtcttcaccatccacggattgagccgacgcatttccttcgtgtggaatccaccgttgtcgatgtccacccagtccatcggcggttcgacgcacggaagatagaacggcgtagcctcaatcacaaagtcgctgatctgcgtaatcagcttgcgcacctcgtcagtcagcacgatcttgacgtgagtcttggtctggaacttgcggtacgctgcgcctgcactggcagcagtctcggttactacgccaatctccaacatgcccaactgggcgagctgatcgcacaggtacgcgccgacctgatcgcgctgcgcttgcccccactccatgaactcgatgccgttcttgcggccctgcatcttcatcaccgtcatgcggtggttctcgttgacagagagcttgcggtccatgtcgttcatcaggtggtagaacagcgtcggctcagcgtcggcgaactgcgtcagcaggtactcgtggtacacgttgatgccaacgttcttcagcacgtcgcggtcgctgccttcgccgtgcttgtcccgcatgcaggaggtaagggcaccacgaacggcaacgaaggccacagcctcgtaccactcgcgtgcctgttcctcggcgctgacgggctgtccacgcttgttctgacgctcgggatcatacttggcgcgcagaagtggcacgtgcgcttgggcacgaccgatgcgcggggagtcgatgtccgcacggatgcgctccgcaagcggaagcacgaaccggcgatacactgcttgggcgtaggggttgttgtccgcgccgcccttctcctcgttgcgggcgatggacttctccatgcgctccttaccgaaggcgtaggtttccagttcgagttccacttgcgagagcatgctacctccgttgcttgatggtgaagtccgtcggcgggtagcgcttcaggatcatgcagaccagtgcggtgtgcatttcgttgatgatgtgcggccacgcaggaccaccgacctcgtagctcgggatgcactggcggttgaagaactgctcggtgccgcaccacgcggtggcagtcacagtgacgtgacctccaccgtagggagagaagcggtcaccgtcgaaatccagctcgggctttccgaatcgaatgtccatcagcccctccgttcggcgaggaagcggtccagcgattcgatcaccgcatcgcgcaccgtctcgttcggccacagggaaccggcgtactcacggaacgggatgctcactcgcacctccaccgtgtcgcgctccatgttatgccacacttcggtctgaacgttgctcaccggtcggcctccttcttgtcatggcggatgcccttgtagcgcggctcgcgcagcaggccgtacttgctgaaggacatggcttcgatttccacgatgtcgccgactacgggaacttgcgaaagctggtgcggcacgccgctcccgacctcctgctccttaccatcgccgaggtccacgaacacggtgtagacatcgcgcccggtcttctcgccgacagcacggccgatgcgtagcacacgcaggtccagcgtcagggtaggcttgaccttgacgacttcgccgttcgtgcccttgtcgcccttcacccacttaccgctcggcttgcgcaggatcaggccgtcgtatgcgccgccctcgcacaacagcttcgccgcctccatgctgcccagctcttggtcgatcaggaagccctgcgactctgcgtagaacaccggagcggtgccctctgcgatggcatggcccatgctcggcaggcggctgacgcgctcctgatacacgaggtcgctgaaaccctgctcccattcttccagcgtcacgaagtcgaacaccacgaacatcggctcggtgtactgcgtgccatccttcttgcggaacatgccgctgacggtgggctggtcgatctgcgggtgccagtattccccgaagtacacgccgaccgggaagaacggcgcggatgcgagagcgttctcgatgtggtgcgcgctgacgacctgctcgccagtccgagagaacaggtcaaccaccccgcgatccaccggctgcatctgcacgtcgcccaccttgattgcgtgcagacccttgttcactgtcggcacccagtggccgcgcttgatggcgaccatgttgcacccgtcgtacttcggctgtgcgatgtactcggtgcgcagctgctcctcggtaggccgcagcttcttcttgatcttgtcctgctcgactgccttgtggacgatgtagctcatgcgtggtccctccaaatctggaacatggcgagcggcacttcgtaccacggaacgtaacgctcccagtacgtggccttgccgtcgtaccactgcacgcggaagttgcccttggtgaaggcgcggttgatcttgaagccgcgcttgcgcttcttgtagccgggagcgacccggacattgctgcgaggcacatcaaacatcggcgctgtcctccttcttggtgccgtcacccagtgcagcgttgaactgcgcgatgcgggatgacatgaacttgttgacgatgccgccgatccacagcttgcgaggggcgagggaaccacggtacccttcccactcgtcggcgatgcgggtatacagctcggcctgagcctcgtcgggcaggttcgggaacccggccttgaccgcgttctgcaacgcctcctcgtggtcagcactctcgccccacgcaacggcgttctcgtaggacttgataagcatggcggtctggttcttgtagagcattcatttctccttcgacgggaatggaacgaaacctgcgaggcccttcatcacgaggatgcagaaggcgtcgtcagggtatgtacgatgccagagcgagttggcccacccggcatcgaactgcttgcgggtacggtgctcctctaggaagcgcgcccactcggcctcatgtgggacgtaccgatgcacttggccgcagcgggcgcaggccattagtcacccttgctgaaccaacggcggatgatgtactggcggatgaagcttatcgccgtgaacgcaatgccgatggcgtgcgccgaaagcagcgggtgctcgggatgccacagcaccggcagcagggcgatgttcgctgcgtagttgatgctgtacccgatgccgatgttcacccaagcctctttgatcgagcgcgccttactctgcgccacgggccttctcctcctcgcgcagttccagctccaacaggaacagctcgttgatgatgtggtgcgcccggtggtggattcccgtctccgggtccagcttctcgccgaggcagcgcttgttgtcgtgccggtagctcgcgtcctgataacgttcgagcgccttctccacgtgctgccacgaatgcgccttgtacttctgcgcaccgaaggtcagggtgtcgatgacacgggccagtgcacgcggcacgccctcgtgcagcagccgcgcctgcggcttaccgccatcatccttcagcccgacaccacggtcggacagtgtgcgacgatcttcgtcacggtagttcagtgcttctggcaagggaacctcccttcgtgcggtggtgacacctcccacgcccatcaggcgagtgaggaactgcgggcggatgatagattccttcagctgcccgtcgaacagaactccaacatcaacggcgctgatcgagcgaaccacgccggacctaccgacgaggcccggagcggagccggtatagcgtacgcggtcgccgtggcgaacgtcggtaagtctcatgcgcttctccttacgcgggaacggtgatgtgcttgcgagcctcggcgctggtcgtgagcttgcgcccacggctgtagccgtcgcacacggtgcactgaagcaggaggtacgttccgacctgcgtacgggccggatcatcctgcgggatcatttcgttgcagccgcacttgttgcagcgatgctcgctgccatcggccttgtagtacactgcgacgttcgggtgctgcgagtaccaaccgcgcagcttcttgtactccaacttcatggacttcacgtcgattcggttgtacgcttcgcactcgtcccatgcgccgggcaagctctgcatgcaggccacccacaggtcgaagccggggaagttgtggtggtcgtacttgcgcagctccggcacgatcacgccggtggtgtactccaacttctgcgaggtgaaggcgaactcggtgcggttcagcagcagtgggtcgatcacctgcaccggagacacgggcgggaacccgaggatggcgaggcgcgccttgatcttgcgcaggtcgaacttcttgccgttgcgagcgagcacgaagtcggcggcgttgagcagtgcccacagcgccttgccttgcttgcgatcatcgaacacatcacgcacgttgcgctgatccatgtagaacgactcgtcatcgtccagccactcgcaagcgaacgacatcagcgaccagtcacgcttgatctgcttgacgctgaagttgttgttgaacatgccccagccgtagaactcgatggggaatgtctcgatgtcgaggcagagaatcttcgggccgcgcttcggtgctcggcgaatgaactgggtaagggtcacggtgtctccttgttgatagcccgacgctttcgcgccttcgcattgcgagcgatgcgcttctcgtcgtcggtcttgaaggtaggatgcaggtaccccgtgatgttggtgaggtgcgaccgcaggtagttggggatgcccgcacagaatgcgaacacgtcgcgcacgccgtaccggcctgcgttgttctcgaccttgccaagcagcgagttgcatccgcgatggagcaccccgcgcacagcgccggtcttgtggtcgtggtcgagcaccggatcgagcggagccttcaggccgaactgtccctgacagagacagcaccggttgccttgctccgctgcgagcttgatgcgcagcagcttgacctgtgttgcagtgagtcgcttcatgctttgtatgcctccaagattgcgcgcttctcgttcacgtcctcggcgaggtcatagaacgcctgcttcagcttcggcccaaacacgtcgagcttcagcacgtcgagcagttcagcgtcacgatccgtccgcatccacaacagcacggcttgctcggcgaaggtcttgcgccagtcggaacccagcacctcgctgtacttgccacgcaccagcatcgctgcctcggcgttgtccttggtaccgaacagcaacgtctcggcagtgaccttgcccacgtcaggcaggccggggatgtggtcggcgctgtcaccgtggagcatctgcatccagaaccacttgtggccgtactgcaaaccgttctcgcccacgatgtcgtaagcgccaagcggaacctcggtgatgtcgtagccgtcccagtctacgtgcacgccgcagaacattcgcatgtccttgtcggcgctgtgcaccacgtgcaggatgttgtggtgcaatgctgcaccctcgttgacgtacgcgatgccgtcgtcggcctcacgagtcagccagattttgggagtgaaagcgtcgccctcgtatgtctccatccactcacgaaggaacgcccagttgttgggcttgcggcctgcttggcgctgaccctgatacggctgcgtggtagcagcgaggaagcgatcacccttggtagacgcggcgtgcgtcaggtgcatgacgatcttgcccgctccgctgacatgcttcagctgtgcgcagcgggagagcacgttgcgtcgtgcatcccccgccgagcagttctcgctaccagccgcgaagtacgccatgtagtccccgtcaacgtgagcgatcacgcgcgggttgtgctgacgtaccacttgcaccggcatcggggagcgctcaccggccgctgccatgagagcgctcaggtccatcaggcgatgcccgccatcgggtcgctaccatccaccgggaacggcggcttgtcgtcagccggagcagcgtcggtagccgcagcgttcgccacgtcgccgaccacttcgtccagcgcatcgacgccttccttggtgaccgtgctgctgcccgacaacttggcggcggcgtagtcgtagcacggcaggcccttgaagttcagcgccgcagcgatgcgcagctgcgtcttgttcttcgactgcgcttcgtgagtgaccttgccggtcttctcgtccttgcgctccgggtactcgccggggatgtagatgctgtcccacatgtcggcatcggcgaagtcccacacgaacgcacccagcggggtgatctgctgcggtaccgggatcacggtgtccacgaacttgccggtggggataccgttctccatttccggcaccggcatgaccggcttgcggatggaagccttgtcgatttcggcgaaggtcttgttcgggtcgcgcttgcccggcttgtggatgacttccagcagcacgccctgacccagcagctgcacgaagtgtcgctcctcggtgcgcaggcggctgaagattttgaagtagtgcgccttctcgttggtggacaggccgagggtcagcgtcatgcgcaccggcaccggaccgttgtccgtgtcgatgtgcgggtgctgcttgccggtcagctcgaacacgatggcgacttcatcctgcgtcttcttcttgccctcgaactcgaactcgtgcttgcccagctcgtagtacccgacgatgcgggcggtggtcacaccagcagcgggcggggtgtagtcgaagttgccaccactggcaaccgactgatccttaccctgcgtggcgaccttgttcaacagtgcgtcaagactcatgcgtgttgttctccttattcaaacgacgggttgtgattaccaacgaagtccttgcggatcgacgctcggtactcgatgaccagaccggcgaactctgcgggagggttcttctcctccatcatgttgtcgcccatcttggtttcacacgggacgccaagtggcagcgtccagttgaaccaccactccatatacaccgacgcttccagcatcgaggcgtgcagcagagcagaggccttggttgcgatgtcgccgtgtgcatccacgtagacggcatcgtgcacctgattcacgagcagcgcgcggcccaaccattccttcggttcggtcacgtacttccggtagaaggcgcgcaggctgacgtacatcgccgccttggcccactcaccaccggtgccctgcatcgggtagttcttgatttccgtaggcgagaacgactgcgcacagccacccttgctcgcgggcttgttggcgatgaacaccggggacggtgactcgctgaaggaatacatcttgccgtccggagtggtccagtgcgaccggccaagctgacacgtaagcccatgtggcacgccttgctgcccggcgttgggatgcggaacgaagcgttgcgtgctgacgcggttgcgcttgatgtgctcgaccatgcggtcgatgtactcgcccagctccgggtaacgctcggcctcaccacgcaccagcgcctcgacttcttcctccgacatgccggtggtcgcagcgatcttcgccacgcccgcaccgtacgcacgctggaaggagaacaccttcgcgtttccgcgcttcttcttccacttcttgtgctcgggatgcttgtcgtccttgctcgccttcaggatgaagtcgtagtcgtacttgccttgctcgccccacgcctgctctgcacgcaagcagtgcatgtcgaggccccgcttcaagtcctcgatcagctgacggcactcggtgaggattgcctgcacgtagatttcgagggaggtgtagtccgactggatgatcttgccacccttgtgtcgggacacgaaggcgcgcttgatctgcgaacccttctcctccaacgtctcctcgtccagctcacccttactcacgttctgcaagttcggatcgctggaagacaagcggcccgtgaccgtgttggtcatgttgagcttgtggtggatgatgccgtccggcccgaccagcgtgagcattcccttctgctcgccagtcttctcgtccgtcgtgatgtagtacgtggacaagtccttgtgcaagtcagcgcgccgggcaagcgccttggtgaacggcaggttgcggtagcccagcgcctcgatcacatcggcggcggtggagtacacaccctcgtcgctcttgctttcccacgcagcatcaggctcggtgtagccggggaactcgaacagcatgtcctcgttgcggaacttctgcttggtcaagtcatcgaccttaaccttcttggtcttgtactcccccttgttcttgccgctgccgtacgtggtgtagcgccacaggttgtcgaagtcctcggccgggggcgtcgccgtcgtagtaccatcgaccagcacgtagtgcacctcgtccttctgcacgtacgtcggcccgccctcggtggacatgatcggaaccttggccgtgtacttcaccttgccaccgaagatcagcgcgctcttgtggaagcggctgttccagttgaaggtcagaccctcgggcaactcggggatgaagccgttgagttcggcggtcgccgttgcaagctcgacctccaactccttcgccttcgcaagcgcccagtccttgtccacgtacatgccgttgtactcggcttcgatggtgaagcacagcgcacccatgttgagcagcgccgagcgcaaaccaccacgtgcacggaaggcagcgagctgaccgaggaacatcttctcggtgttgccgatgtcgcccacgtcgtcggtgtcgttggtgccgaggagataatccatcagcagcgtcttgtcgatgtcgcaggtgtccacgcccgcagcccacagggacttgactgcatcgtccttcaggttgccgccgtagcgtggggccgtctcgtccatgctcgccatgtggaactcttgcgtcataccatgaagcaggtactccgcaagctggcagtcccacaccatgccgccgccgtcgatgaactcgatccatgcctgccgattgagcgggccttggcagatggcgtgcaggatgtcgaacttgatgttgaacccgacgaggaactgctgcccgtaacacagctcgcgcagccacccatcgggtgcgccgcccatgtactggttgtcgattccgatgcgggtgtcgtagtacaggccggtgttccgtgcgtcgcccttccgcttgtagccaatcgccacgatcttgttcatatcgtagaacggattggccttgcgcttcaggatggcacggatcgtggtttcgaggtcgaaggaagtgaagctcacagcggccaccgttgcagggccagctcgtacatttcgtcggacgcatcgccatccaagtcaagcccgtcacgcacccaacggaacacgatgatgcggtcctgcttgtccttgatgttgcggcgcttgcagatggtggtggcctcgaccgcgcgctgataccagccggagtcggcggtcaccatgacgttgaacacgccgttgcgcagcgcataccacgtgtcgctgtagtcctcgtcctcctcgtagtgcccatcggcaccggagcacagggtccatcccgcctcgaccagcttggcgatggcctcgtggaagtcctgcaccagcacgaggtagtcgatgtccgtgttggttacgggcggctcgacggtgtagctgctgccggtacgactggacgtgatgacgcccacgttgcgcggcaggtagatattcggttcggtactcacggcgtgttacctccgggcttggtgatccacagcgtgaagcacgggatcaggttgatgcaccagcgcttgttgtgcggcgagtagtgcacgccgatccatgtgctgtgcttgttgcgcaaccatccccacttccactgcggagcatcgttgcggccttcgatgtagcctgcgtcgtgtaccttgcgcatcataccagcgaggaagttagcctgcgctgtcgatgcacactggtacgactgcccaccgaagtggacctgcgcacacccatcgacgtggattttgtccttcgtcatgctgcctcctgatagaagcgggcacgctctgcgtccatcatcacttcttcccgaacgtcacgcttaccgcctgcgcggtgcagcttgttcttcggggtgccgatgtagcggaagcgttccatcgctgggtcattgagcttgccgcccatgatgatgaagtcgcacgcaccctgcttgccggtcttgctgtccttcagtgcggactgcggcgggtactgaatgccctcaccctcagcgctgatctgcgaagtcgccacgcccacggcgtcgtacttcacacaccagttgcgagcggcctgatacatcgcctccaacatctgatcggtacgctgtccgccgttggtcatgccaccggtgaacgtgatgttgtcgatcatgtcgaagatgatgaagccggggttggtctgcttgatgatggcctcgacctcaccggagttgaacccgtggatgtcgtagaactgcatgcggtggatgtccccgcccatcgcatcttcgatgcgcttgcggatgctgccatccttcgcccactccaccatctcagggatggtagcgccgagcagcgactgataccaccgctgcttgatgcgcttgcccggtccctcgttgttgagccagatgccggtgcgcttctggtccggccacaccgcatcgagctgcgtgatccagtgactagactcgctcgttaggaacgtggtcttgcctgcgtcgggacgcatggcgtagataccgaagtcaccgccacgcatagcacgcaggttgcgcgccaatgtgggcagtcggaagtggatgccgatgtcgtgctcgtccatttccatcagttcttccggcgtctccttgaccagcgggagccgcgccttacgatccatccggtcggtgatagtctcggccaatccgtacagctcgtcgcgcaggctgaactccgctccgccattccactgcacgatcttactgaccgcagtggtggcaagctccaactccaacagcttctcgatcatgccctgctctgcctcgggcgggaccggctcgcgcatctgcttcagcagaactttgagcagggacttcttgtcgtcggcctgcgtcttccacttgaactccatggcccagccatcgaacacatcgaacggcaagtccttcgtgtccgggaactccttgtagtacgcacgcaacgcatcgagcatcagcacggtcagctcgtccagcccatcacgtggtgcactgggtaccagccggtcgaacttgccacggttggtgcacaaccgcagcagcgtggtgtcaagactcatcaggttctccttcgggttcgtacttggaatcgagctggtgataccgtgtgttgcgcgtctcgaacttgcgcccgccgtccgtcacgtacagcaccgtcgaggtgtgcacgatgtcgcagtcgccgaggttcggatgcgcaagcacgtcgccgagcgtggcacggaagccaacgacgggcgggatgatggcgcgccgatagcgcacgatgggtttgctcattgcagcttctccttgatgtagtcggtcgtgtaatacttcgggtcacgtggtgacgtgatgttcctgtagtccagaccaaacgcacgtagacgcgcagcgattactcgcgcgctgtcttggccgggattgctaccgttgcttctacctctgtcgtcatcgagccacgttgctacacgttggcctcgatcagtcagctgcttcaacactttgttgtgcagcttggtgccgagcaacgaccacgcttctgtgcactggcccaccttgaaggcggatagcgggtcttcgcatagcacgatggtgtcccccttgcccacgccgtagcgtgcgacaagcccatccttcggcacatcaggagtcagccatttgggctgacggcttgtgcttcgtgctgtccagtacacaacgtcgtcgccttcagtgatcggtagtaccacccgcccgatgctcgggcaccagtacagccgcagcttgtcgatcatctgaagcgagagtcccatcttaaagaaccacaccttcgcatcgagcggccactctcgggtgtcgtatacccgtggctctggcaactcaacagtcgcacgcactctgcgttcgctcgtctgctcggcgtggattcgtgcaagcttggcctctatactctcgtgctcacgcttgaatcctgtgccaccgcacctgaaacagaatgcggtggacttgtcatgctcccgagtgataagcaagggagtcccttccccgcaatcatgcggcactcgggtgcggtggccgacctgtagtcgctccgcatggtgcagccaatcgctgtcgggaagggtctcgctcatgctatcctcgcttgattactcgaacacctcgaagatgtcgttgtcggtggcgtacagcacggagccgttgccatcggtgctgacgatcagccggtcaccagactcgctggtcagcttggacaccacgaaaggcgtgcccttggtcagcttgttggtctgccgggtgtcgatcaggtacgcggtggtgccgggcttcagctcgtcgccgcgcttgactgatgcactgaccggggccgggctggacaggctcacgactgcccgccttcaccggcagcagccttggcggcggcagcttcggcggcgaggcgctgtgcctcggcaacggcggcgtcgatttcttcctgcgccttcagcacttcttcggccgacatcagcagggcgctgctgtcgatcaggttcagctcggcatccagaccttcgccggtctgcaccttcagttgcagcacgcccttgtcgttcttgccggtggcgacgatcacgccggacaggacacgcttgttcagggcacgaccgaacaggtaggacacggcgtcgccggacttcagcgcttcgatggctgcgctgttggcctcgaccgcatccagcttggcgagcttgtcgttcagcgcatcgaccttggcctgcgccttggcgatgtcttccagcagctcggcgcgcttggcttcgtagtggctgacggaggtggtctgttcggtggtgttttcgttcgacatgcggtgtatctcctttcattgacgggtttggttggtggaccgtaacgtgggccagtcggcacagttcagtgctggattactggaagatcagctcgctgttgtacccaccgccgccattgtagaagcgacggcgcagcacgctctcctcgccgagcaccagcaggcggtccacgatggcgcggatggcgctcatgtactggtccaccagctcgctctgcaagttcatgtcgaagcggatcacggtcaccgcctcgtcatccagtgcgccggtatccttgcggacgtacaggccacgggcattggtcatcgtcgcgccaccgatcagcttgacggcggcggcaatctccggctgcacgttgagcagtcggctgtcgggcacggtcacctcgacccagcttcccatgcgcaggctcatgctgcacctgccagtgcggactgcacgttcggctgcaacgatgcaccagcacgcagctcggcagcacgacgcttcatgcgggagcgcagcttgcggcgctgcttgttgttgtcgccgaggctatcggccacacgcttcagctggttgttgccgacgatgcgggtctgaccctgccccttctgcacggggaagtagtcctgccccagcatcttgcgcagcaccgggttgtcgatggggatcagcggcacgctgacgtgcaggtaccggctggtatccggtgcgggcggcggcgtgtcatcgtcgtcgtgctgcggcttcaccgctgcaaccaccttgtccttcacccagttggcggcaccgcgaatcttgccgccgacgttcttgatcttttccatgaatcccatggtttacttcctcctcgtgccgaagtgattgaactccgtctcgtgccacacatagtacgtggtgccgagcgggtcggtgtctgcctgccagttgcgctgggtgcagtagtcgttggctgcgtcgaggtcatcgaacgtcagcgagaacccggtggaagccgggccggtgcggaaccggcacagcctaccgtcgtcgtcatggtactgcccgacgacaacccacggtccacgacccacgatccagtacagcaggatcaggatacgcagccagagtttacgcatacaccgcctcgatgtagtagcccgagggattctgcttgctgcgcttgtcaccgatggtattatcgatgatgtcacgggcggcggcgcgagtcgggaacagcaggttgtcctcgctgttgttctcttcgtcaccatcgacgcgcaccgttgcgccgtctttgtagcagctggtgtagtcaccgtcgtacttgatacgctagcccttcacctgacgcaccggcttgcggatgctatcgcccacttcgatgatgtgccagttgaacaggccaccaccgttgaaggagttcaggatgtcggcctcggcacgggcggcggcacggcgctcgaaggcggacaccgggccgggataggtggcgtcgcgcaggctgtccagcagggactgcgttgcgcccttggtgcgcagcagctcgaccagtgccgtcacttcctcggcggtggcgttgcggcccgtgccattggcgacgacgccagtgatgacgccatcctttgcggtggccgggatcgaagcgatgaagtacagcttacgcatggtggttctcctcattgacgggtgggatttcgatttcctctacggtgtagagagtgggcaccttctcgtggtgcagacggtggtgtgcgatggcctgctcgcacgcctcgtggctggtgtggtgcccgccgaggatataatccccgacagcccaaccctgcacggtaacgagcggcagcgccttcaccacaaggcgcaggctgacctcacgcataccagcgctccacgctgtgctcatgggtcacgaactctttccactggcggggcttctcgcacagctggatcggcttgcgctttccactacggatgcgcttgtagacgatagggatcatgcaatatgccctcctgttgggcgtggttccaaagctacgccctcgttagaaggcgcagcggtagatcacgcgtggttcgggtgccacttcactcggtagcgacgcagacggttcgcatcgttgccgacgtgcgcagcgatggcattgcgtgcagcttgcgcagtggtgaccgttccgttgagaccggtcacgctggacgtgttccatcccagctgcgactgacgggcggcgtgcttggtgaagaactcggcggtgtagaagccgcgatccttctccgggccatcgggagtaccttccggcaccacacggtacgcatcctcgctgataccctgcgccttggcccgcgccttcagcatgcggtacgctgcattgcggctgcgctgcggcaggcccagctcacgcacctgtgcccagttggcaagggcgatgccgccgtggcgcagattgaactgcacgatccagcccttggcctgcggcttgttgaccagcccggtctgcgatgcagtcagggccacgtggcgtgcgctctgatcgtccatcagtacatccggcagcttacgcggcaggttgtcgggcattgccgggccgggcaacaccatgcggccggtcacgctgccgaggaagtccagctgcgaggcatccaacaccaccggaggcaacggagacagcaggcacgccatcacccgcgcctcgatagcagcgaagtcaagttcacgcatgccgtagcccacggtgaacgtcggcggtgcgaacaggtcacgcagcagctgcgcctcggcattgctgtcccggcaggccgcgataacgtcgtcctcgaattgcaggataccgtcacggtcgaagctctcgattccgaagtctcgcagctcaccgtgcagagtggagaactcgtcggcgaggtctttgcgagcatacggctgcgctttggcggtcagcgcacaggcaatgtgcagggcagcacgcagcagggacgcttcgcgctgggtcactcgcaagttgatcttgggttccatcatggctccttgaatcggtgggtgtggaaggctgtgcggtcgccgaagtcatcgacaaccacccagtattcgggaaaggtgaatccgttctccatcgtgacgctcgggaccacctcgactacggtgtattccttgccgccagtcaggcggaacagggccgtgtgcttggatacaacgacggtcccggattccatcacgcagtcgccttcaccttggcaggcttgggcacggcgcgggcagcgttgatgacggcctgttcttcctcggtcgggacataaccgccctcggtcgccttttccagacggcccagcagcttgtgcaggtcggcggcgaaggagaacgcctcggcgggcttctcggtcttgaagtcgtaccacgccttcgcggcggcacgttccagcatttcggccagagcttcgccctcgacgcgcttgctcttggcaaacttcatcggcgcgctcgccttggtttccttgtcgtcgttcggagccatcgggccgaactcggacaggtacaggcgcagggcctcatgcttcatgccgttgcccacggcgagacacagatcggaggcaagcgtaacgtcgccgtggatgtgtgcatggttgatgaccgcaatcgcggcctgctgaatctggtccaccagcttggtgcgggcggtgttgatcgacttgatggtgcgcttgatgtcagcgcttccggtgatgatgtccatggtggttcccttcaggttgggtccgtgccgattgcacgacactaggccctcttgcgaaggcccagtagcttgcattcagtggatggtgggtgcagcgagcttgatgtcataggtccagcgtgcgccggtccattgcaggttcgatacagcgcccggcggatgcttcgccattgcccgttcgtggcttgccatggcgttgcggctgtaccctgcggcgaagtagaatcggatcacaggtaagccctccggtcagcggcgtggttcgcccggttcgtcccgctgttgccctcgacaacaaacacagatcgctttccagcggttccgtggcgggcttcgtagcgttcggcttgtcgcttgcgctcggcgagcttgcggtcatgctccgtggtgcgcaggtccatcacgcttgcagtccgggtgaactggcagaagcggcgcttacgctgggtgcggtcgagattggcattgatcgagccttgcatgttgtgcctccatttggcactggtgggaaaaactaacagattgatgcgccctcagaaagccgtcgagtcggtcaatccctcattctcgattagagccgttgcatcgcctatcgtgggcgcacactgaccaccggatttgcctgcatggtcatcgcaaagggagggcgcatcaatctgctagcccttcgggctgtcaaccctactccggctagcagtgccattgtcaccgtgtggcccatagagccttttcacgaaacgcacagtattccatgcgataggaggctcaccacctccttatgaccggcttcccacctttggcagtgggttacgctgcgtggccgactctcacggcaaatgcaggccctaagcgttaggcttaggtaaagcggcaccagtgttgctagtctggtggattctatgggcctttgacatcccagttcatccggttatccgctagtgctacgttgtagcttggcgttccacccgtgggcttcacgttacaccctacccgttagcggtagtcctacccggtccagtgccggtggtcctcagaccgtggtgccatactagcaccctgtttgcatcctgtcaagcccttggctcgattcgggtctctaacccgttgggcgtcctgtcgccaccatcctaccatgtatgccggtagtccgcaaggtgctagctgctccgctgttccggtggctaccacttgccgcctatcatagctcactgctagcttagtgtcaagcgtggttcggtagctcctcgcatcccttaccagtgactcccatgtgcccttagcccacttgttggcggcgccactacggatcacgtcactcgacttgcgttgcagcttactaccattgcggccgtgtgtcaaccgttggcctagcgggtagctaactaatcagctcgacagagtaccgatagacggtgattcaggttgagccgactgtgtgctataggtgtaccaaaaggccgaaacgatacagatggccctcacacgcctacagctgcggttcgcatggtacccggtaggtatgtacctgtcaagccccttgcggccctcctgcggccctgtcgctgcgcctgacgcggtgtcaggtgtcgcggtagctcctcagtgacgccagtagaccacac

SEQ ID NO: 7 - DNA, 44415 bp, unidentified
  source 1..44415: mol_type = genomic DNA
tgattgcggtgggcatgaacaacgtcaaccgcctgcaatggaagctcgtcggcaatcccgacgactggccctaacctacaggagaacagcatgaccccgccgagtgtggtcaatgaggtcgtccgaacctcgccgcttacgctcggcgcggtctacctcaacttcatcagcacgtacggtgctgccatcgtaactacgctcgccattctgtacgccgtcgctcagttctactggcgggcacgcgagcaccgaaagatcatgggaggcaaggatgtcgaatccggcaagtgagggcgcactcggtgcgctgcacgaactggtcgcgcgtgcgctgatgcagcgcatccaagatggcgagctgtgcaccgcagccgacatcaatgcggcgatcaagttcctgaaggacaacaacatcacggcgacgcgcgaggccaacaaggcactcggcgagctggaagacgagctgggcaagcactcgctgcctccggctgacgacgacgagttgcagcgtgcactcgacaacatcgttcactttccggggagcgtagccaacaatgcgtgaatcagctgaagcggccgacgtgcgccgcaagaagttggagctgttgcagaaccactaccggcacttcgccaccttcatgcgcgacattatgaaggtgctggggttcgagccgacgtggatgcagtacgacatcgccaactacatgcagtatggcccgcacctcgcaatggtgcaggcgcagcgaggcgaggcgaagtccaccatcgctgccatctacgccgtcttctgcctgatccacgatcccactcaccgtgtgctgatcgtatcggcaggcggcacgcaggcatccgagattgctacgctgattcagcgcatcatcctcacggtgccgacgttggagtgcatccgcccggacaagaacgcgggcgaccgtacctccgtggatgcgttcgacgtgcaccactcgctgaagggaatcgacaagtccccgagcgtggcgtgcatcggcgtcaccggcaacctgccgggtaagcgtgcggacctgctgatcgccgacgacgtggagtccaacaagaacagccgcactgccgcgaaccgtgagctgctgctgaccatcacgttggagttctcggccatctgcaccggcaagcccggtactccgggtcgcatcctgtacctcggcacgccgcagaccggcgactccatctacaacaccctgcccggacgtggctacgacgttcgcatctggcccggtcgctacccgaccccggcacagcgcgagcactacggcccgcatctggcaccgtctatcgtgcagcgcctagaagccgacccgatgttggcgttcggtggtggcccgatgggcgacgagggccagtgcaccgacgagctgttggccggtgagcagaagcaccagtccgagctgcgtcagcgtggaccgtccagctatcagctgaactacatgctcaacacgcggctgatggatgcgctgcgcttcccgctgaagaccgagaacctgatcgtgatccccggtggtggcgaccgcttcccgctgacgatcacccgtggcctgagcaacgctcaccagcgcagcttccagtccagtgggtacggcttcgtgatgatgatgccgcacgacatgagcaccgagactgcccccgtgcagggcgtgcacatgcagatcgacccggccggtggtggtgccaacggagacgagacggccttcgccgtgaccgccttcctcaactccaccgtgtacgtgttggccgtgggagctgtgcccggtggctacgacggtgatggcttgctagaactgcgccgcattgcggtgaagtacaagccgaacgtcatcagcatcgaaaagaacatgggctacggcgcgttcgccaaggtgttcctgcctgtcctgcgagaagatcgcggcacggagaagggatacaagggcgacatccgcgaggagttcgtgaccggcaacaaggaagcccgtatcatcggcactctcgaacctgtcatggctcgcggctcgctggtcatgctggaatccgtggttgaaatggatcacgagtacacccagcgctacgccaccagcggcaagcgtcaggtctacagcctgttccaccagatggcgaagatcacgcagcagaagggcagcatcgcacacgatgaccggctcgatgcactggaaggtagcgtgcgtcactgggttgcgcagcttgcactggaccagaacaaggccatcgccaagcagcagcagcgagagttccaagactggatcaacgatccgaccggcatgaaggcagcgacccgcaagagtccgctgcaacgtggccgtccatccctactcgaccgttaccggaggtaaccaatgcagaagtccgacttcaccagcaactacacgggtctgttcggccgtggcaactacctgcaccgcgaactgctcgccctcatggagcacgcagagcagcatcccgcaaccgcagcgcagctgctcgcgcagttccagaaggacgccaccctcgtgctggacgccctgatcgctgcgggcgcacgcaccgcgtcctcgggtccgaactccggcccgcacactccggtcgatctggacccggatgacgatccactgaccccgtaaggagcaaccatgaaccagcagcagaaccaagataccagcaacaaggggctgttcggcctgatcggcggcatcttcatcggcatttcggcaacgctgctgtcattcacccaaggccacgaaggggtacgctacgctgcgtacctcgacaccggccgggtgccgaccatctgctacggccacaccaagggcgtagcgatgggcatgacggcaacgaaggcacagtgcgacaagtggctgatcgaagacctacagatcgcccagcagggcgtgcgcaagcacctgaaggcccccgttaaccgcaaccagatcgacgcctacacagacttcgtgttcaacgtaggtgagaaggcgttcgccgacagcaccatgctgcgcaaagcgaacgcaggggatcgtgaaggtagctgcaaggagttcctgcgctgggtctacgtcggtaagctcgactgccgactgtccagcagccgttgctccggcatccccaagcgccgcgacgcagagtttgctctgtgcttgcgccccaacaacgaggtgatccaaccgtggaaaccccaagtgaagtgatcgcgcggctcggcggcaagctggttggcttgctgctggtcgtgaccatgttcgtgtgcttcggtctgtacgtctacggcctgcaacgcaaggtggagaagctggaaactgcccaagtcggcacgaccgctaccgccaaggcggcgcagacgcaggctaccgggtacgcgacctacatcaaagagaaggaggacgtgcgtgttcgcactgaagaagttcttgacgctgccccggagtaccgggatggcactgttcctgctgatgtcgctgacctcctgcgcgaacctgccggtccctgacgactccctgcttgcagactgccacatcacctacctcggtggggagaagggcaccacctcctcgcaggacaaggtggtcaagctcgcgcaggaccgccgcatggacaccgttctgtgcaacaaggacaaggctgcgctgcgtgcgtggaaggccgaggtgtgcggtaccggtaagcgccggtgtacgggtgacaaatgaccaccatcgcatgggacggcaagcacctgtgggccgatagtcaggccacgcagggcgaccacaagcacaccgtgcgtaagatcatgcccgtatcgacacccaccggccctgtgctgctgggtgtcaccggggatttcacagtgcttcgcccggttctcgctgcgcttaaagcgggcgaaggctacgaggagcacgttggcaagtccgcgacggtgcttgtggttaaggacggcgtactcacggtcactactggtaagcagcagtgggtcgaggaggctccgtacttcgatggcagtggcaaggcgctagctctaggggcctatcatgcgagcaagtctgtggctaaggccatggctgctgcgatagctcacgatgtctacagctccgggcctatcgtcaagctaaaggcaccagttcgcgaggcttaggagtaaggccacgtgggtagccggaccaaaatttgcttcggaaatgcgcgggggtcactccaatagaagctcccgcgcgtgcccccgtacgccctcgcgttacgcgcctgcgggtgtgcgtgggtgcgtgcccgcgtgtgcgcctgtgtgcgcgtctgtgcgcccgcgtcaaggttccgcgtgggtgtacccgtgtgcctgcctgcgtgggcctgagcgtgcgtgtgcgtggccgtgcgtgggtgcctgcgggtgggcgtgcgggtgggcgtgcgcctgctgcctgtatggctggaccgcgctgccttggctgaatcgttaataaatctcttggcgaaaggtgttgacgtggccggtgcggtgtggttcaatggcgtcactggggcagcgacagggcttcaggagggccgcaaggggcttgacaggggctaccctacctgctaccatgcgaaccgcagctgtaggcgtgcgagggccatctgtatcgtttcggccttttggtacacctatagcacacagtcggctcaacctgaatcaccgtctatcggtactctgtcgagctgattagttagctacccgctaggccaacggttgacgcttgcgatgcaagcagtagtagacacacggccgcaatggtagtaagctgcaacgcaagtcgagtgacgtgatccgtagtggcgccgccaacaagtgggctaagggtacacgggagtcactggtaagggatgcgaggagctaccgaaccacgcttgacactaagctagcagttagctatgataggcggcaagtggtagccaccggaacagcggagcgacctagcggtaaggctagacgtgagagattacgggtgttgaggctgaggtgagaccgggacaccggtcaagacactaacaggagcgcacatggtcctctaacggatagcttgacaaggcggcacagatagccctttgaggccttgcaacacgtggaccaccgacgtacatggtgggatggtggcgacaggacgcccaacgggttagagacccgagcgagccaagggcttgacaggatgcaacaagggtgctagtatggcaccacgctctgaggagcagccacattggatggcgtaggactaccgctaacgggtagggtgtaacgggaagcgtgccaaccacagccaatagtggccgagagttgacgtggaccgccaagctgcaacgtagcactagcggataaccggatgaactgggatttcaaaggcccatagaatccaccagacttgcaacactggtgccgctttacctaagcctaacgcttagggcttcccatctgccgtgagagtcggccacgggaagtaacccactgccaaggtgggaagccggtcataaggaggtggtgagcctcctatcgcatggaatactgtgcgtttcgtgaaaaggctctacgggccacacggtgacaatggcactgctagccggagtagggttgacagcccgaagggctagcagattgatgcgccctccctttgcgatgaccatgcaggcaaatccggtggtcagtgtgcgcccacgataggcgatgcaacggctctaatcgagaatgagggattgaccgactcgacggctttctgagggcgcatcaatctgttagttttcccaccagtgccaatggaggcacaacatgcaaggctcgatcaatgccaatctcgaccgcacccagcgtaagcgccgcttctgccagttcacccggacggcaagcgtgatggacctgcgcaccacggagcatgaccgcaagcttgccgagcgcaagcgccaagccgagcgctacgaagcccgccacggaaccgccggaaagcgatctgtgtttgttgtcgagggtaacagcgggacgaaccgggcgaaccacgccgctgacaggagggcttacctgtgatccggttcaagttctctcgccactacgtggaagctgcccgcgattcctacaatcgggccatcatgaagcatccggccggctctgtgtcggcgctctacgtcctgccgtgcggtgggcgttcattcgacatccgactcgcttaaatgcaagctactgggccttcgcaagagggcctagtgtcgtgcaatcggcacggacccaacctgaagggaaccaccatggacatcatcaccggaagcgctgacatcaagcgcgccatcaagtcgatcaacaccgcccgcaccaagctggtggaccagattcagcaggccgcgattgcggtcatcaaccacgcacacatccacggcgacgttacgctcgcttccgatctgtgtctcgccgtgggcaacggcatgaagcatgaagccctgcgcctgtacctgtccgagttcggcccgatggctccgaacgacgacaaggaaaccaaggcgagcgcgcccatgaagtttgccaagagcaagcgagtcgagggcgaagctctggccgacgtgctggaacgtgccgccgcgaaggcgtggtacgacttcaagaccgagaagcccgcagaggcgttctcgttcgccgccgacctgcacaagctgctgggccgtctggaaaaggcgaccgaggaaggctacgtgccgaccgaggaggaacaggccgtcatcaacgctgcccgcgctgtgccgaagcccaccaagaagaaggagaacgtgtaacatggaacccaagatcaaccttcgagtgacccagcgcgaagcatccctgctgcgctcggcccttcacatcgcctgtgcactgaccgcaaaggcagacccgtactccaaccgcaagctgtccaatgagttcgccgtgctgcacggtgagctgcgcgacttcggtgtcgagagcttcgagcgtgacgccatcctgcaattcgaggacgacgtgattgcggcctgccgtgacagcgatgtcgaggcacagctgctgcgcgacctgatcgcaccgccgacgttcaccgtgggctacggcatgcgtgaacttgacttcgctgctatcgaggcgcgggtgatggcgtgcctgctgtctccgttgcctccggtggtgttggatgcctcgcagctggacttcctcggcagcgtgaccggccgcatggtgttgcccggcctggcaatgcccgacaacctgccgcgtaagctgccggatgtcctgatggacgaccagagcgcacgccacgtcgccctgactgcatcgcagaccgggctggtcaacaagacgaagaccaagggctggatcgtgcagttcaatctgcgccacggcagcatcgccctcgccaactgggcgcaggtgcgtgagctgggcctgccgcagcgcagccgcaatgctgcgtaccgcatgctgaaggcgcgggccaaggtgcagggcatcagcgaggatgcgtaccgtgtggtgcccgaaggcactcccgatggcccggagaaggatcgcggcttctacaccgccgagttcttcaccaagcatgcgcggcgccctcaccagctgggttggaatacgtccactgtgatcggactcagcggcacgttcaccactgcgcaggctgcacgcaacgccatcgcctcgcacgtcggcaacgatccgaaccgtctccgccgctaccgcgtgaagtggcacccgagccgcgcgtgatctaccgctgcgccttctaacgagggcgtagctttggaaccacgcccaacaggagggcacattgcatgatccccgtaacttacaagcgcatccgtagtggggagcgcaagccgatccagctgtgcgagcagccgcgccagtggaaagagttcgtgacccatgagcacagcgtggagcgctggtatgcgtgaggtcagcctgcgccttgtggtgaaggcgctgccgctcgttaccgtgaagggtgtggctgtcggggattacatcctcggcggacatcacaccagccacgaggcgtgcgagcaagccatcgaacaccaccgcaagcaccacgagaaggtgcccaccctctactcgatagaggaaatcgaaatcccacccgtcaatcaggagaaccaccatgcgtaaggtatacttcatcgtctcgatccccaagaacagcaacgatggcgtcatcactggcgtcgtcgccaatggcaccggccgcaccccgacccaagaggaactggatgcggtgatcgccgagctgcgcaccaagggtgccaccaccagcctgctggactcgctgcgtgacggcacgtacccgaaccagctcgccatcttcgaccgccgcgccgccgtgcgtgccgaggcggatgtgctcaacagctacggcgggtcgttcttcaactggcacatcctcgaagtgggcgagagcatccgcaagccggtgcgcaagccgctgggttggcgtatcacctacgccttcgccgaagaccgcagcgactccgatgtcagctgctacaaccagcacccgagcgccaccgtgcgcatcgacggcaacgagtacaacaagagcgagtacaacgtgctgttcccgacccgcgatgcagcgcgcgccgtgttcaatgccgagtcgctgggcggcgagaacatgggctaccgtgtcgagccgtactatgcgtaagctctggctgcgcatcctgatcctgctgtactggatcgtgggtcgtggcccgtgggttgtcgtcggccagtaccatgacgacgacggcaagctgtgccggttccgcaccggcccggcttccactgggttctcgctgacgttcgatgacctcggcgcagccaacgactactgcgaccagcgcaactggaaggcagacactgacccgctcggcaccacgtactacgtgtggcatgagttggagttcaatcacttcggaacgaggaggaagtaaccatgggtttcatggacaagatcaaggctgcggccaagtacgtcaaggacaaggtggtcgcagcggtgaagccgcgccacgatgacgacgacacgccgccgcctgcgccggacaccagccggcacctgcacgtcagcgtgccgctgattcccatcgacaacccgatcctgcgcaagatgctggggcaggactacttccccgtgcagaaggggcagggtcagacccgcatcgtcggcaacaaccagctgaagcgcgtggccgatagcctcggcgggaacaacaagcagcgtcgcaagctgcgctcccgcatgaagcgtcgtgctgccgagctgcgttccggtgcatcgttgcagcccaacgtgcagtccgcactggcaggtgcagcatgagcctgcgcatgggaagctgggtcgaggtgactgtgcccgacagccgactgctcaacgtgcagccggagattgccgccgccgtgaagctgatcggcggtgcgaccatgaccaatggccgtggcctgtacgtccgcaaggacaccggcgcactggacgacgaggcggtgaccgtgatccgcttcgacctgaacttgcacagcgagctggtggaccagtacatgagcgccatccgcgccatcgtggaccgtctgctggtgctgggtgaggagagcgtgctgcgtcgccgcttctacaatggcggcggtgggtacaacagcgagctgatctttcagtaacccgagccgggtaggctacgactggcccacgtacgggccatcctatcaaccgtcaagaggaaccatctacatgtcgaacgaaaacaccaccgagcagaccaccgtcagccactacgaagccaagcgcgccgagctgctggaagacatcgccaaggcgcaggccaaggtcgatggcctgaacgagaagctcgccaagctggatgccgtcgaggccaacagcgccgccatcgaagcgctgaaggcgggcgacgccgtgtcctacctgttcggtcgtgccctgaacaagcgcgtcctgtccggcgtgatcgtcgccaccggcaagaacgacaagggcgtgctgcaactgaaggtgcagaccggcgaaggtctggatgccgagctgaacctgatcgacagcagcgccctgctgatgtcggccgaggaagtgctgaaggcgcaggaagaaatcgacgccgccgttgccgaggcccagcgcctcgccgccgaagccgctgccgccaaggctgcgggtggcgaaggcgggcagtcgtgagcctcgccccgccgtcacccagcgtggccgtcgtcaagcgtggcgacgagctgaagcccggccagaatgcgtacctgatcgacacgcggcagaccaacaagctgccgaagggcaccgggttcgtcgtgtccaagctgaccagtgaagacggctcccgtctgatcgtcagcacggacggcaacggctccgtcctgtacgccaccagccacgacatcttcgaggtctgggaataaccaagcgaggatagcatgagcgatacccttcccgacaacgactggctaccacatgccgagcgcctgcctgttggtggccgcacacgtgtggcccatgagtgcggggagggtacgcccttgcttatctcacgagagcacgacaagtccaccgcattctgtttcaggtgcggtggcacaggattcaagcgtgagcacgagagtatcgaggccaagcttgcacgaatccacgccgagcagacgagcgaacgcagagtgcgtgcgactgttgagttgccagagccacgggtatacgacacccgcgagtggccgctcgacgctaaggtgtggttcttcaagatgggactctcgcttcagatgatcgagaagctgcggctgtactggtgcccaagcatcgggcgggtggtactaccgatcactgaaggcgacaacgtggtatactggacagcccggtcggcaacgagacagccgaagtggctaacacctgacgttccgaaagacggacttgtcgcacgctacggcgtgggcacaggtgacaccatcgtactgtgcgaagacccgctcagtgcatacaaggtgggactggtaaccgaagcgtggtcgttgctcggcaccaagctgcacaacaaagtgttgaagcagctgactgatcgaggccaacgtgtagcgacgtggctcgatgacgacagaggtagaagcaacggtagcaatcccggccaagacagtgcgcgagtaatcgctgcgcgtctacgtgcgtttggtctggactacaggaacatcacgtcaccacgtgacccgaagtattacacgaccgactacatcaaggagaagctgcaatgagcaaacccatcgtgcgctaccggcgcgctatcatcccgcccgtcgttggcttccgtgccacgctcggcggcgtgcttgcgcatccgaacctcggcgactgcgacatcgtgcacacctcgacggtgctgtatgtggcggacggcgggcgcaagttcgagacgcgcaacacccggtatcaccagctcgattccaagtacgaacccgaaggagaacctgatgagtcttgacaccacgctgctgcggttgtgcaccaaccgtggcaagttcgaccggctggtacccagcgcaccacgtgatgggctggacgagctgaccgtgctgatgctcgatgcgttgcgtgcgtactacaaggagttcccggacacgaaggacttgccgttcgatgtgttcgatggctgggccatggagttcaagtggaagacgcagcccgacgacaagaagtccctgctcaaagttctgctgaagcagatgcgcgagccggtcccgcccgaggcagagcagggcatgatcgagaagctgttggagttggagcttgccaccattgcggtcagcaagatcgtgcagtggaatggcggcgctgagttcagcctgcgcgacgagctgtacggcttggccgagacgatcaccgaccgaatggatcgcaaggcgcggctcccgctggtgcaggagacgcccgaggaactgatgcagatggacgagcacgacatcggcatccacttccgactgcccacgttggcgaagaacctgcgcgctctgcgtggtggtgacttcggcatctacgccatgcgtcccgacgcaggcaagaccacgttcctgaccagcgagtccagccactggatcacgcagctcgacaacgtttggccggaccagaagcgcaccggcatctggctcaacaacgaggggccgggcaagcgcatcaagcagcggtggtatcagtcgctgctcggcgctaccatccctgagatggtggagtgggcgaaggatggtagcatccgcaagcgcatcgaagatgcgatgggcggggacatccaccgcatgcagttctacgacatccacgggttcaactccggtgaagtcgaggccatcatcaagcagaccaaccccggcttcatcatcttcgacatgatcgacaacatcacgttcaccggtggcatgaccaacggcgggcagcgtaccgatcagatgttggaggcgatgtatcaggccgctcgcaactggtgtgtgaagtacgacgccgtgggcgtggcgacttcgcagatcagcgccgagggtgagggaatccagtacccgccgcagtccgcactgaaggacagcaagaccggcaagcagggtgcgtgcgacttcatcatcatgggcggcaagctcaatgacccagcgatggaacgcttccgctacatcggcaccccgaagaacaagctgcaccgcgcaggcggcaagcgtgacgttcgggaagaagtgatgatggatgcagagcgtgcccgcttctatcaggaggcagcatgagcaagccaattcacatcgtagccaccgggttcacggtgtcggtcagcttccccggtgaatccaccgaggcgaagaccttcaactgcgtgagcaacgcgcaagcaatccaccttgccaagctgctgcgcaaggtgcacgacgcaggctacatcgaaggccgcaacgacgcgccgcagtggaagtggggatggctgcggaacaaacacagcacttggatcggcgtgcactactcgccgcacaacaagcgctggtgcatcaatctgatcccgtgcttcacgttctggatcaccaagcccggaggtaacacaccgtgagtaccgaaccgaacatctacctgccgcgcaacgtgggcgtcatcacgtccagccgcaccggcagcagctacacagtcgagccgcccgtgaccgacacggacatcgacttcctcgtgctggtgcaggacttccacgaggccatcgaaaagctggtcgatcagggatggaccctgtgctccggtgccgatggacactacgaggaggacgaggactacagcaccacgtggtatgcgctgcgcaacggcgtgttcaacgtcatggtgaccgccgactccggctggtatcagcgcgcggtcgaggccaccaccatctgcaagcgccgcaacatcaaggacaagcaggaccgcatcatcgtgttccgttgggtgcgcgacgggctggacttggatggcgatgcgtcggatgaaatgtaccagctggccctgcaacggtggccgctgtgagcttcacttccttcgacctcgaaaccacgatccgttccatcctgaagcgcaaggccaatccgttctacgacatgaacaagatcgtggcgattggctacaagcggaagggtgacgcacggaacaccggcctgtactacgacacccgagtcgggatagacaaccagtacatgggcggcgcacccgatgggtggctgcgtgagctgtgttacgggcagcagttcctcgtcgggttcaacatcaagttcgacatcctgcacgccatctgccaaggcccactcaaccggcaggcatggatcgagttcatcgacggcggcggcatggtgtgggactgccagcttgcggagtacctgctgcacggcatgacgcaagagttccacatggcgagcatggacgagacggctccacgctacggcggcaacttgaaggacgatgcagtcaagtccctgtgggctgcgggcgtggacacctgcgacatcgacaagacgctgctgatggattacctcctcggcaccaacgacaccgacgacgtgggcgacatcggtaacaccgagaagatgttcctcggacagctcgccgccttccgtgcacgtggtggtctgcgctcggcgctcctcaacatgggtgcgctgtgcttcaccatcgaagccgagtacaacggcatgtacgtggacaaggactgggcgcttacgaaggcgaaggagttggaggtcgagcttgcaacggcgaccgccgaactcaacggcttcatccccgagctgcccgagggcctgaccttcaactggaacagccgcttccacaagagcgcgctgatcttcggcggcaaggtgaagtacacggccaaggttccgatcatgtccaccgagggtgggccgacttacgtgcagaaggacgaggtgcactacgtgctggtcgatggtaccacgacggcgacgccaccggccgaggacttcgacaacctctggcgctacaccacgtacggcagcggcaagaacaagggagagtacaagaccaagaaggtgaaggtcgatgacttgaccaagcagaagttccgcaacgaggacatgctgttcgagttccctggctacaccgagcctgatgctgcatgggaaagcaagagcgatcccggcgtgtactccaccgctgccgacgtgatcgaggcgctgggctaccgcaacctgccgttcaccaaggcgcttgccagacgcgacgacatccacaaggacttgtccacgtactacatcacgacggacgagaagaccggagagcagaagggcatgctcacgctggtgggaccggacggcatcatccaccacaagctcaacatgaccaacacggttaccggccgcttgtcttccagcgatccgaacttgcagaacgtgagcaagggcgagctggacgaggagacgttggaggagaagggttcgcagatcaagcgcgccttcgtgtcccggcaccggggtggcaagatcatccagtcggactacacctccctcgaaatctacgtgcaggcaatcctcaccgagtgccgtcagctgatcgaggacttgaagcagggcctcgacatgcactgcctccgtgcagagcaggcgtggggtgagcaaggcaagtacgactacgacttcatcctgaaggcgagcaaggacgacaagcatcccgagcacaagaagtggaagaagaagcgcagcaacgcgaaggtgttctccttccagcgtgcgtacggtgcgggcgtggcgaagatcgctgcgaccaccggcatgtcggaggaagaagtcgaggcgctggtgcgcggtgaggccgagcgttacccggagctgggcgagtacatcgaccgcatggtcgagcacatcaagcgcaaccgcgtcagcactcagcgcttcgttccgcatcccaacgcggggcagcaaggcgtgccgcatgggctgacgtgtcagcttggccggtcgcactggaccacgccggacggcaagatgtattccttcagcgagtcaccgtccccggtgttcatcgccaacaagcccgcgagcaagggtggctgtgcgcagtcgttctcgcccacggaaatcaagaactacccgatgcaaggcaccggtggtgaatgggccaaggcggcgatgtacgtcagcctgcgcgccttctaccggaagtacgtgaccgaaccgaaggaatggttgggccgtgcgttgctcgtgaatcaggtgcacgatgccgtctacgtggatgcacacggcgacatcgcaaccaaggccgctgctctgctgcacgcctcgatgctggaagcgtcggtgtatatggagtggtggttcaactggacgctgccgcttggcgtcccgtgtgaaaccaagatgggcgacaacatgatggaggagaagaaccctcccgcagagttcgccggtctggtcatcgagtaccgcgcgtcgatccgcaaggacttcgtaggtaatcacaacccgtcgtttgaataaggagaacaacacgcatgagtcttgacgcactgttgaacaaggtcgccacgcagggtaaggatcagtcggtcgccagtggtggcagcttcgactacaccccgcccgctgccggtgtgaccaccgcccgcatcgtcgggtactacgagctgggcaagcacgagttcgagttcgagggcaagaagaagacgcaggatgaagtcgccatcgtgttcgagctgaccggtaagcagcacccgcacatcgaaaccgacaatggtccggtgccggtgcgcatgacgctgaccctcggcctgtccaccaacgagaaggcgcactacttcaaaatcttcagccgcctgcgcaccgaggagcgccacttcgtgcagctgctgggtcagggtgtgctgctggaagtcatccacaagccgggcaagcgcgacccgaacaagaccttcgccgaaatcgacaaggcttccatccgcaagccggtcatgccggtgccggaaatggagaacggcatcccgaccggcaagttcgtggacaccgtgatcccggtgccgcagcagatcaccccgctgggtgcgttcgtgtgggacttcgccgacgccgacatgtgggacagcatctacatccccggcgagtacccggagcgcaaggacgagaagaccggcaaggtcacccacgaggcgcagtcgaagaacaagacgcagctgcgcatcgctgcggcgctgaacttcaagggtcttccgtgctacgactacgccgccgccaagttggcgggcagcaccacggtcaccaaggaaggcgtcgatgcgctggacgaagtggtcggcgacgtggcgaacgccgcgcccaccgacgctgctccggccgacgacaagccgccgttcccggtggacggtagcgacccgatggcaggcatcgcctgatggacctgagcgctctcatggcagcggccggtgagcgctccccgatgccggtgcaggtggtacgtcagcacaacccgcgcgtgatcgctcacgttgatggggactacatggcgtacttcgcggctggtagcgagaactgctcggcgggggatgcacgacgcaacgtgctctcccgctgcgcacagctgaagcatgtcagcggagcgggcaagatcgtcatgcacctgacgcacgccgcgtctaccaagggtgatcgcttcctcgctgctaccacgcagccgtatcagggtcagcgccaagcaggccgcaagcccaacaactgggcgttccttcgtgagtggatggagacatacgagggcgacgctttcactcccaaaatctggctgacccgtgaggccgacgatggcatcgcgtacgtcaacgagggtgcagcattgcaccacaacatcctgcacgtggtgcacagcgccgacaaggacatgcgaatgttctgcggcgtgcacgtagactgggacggctacgacatcacagaggttccgctcggcgcttacgacatcgttggcgagaacggattgcagtacggtcacaagtggttctggatgcagatgctccacggcgacaccgccgacaacataccgggtctgccgaaggtgggcaaggtgacagcggagcagctgctgttcgagacgaagaccaacctcgaagcggtgcagatcgtgagcggcaagtacagcgaagtgttgggtgccgactggcgcaagacattcgccgagcaagccgtgctgctgtggatgcggacggatcgtgacgcagaactgctcgacgtgctgaagctcgacgtgttcgggccgaagctgaagcaggcgttctatgacctcgccgaggacgtgaacgagaagcgtgcaatcttggaggcatacaaagcatgaagcgactcactgcaacacaggtcaagctgctgcgcatcaagctcgcagcggagcaaggcaaccggtgctgtctctgtcagggacagttcggcctgaaggctccgctcgatccggtgctggaccatgaccacaagaccggcgctgtgcgcggggtgctccatcgcggatgcaactccctgctcggcaaggtcgagaacaacgcaggccggtacggcgtgcgcgacgtgttcgcattctgtgcgggcatccccaactacctgcggtcgcacctcaccaacatcacggggtacctgcatcctacctacaagaccgacgacgagaagcgtatcgctcgcaatgcgaaagcgcgaaagcgtcgggctatcaacaaggagacaccgtgacccttacccagttcattcgccgagcaccgaagcgcggcccgaagattctctgcctcgacatcgagacgttccccatcgagttctatggctggggcatgttcaacaacaacttcagcgtcaagcagatcaagcgtgactggtcgctgatgtcgttcgcttgcgaatggctggacgacgaggcgtcgttctacatggaccagcgcaacgtgcgcgacgtgttcgatgatcgcaagcagggcaaggcgctgtgggcactgctcaacgccgccgacttcgtgctcgctcgcaacggcaagaagttcgaccttcgcaagatcaaggctcgcctcgcaatcctcggcctgccgcccgtgtctccggtgcaggtgatcgacccgatgctgctgaaccgcaccgagttcgccttcacctcgcagaagttggagtacaccaccggcgtgatcgtgccggagctgcgcaagtacgaccaccacaacttccccggcttcgacctgtgggtggcctgcatgcagagcctgcccggagcatgggacgagtgcgaagcgtacaaccgcatcgacgtgaagtccatgaagttggagtacaagaagctgcgcggttggtactcgcagcatccgaacgtcgcagtgtactacaaggccgacggcagcgagcaccgctgcaacaagtgcggctgcaacgaaatgatcccgcaggatgatccggcccgcacgcaggtcggtacctacctcctgcttcagtgcaccgtgtgcgacggctacagccgtgggcgcaagctcacgaccagcgccgaggcgcgcaagcacatcaccgtcccggcataaggaaccgacatgaagatcaccgacatccgcagcggcatgcgggtacagtacatcggcaatgcgcccgcaatgatcgggctgcgtggacaggtaagccgcgtgttcgctcgtgatgtcgaggtcttcttcgacggtcgagttaagccgagctgctgcgttcccgattccctccgacagcttctcagcatcggaggcgtgaccaccaccagacgagaggtaccaatgcccgaactgagctaccgcgacgaggaccgtcgcacactgtccgaccgtggcgtcggcctgaaggatgacgggggcaagccgcaggcccgtctgctgcatgagggcgtgccgcgtgcactggcccgagtcatcgacaccctgaccttcggcgcgcagaagtacaaagcgcactcgtggcagcatgtcgagaaggcgctcgaacggtatcaggacgcgagctaccgacacgacaacaagcgctgcctcggcgagaagctggacccggagacgggcatccaccaccgggcgcaccacatcatcaacgagctgttcctgttggagctggaactgcgcgaggaggagaaggccagtggcgcagagtaaggcgcgctccatcaaagaggcttgggtgaacatcggcatcggctacagcatcaactacgcagcgaacatcgcgctgcttccggtgctgtggcatcccgagcatccgctgctgtcggcgcacgccatcggcattgcgttcacagcgatcagcttcatccgccagtacatcatccgccgctggttcagcaagggtgactgatggcctgcgcccgctgcggccaagtgcatcggtacgtcccacatgaggccgagtgggcgcgcttcctagaggagcaccgtacccgcaagcagttcgatgtcgagtgggccaactcactctggcatcgtacataccctgacgacgcattctgcatcctcgtgatgaggggcctcgcaggtttcgttccattcccgtcgaaggagaactgaatgctctacaagaaccagaccgccatgctcatcaagtcctacgagaacgccgttgcgtggggcgagagtgccgaccacgaggaggcattgcagaatgcggtcaaggccgggttcccgaacctgcccgacgaagatcaggccgagctgtatacccgcatcgccgatgcgtgggaaggctaccgtggttcgctcgctccgcgcaagctgtggatcggcaccatcgtcaaccagttcatgtcgtcccgcatcgcacggttcaacgccgcgctgggtgacggcaccaagaaggaggacagcgccgatgtttgatgtgcctcgccagaatgtccgggttgctcccggctacaagaagcgcaagcgcggcttcaagatcaaccgcgccttcaccaagggcaacttccgcgtgcagtggtacgacggcaaggccacgtactgggagcgctacgttccgtggtacgaagtgccgctcgccatgttccagatttggagggactacgcatgagctacatcgtccacaaggcagtcgagcaggacaagatcaagaagaagctgcggcccaccgaggagcagcttcgcaccgagtacatcgcacagccgaagtacgacggctgcaacatggtcgccatcaagcgcggccactgggtgcccacggtgaacaagggcctgcatgccatcaaggtgggcgacgtgcagatgcagccggtggatcgtggcgtggttgacctgttctcccgcaccggtgagcaggtcgtcagcgcacaccacatcgagaacgctctcgcatccgcgccgttcttcccggtcggcgtgtacttcggcgaatactggcacccgcagatcgaccagcccaccgtcagcggcatgttccgcaagaaggacggcacgcagtacaccgagccgatgttcgtggtgttcgacttcgtgacgctggaagaatgggagcagggtttcagcgacctcgtgtatcaggagcgcgtcagccgcctgccgagcatgggccacgccatcgccgagggcaccgcgccggtgttctacgccgagtcgcagggcttcctgatcgaccaagagctgggcagcatggaagcggcgaagctgctgtgcgagggcggcgcgtacgacgggctgatcctgcgcaagccgagcggcaagtgggtgaagggcgacaagggaaccaacggcgaagtcgtcaagatcaagccgaccctgacgctggacctgcgtgtgctcggcatcaacgaagcagtcggcgagaagaccggccgcgccgtgtacacggtcgtcgttgacctcggagaaggcaagacgcaggaggttggcagcggcgtgccgcacagcgagagcgagctgcctagcgtgggaggcatcgtggaaatcgaggcgatgtccttcagcaagtacggcctgctgcgcgagccgcgatacaagggcatccgtcacgacaagaaggaggcagacctgtgagcgtcgaggtgcaagcatggcacaacatggagcgcgacacggtggagctgcgcatcagcgttcctttcggcgagtacgccggttccctgtggccgaacgagacgctgcgcgacaaggtgcaggaagcgttcgccaagttccttgacgagcggaggggctgatggacgcgatcactttcgagaagccggagctggacttcagccagtcctcggcatggatgggccgcgtcgaggtttcggtgcgcgcccggtacggtgccgacttgttcggcgctgctgccacgtgcatggccgaggatatcggcggtgaggcgtggccgcacatcatccacgacctgcacatggaaatcatgcgcggtatcctgaaacgctacccgccgcgcgactacaccgtgcggcagcaacggaggtaacaatgctctcgcaagtggaactcgaactggaaacctacgccttcggtaaggagcgcatggagaagtccatcgcccgcaacgaggagaagggcggcgcggacaacaacccctacgcccaagcagtgtatcgccggttcgtgcttccgcttgcggagcgcatccgtgcggacatcgactctccgcgaatcggccgtgcgcaagcgcacgtgccacttctgcgcgccaagtacgatcccgagcgtcagaacaagcgtggacagcccgtcagcgccgaggaacaggcacgcgagtggtacgaggctgtggccttcgtcgccgttcgcggtgcccttacctcctgcatgcgagacaagcacggcgaaggcagcgaccgcgacgtgttgaagaacgttggcatcaacgtgtaccatgagtacctgctgacgcagttcgccgacgcggagccgactctgttctaccacctgatgaacgacatggaccgcaagctctctgtcaacgagaaccaccgcatgacggtgatgaagatgcaaggacgcaagaacggcatcgagttcgtggagtggggacaggcacagcgcgatcaggtcggcgcgtacctgtgcgatcagcttgcgcagctgggcatgttggagattggcgtggtcaccgagactgctgccagtgcaggcgcagcgtaccgcaagttccagaccaagacgcacgtcaagatcgtgctgaccgacgaggtgcgcaagctgattactcagatcagcgacttcgtgatcgaggccacgccgttctacctgccgtgcgtcgagccgccgatggactgggtggacatcgacaacggtggattccacacgaaggaaatgcgccgactcaatccgtggatggtgaagacctacgctcagacccgcgacgagtaccgcgctgccgagctgcgcaacgagatggctgcgatcaacgcattgcagcgcgtgccgtggcgcatcaacaagcgactgatggaagctgtgtcggccatcgccaaggtgcacgacatggaggaaatcatttctcagggcgagctgccgaagccgcgcaagccggagtggctgacgaaggacatgaccaaggaaaccatgtcccacaatcaggagttggagttcaagcagtggaagcgcgacatgtccaactggcacaccgacgagcgcctgcgacagaacaagggcaatcgtttctacaacgcaatgaaggtggcgcgcaagttcgccgagtacccgagcatctacttcgtgtacttcgctgacttccgtggccgcaagtacgttcagaccaccggcgtgtcgccgcagggttcggacttgcagaaggcgctcttggagttcgccgatggcaagccgctgctgactaaggacgcgaaggattggttctgcatcacaggagcaaaccgatggggatacgacaaggcgtctctgccggatcgtgtgaagtgggtagcggagcatcacgaccagatcatggcgttcgctgcggacccggtgaacaacgacgagtggaagaccgccgacaagccgctgcaatttctgagctggtgcatggagtacgagcagtggcaagtgttcggggatcgcttcctgagccgcatcgcagtcggcatggacggttcgtgcaatgggcttcagaacttctcggcgatgctgcgcgacgcagcaggcggcgtggcgacgaacctgatcccagcaccgctgccgaatgacatctaccagatggtggcagaccgcgtgactgccgtcctgctaggcgaggacgaggatgccgaagggtaccgcacgctgtggctcgaccacggcctcacacgctcgctggtgaagcgcagcgtgatgaccctgccgtacggctcgcggcagtcctcgtgggcggacttcatcatcgaagactacctgaagtgtgggaagttcccctcgctcgacaaggccctgtacggccccgcagcgcgcttcctgagcaagcgcatgggtgaggccatcgccgacaccgtggtcgccgcagcgggcgcgatggagtggttgcagcgcggctccgggtcgatcctcaaccaagggtacgaccgcatccggtggatcacgccgtccgggttcccggtggtgcaggtctactgggagtccgaggagcaccgcatcaacaccaagctgtgcggcaacgccaagctgtccctgcgcaagagcacggacgcggtgaagaagtcccggcaccgcaacggcatcgccccgaacttcgtgcacagcctcgacgcaagccacctgacgctggtggtcaacgcggccaaggccgaaggcatcgacgccttcgccatgattcacgacgacttcggcacccacgccgccgacagcgcggcactgtaccggatcatccgggaggtgttcgtgtcgatgtacgagcggcacgacgtgctgtcggccttccactcggcctacccgttcctgccggagccgccgccgatgggcgagctggaccttcggcaagtccttgattctccgtacttcttcagctgacggagtttcagtacacctatagcacgaggcaactgaggtccggttggagcggccgcgaaggtaagcggaaccggtgccggaccttttggtacacctatagcacagaggagacaccatggccgaagacgccaaagtgaaagtcctgatgacgctccacccgaaccagctggccgccgtgcggaagctgtccgggctgtcgctgtccgtcaactcgaataccacgcccttggaggcaggtatgcagttggggatggcccgcgtcctgaacatcttacaggagggtttcaccgttgattcctccgtaccgaacaccaacgacgggtgatagtgagcagatcaaggcggctttaacggccgctttgtatctgtcatctagagaagatagtaaggtagacaacagagaatcttctgtgagctacaactgtgatgaccctgattacacagtggccctgataacacagggtctagtggatgcagtaatcattgatgaagcctacctgctgtgctttgccattgtcacaccgtggtactccaagaaccgtactacgttcgttgagaacatggtgctgcgaattgggccgggcagttccttcgaccggtacatagccgtgatggaacatctggctgacatcaaccactgcgactcactgagcgcaggcggtgcactagctcggaactcccgagcactcacacggatgtatgcacgctacggctacctgctggaacggcatgctccccaattcaccaagcgaaggagttaacctatgggtagcatcgttggtggtgggtccgccaagcgagcagcgctgaagcaagctgctgctatcgacaagcagaccaacctccaaactcaatccacgaactaccagattcaggcgatggccgatcagatggcacaggcagctgcacagcaggccgcatctgagtacgccgagaagttgctgagtgcccccgtcgataccgtcgatgtgcggctgggaacttccgacctcgacttgcagactgccgacctgatcggccgacgcaagaccgcccgctccacttacacccgacccgtgaccacgaccgcagcttcccggctgacgaccgtggccgggtcagacctgttgtgaggtgagcatggaccatccgatccaaaccgctcaccgccagttcgaggcttacgacaacaagcgacagggcatcatgtaccgactcgaacgctattcgagctggaccgtgcccaagctgttccctcgcaagaaccgcgatcaggacaccgagccgctgacccacgggttccagtctctcggcgcgcaggcagtgaaccatctggcgaacaagctgatgatgtcgctgttcgcaccgtcccgcccgttcttccggttggagctgaagcgcaaggcgaagcaggctgcgcaggagcaaggcgctgacttgcaggccatgcaggcgatgcttgcgaaggccgagcaggatgccagtctcgaactggacaagcgctccatccgctcccggctgtacgacctgctgaagatgctgatcgtgctgggcaacgccctcatggtgttggagaaggacacgatccgcgtgctcaacatgcggcactacgtggtcaagcgcacccgcaccggcgaggtctacgaactgatccttcgggagaaggtgcacaagacccagctggaacccgcagcgctcgctgccattgtcgcgcacccggacttcaagcccgatgacgacggcatggtgtgggagtacaagtgggtcaagctggaccacaagaccggcaagtacaacgaagacgtgtggatttgcaactgcaagctgcccgccaacttctcctcgacctacaccgcagacaagctgccctaccgggcggttagctgggacttggccgcaggcgatgactacggctccggcttggtcgaagactacgaggccgacttccagtcgctctcgatgctgtccgaggccgcagtgcagggcgcgatcctcgcctccgagttccggtggctggttaaccccgcaggtcagacctccgtcgaggacttcatggcgtcgcccaatggcgcggccattcccggcatgaagggtgacatcgagctgattaacgcaggcgtcgatggcgtgctgcaaaccaaccaagcaatccagtccacctacatcaaccgcatcggcgcaggcttcctgttgcagacggcggtgactcgtcaggcggaacgtgtgaccgcgcaggaaatccgcatggtcgccgaagaactggaaggcgggctgggtggcggctactcccggatcgctgcggacgtgcaggtaccagtcgccttttgggtgatgaacctgacgggccgcgacatccgaggcaaggacttggagcctgtcatcatcaccggcttggccgcgctctcccgtacgggtgaccgtgaccggctgttggagttcggcagcaacctcgccaacgtcctcgcactgccgccgcagattctcgaacgactgaagctgtccgcgtggatcgcagacctcgccgccgctggtggcttggacccgaacgtctacgtgctgactgaggccgagtacggccagatgatgcagcagcgtgcacagcagcagctcgccatgcagaacgcatcccagcagatcgacaacgccaacaacatggagacacagacacaatgagttccaacgcacctccgggcggtggtcccggcgcaaccgtgatcgcaacctcgaacggcaaccagcccgcaccggcagctccggctcccgcagacgacaagctgttgcccaacggccagcccgctccggccgcaccggcacagcccgcagctcctgctgcacctccggctgctgacgcgctgagtctcgaacctgccgctcccgcacagcccgccgccccggcgaacgctgcgccgactgcggtgtcgatcccggactacggcgacaacggcctgaacatcgcggccgaatacttcgtcaacaccgtgggcctcgacatcgacagccgcgaactgaccgaagcagcgaagggcaacttcgccctgctggaagccaagctggaagtcctcggcgacaaggccaagggttccgcaccgatcctcgctctggcgaaggagagcatcgctcgtgtcaccgccgctgcaaccgcagcgcacgccgcgaacgttgctgctgtccacgaagccgtgggtggcgcagagaactgggctgcgatccagcagttcgcacgggccaacctgcccgccgaccaactgaagcaggcaagcgaatcgctgtcggctggtggcttcggcgctcaggcgaccgcgcgttacctgatggctctggcacaggccaatcccgcgacgaccgtcaagggcgcaccggctaccaacgccgccgcccccgccgcgtcgatcaacggcgtcgctcctatcacgaaggagcagtaccgcgctgagtaccgcaagctggttgccgagaagggcatccgtggtgcggcccactccgaagaactgcgtgcactcaacgcgcgcgtcatccactaagaccaaggagcaacacaaagcatgagcaccatcttcccgactgtcccggttctgccgaatcaggtcaaccagtccggcaacgagaacgccctgatcctcgaacagttcaccggcgatgtcgagcacacctacgtgtccagctcggtgctggaaaagttcttcccgcgcaagcaggtcaagggcaccaacaccctgaccaagaaggccatcggccgtaccaagcttcagaagctgaagcgcggtgacgcgccggacggcaccccggtggacttcagcaaggcgtcggtgaccgtcgataccatgctgctgtcgcgtcacagcatctggcagctggacgaaatcttcaccgacatcgacacccgcaaggaaatcgccatcgagcagggtcaggaaatcgccgagttcgtggacctgaccatcagcatcgccgccgcgaaggccgctgctgccacgcagtcgatcttcacccgcaacggccgcgcgcccgagggccacttcggtgccacgcaggtcgtgctgtccgccgctggtgacgagaacgatccggccaaggtgtacgccgccatcggcaaactgttctcccgcatggaggaggagaagaaggtcaagccgcagcgcgatggcgtggtcctgatcgtgcgcccggcgatcttctacctgttgcagcaggccgagcagatcagcaacggcgagtacctgacctcggacggcaacaagctgaccggcatcccgaccttccacggctggggcgtcccggtgctgtcgagcgagaacctgccgaacaccgtgatcgaaggtcacctgctgtcgaacgacgacaacgacgacttctacgacggcgacttcagcaccctgatcgccgtggccgtgtcgccgaaggccctgctgatcgccgaagcgctgccgttgcagtcctcggtgtggtggagcgatgcctcgaagtgctacttcgtggactcgtggatgtccttcgccgttggtctggatcgcgtcgagaacgcgggccgcatcgacaaggttgcctaatccgctgggcgcggtccctgaatccttcgggtaactcaaaccgcgcccttcttccaccaacacaggagcaacatcatggtctttgaccgaccgttcgagatttccaaccgcgtcgtcgccgcaactggcgtggccggtctgcccgccaactccgttggtaccgtcgtcggcgtccactacgacacccgtggcaccgcaggctgggtcgtccgtgtccgtttcgtggacgacgaaatcggctcgcaggacatcgagtacgcaccggccgctctggctctggctgcggactaagcaacatcccggcaggggcgctccggcgtctctgccttgttcctctcaggagacaccatggcattcatcaccaagctcgacatcgtgaacgcctgcttgaagacgatgggcgagacgaagctcaacacgctggaagatgaccacgtatacaaggacgacgccgttgacttgatcgaccgcgtgcaccgtgacgtgtcctcactctcgctgtggttcaacaccgaatgggtggagctgaagccgcaggcaacgagcaagtacatcatggtccccacggacgtgctgaagctggactgcaacccgagccggttcggccacgtggtgcagcgcggacgccgactgtacgaccgcaagcgcaacacctacgagttcgaccacaacgtgcaggccaagctggtgcggctgctggacttcgatgacctcccctacgaggtgcagatgttcgtgcgcgacgactcggtgctgcggttccagtctgacttcgacggcgacaacaccaagtacgccaagatcaagcagcagcgcgatgacagttacatcaacttgaaggccgagcacatccgccagatcaaggcgaacccgctgttcgctcgcgcatccgtggacgtgctgcgttcccgttactggaactacagcggtcacccgtggcacagccacgtcacattccccggctaaggagacaacatggcaaaggcaggcggaacctatcccgacatccttcagggtgtcagtcagaaaccggcgcatcgtcgtcggccgggacagacgcacgagcagatcaacgtgctgtccgatccggtgaacggcctcgtgcgccgtcgtggtacgcggttcgctgcttcccaagccgttgtcacctcggccgagctgcgcaacatggacgtgttcgacttcatgcaggagggcaaggagtacgcgctgctgtaccggcgcgacgcctcgaccttgggcagcgagtccttcgcgttcctctacaacaagacggacgagtcgttcatccctctggtgtacgagaacagcacgtgggtcaacacgctggtcagcggaggcgcatcgtcgctcacggccatcggcagctacgtctacatcgcgggcaacaccacgatcccctcggccaccagcacgaacgtgtggcaggagcagacgaacatccagcgcctcgcagcatgggtgcgcaccgggaagtacaacaccacgtacacggtgaacctgacgcggacggacaacacggtgctgacggtaacgttcaagacggttaccgcatcgtaccccggaacgctcgacaccagcgacatcccgttctaccttcccggtggcacggagccggacgcggcgtaccagaagtacgtcaacgaccgagtgaacgagtacaactctgcggtcaacgagtggatcgtgacgagcgctgagcagacgcgcccggagtacatcgcggagcagctgtcggatttgctggtcgatgcaggcgtgtcggcaacgtacatcaagggcgggatcatcattgacgatgaccagttcaaggacatcacggttgacgacgagggagacggcacgaccttctacgccgcagggcaggaaattacagacgcgacctacgccgtcaagttccactggcacggcaaggtcattcgcgtgcggccgagtggtgcaggcgcggacgagtcgtactacctgcgcgctgagttggagaacggcgagacttccggctacgggtcggtggactggtacgaagcgcccggcgtggagtgcaccatcgacaacctcgtgtcgcagctctacatctacaacggtgtaggctacatcgcacgcaacggtgcgggcctcacgtctctggctccgagcagcggcgagcatccggcctacggtgcgcgagtggcaggcgatggtctgacctcgccgatcccgtggttcatcgacaagccgatcacgatgctgtccgtcttccaagaccggctggtcatcggcgcacagaactacgtcaacgcctcacgctcggcggactacctgaacttctggcgcggctcggccgtcaccatcgaagacagcgaccccatcgaaatcttcgcgcacggcagcgagggcgatgtgctccggcacgcgacgctctacaacggcaacctcgtgatcttcggtgaccgtcagcagtacggcatcagcggcgactcggtgttcagtccgaagaatccgctgattaaagcgttcagtgccaacaaggattcggttgacgcgaaggcgcagacctcgggcaactacatcttttatgcgcagtacggcagcgaaggcacgagcctgcaccagatgcgagtgggcgcgctcaacgggcagcagacggtgacggacgaaatgtccaacgagctggactcgtggctgtcgggcactccgttgcagatcaccccgctcactgcgccgaacctcgtcatgttccgcactcgcgagcacccgcaggacttctacctgtaccggtacgaggacaacaagaacaacgggcagcgcatcgtggatgcgtggtcgaagttccggtaccacccggcgctgggcgaaatcatcggcgtgagcagctacaagaagaacggcctcgtgttcactgcgcgcgggtcgctggtggcgtgcgacgtgttcgacccgaagggcgagccggactcgcatgcgtgcctcgacagctgggcgagttttggtacacctacgggcgtacagactgcgagcgcaagcatcgccgtcaatagcactagcccgtacttcctgctgggttgtccctacgcgcaggcgtctgacttccttaaccagttcgatgacctcgctgctggtgcgctggaatacggcgtggtgtccgaagctctggtgatcccgaccaatccgttccctcgggaccagaacggtcaggccgtactcgatggacgcatgtccctcaacaaggtgacggtggacgtggagaacacggcaggcatgatcgccacggtggcaacccgcaacagcaatgtgaccactacggacttcgagggccgcatcctcggcgactccgacaatctgatcgcgcggcaaccggtgtaccgggggcagctcaacatcagcgtcgggcgcgaagtgcgcgagtgcacctacgagattcgcagcaaggattggctcccgctccgggtgaccggcctgagctggacgggtcagactttcaacaatgtacggagggttagctaatgggttcggttaatacgatcctgcaagcgaacaacaccacccgcgttgcccgtgcgaactaccgtgcagccgttgcgcagaccgacaaccagaaccgcagcgaggtcgccaagaccggcttcgctgatttcatgcggtccctgaagaacaacgcccaactggacgccgccgcgaaggagtacaactccaacatggaagcgctgtccgaggagctgcgtgcgcgccaaggggctgggcttaactcccagctccaactggcgaacgcgcgtggcgcacttcaggcgcaggctggtgctgtcggtgtcggcggctcgtccgcagacctgatggattcgatggtgcggttgcaggcggaaatggatcaggagacgcaggccaacgctgtctcgctcctcgcctcgcggggcgcatcgcagactgcgcagatcatgtcgcgcgcgtggaacgggatggacatgagccgttcgttcgggcagttcgactactcgcagcacatcgagccgcaggcaatgaagcgtcgcttgggcaagctgatcggcgtggccgtggctacctacttcggtgggccgatggcaggcgaggccgtggcagacttcgcggtcggcacgtggcaggcggacaacggcaacttcactggtgcctctcagtccttcagcaacgcagcgcagaacggtatgcaggcgtggcagcagtccaatgatcgcggcggcaagtcgtgggcgtccactaccttcgggtacaacgacggcaccggcaagcagtccgtgactggggcgaaggtcaccggcaacttcggcaacaactacgacaacttctccaccactacgtccggcctcggctggttcgatagcggcagcggaggcaactcaggaggtgcatggtaatggctgacatcggcacggttaccttcaacacgcagtccgcattgcagggtggcatcaacgccaccccagcactgtcgggcaacaccagcattcaaggcgctggtgtgaatcaggtcgggccggttcaatccggcaacgactggttcgcaagcactggtggtatgacgatgccggacagcaacctgccagagttcttgcaggagctggcagcgccgaacaccgccaagctgaagcagcagcagatgtgggacggcttcgttgccgcccgcgctggtaagaccatggacgagattgctgcgaccgaaccgtggtacaagaaaatcttcggagacaccaactacgagattggcgcgagcatgtataacacgctctcgcaggtcaacgaaatggagagcgacttgcttcggcgtatgccggagttgcgtcagcttcctcccgaggcgatggcgaaggagttcaacgacctcgccactgcccgcatgaccggcaacggtttcgcggacacggtgttgcagaagaccttcatggatcgcgcgggttccctcatggacctgcacaccaaggagcgcacggcatggcagcagcaggagctggtgaaggcgcagtacgctgcgaactcgtcggcgtccaccggcttcaacgaactggcgaagcgcacggcgatgctcggtaccaaccgtcccatggacgagaaggccaccgaggcgctgacgcaggcgcagctgtccctgctggacggactgtcgccctcgcgctaccagacggacgagtcgtacaagtccgcgatcactgcgttctatcgtggcgctgcggatcgcggcgagttccacacgctgaagttcctcaacagcaagggcgttctgaacgccatcgacccggacgggcagctgggaatccagcagtacgtgaagcaggcgcaggatcgttaccgttccgactggctcgatgccaacccggagcaggccgagaagatggcgctcgtctccatgtacgcatcggagggcattggtgccaagccgtcgcaggcgatgatcgaggaaatgaactcgacctacgccgccgagactggaagcgacgcaccgctgtactccggtacgcagttggcttcgatcatggcacagtccgcaggcgcgcacatccgcgcacaggaagccgtcatcaaccagcgtaacgctgcggccaaggccgcgctgaccgaccagcagaagctggccgcgcaggaggaggacatccgtggtggcatcgaagcgttcaagcgcggcacgtacgcgcagacgatcaacatccccggcgtggacaaggagctgatcgaggcgaacacggtgcaggcatggaatgccacgatggccgcgaaccccaaggtcgccatgtcgcagctggtgtggaacgccaacaccgggcgaggcgctgtgctgaagggtgtggccgaccagttccagaccacggcgcgcgctgtgctccgcgatcagccgaacacggcagcggctgcactgtaccagcagtggaaggaactgaagcagaccaccgccgcacgcatcgacacgaacggtcagcccgtgcagggccgactgactggcgcgactaccgctgcgctgtacttcggagatagcgtcaacacgttcttcaacaagctgcaagcgttggagaatggtggcgtgaacttcgagcttgcttacgaggtggcccgtggagaaatcaccaccgacgatccgacgcagttcgacgcgaacagccgtaaggaatccgaggctactcaggctcgtgttacggaagctatcgccaagctcaaccccaagtacctcggcatgttcggcaacaagctgggcgactctggccgcgctgcgtatgctcgcgccatcgtccgctcggtcactgacaccggtggtctgctggacacttctgcggaaggcttgcaggctgcggctactcacgccaagctggcctacggtctggaagacgcaggcaagtacgcatgggaaaacggacgcgacgacgaaggccgagtgatcggcagcgtcggtgcatggctgggcttcatggacacgaaggaaaccggacccgccatcgagaaggccatcgacgcagcactgcgccgggtcaacatcgagccgagcaccgggctgaaggctgacgtgttccgcatgaaggacagcgagaacggcgagccggtgctgtacgtcaacgctgttggcgagaagggctggaaggttgtgccggtgtacgggcgcgacatcaaggacgagtacgagaagcacaccaagcagcagcgtcagttgcaggccccggtaccgcagggctacgttcgcatgaacgacggtacgattcagcagagcatttccatccaacccaaactgtaaggagatagacaatggcactcgatctttcggggctgacccaagaccagcagattgccaaggctgccgcttatgcgggagtgccggagtccatcgtgcgcggtcagtggcgagtagagtccggcaacgggcgtgccgccaaggacgctgacggtgtgatccgcagcaaggcaggagcacagggcgacttccaagtcatgcccaccacgcaggcaacgtgggaagcgcgcaacggtcgcaagtacgacatgcgcaacttccaagacagcatcgagctgtatgccgacatcatgcgcgagaacatgcagcttgccaagggcgacgtgacgaaggcgctgcgcatctaccaaggcggcaccaatccgaagaactgggggcaggagaacgcagcctatgcaccgagcgtgctgggcggtgcgtccgctcccgcagtgtcggcgcagccgcgcagcctgaccaccacgcaggcagacctcaacgccgcatggcagggcaacccgaacatgcgcgaccgtacgtggtccggtgcgtccatcccggatgcgtggacgggtgcgcccatcgaaggccgcaacgctctggcgtcggcagcgaaggaacacatcggcaagattcgtgcgggcatcgccgagctgtcgatgggtcaggtagcacaggaaggtggcaccgccgcgcaggccgtaggcaaggctcaggctgtccgtgcatcggatcaggttgtgccgtggtgggtgcgtcaggaagtggacgtgctgaacaccggcgctcgcaaggcgctgctggatcagaccgaacaggcgctcgcgcaggaccgcgcggacgaggagctgcgcaactcgctgaccttcctcgacaagtggggcgctgcgttcgacagcggcatcggtgctgcgatcagcaaccagtttgcgcgcgaggacgagaacgttccggaaggttggaagtacgacccgaaggaatgggagaagccgtggatgactgccgacgaactcgaagacatccgcgatgcagcgtactcgccgaacgagctgaagtacgtcagcgaccgacagttcctgcgccgccactccatgcgcatcaaggatcagcagactggctggggtagcttcggttacgacatggtggcaggcttcaccgatccgggcaactgggctatcggcggcgtcactgccgcaggcgctaaggcgctgggcatcggctcggctgcactcgttgccgaagggcgcgtgggcgcgtcgctcgcgtcggctgctgcggagaacgcggtcggttccgtcatcacggacgccgcgctggttggcatgggcgagcgccgcaacttcgcggacttcatgaccgacgctgcattcgctaccaccataggcaccgcgatgcacattccgggcgtgcgctcggctgcgcagattcgtgacaaggcaaccatcgacctgtccgcaggcaacgctgccgcttacggcgaagcgtggtcggccgacctgaaggcgcgcgctgtggccgagctgggcgaggacgccaacccggtgctggtgaacaaccgcatccaccagcttgccaagcaggaggctgtggattggctgcgcgctggtatggccgacgtgcctgacgacttccgtatcttcgcccgtcccgacgtgcaggagacgaccaccaccgcaggcaccactggtgcactcgcacgggacgcgggcaacgtggacgcaacgaccgggcggtacaacgacagcgtgggtggccgggtcgatcagcatgacccgctgctggaacgcgcatggaagaccgcaggtatcaagggcggtaacgtcgatggcgtgctgaagtatctggaatccaacgcctctatcccggaggacgtgcgtgctatcgccaacgcgctgaagcgtggcgggcggctgagcacggtgaagatcgtgccggaatcggaactcgacaagtggttcgccggtgccaacatgggtccgggtatgcgtgtggccggtggctacaacgccggactggacgcgatggcgatgcggaactacacgccggaagtggtggtgcacgaaatgctgcacgctgccacgctgcgtgagctgcgcagcaactcggtgttcgggcaggaaatggaagaactgctgacccatatcaacaacagcatcggcagtgtggactccacgctgaccaccgctgcgatggagacgcgcatcaaccagccgcaggcaggcttcctcgccaacactgacgagctgatttcctacggcctgacgaaccgcgctgtgcaggcggtgctgcgtcagatgcccgcgccgggcaacacccgcccgaatgcgtgggagtggctgaaggataagatcgcgcgagtgatgggtctgaagaatcaggagtccgcgctcgaacgcctgatgtcggtcgtcggtgacaacctcggcgcggaagtgcgcgacacgcaggccggtacccggcagacgcgtggcatgctcgccaactcgatcttcaagtcgaaccgcgagcgcaaggctttctaccagcgcaccggtctggacaagtccgtcagtgatgacgcgatgcgtgtgcaggtcgccgaagtgatggcacgctccgaacgcttcagtgcgcagtacggcatcgacgcggcgaagctgtccaccatcatgcagcgcttcgggctggaagctacgagcacgactctaatgtcgtccaagtcgccagttgcccgcatgcttgcgatcaccctgttggagaatcccgagggtgcagcaggccgacacagcaccgcagcgatggatcggcatggtcggtttgagtcgttcatgggcacccgcccgcgtcagtgggaagcggcctatcgcctgtggcgtgcggacgtgcgcggtatcggtgcgatcaaggacttcgccacgggctggaaggctcgcgcggacttcgagtacgcagtgaagctgtaccgcgagactcgcttcaacggcggggacatcccggatgcgcacgaggcagtgaaggcaatggcccgtgagttggaccgtggctacaaccgcatggcagcagagcagcgcgcggccggtacggtgggcgcacagcgtctgccggaggaggacgtggagggctacgagtcccgtacgtggctgggcggcagcatcgctgctgctggtccggtgcgacgcgagggtatccgtcaggcgatgcgcgatcagttcgaggtgatgggcgagctgtatggggacgacttcctcgataagttcgctaccaagtatctggaacgcatcgagcgcaaggctgcgggtgtcatcgaagcgccgggtcaggtcttctcggagtcgcaggcggacacgctgcgcgacactctgcgggcgatgtcgctcaacgaggaggagattcagaaggtcatgggcaagtacagccgtggcggtgcgaagcacaccaaggcgcgtatcgacctcgacgtgaccaagcagtacgaggacgctgacggtaagttccgtctgatggactatctcgacaaccgcgtgatggacaactaccgcaagtacgcgggacgtgttgctggtgacatcgctctggcgaagcacggcatcctcggcgacgcaggcatcaacgtggcgcgcgaagcaatgcgcctgaccggtgccaacgatgtggagctgaaggcgttcgagcaggtgatgtccgagttccttggtcgcccggtcggtaccggcgatccgactgttctggcgaatgcgcgtctgctgacctcggccatccagctgggcggcgcgggcatcaatcaggcagcggagtacagcaacggcctcgccgctgttggtgctgctggtgtggctgacgcaatccgtatcgctccccgcatgcgcagcgaaatcatgcgcatcctgaagggcgaggacagcggcaaccaaatcctcgacggcttcgagttcatcagcggtcgcggcttcggtctcgccggttacgacctacacatgttcaactcgctggacacgcaggcgtcgatgtatggtagcgagcgcgcaggcttcctgacctcgctggtgcagaaggcagcgcatgcgaaccgcatcctctcggggcagcgggccgtgcttgctgtgcagcagcgtggcttcgcggaagtgctgatcgccaagggcgtgaagttcctgcgtgatggtgctgaagctgacaccgccctgaaggacatgggcattgacgacaacctgctgaaccgcctgcgggctacgcaggatcaggtcgtgcgctggggcgcggatggtaagctggaagcagtagacccgcgcaacgtcgaggggctggcggatcggcaggcatggttggcgttctacaacgcgatcaaccgtggcacctcgcagattcttcaggacaccttcatcggcgagactggcaagtgggcgcacaacggctggctgaagctgctgttccagcaccgcacgttctcgctggtcgcgcagcagaagcagctgggccggtacgtgggcaactacggtgcatggcagacggcgggcctgatcgctgctgcgatggctgtggcggctccgctgcaagccctgcgggtgctgtcccgcgtggccctgatgaacgatcaggagcgcgacgaggccatcgaccagaacatcctgtcgcctctggcgctgggcaaggccacgctgaactacgtgtcggcgacgggtatgctcaacgatgtgctggacgtgggcactggcgtggcgggcggctggtacgagtacgccaccgatacgcagggtccgacgtggctgaagcagctggccggtgggcagttcggcaaccgcaaggaagtggtgggcgggcagttcgcgccgtcgctgggagtcatcaacgacttcgctcagggcattgctggcaagccggagaatctggccgacgtgattccgggcgggcgactgccgatggtgatcccgctgctgaagggcgcagccagccagtggaaggaggagtaagatcagggccaaggacggcccacccttttggtacacctatagcaaacaggaggcagcatggcagttccagacccgcagctgcgctacgcgacagacgtgttcgacgccgatggcgtgaccactgactggcagatcagctttaccggtggctacatcaacccgtcccacgtgtacgccatgagcggactgctggacgaggagactcagctgctgaccgaccggactccgcacaccgtggaagtcctgagcgaagacgatgacgctagtaccgtccgagtctcgcctgccgtcgccgctgggcgcaagctctacatctaccgcagcactccggtgcagcagatgctcgttgactacgttaacggtagcatcatcagcaagacaaaccttaacctcagcaacgaccagctcctgaagatcattcaggaaatgttcgactcactcaacatcgccacccttagcatcgaccagcaggtcggtgtgatcgtggacctgaacgagattatccagaacatctacaagcaggtcaccgagttgctggcagctggtggtatcgtgtccgtcgccccgcgcgtctggtccggtgcttggactggcgatcaggtgggtgacaccgacttcgacatggtgggcgcggacgtatccggcgcgggcttctacgacgtgtacgtcaacggcatcggcatgcagccggacgtggactatcaggtcacgctcgctgacggcaccgatcccagcttcatccgcttcgccacggttcctgccgagggcagcatctggttcgccgtgctgcgtggttacgccaagccctacaccgggcctgcgccgatcaccgctgcgagcctgcgggtgccgatcatcacggcagagggtccgacttactacgccgccaaggctaccgagtacggactcgtgcgctgcacgtacgccggaggttgcgccgtcaacatcaacctgatccccgaagtgggcgacggtgaaaccaagctcgcctcgggcagctacttcagcgtgcagcagaaggcaggccctgtggtcatcactggcgacgtgggcgtgacgctcgaagtcccggtcggctgcaccgccgcaactcgcggcaccaactccgtcatcactgcaacgtgcatcgacggcgacaccaacacgtggttgctctcgggcgacttggctaaggagtaagcatggctaatcacttcaggctgtacggccgaccgctcatggcggacgaggttgcagatggcctgtcggtgacgggcgtgctggaagggtacacggcgggcgaggcttacgagtctcgcctgtccatcaacaacccagtcggccgctgcaccgtggaggtcatcgaatcgacgctcccttcgggcgctgcggtacgggtggacaacatcaccaaggaagtcgtcgtcaagtgggcggctttcactgaagtcgtggacgaggaaaccctcgtgcccaacggcgacttcgaggcaggcgacgacggcacgtggttgccgggcggtggatcgaatggcgaaggctggtcgattggcactggctcagactacgacaccgacagcggcgtgtacagcgcgcgcttcgccaacatcaagacgggcggcagcgacctgctcaacccgctgatccctgccaaggtcaacgactacatccgatgcaccgccgaggtccagcagggcgcaagctccaagggcaaggccggtgctcgtgtgtcgatcatctaccgcaaggaggatgggaccgagctgcaacgcaactggggcaacatggtttcctccggcagcaacggtgcgtggcaccagtccgttgccgaaggcgctgcgcccaaggacacgaagtacgtgcaggttgtactgtcggcgttccgcagcaagcagaacaaaccgctgtgggtggacaccgttaagtggaaccacaagtacgtactgggtcagaacgacgacagctcctacttccttagcatcaaggtcacggacgggttgaaccgtgtggcctactggtccggtcgtatcgaggagcagggcatctacgttacgtccaagctctacagcttctaccagttcgatgccgcgatgctgaccagcagctttgctgggtacagcaacatcgacatgctccagcctttggatactgcgtcgctgggttcctccttcgtaagctgggaactccgaagctctaggcaggattatgccgccgacccggagagcacgttgtacgggagcgctttcgtttcgttcgacatccgatccatccgtaaggactacacgcctgacccggagacggcgaagctgtcgagttctttccattccttcaccctgaagcagcaccctgtagtcaaccagccgctcgacgcgactgcacgactccggtctggcttcgtatcatggagcttcgcatgatccacaatcacctcggcattgctggcgtgttcaccatcagcaagggtaagtccctcgatactctcgaagttgtagccgactggcagagcaaccttatcacggacggtggtatggacgcactgggtgataccggcagcggctatcctcgcagcatgtacgacctcattgcttacttggcagtcggtagtggcagcgccaccccggcattcaccgataccgctcttggtgcacaggtggcgcaggttggtcgtacgtcctcggacagcggtgggactaccactgccccgtactacgcctactcccgctgccagtaccagttcccggctggtaccgctactggcgttctgtcggagcttggtgccaaagcatacaacaacaataccggcgcgtacatcctgaccacccgtgcgcttatcaaggactccgcaggtaacccgaccaccatcacggtgctgtcggatgaaatcctcgtggttacttacgagctgcgcatgtacgcagataccacgccggttgtcactactgagacgatcaagggtgttagcaccactgttacctgtaagcctattgcaatgggccgcagcggcggtatgaacggtcagtcggcagtcgcttggtcggactacgtgtgggggtgctactacttctacggcggtactggcgacggcaccggagctatcaccgaccagtatccgccggggacgattgccagcttctctgacttgcagcttcagcaggtagcctatgttccgggtacttactaccgtgactgcgtttgccggatgtcgatcaacaacgtgcccggtggtccgatcacggctgcaatgggactctccgcgtgcgtgaccttccaagtcggcttcaatccgggtatcaccaagaccggatcggagacggcgaacttgcgcatgcgggtttcttggagccggtacacgccatgatccccactgtctcccaaagcatccaacgcggtgactgggtggagcagcagaatcggcgcacccgcccgctcattgacttcgagcagggcgggctgactctcaacgcagcagtggacgacctccaagctgcgctgtggactgccgagagtgacggcagcagcgtcgtcgtttaccgcgacggcgttgccccggtcaccgtgctgaccgactccgggatcacgcagatcgcactggccttcgaccagaccatgcgcccgcacgtggcgtacatggcgggcggtgtgtgcaagttctactggtacgacacggtggctgcttcgatgcagaccatggtgatccccggtgctaccactccgcgcctgtgcatggacgagaagcgggctgtcttcgccacgcagagcgacgtgctcctgtcgtacaagaacggcagcaacctgtgcgtacgcgcgcagcgtgagcgcttcgcaaccgaacatgtgatcgcctcgggaatccccggcgacc

SEQ ID NO: 8 - DNA, 44427 bp, unidentified
  source 1..44427: mol_type = genomic DNA
gcgctgccttggctgaatcgttaataaatctcttggcgaaaggtgttgacgtggccggtgcggtgtggttcaatggcgtcactggggcagcgacagggcttcaggagggccgcaaggggcttgacaggggctaccctacctgctaccatgcgaaccgcagctgtaggcgtgcgagggccatctgtatcgtttcggccttttggtacacctatagcacacagtcggctcaacctgaatcaccgtctatcggtactctgtcgagctgattagttagctacccgctaggccaacggttgacgcttgcgatgcaagcagtagtagacacacggccgcaatggtagtaagctgcaacgcaagtcgagtgacgtgatccgtagtggcgccgccaacaagtgggctaagggtacacgggagtcactggtaagggatgcgaggagctaccgaaccacgcttgacactaagctagcagttagctatgataggcggcaagtggtagccaccggaacagcggagcgacctagcggtaaggctagacgtgagagattacgggtgttgaggctgaggtgagaccgggacaccggtcaagacactaacaggagcgcacatggtcctctaacggatagcttgacaaggcggcacagatagccctttgaggccttgcaacacgtggaccaccgacgtacatggtgggatggtggcgacaggacgcccaacgggttagagacccgagcgagccaagggcttgacaggatgcaacaagggtgctagtatggcaccacgctctgaggagcagccacattggatggcgtaggactaccgctaacgggtagggtgtaacgggaagcgtgccaaccacagccaatagtggccgagagttgacgtggaccgccaagctgcaacgtagcactagcggataaccggatgaactgggatttcaaaggcccatagaatccaccagacttgcaacactggtgccgctttacctaagcctaacgcttagggcttcccatctgccgtgagagtcggccacgggaagtaacccactgccaaggtgggaagccggtcataaggaggtggtgagcctcctatcgcatggaatactgtgcgtttcgtgaaaaggctctacgggccacacggtgacaatggcactgctagccggagtagggttgacagcccgaagggctagcagattgatgcgccctccctttgcgatgaccatgcaggcaaatccggtggtcagtgtgcgcccacgataggcgatgcaacggctctaatcgagaatgagggattgaccgactcgacggctttctgagggcgcatcaatctgttagttttcccaccagtgccaatggaggcacaacatgcaaggctcgatcaatgccaatctcgaccgcacccagcgtaagcgccgcttctgccagttcacccggacggcaagcgtgatggacctgcgcaccacggagcatgaccgcaagcttgccgagcgcaagcgccaagccgagcgctacgaagcccgccacggaaccgccggaaagcgatctgtgtttgttgtcgagggtaacagcgggacgaaccgggcgaaccacgccgctgacaggagggcttacctgtgatccggttcaagttctctcgccactacgtggaagctgcccgcgattcctacaatcgggccatcatgaagcatccggccggctctgtgtcggcgctctacgtcctgccgtgcggtgggcgttcattcgacatccgactcgcttaaatgcaagctactgggccttcgcaagagggcctagtgtcgtgcaatcggcacggacccaacctgaagggaaccaccatggacatcatcaccggaagcgctgacatcaagcgcgccatcaagtcgatcaacaccgcccgcaccaagctggtggaccagattcagcaggccgcgattgcggtcatcaaccacgcacacatccacggcgacgttacgctcgcttccgatctgtgtctcgccgtgggcaacggcatgaagcatgaagccctgcgcctgtacctgtccgagttcggcccgatggctccgaacgacgacaaggaaaccaaggcgagcgcgcccatgaagtttgccaagagcaagcgagtcgagggcgaagctctggccgacgtgctggaacgtgccgccgcgaaggcgtggtacgacttcaagaccgagaagcccgcagaggcgttctcgttcgccgccgacctgcacaagctgctgggccgtctggaaaaggcgaccgaggaaggctacgtgccgaccgaggaggaacaggccgtcatcaacgctgcccgcgctgtgccgaagcccaccaagaagaaggagaacgtgtaacatggaacccaagatcaaccttcgagtgacccagcgcgaagcatccctgctgcgctcggcccttcacatcgcctgtgcactgaccgcaaaggcagacccgtactccaaccgcaagctgtccaatgagttcgccgtgctgcacggtgagctgcgcgacttcggtgtcgagagcttcgagcgtgacgccatcctgcaattcgaggacgacgtgattgcggcctgccgtgacagcgatgtcgaggcacagctgctgcgcgacctgatcgcaccgccgacgttcaccgtgggctacggcatgcgtgaacttgacttcgctgctatcgaggcgcgggtgatggcgtgcctgctgtctccgttgcctccggtggtgttggatgcctcgcagctggacttcctcggcagcgtgaccggccgcatggtgttgcccggcctggcaatgcccgacaacctgccgcgtaagctgccggatgtcctgatggacgaccagagcgcacgccacgtcgccctgactgcatcgcagaccgggctggtcaacaagacgaagaccaagggctggatcgtgcagttcaatctgcgccacggcagcatcgccctcgccaactgggcgcaggtgcgtgagctgggcctgccgcagcgcagccgcaatgctgcgtaccgcatgctgaaggcgcgggccaaggtgcagggcatcagcgaggatgcgtaccgtgtggtgcccgaaggcactcccgatggcccggagaaggatcgcggcttctacaccgccgagttcttcaccaagcatgcgcggcgccctcaccagctgggttggaatacgtccactgtgatcggactcagcggcacgttcaccactgcgcaggctgcacgcaacgccatcgcctcgcacgtcggcaacgatccgaaccgtctccgccgctaccgcgtgaagtggcacccgagccgcgcgtgatctaccgctgcgccttctaacgagggcgtagctttggaaccacgcccaacaggagggcacattgcatgatccccgtaacttacaagcgcatccgtagtggggagcgcaagccgatccagctgtgcgagcagccgcgccagtggaaagagttcgtgacccatgagcacagcgtggagcgctggtatgcgtgaggtcagcctgcgccttgtggtgaaggcgctgccgctcgttaccgtgaagggtgtggctgtcggggattacatcctcggcggacatcacaccagccacgaggcgtgcgagcaagccatcgaacaccaccgcaagcaccacgagaaggtgcccaccctctactcgatagaggaaatcgaaatcccacccgtcaatcaggagaaccaccatgcgtaaggtatacttcatcgtctcgatccccaagaacagcaacgatggcgtcatcactggcgtcgtcgccaatggcaccggccgcaccccgacccaagaggaactggatgcggtgatcgccgagctgcgcaccaagggtgccaccaccagcctgctggactcgctgcgtgacggcacgtacccgaaccagctcgccatcttcgaccgccgcgccgccgtgcgtgccgaggcggatgtgctcaacagctacggcgggtcgttcttcaactggcacatcctcgaagtgggcgagagcatccgcaagccggtgcgcaagccgctgggttggcgtatcacctacgccttcgccgaagaccgcagcgactccgatgtcagctgctacaaccagcacccgagcgccaccgtgcgcatcgacggcaacgagtacaacaagagcgagtacaacgtgctgttcccgacccgcgatgcagcgcgcgccgtgttcaatgccgagtcgctgggcggcgagaacatgggctaccgtgtcgagccgtactatgcgtaagctctggctgcgcatcctgatcctgctgtactggatcgtgggtcgtggcccgtgggttgtcgtcggccagtaccatgacgacgacggcaagctgtgccggttccgcaccggcccggcttccactgggttctcgctgacgttcgatgacctcggcgcagccaacgactactgcgaccagcgcaactggaaggcagacactgacccgctcggcaccacgtactacgtgtggcatgagttggagttcaatcacttcggaacgaggaggaagtaaccatgggtttcatggacaagatcaaggctgcggccaagtacgtcaaggacaaggtggtcgcagcggtgaagccgcgccacgatgacgacgacacgccgccgcctgcgccggacaccagccggcacctgcacgtcagcgtgccgctgattcccatcgacaacccgatcctgcgcaagatgctggggcaggactacttccccgtgcagaaggggcagggtcagacccgcatcgtcggcaacaaccagctgaagcgcgtggccgatagcctcggcgggaacaacaagcagcgtcgcaagctgcgctcccgcatgaagcgtcgtgctgccgagctgcgttccggtgcatcgttgcagcccaacgtgcagtccgcactggcaggtgcagcatgagcctgcgcatgggaagctgggtcgaggtgactgtgcccgacagccgactgctcaacgtgcagccggagattgccgccgccgtgaagctgatcggcggtgcgaccatgaccaatggccgtggcctgtacgtccgcaaggacaccggcgcactggacgacgaggcggtgaccgtgatccgcttcgacctgaacttgcacagcgagctggtggaccagtacatgagcgccatccgcgccatcgtggaccgtctgctggtgctgggtgaggagagcgtgctgcgtcgccgcttctacaatggcggcggtgggtacaacagcgagctgatctttcagtaacccgagccgggtaggctacgactggcccacgtacgggccatcctatcaaccgtcaagaggaaccatctacatgtcgaacgaaaacaccaccgagcagaccaccgtcagccactacgaagccaagcgcgccgagctgctggaagacatcgccaaggcgcaggccaaggtcgatggcctgaacgagaagctcgccaagctggatgccgtcgaggccaacagcgccgccatcgaagcgctgaaggcgggcgacgccgtgtcctacctgttcggtcgtgccctgaacaagcgcgtcctgtccggcgtgatcgtcgccaccggcaagaacgacaagggcgtgctgcaactgaaggtgcagaccggcgaaggtctggatgccgagctgaacctgatcgacagcagcgccctgctgatgtcggccgaggaagtgctgaaggcgcaggaagaaatcgacgccgccgttgccgaggcccagcgcctcgccgccgaagccgctgccgccaaggctgcgggtggcgaaggcgggcagtcgtgagcctcgccccgccgtcacccagcgtggccgtcgtcaagcgtggcgacgagctgaagcccggccagaatgcgtacctgatcgacacgcggcagaccaacaagctgccgaagggcaccgggttcgtcgtgtccaagctgaccagtgaagacggctcccgtctgatcgtcagcacggacggcaacggctccgtcctgtacgccaccagccacgacatcttcgaggtctgggaataaccaagcgaggatagcatgagcgatacccttcccgacaacgactggctaccacatgccgagcgcctgcctgttggtggccgcacacgtgtggcccatgagtgcggggagggtacgcccttgcttatctcacgagagcacgacaagtccaccgcattctgtttcaggtgcggtggcacaggattcaagcgtgagcacgagagtatcgaggccaagcttgcacgaatccacgccgagcagacgagcgaacgcagagtgcgtgcgactgttgagttgccagagccacgggtatacgacacccgcgagtggccgctcgacgctaaggtgtggttcttcaagatgggactctcgcttcagatgatcgagaagctgcggctgtactggtgcccaagcatcgggcgggtggtactaccgatcactgaaggcgacaacgtggtatactggacagcccggtcggcaacgagacagccgaagtggctaacacctgacgttccgaaagacggacttgtcgcacgctacggcgtgggcacaggtgacaccatcgtactgtgcgaagacccgctcagtgcatacaaggtgggactggtaaccgaagcgtggtcgttgctcggcaccaagctgcacaacaaagtgttgaagcagctgactgatcgaggccaacgtgtagcgacgtggctcgatgacgacagaggtagaagcaacggtagcaatcccggccaagacagtgcgcgagtaatcgctgcgcgtctacgtgcgtttggtctggactacaggaacatcacgtcaccacgtgacccgaagtattacacgaccgactacatcaaggagaagctgcaatgagcaaacccatcgtgcgctaccggcgcgctatcatcccgcccgtcgttggcttccgtgccacgctcggcggcgtgcttgcgcatccgaacctcggcgactgcgacatcgtgcacacctcgacggtgctgtatgtggcggacggcgggcgcaagttcgagacgcgcaacacccggtatcaccagctcgattccaagtacgaacccgaaggagaacctgatgagtcttgacaccacgctgctgcggttgtgcaccaaccgtggcaagttcgaccggctggtacccagcgcaccacgtgatgggctggacgagctgaccgtgctgatgctcgatgcgttgcgtgcgtactacaaggagttcccggacacgaaggacttgccgttcgatgtgttcgatggctgggccatggagttcaagtggaagacgcagcccgacgacaagaagtccctgctcaaagttctgctgaagcagatgcgcgagccggtcccgcccgaggcagagcagggcatgatcgagaagctgttggagttggagcttgccaccactgcggtcagcaagatcgtgcagtggaatggcggcgctgagttcagcctgcgcgacgagctgtacggcttggccgagacgatcaccgaccgaatggatcgcaaggcgcggctcccgctggtgcaggagacgcccgaggaactgatgcagatggacgagcacgacatcggcatccacttccgactgcccacgttggcgaagaacctgcgcgctctgcgtggtggtgacttcggcatctacgccatgcgtcccgacgcaggcaagaccacgttcctgaccagcgagtccagccactggatcacgcagctcgacaacgtttggccggaccagaagcgcaccggcatctggctcaacaacgaggggccgggcaagcgcatcaagcagcggtggtatcagtcgctgctcggcgctaccatccctgagatggtggagtgggcgaaggatggtagcatccgcaagcgcatcgaagatgcgatgggcggggacatccaccgcatgcagttctacgacatccacgggttcaactccggtgaagtcgaggccatcatcaagcagaccaaccccggcttcatcatcttcgacatgatcgacaacatcacgttcaccggtggcatgaccaacggcgggcagcgtaccgatcagatgttggaggcgatgtatcaggccgctcgcaactggtgtgtgaagtacgacgccgtgggcgtggcgacttcgcagatcagcgccgagggtgagggaatccagtacccgccgcagtccgcactgaaggacagcaagaccggcaagcagggtgcgtgcgacttcatcatcatgggcggcaagctcaatgacccagcgatggaacgcttccgctacatcggcaccccgaagaacaagctgcaccgcgcaggcggcaagcgtgacgttcgggaagaagtgatgatggatgcagagcgtgcccgcttctatcaggaggcagcatgagcaagccaattcacatcgtagccaccgggttcacggtgtcggtcagcttccccggtgaatccaccgaggcgaagaccttcaactgcgtgagcaacgcgcaagcaatccaccttgccaagctgctgcgcaaggtgcacgacgcaggctacatcgaaggccgcaacgacgcgccgcagtggaagtggggatggctgcggaacaaacacagcacttggatcggcgtgcactactcgccgcacaacaagcgctggtgcatcaatctgatcccgtgcttcacgttctggatcaccaagcccggaggtaacacaccgtgagtaccgaaccgaacatctacctgccgcgcaacgtgggcgtcatcacgtccagccgcaccggcagcagctacacagtcgagccgcccgtgaccgacacggacatcgacttcctcgtgctggtgcaggacttccacgaggccatcgaaaagctggtcgatcagggatggaccctgtgctccggtgccgatggacactacgaggaggacgaggactacagcaccacgtggtatgcgctgcgcaacggcgtgttcaacgtcatggtgaccgccgactccggctggtatcagcgcgcggtcgaggccaccaccatctgcaagcgccgcaacatcaaggacaagcaggaccgcatcatcgtgttccgttgggtgcgcgacgggctggacttggatggcgatgcgtcggatgaaatgtaccagctggccctgcaacggtggccgctgtgagcttcacttccttcgacctcgaaaccacgatccgttccatcctgaagcgcaaggccaatccgttctacgacatgaacaagatcgtggcgattggctacaagcggaagggtgacgcacggaacaccggcctgtactacgacacccgagtcgggatagacaaccagtacatgggcggcgcacccgatgggtggctgcgtgagctgtgttacgggcagcagttcctcgtcgggttcaacatcaagttcgacatcctgcacgccatctgccaaggcccactcaaccggcaggcatggatcgagttcatcgacggcggcggcatggtgtgggactgccagcttgcggagtacctgctgcacggcatgacgcaagagttccacatggcgagcatggacgagacggctccacgctacggcggcaacttgaaggacgatgcagtcaagtccctgtgggctgcgggcgtggacacctgcgacatcgacaagacgctgctgatggattacctcctcggcaccaacgacaccgacgacgtgggcgacatcggtaacaccgagaagatgttcctcggacagctcgccgccttccgtgcacgtggtggtctgcgctcggcgctcctcaacatgggtgcgctgtgcttcaccatcgaagccgagtacaacggcatgtacgtggacaaggactgggcgcttacgaaggcgaaggagttggaggtcgagcttgcaacggcgaccgccgaactcaacggcttcatccccgagctgcccgagggcctgaccttcaactggaacagccgcttccacaagagcgcgctgatcttcggcggcaaggtgaagtacacggccaaggttccgatcatgtccaccgagggtgggccgacttacgtgcagaaggacgaggtgcactacgtgctggtcgatggtaccacgacggcgacgccaccggccgaggacttcgacaacctctggcgctacaccacgtacggcagcggcaagaacaagggagagtacaagaccaagaaggtgaaggtcgatgacttgaccaagcagaagttccgcaacgaggacatgctgttcgagttccctggctacaccgagcctgatgctgcatgggaaagcaagagcgatcccggcgtgtactccaccgctgccgacgtgatcgaggcgctgggctaccgcaacctgccgttcaccaaggcgcttgccagacgcgacgacatccacaaggacttgtccacgtactacatcacgacggacgagaagaccggagagcagaagggcatgctcacgctggtgggaccggacggcatcatccaccacaagctcaacatgaccaacacggttaccggccgcttgtcttccagcgatccgaacttgcagaacgtgagcaagggcgagctggacgaggagacgttggaggagaagggttcgcagatcaagcgcgccttcgtgtcccggcaccggggtggcaagatcatccagtcggactacacctccctcgaaatctacgtgcaggcaatcctcaccgagtgccgtcagctgatcgaggacttgaagcagggcctcgacatgcactgcctccgtgcagagcaggcgtggggtgagcaaggcaagtacgactacgacttcatcctgaaggcgagcaaggacgacaagcatcccgagcacaagaagtggaagaagaagcgcggcaacgcgaaggtgttctccttccagcgtgcgtacggtgcgggcgtggcgaagatcgctgcgaccaccggcatgtcggaggaagaagtcgaggcgctggtgcgcggtgaggccgagcgttacccggagctgggcgagtacatcgaccgcatggtcgagcacatcaagcgcaaccgcgtcagcactcagcgcttcgttccgcatcccaacgcggggcagcaaggcgtgccgcatgggctgacgtgtcagcttggccggtcgcactggaccacgccggacggcaagatgtattccttcagcgagtcaccgtccccggtgttcatcgccaacaagcccgcgagcaagggtggctgtgcgcagtcgttctcgcccacggaaatcaagaactacccgatgcaaggcaccggtggtgaatgggccaaggcggcgatgtacgtcagcctgcgcgccttctaccggaagtacgtgaccgaaccgaaggaatggttgggccgtgcgttgctcgtgaatcaggtgcacgatgccgtctacgtggatgcacacggcgacatcgcaaccaaggccgctgctctgctgcacgcctcgatgctggaagcgtcggtgtatatggagtggtggttcaactggacgctgccgcttggcgtcccgtgtgaaaccaagatgggcgacaacatgatggaggagaagaaccctcccgcagagttcgccggtctggtcatcgagtaccgcgcgtcgatccgcaaggacttcgtaggtaatcacaacccgtcgtttgaataaggagaacaacacgcatgagtcttgacgcactgttgaacaaggtcgccacgcagggtaaggatcagtcggtcgccagtggtggcagcttcgactacaccccgcccgctgccggtgtgaccaccgcccgcatcgtcgggtactacgagctgggcaagcacgagttcgagttcgagggcaagaagaagacgcaggatgaagtcgccatcgtgttcgagctgaccggtaagcagcacccgcacatcgaaaccgacaatggtccggtgccggtgcgcatgacgctgaccctcggcctgtccaccaacgagaaggcgcactacttcaaaatcttcagccgcctgcgcaccgaggagcgccacttcgtgcagctgctgggtcagggtgtgctgctggaagtcatccacaagccgggcaagcgcgacccgaacaagaccttcgccgaaatcgacaaggcttccatccgcaagccggtcatgccggtgccggaaatggagaacggcatcccgaccggcaagttcgtggacaccgtgatcccggtgccgcagcagatcaccccgctgggtgcgttcgtgtgggacttcgccgacgccgacatgtgggacagcatctacatccccggcgagtacccggagcgcaaggacgagaagaccggcaaggtcacccacgaggcgcagtcgaagaacaagacgcagctgcgcatcgctgcggcgctgaacttcaagggtcttccgtgctacgactacgccgccgccaagttggcgggcagcaccacggtcaccaaggaaggcgtcgatgcgctggacgaagtggtcggcgacgtggcgaacgccgcgcccaccgacgctgctccggccgacgacaagccgccgttcccggtggacggtagcgacccgatggcaggcatcgcctgatggacctgagcgctctcatggcagcggccggtgagcgctccccgatgccggtgcaggtggtacgtcagcacaacccgcgcgtgatcgctcacgttgatggggactacatggcgtacttcgcggctggtagcgagaactgctcggcgggggatgcacgacgcaacgtgctctcccgctgcgcacagctgaagcatgtcagcggagcgggcaagatcgtcatgcacctgacgcacgccgcgtctaccaagggtgatcgcttcctcgctgctaccacgcagccgtatcagggtcagcgccaagcaggccgcaagcccaacaactgggcgttccttcgtgagtggatggagacatacgagggcgacgctttcactcccaaaatctggctgacccgtgaggccgacgatggcatcgcgtacgtcaacgagggtgcagcattgcaccacaacatcctgcacgtggtgcacagcgccgacaaggacatgcgaatgttctgcggcgtgcacgtagactgggacggctacgacatcacagaggttccgctcggcgcttacgacatcgttggcgagaacggattgcagtacggtcacaagtggttctggatgcagatgctccacggcgacaccgccgacaacataccgggtctgccgaaggtgggcaaggtgacagcggagcagctgctgttcgagacgaagaccaacctcgaagcggtgcagatcgtgagcggcaagtacagcgaagtgttgggtgccgactggcgcaagacattcgccgagcaagccgtgctgctgtggatgcggacggatcgtgacgcagaactgctcgacgtgctgaagctcgacgtgttcgggccgaagctgaagcaggcgttctatgacctcgccgaggacgtgaacgagaagcgtgcaatcttggaggcatacaaagcatgaagcgactcactgcaacacaggtcaagctgctgcgcatcaagctcgcagcggagcaaggcaaccggtgctgtctctgtcagggacagttcggcctgaaggctccgctcgatccggtgctggaccatgaccacaagaccggcgctgtgcgcggggtgctccatcgcggatgcaactccctgctcggcaaggtcgagaacaacgcaggccggtacggcgtgcgcgacgtgttcgcattctgtgcgggcatccccaactacctgcggtcgcacctcaccaacatcacggggtacctgcatcctacctacaagaccgacgacgagaagcgtatcgctcgcaatgcgaaagcgcgaaagcgtcgggctatcaacaaggagacaccgtgacccttacccagttcattcgccgagcaccgaagcgcggcccgaagattctctgcctcgacatcgagacgttccccatcgagttctatggctggggcatgttcaacaacaacttcagcgtcaagcagatcaagcgtgactggtcgctgatgtcgttcgcttgcgaatggctggacgacgaggcgtcgttctacatggaccagcgcaacgtgcgcgacgtgttcgatgatcgcaagcagggcaaggcgctgtgggcactgctcaacgccgccgacttcgtgctcgctcgcaacggcaagaagttcgaccttcgcaagatcaaggctcgcctcgcaatcctcggcctgccgcccgtgtctccggtgcaggtgatcgacccgatgctgctgaaccgcaccgagttcgccttcacctcgcagaagttggagtacaccaccggcgtgatcgtgccggagctgcgcaagtacgaccaccacaacttccccggcttcgacctgtgggtggcctgcatgcagagcctgcccggagcatgggacgagtgcgaagcgtacaaccgcatcgacgtgaagtccatgaagttggagtacaagaagctgcgcggttggtactcgcagcatccgaacgtcgcagtgtactacaaggccgacggcagcgagcaccgctgcaacaagtgcggctgcaacgaaatgatcccgcaggatgatccggcccgcacgcaggtcggtacctacctcctgcttcagtgcaccgtgtgcgacggctacagccgtgggcgcaagctcacgaccagcgccgaggcgcgcaagcacatcaccgtcccggcataaggaaccgacatgaagatcaccgacatccgcagcggcatgcgggtacagtacatcggcaatgcgcccgcaatgatcgggctgcgtggacaggtaagccgcgtgttcgctcgtgatgtcgaggtcttcttcgacggtcgagttaagccgagctgctgcgttcccgattccctccgacagcttctcagcatcggaggcgtgaccaccaccagacgagaggtaccaatgcccgaactgagctaccgcgacgaggaccgtcgcacactgtccgaccgtggcgtcggcctgaaggatgacgggggcaagccgcaggcccgtctgctgcatgagggcgtgccgcgtgcactggcccgagtcatcgacaccctgaccttcggcgcgcagaagtacaaagcgcactcgtggcagcatgtcgagaaggcgctcgaacggtatcaggacgcgagctaccgacacgacaacaagcgctgcctcggcgagaagctggacccggagacgggcatccaccaccgggcgcaccacatcatcaacgagctgttcctgttggagctggaactgcgcgaggaggagaaggccagtggcgcagagtaaggcgcgctccatcaaagaggcttgggtgaacatcggcatcggctacagcatcaactacgcagcgaacatcgcgctgcttccggtgctgtggcatcccgagcatccgctgctgtcggcgcacgccatcggcattgcgttcacagcgatcagcttcatccgccagtacatcatccgccgctggttcagcaagggtgactgatggcctgcgcccgctgcggccaagtgcatcggtacgtcccacatgaggccgagtgggcgcgcttcctagaggagcaccgtacccgcaagcagttcgatgtcgagtgggccaactcactctggcatcgtacataccctgacgacgcattctgcatcctcgtgatgaggggcctcgcaggtttcgttccattcccgtcgaaggagaactgaatgctctacaagaaccagaccgccatgctcatcaagtcctacgagaacgccgttgcgtggggcgagagtgccgaccacgaggaggcattgcagaatgcggtcaaggccgggttcccgaacctgcccgacgaagatcaggccgagctgtatacccgcatcgccgatgcgtgggaaggctaccgtggttcgctcgctccgcgcaagctgtggatcggcaccatcgtcaaccagttcatgtcgtcccgcatcgcacggttcaacgccgcgctgggtgacggcaccaagaaggaggacagcgccgatgtttgatgtgcctcgccagaatgtccgggttgctcccggctacaagaagcgcaagcgcggcttcaagatcaaccgcgccttcaccaagggcaacttccgcgtgcagtggtacgacggcaaggccacgtactgggagcgctacgttccgtggtacgaagtgccgctcgccatgttccagatttggagggactacgcatgagctacatcgtccacaaggcagtcgagcaggacaagatcaagaagaagctgcggcccaccgaggagcagcttcgcaccgagtacatcgcacagccgaagtacgacggctgcaacatggtcgccatcaagcgcggccactgggtgcccacggtgaacaagggcctgcatgccatcaaggtgggcgacgtgcagatgcagccggtggatcgtggcgtggttgacctgttctcccgcaccggtgagcaggtcgtcagcgcacaccacatcgagaacgctctcgcatccgcgccgttcttcccggtcggcgtgtacttcggcgaatactggcacccgcagatcgaccagcccaccgtcagcggcatgttccgcaagaaggacggcacgcagtacaccgagccgatgttcgtggtgttcgacttcgtgacgctggaagaatgggagcagggtttcagcgacctcgtgtatcaggagcgcgtcagccgcctgccgagcatgggccacgccatcgccgagggcaccgcgccggtgttctacgccgagtcgcagggcttcctgatcgaccaagagctgggcagcatggaagcggcgaagctgctgtgcgagggcggcgcgtacgacgggctgatcctgcgcaagccgagcggcaagtgggtgaagggcgacaagggaaccaacggcgaagtcgtcaagatcaagccgaccctgacgctggacctgcgtgtgctcggcatcaacgaagcagtcggcgagaagaccggccgcgccgtgtacacggtcgtcgttgacctcggagaaggcaagacgcaggaggttggcagcggcgtgccgcacagcgagagcgagctgcctagcgtgggaggcatcgtggaaatcgaggcgatgtccttcagcaagtacggcctgctgcgcgagccgcgatacaagggcatccgtcacgacaagaaggaggcagacctgtgagcgtcgaggtgcaagcatggcacaacatggagcgcgacacggtggagctgcgcatcagcgttcctttcggcgagtacgccggttccctgtggccgaacgagacgctgcgcgacaaggtgcaggaagcgttcgccaagttccttgacgagcggaggggctgatggacgcgatcactttcgagaagccggagctggacttcagccagtcctcggcatggatgggccgcgtcgaggtttcggtgcgcgcccggtacggtgccgacttgttcggcgctgctgccacgtgcatggccgaggatatcggcggtgaggcgtggccgcacatcatccacgacctgcacatggaaatcatgcgcggtatcctgaaacgctacccgccgcgcgactacaccgtgcggcagcaacggaggtaacaatgctctcgcaagtggaactcgaactggaaacctacgccttcggtaaggagcgcatggagaagtccatcgcccgcaacgaggagaagggcggcgcggacaacaacccctacgcccaagcagtgtatcgccggttcgtgcttccgcttgcggagcgcatccgtgcggacatcgactctccgcgaatcggccgtgcgcaagcgcacgtgccacttctgcgcgccaagtacgatcccgagcgtcagaacaagcgtggacagcccgtcagcgccgaggaacaggcacgcgagtggtacgaggctgtggccttcgtcgccgttcgcggtgcccttacctcctgcatgcgagacaagcacggcgaaggcagcgaccgcgacgtgttgaagaacgttggcatcaacgtgtaccatgagtacctgctgacgcagttcgccgacgcggagccgactctgttctaccacctgatgaacgacatggaccgcaagctctctgtcaacgagaaccaccgcatgacggtgatgaagatgcaaggacgcaagaacggcatcgagttcgtggagtggggacaggcacagcgcgatcaggtcggcgcgtacctgtgcgatcagcttgcgcagctgggcatgttggagattggcgtggtcaccgagactgctgccagtgcaggcgcagcgtaccgcaagttccagaccaagacgcacgtcaagatcgtgctgaccgacgaggtgcgcaagctgattactcagatcagcgacttcgtgatcgaggccacgccgttctacctgccgtgcgtcgagccgccgatggactgggtggacatcgacaacggtggattccacacgaaggaaatgcgccgactcaatccgtggatggtgaagacctacgctcagacccgcgacgagtaccgcgctgccgagctgcgcaacgagatggctgcgatcaacgcattgcagcgcgtgccgtggcgcatcaacaagcgactgatggaagctgtgtcggccatcgccaaggtgcacgacatggaggaaatcatttctcagggcgagctgccgaagccgcgcaagccggagtggctgacgaaggacatgaccaaggaaaccatgtcccacaatcaggagttggagttcaagcagtggaagcgcgacatgtccaactggcacaccgacgagcgcctgcgacagaacaagggcaatcgtttctacaacgcaatgaaggtggcgcgcaagttcgccgagtacccgagcatctacttcgtgtacttcgctgacttccgtggccgcaagtacgttcagaccaccggcgtgtcgccgcagggttcggacttgcagaaggcgctcttggagttcgccgatggcaagccgctgctgactaaggacgcgaaggattggttctgcatcacaggagcaaaccgatggggatacgacaaggcgtctctgccggatcgtgtgaagtgggtagcggagcatcacgaccagatcatggcgttcgctgcggacccggtgaacaacgacgagtggaagaccgccgacaagccgctgcaatttctgagctggtgcatggagtacgagcagtggcaagtgttcggggatcgcttcctgagccgcatcgcagtcggcatggacggttcgtgcaatgggcttcagaacttctcggcgatgctgcgcgacgcagcaggcggcgtggcgacgaacctgatcccagcaccgctgccgaatgacatctaccagatggtggcagaccgcgtgactgccgtcctgctaggcgaggacgaggatgccgaagggtaccgcacgctgtggctcgaccacggcctcacacgctcgctggtgaagcgcagcgtgatgaccctgccgtacggctcgcggcagtcctcgtgggcggacttcatcatcgaagactacctgaagtgtgggaagttcccctcgctcgacaaggccctgtacggccccgcagcgcgcttcctgagcaagcgcatgggtgaggccatcgccgacaccgtggtcgccgcagcgggcgcgatggagtggttgcagcgcggctccgggtcgatcctcaaccaagggtacgaccgcatccggtggatcacgccgtccgggttcccggtggtgcaggtctactgggagtccgaggagcaccgcatcaacaccaagctgtgcggcaacgccaagctgtccctgcgcaagagcacggacgcggtgaagaagtcccggcaccgcaacggcatcgccccgaacttcgtgcacagcctcgacgcaagccacctgacgctggtggtcaacgcggccaaggccgaaggcatcgacgccttcgccatgattcacgacgacttcggcacccacgccgccgacagcgcggcactgtaccggatcatccgggaggtgttcgtgtcgatgtacgagcggcacgacgtgctgtcggccttccactcggcctacccgttcctgccggagccgccgccgatgggcgagctggaccttcggcaagtccttgattctccgtacttcttcagctgacggagtttcagtacacctatagcacgaggcaactgaggtccggttggagcggccgcgaaggtaagcggaaccggtgccggaccttttggtacacctatagcacagaggagacaccatggccgaagacgccaaagtgaaagtcctgatgacgctccacccgaaccagctggccgccgtgcggaagctgtccgggctgtcgctgtccgtcaactcgaataccacgcccttggaggcaggtatgcagttggggatggcccgcgtcctgaacatcttacaggagggtttcaccgttgattcctccgtaccgaacaccaacgacgggtgatagtgagcagatcaaggcggctttaacggccgctttgtatctgtcatctagagaagatagtaaggtagacaacagagaatcttctgtgagctacaactgtgatgaccctgattacacagtggccctgataacacagggtctagtggatgcagtaatcattgatgaagcctacctgctgtgctttgccattgtcacaccgtggtactccaagaaccgtactacgttcgttgagaacatggtgctgcgaattgggccgggcagttccttcgaccggtacatagccgtgatggaacatctggctgacatcaaccactgcgactcactgagcgcaggcggtgcactagctcggaactcccgagcactcacacggatgtatgcacgctacggctacctgctggaacggcatgctccccaattcaccaagcgaaggagttaacctatgggtagcatcgttggtggtgggtccgccaagcgagcagcgctgaagcaagctgctgctatcgacaagcagaccaacctccaaactcaatccacgaactaccagattcaggcgatggccgatcagatggcacaggcagctgcacagcaggccgcatctgagtacgccgagaagttgctgagtgcccccgtcgataccgtcgatgtgcggctgggaacttccgacctcgacttgcagactgccgacctgatcggccgacgcaagaccgcccgctccacttacacccgacccgtgaccacgaccgcagcttcccggctgacgaccgtggccgggtcagacctgttgtgaggtgagcatggaccatccgatccaaaccgctcaccgccagttcgaggcttacgacaacaagcgacagggcatcatgtaccgactcgaacgctattcgagctggaccgtgcccaagctgttccctcgcaagaaccgcgatcaggacaccgagccgctgacccacgggttccagtctctcggcgcgcaggcagtgaaccatctggcgaacaagctgatgatgtcgctgttcgcaccgtcccgcccgttcttccggttggagctgaagcgcaaggcgaagcaggctgcgcaggagcaaggcgctgacttgcaggccatgcaggcgatgcttgcgaaggccgagcaggatgccagtctcgaactggacaagcgctccatccgctcccggctgtacgacctgctgaagatgctgatcgtgctgggcaacgccctcatggtgttggagaaggacacgatccgcgtgctcaacatgcggcactacgtggtcaagcgcacccgcaccggcgaggtctacgaactgatccttcgggagaaggtgcacaagacccagctggaacccgcagcgctcgctgccattgtcgcgcacccggacttcaagcccgatgacgacggcatggtgtgggagtacaagtgggtcaagctggaccacaagaccggcaagtacaacgaagacgtgtggatttgcaactgcaagctgcccgccaacttctcctcgacctacaccgcagacaagctgccctaccgggcggttagctgggacttggccgcaggcgatgactacggctccggcttggtcgaagactacgaggccgacttccagtcgctctcgatgctgtccgaggccgcagtgcagggcgcgatcctcgcctccgagttccggtggctggttaaccccgcaggtcagacctccgtcgaggacttcatggcgtcgcccaatggcgcggccattcccggcatgaagggtgacatcgagctgattaacgcaggcgtcgatggcgtgctgcaaaccaaccaagcaatccagtccacctacatcaaccgcatcggcgcaggcttcctgttgcagacggcggtgactcgtcaggcggaacgtgtgaccgcgcaggaaatccgcatggtcgccgaagaactggaaggcgggctgggtggcggctactcccggatcgctgcggacgtgcaggtaccagtcgccttttgggtgatgaacctgacgggccgcgacatccgaggcaaggacttggagcctgtcatcatcaccggcttggccgcgctctcccgtacgggtgaccgtgaccggctgttggagttcggcagcaacctcgccaacgtcctcgcactgccgccgcagattctcgaacgactgaagctgtccgcgtggatcgcagacctcgccgccgctggtggcttggacccgaacgtctacgtgctgactgaggccgagtacggccagatgatgcagcagcgtgcacagcagcagctcgccatgcagaacgcatcccagcagatcgacaacgccaacaacatggagacacagacacaatgagttccaacgcacctccgggcggtggtcccggcgcaaccgtgatcgcaacctcgaacggcaaccagcccgcaccggcagctccggctcccgcagacgacaagctgttgcccaacggccagcccgctccggccgcaccggcacagcccgcagctcctgctgcacctccggctgctgacgcgctgagtctcgaacctgccgctcccgcacagcccgccgccccggcgaacgctgcgccgactgcggtgtcgatcccggactacggcgacaacggcctgaacatcgcggccgaatacttcgtcaacaccgtgggcctcgacatcgacagccgcgaactgaccgaagcagcgaagggcaacttcgccctgctggaagccaagctggaagtcctcggcgacaaggccaagggttccgcaccgatcctcgctctggcgaaggagagcatcgctcgtgtcaccgccgctgcaaccgcagcgcacgccgcgaacgttgctgctgtccacgaagccgtgggtggcgcagagaactgggctgcgatccagcagttcgcacgggccaacctgcccgccgaccaactgaagcaggcaagcgaatcgctgtcggctggtggcttcggcgctcaggcgaccgcgcgttacctgatggctctggcacaggccaatcccgcgacgaccgtcaagggcgcaccggctaccaacgccgccgcccccgccgcgtcgatcaacggcgtcgctcctatcacgaaggagcagtaccgcgctgagtaccgcaagctggttgccgagaagggcatccgtggtgcggcccactccgaagaactgcgtgcactcaacgcgcgcgtcatccactaagaccaaggagcaacacaaagcatgagcaccatcttcccgactgtcccggttctgccgaatcaggtcaaccagtccggcaacgagaacgccctgatcctcgaacagttcaccggcgatgtcgagcacacctacgtgtccagctcggtgctggaaaagttcttcccgcgcaagcaggtcaagggcaccaacaccctgaccaagaaggccatcggccgtaccaagcttcagaagctgaagcgcggtgacgcgccggacggcaccccggtggacttcagcaaggcgtcggtgaccgtcgataccatgctgctgtcgcgtcacagcatctggcagctggacgaaatcttcaccgacatcgacacccgcaaggaaatcgccatcgagcagggtcaggaaatcgccgagttcgtggacctgaccatcagcatcgccgccgcgaaggccgctgctgccacgcagtcgatcttcacccgcaacggccgcgcgcccgagggccacttcggtgccacgcaggtcgtgctgtccgccgctggtgacgagaacgatccggccaaggtgtacgccgccatcggcaaactgttctcccgcatggaggaggagaagaaggtcaagccgcagcgcgatggcgtggtcctgatcgtgcgcccggcgatcttctacctgttgcagcaggccgagcagatcagcaacggcgagtacctgacctcggacggcaacaagctgaccggcatcccgaccttccacggctggggcgtcccggtgctgtcgagcgagaacctgccgaacaccgtgatcgaaggtcacctgctgtcgaacgacgacaacgacgacttctacgacggcgacttcagcaccctgatcgccgtggccgtgtcgccgaaggccctgctgatcgccgaagcgctgccgttgcagtcctcggtgtggtggagcgatgcctcgaagtgctacttcgtggactcgtggatgtccttcgccgttggtctggatcgcgtcgagaacgcgggccgcatcgacaaggttgcctaatccgctgggcgcggtccctgaatccttcgggtaactcaaaccgcgcccttcttccaccaacacaggagcaacatcatggtctttgaccgaccgttcgagatttccaaccgcgtcgtcgccgcaactggcgtggccggtctgcccgccaactccgttggtaccgtcgtcggcgtccactacgacacccgtggcaccgcaggctgggtcgtccgtgtccgtttcgtggacgacgaaatcggctcgcaggacatcgagtacgcaccggccgctctggctctggctgcggactaagcaacatcccggcaggggcgctccggcgtctctgccttgttcctctcaggagacaccatggcattcatcaccaagctcgacatcgtgaacgcctgcttgaagacgatgggcgagacgaagctcaacacgctggaagatgaccacgtatacaaggacgacgccgttgacttgatcgaccgcgtgcaccgtgacgtgtcctcactctcgctgtggttcaacaccgaatgggtggagctgaagccgcaggcaacgagcaagtacatcatggtccccacggacgtgctgaagctggactgcaacccgagccggttcggccacgtggtgcagcgcggacgccgactgtacgaccgcaagcgcaacacctacgagttcgaccacaacgtgcaggccaagctggtgcggctgctggacttcgatgacctcccctacgaggtgcagatgttcgtgcgcgacgactcggtgctgcggttccagtctgacttcgacggcgacaacaccaagtacgccaagatcaagcagcagcgcgatgacagttacatcaacttgaaggccgagcacatccgccagatcaaggcgaacccgctgttcgctcgcgcatccgtggacgtgctgcgttcccgttactggaactacagcggtcacccgtggcacagccacgtcacattccccggctaaggagacaacatggcaaaggcaggcggaacctatcccgacatccttcagggtgtcagtcagaaaccggcgcatcgtcgtcggccgggacagacgcacgagcagatcaacgtgctgtccgatccggtgaacggcctcgtgcgccgtcgtggtacgcggttcgctgcttcccaagccgttgtcacctcggccgagctgcgcaacatggacgtgttcgacttcatgcaggagggcaaggagtacgcgctgctgtaccggcgcgacgcctcgaccttgggcagcgagtccttcgcgttcctctacaacaagacggacgagtcgttcatccctctggtgtacgagaacagcacgtgggtcaacacgctggtcagcggaggcgcatcgtcgctcacggccatcggcagctacgtctacatcgcgggcaacaccacgatcccctcggccaccagcacgaacgtgtggcaggagcagacgaacatccagcgcctcgcagcatgggtgcgcaccgggaagtacaacaccacgtacacggtgaacctgacgcggacggacaacacggtgctgacggtaacgttcaagacggttaccgcatcgtaccccggaacgctcgacaccagcgacatcccgttctaccttcccggtggcacggagccggacgcggcgtaccagaagtacgtcaacgaccgagtgaacgagtacaactctgcggtcaacgagtggatcgtgacgagcgctgagcagacgcgcccggagtacatcgcggagcagctgtcggatttgctggtcgatgcaggcgtgtcggcaacgtacatcaagggcgggatcatcattgacgatgaccagttcaaggacatcacggttgacgacgagggagacggcacgaccttctacgccgcagggcaggaaattacagacgcgacctacgccgtcaagttccactggcacggcaaggtcattcgcgtgcggccgagtggtgcaggcgcggacgagtcgtactacctgcgcgctgagttggagaacggcgagacttccggctacgggtcggtggactggtacgaagcgcccggcgtggagtgcaccatcgacaacctcgtgtcgcagctctacatctacaacggtgtaggctacatcgcacgcaacggtgcgggcctcacgtctctggctccgagcagcggcgagcatccggcctacggtgcgcgagtggcaggcgatggtctgacctcgccgatcccgtggttcatcgacaagccgatcacgatgctgtccgtcttccaagaccggctggtcatcggcgcacagaactacgtcaacgcctcacgctcggcggactacctgaacttctggcgcggctcggccgtcaccatcgaagacagcgaccccatcgaaatcttcgcgcacggcagcgagggcgatgtgctccggcacgcgacgctctacaacggcaacctcgtgatcttcggtgaccgtcagcagtacggcatcagcggcgactcggtgttcagtccgaagaatccgctgattaaagcgttcagtgccaacaaggattcggttgacgcgaaggcgcagacctcgggcaactacatcttttatgcgcagtacggcagcgaaggcacgagcctgcaccagatgcgagtgggcgcgctcaacgggcagcagacggtgacggacgaaatgtccaacgagctggactcgtggctgtcgggcactccgttgcagatcaccccgctcactgcgccgaacctcgtcatgttccgcactcgcgagcacccgcaggacttctacctgtaccggtacgaggacaacaagaacaacgggcagcgcatcgtggatgcgtggtcgaagttccggtaccacccggcgctgggcgaaatcatcggcgtgagcagctacaagaagaacggcctcgtgttcactgcgcgcgggtcgctggtggcgtgcgacgtgttcgacccgaagggcgagccggactcgcatgcgtgcctcgacagctgggcgagttttggtacacctacgggcgtacagactgcgagcgcaagcatcgccgtcaatagcactagcccgtacttcctgctgggttgtccctacgcgcaggcgtctgacttccttaaccagttcgatgacctcgctgctggtgcgctggaatacggcgtggtgtccgaagctctggtgatcccgaccaatccgttccctcgggaccagaacggtcaggccgtactcgatggacgcatgtccctcaacaaggtgacggtggacgtggagaacacggcaggcatgatcgccacggtggcaacccgcaacagcaatgtgaccactacggacttcgagggccgcatcctcggcgactccgacaatctgatcgcgcggcaaccggtgtaccgggggcagctcaacatcagcgtcgggcgcgaagtgcgcgagtgcacctacgagattcgcagcaaggattggctcccgctccgggtgaccggcctgagctggacgggtcagactttcaacaatgtacggagggttagctaatgggttcggttaatacgatcctgcaagcgaacaacaccacccgcgttgcccgtgcgaactaccgtgcagccgttgcgcagaccgacaaccagaaccgcagcgaggtcgccaagaccggcttcgctgatttcatgcggtccctgaagaacaacgcccaactggacgccgccgcgaaggagtacaactccaacatggaagcgctgtccgaggagctgcgtgcgcgccaaggggctgggcttaactcccagctccaactggcgaacgcgcgtggcgcacttcaggcgcaggctggtgctgtcggtgtcggcggctcgtccgcagacctgatggattcgatggtgcggttgcaggcggaaatggatcaggagacgcaggccaacgctgtctcgctcctcgcctcgcggggcgcatcgcagactgcgcagatcatgtcgcgcgcgtggaacgggatggacatgagccgttcgttcgggcagttcgactactcgcagcacatcgagccgcaggcaatgaagcgtcgcttgggcaagctgatcggcgtggccgtggctacctacttcggtgggccgatggcaggcgaggccgtggcagacttcgcggtcggcacgtggcaggcggacaacggcaacttcactggtgcctctcagtccttcagcaacgcagcgcagaacggtatgcaggcgtggcagcagtccaatgatcgcggcggcaagtcgtgggcgtccactaccttcgggtacaacgacggcaccggcaagcagtccgtgactggggcgaaggtcaccggcaacttcggcaacaactacgacaacttctccaccactacgtccggcctcggctggttcgatagcggcagcggaggcaactcaggaggtgcatggtaatggctgacatcggcacggttaccttcaacacgcagtccgcattgcagggtggcatcaacgccaccccagcactgtcgggcaacaccagcattcaaggcgctggtgtgaatcaggtcgggccggttcaatccggcaacgactggttcgcaagcactggtggtatgacgatgccggacagcaacctgccagagttcttgcaggagctggcagcgccgaacaccgccaagctgaagcagcagcagatgtgggacggcttcgttgccgcccgcgctggtaagaccatggacgagattgctgcgaccgaaccgtggtacaagaaaatcttcggagacaccaactacgagattggcgcgagcatgtataacacgctctcgcaggtcaacgaaatggagagcgacttgcttcggcgtatgccggagttgcgtcagcttcctcccgaggcgatggcgaaggagttcaacgacctcgccactgcccgcatgaccggcaacggtttcgcggacacggtgttgcagaagaccttcatggatcgcgcgggttccctcatggacctgcacaccaaggagcgcacggcatggcagcagcaggagctggtgaaggcgcagtacgctgcgaactcgtcggcgtccaccggcttcaacgaactggcgaagcgcacggcgatgctcggtaccaaccgtcccatggacgagaaggccaccgaggcgctgacgcaggcgcagctgtccctgctggacggactgtcgccctcgcgctaccagacggacgagtcgtacaagtccgcgatcactgcgttctatcgtggcgctgcggatcgcggcgagttccacacgctgaagttcctcaacagcaagggcgttctgaacgccatcgacccggacgggcagctgggaatccagcagtacgtgaagcaggcgcaggatcgttaccgttccgactggctcgatgccaacccggagcaggccgagaagatggcgctcgtctccatgtacgcatcggagggcattggtgccaagccgtcgcaggcgatgatcgaggaaatgaactcgacctacgccgccgagactggaagcgacgcaccgctgtactccggtacgcagttggcttcgatcatggcacagtccgcaggcgcgcacatccgcgcacaggaagccgtcatcaaccagcgtaacgctgcggccaaggccgcgctgaccgaccagcagaagctggccgcgcaggaggaggacatccgtggtggcatcgaagcgttcaagcgcggcacgtacgcgcagacgatcaacatccccggcgtggacaaggagctgatcgaggcgaacacggtgcaggcatggaatgccacgatggccgcgaaccccaaggtcgccatgtcgcagctggtgtggaacgccaacaccgggcgaggcgctgtgctgaagggtgtggccgaccagttccagaccacggcgcgcgctgtgctccgcgatcagccgaacacggcagcggctgcactgtaccagcagtggaaggaactgaagcagaccaccgccgcacgcatcgacacgaacggtcagcccgtgcagggccgactgactggcgcgactaccgctgcgctgtacttcggagatagcgtcaacacgttcttcaacaagctgcaagcgttggagaatggtggcgtgaacttcgagcttgcttacgaggtggcccgtggagaaatcaccaccgacgatccgacgcagttcgacgcgaacagccgtaaggaatccgaggctactcaggctcgtgttacggaagctatcgccaagctcaaccccaagtacctcggcatgttcggcaacaagctgggcgactctggccgcgctgcgtatgctcgcgccatcgtccgctcggtcactgacaccggtggtctgctggacacttctgcggaaggcttgcaggctgcggctactcacgccaagctggcctacggtctggaagacgcaggcaagtacgcatgggaaaacggacgcgacgacgaaggccgagtgatcggcagcgtcggtgcatggctgggcttcatggacacgaaggaaaccggacccgccatcgagaaggccatcgacgcagcactgcgccgggtcaacatcgagccgagcaccgggctgaaggctgacgtgttccgcatgaaggacagcgagaacggcgagccggtgctgtacgtcaacgctgttggcgagaagggctggaaggttgtgccggtgtacgggcgcgacatcaaggacgagtacgagaagcacaccaagcagcagcgtcagttgcaggccccggtaccgcagggctacgttcgcatgaacgacggtacgattcagcagagcatttccatccaacccaaactgtaaggagatagacaatggcactcgatctttcggggctgacccaagaccagcagattgccaaggctgccgcttatgcgggagtgccggagtccatcgtgcgcggtcagtggcgagtagagtccggcaacgggcgtgccgccaaggacgctgacggtgtgatccgcagcaaggcaggagcacagggcgacttccaagtcatgcccaccacgcaggcaacgtgggaagcgcgcaacggtcgcaagtacgacatgcgcaacttccaagacagcatcgagctgtatgccgacatcatgcgcgagaacatgcagcttgccaagggcgacgtgacgaaggcgctgcgcatctaccaaggcggcaccaatccgaagaactgggggcaggagaacgcagcctatgcaccgagcgtgctgggcggtgcgtccgctcccgcagtgtcggcgcagccgcgcagcctgaccaccacgcaggcagacctcaacgccgcatggcagggcaacccgaacatgcgcgaccgtacgtggtccggtgcgtccatcccggatgcgtggacgggtgcgcccatcgaaggccgcaacgctctggcgtcggcagcgaaggaacacatcggcaagattcgtgcgggcatcgccgagctgtcgatgggtcaggtagcacaggaaggtggcaccgccgcgcaggccgtaggcaaggctcaggctgtccgtgcatcggatcaggttgtgccgtggtgggtgcgtcaggaagtggacgtgctgaacaccggcgctcgcaaggcgctgctggatcagaccgaacaggcgctcgcgcaggaccgcgcggacgaggagctgcgcaactcgctgaccttcctcgacaagtggggcgctgcgttcgacagcggcatcggtgctgcgatcagcaaccagtttgcgcgcgaggacgagaacgttccggaaggttggaagtacgacccgaaggaatgggagaagccgtggatgactgccgacgaactcgaagacatccgcgatgcagcgtactcgccgaacgagctgaagtacgtcagcgaccgacagttcctgcgccgccactccatgcgcatcaaggatcagcagactggctggggtagcttcggttacgacatggtggcaggcttcaccgatccgggcaactgggctatcggcggcgtcactgccgcaggcgctaaggcgctgggcatcggctcggctgcactcgttgccgaagggcgcgtgggcgcgtcgctcgcgtcggctgctgcggagaacgcggtcggttccgtcatcacggacgccgcgctggttggcatgggcgagcgccgcaacttcgcggacttcatgaccgacgctgcattcgctaccaccataggcaccgcgatgcacattccgggcgtgcgctcggctgcgcagattcgtgacaaggcaaccatcgacctgtccgcaggcaacgctgccgcttacggcgaagcgtggtcggccgacctgaaggcgcgcgctgtggccgagctgggcgaggacgccaacccggtgctggtgaacaaccgcatccaccagcttgccaagcaggaggctgtggattggctgcgcgctggtatggccgacgtgcctgacgacttccgtatcttcgcccgtcccgacgtgcaggagacgaccaccaccgcaggcaccactggtgcactcgcacgggacgcgggcaacgtggacgcaacgaccgggcggtacaacgacagcgtgggtggccgggtcgatcagcatgacccgctgctggaacgcgcatggaagaccgcaggtatcaagggcggtaacgtcgatggcgtgctgaagtatctggaatccaacgcctctatcccggaggacgtgcgtgctatcgccaacgcgctgaagcgtggcgggcggctgagcacggtgaagatcgtgccggaatcggaactcgacaagtggttcgccggtgccaacatgggtccgggtatgcgtgtggccggtggctacaacgccggactggacgcgatggcgatgcggaactacacgccggaagtggtggtgcacgaaatgctgcacgctgccacgctgcgtgagctgcgcagcaactcggtgttcgggcaggaaatggaagaactgctgacccatatcaacaacagcatcggcagtgtggactccacgctgaccaccgctgcgatggagacgcgcatcaaccagccgcaggcaggcttcctcgccaacactgacgagctgatttcctacggcctgacgaaccgcgctgtgcaggcggtgctgcgtcagatgcccgcgccgggcaacacccgcccgaatgcgtgggagtggctgaaggataagatcgcgcgagtgatgggtctgaagaatcaggagtccgcgctcgaacgcctgatgtcggtcgtcggtgacaacctcggcgcggaagtgcgcgacacgcaggccggtacccggcagacgcgtggcatgctcgccaactcgatcttcaagtcgaaccgcgagcgcaaggctttctaccagcgcaccggtctggacaagtccgtcagtgatgacgcgatgcgtgtgcaggtcgccgaagtgatggcacgctccgaacgcttcagtgcgcagtacggcatcgacgcggcgaagctgtccaccatcatgcagcgcttcgggctggaagctacgagcacgactctaatgtcgtccaagtcgccagttgcccgcatgcttgcgatcaccctgttggagaatcccgagggtgcagcaggccgacacagcaccgcagcgatggatcggcatggtcggtttgagtcgttcatgggcacccgcccgcgtcagtgggaagcggcctatcgcctgtggcgtgcggacgtgcgcggtatcggtgcgatcaaggacttcgccacgggctggaaggctcgcgcggacttcgagtacgcagtgaagctgtaccgcgagactcgcttcaacggcggggacatcccggatgcgcacgaggcagtgaaggcaatggcccgtgagttggaccgtggctacaaccgcatggcagcagagcagcgcgcggccggtacggtgggcgcacagcgtctgccggaggaggacgtggagggctacgagtcccgtacgtggctgggcggcagcatcgctgctgctggtccggtgcgacgcgagggtatccgtcaggcgatgcgcgatcagttcgaggtgatgggcgagctgtatggggacgacttcctcgataagttcgctaccaagtatctggaacgcatcgagcgcaaggctgcgggtgtcatcgaagcgccgggtcaggtcttctcggagtcgcaggcggacacgctgcgcgacactctgcgggcgatgtcgctcaacgaggaggagattcagaaggtcatgggcaagtacagccgtggcggtgcgaagcacaccaaggcgcgtatcgacctcgacgtgaccaagcagtacgaggacgctgacggtaagttccgtctgatggactatctcgacaaccgcgtgatggacaactaccgcaagtacgcgggacgtgttgctggtgacatcgctctggcgaagcacggcatcctcggcgacgcaggcatcaacgtggcgcgcgaagcaatgcgcctgaccggtgccaacgatgtggagctgaaggcgttcgagcaggtgatgtccgagttccttggtcgcccggtcggtaccggcgatccgactgttctggcgaatgcgcgtctgctgacctcggccatccagctgggcggcgcgggcatcaatcaggcagcggagtacagcaacggcctcgccgctgttggtgctgctggtgtggctgacgcaatccgtatcgctccccgcatgcgcagcgaaatcatgcgcatcctgaagggcgaggacagcggcaaccaaatcctcgacggcttcgagttcatcagcggtcgcggcttcggtctcgccggttacgacctacacatgttcaactcgctggacacgcaggcgtcgatgtatggtagcgagcgcgcaggcttcctgacctcgctggtgcagaaggcagcgcatgcgaaccgcatcctctcggggcagcgggccgtgcttgctgtgcagcagcgtggcttcgcggaagtgctgatcgccaagggcgtgaagttcctgcgtgatggtgctgaagctgacaccgccctgaaggacatgggcattgacgacaacctgctgaaccgcctgcgggctacgcaggatcaggtcgtgcgctggggcgcggatggtaagctggaagcagtagacccgcgcaacgtcgaggggctggcggatcggcaggcatggttggcgttctacaacgcgatcaaccgtggcacctcgcagattcttcaggacaccttcatcggcgagactggcaagtgggcgcacaacggctggctgaagctgctgttccagcaccgcacgttctcgctggtcgcgcagcagaagcagctgggccggtacgtgggcaactacggtgcatggcagacggcgggcctgatcgctgctgcgatggctgtggcggctccgctgcaagccctgcgggtgctgtcccgcgtggccctgatgaacgatcaggagcgcgacgaggccatcgaccagaacatcctgtcgcctctggcgctgggcaaggccacgctgaactacgtgtcggcgacgggtatgctcaacgatgtgctggacgtgggcactggcgtggcgggcggctggtacgagtacgccaccgatacgcagggtccgacgtggctgaagcagctggccggtgggcagttcggcaaccgcaaggaagtggtgggcgggcagttcgcgccgtcgctgggagtcatcaacgacttcgctcagggcattgctggcaagccggagaatctggccgacgtgattccgggcgggcgactgccgatggtgatcccgctgctgaagggcgcagccagccagtggaaggaggagtaagatcagggccaaggacggcccacccttttggtacacctatagcaaacaggaggcagcatggcagttccagacccgcagctgcgctacgcgacagacgtgttcgacgccgatggcgtgaccactgactggcagatcagctttaccggtggctacatcaacccgtcccacgtgtacgccatgagcggactgctggacgaggagactcagctgctgaccgaccggactccgcacaccgtggaagtcctgagcgaagacgatgacgctagtaccgtccgagtctcgcctgccgtcgccgctgggcgcaagctctacatctaccgcagcactccggtgcagcagatgctcgttgactacgttaacggtagcatcatcagcaagacaaaccttaacctcagcaacgaccagctcctgaagatcattcaggaaatgttcgactcactcaacatcgccacccttagcatcgaccagcaggtcggtgtgatcgtggacctgaacgagattatccagaacatctacaagcaggtcaccgagttgctggcagctggtggtatcgtgtccgtcgccccgcgcgtctggtccggtgcttggactggcgatcaggtgggtgacaccgacttcgacatggtgggcgcggacgtatccggcgcgggcttctacgacgtgtacgtcaacggcatcggcatgcagccggacgtggactatcaggtcacgctcgctgacggcaccgatcccagcttcatccgcttcgccacggttcctgccgagggcagcatctggttcgccgtgctgcgtggttacgccaagccctacaccgggcctgcgccgatcaccgctgcgagcctgcgggtgccgatcatcacggcagagggtccgacttactacgccgccaaggctaccgagtacggactcgtgcgctgcacgtacgccggaggttgcgccgtcaacatcaacctgatccccgaagtgggcgacggtgaaaccaagctcgcctcgggcagctacttcagcgtgcagcagaaggcaggccctgtggtcatcactggcgacgtgggcgtgacgctcgaagtcccggtcggctgcaccgccgcaactcgcggcaccaactccgtcatcactgcaacgtgcatcgacggcgacaccaacacgtggttgctctcgggcgacttggctaaggagtaagcatggctaatcacttcaggctgtacggccgaccgctcatggcggacgaggttgcagatggcctgtcggtgacgggcgtgctggaagggtacacggcgggcgaggcttacgagtctcgcctgtccatcaacaacccagtcggccgctgcaccgtggaggtcatcgaatcgacgctcccttcgggcgctgcggtacgggtggacaacatcaccaaggaagtcgtcgtcaagtgggcggctttcactgaagtcgtggacgaggaaaccctcgtgcccaacggcgacttcgaggcaggcgacgacggcacgtggttgccgggcggtggatcgaatggcgaaggctggtcgattggcactggctcagactacgacaccgacagcggcgtgtacagcgcgcgcttcgccaacatcaagacgggcggcagcgacctgctcaacccgctgatccctgccaaggtcaacgactacatccgatgcaccgccgaggtccagcagggcgcaagctccaagggcaaggccggtgctcgtgtgtcgatcatctaccgcaaggaggatgggaccgagctgcaacgcaactggggcaacatggtttcctccggcagcaacggtgcgtggcaccagtccgttgccgaaggcgctgcgcccaaggacacgaagtacgtgcaggttgtactgtcggcgttccgcagcaagcagaacaaaccgctgtgggtggacaccgttaagtggaaccacaagtacgtactgggtcagaacgacgacagctcctacttccttagcatcaaggtcacggacgggttgaaccgtgtggcctactggtccggtcgtatcgaggagcagggcatctacgttacgtccaagctctacagcttctaccagttcgatgccgcgatgctgaccagcagctttgctgggtacagcaacatcgacatgctccagcctttggatactgcgtcgctgggttcctccttcgtaagctgggaactccgaagctctaggcaggattatgccgccgacccggagagcacgttgtacgggagcgctttcgtttcgttcgacatccgatccatccgtaaggactacacgcctgacccggagacggcgaagctgtcgagttctttccattccttcaccctgaagcagcaccctgtagtcaaccagccgctcgacgcgactgcacgactccggtctggcttcgtatcatggagcttcgcatgatccacaatcacctcggcattgctggcgtgttcaccatcagcaagggtaagtccctcgatactctcgaagttgtagccgactggcagagcaaccttatcacggacggtggtatggacgcactgggtgataccggcagcggctatcctcgcagcatgtacgacctcattgcttacttggcagtcggtagtggcagcgccaccccggcattcaccgataccgctcttggtgcacaggtggcgcaggttggtcgtacgtcctcggacagcggtgggactaccactgccccgtactacgcctactcccgctgccagtaccagttcccggctggtaccgctactggcgttctgtcggagcttggtgccaaagcatacaacaacaataccggcgcgtacatcctgaccacccgtgcgcttatcaaggactccgcaggtaacccgaccaccatcacggtgctgtcggatgaaatcctcgtggttacttacgagctgcgcatgtacgcagataccacgccggttgtcactactgagacgatcaagggtgttagcaccactgttacctgtaagcctattgcaatgggccgcagcggcggtatgaacggtcagtcggcagtcgcttggtcggactacgtgtgggggtgctactacttctacggcggtactggcgacggcaccggagctatcaccgaccagtatccgccggggacgattgccagcttctctgacttgcagcttcagcaggtagcctatgttccgggtacttactaccgtgactgcgtttgccggatgtcgatcaacaacgtgcccggtggtccgatcacggctgcaatgggactctccgcgtgcgtgaccttccaagtcggcttcaatccgggtatcaccaagaccggatcggagacggcgaacttgcgcatgcgggtttcttggagccggtacacgccatgatccccactgtctcccaaagcatccaacgcggtgactgggtggagcagcagaatcggcgcacccgcccgctcattgacttcgagcagggcgggctgactctcaacgcagcagtggacgacctccaagctgcgctgtggactgccgagagtgacggcagcagcgtcgtcgtttaccgcgacggcgttgccccggtcaccgtgctgaccgactccgggatcacgcagatcgcactggccttcgaccagaccatgcgcccgcacgtggcgtacatggcgggcggtgtgtgcaagttctactggtacgacacggtggctgcttcgatgcagaccatggtgatccccggtgctaccactccgcgcctgtgcatggacgagaagcgggctgtcttcgccacgcagagcgacgtgctcctgtcgtacaagaacggcagcaacctgtgcgtacgcgcgcagcgtgagcgcttcgcaaccgaacatgtgatcgcctcgggaatccccggcgacctgattgcggtgggcatgaacaacgtcaaccgcctgcaatggaagctcgtcggcaatcccgacgactggccctaacctacaggagaacagcatgaccccgccgagtgtggtcaatgaggtcgtccgaacctcgccgcttacgctcggcgcggtctacctcaacttcatcagcacgtacggtgctgccatcgtaactacgctcgccattctgtacgccgtcgctcagttctactggcgggcacgcgagcaccgaaagatcatgggaggcaaggatgtcgaatccggcaagtgagggcgcactcggtgcgctgcacgaactggtcgcgcgtgcgctgatgcagcgcatccaagatggcgagctgtgcaccgcagccgacatcaatgcggcgatcaagttcctgaaggacaacaacatcacggcgacgcgcgaggccaacaaggcactcggcgagctggaagacgagctgggcaagcactcgctgcctccggctgacgacgacgagttgcagcgtgcactcgacaacatcgttcactttccggggagcgtagccaacaatgcgtgaatcagctgaagcggccgacgtgcgccgcaagaagttggagctgttgcagaaccactaccggcacttcgccaccttcatgcgcgacattatgaaggtgctggggttcgagccgacgtggatgcagtacgacatcgccaactacatgcagtatggcccgcacctcgcaatggtgcaggcgcagcgaggcgaggcgaagtccaccatcgctgccatctacgccgtcttctgcctgatccacgatcccactcaccgtgtgctgatcgtatcggcaggcggcacgcaggcatccgagattgctacgctgattcagcgcatcatcctcacggtgccgacgttggagtgcatccgcccggacaagaacgcgggcgaccgtacctccgtggatgcgttcgacgtgcaccactcgctgaagggaatcgacaagtccccgagcgtggcgtgcatcggcgtcaccggcaacctgccgggtaagcgtgcggacctgctgatcgccgacgacgtggagtccaacaagaacagccgcactgccgcgaaccgtgagctgctgctgaccatcacgttggagttctcggccatctgcaccggcaagcccggtactccgggtcgcatcctgtacctcggcacgccgcagaccggcgactccatctacaacaccctgcccggacgtggctacgacgttcgcatctggcccggtcgctacccgaccccggcacagcgcgagcactacggcccgcatctggcaccgtctatcgtgcagcgcctagaagccgacccgatgttggcgttcggtggtggcccgatgggcgacgagggccagtgcaccgacgagctgttggccggtgagcagaagcaccagtccgagctgcgtcagcgtggaccgtccagctatcagctgaactacatgctcaacacgcggctgatggatgcgctgcgcttcccgctgaagaccgagaacctgatcgtgatccccggtggtggcgaccgcttcccgctgacgatcacccgtggcctgagcaacgctcaccagcgcagcttccagtccagtgggtacggcttcgtgatgatgatgccgcacgacatgagcaccgagactgcccccgtgcagggcgtgcacatgcagatcgacccggccggtggtggtgccaacggagacgagacggccttcgccgtgaccgccttcctcaactccaccgtgtacgtgttggccgtgggagctgtgcccggtggctacgacggtgatggcttgctagaactgcgccgcattgcggtgaagtacaagccgaacgtcatcagcatcgaaaagaacatgggctacggcgcgttcgccaaggtgttcctgcctgtcctgcgagaagatcgcggcacggagaagggatacaagggcgacatccgcgaggagttcgtgaccggcaacaaggaagcccgtatcatcggcactctcgaacctgtcatggctcgcggctcgctggtcatgctggaatccgtggttgaaatggatcacgagtacacccagcgctacgccaccagcggcaagcgtcaggtctacagcctgttccaccagatggcgaagatcacgcagcagaagggcagcatcgcacacgatgaccggctcgatgcactggaaggtagcgtgcgtcactgggttgcgcagcttgcactggaccagaacaaggccatcgccaagcagcagcagcgagagttccaagactggatcaacgatccgaccggcatgaaggcagcgacccgcaagagtccgctgcaacgtggccgtccatccctactcgaccgttaccggaggtaaccaatgcagaagtccgacttcaccagcaactacacgggtctgttcggccgtggcaactacctgcaccgcgaactgctcgccctcatggagcacgcagagcagcatcccgcaaccgcagcgcagctgctcgcgcagttccagaaggacgccaccctcgtgctggacgccctgatcgctgcgggcgcacgcaccgcgtcctcgggtccgaactccggcccgcacactccggtcgatctggacccggatgacgacccactgaccccgtaaggagcaaccatgaaccagcagcagaaccaagataccagcaacaaggggctgttcggcctgatcggcggcatcttcatcggcatttcggcaacgctgctgtcattcacccaaggccacgaaggggtacgctacgctgcgtacctcgacaccggccgggtgccgaccatctgctacggccacaccaagggcgtagcgatgggcatgacggcaacgaaggcacagtgcgacaagtggctgatcgaagacctacagatcgcccagcagggcgtgcgcaagcacctgaaggcccccgttaaccgcaaccagatcgacgcctacacagacttcgtgttcaacgtaggtgagaaggcgttcgccgacagcaccatgctgcgcaaagcgaacgcaggggatcgtgaaggtagctgcaaggagttcctgcgctgggtctacgtcggtaagctcgactgccgactgtccagcagccgttgctccggcatccccaagcgccgcgacgcagagtttgctctgtgcttgcgccccaacaacgaggtgatccaaccgtggaaaccccaagtgaagtgatcgcgcggctcggcggcaagctggttggcttgctgctggtcgtgaccatgttcgtgtgcttcggtctgtacgtctacggcctgcaacgcaaggtggagaagctggaaactgcccaagtcggcacgaccgctaccgccaaggcggcgcagacgcaggctaccgggtacgcgacctacatcaaagagaaggaggacgtgcgtgttcgcactgaagaagttcttgacgctgccccggagtaccgggatggcactgttcctgctgatgtcgctgacctcctgcgcgaacctgccggtccctgacgactccctgcttgcagactgccacatcacctacctcggtggggagaagggcaccacctcctcgcaggacaaggtggtcaagctcgcgcaggaccgccgcatggacaccgttctgtgcaacaaggacaaggctgcgctgcgtgcgtggaaggccgaggtgtgcggtaccggtaagcgccggtgtacgggtgacaaatgaccaccatcgcatgggacggcaagcacctgtgggccgatagtcaggccacgcagggcgaccacaagcacaccgtgcgtaagatcatgcccgtatcgacacccaccggccctgtgctgctgggtgtcaccggggatttcacagtgcttcgcccggttctcgctgcgcttaaagcgggcgaaggctacgaggagcacgttggcaagtccgcgacggtgcttgtggttaaggacggcgtactcacggtcactactggtaagcagcagtgggtcgaggaggctccgtacttcgatggcagtggcaaggcgctagctctaggggcctatcatgcgagcaagtctgtggctaaggccatggctgctgcgatagctcacgatgtctacagctccgggcctatcgtcaagctaaaggcaccagttcgcgaggcttaggagtaaggccacgtgggtagccggaccaaaatttgcttcggaaatgcgcgggggtcactccaatagaagctcccgcgcgtgcccccgtacgccctcgcgttacgcgcctgcgggtgtgcgtgggtgcgtgcccgcgtgtgcgcctgtgtgcgcgtctgtgcgcccgcgtcaaggttccgcgtgggtgtacccgtgtgcctgcctgcgtgggcctgagcgtgcgtgtgcgtggccgtgcgtgggtgcctgcgggtgggcgtgcgggtgggcgtgcgggtgggcgtgcgcctgctgcctgtatggctggacc

SEQ ID NO: 9 - DNA, 44415 bp, unidentified
  source 1..44415: mol_type = genomic DNA
ctgcttgtccttgatgttgcggcgcttgcagatggtggtggcctcgaccgcgcgctgataccagccggagtcggcggtcaccatgacgttgaacacgccgttgcgcagcgcataccacgtggtgctgtagtcctcgtcctcctcgtagtgtccatcggcaccggagcacagggtccatccctgatcgaccagcttttcgatggcctcgtggaagtcctgcaccagcacgaggaagtcgatgtccgtgtcggtcacgggcggctcgactgtgtagctgctgccggtgcggctggacgtgatgacgcccacgttgcgcggcaggtagatgttcggttcggtactcacggtgtgttacctccgggcttggtgatccagaacgtgaagcacgggatcagattgatgcaccagcgcttgttgtgcggcgagtagtgcacgccgatccaagtgctgtgtttgttccgcagccatccccacttccactgcggcgcgtcgttgcggccttcgatgtagcctgcgtcgtgcaccttgcgcagcagcttggcaaggtggattgcttgcgcgttgctcacgcagttgaaggtcttcgcctcggtggattcaccggggaagctgaccgacaccgtgaacccggtggctacgatgtgaattggcttgctcatgctgcctcctgatagaagcgggcacgctctgcatccatcatcacttcttcccgaacgtcacgcttgccgcctgcgcggtgcagcttgttcttcggggtgccgatgtagcggaagcgttccatcgctgggtcattgagcttgccgcccatgatgatgaagtcgcacgcaccctgcttgccggtcttgctgtccttcagtgcggactgcggcgggtactggattccctcaccctcggcgctgatctgcgaagtcgccacgcccacggcgtcgtacttcacacaccagttgcgagcggcctgatacatcgcctccaacatctgatcggtacgctgcccgccgttggtcatgccaccggtgaacgtgatgttgtcgatcatgtcgaagatgatgaagccggggttggtctgcttgatgatggcctcgacttcaccggagttgaacccgtggatgtcgtagaactgcatgcggtggatgtccccgcccatcgcatcttcgatgcgcttgcggatgctaccatccttcgcccactccaccatctcagggatggtagcgccgagcagcgactgataccaccgctgcttgatgcgcttgcccggcccctcgttgttgagccagatgccggtgcgcttctggtccggccaaacgttgtcgagctgcgtgatccagtggctggactcgctggtcaggaacgtggtcttgcctgcgtcgggacgcatggcgtagatgccgaagtcaccaccacgcagagcgcgcaggttcttcgccaacgtgggcagtcggaagtggatgccgatgtcgtgctcgtccatctgcatcagttcctcgggcgtctcctgcaccagcgggagccgcgccttgcgatccattcggtcggtgatcgtctcggccaagccgtacagctcgtcgcgcaggctgaactcagcgccgccattccactgcacgatcttgctgaccgcagtggtggcaagctccaactccaacagcttctcgatcatgccctgctctgcctcgggcgggaccggctcgcgcatctgcttcagcagaactttgagcagggacttcttgtcgtcgggctgcgtcttccacttgaactccatggcccagccatcgaacacatcgaacggcaagtccttcgtgtccgggaactccttgtagtacgcacgcaacgcatcgagcatcagcacggtcagctcgtccagcccatcacgtggtgcgctgggtaccagccggtcgaacttgccacggttggtgcacaaccgcagcagcgtggtgtcaagactcatcaggttctccttcgggttcgtacttggaatcgagctggtgataccgggtgttgcgcgtctcgaacttgcgcccgccgtccgccacatacagcaccgtcgaggtgtgcacgatgtcgcagtcgccgaggttcggatgcgcaagcacgccgccgagcgtggcacggaagccaacgacgggcgggatgatagcgcgccggtagcgcacgatgggtttgctcattgcagcttctccttgatgtagtcggtcgtgtaatacttcgggtcacgtggtgacgtgatgttcctgtagtccagaccaaacgcacgtagacgcgcagcgattactcgcgcactgtcttggccgggattgctaccgttgcttctacctctgtcgtcatcgagccacgtcgctacacgttggcctcgatcagtcagctgcttcaacactttgttgtgcagcttggtgccgagcaacgaccacgcttcggttaccagtcccaccttgtatgcactgagcgggtcttcgcacagtacgatggtgtcacctgtgcccacgccgtagcgtgcgacaagtccgtctttcggaacgtcaggtgttagccacttcggctgtctcgttgccgaccgggctgtccagtataccacgttgtcgccttcagtgatcggtagtaccacccgcccgatgcttgggcaccagtacagccgcagcttctcgatcatctgaagcgagagtcccatcttgaagaaccacaccttagcgtcgagcggccactcgcgggtgtcgtatacccgtggctctggcaactcaacagtcgcacgcactctgcgttcgctcgtctgctcggcgtggattcgtgcaagcttggcctcgatactctcgtgctcacgcttgaatcctgtgccaccgcacctgaaacagaatgcggtggacttgtcgtgctctcgtgagataagcaagggcgtaccctccccgcactcatgggccacacgtgtgcggccaccaacaggcaggcgctcggcatgtggtagccagtcgttgtcgggaagggtatcgctcatgctatcctcgcttggttattcccagacctcgaagatgtcgtggctggtggcgtacaggacggagccgttgccgtccgtgctgacgatcagacgggagccgtcttcactggtcagcttggacacgacgaacccggtgcccttcggcagcttgttggtctgccgcgtgtcgatcaggtacgcattctggccgggcttcagctcgtcgccacgcttgacgacggccacgctgggtgacggcggggcgaggctcacgactgcccgccttcgccacccgcagccttggcggcagcggcttcggcggcgaggcgctgggcctcggcaacggcggcgtcgatttcttcctgcgccttcagcacttcctcggccgacatcagcagggcgctgctgtcgatcaggttcagctcggcatccagaccttcgccggtctgcaccttcagttgcagcacgcccttgtcgttcttgccggtggcgacgatcacgccggacaggacgcgcttgttcagggcacgaccgaacaggtaggacacggcgtcgcccgccttcagcgcttcgatggcggcgctgttggcctcgacggcatccagcttggcgagcttctcgttcaggccatcgaccttggcctgcgccttggcgatgtcttccagcagctcggcgcgcttggcttcgtagtggctgacggtggtctgctcggtggtgttttcgttcgacatgtagatggttcctcttgacggttgataggatggcccgtacgtgggccagtcgtagcctacccggctcgggttactgaaagatcagctcgctgttgtacccaccgccgccattgtagaagcggcgacgcagcacgctctcctcacccagcaccagcagacggtccacgatggcgcggatggcgctcatgtactggtccaccagctcgctgtgcaagttcaggtcgaagcggatcacggtcaccgcctcgtcgtccagtgcgccggtgtccttgcggacgtacaggccacggccattggtcatggtcgcaccgccgatcagcttcacggcggcggcaatctccggctgcacgttgagcagtcggctgtcgggcacagtcacctcgacccagcttcccatgcgcaggctcatgctgcacctgccagtgcggactgcacgttgggctgcaacgatgcaccggaacgcagctcggcagcacgacgcttcatgcgggagcgcagcttgcgacgctgcttgttgttcccgccgaggctatcggccacgcgcttcagctggttgttgccgacgatgcgggtctgaccctgccccttctgcacggggaagtagtcctgccccagcatcttgcgcaggatcgggttgtcgatgggaatcagcggcacgctgacgtgcaggtgccggctggtgtccggcgcaggcggcggcgtgtcgtcgtcatcgtggcgcggcttcaccgctgcgaccaccttgtccttgacgtacttggccgcagccttgatcttgtccatgaaacccatggttacttcctcctcgttccgaagtgattgaactccaactcatgccacacgtagtacgtggtgccgagcgggtcagtgtctgccttccagttgcgctggtcgcagtagtcgttggctgcgccgaggtcatcgaacgtcagcgagaacccagtggaagccgggccggtgcggaaccggcacagcttgccgtcgtcgtcatggtactggccgacgacaacccacgggccacgacccacgatccagtacagcaggatcaggatgcgcagccagagcttacgcatagtacggctcgacacggtagcccatgttctcgccgcccagcgactcggcattgaacacggcgcgcgctgcatcgcgggtcgggaacagcacgttgtactcgctcttgttgtactcgttgccgtcgatgcgcacggtggcgctcgggtgctggttgtagcagctgacatcggagtcgctgcggtcttcggcgaaggcgtaggtgatacgccaacccagcggcttgcgcaccggcttgcggatgctctcgcccacttcgaggatgtgccagttgaagaacgacccgccgtagctgttgagcacatccgcctcggcacgcacggcggcgcggcggtcgaagatggcgagctggttcgggtacgtgccgtcacgcagcgagtccagcaggctggtggtggcacccttggtgcgcagctcggcgatcaccgcatccagttcctcttgggtcggggtgcggccggtgccattggcgacgacgccagtgatgacgccatcgttgctgttcttggggatcgagacgatgaagtataccttacgcatggtggttctcctgattgacgggtgggatttcgatttcctctatcgagtagagggtgggcaccttctcgtggtgcttgcggtggtgttcgatggcttgctcgcacgcctcgtggctggtgtgatgtccgccgaggatgtaatccccgacagccacacccttcacggtaacgagcggcagcgccttcaccacaaggcgcaggctgacctcacgcataccagcgctccacgctgtgctcatgggtcacgaactctttccactggcgcggctgctcgcacagctggatcggcttgcgctccccactacggatgcgcttgtaagttacggggatcatgcaatgtgccctcctgttgggcgtggttccaaagctacgccctcgttagaaggcgcagcggtagatcacgcgcggctcgggtgccacttcacgcggtagcggcggagacggttcggatcgttgccgacgtgcgaggcgatggcgttgcgtgcagcctgcgcagtggtgaacgtgccgctgagtccgatcacagtggacgtattccaacccagctggtgagggcgccgcgcatgcttggtgaagaactcggcggtgtagaagccgcgatccttctccgggccatcgggagtgccttcgggcaccacacggtacgcatcctcgctgatgccctgcaccttggcccgcgccttcagcatgcggtacgcagcattgcggctgcgctgcggcaggcccagctcacgcacctgcgcccagttggcgagggcgatgctgccgtggcgcagattgaactgcacgatccagcccttggtcttcgtcttgttgaccagcccggtctgcgatgcagtcagggcgacgtggcgtgcgctctggtcgtccatcaggacatccggcagcttacgcggcaggttgtcgggcattgccaggccgggcaacaccatgcggccggtcacgctgccgaggaagtccagctgcgaggcatccaacaccaccggaggcaacggagacagcaggcacgccatcacccgcgcctcgatagcagcgaagtcaagttcacgcatgccgtagcccacggtgaacgtcggcggtgcgatcaggtcgcgcagcagctgtgcctcgacatcgctgtcacggcaggccgcaatcacgtcgtcctcgaattgcaggatggcgtcacgctcgaagctctcgacaccgaagtcgcgcagctcaccgtgcagcacggcgaactcattggacagcttgcggttggagtacgggtctgcctttgcggtcagtgcacaggcgatgtgaagggccgagcgcagcagggatgcttcgcgctgggtcactcgaaggttgatcttgggttccatgttacacgttctccttcttcttggtgggcttcggcacagcgcgggcagcgttgatgacggcctgttcctcctcggtcggcacgtagccttcctcggtcgccttttccagacggcccagcagcttgtgcaggtcggcggcgaacgagaacgcctctgcgggcttctcggtcttgaagtcgtaccacgccttcgcggcggcacgttccagcacgtcggccagagcttcgccctcgactcgcttgctcttggcaaacttcatgggcgcgctcgccttggtttccttgtcgtcgttcggagccatcgggccgaactcggacaggtacaggcgcagggcttcatgcttcatgccgttgcccacggcgagacacagatcggaagcgagcgtaacgtcgccgtggatgtgtgcgtggttgatgaccgcaatcgcggcctgctgaatctggtccaccagcttggtgcgggcggtgttgatcgacttgatggcgcgcttgatgtcagcgcttccggtgatgatgtccatggtggttcccttcaggttgggtccgtgccgattgcacgacactaggccctcttgcgaaggcccagtagcttgcatttaagcgagtcggatgtcgaatgaacgcccaccgcacggcaggacgtagagcgccgacacagagccggccggatgcttcatgatggcccgattgtaggaatcgcgggcagcttccacgtagtggcgagagaacttgaaccggatcacaggtaagccctcctgtcagcggcgtggttcgcccggttcgtcccgctgttaccctcgacaacaaacacagatcgctttccggcggttccgtggcgggcttcgtagcgctcggcttggcgcttgcgctcggcaagcttgcggtcatgctccgtggtgcgcaggtccatcacgcttgccgtccgggtgaactggcagaagcggcgcttacgctgggtgcggtcgagattggcattgatcgagccttgcatgttgtgcctccattggcactggtgggaaaactaacagattgatgcgccctcagaaagccgtcgagtcggtcaatccctcattctcgattagagccgttgcatcgcctatcgtgggcgcacactgaccaccggatttgcctgcatggtcatcgcaaagggagggcgcatcaatctgctagcccttcgggctgtcaaccctactccggctagcagtgccattgtcaccgtgtggcccgtagagccttttcacgaaacgcacagtattccatgcgataggaggctcaccacctccttatgaccggcttcccaccttggcagtgggttacttcccgtggccgactctcacggcagatgggaagccctaagcgttaggcttaggtaaagcggcaccagtgttgcaagtctggtggattctatgggcctttgaaatcccagttcatccggttatccgctagtgctacgttgcagcttggcggtccacgtcaactctcggccactattggctgtggttggcacgcttcccgttacaccctacccgttagcggtagtcctacgccatccaatgtggctgctcctcagagcgtggtgccatactagcacccttgttgcatcctgtcaagcccttggctcgctcgggtctctaacccgttgggcgtcctgtcgccaccatcccaccatgtacgtcggtggtccacgtgttgcaaggcctcaaagggctatctgtgccgccttgtcaagctatccgttagaggaccatgtgcgctcctgttagtgtcttgaccggtgtcccggtctcacctcagcctcaacacccgtaatctctcacgtctagccttaccgctaggtcgctccgctgttccggtggctaccacttgccgcctatcatagctaactgctagcttagtgtcaagcgtggttcggtagctcctcgcatcccttaccagtgactcccgtgtacccttagcccacttgttggcggcgccactacggatcacgtcactcgacttgcgttgcagcttactaccattgcggccgtgtgtctactactgcttgcatcgcaagcgtcaaccgttggcctagcgggtagctaactaatcagctcgacagagtaccgatagacggtgattcaggttgagccgactgtgtgctataggtgtaccaaaaggccgaaacgatacagatggccctcgcacgcctacagctgcggttcgcatggtagcaggtagggtagcccctgtcaagccccttgcggccctcctgaagccctgtcgctgccccagtgacgccattgaaccacaccgcaccggccacgtcaacacctttcgccaagagatttattaacgattcagccaaggcagcgcggtccagccatacaggcagcaggcgcacgcccacccgcacgcccacccgcaggcacccacgcacggccacgcacacgcacgctcaggcccacgcaggcaggcacacgggtacacccacgcggaaccttgacgcgggcgcacagacgcgcacacaggcgcacacgcgggcacgcacccacgcacacccgcaggcgcgtaacgcgagggcgtacgggggcacgcgcgggagcttctattggagtgacccccgcgcatttccgaagcaaattttggtccggctacccacgtggccttactcctaagcctcgcgaactggtgcctttagcttgacgataggcccggagctgtagacatcgtgagctatcgcagcagccatggccttagccacagacttgctcgcatgataggcccctagagctagcgccttgccactgccatcgaagtacggagcctcctcgacccactgctgcttaccagtagtgaccgtgagtacgccgtccttaaccacaagcaccgtcgcggacttgccaacgtgctcctcgtagccttcgcccgctttaagcgcagcgagaaccgggcgaagcactgtgaaatccccggtgacacccagcagcacagggccggtgggtgtcgatacgggcatgatcttacgcacggtgtgcttgtggtcgccctgcgtggcctgactatcggcccacaggtgcttgccgtcccatgcgatggtggtcatttgtcacccgtacaccggcgcttaccggtaccgcacacctcggccttccacgcacgcagcgcagccttgtccttgttgcacagaacggtgtccatgcggcggtcctgcgcgagcttgaccaccttgtcctgcgaggaggtggtgcccttctccccaccgaggtaggtgatgtggcagtctgcaagcagggagtcgtcagggaccggcaggttcgcgcaggaggtcagcgacatcagcaggaacagtgccatcccggtactccggggcagcgtcaagaacttcttcagtgcgaacacgcacgtcctccttctctttgatgtaggtcgcgtacccggtagcctgcgtctgcgccgccttggcggtagcggtcgtgccgacttgggcagtttccagcttctccaccttgcgttgcaggccgtagacgtacagaccgaagcacacgaacatggtcacgaccagcagcaagccaaccagcttgccgccgagccgcgcgatcacttcacttggggtttccacggttggatcacctcgttgttggggcgcaagcacagagcaaactctgcgtcgcggcgcttggggatgccggagcaacggctgctggacagtcggcagtcgagcttaccgacgtagacccagcgcaggaactccttgcagctaccttcacgatcccctgcgttcgctttgcgcagcatggtgctgtcggcgaacgccttctcacctacgttgaacacgaagtctgtgtaggcgtcgatctggttgcggttaacgggggccttcaggtgcttgcgcacgccctgctgggcgatctgtaggtcttcgatcagccacttgtcgcactgtgccttcgttgccgtcatgcccatcgctacgcccttggtgtggccgtagcagatggtcggcacccggccggtgtcgaggtacgcagcgtagcgtaccccttcgtggccttgggtgaatgacagcagcgttgccgaaatgccgatgaagatgccgccgatcaggccgaacagccccttgttgctggtatcttggttctgctgctggttcatggttgctccttacggggtcagtgggtcgtcatccgggtccagatcgaccggagtgtgcgggccggagttcggacccgaggacgcggtgcgtgcgcccgcagcgatcagggcgtccagcacgagggtggcgtccttctggaactgcgcgagcagctgcgctgcggttgcgggatgctgctctgcgtgctccatgagggcgagcagttcgcggtgcaggtagttgccacggccgaacagacccgtgtagttgctggtgaagtcggacttctgcattggttacctccggtaacggtcgagtagggatggacggccacgttgcagcggactcttgcgggtcgctgccttcatgccggtcggatcgttgatccagtcttggaactctcgctgctgctgcttggcgatggccttgttctggtccagtgcaagctgcgcaacccagtgacgcacgctaccttccagtgcatcgagccggtcatcgtgtgcgatgctgcccttctgctgcgtgatcttcgccatctggtggaacaggctgtagacctgacgcttgccgctggtggcgtagcgctgggtgtactcgtgatccatttcaaccacggattccagcatgaccagcgagccgcgagccatgacaggttcgagagtgccgatgatacgggcttccttgttgccggtcacgaactcctcgcggatgtcgcccttgtatcccttctccgtgccgcgatcttctcgcaggacaggcaggaacaccttggcgaacgcgccgtagcccatgttcttttcgatgctgatgacgttcggcttgtacttcaccgcaatgcggcgcagttctagcaagccatcaccgtcgtagccaccgggcacagctcccacggccaacacgtacacggtggagttgaggaaggcggtcacggcgaaggccgtctcgtctccgttggcaccaccaccggccgggtcgatctgcatgtgcacgccctgcacgggggcagtctcggtgctcatgtcgtgcggcatcatcatcacgaagccgtacccactggactggaagctgcgctggtgagcgttgctcaggccacgggtgatcgtcagcgggaagcggtcgccaccaccggggatcacgatcaggttctcggtcttcagcgggaagcgcagcgcatccatcagccgcgtgttgagcatgtagttcagctgatagctggacggtccacgctgacgcagctcggactggtgcttctgctcaccggccaacagctcgtcggtgcactggccctcgtcgcccatcgggccaccaccgaacgccaacatcgggtcggcttctaggcgctgcacgatagacggtgccagatgcgggccgtagtgctcgcgctgtgccggggtcgggtagcgaccgggccagatgcgaacgtcgtagccacgtccgggcagggtgttgtagatggagtcgccggtctgcggcgtgccgaggtacaggatgcgacccggagtaccgggcttgccggtgcagatggccgagaactccaacgtgatggtcagcagcagctcacggttcgcggcagtgcggctgttcttgttggactccacgtcgtcggcgatcagcaggtccgcacgcttacccggcaggttgccggtgacgccgatgcacgccacgctcggggacttgtcgattcccttcagcgagtggtgcacgtcgaacgcatccacggaggtacggtcgcccgcgttcttgtccgggcggatgcactccaacgtcggcaccgtgaggatgatgcgctgaatcagcgtagcaatctcggatgcctgcgtgccgcctgccgatacgatcagcacacggtgagtgggatcgtggatcaggcagaagacggcgtagatggcagcgatggtggacttcgcctcgcctcgctgcgcctgcaccattgcgaggtgcgggccatactgcatgtagttggcgatgtcgtactgcatccacgtcggctcgaaccccagcaccttcataatgtcgcgcatgaaggtggcgaagtgccggtagtggttctgcaacagctccaacttcttgcggcgcacgtcggccgcttcagctgattcacgcattgttggctacgctccccggaaagtgaacgatgttgtcgagtgcacgctgcaactcgtcgtcgtcagccggaggcagcgagtgcttgcccagctcgtcttccagctcgccgagtgccttgttggcctcgcgcgtcgccgtgatgttgttgtccttcaggaacttgatcgccgcattgatgtcggctgcggtgcacagctcgccatcttggatgcgctgcatcagcgcacgcgcgaccagttcgtgcagcgcaccgagtgcgccctcacttgccggattcgacatccttgcctcccatgatctttcggtgctcgcgtgcccgccagtagaactgagcgacggcgtacagaatggcgagcgtagttacgatggcagcaccgtacgtgctgatgaagttgaggtagaccgcgccgagcgtaagcggcgaggttcggacgacctcattgaccacactcggcggggtcatgctgttctcctgtaggttagggccagtcgtcgggattgccgacgagcttccattgcaggcggttgacgttgttcatgcccaccgcaatcaggtcgccggggattcccgaggcgatcacatgttcggttgcgaagcgctcacgctgcgcgcgtacgcacaggttgctgccgttcttgtacgacaggagcacgtcgctctgcgtggcgaagacagcccgcttctcgtccatgcacaggcgcggagtggtagcaccggggatcaccatggtctgcatcgaagcagccaccgtgtcgtaccagtagaacttgcacacaccgcccgccatgtacgccacgtgcgggcgcatggtctggtcgaaggccagtgcgatctgcgtgatcccggagtcggtcagcacggtgaccggggcaacgccgtcgcggtaaacgacgacgctgctgccgtcactctcggcagtccacagcgcagcttggaggtcgtccactgctgcgttgagagtcagcccgccctgctcgaagtcaatgagcgggcgggtgcgccgattctgctgctccacccagtcaccgcgttggatgctttgggagacagtggggatcatggcgtgtaccggctccaagaaacccgcatgcgcaagttcgccgtctccgatccggtcttggtgatacccggattgaagccgacttggaaggtcacgcacgcggagagtcccattgcagccgtgatcggaccaccgggcacgttgttgatcgacatccggcaaacgcagtcacggtagtaagtacccggaacataggctacctgctgaagctgcaagtcagagaagctggcaatcgtccccggcggatactggtcggtgatagctccggtgccgtcgccagtaccgccgtagaagtagtagcacccccacacgtagtccgaccaagcgactgccgactgaccgttcataccgccgctgcggcccattgcaataggcttacaggtaacagtggtgctaacacccttgatcgtctcagtagtgacaaccggcgtggtatctgcgtacatgcgcagctcgtaagtaaccacgaggatttcatccgacagcaccgtgatggtggtcgggttacctgcggagtccttgataagcgcacgggtggtcaggatgtacgcgccggtattgttgttgtatgctttggcaccaagctccgacagaacgccagtagcggtaccagccgggaactggtactggcagcgggagtaggcgtagtacggggcagtggtagtcccaccgctgtccgaggacgtacgaccaacctgcgccacctgtgcaccaagagcggtatcggtgaatgccggggtggcgctgccactaccgactgccaagtaagcaatgaggtcgtacatgctgcgaggatagccgctgccggtatcacccagtgcgtccataccaccgtccgtgataaggttgctctgccagtcggctacaacttcgagagtatcgagggacttacccttgctgatggtgaacacgccagcaatgccgaggtgattgtggatcatgcgaagctccatgatacgaagccagaccggagtcgtgcagtcgcgtcgagcggctggttgactacagggtgctgcttcagggtgaaggaatggaaagaactcgacagcttcgccgtctccgggtcaggcgtgtagtccttacggatggatcggatgtcgaacgaaacgaaagcgctcccgtacaacgtgctctccgggtcggcggcataatcctgcctagagcttcggagttcccagcttacgaaggaggaacccagcgacgcagtatccaaaggctggagcatgtcgatgttgctgtacccagcaaagctgctggtcagcatcgcggcatcgaactggtagaagctgtagagcttggacgtaacgtagatgccctgctcctcgatacgaccggaccagtaggccacacggttcaacccgtccgtgaccttgatgctaaggaagtaggagctgtcgtcgttctgacccagtacgtacttgtggttccacttaacggtgtccacccacagcggtttgttctgcttgctgcggaacgccgacagtacaacctgcacgtacttcgtgtccttgggcgcagcgccttcggcaacggactggtgccacgcaccgttgctgccggaggaaaccatgttgccccagttgcgttgcagctcggtcccatcctccttgcggtagatgatcgacacacgagcaccggccttgcccttggagcttgcgccctgctggacctcggcggtgcatcggatgtagtcgttgaccttggcagggatcagcgggttgagcaggtcgctgccgcccgtcttgatgttggcgaagcgcgcgctgtacacgccgctgtcggtgtcgtagtctgagccagtgccaatcgaccagccttcgccattcgatccaccgcccggcaaccacgtgccgtcgtcgcctgcctcgaagtcgccgttgggcacgagggtttcctcgtccacgacttcagtgaaagccgcccacttgacgacgacttccttggtgatgttgtccacccgtaccgcagcgcccgaagggagcgtcgattcgatgacctccacggtgcagcggccgactgggttgttgatggacaggcgagactcgtaagcctcgcccgccgtgtacccttccagcacgcccgtcaccgacaggccatctgcaacctcgtccgccatgagcggtcggccgtacagcctgaagtgattagccatgcttactccttagccaagtcgcccgagagcaaccacgtgttggtgtcgccgtcgatgcacgttgcagtgatgacggagttggtgccgcgagttgcggcggtgcagccgaccgggacttcgagcgtcacgcccacgtcgccagtgatgaccacagggcctgccttctgctgcacgctgaagtagctgcccgaggcgagcttggtttcaccgtcgcccacttcggggatcaggttgatgttgacggcgcaacctccggcgtacgtgcagcgcacgagtccgtactcggtagccttggcggcgtagtaagtcggaccctctgccgtgatgatcggcacccgcaggctcgcagcggtgatcggcgcaggcccggtgtagggcttggcgtaaccacgcagcacggcgaaccagatgctgccctcggcaggaaccgtggcgaagcggatgaagctgggatcggtgccgtcagcgagcgtgacctgatagtccacgtccggctgcatgccgatgccgttgacgtacacgtcgtagaagcccgcgccggatacgtccgcgcccaccatgtcgaagtcggtgtcacccacctgatcgccagtccaagcaccggaccagacgcgcggggcgacggacacgataccaccagctgccagcaactcggtgacctgcttgtagatgttctggataatctcgttcaggtccacgatcacaccgacctgctggtcgatgctaagggtggcgatgttgagtgagtcgaacatttcctgaatgatcttcaggagctggtcgttgctgaggttaaggtttgtcttgctgatgatgctaccgttaacgtagtcaacgagcatctgctgcaccggagtgctgcggtagatgtagagcttgcgcccagcggcgacggcaggcgagactcggacggtactagcgtcatcgtcttcgctcaggacttccacggtgtgcggagtccggtcggtcagcagctgagtctcctcgtccagcagtccgctcatggcgtacacgtgggacgggttgatgtagccaccggtaaagctgatctgccagtcagtggtcacgccatcggcgtcgaacacgtctgtcgcgtagcgcagctgcgggtctggaactgccatgctgcctcctgtttgctataggtgtaccaaaagggtgggccgtccttggccctgatcttactcctccttccactggctggctgcgcccttcagcagcgggatcaccatcggcagtcgcccgcccggaatcacgtcggccagattctccggcttgccagcaatgccctgagcgaagtcgttgatgactcccagcgacggcgcgaactgcccgcccaccacttccttgcggttgccgaactgcccaccggccagctgcttcagccacgtcggaccctgcgtatcggtggcgtactcgtaccagccgcccgccacgccagtgcccacgtccagcacatcgttgagcatacccgtcgccgacacgtagttcagcgtggccttgcccagcgccagaggcgacaggatgttctggtcgatggcctcgtcgcgctcctgatcgttcatcagggccacgcgggacagcacccgcagggcttgcagcggagccgccacagccatcgcagcagcgatcaggcccgccgtctgccatgcaccgtagttgcccacgtaccggcccagctgcttctgctgcgcgaccagcgagaacgtgcggtgctggaacagcagcttcagccagccgttgtgcgcccacttgccagtctcgccgatgaaggtgtcctgaagaatctgcgaggtgccacggttgatcgcgttgtagaacgccaaccatgcctgccgatccgccagcccctcgacgttgcgcgggtctactgcttccagcttaccatccgcgccccagcgcacgacctgatcctgcgtagcccgcaggcggttcagcaggttgtcgtcaatgcccatgtccttcagggcggtgtcagcttcagcaccatcacgcaggaacttcacgcccttggcgatcagcacttccgcgaagccacgctgctgcacagcaagcacggcccgctgccccgagaggatgcggttcgcatgcgctgccttctgcaccagcgaggtcaggaagcctgcgcgctcgctaccatacatcgacgcctgcgtgtccagcgagttgaacatgtgtaggtcgtaaccggcgagaccgaagccgcgaccgctgatgaactcgaagccgtcgaggatttggttgccgctgtcctcgcccttcaggatgcgcatgatttcgctgcgcatgcggggagcgatacggattgcgtcagccacaccagcagcaccaacagcggcgaggccgttgctgtactccgctgcctgattgatgcccgcgccgcccagctggatggccgaggtcagcagacgcgcattcgccagaacagtcggatcgccggtaccgaccgggcgaccaaggaactcggacatcacctgctcgaacgccttcagctccacatcgttggcaccggtcaggcgcattgcttcgcgcgccacgttgatgcctgcgtcgccgaggatgccgtgcttcgccagagcgatgtcaccagcaacacgtcccgcgtacttgcggtagttgtccatcacgcggttgtcgagatagtccatcagacggaacttaccgtcagcgtcctcgtactgcttggtcacgtcgaggtcgatacgcgccttggtgtgcttcgcaccgccacggctgtacttgcccatgaccttctgaatctcctcctcgttgagcgacatcgcccgcagagtgtcgcgcagcgtgtccgcctgcgactccgagaagacctgacccggcgcttcgatgacacccgcagccttgcgctcgatgcgttccagatacttggtagcgaacttatcgaggaagtcgtccccatacagctcgcccatcacctcgaactgatcgcgcatcgcctgacggataccctcgcgtcgcaccggaccagcagcagcgatgctgccgcccagccacgtacgggactcgtagccctccacgtcctcctccggcagacgctgtgcgcccaccgtaccggccgcgcgctgctctgctgccatgcggttgtagccacggtccaactcacgggccattgccttcactgcctcgtgcgcatccgggatgtccccgccgttgaagcgagtctcgcggtacagcttcactgcgtactcgaagtccgcgcgagccttccagcccgtggcgaagtccttgatcgcaccgataccgcgcacgtccgcacgccacaggcgataggccgcttcccactgacgcgggcgggtgcccatgaacgactcaaaccgaccatgccgatccatcgctgcggtgctgtgtcggcctgctgcaccctcgggattctccaacagggtgatcgcaagcatgcgggcaactggcgacttggacgacattagagtcgtgctcgtagcttccagcccgaagcgctgcatgatggtggacagcttcgccgcgtcgatgccgtactgcgcactgaagcgttcggagcgtgccatcacttcggcgacctgcacacgcatcgcgtcatcactgacggacttgtccagaccggtgcgctggtagaaagccttgcgctcgcggttcgacttgaagatcgagttggcgagcatgccacgcgtctgccgggtaccggcctgcgtgtcgcgcacttccgcgccgaggttgtcaccgacgaccgacatcaggcgttcgagcgcggactcctgattcttcagacccatcactcgcgcgatcttatccttcagccactcccacgcattcgggcgggtgttgcccggcgcgggcatctgacgcagcaccgcctgcacagcgcggttcgtcaggccgtaggaaatcagctcgtcagtgttggcgaggaagcctgcctgcggctggttgatgcgcgtctccatcgcagcggtggtcagcgtggagtccacactgccgatgctgttgttgatatgggtcagcagttcttccatttcctgcccgaacaccgagttgctgcgcagctcacgcagcgtggcagcgtgcagcatttcgtgcaccaccacttccggcgtgtagttccgcatcgccatcgcgtccagtccggcgttgtagccaccggccacacgcatacccggacccatgttggcaccggcgaaccacttgtcgagttccgattccggcacgatcttcaccgtgctcagccgcccgccacgcttcagcgcgttggcgatagcacgcacgtcctccgggatagaggcgttggattccagatacttcagcacgccatcgacgttaccgcccttgatacctgcggtcttccatgcgcgttccagcagcgggtcatgctgatcgacccggccacccacgctgtcgttgtaccgcccggtcgttgcgtccacgttgcccgcgtcccgtgcgagtgcaccagtggtgcctgcggtggtggtcgtctcctgcacgtcgggacgggcgaagatacggaagtcgtcaggcacgtcggccataccagcgcgcagccaatccacagcctcctgcttggcaagctggtggatgcggttgttcaccagcaccgggttggcgtcctcgcccagctcggccacagcgcgcgccttcaggtcggccgaccacgcttcgccgtaagcggcagcgttgcctgcggacaggtcgatggttgccttgtcacgaatctgcgcagccgagcgcacgcccggaatgtgcatcgcggtgcctatggtggtagcgaatgcagcgtcggtcatgaagtccgcgaagttgcggcgctcgcccatgccaaccagcgcggcgtccgtgatgacggaaccgaccgcgttctccgcagcagccgacgcgagcgacgcgcccacgcgcccttcggcaacgagtgcagccgagccgatgcccagcgccttagcgcctgcggcagtgacgccgccgatagcccagttgcccggatcggtgaagcctgccaccatgtcgtaaccgaagctaccccagccagtctgctgatccttgatgcgcatggagtggcggcgcaggaactgtcggtcgctgacgtacttcagctcgttcggcgagtacgctgcatcgcggatgtcttcgagttcgtcggcagtcatccacggcttctcccattccttcgggtcgtacttccaaccttccggaacgttctcgtcctcgcgcgcaaactggttgctgatcgcagcaccgatgccgctgtcgaacgcagcgccccacttgtcgaggaaggtcagcgagttgcgcagctcctcgtccgcgcggtcctgcgcgagcgcctgttcggtctgatccagcagcgccttgcgagcgccggtgttcagcacgtccacttcctgacgcacccaccacggcacaacctgatccgatgcacggacagcctgagccttgcctacggcctgcgcggcggtgccaccttcctgtgctacctgacccatcgacagctcggcgatgcccgcacgaatcttgccgatgtgttccttcgctgccgacgccagagcgttgcggccttcgatgggcgcacccgtccacgcatccgggatggacgcaccggaccacgtacggtcgcgcatgttcgggttgccctgccatgcggcgttgaggtctgcctgcgtggtggtcaggctgcgcggctgcgccgacactgcgggagcggacgcaccgcccagcacgctcggtgcataggctgcgttctcctgcccccagttcttcggattggtgccgccttggtagatgcgcagcgccttcgtcacgtcgcccttggcaagctgcatgttctcgcgcatgatgtcggcatacagctcgatgctgtcttggaagttgcgcatgtcgtacttgcgaccgttgcgcgcttcccacgttgcctgcgtggtgggcatgacttggaagtcgccctgtgctcctgccttgctgcggatcacaccgtcagcgtccttggcggcacgcccgttgccggactctactcgccactgaccgcgcacgatggactccggcactcccgcataagcggcagccttggcaatctgctggtcttgggtcagccccgaaagatcgagtgccattgtctatctccttacagtttgggttggatggaaatgctctgctgaatcgtaccgtcgttcatgcgaacgtagccctgcggtaccggggcctgcaactgacgctgctgcttggtgtgcttctcgtactcgtccttgatgtcgcgcccgtacaccggcacaaccttccagcccttctcgccaacagcgttgacgtacagcaccggctcgccgttctcgctgtccttcatgcggaacacgtcagccttcagcccggtgctcggctcgatgttgacccggcgcagtgctgcgtcgatggccttctcgatggcgggtccggtttccttcgtgtccatgaagcccagccatgcaccgacgctgccgatcactcggccttcgtcgtcgcgtccgttttcccatgcgtacttgcctgcgtcttccagaccgtaggccagcttggcgtgagtagccgcagcctgcaagccttccgcagaagtgtccagcagaccaccggtgtcagtgaccgagcggacgatggcgcgagcatacgcagcgcggccagagtcgcccagcttgttgccgaacatgccgaggtacttggggttgagcttggcgatagcttccgtaacacgagcctgagtagcctcggattccttacggctgttcgcgtcgaactgcgtcggatcgtcggtggtgatttctccacgggccacctcgtaagcaagctcgaagttcacgccaccattctccaacgcttgcagcttgttgaagaacgtgttgacgctatctccgaagtacagcgcagcggtagtcgcgccagtcagtcggccctgcacgggctgaccgttcgtgtcgatgcgtgcggcggtggtctgcttcagttccttccactgctggtacagtgcagccgctgccgtgttcggctgatcgcggagcacagcgcgcgccgtggtctggaactggtcggccacacccttcagcacagcgcctcgcccggtgttggcgttccacaccagctgcgacatggcgaccttggggttcgcggccatcgtggcattccatgcctgcaccgtgttcgcctcgatcagctccttgtccacgccggggatgttgatcgtctgcgcgtacgtgccgcgcttgaacgcttcgatgccaccacggatgtcctcctcctgcgcggccagcttctgctggtcggtcagcgcggccttggccgcagcgttacgctggttgatgacggcttcctgtgcgcggatgtgcgcgcctgcggactgtgccatgatcgaagccaactgcgtaccggagtacagcggtgcgtcgcttccagtctcggcggcgtaggtcgagttcatttcctcgatcatcgcctgcgacggcttggcaccaatgccctccgatgcgtacatggagacgagcgccatcttctcggcctgctccgggttggcatcgagccagtcggaacggtaacgatcctgcgcctgcttcacgtactgctggattcccagctgcccgtccgggtcgatggcgttcagaacgcccttgctgttgaggaacttcagcgtgtggaactcgccgcgatccgcagcgccacgatagaacgcagtgatcgcggacttgtacgactcgtccgtctggtagcgcgagggcgacagtccgtccagcagggacagctgcgcctgcgtcagcgcctcggtggccttctcgtccatgggacggttggtaccgagcatcgccgtgcgcttcgccagttcgttgaagccggtggacgccgacgagttcgcagcgtactgcgccttcaccagctcctgctgctgccatgccgtgcgctccttggtgtgcaggtccatgagggaacccgcgcgatccatgaaggtcttctgcaacaccgtgtccgcgaaaccgttgccggtcatgcgggcagtggcgaggtcgttgaactccttcgccatcgcctcgggaggaagctgacgcaactccggcatacgccgaagcaagtcgctctccatttcgttgacctgcgagagcgtgttatacatgctcgcgccaatctcgtagttggtgtctccgaagattttcttgtaccacggttcggtcgcagcaatctcgtccatggtcttaccagcgcgggcggcaacgaagccgtcccacatctgctgctgcttcagcttggcggtgttcggcgctgccagctcctgcaagaactctggcaggttgctgtccggcatcgtcataccaccagtgcttgcgaaccagtcgttgccggattgaaccggcccgacctgattcacaccagcgccttgaatgctggtgttgcccgacagtgctggggtggcgttgatgccaccctgcaatgcggactgcgtgttgaaggtaaccgtgccgatgtcagccattaccatgcacctcctgagttgcctccgctgccgctatcgaaccagccgaggccggacgtagtggtggagaagttgtcgtagttgttgccgaagttgccggtgaccttcgccccagtcacggactgcttgccggtgccgtcgttgtacccgaaggtagtggacgcccacgacttgccgccgcgatcattggactgctgccacgcctgcataccgttctgcgctgcgttgctgaaggactgagaggcaccagtgaagttgccgttgtccgcctgccacgtgccgaccgcgaagtctgccacggcctcgcctgccatcggcccaccgaagtaggtagccacggccacgccgatcagcttgcccaagcgacgcttcattgcctgcggctcgatgtgctgcgagtagtcgaactgcccgaacgaacggctcatgtccatcccgttccacgcgcgcgacatgatctgcgcagtctgcgatgcgccccgcgaggcgaggagcgagacagcgttggcctgcgtctcctgatccatttccgcctgcaaccgcaccatcgaatccatcaggtctgcggacgagccgccgacaccgacagcaccagcctgcgcctgaagtgcgccacgcgcgttcgccagttggagctgggagttaagcccagccccttggcgcgcacgcagctcctcggacagcgcttccatgttggagttgtactccttcgcggcggcgtccagttgggcgttgttcttcagggaccgcatgaaatcagcgaagccggtcttggcgacctcgctgcggttctggttgtcggtctgcgcaacggctgcacggtagttcgcacgggcaacgcgggtggtgttgttcgcttgcaggatcgtattaaccgaacccattagctaaccctccgtacattgttgaaagtctgacccgtccagctcaggccggtcacccggagcgggagccaatccttgctgcgaatctcgtaggtgcactcgcgcacttcgcgcccgacgctgatgttgagctgcccccggtacaccggttgccgcgcgatcagattgtcggagtcgccgaggatgcggccctcgaagtccgtagtggtcacattgctgttgcgggttgccaccgtggcgatcatgcctgccgtgttctccacgtccaccgtcaccttgttgagggacatgcgtccatcgagtacggcctgaccgttctggtcccgagggaacggattggtcgggatcaccagagcttcggacaccacgccgtattccagcgcaccagcagcgaggtcatcgaactggttaaggaagtcagacgcctgcgcgtagggacaacccagcaggaagtacgggctagtgctattgacggcgatgcttgcgctcgcagtctgtacgcccgtaggtgtaccaaaactcgcccagctgtcgaggcacgcatgcgagtccggctcgcccttcgggtcgaacacgtcgcacgccaccagcgacccgcgcgcagtgaacacgaggccgttcttcttgtagctgctcacgccgatgatttcgcccagcgccgggtggtaccggaacttcgaccacgcatccacgatgcgctgcccgttgttcttgttgtcctcgtaccggtacaggtagaagtcctgcgggtgctcgcgagtgcggaacatgacgaggttcggcgcagtgagcggggtgatctgcaacggagtgcccgacagccacgagtccagctcgttggacatttcgtccgtcaccgtctgctgcccgttgagcgcgcccactcgcatctggtgcaggctcgtgccttcgctgccgtactgcgcataaaagatgtagttgcccgaggtctgcgccttcgcgtcaaccgaatccttgttggcactgaacgctttaatcagcggattcttcggactgaacaccgagtcgccgctgatgccgtactgctgacggtcaccgaagatcacgaggttgccgttgtagagcgtcgcgtgccggagcacatcgccctcgctgccgtgcgcgaagatttcgatggggtcgctgtcttcgatggtgacggccgagccgcgccagaagttcaggtagtccgccgagcgtgaggcgttgacgtagttctgtgcgccgatgaccagccggtcttggaagacggacagcatcgtgatcggcttgtcgatgaaccacgggatcggcgaggtcagaccatcgcctgccactcgcgcaccgtaggccggatgctcgccgctgctcggagccagagacgtgaggcccgcaccgttgcgtgcgatgtagcctacaccgttgtagatgtagagctgcgacacgaggttgtcgatggtgcactccacgccgggcgcttcgtaccagtccaccgacccgtagccggaagtctcgccgttctccaactcagcgcgcaggtagtacgactcgtccgcgcctgcaccactcggccgcacgcgaatgaccttgccgtgccagtggaacttgacggcgtaggtcgcgtctgtaatttcctgccctgcggcgtagaaggtcgtgccgtctccctcgtcgtcaaccgtgatgtccttgaactggtcatcgtcaatgatgatcccgcccttgatgtacgttgccgacacgcctgcatcgaccagcaaatccgacagctgctccgcgatgtactccgggcgcgtctgctcagcgctcgtcacgatccactcgttgaccgcagagttgtactcgttcactcggtcgttgacgtacttctggtacgccgcgtccggctccgtgccaccgggaaggtagaacgggatgtcgctggtgtcgagcgttccggggtacgatgcggtaaccgtcttgaacgttaccgtcagcaccgtgttgtccgtccgcgtcaggttcaccgtgtacgtggtgttgtacttcccggtgcgcacccatgctgcgaggcgctggatgttcgtctgctcctgccacacgttcgtgctggtggccgaggggatcgtggtgttgcccgcgatgtagacgtagctgccgatggccgtgagcgacgatgcgcctccgctgaccagcgtgttgacccacgtgctgttctcgtacaccagagggatgaacgactcgtccgtcttgttgtagaggaacgcgaaggactcgctgcccaaggtcgaggcgtcgcgccggtacagcagcgcgtactccttgccctcctgcatgaagtcgaacacgtccatgttgcgcagctcggccgaggtgacaacggcttgggaagcagcgaaccgcgtaccacgacggcgcacgaggccgttcaccggatcggacagcacgttgatctgctcgtgcgtctgtcccggccgacgacgatgcgccggtttctgactgacaccctgaaggatgtcgggataggttccgcctgcctttgccatgttgtctccttagccggggaatgtgacgtggctgtgccacgggtgaccgctgtagttccagtaacgggaacgcagcacgtccacggatgcgcgagcgaacagcgggttcgccttgatctggcggatgtgctcggccttcaagttgatgtaactgtcatcgcgctgctgcttgatcttggcgtacttggtgttgtcgccgtcgaagtcagactggaaccgcagcaccgagtcgtcgcgcacgaacatctgcacctcgtaggggaggtcatcgaagtccagcagccgcaccagcttggcctgcacgttgtggtcgaactcgtaggtgttgcgcttgcggtcgtacagtcggcgtccgcgctgcaccacgtggccgaaccggctcgggttgcagtccagcttcagcacgtccgtggggaccatgatgtacttgctcgttgcctgcggcttcagctccacccattcggtgttgaaccacagcgagagtgaggacacgtcacggtgcacgcggtcgatcaagtcaacggcgtcgtccttgtatacgtggtcatcttccagcgtgttgagcttcgtctcgcccatcgtcttcaagcaggcgttcacgatgtcgagcttggtgatgaatgccatggtgtctcctgagaggaacaaggcagagacgccggagcgcccctgccgggatgttgcttagtccgcagccagagccagagcggccggtgcgtactcgatgtcctgcgagccgatttcgtcgtccacgaaacggacacggacgacccagcctgcggtgccacgggtgtcgtagtggacgccgacgacggtaccaacggagttggcgggcagaccggccacgccagttgcggcgacgacgcggttggaaatctcgaacggtcggtcaaagaccatgatgttgctcctgtgttggtggaagaagggcgcggtttgagttacccgaaggattcagggaccgcgcccagcggattaggcaaccttgtcgatgcggcccgcgttctcgacgcgatccagaccaacggcgaaggacatccacgagtccacgaagtagcacttcgaggcatcgctccaccacaccgaggactgcaacggcagcgcttcggcgatcagcagggccttcggcgacacggccacggcgatcagggtgctgaagtcgccgtcgtagaagtcgtcgttgtcgtcgttcgacagcaggtgaccttcgatcacggtgttcggcaggttctcgctcgacagcaccgggacgccccagccgtggaaggtcgggatgccggtcagcttgttgccgtccgaggtcaggtactcgccgttgctgatctgctcggcctgctgcaacaggtagaagatcgccgggcgcacgatcaggaccacgccatcgcgctgcggcttgaccttcttctcctcctccatgcgggagaacagtttgccgatggcggcgtacaccttggccggatcgttctcgtcaccagcggcggacagcacgacctgcgtggcaccgaagtggccctcgggcgcgcggccgttgcgggtgaagatcgactgcgtggcagcagcggccttcgcggcggcgatgctgatggtcaggtccacgaactcggcgatttcctgaccctgctcgatggcgatttccttgcgggtgtcgatgtcggtgaagatttcgtccagctgccagatgctgtgacgcgacagcagcatggtatcgacggtcaccgacgccttgctgaagtccaccggggtgccgtccggcgcgtcaccgcgcttcagcttctgaagcttggtacggccgatggccttcttgatcagggtgttggtgcccttgacctgcttgcgcgggaagaacttttccagcaccgagctggacacgtaggtgtgctcgacatcgccggtgaactgttcgaggatcagggcgttctcgttgccggactggttgacctgattcggcagaaccgggacagtcgggaagatggtgctcatgctttgtgttgctccttggtcttagtggatgacgcgcgcgttgagtgcacgcagttcttcggagtgggccgcaccacggatgcccttctcggcaaccagcttgcggtactcagcgcggtactgctccttcgtgataggagcgacgccgttgatcgacgcggcgggggcggcggcgttggtagccggtgcgcccttgacggtcgtcgcgggattggcctgtgccagagccatcaggtaacgcgcggtcgcctgagcgccgaagccaccagccgacagcgattcgcttgcctgcttcagttggtcggcgggcaggttggcccgtgcgaactgctggatcgcagcccagttctctgcgccacccacggcttcgtggacagcagcaacgttcgcggcgtgcgctgcggttgcagcggcggtgacacgagcgatgctctccttcgccagagcgaggatcggtgcggaacccttggccttgtcgccgaggacttccagcttggcttccagcagggcgaagttgcccttcgctgcttcggtcagttcgcggctgtcgatgtcgaggcccacggtgttgacgaagtattcggccgcgatgttcaggccgttgtcgccgtagtccgggatcgacaccgcagtcggcgcagcgttcgccggggcggcgggctgtgcgggagcggcaggttcgagactcagcgcgtcagcagccggaggtgcagcaggagctgcgggctgtgccggtgcggccggagcgggctggccgttgggcaacagcttgtcgtctgcgggagccggagctgccggtgcgggctggttgccgttcgaggttgcgatcacggttgcgccgggaccaccgcccggaggtgcgttggaactcattgtgtctgtgtctccatgttgttggcgttgtcgatctgctgggatgcgttctgcatggcgagctgctgctgtgcacgctgctgcatcatctggccgtactcggcctcagtcagcacgtagacgttcgggtccaagccaccagcggcggcgaggtctgcgatccacgcggacagcttcagtcgttcgagaatctgcggcggcagtgcgaggacgttggcgaggttgctgccgaactccaacagccggtcacggtcacccgtacgggagagcgcggccaagccggtgatgatgacaggctccaagtccttgcctcggatgtcgcggcccgtcaggttcatcacccaaaaggcgactggtacctgcacgtccgcagcgatccgggagtagccgccacccagcccgccttccagttcttcggcgaccatgcggatttcctgcgcggtcacacgttccgcctgacgagtcaccgccgtctgcaacaggaagcctgcgccgatgcggttgatgtaggtggactggattgcttggttggtttgcagcacgccatcgacgcctgcgttaatcagctcgatgtcacccttcatgccgggaatggccgcgccattgggcgacgccatgaagtcctcgacggaggtctgacctgcggggttaaccagccaccggaactcggaggcgaggatcgcgccctgcactgcggcctcggacagcatcgagagcgactggaagtcggcctcgtagtcttcgaccaagccggagccgtagtcatcgcctgcggccaagtcccagctaaccgcccggtagggcagcttgtctgcggtgtaggtcgaggagaagttggcgggcagcttgcagttgcaaatccacacgtcttcgttgtacttgccggtcttgtggtccagcttgacccacttgtactcccacaccatgccgtcgtcatcgggcttgaagtccgggtgcgcgacaatggcagcgagcgctgcgggttccagctgggtcttgtgcaccttctcccgaaggatcagttcgtagacctcgccggtgcgggtgcgcttgaccacgtagtgccgcatgttgagcacgcggatcgtgtccttctccaacaccatgagggcgttgcccagcacgatcagcatcttcagcaggtcgtacagccgggagcggatggagcgcttgtccagttcgagactggcatcctgctcggccttcgcaagcatcgcctgcatggcctgcaagtcagcgccttgctcctgcgcagcctgcttcgccttgcgcttcagctccaaccggaagaacgggcgggacggtgcgaacagcgacatcatcagcttgttcgccagatggttcactgcctgcgcgccgagagactggaacccgtgggtcagcggctcggtgtcctgatcgcggttcttgcgagggaacagcttgggcacggtccagctcgaatagcgttcgagtcggtacatgatgccctgtcgcttgttgtcgtaagcctcgaactggcggtgagcggtttggatcggatggtccatgctcacctcacaacaggtctgacccggccacggtcgtcagccgggaagctgcggtcgtggtcacgggtcgggtgtaagtggagcgggcggtcttgcgtcggccgatcaggtcggcagtctgcaagtcgaggtcggaagttcccagccgcacatcgacggtatcgacgggggcactcagcaacttctcggcgtactcagatgcggcctgctgtgcagctgcctgtgccatctgatcggccatcgcctgaatctggtagttcgtggattgagtttggaggttggtctgcttgtcgatagcagcagcttgcttcagcgctgctcgcttggcggacccaccaccaacgatgctacccataggttaactccttcgcttggtgaattggggagcatgccgttccagcaggtagccgtagcgtgcatacatccgtgtgagtgctcgggagttccgagctagtgcaccgcctgcgctcagtgagtcgcagtggttgatgtcagccagatgttccatcacggctatgtaccggtcgaaggaactgcccggcccaattcgcagcaccatgttctcaacgaacgtagtacggttcttggagtaccacggtgtgacaatggcaaagcacagcaggtaggcttcatcaatgattactgcatccactagaccctgtgttatcagggccactgtgtaatcagggtcatcacagttgtagctcacagaagattctctgttgtctaccttactatcttctctagatgacagatacaaagcggccgttaaagccgccttgatctgctcactatcacccgtcgttggtgttcggtacggaggaatcaacggtgaaaccctcctgtaagatgttcaggacgcgggccatccccaactgcatacctgcctccaagggcgtggtattcgagttgacggacagcgacagcccggacagcttccgcacggcggccagctggttcgggtggagcgtcatcaggactttcactttggcgtcttcggccatggtgtctcctctgtgctataggtgtaccaaaaggtccggcaccggttccgcttaccttcgcggccgctccaaccggacctcagttgcctcgtgctataggtgtactgaaactccgtcagctgaagaagtacggagaatcaaggacttgccgaaggtccagctcgcccatcggcggcggctccggcaggaacgggtaggccgagtggaaggccgacagcacgtcgtgccgctcgtacatcgacacgaacacctcccggatgatccggtacagtgccgcgctgtcggcggcgtgggtgccgaagtcgtcgtgaatcatggcgaaggcgtcgatgccttcggccttggccgcgttgaccaccagcgtcaggtggcttgcgtcgaggctgtgcacgaagttcggggcgatgccgttgcggtgccgggacttcttcaccgcgtccgtgctcttgcgcagggacagcttggcgttgccgcacagcttggtgttgatgcggtgctcctcggactcccagtagacctgcaccaccgggaacccggacggcgtgatccaccggatgcggtcgtacccttggttgaggatcgacccggagccgcgctgcaaccactccatcgcgcccgctgcggcgaccacggtgtcggcgatggcctcacccatgcgcttgctcaggaagcgcgctgcggggccgtacagggccttgtcgagcgaggggaacttcccacacttcaggtagtcttcgatgatgaagtccgcccacgaggactgccgcgagccgtacggcagggtcatcacgctgcgcttcaccagcgagcgtgtgaggccgtggtcgagccacagcgtgcggtacccttcggcatcctcgtcctcgcctagcaggacggcagtcacgcggtctgccaccatctggtagatgtcattcggcagcggtgctgggatcaggttcgtcgccacgccgcctgctgcgtcgcgcagcatcgccgagaagttctgaagcccattgcacgaaccgtccatgccgactgcgatgcggctcaggaagcgatccccgaacacttgccactgctcgtactccatgcaccagctcagaaattgcagcggcttgtcggcggtcttccactcgtcgttgttcaccgggtccgcagcgaacgccatgatctggtcgtgatgctccgctacccacttcacacgatccggcagagacgccttgtcgtatccccatcggtttgctcctgtgatgcagaaccaatccttcgcgtccttagtcagcagcggcttgccatcggcgaactccaagagcgccttctgcaagtccgaaccctgcggcgacacgccggtggtctgaacgtacttgcggccacggaagtcagcgaagtacacgaagtagatgctcgggtactcggcgaacttgcgcgccaccttcattgcgttgtagaaacgattgcccttgttctgtcgcaggcgctcgtcggtgtgccagttggacatgtcgcgcttccactgcttgaactccaactcctgattgtgggacatggtttccttggtcatgtccttcgtcagccactccggcttgcgcggcttcggcagctcgccctgagaaatgatttcctccatgtcgtgcaccttggcgatggccgacacagcttccatcagtcgcttgttgatgcgccacggcacgcgctgcaatgcgttgatcgcagccatctcgttgcgcagctcggcagcgcggtactcgtcgcgggtctgagcgtaggtcttcaccatccacggattgagtcggcgcatttccttcgtgtggaatccaccgttgtcgatgtccacccagtccatcggcggctcgacgcacggcaggtagaacggcgtggcctcgatcacgaagtcgctgatctgagtaatcagcttgcgcacctcgtcggtcagcacgatcttgacgtgcgtcttggtctggaacttgcggtacgctgcgcctgcactggcagcagtctcggtgaccacgccaatctccaacatgcccagctgcgcaagctgatcgcacaggtacgcgccgacctgatcgcgctgtgcctgtccccactccacgaactcgatgccgttcttgcgtccttgcatcttcatcaccgtcatgcggtggttctcgttgacagagagcttgcggtccatgtcgttcatcaggtggtagaacagagtcggctccgcgtcggcgaactgcgtcagcaggtactcatggtacacgttgatgccaacgttcttcaacacgtcgcggtcgctgccttcgccgtgcttgtctcgcatgcaggaggtaagggcaccgcgaacggcgacgaaggccacagcctcgtaccactcgcgtgcctgttcctcggcgctgacgggctgtccacgcttgttctgacgctcgggatcgtacttggcgcgcagaagtggcacgtgcgcttgcgcacggccgattcgcggagagtcgatgtccgcacggatgcgctccgcaagcggaagcacgaaccggcgatacactgcttgggcgtaggggttgttgtccgcgccgcccttctcctcgttgcgggcgatggacttctccatgcgctccttaccgaaggcgtaggtttccagttcgagttccacttgcgagagcattgttacctccgttgctgccgcacggtgtagtcgcgcggcgggtagcgtttcaggataccgcgcatgatttccatgtgcaggtcgtggatgatgtgcggccacgcctcaccgccgatatcctcggccatgcacgtggcagcagcgccgaacaagtcggcaccgtaccgggcgcgcaccgaaacctcgacgcggcccatccatgccgaggactggctgaagtccagctccggcttctcgaaagtgatcgcgtccatcagcccctccgctcgtcaaggaacttggcgaacgcttcctgcaccttgtcgcgcagcgtctcgttcggccacagggaaccggcgtactcgccgaaaggaacgctgatgcgcagctccaccgtgtcgcgctccatgttgtgccatgcttgcacctcgacgctcacaggtctgcctccttcttgtcgtgacggatgcccttgtatcgcggctcgcgcagcaggccgtacttgctgaaggacatcgcctcgatttccacgatgcctcccacgctaggcagctcgctctcgctgtgcggcacgccgctgccaacctcctgcgtcttgccttctccgaggtcaacgacgaccgtgtacacggcgcggccggtcttctcgccgactgcttcgttgatgccgagcacacgcaggtccagcgtcagggtcggcttgatcttgacgacttcgccgttggttcccttgtcgcccttcacccacttgccgctcggcttgcgcaggatcagcccgtcgtacgcgccgccctcgcacagcagcttcgccgcttccatgctgcccagctcttggtcgatcaggaagccctgcgactcggcgtagaacaccggcgcggtgccctcggcgatggcgtggcccatgctcggcaggcggctgacgcgctcctgatacacgaggtcgctgaaaccctgctcccattcttccagcgtcacgaagtcgaacaccacgaacatcggctcggtgtactgcgtgccgtccttcttgcggaacatgccgctgacggtgggctggtcgatctgcgggtgccagtattcgccgaagtacacgccgaccgggaagaacggcgcggatgcgagagcgttctcgatgtggtgtgcgctgacgacctgctcaccggtgcgggagaacaggtcaaccacgccacgatccaccggctgcatctgcacgtcgcccaccttgatggcatgcaggcccttgttcaccgtgggcacccagtggccgcgcttgatggcgaccatgttgcagccgtcgtacttcggctgtgcgatgtactcggtgcgaagctgctcctcggtgggccgcagcttcttcttgatcttgtcctgctcgactgccttgtggacgatgtagctcatgcgtagtccctccaaatctggaacatggcgagcggcacttcgtaccacggaacgtagcgctcccagtacgtggccttgccgtcgtaccactgcacgcggaagttgcccttggtgaaggcgcggttgatcttgaagccgcgcttgcgcttcttgtagccgggagcaacccggacattctggcgaggcacatcaaacatcggcgctgtcctccttcttggtgccgtcacccagcgcggcgttgaaccgtgcgatgcgggacgacatgaactggttgacgatggtgccgatccacagcttgcgcggagcgagcgaaccacggtagccttcccacgcatcggcgatgcgggtatacagctcggcctgatcttcgtcgggcaggttcgggaacccggccttgaccgcattctgcaatgcctcctcgtggtcggcactctcgccccacgcaacggcgttctcgtaggacttgatgagcatggcggtctggttcttgtagagcattcagttctccttcgacgggaatggaacgaaacctgcgaggcccctcatcacgaggatgcagaatgcgtcgtcagggtatgtacgatgccagagtgagttggcccactcgacatcgaactgcttgcgggtacggtgctcctctaggaagcgcgcccactcggcctcatgtgggacgtaccgatgcacttggccgcagcgggcgcaggccatcagtcacccttgctgaaccagcggcggatgatgtactggcggatgaagctgatcgctgtgaacgcaatgccgatggcgtgcgccgacagcagcggatgctcgggatgccacagcaccggaagcagcgcgatgttcgctgcgtagttgatgctgtagccgatgccgatgttcacccaagcctctttgatggagcgcgccttactctgcgccactggccttctcctcctcgcgcagttccagctccaacaggaacagctcgttgatgatgtggtgcgcccggtggtggatgcccgtctccgggtccagcttctcgccgaggcagcgcttgttgtcgtgtcggtagctcgcgtcctgataccgttcgagcgccttctcgacatgctgccacgagtgcgctttgtacttctgcgcgccgaaggtcagggtgtcgatgactcgggccagtgcacgcggcacgccctcatgcagcagacgggcctgcggcttgcccccgtcatccttcaggccgacgccacggtcggacagtgtgcgacggtcctcgtcgcggtagctcagttcgggcattggtacctctcgtctggtggtggtcacgcctccgatgctgagaagctgtcggagggaatcgggaacgcagcagctcggcttaactcgaccgtcgaagaagacctcgacatcacgagcgaacacgcggcttacctgtccacgcagcccgatcattgcgggcgcattgccgatgtactgtacccgcatgccgctgcggatgtcggtgatcttcatgtcggttccttatgccgggacggtgatgtgcttgcgcgcctcggcgctggtcgtgagcttgcgcccacggctgtagccgtcgcacacggtgcactgaagcaggaggtaggtaccgacctgcgtgcgggccggatcatcctgcgggatcatttcgttgcagccgcacttgttgcagcggtgctcgctgccgtcggccttgtagtacactgcgacgttcggatgctgcgagtaccaaccgcgcagcttcttgtactccaacttcatggacttcacgtcgatgcggttgtacgcttcgcactcgtcccatgctccgggcaggctctgcatgcaggccacccacaggtcgaagccggggaagttgtggtggtcgtacttgcgcagctccggcacgatcacgccggtggtgtactccaacttctgcgaggtgaaggcgaactcggtgcggttcagcagcatcgggtcgatcacctgcaccggagacacgggcggcaggccgaggattgcgaggcgagccttgatcttgcgaaggtcgaacttcttgccgttgcgagcgagcacgaagtcggcggcgttgagcagtgcccacagcgccttgccctgcttgcgatcatcgaacacgtcgcgcacgttgcgctggtccatgtagaacgacgcctcgtcgtccagccattcgcaagcgaacgacatcagcgaccagtcacgcttgatctgcttgacgctgaagttgttgttgaacatgccccagccatagaactcgatggggaacgtctcgatgtcgaggcagagaatcttcgggccgcgcttcggtgctcggcgaatgaactgggtaagggtcacggtgtctccttgttgatagcccgacgctttcgcgctttcgcattgcgagcgatacgcttctcgtcgtcggtcttgtaggtaggatgcaggtaccccgtgatgttggtgaggtgcgaccgcaggtagttggggatgcccgcacagaatgcgaacacgtcgcgcacgccgtaccggcctgcgttgttctcgaccttgccgagcagggagttgcatccgcgatggagcaccccgcgcacagcgccggtcttgtggtcatggtccagcaccggatcgagcggagccttcaggccgaactgtccctgacagagacagcaccggttgccttgctccgctgcgagcttgatgcgcagcagcttgacctgtgttgcagtgagtcgcttcatgctttgtatgcctccaagattgcacgcttctcgttcacgtcctcggcgaggtcatagaacgcctgcttcagcttcggcccgaacacgtcgagcttcagcacgtcgagcagttctgcgtcacgatccgtccgcatccacagcagcacggcttgctcggcgaatgtcttgcgccagtcggcacccaacacttcgctgtacttgccgctcacgatctgcaccgcttcgaggttggtcttcgtctcgaacagcagctgctccgctgtcaccttgcccaccttcggcagacccggtatgttgtcggcggtgtcgccgtggagcatctgcatccagaaccacttgtgaccgtactgcaatccgttctcgccaacgatgtcgtaagcgccgagcggaacctctgtgatgtcgtagccgtcccagtctacgtgcacgccgcagaacattcgcatgtccttgtcggcgctgtgcaccacgtgcaggatgttgtggtgcaatgctgcaccctcgttgacgtacgcgatgccatcgtcggcctcacgggtcagccagattttgggagtgaaagcgtcgccctcgtatgtctccatccactcacgaaggaacgcccagttgttgggcttgcggcctgcttggcgctgaccctgatacggctgcgtggtagcagcgaggaagcgatcacccttggtagacgcggcgtgcgtcaggtgcatgacgatcttgcccgctccgctgacatgcttcagctgtgcgcagcgggagagcacgttgcgtcgtgcatcccccgccgagcagttctcgctaccagccgcgaagtacgccatgtagtccccatcaacgtgagcgatcacgcgcgggttgtgctgacgtaccacctgcaccggcatcggggagcgctcaccggccgctgccatgagagcgctcaggtccatcaggcgatgcctgccatcgggtcgctaccgtccaccgggaacggcggcttgtcgtcggccggagcagcgtcggtgggcgcggcgttcgccacgtcgccgaccacttcgtccagcgcatcgacgccttccttggtgaccgtggtgctgcccgccaacttggcggcggcgtagtcgtagcacggaagacccttgaagttcagcgccgcagcgatgcgcagctgcgtcttgttcttcgactgcgcctcgtgggtgaccttgccggtcttctcgtccttgcgctccgggtactcgccggggatgtagatgctgtcccacatgtcggcgtcggcgaagtcccacacgaacgcacccagcggggtgatctgctgcggcaccgggatcacggtgtccacgaacttgccggtcgggatgccgttctccatttccggcaccggcatgaccggcttgcggatggaagccttgtcgatttcggcgaaggtcttgttcgggtcgcgcttgcccggcttgtggatgacttccagcagcacaccctgacccagcagctgcacgaagtggcgctcctcggtgcgcaggcggctgaagattttgaagtagtgcgccttctcgttggtggacaggccgagggtcagcgtcatgcgcaccggcaccggaccattgtcggtttcgatgtgcgggtgctgcttaccggtcagctcgaacacgatggcgacttcatcctgcgtcttcttcttgccctcgaactcgaactcgtgcttgcccagctcgtagtacccgacgatgcgggcggtggtcacaccggcagcgggcggggtgtagtcgaagctgccaccactggcgaccgactgatccttaccctgcgtggcgaccttgttcaacagtgcgtcaagactcatgcgtgttgttctccttattcaaacgacgggttgtgattacctacgaagtccttgcggatcgacgcgcggtactcgatgaccagaccggcgaactctgcgggagggttcttctcctccatcatgttgtcgcccatcttggtttcacacgggacgccaagcggcagcgtccagttgaaccaccactccatatacaccgacgcttccagcatcgaggcgtgcagcagagcagcggccttggttgcgatgtcgccgtgtgcatccacgtagacggcatcgtgcacctgattcacgagcaacgcacggcccaaccattccttcggttcggtcacgtacttccggtagaaggcgcgcaggctgacgtacatcgccgccttggcccattcaccaccggtgccttgcatcgggtagttcttgatttccgtgggcgagaacgactgcgcacagccacccttgctcgcgggcttgttggcgatgaacaccggggacggtgactcgctgaaggaatacatcttgccgtccggcgtggtccagtgcgaccggccaagctgacacgtcagcccatgcggcacgccttgctgccccgcgttgggatgcggaacgaagcgctgagtgctgacgcggttgcgcttgatgtgctcgaccatgcggtcgatgtactcgcccagctccgggtaacgctcggcctcaccgcgcaccagcgcctcgacttcttcctccgacatgccggtggtcgcagcgatcttcgccacgcccgcaccgtacgcacgctggaaggagaacaccttcgcgttgccgcgcttcttcttccacttcttgtgctcgggatgcttgtcgtccttgctcgccttcaggatgaagtcgtagtcgtacttgccttgctcaccccacgcctgctctgcacggaggcagtgcatgtcgaggccctgcttcaagtcctcgatcagctgacggcactcggtgaggattgcctgcacgtagatttcgagggaggtgtagtccgactggatgatcttgccaccccggtgccgggacacgaaggcgcgcttgatctgcgaacccttctcctccaacgtctcctcgtccagctcgcccttgctcacgttctgcaagttcggatcgctggaagacaagcggccggtaaccgtgttggtcatgttgagcttgtggtggatgatgccgtccggtcccaccagcgtgagcatgcccttctgctctccggtcttctcgtccgtcgtgatgtagtacgtggacaagtccttgtggatgtcgtcgcgtctggcaagcgccttggtgaacggcaggttgcggtagcccagcgcctcgatcacgtcggcagcggtggagtacacgccgggatcgctcttgctttcccatgcagcatcaggctcggtgtagccagggaactcgaacagcatgtcctcgttgcggaacttctgcttggtcaagtcatcgaccttcaccttcttggtcttgtactctcccttgttcttgccgctgccgtacgtggtgtagcgccagaggttgtcgaagtcctcggccggtggcgtcgccgtcgtggtaccatcgaccagcacgtagtgcacctcgtccttctgcacgtaagtcggcccaccctcggtggacatgatcggaaccttggccgtgtacttcaccttgccgccgaagatcagcgcgctcttgtggaagcggctgttccagttgaaggtcaggccctcgggcagctcggggatgaagccgttgagttcggcggtcgccgttgcaagctcgacctccaactccttcgccttcgtaagcgcccagtccttgtccacgtacatgccgttgtactcggcttcgatggtgaagcacagcgcacccatgttgaggagcgccgagcgcagaccaccacgtgcacggaaggcggcgagctgtccgaggaacatcttctcggtgttaccgatgtcgcccacgtcgtcggtgtcgttggtgccgaggaggtaatccatcagcagcgtcttgtcgatgtcgcaggtgtccacgcccgcagcccacagggacttgactgcatcgtccttcaagttgccgccgtagcgtggagccgtctcgtccatgctcgccatgtggaactcttgcgtcatgccgtgcagcaggtactccgcaagctggcagtcccacaccatgccgccgccgtcgatgaactcgatccatgcctgccggttgagtgggccttggcagatggcgtgcaggatgtcgaacttgatgttgaacccgacgaggaactgctgcccgtaacacagctcacgcagccacccatcgggtgcgccgcccatgtactggttgtctatcccgactcgggtgtcgtagtacaggccggtgttccgtgcgtcacccttccgcttgtagccaatcgccacgatcttgttcatgtcgtagaacggattggccttgcgcttcaggatggaacggatcgtggtttcgaggtcgaaggaagtgaagctcacagcggccaccgttgcagggccagctggtacatttcatccgacgcatcgccatccaagtccagcccgtcgcgcacccaacggaacacgatgatgcggtc

SEQ ID NO: 10 - DNA, 44415 bp, unidentified
  source 1..44415: mol_type = genomic DNA
gcgagaacatgggctaccgtgtcgagccgtactatgcgtaagctctggctgcgcatcctgatcctgctgtactggatcgtgggtcgtggcccgtgggttgtcgtcggccagtaccatgacgacgacggcaagctgtgccggttccgcaccggcccggcttccactgggttctcgctgacgttcgatgacctcggcgcagccaacgactactgcgaccagcgcaactggaaggcagacactgacccgctcggcaccacgtactacgtgtggcatgagttggagttcaatcacttcggaacgaggaggaagtaaccatgggtttcatggacaagatcaaggctgcggccaagtacgtcaaggacaaggtggtcgcagcggtgaagccgcgccacgatgacgacgacacgccgccgcctgcgccggacaccagccggcacctgcacgtcagcgtgccgctgattcccatcgacaacccgatcctgcgcaagatgctggggcaggactacttccccgtgcagaaggggcagggtcagacccgcatcgtcggcaacaaccagctgaagcgcgtggccgatagcctcggcgggaacaacaagcagcgtcgcaagctgcgctcccgcatgaagcgtcgtgctgccgagctgcgttccggtgcatcgttgcagcccaacgtgcagtccgcactggcaggtgcagcatgagcctgcgcatgggaagctgggtcgaggtgactgtgcccgacagccgactgctcaacgtgcagccggagattgccgccgccgtgaagctgatcggcggtgcgaccatgaccaatggccgtggcctgtacgtccgcaaggacaccggcgcactggacgacgaggcggtgaccgtgatccgcttcgacctgaacttgcacagcgagctggtggaccagtacatgagcgccatccgcgccatcgtggaccgtctgctggtgctgggtgaggagagcgtgctgcgtcgccgcttctacaatggcggcggtgggtacaacagcgagctgatctttcagtaacccgagccgggtaggctacgactggcccacgtacgggccatcctatcaaccgtcaagaggaaccatctacatgtcgaacgaaaacaccaccgagcagaccaccgtcagccactacgaagccaagcgcgccgagctgctggaagacatcgccaaggcgcaggccaaggtcgatggcctgaacgagaagctcgccaagctggatgccgtcgaggccaacagcgccgccatcgaagcgctgaaggcgggcgacgccgtgtcctacctgttcggtcgtgccctgaacaagcgcgtcctgtccggcgtgatcgtcgccaccggcaagaacgacaagggcgtgctgcaactgaaggtgcagaccggcgaaggtctggatgccgagctgaacctgatcgacagcagcgccctgctgatgtcggccgaggaagtgctgaaggcgcaggaagaaatcgacgccgccgttgccgaggcccagcgcctcgccgccgaagccgctgccgccaaggctgcgggtggcgaaggcgggcagtcgtgagcctcgccccgccgtcacccagcgtggccgtcgtcaagcgtggcgacgagctgaagcccggccagaatgcgtacctgatcgacacgcggcagaccaacaagctgccgaagggcaccgggttcgtcgtgtccaagctgaccagtgaagacggctcccgtctgatcgtcagcacggacggcaacggctccgtcctgtacgccaccagccacgacatcttcgaggtctgggaataaccaagcgaggatagcatgagcgatacccttcccgacaacgactggctaccacatgccgagcgcctgcctgttggtggccgcacacgtgtggcccatgagtgcggggagggtacgcccttgcttatctcacgagagcacgacaagtccaccgcattctgtttcaggtgcggtggcacaggattcaagcgtgagcacgagagtatcgaggccaagcttgcacgaatccacgccgagcagacgagcgaacgcagagtgcgtgcgactgttgagttgccagagccacgggtatacgacacccgcgagtggccgctcgacgctaaggtgtggttcttcaagatgggactctcgcttcagatgatcgagaagctgcggctgtactggtgcccaagcatcgggcgggtggtactaccgatcactgaaggcgacaacgtggtatactggacagcccggtcggcaacgagacagccgaagtggctaacacctgacgttccgaaagacggacttgtcgcacgctacggcgtgggcacaggtgacaccatcgtactgtgcgaagacccgctcagtgcatacaaggtgggactggtaaccgaagcgtggtcgttgctcggcaccaagctgcacaacaaagtgttgaagcagctgactgatcgaggccaacgtgtagcgacgtggctcgatgacgacagaggtagaagcaacggtagcaatcccggccaagacagtgcgcgagtaatcgctgcgcgtctacgtgcgtttggtctggactacaggaacatcacgtcaccacgtgacccgaagtattacacgaccgactacatcaaggagaagctgcaatgagcaaacccatcgtgcgctaccggcgcgctatcatcccgcccgtcgttggcttccgtgccacgctcggcggcgtgcttgcgcatccgaacctcggcgactgcgacatcgtgcacacctcgacggtgctgtatgtggcggacggcgggcgcaagttcgagacgcgcaacacccggtatcaccagctcgattccaagtacgaacccgaaggagaacctgatgagtcttgacaccacgctgctgcggttgtgcaccaaccgtggcaagttcgaccggctggtacccagcgcaccacgtgatgggctggacgagctgaccgtgctgatgctcgatgcgttgcgtgcgtactacaaggagttcccggacacgaaggacttgccgttcgatgtgttcgatggctgggccatggagttcaagtggaagacgcagcccgacgacaagaagtccctgctcaaagttctgctgaagcagatgcgcgagccggtcccgcccgaggcagagcagggcatgatcgagaagctgttggagttggagcttgccaccactgcggtcagcaagatcgtgcagtggaatggcggcgctgagttcagcctgcgcgacgagctgtacggcttggccgagacgatcaccgaccgaatggatcgcaaggcgcggctcccgctggtgcaggagacgcccgaggaactgatgcagatggacgagcacgacatcggcatccacttccgactgcccacgttggcgaagaacctgcgcgctctgcgtggtggtgacttcggcatctacgccatgcgtcccgacgcaggcaagaccacgttcctgaccagcgagtccagccactggatcacgcagctcgacaacgtttggccggaccagaagcgcaccggcatctggctcaacaacgaggggccgggcaagcgcatcaagcagcggtggtatcagtcgctgctcggcgctaccatccctgagatggtggagtgggcgaaggatggtagcatccgcaagcgcatcgaagatgcgatgggcggggacatccaccgcatgcagttctacgacatccacgggttcaactccggtgaagtcgaggccatcatcaagcagaccaaccccggcttcatcatcttcgacatgatcgacaacatcacgttcaccggtggcatgaccaacggcgggcagcgtaccgatcagatgttggaggcgatgtatcaggccgctcgcaactggtgtgtgaagtacgacgccgtgggcgtggcgacttcgcagatcagcgccgagggtgagggaatccagtacccgccgcagtccgcactgaaggacagcaagaccggcaagcagggtgcgtgcgacttcatcatcatgggcggcaagctcaatgacccagcgatggaacgcttccgctacatcggcaccccgaagaacaagctgcaccgcgcaggcggcaagcgtgacgttcgggaagaagtgatgatggatgcagagcgtgcccgcttctatcaggaggcagcatgagcaagccaattcacatcgtagccaccgggttcacggtgtcggtcagcttccccggtgaatccaccgaggcgaagaccttcaactgcgtgagcaacgcgcaagcaatccaccttgccaagctgctgcgcaaggtgcacgacgcaggctacatcgaaggccgcaacgacgcgccgcagtggaagtggggatggctgcggaacaaacacagcacttggatcggcgtgcactactcgccgcacaacaagcgctggtgcatcaatctgatcccgtgcttcacgttctggatcaccaagcccggaggtaacacaccgtgagtaccgaaccgaacatctacctgccgcgcaacgtgggcgtcatcacgtccagccgcaccggcagcagctacacagtcgagccgcccgtgaccgacacggacatcgacttcctcgtgctggtgcaggacttccacgaggccatcgaaaagctggtcgatcagggatggaccctgtgctccggtgccgatggacactacgaggaggacgaggactacagcaccacgtggtatgcgctgcgcaacggcgtgttcaacgtcatggtgaccgccgactccggctggtatcagcgcgcggtcgaggccaccaccatctgcaagcgccgcaacatcaaggacaagcaggaccgcatcatcgtgttccgttgggtgcgcgacgggctggacttggatggcgatgcgtcggatgaaatgtaccagctggccctgcaacggtggccgctgtgagcttcacttccttcgacctcgaaaccacgatccgttccatcctgaagcgcaaggccaatccgttctacgacatgaacaagatcgtggcgattggctacaagcggaagggtgacgcacggaacaccggcctgtactacgacacccgagtcgggatagacaaccagtacatgggcggcgcacccgatgggtggctgcgtgagctgtgttacgggcagcagttcctcgtcgggttcaacatcaagttcgacatcctgcacgccatctgccaaggcccactcaaccggcaggcatggatcgagttcatcgacggcggcggcatggtgtgggactgccagcttgcggagtacctgctgcacggcatgacgcaagagttccacatggcgagcatggacgagacggctccacgctacggcggcaacttgaaggacgatgcagtcaagtccctgtgggctgcgggcgtggacacctgcgacatcgacaagacgctgctgatggattacctcctcggcaccaacgacaccgacgacgtgggcgacatcggtaacaccgagaagatgttcctcggacagctcgccgccttccgtgcacgtggtggtctgcgctcggcgctcctcaacatgggtgcgctgtgcttcaccatcgaagccgagtacaacggcatgtacgtggacaaggactgggcgcttacgaaggcgaaggagttggaggtcgagcttgcaacggcgaccgccgaactcaacggcttcatccccgagctgcccgagggcctgaccttcaactggaacagccgcttccacaagagcgcgctgatcttcggcggcaaggtgaagtacacggccaaggttccgatcatgtccaccgagggtgggccgacttacgtgcagaaggacgaggtgcactacgtgctggtcgatggtaccacgacggcgacgccaccggccgaggacttcgacaacctctggcgctacaccacgtacggcagcggcaagaacaagggagagtacaagaccaagaaggtgaaggtcgatgacttgaccaagcagaagttccgcaacgaggacatgctgttcgagttccctggctacaccgagcctgatgctgcatgggaaagcaagagcgatcccggcgtgtactccaccgctgccgacgtgatcgaggcgctgggctaccgcaacctgccgttcaccaaggcgcttgccagacgcgacgacatccacaaggacttgtccacgtactacatcacgacggacgagaagaccggagagcagaagggcatgctcacgctggtgggaccggacggcatcatccaccacaagctcaacatgaccaacacggttaccggccgcttgtcttccagcgatccgaacttgcagaacgtgagcaagggcgagctggacgaggagacgttggaggagaagggttcgcagatcaagcgcgccttcgtgtcccggcaccggggtggcaagatcatccagtcggactacacctccctcgaaatctacgtgcaggcaatcctcaccgagtgccgtcagctgatcgaggacttgaagcagggcctcgacatgcactgcctccgtgcagagcaggcgtggggtgagcaaggcaagtacgactacgacttcatcctgaaggcgagcaaggacgacaagcatcccgagcacaagaagtggaagaagaagcgcggcaacgcgaaggtgttctccttccagcgtgcgtacggtgcgggcgtggcgaagatcgctgcgaccaccggcatgtcggaggaagaagtcgaggcgctggtgcgcggtgaggccgagcgttacccggagctgggcgagtacatcgaccgcatggtcgagcacatcaagcgcaaccgcgtcagcactcagcgcttcgttccgcatcccaacgcggggcagcaaggcgtgccgcatgggctgacgtgtcagcttggccggtcgcactggaccacgccggacggcaagatgtattccttcagcgagtcaccgtccccggtgttcatcgccaacaagcccgcgagcaagggtggctgtgcgcagtcgttctcgcccacggaaatcaagaactacccgatgcaaggcaccggtggtgaatgggccaaggcggcgatgtacgtcagcctgcgcgccttctaccggaagtacgtgaccgaaccgaaggaatggttgggccgtgcgttgctcgtgaatcaggtgcacgatgccgtctacgtggatgcacacggcgacatcgcaaccaaggccgctgctctgctgcacgcctcgatgctggaagcgtcggtgtatatggagtggtggttcaactggacgctgccgcttggcgtcccgtgtgaaaccaagatgggcgacaacatgatggaggagaagaaccctcccgcagagttcgccggtctggtcatcgagtaccgcgcgtcgatccgcaaggacttcgtaggtaatcacaacccgtcgtttgaataaggagaacaacacgcatgagtcttgacgcactgttgaacaaggtcgccacgcagggtaaggatcagtcggtcgccagtggtggcagcttcgactacaccccgcccgctgccggtgtgaccaccgcccgcatcgtcgggtactacgagctgggcaagcacgagttcgagttcgagggcaagaagaagacgcaggatgaagtcgccatcgtgttcgagctgaccggtaagcagcacccgcacatcgaaaccgacaatggtccggtgccggtgcgcatgacgctgaccctcggcctgtccaccaacgagaaggcgcactacttcaaaatcttcagccgcctgcgcaccgaggagcgccacttcgtgcagctgctgggtcagggtgtgctgctggaagtcatccacaagccgggcaagcgcgacccgaacaagaccttcgccgaaatcgacaaggcttccatccgcaagccggtcatgccggtgccggaaatggagaacggcatcccgaccggcaagttcgtggacaccgtgatcccggtgccgcagcagatcaccccgctgggtgcgttcgtgtgggacttcgccgacgccgacatgtgggacagcatctacatccccggcgagtacccggagcgcaaggacgagaagaccggcaaggtcacccacgaggcgcagtcgaagaacaagacgcagctgcgcatcgctgcggcgctgaacttcaagggtcttccgtgctacgactacgccgccgccaagttggcgggcagcaccacggtcaccaaggaaggcgtcgatgcgctggacgaagtggtcggcgacgtggcgaacgccgcgcccaccgacgctgctccggccgacgacaagccgccgttcccggtggacggtagcgacccgatggcaggcatcgcctgatggacctgagcgctctcatggcagcggccggtgagcgctccccgatgccggtgcaggtggtacgtcagcacaacccgcgcgtgatcgctcacgttgatggggactacatggcgtacttcgcggctggtagcgagaactgctcggcgggggatgcacgacgcaacgtgctctcccgctgcgcacagctgaagcatgtcagcggagcgggcaagatcgtcatgcacctgacgcacgccgcgtctaccaagggtgatcgcttcctcgctgctaccacgcagccgtatcagggtcagcgccaagcaggccgcaagcccaacaactgggcgttccttcgtgagtggatggagacatacgagggcgacgctttcactcccaaaatctggctgacccgtgaggccgacgatggcatcgcgtacgtcaacgagggtgcagcattgcaccacaacatcctgcacgtggtgcacagcgccgacaaggacatgcgaatgttctgcggcgtgcacgtagactgggacggctacgacatcacagaggttccgctcggcgcttacgacatcgttggcgagaacggattgcagtacggtcacaagtggttctggatgcagatgctccacggcgacaccgccgacaacataccgggtctgccgaaggtgggcaaggtgacagcggagcagctgctgttcgagacgaagaccaacctcgaagcggtgcagatcgtgagcggcaagtacagcgaagtgttgggtgccgactggcgcaagacattcgccgagcaagccgtgctgctgtggatgcggacggatcgtgacgcagaactgctcgacgtgctgaagctcgacgtgttcgggccgaagctgaagcaggcgttctatgacctcgccgaggacgtgaacgagaagcgtgcaatcttggaggcatacaaagcatgaagcgactcactgcaacacaggtcaagctgctgcgcatcaagctcgcagcggagcaaggcaaccggtgctgtctctgtcagggacagttcggcctgaaggctccgctcgatccggtgctggaccatgaccacaagaccggcgctgtgcgcggggtgctccatcgcggatgcaactccctgctcggcaaggtcgagaacaacgcaggccggtacggcgtgcgcgacgtgttcgcattctgtgcgggcatccccaactacctgcggtcgcacctcaccaacatcacggggtacctgcatcctacctacaagaccgacgacgagaagcgtatcgctcgcaatgcgaaagcgcgaaagcgtcgggctatcaacaaggagacaccgtgacccttacccagttcattcgccgagcaccgaagcgcggcccgaagattctctgcctcgacatcgagacgttccccatcgagttctatggctggggcatgttcaacaacaacttcagcgtcaagcagatcaagcgtgactggtcgctgatgtcgttcgcttgcgaatggctggacgacgaggcgtcgttctacatggaccagcgcaacgtgcgcgacgtgttcgatgatcgcaagcagggcaaggcgctgtgggcactgctcaacgccgccgacttcgtgctcgctcgcaacggcaagaagttcgaccttcgcaagatcaaggctcgcctcgcaatcctcggcctgccgcccgtgtctccggtgcaggtgatcgacccgatgctgctgaaccgcaccgagttcgccttcacctcgcagaagttggagtacaccaccggcgtgatcgtgccggagctgcgcaagtacgaccaccacaacttccccggcttcgacctgtgggtggcctgcatgcagagcctgcccggagcatgggacgagtgcgaagcgtacaaccgcatcgacgtgaagtccatgaagttggagtacaagaagctgcgcggttggtactcgcagcatccgaacgtcgcagtgtactacaaggccgacggcagcgagcaccgctgcaacaagtgcggctgcaacgaaatgatcccgcaggatgatccggcccgcacgcaggtcggtacctacctcctgcttcagtgcaccgtgtgcgacggctacagccgtgggcgcaagctcacgaccagcgccgaggcgcgcaagcacatcaccgtcccggcataaggaaccgacatgaagatcaccgacatccgcagcggcatgcgggtacagtacatcggcaatgcgcccgcaatgatcgggctgcgtggacaggtaagccgcgtgttcgctcgtgatgtcgaggtcttcttcgacggtcgagttaagccgagctgctgcgttcccgattccctccgacagcttctcagcatcggaggcgtgaccaccaccagacgagaggtaccaatgcccgaactgagctaccgcgacgaggaccgtcgcacactgtccgaccgtggcgtcggcctgaaggatgacgggggcaagccgcaggcccgtctgctgcatgagggcgtgccgcgtgcactggcccgagtcatcgacaccctgaccttcggcgcgcagaagtacaaagcgcactcgtggcagcatgtcgagaaggcgctcgaacggtatcaggacgcgagctaccgacacgacaacaagcgctgcctcggcgagaagctggacccggagacgggcatccaccaccgggcgcaccacatcatcaacgagctgttcctgttggagctggaactgcgcgaggaggagaaggccagtggcgcagagtaaggcgcgctccatcaaagaggcttgggtgaacatcggcatcggctacagcatcaactacgcagcgaacatcgcgctgcttccggtgctgtggcatcccgagcatccgctgctgtcggcgcacgccatcggcattgcgttcacagcgatcagcttcatccgccagtacatcatccgccgctggttcagcaagggtgactgatggcctgcgcccgctgcggccaagtgcatcggtacgtcccacatgaggccgagtgggcgcgcttcctagaggagcaccgtacccgcaagcagttcgatgtcgagtgggccaactcactctggcatcgtacataccctgacgacgcattctgcatcctcgtgatgaggggcctcgcaggtttcgttccattcccgtcgaaggagaactgaatgctctacaagaaccagaccgccatgctcatcaagtcctacgagaacgccgttgcgtggggcgagagtgccgaccacgaggaggcattgcagaatgcggtcaaggccgggttcccgaacctgcccgacgaagatcaggccgagctgtatacccgcatcgccgatgcgtgggaaggctaccgtggttcgctcgctccgcgcaagctgtggatcggcaccatcgtcaaccagttcatgtcgtcccgcatcgcacggttcaacgccgcgctgggtgacggcaccaagaaggaggacagcgccgatgtttgatgtgcctcgccagaatgtccgggttgctcccggctacaagaagcgcaagcgcggcttcaagatcaaccgcgccttcaccaagggcaacttccgcgtgcagtggtacgacggcaaggccacgtactgggagcgctacgttccgtggtacgaagtgccgctcgccatgttccagatttggagggactacgcatgagctacatcgtccacaaggcagtcgagcaggacaagatcaagaagaagctgcggcccaccgaggagcagcttcgcaccgagtacatcgcacagccgaagtacgacggctgcaacatggtcgccatcaagcgcggccactgggtgcccacggtgaacaagggcctgcatgccatcaaggtgggcgacgtgcagatgcagccggtggatcgtggcgtggttgacctgttctcccgcaccggtgagcaggtcgtcagcgcacaccacatcgagaacgctctcgcatccgcgccgttcttcccggtcggcgtgtacttcggcgaatactggcacccgcagatcgaccagcccaccgtcagcggcatgttccgcaagaaggacggcacgcagtacaccgagccgatgttcgtggtgttcgacttcgtgacgctggaagaatgggagcagggtttcagcgacctcgtgtatcaggagcgcgtcagccgcctgccgagcatgggccacgccatcgccgagggcaccgcgccggtgttctacgccgagtcgcagggcttcctgatcgaccaagagctgggcagcatggaagcggcgaagctgctgtgcgagggcggcgcgtacgacgggctgatcctgcgcaagccgagcggcaagtgggtgaagggcgacaagggaaccaacggcgaagtcgtcaagatcaagccgaccctgacgctggacctgcgtgtgctcggcatcaacgaagcagtcggcgagaagaccggccgcgccgtgtacacggtcgtcgttgacctcggagaaggcaagacgcaggaggttggcagcggcgtgccgcacagcgagagcgagctgcctagcgtgggaggcatcgtggaaatcgaggcgatgtccttcagcaagtacggcctgctgcgcgagccgcgatacaagggcatccgtcacgacaagaaggaggcagacctgtgagcgtcgaggtgcaagcatggcacaacatggagcgcgacacggtggagctgcgcatcagcgttcctttcggcgagtacgccggttccctgtggccgaacgagacgctgcgcgacaaggtgcaggaagcgttcgccaagttccttgacgagcggaggggctgatggacgcgatcactttcgagaagccggagctggacttcagccagtcctcggcatggatgggccgcgtcgaggtttcggtgcgcgcccggtacggtgccgacttgttcggcgctgctgccacgtgcatggccgaggatatcggcggtgaggcgtggccgcacatcatccacgacctgcacatggaaatcatgcgcggtatcctgaaacgctacccgccgcgcgactacaccgtgcggcagcaacggaggtaacaatgctctcgcaagtggaactcgaactggaaacctacgccttcggtaaggagcgcatggagaagtccatcgcccgcaacgaggagaagggcggcgcggacaacaacccctacgcccaagcagtgtatcgccggttcgtgcttccgcttgcggagcgcatccgtgcggacatcgactctccgcgaatcggccgtgcgcaagcgcacgtgccacttctgcgcgccaagtacgatcccgagcgtcagaacaagcgtggacagcccgtcagcgccgaggaacaggcacgcgagtggtacgaggctgtggccttcgtcgccgttcgcggtgcccttacctcctgcatgcgagacaagcacggcgaaggcagcgaccgcgacgtgttgaagaacgttggcatcaacgtgtaccatgagtacctgctgacgcagttcgccgacgcggagccgactctgttctaccacctgatgaacgacatggaccgcaagctctctgtcaacgagaaccaccgcatgacggtgatgaagatgcaaggacgcaagaacggcatcgagttcgtggagtggggacaggcacagcgcgatcaggtcggcgcgtacctgtgcgatcagcttgcgcagctgggcatgttggagattggcgtggtcaccgagactgctgccagtgcaggcgcagcgtaccgcaagttccagaccaagacgcacgtcaagatcgtgctgaccgacgaggtgcgcaagctgattactcagatcagcgacttcgtgatcgaggccacgccgttctacctgccgtgcgtcgagccgccgatggactgggtggacatcgacaacggtggattccacacgaaggaaatgcgccgactcaatccgtggatggtgaagacctacgctcagacccgcgacgagtaccgcgctgccgagctgcgcaacgagatggctgcgatcaacgcattgcagcgcgtgccgtggcgcatcaacaagcgactgatggaagctgtgtcggccatcgccaaggtgcacgacatggaggaaatcatttctcagggcgagctgccgaagccgcgcaagccggagtggctgacgaaggacatgaccaaggaaaccatgtcccacaatcaggagttggagttcaagcagtggaagcgcgacatgtccaactggcacaccgacgagcgcctgcgacagaacaagggcaatcgtttctacaacgcaatgaaggtggcgcgcaagttcgccgagtacccgagcatctacttcgtgtacttcgctgacttccgtggccgcaagtacgttcagaccaccggcgtgtcgccgcagggttcggacttgcagaaggcgctcttggagttcgccgatggcaagccgctgctgactaaggacgcgaaggattggttctgcatcacaggagcaaaccgatggggatacgacaaggcgtctctgccggatcgtgtgaagtgggtagcggagcatcacgaccagatcatggcgttcgctgcggacccggtgaacaacgacgagtggaagaccgccgacaagccgctgcaatttctgagctggtgcatggagtacgagcagtggcaagtgttcggggatcgcttcctgagccgcatcgcagtcggcatggacggttcgtgcaatgggcttcagaacttctcggcgatgctgcgcgacgcagcaggcggcgtggcgacgaacctgatcccagcaccgctgccgaatgacatctaccagatggtggcagaccgcgtgactgccgtcctgctaggcgaggacgaggatgccgaagggtaccgcacgctgtggctcgaccacggcctcacacgctcgctggtgaagcgcagcgtgatgaccctgccgtacggctcgcggcagtcctcgtgggcggacttcatcatcgaagactacctgaagtgtgggaagttcccctcgctcgacaaggccctgtacggccccgcagcgcgcttcctgagcaagcgcatgggtgaggccatcgccgacaccgtggtcgccgcagcgggcgcgatggagtggttgcagcgcggctccgggtcgatcctcaaccaagggtacgaccgcatccggtggatcacgccgtccgggttcccggtggtgcaggtctactgggagtccgaggagcaccgcatcaacaccaagctgtgcggcaacgccaagctgtccctgcgcaagagcacggacgcggtgaagaagtcccggcaccgcaacggcatcgccccgaacttcgtgcacagcctcgacgcaagccacctgacgctggtggtcaacgcggccaaggccgaaggcatcgacgccttcgccatgattcacgacgacttcggcacccacgccgccgacagcgcggcactgtaccggatcatccgggaggtgttcgtgtcgatgtacgagcggcacgacgtgctgtcggccttccactcggcctacccgttcctgccggagccgccgccgatgggcgagctggaccttcggcaagtccttgattctccgtacttcttcagctgacggagtttcagtacacctatagcacgaggcaactgaggtccggttggagcggccgcgaaggtaagcggaaccggtgccggaccttttggtacacctatagcacagaggagacaccatggccgaagacgccaaagtgaaagtcctgatgacgctccacccgaaccagctggccgccgtgcggaagctgtccgggctgtcgctgtccgtcaactcgaataccacgcccttggaggcaggtatgcagttggggatggcccgcgtcctgaacatcttacaggagggtttcaccgttgattcctccgtaccgaacaccaacgacgggtgatagtgagcagatcaaggcggctttaacggccgctttgtatctgtcatctagagaagatagtaaggtagacaacagagaatcttctgtgagctacaactgtgatgaccctgattacacagtggccctgataacacagggtctagtggatgcagtaatcattgatgaagcctacctgctgtgctttgccattgtcacaccgtggtactccaagaaccgtactacgttcgttgagaacatggtgctgcgaattgggccgggcagttccttcgaccggtacatagccgtgatggaacatctggctgacatcaaccactgcgactcactgagcgcaggcggtgcactagctcggaactcccgagcactcacacggatgtatgcacgctacggctacctgctggaacggcatgctccccaattcaccaagcgaaggagttaacctatgggtagcatcgttggtggtgggtccgccaagcgagcagcgctgaagcaagctgctgctatcgacaagcagaccaacctccaaactcaatccacgaactaccagattcaggcgatggccgatcagatggcacaggcagctgcacagcaggccgcatctgagtacgccgagaagttgctgagtgcccccgtcgataccgtcgatgtgcggctgggaacttccgacctcgacttgcagactgccgacctgatcggccgacgcaagaccgcccgctccacttacacccgacccgtgaccacgaccgcagcttcccggctgacgaccgtggccgggtcagacctgttgtgaggtgagcatggaccatccgatccaaaccgctcaccgccagttcgaggcttacgacaacaagcgacagggcatcatgtaccgactcgaacgctattcgagctggaccgtgcccaagctgttccctcgcaagaaccgcgatcaggacaccgagccgctgacccacgggttccagtctctcggcgcgcaggcagtgaaccatctggcgaacaagctgatgatgtcgctgttcgcaccgtcccgcccgttcttccggttggagctgaagcgcaaggcgaagcaggctgcgcaggagcaaggcgctgacttgcaggccatgcaggcgatgcttgcgaaggccgagcaggatgccagtctcgaactggacaagcgctccatccgctcccggctgtacgacctgctgaagatgctgatcgtgctgggcaacgccctcatggtgttggagaaggacacgatccgcgtgctcaacatgcggcactacgtggtcaagcgcacccgcaccggcgaggtctacgaactgatccttcgggagaaggtgcacaagacccagctggaacccgcagcgctcgctgccattgtcgcgcacccggacttcaagcccgatgacgacggcatggtgtgggagtacaagtgggtcaagctggaccacaagaccggcaagtacaacgaagacgtgtggatttgcaactgcaagctgcccgccaacttctcctcgacctacaccgcagacaagctgccctaccgggcggttagctgggacttggccgcaggcgatgactacggctccggcttggtcgaagactacgaggccgacttccagtcgctctcgatgctgtccgaggccgcagtgcagggcgcgatcctcgcctccgagttccggtggctggttaaccccgcaggtcagacctccgtcgaggacttcatggcgtcgcccaatggcgcggccattcccggcatgaagggtgacatcgagctgattaacgcaggcgtcgatggcgtgctgcaaaccaaccaagcaatccagtccacctacatcaaccgcatcggcgcaggcttcctgttgcagacggcggtgactcgtcaggcggaacgtgtgaccgcgcaggaaatccgcatggtcgccgaagaactggaaggcgggctgggtggcggctactcccggatcgctgcggacgtgcaggtaccagtcgccttttgggtgatgaacctgacgggccgcgacatccgaggcaaggacttggagcctgtcatcatcaccggcttggccgcgctctcccgtacgggtgaccgtgaccggctgttggagttcggcagcaacctcgccaacgtcctcgcactgccgccgcagattctcgaacgactgaagctgtccgcgtggatcgcagacctcgccgccgctggtggcttggacccgaacgtctacgtgctgactgaggccgagtacggccagatgatgcagcagcgtgcacagcagcagctcgccatgcagaacgcatcccagcagatcgacaacgccaacaacatggagacacagacacaatgagttccaacgcacctccgggcggtggtcccggcgcaaccgtgatcgcaacctcgaacggcaaccagcccgcaccggcagctccggctcccgcagacgacaagctgttgcccaacggccagcccgctccggccgcaccggcacagcccgcagctcctgctgcacctccggctgctgacgcgctgagtctcgaacctgccgctcccgcacagcccgccgccccggcgaacgctgcgccgactgcggtgtcgatcccggactacggcgacaacggcctgaacatcgcggccgaatacttcgtcaacaccgtgggcctcgacatcgacagccgcgaactgaccgaagcagcgaagggcaacttcgccctgctggaagccaagctggaagtcctcggcgacaaggccaagggttccgcaccgatcctcgctctggcgaaggagagcatcgctcgtgtcaccgccgctgcaaccgcagcgcacgccgcgaacgttgctgctgtccacgaagccgtgggtggcgcagagaactgggctgcgatccagcagttcgcacgggccaacctgcccgccgaccaactgaagcaggcaagcgaatcgctgtcggctggtggcttcggcgctcaggcgaccgcgcgttacctgatggctctggcacaggccaatcccgcgacgaccgtcaagggcgcaccggctaccaacgccgccgcccccgccgcgtcgatcaacggcgtcgctcctatcacgaaggagcagtaccgcgctgagtaccgcaagctggttgccgagaagggcatccgtggtgcggcccactccgaagaactgcgtgcactcaacgcgcgcgtcatccactaagaccaaggagcaacacaaagcatgagcaccatcttcccgactgtcccggttctgccgaatcaggtcaaccagtccggcaacgagaacgccctgatcctcgaacagttcaccggcgatgtcgagcacacctacgtgtccagctcggtgctggaaaagttcttcccgcgcaagcaggtcaagggcaccaacaccctgaccaagaaggccatcggccgtaccaagcttcagaagctgaagcgcggtgacgcgccggacggcaccccggtggacttcagcaaggcgtcggtgaccgtcgataccatgctgctgtcgcgtcacagcatctggcagctggacgaaatcttcaccgacatcgacacccgcaaggaaatcgccatcgagcagggtcaggaaatcgccgagttcgtggacctgaccatcagcatcgccgccgcgaaggccgctgctgccacgcagtcgatcttcacccgcaacggccgcgcgcccgagggccacttcggtgccacgcaggtcgtgctgtccgccgctggtgacgagaacgatccggccaaggtgtacgccgccatcggcaaactgttctcccgcatggaggaggagaagaaggtcaagccgcagcgcgatggcgtggtcctgatcgtgcgcccggcgatcttctacctgttgcagcaggccgagcagatcagcaacggcgagtacctgacctcggacggcaacaagctgaccggcatcccgaccttccacggctggggcgtcccggtgctgtcgagcgagaacctgccgaacaccgtgatcgaaggtcacctgctgtcgaacgacgacaacgacgacttctacgacggcgacttcagcaccctgatcgccgtggccgtgtcgccgaaggccctgctgatcgccgaagcgctgccgttgcagtcctcggtgtggtggagcgatgcctcgaagtgctacttcgtggactcgtggatgtccttcgccgttggtctggatcgcgtcgagaacgcgggccgcatcgacaaggttgcctaatccgctgggcgcggtccctgaatccttcgggtaactcaaaccgcgcccttcttccaccaacacaggagcaacatcatggtctttgaccgaccgttcgagatttccaaccgcgtcgtcgccgcaactggcgtggccggtctgcccgccaactccgttggtaccgtcgtcggcgtccactacgacacccgtggcaccgcaggctgggtcgtccgtgtccgtttcgtggacgacgaaatcggctcgcaggacatcgagtacgcaccggccgctctggctctggctgcggactaagcaacatcccggcaggggcgctccggcgtctctgccttgttcctctcaggagacaccatggcattcatcaccaagctcgacatcgtgaacgcctgcttgaagacgatgggcgagacgaagctcaacacgctggaagatgaccacgtatacaaggacgacgccgttgacttgatcgaccgcgtgcaccgtgacgtgtcctcactctcgctgtggttcaacaccgaatgggtggagctgaagccgcaggcaacgagcaagtacatcatggtccccacggacgtgctgaagctggactgcaacccgagccggttcggccacgtggtgcagcgcggacgccgactgtacgaccgcaagcgcaacacctacgagttcgaccacaacgtgcaggccaagctggtgcggctgctggacttcgatgacctcccctacgaggtgcagatgttcgtgcgcgacgactcggtgctgcggttccagtctgacttcgacggcgacaacaccaagtacgccaagatcaagcagcagcgcgatgacagttacatcaacttgaaggccgagcacatccgccagatcaaggcgaacccgctgttcgctcgcgcatccgtggacgtgctgcgttcccgttactggaactacagcggtcacccgtggcacagccacgtcacattccccggctaaggagacaacatggcaaaggcaggcggaacctatcccgacatccttcagggtgtcagtcagaaaccggcgcatcgtcgtcggccgggacagacgcacgagcagatcaacgtgctgtccgatccggtgaacggcctcgtgcgccgtcgtggtacgcggttcgctgcttcccaagccgttgtcacctcggccgagctgcgcaacatggacgtgttcgacttcatgcaggagggcaaggagtacgcgctgctgtaccggcgcgacgcctcgaccttgggcagcgagtccttcgcgttcctctacaacaagacggacgagtcgttcatccctctggtgtacgagaacagcacgtgggtcaacacgctggtcagcggaggcgcatcgtcgctcacggccatcggcagctacgtctacatcgcgggcaacaccacgatcccctcggccaccagcacgaacgtgtggcaggagcagacgaacatccagcgcctcgcagcatgggtgcgcaccgggaagtacaacaccacgtacacggtgaacctgacgcggacggacaacacggtgctgacggtaacgttcaagacggttaccgcatcgtaccccggaacgctcgacaccagcgacatcccgttctaccttcccggtggcacggagccggacgcggcgtaccagaagtacgtcaacgaccgagtgaacgagtacaactctgcggtcaacgagtggatcgtgacgagcgctgagcagacgcgcccggagtacatcgcggagcagctgtcggatttgctggtcgatgcaggcgtgtcggcaacgtacatcaagggcgggatcatcattgacgatgaccagttcaaggacatcacggttgacgacgagggagacggcacgaccttctacgccgcagggcaggaaattacagacgcgacctacgccgtcaagttccactggcacggcaaggtcattcgcgtgcggccgagtggtgcaggcgcggacgagtcgtactacctgcgcgctgagttggagaacggcgagacttccggctacgggtcggtggactggtacgaagcgcccggcgtggagtgcaccatcgacaacctcgtgtcgcagctctacatctacaacggtgtaggctacatcgcacgcaacggtgcgggcctcacgtctctggctccgagcagcggcgagcatccggcctacggtgcgcgagtggcaggcgatggtctgacctcgccgatcccgtggttcatcgacaagccgatcacgatgctgtccgtcttccaagaccggctggtcatcggcgcacagaactacgtcaacgcctcacgctcggcggactacctgaacttctggcgcggctcggccgtcaccatcgaagacagcgaccccatcgaaatcttcgcgcacggcagcgagggcgatgtgctccggcacgcgacgctctacaacggcaacctcgtgatcttcggtgaccgtcagcagtacggcatcagcggcgactcggtgttcagtccgaagaatccgctgattaaagcgttcagtgccaacaaggattcggttgacgcgaaggcgcagacctcgggcaactacatcttttatgcgcagtacggcagcgaaggcacgagcctgcaccagatgcgagtgggcgcgctcaacgggcagcagacggtgacggacgaaatgtccaacgagctggactcgtggctgtcgggcactccgttgcagatcaccccgctcactgcgccgaacctcgtcatgttccgcactcgcgagcacccgcaggacttctacctgtaccggtacgaggacaacaagaacaacgggcagcgcatcgtggatgcgtggtcgaagttccggtaccacccggcgctgggcgaaatcatcggcgtgagcagctacaagaagaacggcctcgtgttcactgcgcgcgggtcgctggtggcgtgcgacgtgttcgacccgaagggcgagccggactcgcatgcgtgcctcgacagctgggcgagttttggtacacctacgggcgtacagactgcgagcgcaagcatcgccgtcaatagcactagcccgtacttcctgctgggttgtccctacgcgcaggcgtctgacttccttaaccagttcgatgacctcgctgctggtgcgctggaatacggcgtggtgtccgaagctctggtgatcccgaccaatccgttccctcgggaccagaacggtcaggccgtactcgatggacgcatgtccctcaacaaggtgacggtggacgtggagaacacggcaggcatgatcgccacggtggcaacccgcaacagcaatgtgaccactacggacttcgagggccgcatcctcggcgactccgacaatctgatcgcgcggcaaccggtgtaccgggggcagctcaacatcagcgtcgggcgcgaagtgcgcgagtgcacctacgagattcgcagcaaggattggctcccgctccgggtgaccggcctgagctggacgggtcagactttcaacaatgtacggagggttagctaatgggttcggttaatacgatcctgcaagcgaacaacaccacccgcgttgcccgtgcgaactaccgtgcagccgttgcgcagaccgacaaccagaaccgcagcgaggtcgccaagaccggcttcgctgatttcatgcggtccctgaagaacaacgcccaactggacgccgccgcgaaggagtacaactccaacatggaagcgctgtccgaggagctgcgtgcgcgccaaggggctgggcttaactcccagctccaactggcgaacgcgcgtggcgcacttcaggcgcaggctggtgctgtcggtgtcggcggctcgtccgcagacctgatggattcgatggtgcggttgcaggcggaaatggatcaggagacgcaggccaacgctgtctcgctcctcgcctcgcggggcgcatcgcagactgcgcagatcatgtcgcgcgcgtggaacgggatggacatgagccgttcgttcgggcagttcgactactcgcagcacatcgagccgcaggcaatgaagcgtcgcttgggcaagctgatcggcgtggccgtggctacctacttcggtgggccgatggcaggcgaggccgtggcagacttcgcggtcggcacgtggcaggcggacaacggcaacttcactggtgcctctcagtccttcagcaacgcagcgcagaacggtatgcaggcgtggcagcagtccaatgatcgcggcggcaagtcgtgggcgtccactaccttcgggtacaacgacggcaccggcaagcagtccgtgactggggcgaaggtcaccggcaacttcggcaacaactacgacaacttctccaccactacgtccggcctcggctggttcgatagcggcagcggaggcaactcaggaggtgcatggtaatggctgacatcggcacggttaccttcaacacgcagtccgcattgcagggtggcatcaacgccaccccagcactgtcgggcaacaccagcattcaaggcgctggtgtgaatcaggtcgggccggttcaatccggcaacgactggttcgcaagcactggtggtatgacgatgccggacagcaacctgccagagttcttgcaggagctggcagcgccgaacaccgccaagctgaagcagcagcagatgtgggacggcttcgttgccgcccgcgctggtaagaccatggacgagattgctgcgaccgaaccgtggtacaagaaaatcttcggagacaccaactacgagattggcgcgagcatgtataacacgctctcgcaggtcaacgaaatggagagcgacttgcttcggcgtatgccggagttgcgtcagcttcctcccgaggcgatggcgaaggagttcaacgacctcgccactgcccgcatgaccggcaacggtttcgcggacacggtgttgcagaagaccttcatggatcgcgcgggttccctcatggacctgcacaccaaggagcgcacggcatggcagcagcaggagctggtgaaggcgcagtacgctgcgaactcgtcggcgtccaccggcttcaacgaactggcgaagcgcacggcgatgctcggtaccaaccgtcccatggacgagaaggccaccgaggcgctgacgcaggcgcagctgtccctgctggacggactgtcgccctcgcgctaccagacggacgagtcgtacaagtccgcgatcactgcgttctatcgtggcgctgcggatcgcggcgagttccacacgctgaagttcctcaacagcaagggcgttctgaacgccatcgacccggacgggcagctgggaatccagcagtacgtgaagcaggcgcaggatcgttaccgttccgactggctcgatgccaacccggagcaggccgagaagatggcgctcgtctccatgtacgcatcggagggcattggtgccaagccgtcgcaggcgatgatcgaggaaatgaactcgacctacgccgccgagactggaagcgacgcaccgctgtactccggtacgcagttggcttcgatcatggcacagtccgcaggcgcgcacatccgcgcacaggaagccgtcatcaaccagcgtaacgctgcggccaaggccgcgctgaccgaccagcagaagctggccgcgcaggaggaggacatccgtggtggcatcgaagcgttcaagcgcggcacgtacgcgcagacgatcaacatccccggcgtggacaaggagctgatcgaggcgaacacggtgcaggcatggaatgccacgatggccgcgaaccccaaggtcgccatgtcgcagctggtgtggaacgccaacaccgggcgaggcgctgtgctgaagggtgtggccgaccagttccagaccacggcgcgcgctgtgctccgcgatcagccgaacacggcagcggctgcactgtaccagcagtggaaggaactgaagcagaccaccgccgcacgcatcgacacgaacggtcagcccgtgcagggccgactgactggcgcgactaccgctgcgctgtacttcggagatagcgtcaacacgttcttcaacaagctgcaagcgttggagaatggtggcgtgaacttcgagcttgcttacgaggtggcccgtggagaaatcaccaccgacgatccgacgcagttcgacgcgaacagccgtaaggaatccgaggctactcaggctcgtgttacggaagctatcgccaagctcaaccccaagtacctcggcatgttcggcaacaagctgggcgactctggccgcgctgcgtatgctcgcgccatcgtccgctcggtcactgacaccggtggtctgctggacacttctgcggaaggcttgcaggctgcggctactcacgccaagctggcctacggtctggaagacgcaggcaagtacgcatgggaaaacggacgcgacgacgaaggccgagtgatcggcagcgtcggtgcatggctgggcttcatggacacgaaggaaaccggacccgccatcgagaaggccatcgacgcagcactgcgccgggtcaacatcgagccgagcaccgggctgaaggctgacgtgttccgcatgaaggacagcgagaacggcgagccggtgctgtacgtcaacgctgttggcgagaagggctggaaggttgtgccggtgtacgggcgcgacatcaaggacgagtacgagaagcacaccaagcagcagcgtcagttgcaggccccggtaccgcagggctacgttcgcatgaacgacggtacgattcagcagagcatttccatccaacccaaactgtaaggagatagacaatggcactcgatctttcggggctgacccaagaccagcagattgccaaggctgccgcttatgcgggagtgccggagtccatcgtgcgcggtcagtggcgagtagagtccggcaacgggcgtgccgccaaggacgctgacggtgtgatccgcagcaaggcaggagcacagggcgacttccaagtcatgcccaccacgcaggcaacgtgggaagcgcgcaacggtcgcaagtacgacatgcgcaacttccaagacagcatcgagctgtatgccgacatcatgcgcgagaacatgcagcttgccaagggcgacgtgacgaaggcgctgcgcatctaccaaggcggcaccaatccgaagaactgggggcaggagaacgcagcctatgcaccgagcgtgctgggcggtgcgtccgctcccgcagtgtcggcgcagccgcgcagcctgaccaccacgcaggcagacctcaacgccgcatggcagggcaacccgaacatgcgcgaccgtacgtggtccggtgcgtccatcccggatgcgtggacgggtgcgcccatcgaaggccgcaacgctctggcgtcggcagcgaaggaacacatcggcaagattcgtgcgggcatcgccgagctgtcgatgggtcaggtagcacaggaaggtggcaccgccgcgcaggccgtaggcaaggctcaggctgtccgtgcatcggatcaggttgtgccgtggtgggtgcgtcaggaagtggacgtgctgaacaccggcgctcgcaaggcgctgctggatcagaccgaacaggcgctcgcgcaggaccgcgcggacgaggagctgcgcaactcgctgaccttcctcgacaagtggggcgctgcgttcgacagcggcatcggtgctgcgatcagcaaccagtttgcgcgcgaggacgagaacgttccggaaggttggaagtacgacccgaaggaatgggagaagccgtggatgactgccgacgaactcgaagacatccgcgatgcagcgtactcgccgaacgagctgaagtacgtcagcgaccgacagttcctgcgccgccactccatgcgcatcaaggatcagcagactggctggggtagcttcggttacgacatggtggcaggcttcaccgatccgggcaactgggctatcggcggcgtcactgccgcaggcgctaaggcgctgggcatcggctcggctgcactcgttgccgaagggcgcgtgggcgcgtcgctcgcgtcggctgctgcggagaacgcggtcggttccgtcatcacggacgccgcgctggttggcatgggcgagcgccgcaacttcgcggacttcatgaccgacgctgcattcgctaccaccataggcaccgcgatgcacattccgggcgtgcgctcggctgcgcagattcgtgacaaggcaaccatcgacctgtccgcaggcaacgctgccgcttacggcgaagcgtggtcggccgacctgaaggcgcgcgctgtggccgagctgggcgaggacgccaacccggtgctggtgaacaaccgcatccaccagcttgccaagcaggaggctgtggattggctgcgcgctggtatggccgacgtgcctgacgacttccgtatattcgcccgtcccgacgtgcaggagacgaccaccaccgcaggcaccactggtgcactcgcacgggacgcgggcaacgtggacgcaacgaccgggcggtacaacgacagcgtgggtggccgggtcgatcagcatgacccgctgctggaacgcgcatggaagaccgcaggtatcaagggcggtaacgtcgatggcgtgctgaagtatctggaatccaacgcctctatcccggaggacgtgcgtgctatcgccaacgcgctgaagcgtggcgggcggctgagcacggtgaagatcgtgccggaatcggaactcgacaagtggttcgccggtgccaacatgggtccgggtatgcgtgtggccggtggctacaacgccggactggacgcgatggcgatgcggaactacacgccggaagtggtggtgcacgaaatgctgcacgctgccacgctgcgtgagctgcgcagcaactcggtgttcgggcaggaaatggaagaactgctgacccatatcaacaacagcatcggcagtgtggactccacgctgaccaccgctgcgatggagacgcgcatcaaccagccgcaggcaggcttcctcgccaacactgacgagctgatttcctacggcctgacgaaccgcgctgtgcaggcggtgctgcgtcagatgcccgcgccgggcaacacccgcccgaatgcgtgggagtggctgaaggataagatcgcgcgagtgatgggtctgaagaatcaggagtccgcgctcgaacgcctgatgtcggtcgtcggtgacaacctcggcgcggaagtgcgcgacacgcaggccggtacccggcagacgcgtggcatgctcgccaactcgatcttcaagtcgaaccgcgagcgcaaggctttctaccagcgcaccggtctggacaagtccgtcagtgatgacgcgatgcgtgtgcaggtcgccgaagtgatggcacgctccgaacgcttcagtgcgcagtacggcatcgacgcggcgaagctgtccaccatcatgcagcgcttcgggctggaagctacgagcacgactctaatgtcgtccaagtcgccagttgcccgcatgcttgcgatcaccctgttggagaatcccgagggtgcagcaggccgacacagcaccgcagcgatggatcggcatggtcggtttgagtcgttcatgggcacccgcccgcgtcagtgggaagcggcctatcgcctgtggcgtgcggacgtgcgcggtatcggtgcgatcaaggacttcgccacgggctggaaggctcgcgcggacttcgagtacgcagtgaagctgtaccgcgagactcgcttcaacggcggggacatcccggatgcgcacgaggcagtgaaggcaatggcccgtgagttggaccgtggctacaaccgcatggcagcagagcagcgcgcggccggtacggtgggcgcacagcgtctgccggaggaggacgtggagggctacgagtcccgtacgtggctgggcggcagcatcgctgctgctggtccggtgcgacgcgagggtatccgtcaggcgatgcgcgatcagttcgaggtgatgggcgagctgtatggggacgacttcctcgataagttcgctaccaagtatctggaacgcatcgagcgcaaggctgcgggtgtcatcgaagcgccgggtcaggtcttctcggagtcgcaggcggacacgctgcgcgacactctgcgggcgatgtcgctcaacgaggaggagattcagaaggtcatgggcaagtacagccgtggcggtgcgaagcacaccaaggcgcgtatcgacctcgacgtgaccaagcagtacgaggacgctgacggtaagttccgtctgatggactatctcgacaaccgcgtgatggacaactaccgcaagtacgcgggacgtgttgctggtgacatcgctctggcgaagcacggcatcctcggcgacgcaggcatcaacgtggcgcgcgaagcaatgcgcctgaccggtgccaacgatgtggagctgaaggcgttcgagcaggtgatgtccgagttccttggtcgcccggtcggtaccggcgatccgactgttctggcgaatgcgcgtctgctgacctcggccatccagctgggcggcgcgggcatcaatcaggcagcggagtacagcaacggcctcgccgctgttggtgctgctggtgtggctgacgcaatccgtatcgctccccgcatgcgcagcgaaatcatgcgcatcctgaagggcgaggacagcggcaaccaaatcctcgacggcttcgagttcatcagcggtcgcggcttcggtctcgccggttacgacctacacatgttcaactcgctggacacgcaggcgtcgatgtatggtagcgagcgcgcaggcttcctgacctcgctggtgcagaaggcagcgcatgcgaaccgcatcctctcggggcagcgggccgtgcttgctgtgcagcagcgtggcttcgcggaagtgctgatcgccaagggcgtgaagttcctgcgtgatggtgctgaagctgacaccgccctgaaggacatgggcattgacgacaacctgctgaaccgcctgcgggctacgcaggatcaggtcgtgcgctggggcgcggatggtaagctggaagcagtagacccgcgcaacgtcgaggggctggcggatcggcaggcatggttggcgttctacaacgcgatcaaccgtggcacctcgcagattcttcaggacaccttcatcggcgagactggcaagtgggcgcacaacggctggctgaagctgctgttccagcaccgcacgttctcgctggtcgcgcagcagaagcagctgggccggtacgtgggcaactacggtgcatggcagacggcgggcctgatcgctgctgcgatggctgtggcggctccgctgcaagccctgcgggtgctgtcccgcgtggccctgatgaacgatcaggagcgcgacgaggccatcgaccagaacatcctgtcgcctctggcgctgggcaaggccacgctgaactacgtgtcggcgacgggtatgctcaacgatgtgctggacgtgggcactggcgtggcgggcggctggtacgagtacgccaccgatacgcagggtccgacgtggctgaagcagctggccggtgggcagttcggcaaccgcaaggaagtggtgggcgggcagttcgcgccgtcgctgggagtcatcaacgacttcgctcagggcattgctggcaagccggagaatctggccgacgtgattccgggcgggcgactgccgatggtgatcccgctgctgaagggcgcagccagccagtggaaggaggagtaagatcagggccaaggacggcccacccttttggtacacctatagcaaacaggaggcagcatggcagttccagacccgcagctgcgctacgcgacagacgtgttcgacgccgatggcgtgaccactgactggcagatcagctttaccggtggctacatcaacccgtcccacgtgtacgccatgagcggactgctggacgaggagactcagctgctgaccgaccggactccgcacaccgtggaagtcctgagcgaagacgatgacgctagtaccgtccgagtctcgcctgccgtcgccgctgggcgcaagctctacatctaccgcagcactccggtgcagcagatgctcgttgactacgttaacggtagcatcatcagcaagacaaaccttaacctcagcaacgaccagctcctgaagatcattcaggaaatgttcgactcactcaacatcgccacccttagcatcgaccagcaggtcggtgtgatcgtggacctgaacgagattatccagaacatctacaagcaggtcaccgagttgctggcagctggtggtatcgtgtccgtcgccccgcgcgtctggtccggtgcttggactggcgatcaggtgggtgacaccgacttcgacatggtgggcgcggacgtatccggcgcgggcttctacgacgtgtacgtcaacggcatcggcatgcagccggacgtggactatcaggtcacgctcgctgacggcaccgatcccagcttcatccgcttcgccacggttcctgccgagggcagcatctggttcgccgtgctgcgtggttacgccaagccctacaccgggcctgcgccgatcaccgctgcgagcctgcgggtgccgatcatcacggcagagggtccgacttactacgccgccaaggctaccgagtacggactcgtgcgctgcacgtacgccggaggttgcgccgtcaacatcaacctgatccccgaagtgggcgacggtgaaaccaagctcgcctcgggcagctacttcagcgtgcagcagaaggcaggccctgtggtcatcactggcgacgtgggcgtgacgctcgaagtcccggtcggctgcaccgccgcaactcgcggcaccaactccgtcatcactgcaacgtgcatcgacggcgacaccaacacgtggttgctctcgggcgacttggctaaggagtaagcatggctaatcacttcaggctgtacggccgaccgctcatggcggacgaggttgcagatggcctgtcggtgacgggcgtgctggaagggtacacggcgggcgaggcttacgagtctcgcctgtccatcaacaacccagtcggccgctgcaccgtggaggtcatcgaatcgacgctcccttcgggcgctgcggtacgggtggacaacatcaccaaggaagtcgtcgtcaagtgggcggctttcactgaagtcgtggacgaggaaaccctcgtgcccaacggcgacttcgaggcaggcgacgacggcacgtggttgccgggcggtggatcgaatggcgaaggctggtcgattggcactggctcagactacgacaccgacagcggcgtgtacagcgcgcgcttcgccaacatcaagacgggcggcagcgacctgctcaacccgctgatccctgccaaggtcaacgactacatccgatgcaccgccgaggtccagcagggcgcaagctccaagggcaaggccggtgctcgtgtgtcgatcatctaccgcaaggaggatgggaccgagctgcaacgcaactggggcaacatggtttcctccggcagcaacggtgcgtggcaccagtccgttgccgaaggcgctgcgcccaaggacacgaagtacgtgcaggttgtactgtcggcgttccgcagcaagcagaacaaaccgctgtgggtggacaccgttaagtggaaccacaagtacgtactgggtcagaacgacgacagctcctacttccttagcatcaaggtcacggacgggttgaaccgtgtggcctactggtccggtcgtatcgaggagcagggcatctacgttacgtccaagctctacagcttctaccagttcgatgccgcgatgctgaccagcagctttgctgggtacagcaacatcgacatgctccagcctttggatactgcgtcgctgggttcctccttcgtaagctgggaactccgaagctctaggcaggattatgccgccgacccggagagcacgttgtacgggagcgctttcgtttcgttcgacatccgatccatccgtaaggactacacgcctgacccggagacggcgaagctgtcgagttctttccattccttcaccctgaagcagcaccctgtagtcaaccagccgctcgacgcgactgcacgactccggtctggcttcgtatcatggagcttcgcatgatccacaatcacctcggcattgctggcgtgttcaccatcagcaagggtaagtccctcgatactctcgaagttgtagccgactggcagagcaaccttatcacggacggtggtatggacgcactgggtgataccggcagcggctatcctcgcagcatgtacgacctcattgcttacttggcagtcggtagtggcagcgccaccccggcattcaccgataccgctcttggtgcacaggtggcgcaggttggtcgtacgtcctcggacagcggtgggactaccactgccccgtactacgcctactcccgctgccagtaccagttcccggctggtaccgctactggcgttctgtcggagcttggtgccaaagcatacaacaacaataccggcgcgtacatcctgaccacccgtgcgcttatcaaggactccgcaggtaacccgaccaccatcacggtgctgtcggatgaaatcctcgtggttacttacgagctgcgcatgtacgcagataccacgccggttgtcactactgagacgatcaagggtgttagcaccactgttacctgtaagcctattgcaatgggccgcagcggcggtatgaacggtcagtcggcagtcgcttggtcggactacgtgtgggggtgctactacttctacggcggtactggcgacggcaccggagctatcaccgaccagtatccgccggggacgattgccagcttctctgacttgcagcttcagcaggtagcctatgttccgggtacttactaccgtgactgcgtttgccggatgtcgatcaacaacgtgcccggtggtccgatcacggctgcaatgggactctccgcgtgcgtgaccttccaagtcggcttcaatccgggtatcaccaagaccggatcggagacggcgaacttgcgcatgcgggtttcttggagccggtacacgccatgatccccactgtctcccaaagcatccaacgcggtgactgggtggagcagcagaatcggcgcacccgcccgctcattgacttcgagcagggcgggctgactctcaacgcagcagtggacgacctccaagctgcgctgtggactgccgagagtgacggcagcagcgtcgtcgtttaccgcgacggcgttgccccggtcaccgtgctgaccgactccgggatcacgcagatcgcactggccttcgaccagaccatgcgcccgcacgtggcgtacatggcgggcggtgtgtgcaagttctactggtacgacacggtggctgcttcgatgcagaccatggtgatccccggtgctaccactccgcgcctgtgcatggacgagaagcgggctgtcttcgccacgcagagcgacgtgctcctgtcgtacaagaacggcagcaacctgtgcgtacgcgcgcagcgtgagcgcttcgcaaccgaacatgtgatcgcctcgggaatccccggcgacctgattgcggtgggcatgaacaacgtcaaccgcctgcaatggaagctcgtcggcaatcccgacgactggccctaacctacaggagaacagcatgaccccgccgagtgtggtcaatgaggtcgtccgaacctcgccgcttacgctcggcgcggtctacctcaacttcatcagcacgtacggtgctgccatcgtaactacgctcgccattctgtacgccgtcgctcagttctactggcgggcacgcgagcaccgaaagatcatgggaggcaaggatgtcgaatccggcaagtgagggcgcactcggtgcgctgcacgaactggtcgcgcgtgcgctgatgcagcgcatccaagatggcgagctgtgcaccgcagccgacatcaatgcggcgatcaagttcctgaaggacaacaacatcacggcgacgcgcgaggccaacaaggcactcggcgagctggaagacgagctgggcaagcactcgctgcctccggctgacgacgacgagttgcagcgtgcactcgacaacatcgttcactttccggggagcgtagccaacaatgcgtgaatcagctgaagcggccgacgtgcgccgcaagaagttggagctgttgcagaaccactaccggcacttcgccaccttcatgcgcgacattatgaaggtgctggggttcgagccgacgtggatgcagtacgacatcgccaactacatgcagtatggcccgcacctcgcaatggtgcaggcgcagcgaggcgaggcgaagtccaccatcgctgccatctacgccgtcttctgcctgatccacgatcccactcaccgtgtgctgatcgtatcggcaggcggcacgcaggcatccgagattgctacgctgattcagcgcatcatcctcacggtgccgacgttggagtgcatccgcccggacaagaacgcgggcgaccgtacctccgtggatgcgttcgacgtgcaccactcgctgaagggaatcgacaagtccccgagcgtggcgtgcatcggcgtcaccggcaacctgccgggtaagcgtgcggacctgctgatcgccgacgacgtggagtccaacaagaacagccgcactgccgcgaaccgtgagctgctgctgaccatcacgttggagttctcggccatctgcaccggcaagcccggtactccgggtcgcatcctgtacctcggcacgccgcagaccggcgactccatctacaacaccctgcccggacgtggctacgacgttcgcatctggcccggtcgctacccgaccccggcacagcgcgagcactacggcccgcatctggcaccgtctatcgtgcagcgcctagaagccgacccgatgttggcgttcggtggtggcccgatgggcgacgagggccagtgcaccgacgagctgttggccggtgagcagaagcaccagtccgagctgcgtcagcgtggaccgtccagctatcagctgaactacatgctcaacacgcggctgatggatgcgctgcgcttcccgctgaagaccgagaacctgatcgtgatccccggtggtggcgaccgcttcccgctgacgatcacccgtggcctgagcaacgctcaccagcgcagcttccagtccagtgggtacggcttcgtgatgatgatgccgcacgacatgagcaccgagactgcccccgtgcagggcgtgcacatgcagatcgacccggccggtggtggtgccaacggagacgagacggccttcgccgtgaccgccttcctcaactccaccgtgtacgtgttggccgtgggagctgtgcccggtggctacgacggtgatggcttgctagaactgcgccgcattgcggtgaagtacaagccgaacgtcatcagcatcgaaaagaacatgggctacggcgcgttcgccaaggtgttcctgcctgtcctgcgagaagatcgcggcacggagaagggatacaagggcgacatccgcgaggagttcgtgaccggcaacaaggaagcccgtatcatcggcactctcgaacctgtcatggctcgcggctcgctggtcatgctggaatccgtggttgaaatggatcacgagtacacccagcgctacgccaccagcggcaagcgtcaggtctacagcctgttccaccagatggcgaagatcacgcagcagaagggcagcatcgcacacgatgaccggctcgatgcactggaaggtagcgtgcgtcactgggttgcgcagcttgcactggaccagaacaaggccatcgccaagcagcagcagcgagagttccaagactggatcaacgatccgaccggcatgaaggcagcgacccgcaagagtccgctgcaacgtggccgtccatccctactcgaccgttaccggaggtaaccaatgcagaagtccgacttcaccagcaactacacgggtctgttcggccgtggcaactacctgcaccgcgaactgctcgccctcatggagcacgcagagcagcatcccgcaaccgcagcgcagctgctcgcgcagttccagaaggacgccaccctcgtgctggacgccctgatcgctgcgggcgcacgcaccgcgtcctcgggtccgaactccggcccgcacactccggtcgatctggacccggatgacgacccactgaccccgtaaggagcaaccatgaaccagcagcagaaccaagataccagcaacaaggggctgttcggcctgatcggcggcatcttcatcggcatttcggcaacgctgctgtcattcacccaaggccacgaaggggtacgctacgctgcgtacctcgacaccggccgggtgccgaccatctgctacggccacaccaagggcgtagcgatgggcatgacggcaacgaaggcacagtgcgacaagtggctgatcgaagacctacagatcgcccagcagggcgtgcgcaagcacctgaaggcccccgttaaccgcaaccagatcgacgcctacacagacttcgtgttcaacgtaggtgagaaggcgttcgccgacagcaccatgctgcgcaaagcgaacgcaggggatcgtgaaggtagctgcaaggagttcctgcgctgggtctacgtcggtaagctcgactgccgactgtccagcagccgttgctccggcatccccaagcgccgcgacgcagagtttgctctgtgcttgcgccccaacaacgaggtgatccaaccgtggaaaccccaagtgaagtgatcgcgcggctcggcggcaagctggttggcttgctgctggtcgtgaccatgttcgtgtgcttcggtctgtacgtctacggcctgcaacgcaaggtggagaagctggaaactgcccaagtcggcacgaccgctaccgccaaggcggcgcagacgcaggctaccgggtacgcgacctacatcaaagagaaggaggacgtgcgtgttcgcactgaagaagttcttgacgctgccccggagtaccgggatggcactgttcctgctgatgtcgctgacctcctgcgcgaacctgccggtccctgacgactccctgcttgcagactgccacatcacctacctcggtggggagaagggcaccacctcctcgcaggacaaggtggtcaagctcgcgcaggaccgccgcatggacaccgttctgtgcaacaaggacaaggctgcgctgcgtgcgtggaaggccgaggtgtgcggtaccggtaagcgccggtgtacgggtgacaaatgaccaccatcgcatgggacggcaagcacctgtgggccgatagtcaggccacgcagggcgaccacaagcacaccgtgcgtaagatcatgcccgtatcgacacccaccggccctgtgctgctgggtgtcaccggggatttcacagtgcttcgcccggttctcgctgcgcttaaagcgggcgaaggctacgaggagcacgttggcaagtccgcgacggtgcttgtggttaaggacggcgtactcacggtcactactggtaagcagcagtgggtcgaggaggctccgtacttcgatggcagtggcaaggcgctagctctaggggcctatcatgcgagcaagtctgtggctaaggccatggctgctgcgatagctcacgatgtctacagctccgggcctatcgtcaagctaaaggcaccagttcgcgaggcttaggagtaaggccacgtgggtagccggaccaaaatttgcttcggaaatgcgcgggggtcactccaatagaagctcccgcgcgtgcccccgtacgccctcgcgttacgcgcctgcgggtgtgcgtgggtgcgtgcccgcgtgtgcgcctgtgtgcgcgtctgtgcgcccgcgtcaaggttccgcgtgggtgtacccgtgtgcctgcctgcgtgggcctgagcgtgcgtgtgcgtggccgtgcgtgggtgcctgcgggtgggcgtgcgggtgggcgtgcgcctgctgcctgtatggctggaccgcgctgccttggctgaatcgttaataaatctcttggcgaaaggtgttgacgtggccggtgcggtgtggttcaatggcgtcactggggcagcgacagggcttcaggagggccgcaaggggcttgacaggggctaccctacctgctaccatgcgaaccgcagctgtaggcgtgcgagggccatctgtatcgtttcggccttttggtacacctatagcacacagtcggctcaacctgaatcaccgtctatcggtactctgtcgagctgattagttagctacccgctaggccaacggttgacgcttgcgatgcaagcagtagtagacacacggccgcaatggtagtaagctgcaacgcaagtcgagtgacgtgatccgtagtggcgccgccaacaagtgggctaagggtacacgggagtcactggtaagggatgcgaggagctaccgaaccacgcttgacactaagctagcagttagctatgataggcggcaagtggtagccaccggaacagcggagcgacctagcggtaaggctagacgtgagagattacgggtgttgaggctgaggtgagaccgggacaccggtcaagacactaacaggagcgcacatggtcctctaacggatagcttgacaaggcggcacagatagccctttgaggccttgcaacacgtggaccaccgacgtacatggtgggatggtggcgacaggacgcccaacgggttagagacccgagcgagccaagggcttgacaggatgcaacaagggtgctagtatggcaccacgctctgaggagcagccacattggatggcgtaggactaccgctaacgggtagggtgtaacgggaagcgtgccaaccacagccaatagtggccgagagttgacgtggaccgccaagctgcaacgtagcactagcggataaccggatgaactgggatttcaaaggcccatagaatccaccagacttgcaacactggtgccgctttacctaagcctaacgcttagggcttcccatctgccgtgagagtcggccacgggaagtaacccactgccaaggtgggaagccggtcataaggaggtggtgagcctcctatcgcatggaatactgtgcgtttcgtgaaaaggctctacgggccacacggtgacaatggcactgctagccggagtagggttgacagcccgaagggctagcagattgatgcgccctccctttgcgatgaccatgcaggcaaatccggtggtcagtgtgcgcccacgataggcgatgcaacggctctaatcgagaatgagggattgaccgactcgacggctttctgagggcgcatcaatctgttagttttcccaccagtgccaatggaggcacaacatgcaaggctcgatcaatgccaatctcgaccgcacccagcgtaagcgccgcttctgccagttcacccggacggcaagcgtgatggacctgcgcaccacggagcatgaccgcaagcttgccgagcgcaagcgccaagccgagcgctacgaagcccgccacggaaccgccggaaagcgatctgtgtttgttgtcgagggtaacagcgggacgaaccgggcgaaccacgccgctgacaggagggcttacctgtgatccggttcaagttctctcgccactacgtggaagctgcccgcgattcctacaatcgggccatcatgaagcatccggccggctctgtgtcggcgctctacgtcctgccgtgcggtgggcgttcattcgacatccgactcgcttaaatgcaagctactgggccttcgcaagagggcctagtgtcgtgcaatcggcacggacccaacctgaagggaaccaccatggacatcatcaccggaagcgctgacatcaagcgcgccatcaagtcgatcaacaccgcccgcaccaagctggtggaccagattcagcaggccgcgattgcggtcatcaaccacgcacacatccacggcgacgttacgctcgcttccgatctgtgtctcgccgtgggcaacggcatgaagcatgaagccctgcgcctgtacctgtccgagttcggcccgatggctccgaacgacgacaaggaaaccaaggcgagcgcgcccatgaagtttgccaagagcaagcgagtcgagggcgaagctctggccgacgtgctggaacgtgccgccgcgaaggcgtggtacgacttcaagaccgagaagcccgcagaggcgttctcgttcgccgccgacctgcacaagctgctgggccgtctggaaaaggcgaccgaggaaggctacgtgccgaccgaggaggaacaggccgtcatcaacgctgcccgcgctgtgccgaagcccaccaagaagaaggagaacgtgtaacatggaacccaagatcaaccttcgagtgacccagcgcgaagcatccctgctgcgctcggcccttcacatcgcctgtgcactgaccgcaaaggcagacccgtactccaaccgcaagctgtccaatgagttcgccgtgctgcacggtgagctgcgcgacttcggtgtcgagagcttcgagcgtgacgccatcctgcaattcgaggacgacgtgattgcggcctgccgtgacagcgatgtcgaggcacagctgctgcgcgacctgatcgcaccgccgacgttcaccgtgggctacggcatgcgtgaacttgacttcgctgctatcgaggcgcgggtgatggcgtgcctgctgtctccgttgcctccggtggtgttggatgcctcgcagctggacttcctcggcagcgtgaccggccgcatggtgttgcccggcctggcaatgcccgacaacctgccgcgtaagctgccggatgtcctgatggacgaccagagcgcacgccacgtcgccctgactgcatcgcagaccgggctggtcaacaagacgaagaccaagggctggatcgtgcagttcaatctgcgccacggcagcatcgccctcgccaactgggcgcaggtgcgtgagctgggcctgccgcagcgcagccgcaatgctgcgtaccgcatgctgaaggcgcgggccaaggtgcagggcatcagcgaggatgcgtaccgtgtggtgcccgaaggcactcccgatggcccggagaaggatcgcggcttctacaccgccgagttcttcaccaagcatgcgcggcgccctcaccagctgggttggaatacgtccactgtgatcggactcagcggcacgttcaccactgcgcaggctgcacgcaacgccatcgcctcgcacgtcggcaacgatccgaaccgtctccgccgctaccgcgtgaagtggcacccgagccgcgcgtgatctaccgctgcgccttctaacgagggcgtagctttggaaccacgcccaacaggagggcacattgcatgatccccgtaacttacaagcgcatccgtagtggggagcgcaagccgatccagctgtgcgagcagccgcgccagtggaaagagttcgtgacccatgagcacagcgtggagcgctggtatgcgtgaggtcagcctgcgccttgtggtgaaggcgctgccgctcgttaccgtgaagggtgtggctgtcggggattacatcctcggcggacatcacaccagccacgaggcgtgcgagcaagccatcgaacaccaccgcaagcaccacgagaaggtgcccaccctctactcgatagaggaaatcgaaatcccacccgtcaatcaggagaaccaccatgcgtaaggtatacttcatcgtctcgatccccaagaacagcaacgatggcgtcatcactggcgtcgtcgccaatggcaccggccgcaccccgacccaagaggaactggatgcggtgatcgccgagctgcgcaccaagggtgccaccaccagcctgctggactcgctgcgtgacggcacgtacccgaaccagctcgccatcttcgaccgccgcgccgccgtgcgtgccgaggcggatgtgctcaacagctacggcgggtcgttcttcaactggcacatcctcgaagtgggcgagagcatccgcaagccggtgcgcaagccgctgggttggcgtatcacctacgccttcgccgaagaccgcagcgactccgatgtcagctgctacaaccagcacccgagcgccaccgtgcgcatcgacggcaacgagtacaacaagagcgagtacaacgtgctgttcccgacccgcgatgcagcgcgcgccgtgttcaatgccgagtcgctgggcg

SEQ ID NO: 11 - DNA, 44287 bp, unidentified
  source 1..44287: mol_type = genomic DNA
gtagtcgcgccggggatcaccatggtctgcatcgaagcagccaccgtgtcgtaccagtagaacttgcacacaccgcttgccatgtacgccacgtgcgggcgcatagtctggtcgaatgccagtgcgatctgcgtgataccggagtcggtcagcaccgtgaccggggcaacgccgtcgcggtaaacgacgacgctgctgccgtcactctcggcggtccacagcgcggcttgtaggttgtccactgccgcgttgagagtcagcccgccctgctcgaagtcaatgagcgggcgggtgcgccgattctgctgctccacccagtcaccacgttggatgctttgggagacagtggggatcatggcgtgtagcgactccacgaaacccgcatgcgcaggttggcagtctccgaggtcgtcttggtaactcccggattgaatccaacctgccagctgatagccgcactgattccggcagcggcagtgatgggcgctccggggttgttgttgatcgacatacggcagatgcaatcccggtagtacgtacccggcacgtatggaacgcgctgaagttgcagctcggagaaactgacgtttctgccgggagggtactgatcggtgaccgcgcccgtgccatcaccagtgccgccggtgaagtagtagcagccccacacgtaatcgctccaaaccacagaagacgcgccgctgaggccaccgctgctacccaaggcaagcggcttgcacgttacagtggtgctcacgcccttgatcgtctccgtggtgaccacgggagtcaggtcgggatacaggcgaatctcgtaagttaccacgaggatttcatcggacagcaccgtgatggtggtgggattgcccgaggaatccttgatgagtgcgtgggtagtcagaacgtaagcgccggtgtcgttgttgtagccgaaaccgcccagctctgacagcacaccggttgccgtacccgctgggaactggaactgcatgcgcccgtaagcgtagtagggtgccgtcgtagtcccgccgttgtcgcttgacgtgtaggacacacgagcaacctgagcgccgagcgcagtgtcggtaaacgcgggctcggcactaccactgccaacaccgaggtacccgattaccgtgtagagggactgcggatactcgcggcctccgatgaagtccataccgccgttggtaatgaggttgttttgccagtctgccactacttcaagggagtccagcgacttgcccttgctgatggtgaacacaccagccactcccatcttattgtggatcatgcaaagctccatgatacgaaggcgctctttgccatcgcgctcgcgtctagcggctgattgacaatagggtgctgcttcagggtgaaagaaatgaatcccgaggtaaccttggcactctcggaacctgcgtcgtactccttgcggatcgacttgatttcccagctcacaaacgaggagcctagctcggcatactcgggtgaggctgcgtaatcctgacggctgctgcggacctcccaactcacgaaggaagaaccgaccagcgtgctatccacgggaggaagcatgtcgatgttggagtacccagcaaagctgctggtcagcagcgctgcgtcgaattggtagaagttgtagagcttcgacgtaacgtagatgccctgctcctcgatacggccggaccagtaggccacacggttcaacccgtccgtgaccttgatgctcaggaagtaggagctgtcgtcgttctgcccgagcacgtacttgtggttccacttaacggtgtctacccacagcggcttgttttgcttgctgcggaaagccgacagtacaacctgcacgtacttcgtgtccttgggtgcagcgccctcggcaaccgactggtgccagttaccattgctgccgctgctcaccatgttgccccagttgcgttgcagctcggtcccgtcttccttgcggtagatgatcgacacgcgcgcaccagccttgcccttcgagcttgcgccctgctggacttcggcggtgcatcggatgtagtcgttgacctcggccggtatcagggggttgagcaggtcactgccacccgtcttgatgttggcgaagcgcgcgctgtatacgccgctgtccgtgtcgtagtccgagccagtgccaatcgaccagccttcgccgttcgatccaccgcccggtacccacgtaccgtcgtcgcctgcctcgaagtctccgttgggtacgagagtttcctcgtccacgacttcagtgaaagccgcccacttgacgacgacttccttggtgatgttgtccacccgtaccgcagcgcccgaagggagcgtcgattcgatgacctccacggtgcagcggccgactgggttgttgatggacaggcgagactcgtaagcctcgcccgccgtgtacccttccagcacgcccgtcaccgacaggccatctgcaacctcgtccgccatcagcggtcggccgtacagcctgaagtgattagccatgcttactccttagccaagtcgcccgagagcaaccacgtgttggtgtcgccgtcgatgcacgttgcagtgacgacggagttggtgccgcgagttgcggcggtgcagcctaccgggacttcgagcgttacgcccacgtcgccggtgatgaccacagggcctgccttctgctgcacgctgaagtagctgcccgaggcaagcttcgtctcaccgtcgcccacttcagggatcaggctgatgttgacggcgcagcccccggcgtacgtgcaacgcacgaggccgtactcggtagccttggcggcgtagtaggtcgggccttctgccgggatgataggcacgcgcaagctcgcagcggtgatcggcgcaggcccggtgtagggcttggcgtaaccacgcagcacggcgaaccagatgctgccctcagcgggaaccgtggcgaagcggatgaagctcgggtcggtgtcgtccgcaagcgtgacctgatagtccacgtccggctgcatgccgataccgttgacgtacacgtcgtagaagcccgcgccggacacgtccgcgcccaccatgtcgaagtcggtatcgtccgcctgatcgccagtccaagcaccggaccagacgcgcggggcgacggacacgataccaccagcggccagcaactcggtgacctgcttgtagatgttctggataatctcgttcaggtccacgatcacgccgacctgttggtcgatgctaagggtggcgatgttgagcgagtcgaacatttcctgaatgatcttcaggagctgatcgttgctgaggttaaggttggtcttgctgatgatgctaccgttaacgtagtcaacgagcatctgctgcaccggagtgctgcggtagatgtagagcttgcgcccagcggcgacggcaggcgagactcggacggtactagcgtcatcgtcttcgctgaggacttccacggtatgcggagtccggtcggtcagcagctgagtctcctcgtccagcagtccgctcatggcgtacacgtgggacgggttgatgtagccaccggtaaagctgatctgccagtcagtggtcacgccatcggcgtcgaacacgtctgtcgcgtagcgcagctgcgggtctggaactgccatgctgcctcctgtttgctataggtgtaccaaaagggtgggccgtccttggccctgatcttactcctccttccactggctggctgctcccttcagcagcgggatcaccatcggcagtcgcccgcccggaatcacgtcggccagattctccggcttgccagcaacgccctgagcgaagtcgttgacgactccaagcgacggtgcgaactgcccgccgatcacctccttgcggttgccgaactgcccaccggccagctgcttcagccacgtcggaccttgcgtgtcggtggcgtactcgtaccacccgcccgccacaccggtgcccacgtccaacacatcgttgagcatgcccgtcgccgacacgtagttcagcgtggccttgcccagcgccagaggcgacaggatgttctggtcgatggcctcgtcgcgctcctgatcgttcatcagggccacgcgagagagcacgcgcagggcttgcagcggagccgccacagccatcgccgcagcgatcaggcccgcagtctgccacgcaccgtagttgcccacatagcggcctagctgcttctgttgtgcgaccagcgagaacgtgcggtgctggaacagcagcttcagccagccgttgtgtgcccacttgccagtctcgccgatgaaggtgttctgaagaatctgcgaggtgccacggttgatcgcgttgtagaacgccaaccatgcctgccgatccgccagcccttcgacgttgcgcgggtccactgcttccagcttaccgtcagcgccccagcgaacaacctgatcctgcgtagcccgaaggcgattcagcaggttgtcgtcaatgcccatgtccttcagggcggtgtcagcctcagcgccatcacgcaggaacttcacgcccttggcgatcagcacctccgcgaatccacgctgctgcacggcgagcacagcccgttgccccgagaggatacggttcgcatgcgcagccttctgcaccagagaggtcaggaagcctgcgcgctcgctgccgtacatcgacgcctgagtgtccagcgagttgaacatgtgcaggtcgtaaccggcgaggccgaagccacgaccgctaatgaactcgaagccgtcgaggatttggttgccgctgtcctctcccttcaggatgcgcatgatttcgccacgcatacgaggagcgattcggatggcgtcagccacaccggcagcgccaacagctgcgaggccgttgctgtactccgccgcctgattgatgcccgcgccgcccagctggatagccgaggtcagcaggcgtgcattcgccagaacagtcggatcgccggtgccgacaggacgaccaaggaactcggacatcacctgctcgaacgccttcagctccacatcgttggcaccagtcaggcgcattgcctcgcgcgccacgttgatgcctgcgtcgccgaggatgccgtgcttagccagagcgatgtcacccgcaacacggcccgcgtacttgcggtagttatccatcacgcggttgtcgaggtagtccatcaggcggaacttgccatcggcatcttcgtactgcttggtcacgtcgaggtcgatacgcgccttggtgtgcttcgcaccgccacggctgtacttgcccatcaccttctgaatctcctcctcgttgagcgacatcgcccgcagagtgtcgcgcagcgtgtccgcctgcgactccgagaagacctgacccggtgcttcgatgatccccgcagccttgcgctcgatccgttccagatacttggtggcaaacttttcgaggaagtcatccccgtacagctcacccatcacctcgaactgatcgcgcatagcctgacggatgccctctcggcgaaccggacccgcagctgcaatgctgccgcccagccacgtgcgagactcgtagccctccacgtcttcctccggcagacgctgtgcgcccaccgtaccggccgcgcgctgctctgctgccatgcggttgtagccacgatccagctcacgggccattgccttaactgcctcgtgcgcggccgggatgtcgccaccgttgaagcgagtctcgcggtacagcttcactgcgtactcgaaatcagcgcgcgccttccagcccgttgcgaagtccttgatcgcaccgatgccgcgatcgtccgcacgccacaggcgataggccgcttcccactgacgcggccgcgtgcccatgaacgactcgaaccggccatgccgatccatcgccgccgtgctgtgccggcctgctgcgccctcgggattctccaacagggtgatcgcgagcatgcgggcaactggcgacttggacgacatgagggtcgtgctcgtagcttccagcccgaagcgctgcatgatggtggacagcttcgccgcgtcgatgccgtactgagcactgaagcgttcggagcgggccatcacttctgcgacctgcacacgcatcgcgtcatcgctgacggacttgtccaacccggtgcgctggtagaaagccttgcgctcgcggttcgacttgaagatggagttggcgagcatgccacgggtctgccgggtaccggcctgcgtgtctcgcacttccgctccgaggttgtcaccgaccacagacatcagccgttcgagagcggactcctgattcttcagtcccatcacccgcgcgatcttgtccttcaaccactcccacgcattggggcgggtgttgcccggagcgggcatctgacgcagcaccgcctgcacagcgcggttcgtcaggccgtaggaaatcagctcgtcggtgttggcgaggaagcctgcctgcggctggttgattcgcgtctccatcgcagcggtggtcagcgtggagtccacactgccgatgctgttgttgatgtgcgtcagcagttcttccatttcctgcccgaacaccgagttgctgcgcagctcacgcaaggtagcagcgtgcagcatttcgtgcaccaccacttccggtgtatagttccgcatcgccatcgcatccaatccggcgttgtagccacctgccacgcgcatacccggacccatgttggcaccggcgaaccacttgtcgagttccgattccggcacgatcttcaccgtgctcaggcgtccgccacgcttcagcgcattggcgatagcacgcacgtcctccgggatagaggcgttggattccagatacttcagcacaccctcgacgttgccgccacggatgcccgccgtcttccatgcacgttccagcagcgggtcatgctgatcgacgcgaccacccacactgtcgttgtactgacccgtggttgcgtccacgttgtccacgtccctcgccagtgcaccagtggtgcctgcggtagtggtcgtttcctgcacgtcggggcgggcgaagatgcggaagtcgtccggcacatctgccatgcctgcacgcagccagtccacagcttcctgctttgcaagctggtggatgcggttgttcaccagcaccgggttagcgttctcgcccagctcggccacggcgcgtgccttcaggtcagccgaccacgcttcgccgtaagcggcagcgttgcctgcggacaggtcgatggtagccttgtcacgaatctgcgcagccgagcgcacgcccggaatgtgcatcgcggtgccgatggtcgtggcgaacgctgcgtcggtcataaagtccgcgaagttgcggcgctcacccataccaaccagcgcggcgtccgtaatgacggaaccgaccgcgttctccgcagcagcggacgcgagggacgcaccgacgcggccttcggcaaccagagccgccgagcctacgcccagcaccttggcacccgcagcagtcacgccgccgatggcccagttgcccggatcggtgaagcctgccactaggtcgtagccgaagctcgaccagccggtctgctgatccttgatgcgcattgagctgcgacgcatgtactgtcggtcgctcacgtacttcagctcgttcggcgagtacgcagcatcgcggatgtcttccagttcgtcggcagtcatccacgacttctcccactccttcgggtcgtacttccaaccttccggcacgttctcgtcctcacgcgcgagctggttgctgatcgcagcaccgatgccgctatcgaaagcagcgccccacttgtcgaggaaggtaagcgagttgcgcagttcctcgtccgcacggtcctgtgcgagagcctgctcggtctgatccagcagcgccttgcgtgcgccggtgttcagaacgtccacttcctgacgaacccaccacggcacaacctgatccgatgcacggacagcctgcgccttacccacagcctccgctgcggtgccgccttcctgagccacctgccccatcgacagttcggcgatgcccgcgcgaatcttgccgatgtgttccttcgctgccgacgccagagcgttgcggccttcgatgggcgcgccagtccacgcatccgggatggatgcaccggaccacgtgcggtcgcgcatgttcgggtttccctgccatgcggcgttgaggtctgcctgtgtggtagtcaggctgcgcggctgcgatgacactgcgggagcggatgcgccgcccagcacactcggtgcgtaagccgcgttctcttgcccccagttcttctggttggtaccaccttggtagatgcgcagcgccttcgtcacgtcacccttggcaagctgcatgttctcgcgcatgatgtcggcatacagctcgatgctgtcttggaagttgcgcatgtcgtacttgcgaccgttgcgcgcttcccacgttgcctgcgtggtgggcatgacttggaagtcgccctgtgctcctgccttgctgcggatcacaccgtcagcgtccttggcggcgcgcccgttgccggactctactcgccactgaccgcgcacgatggactccggcactcccgcataagcggcagccttggcaatctgctggtcttgggtcagccccgaaagatcgagtgccattgtctatctccttacagtttgggttggatggaaatgctctgctgaatcgtaccgtcgttcatacgaacgtagccctgcggtaccggggcctgcaactgacgctgctgcttggtgtgcttctcgtactcggccttgatgtcgcgcccatacaccggcacaaccttccagcccttctcgccaacagcgttgacgtacagcaccggctcgccgttctcgctatccttcatgcggaacacgtcagccttcaggccagctcccggctcgatgttgacccggcgtagcgctgcgtcgatggccttctcgatagcgggtccggtttccttcgtgtccatgaagcccagccatgcaccgacgcctccggtcactcgaccttcatcatcgcgcccgttctcccacgcgtacttgcctgcgtcttccagaccgtaggccagcttggcgtgagtagccgcagcctgcaagccttccgcagacgtgtccagcagaccaccgctgtcggtgaccgagcgtacgatggcgcgagcatacgcagcgcggccagagtcgcccagcttgttgccgaacatgccgaggtacttggggttgagcttggcgatagcttccgtaacacgagcctgagtagcctcggattccttacggctggtcgcgtcgaactgcgtagggtcttcggtggtgatttctccacgggccacctcgtaggcaagctcgaagttcacgccaccattctccagagcttgcagcttgttgaagaacgtgttgacgctatccccgaagtacagcgcagcagtagtcgcgccagtcagtcggccctgtacgggctgaccgttcgtgtcgatgcgtgcggcggtggtctgcttcagctccttccactgctggtacagtgcggccgctgccgtgttaggctgatcgcggagcacagcgcgtgccgtggtctggaactggtcggccacccccttcagcacagcgcctcgaccggtgttggcgttccacaccagctgcgacatggcgaccttggggttcgatgccatcgtggcgttccatgcctgcaccgtgtttgcttcgatcagctccttgtccactccggggatgttgatcgtctgcgcgtacgtgccgcgcttgaacgcttcgatgccaccacggatgtcctcctcctgcgcggccagcttctgctgatcggtcagcgcggccttggccgcagcgttgcgctggttgatgacggcttcctgtgcgcggatgtgtgcgcctgcggactgcgccatgatcgaagccagctgtgtgccggagtacagcggtgcgtcgcttcccgtctcggcggcgtaggtcgagttcatttcctcgatcatcgcctgcgacggcttggcaccaatgccctccgatgcgtacatggagacgagcgccatcttctcggcctgctccgggttggcgtcgagccagtcggaacggtaccggtcctgcgcttgcttcacgtactgctggattccaagctgcccatcagggtcaatggcgctcagcacgcccttgctgttgaggaacttcagcgtgtggaactcgccacgatccgcagcgccacggtagaacgccgtgatcgcggacttgtaggactcgtccgtctggtagcgcgaaggcgacagcccatccagcaaggacagctgcgcctgcgtcagcgcctcggtagccttctcgtccattggccggttggtgccgagcatcgccgtgcgcttcgccagttcgttgaagccggtggacgccgacgagttcgcagcgtactgtgctttcaccagctcctgctgctgccacgccgtacgctccttggtgtgcaggtccatgagagaaccagcgcgatccatgaaggtcttctgcaacaccgtgtccgcgaaaccgttgccggtcatccgggcagtggcgaggtcgttgaactccttcgccatcgcctcgggaggaagctgccgcaactccggcatgcggcgcagcaagtcgctctccatttcattgacctgcgagagcgtgttatacatgctcgcgccaatctcgtagttggtgtcgccgaagattttcttgtaccacggttcggtcgcagcaatctcgtccatggtcttaccagcgcgggcggctacgaagccatcccacatctgctgctgcttcagcttggcggtgttcggcgctgccagctcctgcaagaactctggcaggttgctgtccggcatcgtcataccaccagtgcttgcgaaccagtcgttgccggattgaaccgggccgaccggattcacaccagcgccttgaatgctggtgttgcccgacagtgcgggggtggcgttgatgccaccctgcaatgcgggctgcgtgttgaaggtaaccgtgccgatgtcagccattaccatgcacctcctgagttgcccccgctgccgctatcgaaccagccgaggccggacgtagtggtggagaagttgtcgtagttgttgccgaagttgccagtgaccttcgccccagtcacggcctgcttgccggtgccgtcgttgtacccgaaggtagtggacgcccacgacttgccgccgcgatcattggactgctgccatgcctgcatgccgttctgcgctgcgttgctgaaggactgagaggcaccagtgaagttgccgttgtccgcctgccacgtgccgaccgcgaagtctgccacggcctcgcccgccatcggcccaccgaagtaggtagcaacggccacgccgatcagcttgcccaagcgacgcttcatcgcctgcggctcgatgtgctgcgagtagtcgaactgcccgaacgaacggctcatgtccatcccgttccacgcacgcgacatgacctgcgcagtctgcgaggcaccacgcgaggcgaggagagcaacagcgttggcctgcgtctcctgatccatttccgcctgcaaccgcaccatcgaatccatcaggtctgcggacgagccgccgacaccgacagcaccggcctgcgcctgaagtgcaccccgcgcgttcgccagttggagctgggagttaagcccagccccttggcgcgcacgcagctcctccgacagcgcctccatgttggagttgtactccttcgcggctgcgtccagttgggcgttgttcttcagggaccgcatgaaatcagcgaagccggtcttggcgacctcgctgcggttctgattgtcggtctgcgcaacggctgcacggtagttcgcacgggcaactcgggtggtgttgttcgcttgcaggatcgtattaaccgaacccattagctaaccctccgtacattgttgaaagtctgacccgtccagctcaggccggtcacccggagcgggagccaatccttgctgcgaatctcgtaggtgcactcgcgcacttcgcgtccaacgctgatgttgagctgcccccggtacaccggttgccgcgcgatcaggttgtcggagtcgccgaggatgcggccctcgaagtccgtggtggtcacgttgctgttgcgtgtggtcaccgcagcgagcatgcccgcagtatcctctacgtccaccgtcaccttgttgagtgacatgcgtccgtcgagtacggcctgaccattctgatcccgagggaacgggttggtcgggatcaccacagcctcggacaccacaccgtattccagcgcaccagcgtcgaggtcatcgaactgggtaaggaagtcggacgcctgagcgtaaggacagccgagcaggaagtacgggctagtgctattgacggcgatgctcgcgctcgcggtcagtacgcccgtaggtgtaccaaaactcgcccagctatcgaggcacgcatgcgagtccggctcgcccttcgggtcgaacacgtcgcacgccaccagcgatccgcgtgcggtgaacacgaggccgttcttcttgtagctgctcacgccgatgatttcgcccagcgccgggtggtattggaacttcgaccacgagtccacgacacgctgcccgttgttcttgttgtcctcgtaccggtacaggtagaagtcctgcgggtgctctcgcgtgcggaacatgacgaggttcggtgccgtgagcggagtgatctgcaacggcgtgcccgacagccacgagtccagctcgttggacatttcgtccgtcaccgtctgctgcccgttgagtgcgccgactcgcatctgatgcaggctcgtgccttcgctgccgtactgcgcgtagaagatgtagttgcccgaggtctgcgccttcgcatccaccgaatccttgttggcactgaacgccttaatcagtggattcttgggactgaacaccgagtcgccgctgatgccatactgctgccggtcaccgaagatcacgaggtttccgttgtagagcgtagcgtgccggagcacgtcgccctcgctaccgtgagcgaagatttcgatggggtcgctgtcttcgatggtaacggcagagccacgccagaagttcaggtagtccgccgagcgcgaggagttgacgtagttctgtgctccgatcaccagccggtcttggaagacggacagcatcgtgatcggcttgtcgatgaaccacgggatcggcgaggtcagcccgtcgcctgccacccgcgcgccgtaagccggatgctcaccgctgcccggagccagagacgtgaggccagcgccgttacgcgcgatgtagcccacaccgttgtagatgtagagctgggacacgaggttgtcgatggtgcactccacgccgggcgcttcataccagtccaccgagccgtagcccgaagtctccccgttctccaactccgcacgcaggtagtacgactcgtcagcgcctgcaccgctcgggcgcacgcggatgatcttgccgtgccaatggaacttgacggcataggtcgcgtcggtaatctcctgccctgcggcatagaaggtcgtgccgtcgccctcgtcgtcaaccgttatgtccttgaactggtcgtcgtcaatcacgataccgcccttgatgtacgtcgccgacacgcctgcatcgaccagcaaatccgacagctgctcggcgatgtactccgggcgcgtctgctcggcgctcgtcacgatccactcgttgactgcggagttgtactcgttcactctgtcgttgacatacttctggtacgccgggtccggctccgtaccaccgggtaggtagaacgggatgtcgctggtgtcgagcgtgccgggatacgatgcggtcaccgtcttgaacgtcaccgtaagcaccgtgttgtccgtccgcgtcaggttcaccgtgtacgtggtgttgtacttaccgctgcgcacccacgctgcgaggcgctggatgttcgtctgctcctgccacacgttcgtgctagtggcggacgggatcgtggtgttgcccgcgatgtagacgtagctgccgatggctgcgagcgacgatgcgccaccgctgaccagcgtgttgacccacgtgctgttctcgtacaccagcgggatgaacgactcgtccgtcttgttgtagaggaacgcgaaggactcgcttcccaaggtcgaggcgtcgcgccgatacagcagtgcatactccttgccctcctgcatgaagtcgaacacgtccatgttgcgcagctcggccgaggtgacaacggcttgggaagcagcgaaccgcgtaccacgacggcgcacgaggccgttcaccggatcggacagcacgttgatctgctcgtgcgtctggcccggacgacgacggtgcgccggtttctgactgacaccctgaaggatgtcgggataggttccgcctgcctttgccatgttgcctccttagccggggaaagtgtagtggctatgccacgggtgtccgctgtagttgaagtaccgctgacgcagcacgtccacggatgcacgagcgaacagcgggttcgccttgatctggcggatgtgctcggacttcaggttgatgtagctgtcgtcgcgctgctgcttgatctttgcgtacttggtgttgtcgccatcgaagtccgactggaagcgcagcactgcgtcgtcgcgcacgaacatctgcacctcgtaggggaggtcatcgaagtccagcagccgaaccatcttggcctgcacgttgtgatcgaactcgtatgtgttgcgcttgcggtcgtacagtcggcgtccgcgctgtaccacgtggccgaaccggctcgggttacagtccagcttcagcacgtccgtggggaccatgatgtacttgctcgttgcctgcggcttcagctccacccattcggtgttgaaccacagcgcgagcgacgacacgtcgcgggtaacgcggtcgatcaagtcaactgcgtcgtccttgtatacgtggtcatcttccagcgtgttgagcttcgtctcgcccatcgtcttcaagcaggcgttcacgatgtcgagcttggtgatgaatgccatggtgtctcctgagaggaacaaggcagagacgccggagcgcccctgccgggatgttgcttagtccgcagccagagccagcgaggccggtgcgtactcgatgtcctgcgagccgatttcgtcatcaacgaaacggacgcgcacgacccagcccgagccgatggcgtcgtaatggacgcctacgacggtgccaacggagttggcgggcagaccggccacgccagttgcggcgacgacgcggttggaaatctcgaacggtcgatcaaagaccatgatgttgctcctgtgttggtggaaggcgaggcgcggtttgagttacccgaaggattcagggaccgcgcctagcggattaggcaaccttgtcgatgcggcccgcgttctcgacgcgatccagaccaacggcgaaggacatccacgagtccacgaagtagcacttcgaggcgtcgctccaccacaccgaggactgcaacggcagcgcttcggcgatcagcagggccttcggcgacacggccacagcgatcagggtgctgaagtcgccgtcgtagaagtcgtcgttgtcgtcgttcgacagcaggtgaccttcgatcacggtgttcggcaggttctcgctcgacagcaccgggacgccccagccgtggaaggtcgggatgccggtcagcttgttgccgtccgaggtcaggtactcgccgttgctgatctgctctgcctgctgcaacaggtagaagatcgccgggcgcacgatcaggaccacgccatcacgctgcggcttgaccttcttctcctcctccatgcgggagaacagcttgccgatggcggcgtacaccttggccggatcgttctcgtcaccggcggcggcgagcacgacctgcgtggcaccgaagtggccctcgggcgcgcggccgttgcgggtgaagatcgactgcgtggcagcagcggccttggcggcggcgatgctgatggtcaggtccacgaactcggcgatttcctgaccctgctcgatggcgatttccttgcgggtgtcgatgtcggtgaagatttcgtccagctgccagatgctgtgacgcgacagcagcatggtatcgacggtcaccgacgccttgctgaagtccaccggggtgccgtccggcgcgtcaccgcgcttcagcttctgaagcttggtacggccgatggccttcttggtcagggtgttggtgcccttgacctgcttgcgcgggaagaacttttccagcaccgagctggacacgtaggtgtgctcgacatcgccggtgaactgttcgaggatcagcgcgttctcgttgccggactggttgacctgattcggcagaaccgggacggtcgggaagatggtgctcatgctttatgttgctccttggttcttagtggatgacgcgcgcgttgagtgcacgcagttcttcggagtgggccgcaccacggatgcccttctcggcaaccagcttgcggtactcagcgcggtactgctccttcgtgagaggagcgacgccgttgatcgacgcggcgggagcggcggcattggtagccggtgcgcccttgacggtcgtcgcgggattggcctgtgccagagccatcaggtaacgcgcggtcgcctgagcgccgaagccaccagccgacagcgattcgcttgcctgcttcagttggtcggcgggcaggttggcccgtgcgaactgctggatcgcagcccagttctctgcgccacccacggcctcgtggacagcagcaacgttcgcggtgtgtgctgcggttgcggcagcggtgacgcgagcgatgctctccttcgccagagcgaggatcggtgcggaacccttggccttgtcgccgaggacttccagcttggcttccagcagggcgaagttgcccttcgctgcttcggtcagttcgcggctgtcgatgtcgaggcccacggtgttgacgaagtattcggccgcgatgttcaggccgttgtcgccgtagtccgggatcgccacagcagtcggcgcgccattcgccggggcggcgggctgtgcgggagccgcaggttcgagactcagcgcgtcagcagccggaggtgcagcaggagctgcgggctgtgccggtgcggcgggtgcaggctgaccgttgggcagcagcttgtcgtccacgggagccggagctgccggtgcgggctggttgccgttcgaggttgcgatcacggttgcgccgggaccaccgcccggaggtgcgttggaactcattgtgtctgtgtctccatgttgttggcgttatcgacctgctgcgatgcgttctgcatgaccagctgctgctgtgcacgctgctgcatcatctggccgtactcggcctcagtcagtacgtagatgttcgggtccaagccaccagcggcggcgaggtctgcgatccacgcggacagcttcagtcgttcgagaatctgcggcggcagcgcgaggacgttggctaggttgctgccgaactccaacagccggtcacggtcacccgtacgggagagcgcggccaagccggtgatgatgacaggctccaagtccttgcctcggatgtcgcggcccgtcaggttcatcacccaaaaggcaacgggtacctgcacgtcagcggcgatacgggagtaaccaccacccagcccgccttccagttcttcggcgaccatgcggatttcctgcgcggtcacacgttccgcctgacgagtcaccgccgtctgcaacaggaagcctgcgccgatgcggttgatgtaggtggactggattgcttggttggtttgcagcacaccatcgacgcctgcgttaatcagctcgatgtcgcccttcatgccgggaatggctgcgccgtttggcgatgccatgaagtcctcgacggaggtctgacctgcggggttcaccagccaccggaactcggaagcgaggatcgcgccctgtactgcggcctcggacagcatcgagagcgactggaagtcggcctcgtagtcttcgaccaagccggagccgtagtcatcgcctgcggccaagtcccagctcaccgcccggtagggcagcttgtctgcggtgtaggtcgaggagaagttggcgggcagcttgcagttgcaaatccacacgtcttcgttgtacttgccggtcttgtggtccagcttgacccacttgtactcccacaccattccgtcgtcatcgggcttgaagtccgggtgcgcgacaatggcagcgagtgcggctggttccagctgggtcttgtgcaccttctcccgaaggatcagctcgtacacctcgccggtgcgggtgcgcttgaccacgtagtgccgcatgttgagcacgcggatcgtgtccttctccaacaccatgagggcgttgcctagtacgatcagcatcttcagcaggtcgtacagtcgggatcggattgagcgcttgtccagttcgagactggcatcctgctcggccttcgcaagcatcgcctgcatggcctgcaagtcagcgccctgttcctgagcagcctgcttcgccttgcgcttcagctccaatcggaagaagggtcgggacggagcgaacagcgacatcatcagcttgttcgccagatggttcactgcctgcgcgccgagagactggaacccgtgggtcagcggctcggtatcctgatcgcggttcttgcgagggaacagcttcggcacagtccagcccgaatagcgttcgagtcggtacatgatgccctgacgcttgttgtcgtaagcctcgaactggcggtgagcggtttggatcgaatggtccatgctcacctcacaacaggtctgacccggccacagtcgtcagccgggaagctgcggtcgtggtcacgggtcgggtgtaggtggagcgggcggtcttgcgtcggccgatcaggtcggcagtctgcaagtcgaggtcggaagttcccagccgcacatcgacggtatcgacgggggcactcagcaacttctcggcgtactcagatgcggcctgctgtgcagctgcctgtgccatctgatcggccatcgcctgaatctggtagttcgtggattgagtttggaggttggtctgcttgtcgatagcagcagcttgcttcagcgctgcccgcttggcggacccaccaccaacgatgctacccataggttaactccttcgcttggtgaattggggagcatgccgttccagcaggtagccgtagcgtgcatacatccgtgtgagcgctcgtgagttccgagctagtgcaccgcctgcgctcagtgagtcgcagtggttgatgtcagccagatgttccatcacggctatgtaccggtcgaaggaactgcccggcccaattcgcagcaccatgttctcaacgaacgtagtacggttcttggagtaccacggtgtgacaatggcaaagcatagtaggtaagcttcatcaatgattactgcatccactagaccctgtgttatcagggccactgtgtaatcaggatcatcacagttgtagctcacagaagattctctgttgtctaccttactatcttctctagatgacagatacaaagcggccgttaaagccgccttgatctgctcactatcacccgtcgttggtgttcggtacggaggaatcaacggtgaaaccctcctgtaagatgttcaggacgcgggccatccccaactgcatacctgcctccaagggcgtggtatttgagttgacggacagcgacagcccggacagtcgccgcacggcggccagctggttcgggtggagcgtcatcaggactttcactttggcgtcttcggccatggtgtctcctctgtgctataggtgtaccaaaaggtccggcaccggttccgcttactctcgcggccgctccaaccggacctcagttgcctcgtgctataggtgtactgaaactccgtcagctgaagaagtacggagaatcaaggacttgccgcaggtccagctcgcccatcggcggcggctccggcaggaacgggtaggccgagtggaaggccgagagcacatcgtgccgctcgtacatcgacacgaacacctcccggatgatccggtacagggccgcgctgtcggcggcatgggtgccgaagtcgtcgtggatcatggcgaaggcgtcgatgccctcggccttggccgcgttgaccaccagcgtcaggtggcttgcgtcgaggctgtgcacgaagttcggggcgatgccgttgcggtgccgggacttcttcaccgcgtccgtgctcttgcgcagggacagcttggcgttgccgcacagcttggtgttgatgcggtgctcctcggattcccagtagacctgcaccaccgggaatccggacggcgtgatccaccggatgcggtcgtacccttggttgaggatcgacccggagccgcgctgcaaccactccatcgcgcccgctgcggcgaccacggtgtcggcgatggcctcacccatgcgcttgctcaggaagcgcgctgcggggccgtacagggccttgtcgagcgaggggaacttgccgcacttcaggtagtcttcgatgatgaagtccgcccacgaagactgccgggagccgtagggcagggtcatcacgctacgcttcaccagcgaacgtgtgaggccatggtcgagccacagcgtacggtacccttcggcatcctcgtcctcgcccagcaggatcgcagtcacgcggtctgcgaccatctggtagatgtcattcggcagcggtgccgggatcaggttagtcgccaccccgcctgctgcgtcgcgcagcatcgccgagaagttctgaagcccattgcacgaaccgtccatgccgactgcgatgcggctcaggaagcgatccccgaacacttgccactgctcgtactccatgcaccagctcagaaattgcagcggcttgtcggcggtcttccactcgtcgttgtgcaccgggtccgcagcgaacgccattatctggtcgtgatgctccgctacccacttcacacgatccggcagagacgccttgtcgtatccccatcggtttgctcctgtgatgcagaaccaatccttcgcgtccttcgtcagcaacggcttaccatcggcgaactccaagagtgccttctgcaagtccgaaccctgcggcgacacgccggtcgtctgcacgtacttgcggccgcggaagtcagcgaagtacacgaagtagatgctcgggtactcggcgaacttgcgcgccaccttcattgcgttgtagaatcgattgcccttgttatgccgcaggcgctcgtcggtgtgccagttggacatgtcgcgcttccactgcttgaactccaactcctgattgtgggacatggtttccttggtcatgtccttcgtcagccactccggcttgcgcggcttcggcagctcgccttgcgaaatgatttcctccatgtcgtgcaccttggcgatggccgacacggcttccatcagccgcttgttgatgcgccacggcacgcgctgcaatgcgttgatcgcggacatttcgttgcgcagctcggcggcgcggtactcgtctcgcgtctgagcgtaggtcttcaccatccacggattgagccgacgcatttccttcgtgtggaatccaccgttgtcgatgtccacccagtccatcggcggttcgacgcacggaagatagaacggcgtagcctcaatcacaaagtcgctgatctgcgtaatcagcttgcgcacctcgtcagtcagcacgatcttgacgtgagtcttggtctggaacttgcggtacgctgcgcctgcactggcagcagtctcggttactacgccaatctccaacatgcccaactgggcgagctgatcgcacaggtacgcgccgacctgatcgcgctgcgcttgcccccactccatgaactcgatgccgttcttgcggccctgcatcttcatcaccgtcatgcggtggttctcgttgacagagagcttgcggtccatgtcgttcatcaggtggtagaacagcgtcggctcagcgtcggcgaactgcgtcagcaggtactcgtggtacacgttgatgccaacgttcttcagcacgtcgcggtcgctgccttcgccgtgcttgtcccgcatgcaggaggtaagggcaccacgaacggcaacgaaggccacagcctcgtaccactcgcgtgcctgttcctcggcgctgacgggctgtccactcttgttctgacgctcgggatcatacttggcgcgcagaagtggcacgtgcgcttgggcacgaccgatgcgcggggagtcgatgtccgcacggatgcgctccgcaagcggaagcacgaaccggcgatacactgcttgggcgtaggggttgttgtccgcgccgcccttctcctcgttgcgggcgatggacttctccatgcgctccttaccgaaggcgtaggtttccagttcgagttccacttgcgagagcatgctacctccgttgcttgatggtgaagtccgtcggcgggtagcgcttcaggatcatgcagaccagtgcggtgtgcatttcgttgatgatgtgcggccacgcaggaccaccgacctcgtagctcgggatgcactggcggttgaagaactgctcggtgccgcaccacgcggtggcagtcacagtgacgtgacctccaccgtagggagagaagcggtcaccgtcgaaatccagctcgggctttccgaatcgaatgtccatcagcccctccgttcggcgaggaagcggtccagcgattcgatcaccgcatcgcgcaccgtctcgttcggccacagggaaccggcgtactcacggaacgggatgctcactcgcacctccaccgtgtcgcgctccatgttatgccacacttcggtctgaacgttgctcaccggtcggcctccttcttgtcatggcggatgcccttgtagcgcggctcgcgcagcaggccgtacttgctgaaggacatggcttcgatttccacgatgtcgccgactacgggaacttgcgaaagctggtgcggcacgccgctcccgacctcctgctccttaccatcgccgaggtccacgaacacggtgtagacatcgcgcccggtcttctcgccgacagcacggccgatgcgtagcacacgcaggtccagcgtcagggtaggcttgaccttgacgacttcgccgttcgtgcccttgtcgcccttcacccacttaccgctcggcttgcgcaggatcaggccgtcgtatgcgccgccctcgcacaacagcttcgccgcctccatgctgcccagctcttggtcgatcaggaagccctgcgactctgcgtagaacaccggagcggtgccctctgcgatggcatggcccatgctcggcaggcggctgacgcgctcctgatacacgaggtcgctgaaaccctgctcccattcttccagcgtcacgaagtcgaacaccacgaacatcggctcggtgtactgcgtgccatccttcttgcggaacatgccgctgacggtgggctggtcgatctgcgggtgccagtattccccgaagtacacgccgaccgggaagaacggcgcggatgcgagagcgttctcgatgtggtgcgcgctgacgacctgctcgccagtccgagagaacaggtcaaccaccccgcgatccaccggctgcatctgcacgtcgcccaccttgattgcgtgcagacccttgttcactgtcggcacccagtggccgcgcttgatggcgaccatgttgcacccgtcgtacttcggctgtgcgatgtactcggtgcgcagctgctcctcggtaggccgcagcttcttcttgatcttgtcctgctcgactgccttgtggacgatgtagctcatgcgtggtccctccaaatctggaacatggcgagcggcacttcgtaccacggaacgtaacgctcccagtacgtggccttgccgtcgtaccactgcacgcggaagttgcccttggtgaaggcgcggttgatcttgaagccgcgcttgcgcttcttgtagccgggagcgacccggacattgctgcgaggcacatcaaacatcggcgctgtcctccttcttggtgccgtcacccagtgcagcgttgaactgcgcgatgcgggatgacatgaacttgttgacgatgccgccgatccacagcttgcgaggggcgagggaaccacggtacccttcccactcgtcggcgatgcgggtatacagctcggcctgagcctcgtcgggcaggttcgggaacccggccttgaccgcgttctgcaacgcctcctcgtggtcagcactctcgccccacgcaacggcgttctcgtaggacttgataagcatggcggtctggttcttgtagagcattcatttctccttcgacgggaatggaacgaaacctgcgaggcccttcatcacgaggatgcagaaggcgtcgtcagggtatgtacgatgccagagcgagttggcccacacggcatcgaactgcttgcgggtacggtgctcctctaggaagcgcgcccactcggcctcatgtgggacgtaccgatgcacttggccgcagcgggcgcaggccattagtcacccttgctgaaccaacggcggatgatgtactggcggatgaagcttatcgccgtgaacgcaatgccgatggcgtgcgccgaaagcagcgggtgctcgggatgccacagcaccggcagcagggcgatgttcgctgcgtagttgatgctgtacccgatgccgatgttcacccaagcctctttgatcgagcgcgccttactctgcgccacggaccttctcctcctcgcgcagttccagctccaacaggaacagctcgttgatgatgtggtgcgcccggtggtggattcccgtctccgggtccagcttctcgccgaggcagcgcttgttgtcgtgccggtagctcgcgtcctgataacgttcgagcgccttctccacgtgctgccacgaatgcgccttgtacttctgcgcaccgaaggtcagggtgtcgatgacacgggccagtgcacgcggcacgccctcgtgcagcagccgcgcctgcggcttaccgccatcatccttcagcccgacaccacggtcggacagtgtgcgacgatcttcgtcacggtagttcagtgcttctggcaagggaacctcccttcgtgcggtggtgacacctcccacgcccatcaggcgagtgaggaactgcgggcggatgatagattccttcagctgcccgtcgaacagaactccaacatcaacggcgctgatcgagcgaaccacgccggacctaccgacgaggcccggagcggagccggtatagcgtacgcggtcgccgtggcgaacgtcggtaagtctcatgcgcttctccttacgcgggaacggtgatgtgcttgcgagcctcggcgctggtcgtgagcttgcgcccacggctgtagccgtcgcacacggtgcactgaagcaggaggtacgttccgacctgcgtacgggccggatcatcctgcgggatcatttcgttgcagccgcacttgttgcagcgatgctcgctgccatcggccttgtagtacactgcgacgttcgggtgctgcgagtaccaaccgcgcagcttcttgtactccaacttcatggacttcacgtcgattcggttgtacgcttcgcactcgtcccatgcgccgggcaagctctgcatgcaggccacccacaggtcgaagccggggaagttgtggtggtcgtacttgcgcagctccggcacgatcacgccggtggtgtactccaacttctgcgaggtgaaggcgaactcggtgcggttcagcagcagtgggtcgatcacctgcaccggagacacgggcgggaacccgaggatggcgaggcgcgccttgatcttgcgcaggtcgaacttcttgccgttgcgagcgagcacgaagtcggcggcgttgagcagtgcccacagcgccttgccttgcttgcgatcatcgaacacatcacgcacgttgcgctgatccatgtagaacgactcgtcatcgtccagccactcgcaagcgaacgacatcagcgaccagtcacgcttgatctgcttgacgctgaagttgttgttgaacatgccccagccgtagaactcgatggggaatgtctcgatgtcgaggcagagaatcttcgggccgcgcttcggtgctcggcgaatgaactgggtaagggtcacggtgtctccttgttgatagcccgacgctttcgcgccttcgcattgcgagcgatgcgcttctcgtcgtcggtcttgaaggtaggatgcaggtaccccgtgatgttggtgaggtgcgaccgcaggtagttggggatgcccgcacagaatgcgaacacgtcgcgcacgccgtaccggcctgcgttgttctcgaccttgccaagcagcgagttgcatccgcgatggagcaccccgcgcacagcgccggtcttgtggtcgtggtcgagcaccggatcgagcggagccttcaggccgaactgtccctgacagagacagcaccggttgccttgctccgctgcgagcttgatgcgcagcagcttgacctgtgttgcagtgagtcgcttcatgctttgtatgcctccaagattgcgcgcttctcgttcacgtcctcggcgaggtcatagaacgcctgcttcagcttcggcccaaacacgtcgagcttcagcacgtcgagcagttcagcgtcacgatccgtccgcatccacaacagcacggcttgctcggcgaaggtcttgcgccagtcggaacccagcacctcgctgtacttgccacgcaccagcatcgctgcctcggcgttgtccttggtaccgaacagcaacgtctcggcagtgaccttgcccacgtcaggcaggccggggatgtggtcggcgctgtcaccgtggagcatctgcatccagaaccacttgtggccgtactgcaaaccgttctcgcccacgatgtcgtaagcgccaagcggaacctcggtgatgtcgtagccgtcccagtctacgtgcacgccgcagaacattcgcatgtccttgtcggcgctgtgcaccacgtgcaggatgttgtggtgcaatgctgcaccctcgttgacgtacgcgatgccgtcgtcggcctcacgagtcagccagattttgggagtgaaagcgtcgccctcgtatgtctccatccactcacgaaggaacgcccagttgttgggcttgcggcctgcttggcgctgaccctgatacggctgcgtggtagcagcgaggaagcgatcacccttggtagacgcggcgtgcgtcaggtgcatgacgatcttgcccgctccgctgacatgcttcagctgtgcgcagcgggagagcacgttgcgtcgtgcatcccccgccgagcagttctcgctaccagccgcgaagtacgccatgtagtccccgtcaacgtgagcgatcacgcgcgggttgtgctgacgtaccacttgcaccggcatcggggagcgctcaccggccgctgccatgagagcgctcaggtccatcaggcgatgcccgccatcgggtcgctaccatccaccgggaacggcggcttgtcgtcagccggagcagcgtcggtagccgcagcgttcgccacgtcgccgaccacttcgtccagcgcatcgacgccttccttggtgaccgtgctgctgcccgacaacttggcggcggcgtagtcgtagcacggcaggcccttgaagttcagcgccgcagcgatgcgcagctgcgtcttgttcttcgactgcgcttcgtgagtgaccttgccggtcttctcgtccttgcgctccgggtactcgccggggatgtagatgctgtcccacatgtcggcatcggcgaagtcccacacgaacgcacccagcggggtgatctgctgcggtaccgggatcacggtgtccacgaacttgccggtggggataccgttctccatttccggcaccggcatgaccggcttgcggatggaagccttgtcgatttcggcgaaggtcttgttcgggtcgcgcttgcccggcttgtggatgacttccagcagcacgccctgacccagcagctgcacgaagtgtcgctcctcggtgcgcaggcggctgaagattttgaagtagtgcgccttctcgttggtggacaggccgagggtcagcgtcatgcgcaccggcaccggaccgttgtccgtgtcgatgtgcgggtgctgcttgccggtcagctcgaacacgatggcgacttcatcctgcgtcttcttcttgccctcgaactcgaactcgtgcttgcccagctcgtagtacccgacgatgcgggcggtggtcacaccagcagcgggcggggtgtagtcgaagttgccaccactggcaaccgactgatccttaccctgcgtggcgaccttgttcaacagtgcgtcaagactcatgcgtgttgttctccttattcaaacgacgggttgtgattaccaacgaagtccttgcggatcgacgctcggtactcgatgaccagaccggcgaactctgcgggagggttcttctcctccatcatgttgtcgcccatcttggtttcacacgggacgccaagtggcagcgtccagttgaaccaccactccatatacaccgacgcttccagcatcgaggcgtgcagcagagcagaggccttggttgcgatgtcgccgtgtgcatccacgtagacggcatcgtgcacctgattcacgagcagcgcgcggcccaaccattccttcggttcggtcacgtacttccggtagaaggcgcgcaggctgacgtacatcgccgccttggcccactcaccaccggtgccctgcatcgggtagttcttgatttccgtaggcgagaacgactgcgcacagccacccttgctcgcgggcttgttggcgatgaacaccggggacggtgactcgctgaaggaatacatcttgccgtccggagtggtccagtgcgaccggccaagctgacacgtaagcccatgtggcacgccttgctgcccggcgttgggatgcggaacgaagcgttgcgtgctgacgcggttgcgcttgatgtgctcgaccatgcggtcgatgtactcgcccagctccgggtaacgctcggcctcaccacgcaccagcgcctcgacttcttcctccgacatgccggtggtcgcagcgatcttcgccacgcccgcaccgtacgcacgctggaaggagaacaccttcgcgtttccgcgcttcttcttccacttcttgtgctcgggatgcttgtcgtccttgctcgccttcaggatgaagtcgtagtcgtacttgccttgctcgccccacgcctgctctgcacgcaagcagtgcatgtcgaggccccgcttcaagtcctcgatcagctgacggcactcggtgaggattgcctgcacgtagatttcgagggaggtgtagtccgactggatgatcttgccacccttgtgtcgggacacgaaggcgcgcttgatctgcgaacccttctcctccaacgtctcctcgtccagctcacccttactcacgttctgcaagttcggatcgctggaagacaagcggcccgtgaccgtgttggtcatgttgagcttgtggtggatgatgccgtccggcccgaccagcgtgagcattcccttctgctcgccagtcttctcgtccgtcgtgatgtagtacgtggacaagtccttgtgcaagtcagcgcgccgggcaagcgccttggtgaacggcaggttgcggtagcccagcgcctcgatcacatcggcggcggtggagtacacaccctcgtcgctcttgctttcccacgcagcatcaggctcggtgtagccggggaactcgaacagcatgtcctcgttgcggaacttctgcttggtcaagtcatcgaccttaaccttcttggtcttgtactcccccttgttcttgccgctgccgtacgtggtgtagcgccacaggttgtcgaagtcctcggccgggggcgtcgccgtcgtagtaccatcgaccagcacgtagtgcacctcgtccttctgcacgtacgtcggcccgccctcggtggacatgatcggaaccttggccgtgtacttcaccttgccaccgaagatcagcgcgctcttgtggaagcggctgttccagttgaaggtcagaccctcgggcaactcggggatgaagccgttgagttcggcggtcgccgttgcaagctcgacctccaactccttcgccttcgcaagcgcccagtccttgtccacgtacatgccgttgtactcggcttcgatggtgaagcacagcgcacccatgttgagcagcgccgagcgcaaaccaccacgtgcacggaaggcagcgagctgaccgaggaacatcttctcggtgttgccgatgtcgcccacgtcgtcggtgtcgttggtgccgaggagataatccatcagcagcgtcttgtcgatgtcgcaggtgtccacgcccgcagcccacagggacttgactgcatcgtccttcaggttgccgccgtagcgtggggccgtctcgtccatgctcgccatgtggaactcttgcgtcataccatgaagcaggtactccgcaagctggcagtcccacaccatgccgccgccgtcgatgaactcgatccatgcctgccgattgagcgggccttggcagatggcgtgcaggatgtcgaacttgatgttgaacccgacgaggaactgctgcccgtaacacagctcgcgcagccacccatcgggtgcgccgcccatgtactggttgtcgattccgatgcgggtgtcgtagtacaggccggtgttccgtgcgtcgcccttccgcttgtagccaatcgccacgatcttgttcatatcgtagaacggattggccttgcgcttcaggatggcacggatcgtggtttcgaggtcgaaggaagtgaagctcacagcggccaccgttgcagggccagctcgtacatttcgtcggacgcatcgccatccaagtcaagcccgtcacgcacccaacggaacacgatgatgcggtcctgcttgtccttgatgttgcggcgcttgcagatggtggtggcctcgaccgcgcgctgataccagccggagtcggcggtcaccatgacgttgaacacgccgttgcgcagcgcataccacgtgtcgctgtagtcctcgtcctcctcgtagtgcccatcggcaccggagcacagggtccatcccgcctcgaccagcttggcgatggcctcgtggaagtcctgcaccagcacgaggtagtcgatgtccgtgttggttacgggcggctcgacggtgtagctgctgccggtacgactggacgtgatgacgcccacgttgcgcggcaggtagatattcggttcggtactcacggcgtgttacctccgggcttggtgatccacagcgtgaagcacgggatcaggttgatgcaccagcgcttgttgtgcggcgagtagtgcacgccgatccatgtgctgtgcttgttgcgcaaccatccccacttccactgcggagcatcgttgcggccttcgatgtagcctgcgtcgtgtaccttgcgcatcataccagcgaggaagttagcctgcgctgtcgatgcacactggtacgactgcccaccgaagtggacctgcgcacacccatcgacgtggattttgtccttcgtcatgctgcctcctgatagaagcgggcacgctctgcgtccatcatcacttcttcccgaacgtcacgcttaccgcctgcgcggtgcagcttgttcttcggggtgccgatgtagcggaagcgttccatcgctgggtcattgagcttgccgcccatgatgatgaagtcgcacgcaccctgcttgccggtcttgctgtccttcagtgcggactgcggcgggtactgaatgccctcaccctcagcgctgatctgcgaagtcgccacgcccacggcgtcgtacttcacacaccagttgcgagcggcctgatacatcgcctccaacatctgatcggtacgctgtccgccgttggtcatgccaccggtgaacgtgatgttgtcgatcatgtcgaagatgatgaagccggggttggtctgcttgatgatggcctcgacctcaccggagttgaacccgtggatgtcgtagaactgcatgcggtggatgtccccgcccatcgcatcttcgatgcgcttgcggatgctgccatccttcgcccactccaccatctcagggatggtagcgccgagcagcgactgataccaccgctgcttgatgcgcttgcccggtccctcgttgttgagccagatgccggtgcgcttctggtccggccacaccgcatcgagctgcgtgatccagtgactagactcgctcgttaggaacgtggtcttgcctgcgtcgggacgcatggcgtagataccgaagtcaccgccacgcatagcacgcaggttgcgcgccaatgtgggcagtcggaagtggatgccgatgtcgtgctcgtccatttccatcagttcttccggcgtctccttgaccagcgggagccgcgccttacgatccatccggtcggtgatagtctcggccaatccgtacagctcgtcgcgcaggctgaactccgctccgccattccactgcacgatcttactgaccgcagtggtggcaagctccaactccaacagcttctcgatcatgccctgctctgcctcgggcgggaccggctcgcgcatctgcttcagcagaactttgagcagggacttcttgtcgtcggcctgcgtcttccacttgaactccatggcccagccatcgaacacatcgaacggcaagtccttcgtgtccgggaactccttgtagtacgcacgcaacgcatcgagcatcagcacggtcagctcgtccagcccatcacgtggtgcactgggtaccagccggtcgaacttgccacggttggtgcacaaccgcagcagcgtggtgtcaagactcatcaggttctccttcgggttcgtacttggaatcgagctggtgataccgtgtgttgcgcgtctctaacttgcgcccgccgtccgtcacgtacagcaccgtcgaggtgtgcacgatgtcgcagtcgccgaggttcggatgcgcaagcacgtcgccgagcgtggcacggaagccaacgacgggcgggatgatggcgcgccgatagcgcacgatgggtttgctcattgcagcttctccttgatgtagtcggtcgtgtaatacttcgggtcacgtggtgacgtgatgttcctgtagtccagaccaaacgcacgtagacgcgcagcgattactcgcgcgctgtcttggccgggattgctaccgttgcttctacctctgtcgtcatcgagccacgttgctacacgttggcctcgatcagtcagctgcttcaacactttgttgtgcagcttggtgccgagcaacgaccacgcttctgtgcactggcccaccttgaaggcggatagcgggtcttcgcatagcacgatggtgtcccccttgcccacgccgtagcgtgcgacaagcccatccttcggcacatcaggagtcagccatttgggctgacggcttgtgcttcgtgctgtccagtacacaacgtcgtcgccttcagtgatcggtagtaccacccgcccgatgctcgggcaccagtacagccgcagcttgtcgatcatctgaagcgagagtcccatcttaaagaaccacaccttcgcatcgagcggccactctcgggtgtcgtatacccgtggctctggcaactcaacagtcgcacgcactctgcgttcgctcgtctgctcggcgtggattcgtgcaagcttggcctctatactctcgtgctcacgcttgaatcctgtgccaccgcacctgaaacagaatgcggtggacttgtcatgctcccgagtgataagcaagggagtcccttccccgcaatcatgcggcactcgggtgcggtggccgacctgtagtcgctccgcatggtgcagccaatcgctgtcgggaagggtctcgctcatgctatcctcgcttgattactcgaacacctcgaagatgtcgttgtcggtggcgtacagcacggagccgttgccatcggtgctgacgatcagccggtcaccagactcgctggtcagcttggacaccacgaaaggcgtgcccttggtcagcttgttggtctgccgggtgtcgatcaggtacgcggtggtgccgggcttcagctcgtcgccgcgcttgactgatgcactgaccggggccgggctggacaggctcacgactgcccgccttcaccggcagcagccttggcggcggcagcttcggcggcgaggcgctgtgcctcggcaacggcggcgtcgatttcttcctgcgccttcagcacttcttcggccgacatcagcagggcgctgctgtcgatcaggttcagctcggcatccagaccttcgccggtctgcaccttcagttgcagcacgcccttgtcgttcttgccggtggcgacgatcacgccggacaggacacgcttgttcagggcacgaccgaacaggtaggacacggcgtcgccggacttcagcgcttcgatggctgcgctgttggcctcgaccgcatccagcttggcgagcttgtcgttcagcgcatcgaccttggcctgcgccttggcgatgtcttccagcagctcggcgcgcttggcttcgtagtggctgacggaggtggtctgttcggtggtgttttcgttcgacatgcggtgtatctcctttcattgacgggtttggttggtggaccgtaacgtgggccagtcggcacagttcagtgctggattactggaagatcagctcgctgttgtacccaccgccgccattgtagaagcgacggcgcagcacgctctcctcgccgagcaccagcaggcggtccacgatggcgcggatggcgctcatgtactggtccaccagctcgctctgcaagttcatgtcgaagcggatcacggtcaccgcctcgtcatccagtgcgccggtatccttgcggacgtacaggccacgggcattggtcatcgtcgcgccaccgatcagcttgacggcggcggcaatctccggctgcacgttgagcagtcggctgtcgggcacggtcacctcgacccagcttcccatgcgcaggctcatgctgcacctgccagtgcggactgcacgttcggctgcaacgatgcaccagcacgcagctcggcagcacgacgcttcatgcgggagcgcagcttgcggcgctgcttgttgttgtcgccgaggctatcggccacacgcttcagctggttgttgccgacgatgcgggtctgaccctgccccttctgcacggggaagtagtcctgccccagcatcttgcgcagcaccgggttgtcgatggggatcagcggcacgctgacgtgcaggtaccggctggtatccggtgcgggcggcggcgtgtcatcgtcgtcgtgctgcggcttcaccgctgcaaccaccttgtccttcacccagttggcggcaccgcgaatcttgccgccgacgttcttgatcttttccatgaatcccatggtttacttcctcctcgtgccgaagtgattgaactccgtctcgtgccacacatagtacgtggtgccgagcgggtcggtgtctgcctgccagttgcgctgggtgcagtagtcgttggctgcgtcgaggtcatcgaacgtcagcgagaacccggtggaagccgggccggtgcggaaccggcacagcctaccgtcgtcgtcatggtactgcccgacgacaacccacggtccacgacccacgatccagtacagcaggatcaggatacgcagccagagtttacgcatacaccgcctcgatgtagtagcccgagggattctgcttgctgcgcttgtcaccgatggtattatcgatgatgtcacgggcggcggcgcgagtcgggaacagcaggttgtcctcgctgttgttctcttcgtcaccatcgacgcgcaccgttgcgccgtcttcgacggagttgtagcagctggtgtagtcaccgtcgtacttgatacgccagcccttcacctgacgcaccggcttgcggatgctatcgcccacttcgatgatgtgccagttgaacaggccaccaccgttgaaggagttcaggatgtcggcctcggcacgggcggcggcacggcgctcgaaggcggacaccgggccgggataggtggcgtcgcgcaggctgtccagcagggactgcgttgcgcccttggtgcgcagcagctcgaccagtgccgtcacttcctcggcggtggcgttgcggcccgtgccattggcgacgacgccagtgatgacgccatcctttgcggtggccgggatcgaagcgatgaagtacagcttacgcatggtggttctcctcattgacgggtgggatttcgatttcctctacggtgtagagagtgggcaccttctcgtggtgcagacggtggtgtgcgatggcctgctcgcacgcctcgtggctggtgtggtgcccgccgaggatataatccccgacagcccaaccctgcacggtaacgagcggcagcgccttcaccacaaggcgcaggctgacctcacgcataccagcgctccacgctgtgctcatgggtcacgaactctttccactggcggggcttctcgcacagctggatcggcttgcgctttccactacggatgcgcttgtagacgatagggatcatgcaatatgccctcctgttgggcgtggttccaaagctacgccctcgttagaaggcgcagcggtagatcacgcgtggttcgggtgccacttcactcggtagcgacgcagacggttcgcatcgttgccgacgtgcgcagcgatggcattgcgtgcagcttgcgcagtggtgaccgttccgttgagaccggtcacgctggacgtgttccatcccagctgcgactgacgggcggcgtgcttggtgaagaactcggcggtgtagaagccgcgatccttctccgggccatcgggagtaccttccggcaccacacggtacgcatcctcgctgataccctgcgccttggcccgcgccttcagcatgcggtacgctgcattgcggctgcgctgcggcaggcccagctcacgcacctgtgcccagttggcaagggcgatgccgccgtggcgcagattgaactgcacgatccagcccttggcctgcggcttgttgaccagcccggtctgcgatgcagtcagggccacgtggcgtgcgctctgatcgtccatcagtacatccggcagcttacgcggcaggttgtcgggcattgccgggccgggcaacaccatgcggccggtcacgctgccgaggaagtccagctgcgaggcatccaacaccaccggaggcaacggagacagcaggcacgccatcacccgcgcctcgatagcagcgaagtcaagttcacgcatgccgtagcccacggtgaacgtcggcggtgcgaacaggtcacgcagcagctgcgcctcggcattgctgtcccggcaggccgcgataacgtcgtcctcgaattgcaggataccgtcacggtcgaagctctcgattccgaagtctcgcagctcaccgtgcagagtggagaactcgtcggcgaggtctttgcgagcatacggctgcgctttggcggtcagcgcacaggcaatgtgcagggcagcacgcagcagggacgcttcgcgctgggtcactcgcaagttgatcttgggttccatcatggctccttgaatcggtgggtgtggaaggctgtgcggtcgccgaagtcatcgacaaccacccagtattcgggaaaggtgaatccgttctccatcgtgacgctcgggaccacctcgactacggtgtattccttgccgccagtcaggcggaacagggccgtgtgcttggatacaacgacggtcccggattccatcacgcagtcgccttcaccttggcaggcttgggcacggcgcgggcagcgttgatgacggcctgttcttcctcggtcgggacataacctccctcggtcgccttttccagacggcccagcagcttgtgcaggtcggcggcgaaggagaacgcctcggcgggcttctcggtcttgaagtcgtaccacgccttcgcggcggcacgttccagcatttcggccagagcttcgccctcgacgcgcttgctcttggcaaacttcatcggcgcgctcgccttggtttccttgtcgtcgttcggagccatcgggccgaactcggacaggtacaggcgcagggcctcatgcttcatgccgttgcccacggcgagacacagatcggaggcaagcgtaacgtcgccgtggatgtgtgcatggttgatgaccgcaatcgcggcctgctgaatctggtccaccagcttggtgcgggcggtgttgatcgacttgatggtgcgcttgatgtcagcgcttccggtgatgatgtccatggtggttcccttcaggttgggtccgtgccgattgcacgacactaggccctcttgcgaaggcccagtagcttgcattcagtggatggtgggtgcagcgagcttgatgtcataggtccagcgtgcgccggtccattgcaggttcgatacagcgcccggcggatgcttcgccattgcccgttcgtggcttgccatggcgttgcggctgtaccctgcggcgaagtagaatcggatcacaggtaagccctccggtcagcggcgtggttcgcccggttcgtcccgctgttgccctcgacaacaaacacagatcgctttccagcggttccgtggcgggcttcgtagcgttcggcttgtcgcttgcgctcggcgagcttgcggtcatgctccgtggtgcgcaggtccatcacgcttgcagtccgggtgaactggcagaagcggcgcttacgctgggtgcggtcgagattggcattggtcgagccttgcatgttgtgcctccatttggcactggtgggaaaactaacagattgatgcgccctcagaaagccgtcgagtcggtcaatccctcattctcgattagagccgttgcatcgcctatcgtgggcgcacactgaccaccggatttgcctgcatggtcatcgcaaagggagggcgcatcaatctgctagcccttcgggctgtcaaccctactccggctagcagtgccattgtcaccgtgtggcccatagagccttttcacgaaacgcacagtattccatgcgataggaggctcaccacctccttatgaccggcttcccacctttggcagtgggttacgctgcgtggccgactctcacggcaaatgcaggccctaagcgttaggcttaggtaaagcggcaccagtgttgctagtctggtggattctatgggcctttgacatcccagttcatccggttatccgctagtgctacgttgtagcttggcgttccacccgtgggcttcacgttacaccctacccgttagcggtagtcctacccggtccagtgccggtggtcctcagaccgtggtgccatactagcaccctgtttgcatcctgtcaagcccttggctcgattcgggtctctaacccgttgggcgtcctgtcgccaccatcctaccatgtatgccggtagtccgcaaggtgctagctgctccgctgttccggtggctaccacttgccgcctatcatagctcactgctagcttagtgtcaagcgtggttcggtagctcctcgcatcccttaccagtgactcccatgtgcccttagcccacttgttggcggcgccactacggatcacgtcactcgacttgcgttgcagcttactaccattgcggccgtgtgtcaactgttggcctagcgggtagctaactaatcagctcgacagagtaccgatagacggtgattcaggttgagccgactctgtgctataggtgtaccaaaaggtccgaaacgatacagatggccctcacacgcctacagctgcgggtcgcatggtagcaggtaggtatgcacctgtcaagccccttgcggccctcctgaagccctgtcgctgccccagtgacgccattggatcacaccaacggcaccacgtcaacacctttcggcgggagatttatgtacgattcagctagcccaccacgtgccacggcaggagaggaaccacaggcgcacacgcgagcacgcacccatgcgcacccgcaggcgcgtaacgcgagggcgtacgggggcacgcgcgggagcttctattggagtgacccccgcgcatttgggaagcaaattttggtccggctacccgcgtggccttatgactaagccttgcgaactggtgcctttagcttgatgataggcccggagctgtacacatcgtgagctatcgccgcagccattgccttagccacagacttgctcgcatggtacgcccctagagctagcgccttgccgctgccatcgaagtacggagcctcctcgacccactgctgcttaccagtagtgaccgtgagtacgccgtccttaatcacaagcaccgtcgcggacttgccaacgtgctcctcgtagccttcgccgctttaagcgcagcgagaaccgggcgaagcactgtgaagtccccggtgacacccagcagcacagggccggtgggtgtcgatacgggcatgatcttgcgcacggtgtgcttgtggtcaccctgcgtggcctgactatcggcccacagatgcttgccgtcccatgcgatggtggtcatttgtcacccgtgcaccggcgcttaccggtaccgcacacctcggccttccacgcacgcagcgcagccttgtccttgttgcacagaacggtgtccattcggcggtcttgcgcgagcttgaccaccttgtcctgactggaagtgctgcccttcgcgccaccgaggtaggtgatagagcagtccttcagcaggtcatcgctcggaaccggaaggttcgcgcaggaggtcagcaacatcagcaggcacactgccatcgcggtactctggagctgcgtccagaacttcttcggtgcgtacacgcacatcctccttctctttgatgtaggttgcgtagccggtagcctgagtcttggccgcagtggacgacgcggaggtcaccacttgggcgttctccaacttatcgaccttgcgctgcaagccccacacgtacagacccgcgcagacgatgagcaccacgccgagcagcaggccgatggccttaccagcaagacgcgcactcatttcggttggggtttccatggttggattacctcactgttgggccgcatgcacagagctgcctctgcatcgcggcgcttggggataccagcacaacggctggaagacaggcggcagtcgagtttcccgacgtacacccagcggtagaactccttgcagctaccagctcgatcccctgagttcgccttgcgcagcatcgtgctgccgacgaagttcccctcacccacattgaacacgaagctcgtgtaggcgtcgatctggttccgctctgccggtactttcaggtgcttgcgcaccgccttctgcgcgatggcgaggtcttcgaccagccactgcttgcattgagcctcggtcgcggtcatgcccatacgcaccccggccgtgtggccgtagcagatggtgggcactttgccggtgtcgaggtacgccgagtagcgtaccccttcgtggccggtgacaatcgtcagcagcgtggccgatacgccgatcaggatgccgccgacgaggccgaatagccccttgttgctctggtcgttctgctgctgactcatggcttacggctcctcgggttcttccggcgcgggcagcgggccgctgttcgggccactggactcggtgcgggcctgcgcggcggtcagagccgcctgcacgacggcgacatcgccggtgaagatggcctgcaactgctcggcagactgcggatgctgctcggcgtactctaccagaagcagcagctcgcggcggatgtagtcgccacggccatacaggccggtgtactggctggggaaatcggacttcaacattgggttacctccggtaacggtcgagtagggatggacggccacgttgcatcggactcttgcgggtcgctgccttcatgccggttggatcgttgatccagtcttggaactctcgctgctgctgcttggcgatggccttgttctggtccagtgcaagctgcgcaacccagtggcgcacgctaccttcgagtgcatcgagcctgtcatcgtgtgcgatgctgcccttctgctgcgtgatcttcgccatctggtggaacaggctgtatacctgacgcttgccgctggatgcgtagcgctgggtgtactcgtgatccatttcaaccacggattccagcacgaccagcgagccgcgagccatgacaggttcgagcgtgccgatgatgcgggcttccttgttgccggtcacgaactcctcgcggatgtcgcccttgtatcccttctccgtgccgcgatcttctcgcaggacgggcaggaacaccttggcgaacgcaccgtagcccatgttcttttcgatgctgatgacgttcggcttgtacttcaccgcgatgcggcggagttcgagcaggccatcgccatcgtagccaccgggaacagcgcccacggccaacacgtacacggtggagttgaggaaggcggtcacggcgaaggccgtctcgtctccgttggcaccaccaccggccgggtcgatctgcatgtgcacgccctgcacgggggcagtctcggtgctcatgtcgtgcggcatcatcatcacgaagccgtacccgctggactggaagctgcgctggtgcgcgttgctcaggccacgggtgatagtcagcgggaagcggtcgccaccaccggggatcacgaccagattctcggtcttcagcgggaagcgaagcgcatccatcaaccgcgtgttgagcatgtagttcagctggtagctggacggtccacgctgacgcagttcggactggtgcttctgctcaccggccaacagctcgtcggtgcactggccctcgtcgcccatcgggccaccaccgaacgccaacatcgggtcggcttcgaggcgctgcacgatagctggtgccagatgcgggccgtagtgctcgcgctgtgccggggtcgggtagcgaccgggccagatgcgaacgtcgtagcctcgtccgggcagggtgttgtagatggagtcgccagtctgcggcgtgccgaggtacaggattcggccgggagtaccgggcttgccggtgcagatggccgagaactccaacgtgatggtcagcagcagctcgcggttcgcggcggtgcggctgttcttgttggactccacatcgtcggcgatcagcaggtccgctcgcttacccggcaggttgccggtgacgccgatacacgccacgctcggtgacttgtcgatgcccttcagtgagtgatgcacgtcgaacgcatccacggaggtgcggtcgcccgcgttcttgtccgggcggatgcactccaacgtcggcaccgtgaggatgatgcgctgaatcagcgtagcaatctcggatgcctgcgtgccgcctgccgatacgatcagcacacggtgggtgggatcgtggatcaggcagaagacggcgtagatcgcagcgatggtagacttcgcctcgcctcgctgtgcctgcaccattgcgaggtgcgggccgtactgcatgtagttggcgatgtcgtactgcatccacgtcggctcgaaccccagcaccttcataatgtcgcgcatgaaggtggcgaagtggcggtagtggttctgcaacagctccaacttgcggcgacggatgtctgccgcttcggctgattcacgcatggttggctacactccccggaaagttcacgatgttgtcgagcgctgcttgcagctcggtgtcgtcggcctgcggcagcgagtgcttgccgagttcgtcttccagttcgccgagcgccttgttggcctcacgcgtcgccgtgatgttgttgtccttcaggaacttgatcgcggcattgatgtcggcggcagtgcacagctcgccattggcgagacgttccttcagtaccgtggcgacgagttcgtgtagcgcgccaagcgcaccctcacttgctgggttcgacatccttacctcccatgatcttgcggtgctcgcgtgtgcgccagtagaactgggcgactgcatacagaatggcgagcgtagttacgatggcagcaccgtacgtgctgatgaagttgaggtagaccgcgccgagcgtaagcggcgaggttcggacgacctcattgaccacactcggcggggtcatgctgttctcctgtaggttaaggccagtcgtcgggattgccgacgagcttccattgcaggcggttgacgttgttcatgccaaccgcgatcaggtcgccggggattccagaggcgatcacgtgttcggttgcgaagcgctcacgctgcgcgcggacgcacaggttgctgccattcttgtacgacagcagtacgtcgctttgtgtggagaagatcgcccgcttctcgtccatgcacaggcggggt

SEQ ID NO: 12 - DNA, 42769 bp, unidentified
  source 1..42769: mol_type = genomic DNA
cgctagaacttacaccgagctccgtaacattgcctacgacagcaccctgtgcgaactggaagtagcgagtgcgggaaccccatacggtggtagcggttcgcatttgctcttcggtggagccggcaagggtatcgctctggtaagtgctgctagtgtaagcgagactcgacgcgagctggatgtcggtgaattctggtgtggtagtgcccacaccaacgtgacagtaggtgaggtagccattggcagttcccaactgatccatgccgctgttggtaatcaggttatcgaacttttcagtgagcttgcggacatgccgcacaccccgctcgtcaactcgtgcagcgaacagctggaactgtccgcgcacctgagcattaagaatcatgttttggtcatccctatgatagttggcataccagtcttagttctatcgacgtagcccgacgtgcggacaacgactttagcgctggtacctccggtgatggtcggcatgctggtcttggtgtagtcttccttcggcagaatgaggcggttaaccgcagactttgaagacatacctacgatatacggcatagcggcgagagcaggggtgtcttccagcacagcaacgcgaagaacggcggatcggctggacaaagacacgacacccggcatacctgctgtggcgtagtctagaaggttggcaccggcaccgagattgagttgtgtagtcggcatgtgtgccgcagcgtcgtcgtaaaccgagacgggatacagctggccgattacgtaagttgcatcgattccgataccgccacgccagtaggccacacggttggcaccgtctgtcaccttgatgtagagcgagtagtcgctgtcatcgtcttggcctagcacgtacttgtggttccacttaacggtgtccacccacagtggcttgttctgcttgcttcggaatgctgacagcaccacttgcacgtactttgtgtccttaggcgcggcgccttcggcgactgactgatgccacgcaccgttgctcccggacttcactaggttgccggagttgcgttgcagctcggttccatcctccttgcggtagatgatcgagacgcgcgcgccggccttgcccttggagcttgcgccctgctgaacttcagcggtgcagcggatgtagtcgttgaccttggcagggacaagcgggttgagcaagtcgctaccgcccgtcttgatgttggcgaagcgcgcgctgtacacgccgctatcggtgtcgtagtctgagccagtaccaatcgaccagccttcgccgttcgatccaccgcccggcacccacgtgccatcgtcgcctgcctcgaagtcgccgttaggcacgagtgtttcctcgtccacgacttcagtgaaagccgcccacttgacgacgacttccttggtgatgttgtccacacgtaccgcagcgcccgaagggagcgtcgattcgatgacctccacggtgcagcggccgactgggttattgatggacaggcgagactcgtaagcctcgcccgccgtgtacccttccagcacgcccgtcaccgacaggctatctgcaacctcgtccgccatcagcggtcggccgtacagcctgaagtgattagccatgcttactccttagccaagtcgcccgagagcaaccacgtgttggtgtcgccgtcgatgcacgttgcagtgacgacggaattggtgccgcgagttgcggcggtgcagccgaccggtacttcgagggtcacgccaacgtcgccggtgatgaccaccgggcctgccttctgctgaacgctgaagtagctgcccgaggctagcttcgtctcaccgtcacccacttcggggatcaggttgatgttgacggcgcagcctccagcatacgtgcagcgcacgagtccgtactcggtagccttcgcggcgtagtagatagggccttctgccgggatgatcggcacgcgcaggctcgcagcagtgatcggaggaggcccggtgtagggcttggcgtaaccacgcagcacggcgaaccagatgctgccctcggcaggaatcgtggcgaagcggatgaagctgggatcgctgccgtcggccagcgtgacctgatagtccacgtccggctgcataccgataccgttgacgtacacgtcgtagaagccagcgccggacacgtcagcgccaaccatgtcgaagtcggtgtcgcccacctgatcaccagtccaagaaccggaccagacgcgcggggctacggacacgataccaccagcggccagtaactcggtgacctgcttgtagatgttctggattatctcgttcaggtccaccaccacacctacctgctggtcgatgctaagggtggcgatgttcagcgaatcgaacatttcctggatgatcttcagcaactggtcattgctgaggttaaggttggtcttgctgatgatgctgccgttaacgtagtcaacgagcatctgctgcaccggagtgctgcggtagatgtagagcttgcgcccatccgcgacggcgggctcaactcgcacggtcgaggagttttcgtcctcggacagtacctccacggtgtgggaggtccggtcggtaagcagctgcgtttcctcgtccagaatgccgctcatcgcgtacacgtgggacgggtcgatgtagccgcccgtgaagctgatttgccagtcagtagtgacgccgttagcgtcaaatacgtccgtcgcgtagcgcagctggggatcgggaactgccatgctgcctcctgtgtttgtcgtatgtgtaccaaaagtcgggccgtccttggcccgccagccttattcctccatctgcgccgccgcgcccttcagtagcgggatcacgtacggcaggcgaccgcccggcagcacgtccgcaaggttctcgggacgcccgctcacgccctgcgcgaagtcgttgatgacccccagcgcaggggcgaagctgccgcccacgatttccttccggttgccgagctggccgcccgcgagctgccgcacccagtccggggagccggtgtcggttgcgtgctcataccagccacccgccacacccgtccccacttccagcacgtcgccgaggaaggccgtcgcgctgatgtagttcatggtgctacggcccatcgccagaggcgacagggcatcctcgatggcctgatcgcgctgctcctccggcaggagggcggcacgcgaggcgacacgcagggcttgcagcggagcgaccacagccatcgccgaagcgatgatgcctgccgtaccccatgcaccgtacaggcccacgtagcgacccagctgcttctgctgtgcgaccagcgagaacgtgcggtgctggaacagcatcttcagccaaccgttgtgcgcccacttgccggtctcaccgatgaaggtgtcctgcaagatttggttagtaccacggtcgatggtgttgtagaacgcgagccacgcctgacggtcgtgcaggttctccagaccacgcgggtccacagcctccagcttaccgtccgcgccccagcgcaccacctgatcctgcgtctgccgcagccgagcaagcagcgtgtcgtcgaggcccatgtccttcagggcagtatcggcagacttaccgtcccgcaggaacttcacacccttggcgatcagcacttccgcgaagccacgctgctgcacagccagtaccgcgcgctgccccgagaggatgcggttggcgttggcagtgcgctggaccagagcagtcaggaagcctgcgcgctcggagccgtacagcgaagcctgcgtgtccatcgagttgaacatgtgcaggtcgtaacccgcgaggccgaagccgcgcccactgatgaactcgaagcccccgaggatgctgttatccgggtcttcgccgcgcagaatcttgccaatctctgcacgcatgcggggagcaatgcggatggcttccgccacaccagcagcacccacagccgggaggccgttggaatactccgccgcttggtttatgcccgcgccgcccagctgtattgccgaggtcagcagtcgcgcattcgccagaacagtcgggtcacccgtgccgattacacgaccagtgaactcggacatcacctgatcgaacgcacgcagctccacgtcgttggcacccgtagcctgcatggccttgcgcaggacagacacacctgcgtcgcccatgatgccgtgcttcgccagagcgatgtcaccagccacacggcccgcgtacttgcggtagttgtccatcacgcggttgtccaagtagtccatcaggcggaactcgccctcggcatccttgtacttgcgcgtcacgtccaagtcgatacggctcttggtgtgtttcgcaccaccacgcgagtaccggcccatcaccttctggatttcctcctcgttgagcgacagcgcgcgcagagtatcacgcagcgtgtcggactggttgtcggagaacaggttgtccggcgcgcggttcatgcccgcagcccgctcctcgatccgctccagatacttgatgctcaggtcgtcgaggaacttgtccccgtacatttcacccatcacgtcgaactgatccctcagtgcctgccggataccttcacgacgcacgcgcccagccgcagcgatcttaccgcccagccaagtgcgggactcgtaaccggccacgtcaccatcgggcaggcgggcagaacccaccgtgccgacagcacgctgctcggcagccatacggttgtagccctcgtccagcgccttcgccatctgcttgatggactcgtgggcgtcggcaatatcgcggcccatatacatggtctcgcggtacagcttcacctcgtactcgaactcgttgcgcatcttccagccggttgcgaagtccttaatcgcaccagccttccgcacgtccgcacgccacaggcgataggccgcttcccactgtctcgggcgcgcacccatgaacgactcgaagcgaccacggcgatccatcgctgctgtgctgtgacgaccagccgcgccttccgggttctccagcagggtgacggcgatcatgcgagcgaccggggactgcgacgacatgagcgtggtgctcgttgcctccagcccgaacttctgcatgatggtggacagcttatccgcgtcgatggcgtacttgccactgaagcgttctgcacggccgattacctcggcaacttggatgcgagttgcattgtcgctgatctgcttgtccagcccggtgcgctgcatgaaagccttgcgctcgcggttgctcttgaagatcgagttgaccagcatgccacgggtctgctgcgatgcagcctgcggagagcgaatctcctgacccaagttctcgccgaccacattcatcaggcgctccaacgcggactccttcccggtcaggcccagcacgcgggcgatcttgtccttcagccattcccacgcggtctgctgcgtcgcacccggaggggcgctgatgttgcgcagcactgcctgcacgtcgcggttggtcagaccgtacgacaccagctcgtcgctgttggcgaggaagcccatgctctgctgatccacacgtccctgcatcgcctgagtcatcaggttgcggtccgcctcggacaggttcgcattgacgtgcgtcagcagctcgtccatctgcgccttgaagttcgcatcctgccgcagcgagcggaaggtagcggcgtgcagcatttcgtgcagcaccacctcggcattgtgtgcggagctgcgcatcgccatcgcgttgagcgacgggttgtacccaccggccacgttcggctggttcgggaaccactgggccagctctgcatcgggagcgatgcggacaccgttcaaccggccgctacgcttcagcgtgttggcgattgcacggaagtcttccggcacgttattcgaggattcgaggtagcgcaggatgtcgtccggcgtgcccttgataccgctcgccttccacgcacgagtcagcagcgggtcagccggagcgttccactccacgctcccgcccacgttgtcggcgtagttgccagtgctcgggtccacgttctccacgtcacgggccagagagccggtggcgttcgaggtggtcggggcttcctgcgccacgtccggacgagcgaacaggcggaagtcatccggcacgtcagccatgcccgcacgaatccagtccattacctcagcgcgcgcgagggagtgaaccttcgcattgagcgccaccgggttgccatcgcccacttcggccacggcgcgggcgcggaggtccgcgttccacgcctcgccgtacatggcggcgttaccggaggccaagtcgatggttgccttgtcacgcaaggccgccgcgctgcggatgcctcgtaggttcatcgccgtgccgataccagctgagaaggcggcgtcggtcataaagtcggcgacggtgcggttctcgcccatgcccaccagtgctgcgtccgtgatgacggaagcagcggcgttctcggcaacgctcgaagcgatgcccgcagccacgcggccctcagcgaacagcgccgccgagccaacgccaagcgcgcgcgcgccaccggaggccaagccacccgttgcccagttgccaggatcggtcaggcccgccacgaggtcatatccaaagctgccccatccggactggttctccttgatccgcatgctgtggcggcgcgtgtcgatgcgatccgacacgtacgacagctcatccggggagtacgctgcatcgcgtatgtcttccagctcatcggctgtgtagtacggcttctcccactgcttcgggtcgtacgtccaaccctccggggtcagctcccgatcacgggtgatctggttggacagcgccgcgccaatgccactatcgaacgacgcgccccacttgtcgaggaacgtgagcgaatcgcggaaggccacctcgtcccggtcggcctgcgtagctgcgatggcagcgcgggtgttgcgctcgttgctctgcgtgtcgatggcagagacttcctgccgcacccaccatgggaccacctcgtcactaccgcgaacggcctgcgcagcagccacgccctgctcggcggtgccaccttccacgacgttctgacccatagccagctcgcccagcccttcgcgcaccttgccgatgtactccttcgtagctctggcaagaccgccacccgcgccttcgatagcatctccccgccatgctgcggggatgcttgccccactccacgtctccgtggtcatgttgcctgcaccggcccaagcggcactgatgctgccctggccgtccgcaccatgcgaagccacagcgggagccgtatcactacccagcactgccggcgcgtatgccgcattttctttaccccaccctcgacggtttggtccgccttggtagatacgcaaagcggtggagatgtcccccttagccatctgcatgttctcgcgcatgatgtgcgcgtacatttcaaggttgtcttggaagttccgtacgtcatacttcttaccagtgcgagcctcgatggtggcctgtgtcggaggcatgacttggaagtcaccttgtgctcccttcttagagcggataaccccatccggatcacgctttgcagtaccactaccggattctacgcgccactgtccacgcacaaccgactccggcactcccgcgtaagcggcagccgcagcgatctgctggtcttgggtcagccccgaaagatcgagtgccattgtctagttctccttagagttttggttggatggaaatgctctgttggatgctaccgtccggcatgcggacgtagccttgcggcaccgggaactcggtgcgggttgctgccttgcggcgcttctcgtactcggccttgatgtctgcgccggtgacggccacgaccttccagccgcgctcgccaacggtgttgacgtacagcaccggctcgccgctctcgctgtcacgcatacggaacacgtcagccttcaggctcttgctcggctccacgttgttggcgcggagggtggcgtcgatggctgcctcgatagcaggcccggtctccttggtgtccaggaagcccagccatgcaccgacgctgcctatgacgtgcccttcgtcgtcacgcccgttctcccagtaatacttgcccgcatcctcgccgccgtacttcagcttggcaaggttgagcgcagcagtgataccttcggaggacgtgtcgagcagcccgccagtttcgcccacggcacgcacgattgcacgtgcagctgcggctcggccggagtctcccagcttgttgccgaagtatccgaagtaggccgggttcgccttctgcaagacgctcgccactcgggactgcaacgcctcggactccttgcgactgttcgcactgaactcggtcgggtcggcggtggtgatttcaccacgcgcaacctcgtaggccagctcgaagttcacgccggattcctccagcgcttgcagcttgttgaacatcgtgttcacgccatcgccgaagtacagggctgctgtggtagcaccggacagcttgccctcgacggggttgccgttgatgtcgatacgcttggcagtcgtgttcttcagcatgcgccactggttgtagaggtcgcgcgctgcgtcgttcggctgctcacgcaggactgcgcgggccgtagtctggtactggtcggccacgcccttcagcacagcaccgcgcccagtgttggcgttccacaccagctgcgacatcgccacttcggggttcttctgcaaggtctggttgaagccctgcaccacgtttgcctccagcagctccttgtccacgcctgggacgttgatcgtctgagcgtaggtgccatgacgccacgagtcgatagcagcacggatgtcctcctgctgcgcagccagctttgcctgctcggtctgcgccaccttggcagccgccgcacgctcacgcatcaccgcttcctgcgcgcggatgtgcgcgcctgcggactgagccatcatgctcatgcgctgggtgccggagtacagcggatcgtcgctgccggtcgcagccgcgtagcccatgttgagctggtcgatctgcgcctcggtcggcttcgcaccgatgccctcggcagcgtacagcgacacgagcgccatctgctccgtagcctgcgggttactgtccagccactcggacttgtactgcgcctgcttctgcttgacgtacgcctgcaactgcaaggcatcgtccgggtccagcgccgacagcacaccacgctggttgaggaacttcagcgtgtagaactctccacggtcagcagcgccacgcacgaacgcggtcatcgccgccttgtagctatcgtccgtctggtaggcggaaggagacagcccatccagcatgctgatctgtgattgcaccagcttctcggcctcggcttcgtcgccgggtgccttgttgcccagcagcgccacccgcttcgccatttcgttgtagctggtggagttgctactgttgctagcatactgcgccttgaccagctcgctctgctgccacgccacacgctccttggtgtgcaggtccatcagcggaccagcacggtccatgaaggtcttctgcaacacggcatccgcataaccgttgccggtcatctgcgactgtgcgagcttgttgaactcctgcgccattgcttccggcggcagcttgcgcagctccggcatgcggtggatcaggtcttgctccatgtctgagaccgaacgcagcacgttgtagttctgcgcgccaatctcatagttcgtagggccgaacagcttgctgtaccacggctgctcggcagagatttcgtccatcgtctgcccgctgcgcgctgcaacgaagccatcccacatctgctgctgttccagcgccttacggttcggggcagtaatctcctccaagaactctgggagattgctgtctggcatagtcatgccgccagtatcggcgaaccaatcatttccgctgcgtaccgcctgaagcggggccacgccactaccttgcacaccggtctgtggaacggcagcggtcgcaccaagcgaaccgccaccgaccgtttcggtgctgaaggtgatcgtacccggatcaccgatagccatgtttcctccttagaaccacccaagcccagaagtgctggtggcgaagttgtcgtagttgttaccaaactgtgtggtgattttagcaggtgcctgccgcccagtaccgtcgttgtagttaaaggtgctggacgcccacgacttgccacctcgtttggacataccctgccacgccccgataccaccttggattgcggagtccatgctcttggacatgccttggaagtccccgttgcttgcctgccactggctgacagcaaggtctgccaccgcctcaccagccataggcccaccgaagtagcttgcgagagcaatacccacaccccacgcgaaccgatttttcatagccttcggctcgatgtgctgctggtaatcgaactgaccgaacgtccggctgatgtccattcccttgtaggcgttggacatgatctgtgccgtctgcgaagctccgcgacttgccatgaggcttatcgcgttctgctgcgtttccaaatccatttcggattgcaggcgcaccatagtatccattaggtcggaggacgagccaccgacaccaacgaagccagattgcgcagccagggcaccgcgcgcggctgcgagttgcacctgtgtattgaggcttgctccttgctttgcacgcagctcctcagacagctgctccatctggaagttgtactcctttgaggccgcgttcaccttcacttggttgttgagcgtgcgcatgtactccgagaagtttcccttcgccacttctagggcgttggtgttcttcgtcttcgcctcagcggcgcgccagttcgctcgtgcaacccgcgtggtgttgttggcctgaaggatagtgtttacgctacccattagctaactctcctgacgttgttaaaggtctgtccaacccacgacaggcccgtcactcggagcgggagccagtccttggagctgatcgtgtaactgcactcgcggacctcgcggcccacggggatcgacagctgcccggaatacaccggctgctgcccgaccaagttgtcgctgtcgccgaggattcggccctcgaagtcgatgctgctctgcactcggttgcgcgtggcgaccacggccaccatacctgcggtgttctgcacgtcggcggtgactcggttgagggccattcgcccgtccagcacagcctgaccgttctggtcacgcgggaacggattggttggcgtcaccgatgcgggactcaccacgccgaactccagcgatgcagggtcgaggtcgtcgaactgggataagaactccgcgatgcgtgccagtggcgtgcccagcaggaagtagtcgctggttgcgttcaccaccaccgagccatccgccacaccattctctgcgcggttcgcgtacgcgatgcgggagtcgatgtacccgtgctcgtccagctcgcccttgaagtccagcacgtccgccaccacaccactcgcgcgtccggtgaacacgatgcccgacttcttgtgggagctgattccgaggatgttgccaagcgtcggtgcgtaggcgaacttgctccacgcctccagctgccgctgcccgttgttcttgttgtcctcgtagcggtacaggtagaacgtgctgggctggttcctcgtgcggaacatcaccacgttcggcgcagtcaccgtggcaatctgcaacggctcacccttcagccagttgtcctgctcctcgctcagctcgtcggtcacggtctgctgcccgttgagggcacccacgcgcatctggtgcaggctcacgccctcgctaccgtactgcgagtagaagatgaagttgccggaggtctgagccttcgcgtcggtgctgtccttgttggcgctcaccgcccggatcaacggagacttcggagtcagcagcgcatcgccgctcacgccgtactgctgccgctcaccgaagatgatgaggttgccgttgtagagcaccgcatgccgcagtacgtcaccctcggaaccgaacgcgaacatttccactgggtcgtcgtcggcgatggtcacgacacttccgcgccagaagtcgaggtagtccccgctcatgcttgcattgacgtagttcgcactaccaacgatcagccggtcttggaagactgacagcatcgtgatgggcttgtcgatgaaccacgggatcggggaggttaggccgtcgccgaccttgcgtgcgccgtaagcggggtggtccccactcgctgggaagatgctcgtaatgcccgcgccgttgcgcgcgatgcacgcctgcccgttgtagatgtagagctgcgcgacgaggttgtcgatggtgcaagtaatgcccgcagtctcgaaccagtccaccgagccgaagcctgaggtctcaccgctttccagctccgctcgcaggtagtacgcctcgtccgtgccagcgccgctcgggcgcacacgaatgacctttccgtggaagtggtacttggtggcgtaggttgcatcggtgatttcctgcccagacgcgaagaacgtggttccatctccttcatcgtccacagtgatgtccacgaactggtcatcgtctattaggatggaacccttcaggtaggttgaggccacgccaccatcaactagcaagtccgacagcttctcggcgatgtactcgggcctagtttgctcggcgctggtgacgatccactcgttaactgcggagttgtattcgttaactcggtcgttgacgtgcttctgataagccgggtcaggctccgtgccgccaggtaggtagaatgggatgtcactggtatccagcgtgccggggtaggcagccgtcaccgtcttgtacgtcacctgcaacgtggtaccgtctgctcggtgcatggtcacggtgtaggtggtgttgaacttgccggtgcgaatccacgcagcaagtcggcgcaggttggtctcctcctgccagaggttggtgctggtcgcgctcgggaggttgtcgttgccagcgatgtagacgtagctgccgatggccgcgagtgacgatgcgccgcctgccaccagcgtgttgacccacgcgctgttctcgtacgtgatcgggatgaactgctcgcccgtcttgtcgtacaggaacgcgaagctcgcggagccgagcgccgaagcctttcggcgatacagcagcgcgtactcgcggccctcctgcgtgaagtcaaatacgtccatgtcttgcagctcgacgcgcgctgcctcgctaagggctagaggcagccgggcagcgaagcgcgtaccgcggcgacgcacaagcccttcgacgggatcggacagaatgttgatctgctcggtcgtctgtcccggtcgccgacgatgcggcggcttgccgctcacgccttgtacaatgtccgggtaggttccgcctgcctttgccatgatgcctccttagccggggaatgtggtgtggctgtgccacgggtgcccgctgtagttgaacacgcgctgacgaagaacgtccacgcttgcccgcgcatacaggggattcgccttgatctgacggatgtgctccgaccgcaggttgatccatgagtcgttgcgctgttgcataatcttctggtacttggtgttgtcgccgtcgaagtccgactggaaacgcagcacgctgtcgtcgcgcacgaacatctgcacctcgtaagggcagtcctcgaagtccagcagcctggccaccttgacggtgacggggccatcgaactcgtacttgttgcgtgcgacatcgtacaggcgtcggccgcgctgggctactcgccgcgcgccgcactgcggcaccgggtccaccttcagcacgtcggtcggaaccatgatgtacttgctggtggcctgcggctggagcttcaaccactccacgttgaaccacagcgcgagcgacgaggtgtcgcgcagcacacggtccacgaggtcgagggcatcatccttgtacgggtgatcttcctccagagtgttgagcttcgtttcgcccatcgtcttcaggcaggcgttcactacgtccaactttgtgatgaacatgatgcctcctagggaacaaggcagagagagcgctgtgctctccctgccggtggatcagtcggccgcgagggtcacggcggacggtgccagctcgaagtcctgcgagccgttctcgtcatcctccacgcgcacgacgatacgccacgcattgtcgcggccgaagacggcgacgacggtgcccagcgtaccggcctcgatgcccagcggcgcgatggcggcggtgatagaaacgcggttggaaatctcgaaggggcggtcatagaccattgtgtcttactccttggtagagggcgcagtttgagttacccgaaggattcagggactgcgcccggacggattagggagccgcgtcgatgcgaccggccagttcgacgcggttgaagccgacggcgaacgacatccagctgtctacgaagaagcacttcgaggcgtcggaccaccacacgctcgactggagcggcagcgcctcggcgatcagcagggcgcgaggcgagaccgccacggccacgaggccggtgaagtcgccgtcgtagaagttgtcgttgtcctcgttcgacagcaggtggccttcgaccacgccgttcggcaggttctcgctcgacaggaccgggacgccccacgccttgaagaccgggatgccggtcagcttgttgccgtcgctggtcaggtactcgccgttgacgatctgctcggcctgctggagggtgtagaacacggtcgggcggacgatcaggacgatgccgtcgcgctgcggcttgaccttcttggtctcctccatttcggagaacagcttgccgatggcagcgtacagcttggccggatcgttctcgtcaccggcagcggcgagcacgacctgcgtggcaccgaagtggccctcgggcgcgcggccgttcttggtgaaggccgaggtggtcatggcggcagccttggcagcagcgatgctgatggtggcgtccacgaactcggcaatctcctgaccctgctcgacagcgatttccttgcgggtgtcgatgtcggtgaagatgtcgtccagctgccagatggagtggcgcgacagcagcatggtgtccacggtcacggacgccttgctgaagtccacctgcgtgccgtccggcgcgtcgccgcgcttcagcttctggagcttggtgcggccgatggccttcttggtcagtgtgttggtgcccttgaccggctttcgcgggaagaacttctccagcacggagctggaaacgaaggtgtgctccacgtcgccggtgaactgctccagaatcagggcgttctcgttgccctgctggttgatctggttcgggaggaccggaacggtcgggaagatggtgctcatgttgtagtgatgctccttggttgttagtggatgacgcgagcgttcagagccttcagctcatcggacttcgctgcaccgctgattcccagcttgtccaccagcttacggtactctgcacggtactgttcgcgggtgagcggggcgacgccctgcaacgactcggacacggcagccggattggtagcgggctgtccctgcacggagacgttcgggttcgaggacgcgaggccgagcaaatgccgggccatcgcaacggcagccaagccgcccgaggacagagcctcactggcctgcttcagctgatcggcgggcaggttggtgcgtgcgtactgctgcacggccttccagttcgcctcaccacccacggcctcgtggaccttggtggcggtttccttgtgcttcgcgtcggcggcggcagtgatgcgcgacaccgagtccttcgccagagcgaggatcgggcctgcgcccttcgccttgtcgcccagcacttcgatcttggcttccagcaggtggaagttgcccttcgccgcttcggtcagctcacggctgttgatgtcgagacccagcgtgttgacgaagtagtcggccgcgatgttcaggccgttgtcgccgtagtccggcagctcggcagcagctggagcctgcggcgcattcggtgccggggcttgcggggcgggttcgaggttcagcgcgttcgggtcggtcacgaccggggctgcgggagcctgcggctgtgccggtgcgaccggctggttcggctggaccttggtctggtcgtcggcgggctgcgtgttgccgttgggctgcgcggtcgagacgatcacgtttgcgttggggccaccgcccggaggtgcgttctgactcattgggtctccatattgttctggttgtcgatctgctgcgaggcgttctgcatggcgagctgctgctgctgtcgcatctgcatcatctgactgtactcctcctcgctcagaacgtaggttgcgggatcaagtccgcgcgctgcggcgaggtcggcgatccacgcggacagcttcaggcggtcgagaatctgcggaggcagactcagcacgccgctgatgtcctgaccgaagcccagcagacggtcacggtccccggtgcgcgagagcgcggcgaggccagtgatgatgacgggttcgatgtcagaaccggcgatgctcttgtcgataagctccatgacccagtaggccacgggaacctgcacgtccacggcaatgcggctgtaaccgccgcccagtccaccttccagctcctcggccaccatgcggatttcttccgccgtcacgcgctcggcttgacgagtcaccgccgtctggagcaggaagcctgcgccgatgcggttgatgtagagctgctggatgttgagattggtctgtagcgtgccttcgacgccggagctaatcagctcgatgtcgcccttctgtccggggattgccgcgccgttgggcgaggccacgaagtcttctactgaagtctgaccagcagggttcaccaaccaccggaactcggaggcaaggatcgctgcttggatggtcgcttcgctcaggagggacagcgcttggaagtcgccctcgtagtcttccacgaggccggtgccgtagtcgtcgcctgccgccaagtcccacgtcacagcgcggtagggcagcttctccaaagtatagttcgacgagaagttggcgggtagctgtacgttgtccagccacacggtctcctcaaacttcgtcccgttgaacttaacccacttgtactcccagcagttaccatcgtcgtccggcttgaactccgggttgccgatgactgcggcgagtgctgcgggcttgatcgcggacttgtgaatcttttcgcggatgatgagttcgcacaccgaaccttggcggtcgcgcttgacgacgtaattgcggaggttcagcacgcgcaccgtgtccttgtcgaacaccatgagtgcattgccaagcactatcagcatcttcagcaggtcgtacagccgggcgcgaatggagcgcttgtctagctccagagaggcttcctgctccagcttcgcaagctgggtctggattgccttcgggtctacacctgactcgctcatcgaggctctggccttgcggttcgcttccagccggaagaacgggcgggacggtgcgaacagggacatcatcagcttgttggcgaggtggttcaccgcctgcgctcccagcgactggaagccgtgggtcagcggctcggtgtcctgatcgcggttcttcttggggaacagcttcgggatggtccacgaagcgtagcgctctagccggttaaggatgccgttacgcttcccgtccagcttctcgaagcgctgttccgcagtggtcgggcacattggattgtccatgctcacctcacaataggtcggtgccggacgtaccggtcagccgtgattgtgctgtggggatgatgcgctggtactgctgccgggtggtacgtcggcggccgatcaggtcatcggtcttcaggtcgaggtcggaggtgccaagggtaacatccaccgtttcgatgggagcactcagcaacttctcggcatactcgctcgcagcctgttgggcggcagcggtagccatctgatcggccatcgcctgaatctggtaattggtctgttgggtctgaaggttggtctgacggtcgatggcagccgcttgcttcagggctgccttcttcgccgagccacctccgacgagggaacccataggctatctccttcgtttggtgagttgcggcgaaccatcctccagctcgaagccgaagcgttggtacagccgagtgattgcccgagatgatcgagctagtgctccgcctgtgactatggcatcgcaatcgttggtctcggctagatgctccagtgtggctactactgcccggaaggaactgcctttaccgatccgtagtaccaagtcctcagacaggactaacctgttcttagagtaccaaggtttaactacagagaataccagtaggtagctttcgtctatcactactgcatctaccatattctgtactaccatttccacagtgtattgtggatcgtcacagaggtagcttaccgaggagctactatgctcactctcactcggggctaaagacagatacagggcagcgtctagcgccaccctgatctgctctctatcacccgtcgttggtgttcggattgctggactcaacggtgaatccctcctgcaagatgcggagaactcgtgccattccgagctgcacacctgcctctaatggcgtggtgttggaattgacggagaggacggaacccgcctgtcgctgcacggcagccagttgcttcgggtccagtcggtagatgatcttggtttcggacatgaggtctcctctgtcgtatgtgtaccaaaagggtttgatgcctgcccacgaagggcgaggcacctttgtcgtatgtgtaccgaaactccatcagctgaagaagtacggagaatcaatgacttgcgagaggtcgaggtcgcccatcggcggcggctcgggcaggaaaccataggccgccctgaactcctccagcacgtcgtgcctggagtacatgtccacgaagacctcccggatgatttcgtacaggcgggccgtgtcggcggcgtgggtgccatagtcgtcgtggatcatggcgaaggcgttgatgccatcggccttggcccggttgaccaccagcgtcaggtggctggcgtcgaggctgtggacgaagttgggggcgatgccgttgcggtgccgggacttcttcacctcgtctgtgcttcggcgcacagagagcttggtgttgccgcacagcttggtgttgatccggtgctcctcagtctcccagtacacctgcgtcaccgggaagccggacggcgtgatccacttgatgcggtcgtagccctcgcgcaggatcgccgtggatgccttctggagccacgccattgcatcggctgccgccactaccgtgtcagcgatggcgacgccgaggcgcttgctcaggaagcgtgcggccctgtcgtagagcttcttgtccagctcagggaacttgtcagccttcaggtagtcgctcacgatgaagtccgcccagctcgattgccgagagccgtatggcagggtcatcaccgagcgcttaaccagcgagcgggtcaggccgtggtccagccacagcctacggaacccttcctcgtcgtccccctcggcttcgaggagcttggtcacgaggtccgccaccatctggtagatgtcattcggcagcggtgccgggatcaggttggtagccttcccgcctgcactgtcgcgcagcattgcggagaagttctgaagcccattgcaggaaccatccatgccgactgcgatgcggctctggaagcgatccccgaacacttgccactgctcgtactccaagcaccaagcgaggaattgcagcggcttgtctgcggtcttccactcgtcgttgttcaccgggtccgcagcaaacgccagaatctggtcgtgatgctcggccacccacttcacacgatccggcagagacgccttgtcgtatccccaccggtttgctcctgtgatgcagaaccagtccttagctgacttggtgagcaagggcttaccctcgccgaactccagcagtgccttctgcaagtccgaaccctgcggagatacgccggtggtctggacatacttgcggccacggaagtccacgaagtaaacgaagtagattgcttggtagtctacgaacttgcgcgccactcgcatggcgttgtagaaccgattgctcttgctgttgcgcagtcgctcgtcggtgtgccagtcggccacctcacgcttccacttcttgaactcgcgctgctgggattcggacatgtcctccttggtcattcctttcgccaaccactccggcttgcgtggcttcggcagctcggcctgcgaaatgatttcctccatgtcgtggacctgtgccactgcggacacagcctccagcatgcgtcggttgattctccactttacctgctgcaacgcattgaccgcagccatttcgttacgcagctcggcggagcggtagtcgtcgcgggtctgagcgtaggtcttcaccatccacgggtgcagcctgcgcatttcgttggtgtggaatccgccgttgtccacgtcggtccagtccttcggtggctcgacgcacggcaggaagtacggggtgctctcgatgacgaactcgctgatctggtggatcagcttgcgcacgtcctcggtaagctcgacgtgcaggttggtcttcgtcctgcgacgtccaccagccacgatggtctcgttcaccacaccggcattcaccatgcccatctgcgcaagctggtcaacgaggtagccaccgacctgatcgcgctgcgcctgcccccactcgtggaactcgacgccgttcttcctgccctgcatcttcatcactgtcatgcggtgcgtctcgttgacgctcagcttacggtccatgtcgttcatcaggtggtagaacagcgtcggctccgcgtctgcgaactgggtcagcaggtactcgtggtacacattggtgccaacctgcttcaccacctcacgaccggcagccttatccttcttgccctgctcggcgatgcaagctgccaagcaaccacggacggccacgaaggcgatagcctcgtaccattcggtggcttgttcttcggcagtgatggcctgcccacgcttgtcctttcgctccgggtcgtacttcgcccgcagaagtggcacatgggcctgcgctctcccgatgcgcggcttgtcgatgtcagcccggattcgctccgcaagcggaagcacgaaccggcgatacaccgcctgagcgtacgggttgttcggcgcaccgccgttctcctcgttgcgctcaatggccttacgcatgcgctcttggccgaaagcgtaggtctccagttcgagttccgcttgtgtgagcatgctacctccgttacctgattgtaaagtccatcacctgtccgccaccgccttgtcgtggcggattcccttgtatcgcggctcgcgcagcaggccgtacttgctgtaggacatggcctcgatctccacgatgtccccgatgcagggcagctggtccgcgctgtgcggcacgccgctgccgacctcctgctccttgccttcgccgaggtccacgaccaccgtccacacgtcgcgcccggtcttctcgccggtgctaatgttgacgtgcatcactcgcaggtccagagtcagggtcggcttgatcttgatgacctcgcccttcgtgcccttgtcgcccttcgtccacgtgccgctcggcttgcgcaggatcaggccatcgtacgggccgctctcgcacaacaggcgggcggcttccatcggcgacagctcctgatccacgaggaagccctgcgactccgcgaggaagaacggagccttgcactcctcgatcttgctcagggtcggcggcagtcggcccacgcggtcaaggtaggtcagcgggctgaatccctgctcccactccccgatgctcacgaagtcgaacaccacgaagaacggttcggtgtactgcgtgccgtccttcttgcggaacatcccgctcacggtcggctggtcgatggtcgggtgccagtattcgccaaggtacacgccgatgggagcgaacggcgcagcggccaacgcttccttgatgtggttcgcggacatcacctcctcgccagtgcggctgaagatcgtgatgtgctcgacggagttggcagcctttaccaccacgcagttgcagccgtcgtacttgggctgcgcgaggtactcggttcgcagcatgtcgtcgctggggcgctgacgcttctgcaccttgtccagctcgacggccttgtgtacgatgtagggcttactcatcggccttggcctccttggtcgggaggttgtttcggacggtcagcccgccgacgttcgatgcgattcggccagacatgaagtctgtgacgatctggccgatccacagcttgcgcggcaccatgccgttgcggtagccttcccacgcatcggcgatgcgagcgtacaactcggctttgccttcgtcgttcagaccggggaacgcagtgttgaccgcatcctgcaacgcttcatcatgatcgccattgccccaagcaacggcaccctcgtaggactggatcagacgctgggtgttggacttgtagttcattcggtctccttcgacgcggtggaagtgttggttgctcgtggcgctcgcggcgctccttcttcttcgagcttcagctgtagcagtgcagcagcacgccacagcacgccttcgtagtcgccctcctgcaagtgtcgcaggatgcaatcttcgtgatcgccactcttgtcacgactccattgcaatggcataccggggttgtgcttctggttactcttgtacgcatgatgcgccagagcattcatggctgctgggaagtacccgaacaacaccgagtacaccggatactccttacgttcctcgctaccgtttggcagattgcttgggaagcgtgccccgtcgttgagcttgtgggtgcgctcgtcctcattacggtagttcagctcgggcagtacaacctcacgccgtgctgtggtaacacctcccacacctataaggcgtgcgagtaactctggctttacgaggctcgtagcgagtgggcggtcatccgttttaatccgcacccacttatcgtcgatcccaaccaccaccccggatttaccgacgaggttgttggctgatccggtgtagcgaacgcggtctctgatgcggacatctgtaagtctcatgttacctccttatgctggaacggtgatgtggcgacgctgctcgatgttggtcgtcagcttgcggccacggctgtgcccaccgcactgtgtgcattgcagcagcaggtaggtgccgacctgagtgcgggccggtgccttctgcgggatcatttcgttgtgcccgcacttgttgcagcggtgctcgctgccgtcggccttgtagtacaccgcgatgttcgggtgcctgctgtaccagccacgcagcttgcggtactcggccttcatggacttcacgtcgatgatgttgtactcctcgcactcgtcccatgcgccgggcaagccctgcatgcacgccacccacaggtcgaagccggggaagttcgcatggtcgtacttgcgcagctcgggaacgatgactccggtggtgtactccagcttctgcgaggtgaacgcgaactcgtcgcggttcagcagcatcgggtcgatcacgctgaccggggagagcggagggaagccgaggatggcaaggcgagccttcaccttgcgcaggtcgaacttcttgccgttgcgagcaagaacgaagtccgccgcgttgagcagggcgtggagaaccttggcctgcttgcggtcgttgaacacgtccttctcgcggcgctggtccacgtagatcgtggcctcgtcgttgtccagccactccgcagcgaacgacatgagagaccagtcgcgcttgatctgcttcgggctgaagttgttgttgaacatctgccatccccaaaactcgatggggaaggtctcgatgtcgaggcacaggatcttcggcccgtgcttcggggcgtgcttcaggaatgtggtgaggttcacgggttctccttcttcattgctcgggccttacgcgctttcgcattgcgagcggtgcgcttctcgtcctcggtcttgtgggtgggatgcagatagcccgtgatgttggtcatgtgctttcgcaggtaattcgcaagtcccccgcagaaggcgaggatgtcccgcactccataacgtgggccattgttctcgaccttgcccagcagcgagttgcacccacgatggagtacgccccgcactgcgccagtgcggtgatcgtgatccagcaccgggtcgagcggtgccttcagtccgagctgcccgccgcacaatgcgcagcggttgctctgctctgctgcgagtttaacccgcaccagcttcacctgtgttgctgtcagacgcttcatcgtttcagttcctccagcgctgcgcgcttatcgttgacatcctcggcgaggtcgtagaacgcctgcttcagcttgtcgccgaacacgtccagctgtagaacgtccagcagatttgcgtcgcgatccgtacgcatccacagcagcaccgcctgctcggcgaagtaccgctgccatccttcgcccttcacctcggcgtacttaccgtacaccaggggcgcggcttcggcgttgctcttggttccgaacagtagctcctccgccgtcaccttgcctaccttcggcaagccggggatgaagtccgccgtatctcccatgagcatctgcatccagaaccacttgtgcccatactgcaagccgtctgcgcccacgaggtcgtaggtgccgagcggaacgtccacgatgtggtagtcctcccacgtgatgtgggtgccgcagaacatacgcatgtccttgtcggcggtgtggatcacgtgcagcacgttgccgtgcttggctgctccggtgctaacgaaggccattccatcgtccgcctcgcgggtcgtccagattttcggtgtgaagtgcgggccgtcgtacgtctccatccactcgcggaggaaggcccagttgttcggcttgcgtcctgactggcgctgcccctgatacggctgagtcgtagcagcgaggaacctgtcacccttcgatgacgcgccatgtgtgaggtgcatgactacacgatccgctccgctgatatgcttcagatgcgagacgcgggagagcacgttgcgtcgtgcgtcccccgcagaacagttctcgctaccagcgcagaagtacgcagcgtagtccccgtccacgtgagcgatcacgtttcggttgtgctgtcgtacttccacgatgggcatcggggagcgctccgcagccgcagccatcagagcgctcaggtccatcaggcgacgcccgccatcgggtcgtccatgtcgaatggcggcttgtcgtcctcgtcgccctgcgcgttgtccacgtcaccgaccgcctcgtccagcgcatccacgccttccttggtgacggtgccgccgaccagcttggaggccgcgtagtcgtagcacggcagccccttgaagttcagcgccttggcgatttccagctggatggtgttcttgctgcgcgcctcggcgatgaccttgccggtcttctcgtccttgcgctccgggtactcgccttcgatgtagatgctgtcccacatgtcggcatcggcgaagtcccacacgaatgccttcagctcggtcatggccgcgcccaccgggaacacctgctccagcaggttgccggtcggctctccgtcttccagctcggggacttggatgatcggcttgcggatggattccttgtcgatgttggcgtacgtcttcttcttgccttccgggccgcgctccacgtggaccacgttcagcagcaccggcttgcccagcagctggacgaagtgcttctcgtcggtgcgcaggcgggagaacatcttgaagtacgcggccttctcgttggtagagaggttgaggcgcaggctcaggcggaccggaatcttgacgccaccatccagttccttcggcggatgcttcttgccgatcagctcgaacacgatgatgacttcgttgttggtcttcttcttgccctcgaactcgctctcgtgctggcccacctcgtagtaggcgacgatgcgagcgccggtctgcccggcctcgggcggagtgtagtcgccgccaccggcggacgccacggactggtcctgacccttttcctgcacctgcttcagcagcttgtcgagactcatgcgttggtttctccttattcaaacgacggattgtgattaccgatgaagtccttgcggatttgcatgcggtactcggggaacaagacggcgaactctgccggagggttgtgctcctccatcatgttgtcgcccatcttggtttcgcatggcacgccgagaggcagcggccacttgaaccaccactccatgtaaacggaggcttcgagcatgcttgcatgcaggagcgccgccgcttccgtggcgatggatgctgcgctgtccacgtataccgcatcgtggacctgattcaccagcagggcttggccgagccagcgctcgggctgggtgacgtacatgcggtagaaggcccgcagcgagacgtacatgctcgccttggcccactctccgccagtaccctgcaccgggtagttcttgatttccgtgggtgagaacgactgcgccacgccgccacgtgaggcgggtttggttgcgatgaacttgggcgaaggcgactcgctgaaggagtacatcttgccatccggcgtggtgaagtgggagcggcccagctgacaggtcagccccggcacgtccggatgctgcacgaagcggccagtcgtcacacggttggccttgatgacctccaccatgtggtcgatgtactcgcccagctccgggtaacgctcggcctcggcgcgcaccagcttctccacttcctcctcggtcatgcccgtggtcgctgcgatcttcgcaacgcctgcgccgtacgcacgctggaaggagaagaccttcgcgttgccgcgcatcttcttccacttgctgtgctccgggtgcgtctcgtccttcgctgccttcaggatgtaggcgtagtccttgccttcggctgcaccccatgcctgctcggcacgcaggacgtgcatgtccagaccagccttcaagtcttcgatcagctttcggcattgggtgaggatcgcctgcacgtagatttccagcgacgtgaagtccgactggatgatcttgccaccggcgtgtcggctgatgaacgcgcgcttgatctggctgcccttctccttaccggtctcctcgtcgtactcccccttgctcacgttctgcaagttcgggtcgctcgacgacaggcggccggtcacggtgttggtcatgttgagcttgtggtgtatgataccgtctggccccaccagagtgagcatgcccttctgctccccagtcttctcgtccgtcgtgatgaagtatgtggacaagtccttgtggatgtcggcgcgcttggcgagcgccttcaggaacgggatgtcacgagcgcccagctcctcaatcacctcggctgcggtggagtacacgcccttgtcggacttgctctcccatcgctcgctgccttcggtgtaaccggggaacacaaacaccatgtcctcgttgcggaacttgggcttggtcaggtcatcgaccttgaccttcttggtcttgcgctcgcccttgttcttgccaccagcgaacaccaccggctccttgccctccggtactccacccgcatcccaccactcggtcgccgcgcagtggtcccaccactcgcaggccatcgtggtgccgtcttcgaggatgtaatgcagctcatccttctggacgtactgctgcttgccggtctcaggcaccagcaccggcaccttcgccacgtacttcacctcgccgccgaagatcagcgcgctcttgtggaagcggctgttccagttgaaggtcaagccctcgggcagctcggggatgtaggactccagctctgccgttgcgtttgcaagctcctgctccagcttcttcgcatgctccagcgcccacggcttgtccacgaacatgccgttgtactcggcttcgatggtaaagcacagcgcgcccatgttgagcagcgccgagcgcagaccgttgcgtgcccggaaggcatcgagctgaccgaggaacatcttctcggtgttgccgatgtcgcccacgtcgtccgtgtcgttggtgcctacgaggtagtccataagcagggtcttatcgatgtcgcacgtatccacccctgcattccacagggacttcaccgcgtcgtccttcaggttgccgccgtacctcggggccacctcgtccatcgcgcacatgtggaactcctgggtcatgccgtacagcaggtactcggcaagctggcagtcccacaccatgccgccacggtcgatgaactcgatccatgccatgcgattctgcgggccttggcagatggcgtgcaggatgtcgaacttgatgttgaatccgacgaggtactgcgcgccgtagcatagctccttcagccaaccatccggcgcaccgccgacgtagttgttgtcttcgtcgcgcccggtggtgaagtaccgaccgctgttcttggcgtcgcccttgcgcttgtggccgatggcgacgatgcggttgaggttgtagaacgggttcgccttgcgcttcagcgtggcgcggatcgtggtctccaagtcgaaggacacgtagctcatagcggccaccgttgcagagccagatggtacatttcatccgacgcatcgccatccaagtcgagaccatcgcgcacccagcggaacacgatgatgcgatcctgcttgtccttgatgttgcgctgcttgcagatggtggtggcctctaccgcgcgctgataccagccgggatcggcagtcaccatgacgttgaacgcgccgttgcgaagcgcataccacgtgctgctgtagtcctcgtcttcctcgtagtgcccatcggcaccagagcatatggtccacccagccttgaccagctgatctagtgcctctccgaagtcctcgaccagcacgaggaaatcaatgtccgtgtcagtcacgggaggttcgacggtgtagctgctgccggtgcggctggacgcgatgacgcccaacgtgggcggcaggtggacgttctgttcggtactcatacttcctccttgacgaagcggcgggcgtggcaccagactttcttgccgtagtcgtcctccaccatcacgtaagcgggccacgtgaagttctgatcgggatactccggctggtagtcgatgacctcgtacaccttgttggtcgtgaagaagtagcctcgggagcctacgcacctcaccttgtctcccacgctcatttcgatcttcatgcttcctcctcgtagaaccgggcgcggtctgcgtcgaacatcacctcggcgcgaggatcacgcttaccgcctgcgcggtgcagcttgttcttcggagtgccgatgtatcggaagcgatccatcgcaggatcgttgagctttccgcccatgatgatgaagtcgcacgcgccctgctttccagtcttgctgtctttcagtgcggactgcggcgggaactggccgccctcgccctcggcgctgatctgcgaagtcgccacgcccacggcgtcgtacttcacgcaccagttgcgcgcggcttggtacatggcttcgagcatctgatcggtacgctgcccaccgttggtcatgcctccggtgaacgtgatgttgtcgatcatgtcgaagatgatgaagccggggttggtctgcttgatgatggcctcgacctctccggaggtgaagccgtggatgtcgtagaactgcatgcggtggatgtcgccacccatcgcttcctcgatccgctttcggatgctgccgtccttcgcccactccaccatttcggggatcgttgcgttgaggagagactgataccagcgctgcttgatgcgcttgcccggcccctcgttgttcaaccagatgccggtgcgcttctggtccggccacacgtcgtccagctgcggcagccagaatgtggactcgctggtgaggaacgtggtcttgcctgcgtcgggacgcatggcgtagatgccgaagtcgcctccgcgcatcgggcgcaggttgcggctcaggctcggcagtcggaagtggattccgatgtcgccctcgtccattgccatcagttcttccggcgtctcctgcaccagcggcagccgggccttgcggtccatgcgctcggtgatgccttcggccagagctgacagctcatcgcgcagggagaactccgcgccaccattccactgcacgatcttgctgacggcggacgtggcaagctccagctccagcatcttttcgatcatgccctgctccgcctcgggcgggacagcctcgcgcatcgcacgcagctgcaacttcagcagggatttcttgtcgtcggggagttgcttgaacttgaactccatcgcccagccgtcgaacacgtcgtgcggcagagccttggtgtcggggaactccttgtagtacgcgcgcagtgcatccagcatcagcacggtcagctcgtccagcccctcgcgcggagcgttcgggaccagccgctcgaacttacccttgtcgctgcacaatcgcagcagtgtgaggtcaagactcatcgggttcctcctcccattcgtacggtgaactcatgtcagttcctcctgccgtttagcttgttgagttctagcacaaaatccagtgctctccggtctcttcccgagaacacccagctagacacgtgataccagtgttggaaccgggaggaccaccggatgcgttctttcacagcagcttctcctctatgtactcggtcggataatacttcgggtcacggtcgctcgtgatgttccgatagtccaagccgaacgcacgaaggcgcgcggcgatttgtttcgcagcatcctgaccgggattgctcccgttcgatctgcccttgtcgtcgtcgagccacgtcgctacacgttggcctcgctcaatcagctgcatcagcaccttgttgtgcagcttggtgccgagcaacgaccacgcttctgtcaccagtcccaccttgtatgcggagagcgggtcttcgcatagaacgatggtgtctcccttgcccacgccgtagcgtgcgacgagtccgtctttcgggacatcgggagtcagccacttcggttgcctcgtagaggaccgggctgtccagtacacagggcggtcgccttccatgatgggtagtatcacgcgcccgatgtccgggcaccagtacaggccaagttcccctatcatgcgaagcgagaggcccatcttgtagaaccacaccttgtcacgcagcggccactcggttgtttcgtagacacgtggctctggcaactcaacagttgcgcgcactctgcgctcgctggtttgctcggcatgggttcgtactagcttggcttctaagctctcgtgctcacgcttgaatcctgtgccaccacacctgaaacagtatgcggtggacttgtcgtgcgagcgagtgatgagcaacgagtttccctcaccacacgcatggttgatccgagtacgggtgccgaccttcagtcgttccgcatgcggcagccagtcgctgtcaggtagttcgttgctcatcttgtcctcgcttagattgtcggaacctgtccgccgctcggcaggaagtacacgaagaaccagtacaccacgtacaaccagcccagcaggaagtgcaggatggcccacgcgatggacttgctcacggtgtaggacaggaacgcgccgccgaagcagccgatcagtgcgacgagccggttcaccagatggcccacacgctggtcgggcttgcggccacggtggtgccggagtgccgctcgatcaggagcgggttgcccttcttgtccttctggtcggtgacgatgaagacgttatcgccgtcgctcgccgcgtcggagtcctgacccagcagcagggttacgtactggcccggcaccagagcaccgggacgcaggatcgtggctgcggtgtaggaacgggaggtagcaggagcgcactgcgcctgcggctggctcgggccgatcattcggcaccgccttcgctgcccttctcggcggaagccttggccgcgtcgatgtcggcctgcgccttctcgatttcttcggcggtgaacagcagggcggtggcgtcgatcaggtggaactcggcgtcgaagccttcaccgtgctcgaccttcagctgcacgatgcccttgtcgttcttcttggtggccgacacggtgccggacaggacgcgcttgttcatggcgcggccatagacgtaggccacggcgtcgcccgccttcagcgcttcgattgcagcctcgttcgcggcgtcgttctccagcgcagcgatcttctcgtcgatcttgttgaccttttccatcgccttcaggcggtcttcgcgcagctcggccagcttgacttcggtgtgcgagacggactgggtggtggtttcgttcgacatttggtgtatctccttgacgttgtgattgagagtgcctcgtaacgtgaggcagacgactctccgagtaggttagtgcttggtcgggccgaagatcagctcggacgtgtagccgccctgcgcccacgggcggccgtagtgcctgcggcggagtacgcactcctcgcccagctccagcagcgtgtccaccaccttgcgggtggcggccctcacttggttgatgtcctcgcgctggatgttgaagtcccagcgcaccacgatgacgtgctcgtagtctgtgctgccgttgtcgttgcggacgtagaagccccgaccctcggtcagagtggcaccgccgatgatggcgacggtgttgtccagcgcctcgcgcagcccgtcgtcggacatgcgggtgctcgggatggtgacttcgatccagctaccgagaagggcgctcattgcgcacccgccaaggcgttgcggacgctcgggttcagcggcgcaccggcacgcagctcggctgctcggcgcttgatcttggaacgcaggcggcggcgctgcttgttgttcgcacccagagaatcagctgcgcgcttcatctcgttgttgcccacgttacgggtctgcccacggcccgacatgtagtcctgacacatcagcttccgcagcagcgggtcttcgattggaaccagcggcaccgagacgtgcaggtagcgggaggtgtccggcgcaggaggcggcgtgttgtcgtcatcatgctgcggcttgaacgcctgcaccaccttgtccttcacgtacttggccgcgcccttgatcttgtcgaggaagcccatcagcgtttctccttgttgtggaagtagttgaactccagctcgtgccacacgtagtacgtggtgccgagcgggtcggtcatttcctgctcgttgcgcagcgtgcagtagtcgttggcctcgtcgaggttgtcgtaggtgcggacccacagcccatcgggagttgccgggatggtgcggaaccggcacagcctaccgtcatcgtcatggtactggccgatgacgatccacggaccacgcccgacgatccagtagagcaggataagtagacgcagggcgagcttacgcatcggcatataccgcttcgatgtagtagccgtacgggttgcccttgctgcgcttgtcgccgatggtgtccagcacggggcgggcggcggcgcgggtcgggaacagtagattgctctcgtcgttgttctcctcgttgccgtcgatgcggacggtggcaccgtgttcgatgctgttgtaggcgctggtgtagtcgccgtcgtacttcagacgccaacccagcacgggctgcacacggcgcaccttgtcgccgaactcgcccacgccgtaatcgaagtgcggggactcgaatgattccagctcgccgatggcggcacgtgcggcagcgcgcttgtcccacaccaccacggtgttcgggtaggtgccgtcgcgcagcgcatcggcgaggctcggcgtcgcagcgggcttgatggtggacaggatggcctgcacttcctcgggggtgaccgggcgagcgccggtcaggttcgtgttggcgacgacaccgacgatggtgttggtgcccttggcacgggtgatgccgaagtaggtcttgctcatggttgattctcctcgttgacgggtgggatttcgtgctcggtgtgggtcacgatgtagccgtgttcctccatcatgccgcaccaagcatcggacatgcgagggtattccaaggtgctgcccgtcctcgggtcgagcacttcggttacgaacaggagccggacctcacgcataccagcgttccacgctgtgctcgttggtcacgaactctttccactggcgcggcttctcgcacagctgggccggcttgcgctttccactacggatgcgcttgtagattacggggatcatgcgttcacactctctttggtcagttcgtcgatcaggaaggacagcaggcggcggctccggccatactcgctgtcctcgtcgtacatgttgccgttgtacagggcgtactcgtccactgcgtcgaagtaggcggcagcggcggcatcgggatcgtcccagtccactgagtccatatcgttgtcggaacggtactcgtagatcatgtcgtcatcttcgcccgacgccgggaccgggtacgtgctgcacccgctccactccggccactcacgatagagctgcgtgcggaggtccacggcagaacccacatcatccgacgtgaggccgtcgcggtatcgtatgtcccgcatctggtcggcgatcttctcgcacagcgcctcgccgagattgttctcgtcgtcgatgtccgcacgggcggcaatggccgcagcgaggaggagcgcaacaacgcgctccccgtagattcccgtgaggcggctcatgccttcacctcggcgctcttgcgcttggtggcgggcttcggcaccttgtgcgcggcctcgatcacggcgcgctcctcgtcgctcggcgtatagccgccatcgacggccttttccagacggcccagcagcttgtgcaggtcggcggcgaagctgaagtcctcggcgggcttctcggtcttgaagtcatgccacatcttggcggcggcgcgctccagcatggcggccagctcctcgccctccagacgcttgctcttggcgtacttcatcggcatggcggccttggtctccttgtcgtcgtttggagccatcggaccgaactcggacaggtacaggcgcagcgcctcgtgcttcatgccgttgcccacggcaaggcacaggtcggcagcgagcgtcacgtcgccgtggacgtgggcatggttaatgacggcgattgcggtctgctgaatcgtgtccaccagcttggtgcgtgccgtattgatggacttgatgctcttgcggatgttggccgcgttggtctcgatgttcatggtatggtcccttcaggttgggtccgtgccgattgcacgacactaggccctcttgcgaaggcctagtagcttgcattacgggagccggatgctgtatgagcgcccgccgcatggtaggatgctcaggcaggacacagcgccctgcggatgcttcaggatggcccgattgtagctgtcgcgggcagattcaacgtggaagcgagagaatttgagcaggatcacaggaaagccctccggtcagcggcatggttcgcccgattggtcccgctatttcctccagcaacaaacacagatcgcttacctgcggtcccgtgtcgtgcctcatagcgctcagcttggcgcttgcgctcggccatgcgtcggtcctgctcggtggtacgcaggtccataacgcttgcagtccgggtgaactggcaaaagcggcgcttggtgctggttcgttcgagattggcgttaccgtgcatcgtttagtcctccttctggacggaattgatttgaatccaatcgaacccagattcggcgcggcgtttccagaactctttgcgcgcctcggattcggaactagcagaaaccatatcagcgtattcccggccgtgctcgccgatacctgcgaggtagaagaaaccgtacatatttgtgcctccattttggcactgtgagaaagcgaaaacatacagattgaagctcactcaggaaagccgtcgagtcggacgatccctcattctcgattagagccgacaagcaaggtttgcgcagtgcactaccgaatgccgggagtgagattcaatctgtatgccccttcgggctgtcaaccttactccgggcatacagtgccatagtcactatgcgagcggagcgctctgttcacaacccgccagattaccggcaaggtgggcaaggtgtcgcgtctgttagggtgcacattccgtgtgccgaattatggactaatccaacctagacgcggcttgcctcttgtgaccggcttcccgtattccgacgggttacgctgctgggccgactctcacggcagatgcaggtcctaggcgttagtcctaggtaaagcggcactggtgttgctagtccagtggattctatgggccttttatatcccagttcatccggttttccgctagtgctacgtttcagcttggcgatccacccatctaggcttctcgttacaccctacccgttagcggtagtcttatatcccggtccatgatgccggtggtccgcagaccgtgaagccatagtaccctatcctacctcccgtgtcaagccctgtggcttaacccgtagcgtcctgtcgccaccatcctaccatgtaagccggtagtccgcttactgatcgctccgcctttaggcttcctgaccgttactgcatagtagcctactattggcttcctgtcaagctatccgggtgtacgctcatttgcgccttgaccggaagtctcacccatgtacccttagcccattgcaagcggcgccactacggtagacttatcactagactgaccactagcttaccactacgctaactgtctgtcaaccccttggctgtcaatgcttgccgtgtggcttgcatcggcgaccggttcctagcttcacgacgctaggagtggagcgtagggaggatgctaggctatctgtagcttactgtcaagcccctgatacactttccggctaaagaccgatacgataatcgtggcaagccattctgtcgtatgtgtaccaaaaggaaaacgatacagatgccgtcctcccgtccctcactgcgtcccaatcatcgcccggtaggtatgcacctgccatgccatgcgtgcgccgtgtaggcccatcggcggccacgtgccgcgcctccaatgggcgggctgtgcttccaacgtggagccattgaatcacactcccaaccagccgtcaagcaccaatcgcaagagatttattaacgattcagtcagcctcctagtgcagtggtgtactacctggccaacacacctccacgcgagaggagagaggcacccgcgcgcacaacacgcgcccacgcgcacgcacaggcacccacaggcgcacgcgcgcacaggcacgggcacacccacacacccgcgctacgcacgcccgtaggcgcgcataggcgcacgcgcatcacgcgggagggcgcacgggggcgcacacgcgagctttgattggagtggcccccgcgcaattctaaatcaaaatttggtccagctcccgatcagcccgtcttaagtctaacgatgggcgcagcggagtacatgtcgatagcgcacgcggcagccacggccttagccgcagatttgctcacgtggtacgctccacgagcaatacccgcgccgctgccaatgaagatcggagcgtcatccggccaagacttcttaccgctaatgacggtcgcctgtccgtccttgatgataagcacggtggagttgccactgaccagcggctcgatggcttctccgcctttgagggcggctaccacggagcggaggacgtgaatctcaccggctacggcgcagaagaccggaccctccgtggtttggacccggagagccttggtcatcgtgcccttcatgtcgtccgcagtgacttggctgtcggcatacaggtgcttgccgtcccacacgatggtcgtcatgggctacttctccaccttgcagcgccaaccgcaggcttgcttgtagccgtcgtaccacgcacgcagggcgcgcttgtccacgttgcagagcttcacgtcgaactccctgtcaatagcgagcttcgctacgtcagagttggtcggatgctcctcggtgaggtacgttacggcgcaatcttcaaggtactgcgcgggcggcgccggtatcgtgacgcaggaggtcagcgacatcagcaggaacagtcccatcagcccactcaggactgcgagcaatggcttgatcgagcgcgacatgcgcgttctccttctcgattactacggttttcagttccttagccgcagtggtagcggccgaggcgttgcccgacgcctgctggtagtcctcttggacgttggcgcgagagttacggaggtgcagagtgtacgcggacaggaggattacggccagaagcagcagccctccgatcagcagttcgattttacggaagatagacataaggtccgtccttcaggcacatggcctgctcctcgtatcgtctggtcacgagaccgcgcagtaccattttgttggcgtaaatccaccgaggatactggttgcagctcccacggcggtctccggcgttgaccttgcgaagcagggtcgatgcccggagattcgactcacccacgttgaagacgaaggacaccatcgcgtcgtactctccctgcttcagaggcacgcgcacgttgcgctgtacggcccgctcagcgacgcggaggtcttcagcataccactggtcgcactgctcgtgtgtggcccgcatgccaggtcggacgcccttggtgtgccctcggcagatggtccaaggtgcgccgccagtggccgggtccgggtaggccaccagccgatagccttcgttggaagcgatctgctgcgccccgtcgagcgagaggtaggttgccccacctccagccagtgcgagggccagcaacgcggccatgacgcgcttgctgacgttcatcatcagccctccggttccggctcaggatcagtcggcaggatttcgccaccggggccggacgattccgtacgggactgggcagcggtaatggcagcctgcacccgtgccacgtcggcgttgaacagagccgccagctgggccgcagtctgcgggtgcttctcggcgtgctcgaccagagccagcagctcgcggacgagatagttgccacggccgaacaggccggtgtagttggagaaattggacttcagcatgttacctccggtaacggtcaaggatggatgggcggcctgcgcggatcggccctcgccgggtcgctgccttcatgccggttggatcgttgatccagtcttggaactccttctgcgcctgcttctcgatggccttgttctggtccagtgcgagcttgctcacccagtgccgcacgctaccttccagtgcgtcgatgcggtcatcatgcgcaaggctgccgcgttgactggtgatcttggcgatctggtggaacagggaatacaccgagcgcttgccgctgttggcgtgccgctgcgtgtactcgtgatccatttcgaccacgctctccagcaccacgagcgagccacgggcgatcacaggctccaaggtgccgatgatacgggcctccttgttgcctgtcacgaactcctcgaccagcgagccgttccacttctcccgcaggatcggaaggaacaccttggcgaaggcaccgtggcccatgttcttctcgatggagaggacgttgggcttgtatttggcggcgatttccgcgaggtggcgcaggccatccccgtcgtaaccacccggcaccgcgccaactgcgagcacgtacacggtggagttgaggaagccagtcactgcgaacgcggtctcgtctccgttggcaccgccaccggcagggtcgatctgcatgtggacaccctgaagctccgcagtctccccggagatttcgtgcggggccatcatcaggaagccgatgccactggactggaacgtgcgctggtgctgctgggacatgccacgagtgatcgtcagcgggtagcgggttccgccgcccggaatcacgatcaggttctccgtcttcagagggaagcgcatggcgtccatgagtcgggtgttcagcatgtagttcagctggaacgaggacgggcctcggtccttcagcttcgcttgcagcttggcctcgtcgtaaatctgctcgtcggtcggctgcccctcgtcgcccatcggaccaccgccaaaggcgagggacgggtctgcttcgaggcgctgtacgatagacggggccagatgcgggccatacgcctcgcgctgtgccggggtagggtagcgaccgggccagatgcgaacgtcgaagccacgacctgggagcgtgttgtagatgctctcgctggtctgcggcgtgccgaggtacaggatgcgtgccgggatgcccggacgacctgtgcagatggcggagaactccagtgtgatgttcagcagcagctcgcggttagcggcggtgcggctgttcttgttggattccacgtcgtcggcgatcagaaggtccgcgcgcttacccggcaggttgccggtgacgccgatacacgccacggatggcgagcggtcgatgcccttcaggctatgatgcacgtcgaaagcctcaaccgaagtgcggtcgcccgcattcttgtcagggcgaaggcattcgagctgcggcacggtcaggatgatgcgctggatcagcgtcgctgtctcgttggcgttggttccgcccgccgaaatcacgaggattcggtgctgcgggtcttggatcagctgccacaccgcgaagatcgcggtgatagtggtcttcgcttctccacgctgcgcctgcaccatcaggttgttcggcccgaattgcaggtagttggcgatgtcgtactgcatccacgtgggcgtgaagcccagcaccttcattatgtcgcgcatgaagacggcgaagtgggcgtagtgcttctggagcacagccagtttcttgcggcgcagctctgccgcttctgcggactcatgcgccattggctacgctccccggaaagttgacaatgttgtccagcgctgcttgcagctcggcctcctcggcctcggacacgtccttgttctccagcgtatcggccagttcgtcgagcgccttgttggcctcgcgcgtggcttggatgttgttgtccttcaggaacttgatcgcggcgttgatgtcggcggcagtgcagagttcatcattgcgtagacggtctttaaggaccgtcgccacgattacgtgcagctcacctagcgcgccttcacttgcgggatttgtcattgtggtctcccatgatctttcggtgctcgcgtgagcgccagtagaactgggcgaccgcatacagaatggcgagcgtagttacgattgcagcaccgtacgtgctgatgaagttgaggtagaccgcgccgagtgtaagcggcgaggtacggacgacctcattgaccacactcggcggggtcatgctgttctccttaaagttttgggtacaccttccactgaaggcggcggttgtttgccattcctacgttgagcagcttactggctgcaaccaacccggagagcagaacgtgctcggtcagcatgcgctctctctgcacacgacacactacctgactgctgttcttcacagcactcactagaacgtcagacagcgcctgcgattcagtctccaccacgtcgaggttgacgcagatgtctttgtagccagcgtactctaccgtgaccatgctaccgaccgaggagtcgtaccaccacaggaaggccgacgacccaccagtctggtagcccacaacggggcgcatcagctggtcgaagtcgaaggccacacgggtgacgttcggaacggagagtagtgttacagcagagccgccatccggcgtagcttggatgttggctccgtcgtagctgctcgtccacagggtgtctcgcttggcgctaaggccaacagctgaggaacccatagcgtagtccacgagcggcgcggtgaagcgccgactcgggagaacgtaggtgctcggatcaatgcctgacaccggtacagggatcatggcgtgtaccgcgaccacgcctgacgaactacgagcgaccacgtgtagttggaagtcttcgtcaggttatccgggaactcgattcggtagttcatccagccaacgtcatacgctacgccgtaccaacgcccgttcgcagcggaaggcggtgcgctgattgtgtactcgaacacaaagctcccgggaacataagtgcttgcaacaaggctagtgccgttgtaagaagacggcgcattcgcagtgcgcccaccagaccacgctgaggacgagagacgaatgtagtttcgactcgctgatccgttgttcttggacatggcgttgccgatgaagttcccgatgctggaagcacccacttggccactcgtgctgtacaaacccgaggtgtagttgtaggtgttaccgtcgaatacgaaggttccggacacgtcagttgcgtcgaggtagaccgacaaggtgtaagcgacgtacaggtactcggacgcgagcaccgtcacgctagtgggatttccttcggagtccttaatcagagtgcgagagaacagtggatagctgctaccggtacctc

SEQ ID NO: 13 - DNA, 20 bp, synthetic construct
  source 1..20: mol_type = other DNA
gcgcagtcatgagatcgaga

SEQ ID NO: 14 - DNA, 20 bp, synthetic construct
  source 1..20: mol_type = other DNA
gttgagtgcaccgagagtga

SEQ ID NO: 15 - DNA, 20 bp, synthetic construct
  source 1..20: mol_type = other DNA
tgggtcacttcggtgttacg

SEQ ID NO: 16 - DNA, 20 bp, synthetic construct
  source 1..20: mol_type = other DNA
gtggtgaaaggtgcggtttc

SEQ ID NO: 17 - DNA, 20 bp, synthetic construct
  source 1..20: mol_type = other DNA
cgtagtcgcgattgtcggta

SEQ ID NO: 18 - DNA, 20 bp, synthetic construct
  source 1..20: mol_type = other DNA
accactgctgacgttcgatt

SEQ ID NO: 19 - DNA, 20 bp, synthetic construct
  source 1..20: mol_type = other DNA
gctaccggtacgactacgtg

SEQ ID NO: 20 - DNA, 20 bp, synthetic construct
  source 1..20: mol_type = other DNA
gatctggaaacagccgtcca

SEQ ID NO: 21 - DNA, 19 bp, synthetic construct
  source 1..19: mol_type = other DNA
tttcggtggcttggatttt

SEQ ID NO: 22 - DNA, 20 bp, synthetic construct
  source 1..20: mol_type = other DNA
atttgcgagaagtacaactg

SEQ ID NO: 23 - DNA, 20 bp, synthetic construct
  source 1..20: mol_type = other DNA
atcccctttgcatcttcaat

SEQ ID NO: 24 - DNA, 20 bp, synthetic construct
  source 1..20: mol_type = other DNA
ttccgtcatctaagggaatc

SEQ ID NO: 25 - DNA, 20 bp, synthetic construct
  source 1..20: mol_type = other DNA
taagcccttcgtaaagttct

SEQ ID NO: 26 - DNA, 20 bp, synthetic construct
  source 1..20: mol_type = other DNA
aagcattgaaaaacgaaacg

SEQ ID NO: 27 - DNA, 21 bp, synthetic construct
  source 1..21: mol_type = other DNA
actaggagaagattagatggc

SEQ ID NO: 28 - DNA, 16 bp, synthetic construct
  source 1..16: mol_type = other DNA
ctggtccgtaagggtg

SEQ ID NO: 29 - DNA, 20 bp, synthetic construct
  source 1..20: mol_type = other DNA
gatatacgagcaacgtcttc

SEQ ID NO: 30 - DNA, 20 bp, synthetic construct
  source 1..20: mol_type = other DNA
atttgcgagaagtacaactg

SEQ ID NO: 31 - DNA, 20 bp, synthetic construct
  source 1..20: mol_type = other DNA
gttattgcgacggttaaaga

SEQ ID NO: 32 - DNA, 20 bp, synthetic construct
  source 1..20: mol_type = other DNA
tggattaaatactacgccga

SEQ ID NO: 33 - DNA, 20 bp, synthetic construct
  source 1..20: mol_type = other DNA
ctggcaaaacaacctcatta

SEQ ID NO: 34 - DNA, 20 bp, synthetic construct
  source 1..20: mol_type = other DNA
agttaccacgaggatttcat

SEQ ID NO: 35 - DNA, 19 bp, synthetic construct
  source 1..19: mol_type = other DNA
gtagatgttcggttcggta

SEQ ID NO: 36 - DNA, 20 bp, synthetic construct
  source 1..20: mol_type = other DNA
caagccaattcacatcgtag

SEQ ID NO: 37 - DNA, 20 bp, synthetic construct
  source 1..20: mol_type = other DNA
attctgtttcaacaaccctg

SEQ ID NO: 38 - DNA, 20 bp, synthetic construct
  source 1..20: mol_type = other DNA
cagacatccaggaacttttc

SEQ ID NO: 39 - DNA, 20 bp, synthetic construct
  source 1..20: mol_type = other DNA
catacctacgatatacggca

SEQ ID NO: 40 - DNA, 20 bp, synthetic construct
  source 1..20: mol_type = other DNA
gactactcgctctacatcaa

SEQ ID NO: 41 - DNA, 20 bp, synthetic construct
  source 1..20: mol_type = other DNA
atggcctttcttcattcttg

SEQ ID NO: 42 - DNA, 20 bp, synthetic construct
  source 1..20: mol_type = other DNA
agaaaatatccgggtgtgat

SEQ ID NO: 43 - DNA, 20 bp, synthetic construct
  source 1..20: mol_type = other DNA
tagattgtgattcacgcaac

SEQ ID NO: 44 - DNA, 20 bp, synthetic construct
  source 1..20: mol_type = other DNA
gaagacgaaaaggcaaaaac

SEQ ID NO: 45 - DNA, 20 bp, synthetic construct
  source 1..20: mol_type = other DNA
atattgaactccgaagtcgt

SEQ ID NO: 46 - DNA, 19 bp, synthetic construct
  source 1..19: mol_type = other DNA
ctaccaaactgggggatag